European Patent Application EP 4 635 975 A1 - sequence listing, part 4

SEQ ID NO: 219 - DNA, 4639646 bp, Escherichia coli (residues 2,319,824-4,639,646 of 4,639,646)
  source 1..4639646: mol_type = genomic DNA; note = MG1655 E.coli strain used
aaagcctcaggaaccgggcttggtctggcgttaagtcaacgcatcattaatgcccatcagggtgatattcgcgtcgccagtttgccgggctacggcgcaaccttcacgcttattttaccgatcaacccgcagggaaatcagactgtatgactgctattaatcgcatccttattgtggatgatgaagataatgttcgccgtatgctgagcaccgcttttgcactacaaggattcgaaacacattgtgcgaacaacggacgcacagcattacacctgtttgccgatattcaccctgatgtggtgttgatggatatccgcatgccagagatggacggcatcaaggcactaaaggagatgcgcagccatgagacccggacacccgttattctgatgacggcctatgcggaagtggaaaccgccgtcgaagcgctacgctgcggagccttcgactatgttattaaaccgtttgatctcgatgagttgaatttaatcgttcagcgcgctttacaactccagtcaatgaaaaaagagatccgtcatctgcaccaggcactgagcaccagctggcaatgggggcacattctcaccaacagcccggcgatgatggacatctgcaaagacaccgccaaaattgccctttctcaggccagcgtcttgattagcggtgaaagcggcaccgggaaagagttgattgccagagcgattcactacaattcgcggcgggcaaaggggccgttcattaaagtcaactgcgcggcgctgccggaatcgttgctcgaaagtgaactgtttggtcatgaaaaaggtgcatttactggtgcacaaaccttgcgtcagggattatttgaacgagccaacgaaggtactctgctcctcgacgaaattggcgaaatgccgctggtactacaagccaaattactacgcattctacaggaacgggaatttgaacggattggcggccatcagaccataaaagttgatatccgcatcattgctgccaccaaccgcgacttgcaggcaatggtaaaagaaggcaccttccgtgaagatctcttttatcgccttaacgttattcatttaatactgccgcctctgcgcgatcgccgggaagatatttccctgttagctaatcactttttgcaaaaattcagtagtgagaatcagcgcgatattatcgacatcgatccgatggcaatgtcactgcttaccgcctggtcatggccgggaaatattcgagagctttccaacgttattgaacgcgccgtcgtgatgaattcaggcccgatcattttttctgaggatcttccgccacagattcgtcagccagtctgtaatgctggcgaggtaaaaacagcccctgtcggtgagcgtaatttaaaagaggaaattaaacgcgtcgaaaaacgcatcattatggaagtgctggaacaacaagaaggaaaccgaacccgcactgctttaatgctgggcatcagtcgccgtgcattgatgtataaactccaggaatacggtatcgatccggcggatgtataacaccaaaacttgctatgcagaaatttgcacagtgcgcaattttctgcatagccgctcattctccttataaatccccatccaatttatcccttcatattcaattagttaaataactaaatccaataatctcattctggcactccccttgctattgcctgactgtacccacaacggtgtatgcaagagggataaaaaatgaaaacaaaattgatgacattacaagacgccaccggcttctttcgtgacggcatgaccatcatggtgggcggatttatggggattggcactccatcccgcctggttgaagcattactggaatctggtgttcgcgacctgacattgatagccaatgataccgcgtttgttgataccggcatcggtccgctcatcgtcaatggtcgagtccgcaaagtgattgcttcacatatcggcaccaacccggaaacaggtcggcgcatgatatctggtgagatggacgtcgttctggtgccgcaaggtacgctaatcgagcaaattcgctgtggtggagctggacttggtggttttctcaccccaacgggtgtcggcaccgtcgtagaggaaggcaaacagacactgacactcgacggtaaaacctggctgctcgaacgcccactgcgcgccgacctggcgctaattcgcgctcatcgttgcgacacacttggcaacctgacctatcaacttagcgcccgcaactttaaccccctgatagcccttgcggctgatatcacgctggtagagccagatgaactggtcgaaaccggcgagctgcaacctgaccatattgtcacccctggtgccgttatcgaccacatcatcgtttcacaggagagcaaataatggatgcgaaacaacgtattgcgcgccgtgtggcgcaagagcttcgtgatggtgacatcgttaacttagggatcggtttacccacaatggtcgccaattatttaccggagggtattcatatcactctgcaatcggaaaacggcttcctcggtttaggcccggtcacgacagcgcatccagatctggtgaacgctggcgggcaaccgtgcggtgttttacccggtgcagccatgtttgatagcgccatgtcatttgcgctaatccgtggcggtcatattgatgcctgcgtgctcggcggtttgcaagtagacgaagaagcaaacctcgcgaactgggtagtgcctgggaaaatggtgcccggtatgggtggcgcgatggatctggtgaccgggtcgcgcaaagtgatcatcgccatggaacattgcgccaaagatggttcagcaaaaattttgcgccgctgcaccatgccactcactgcgcaacatgcggtgcatatgctggttactgaactggctgtctttcgttttattgacggcaaaatgtggctcaccgaaattgccgacgggtgtgatttagccaccgtgcgtgccaaaacagaagctcggtttgaagtcgccgccgatctgaatacgcaacggggtgatttatgattggtcgcatatcgcgttttatgacgcgttttgtcagccggtggcttcccgatccactgatctttgccatgttgctgacattgctaacattcgtgatcgcgctttggttaacaccacaaacgccgatcagcatggtgaaaatgtggggtgacggtttctggaacttgctggcgtttggtatgcagatggcgcttatcatcgttaccggtcatgcccttgccagctctgctccggtgaaaagtttgctgcgtactgccgcctccgccgcaaagacgcccgtacagggcgtcatgctggtcactttcttcggttcagtcgcttgtgtcatcaactggggatttggtttggttgtcggcgcaatgtttgcccgtgaagtcgcccggcgagtccccggttctgattatccgttgctcattgcctgcgcctacattggttttctcacctggggtggcggcttctctggatcaatgcctctgttggctgcaacaccgggcaacccggttgagcatatcgccgggctgatcccggtgggcgatactctgttcagtggttttaacattttcatcactgtggcgttgattgtggtgatgccatttatcacccgcatgatgatgccaaaaccgtctgacgtggtgagtatcgatccaaaactactcatggaagaggctgattttcaaaagcagctaccgaaagatgccccaccatccgagcgactggaagaaagccgcattctgacgttgatcatcggcgcactcggtatcgcttaccttgcgatgtacttcagcgaacatggcttcaacatcaccatcaataccgtcaacctgatgtttatgattgcgggtctgctgctacataaaacgccaatggcttatatgcgtgctatcagcgcggcagcacgcagtactgccggtattctggtgcaattccccttctacgctgggatccaactgatgatggagcattccggtctgggcggactcattaccgaattcttcatcaatgttgcgaacaaagacaccttcccggtaatgaccttttttagttctgcactgattaacttcgccgttccgtctggcggcggtcactgggttattcagggacctttcgtgatacccgcagcccaggcgctgggcgctgatctcggtaaatcggtaatggcgatcgcctacggcgagcaatggatgaacatggcacaaccattctgggcgctgccagcactggcaatcgccggactcggtgtccgcgacatcatgggctactgcatcactgccctgctcttctccggtgtcattttcgtcattggtttaacgctgttctgacggcacccctacaaacagaaggaatataaaatgaaaaattgtgtcatcgtcagtgcggtacgtactgctatcggtagttttaacggttcactcgcttccaccagcgccatcgacctgggggcgacagtaattaaagccgccattgaacgtgcaaaaatcgattcacaacacgttgatgaagtgattatgggtaacgtgttacaagccgggctggggcaaaatccggcgcgtcaggcactgttaaaaagcgggctggcagaaacggtgtgcggattcacggtcaataaagtatgtggttcgggtcttaaaagtgtggcgcttgccgcccaggccattcaggcaggtcaggcgcagagcattgtggcggggggtatggaaaatatgagtttagccccctacttactcgatgcaaaagcacgctctggttatcgtcttggagacggacaggtttatgacgtaatcctgcgcgatggcctgatgtgcgccacccatggttatcatatggggattaccgccgaaaacgtggctaaagagtacggaattacccgtgaaatgcaggatgaactggcgctacattcacagcgtaaagcggcagccgcaattgagtccggtgcttttacagccgaaatcgtcccggtaaatgttgtcactcgaaagaaaaccttcgtcttcagtcaagacgaattcccgaaagcgaattcaacggctgaagcgttaggtgcattgcgcccggccttcgataaagcaggaacagtcaccgctgggaacgcgtctggtattaacgacggtgctgccgctctggtgattatggaagaatctgcggcgctggcagcaggccttacccccctggctcgcattaaaagttatgccagcggtggcgtgccccccgcattgatgggtatggggccagtacctgccacgcaaaaagcgttacaactggcggggctgcaactggcggatattgatctcattgaggctaatgaagcatttgctgcacagttccttgccgttgggaaaaacctgggctttgattctgagaaagtgaatgtcaacggcggggccatcgcgctcgggcatcctatcggtgccagtggtgctcgtattctggtcacactattacatgccatgcaggcacgcgataaaacgctggggctggcaacactgtgcattggcggcggtcagggaattgcgatggtgattgaacggttgaattaatcaataaaaacacccgatagcgaaagttatcgggtgttttcttgaacatcgacggcgaaggtaaccccattaatcaccagtcaaaacttttcaccagcgtcagctcgccagcattacgcatcggtacaataaatgtttcctgtttctcattgaccgatccttcatcggtgatcagcgtcagttgggcggtggttaattccgtttcgctgcgcccaccatagtagttgatatacacctgatagcgcccgtgaattggcgcgggcatggcgaaaatctcgggtccgtaccccgtcgtgacatccatatccagtgcaccactgtttttcagcacggtgttaccgtaccaggcgtgttcgccatcgggcgtaacaacgtgaaggtcgaggtcggtattgtccgtatcccacgagagaaccagccgtaaacgtgcacgaatcgttcctgtacccggcgttgagtaaaactgcattttttgtcggctttgcccatccgggctgatgacctgcacgctgttgctgccttcagtgaaaatataagggcgtgcaaatgaaccatcggattcaattctctgcggcatactggcaccgttgaccaccagccggccctgctgaactttacccgccgcagcataattctttattttgccgcggatctgcgctgagatattttgatcatctgccatgttgacggacgacgccgggtaattgatcgattgtgaaaaactggcatcttcgccctctgccggatgccagcctgagagcggtgcatcaatctcgacttcctgcacaccttcactgtgagcgacaggcgaaagcgccaccagtaacaacggaagaaaaatctttcgcatagcattagtccattaataattgtcgggtcagcgtttcgatatagttctcatcaagcccggtgggataaccatcaaaggccaggtgcagatactcatgggttaaatccagccgatcctgaagcgtaaagaagttacgaataaacagccgtttctgctgccgatcggtataggggaaacctgagactaaacggcaaaccgcaaacacgtctggttcgttgtaccccgtctcagcttgtaatatacgccgccactgcggcatttttttcgccagccaggctttcgctttgggtaataactggcaggttgagcgtggcgctccccagcggctaagactgttgtcgggataagcaaacgcgagtatctgatcgtaacgctctccctgccccgcctgggccgtggcttgccgccaggaaagtgtcccttcggtagcgcgactgccatgataatgaaccggatcgcctgcatagatgagatcctgcgtccaggcggtcatcgttcgcgcccccgtggtcgctggcgaagcagaaacacgctgcgtggcgctgctgtcggggatggtcaggcaatcgccttcccgattggcgttttgctgtaaaaaagtgcgaatcgccacggtcatggctttcgctgcctcagggggcgtacttttcgcctcgcgatccagaactctggcaacgtactcttcacgatcgagatgcgactgcaatttcagtttgcccttttcgctcagtaaggtcgtctcaccgtggctgacaaacgtaatgtggttaccattagtaaacgtcacacgatagcgcccattaagtacgccgggatttactgccgtcgtactcttttccgctgtgattttcttcagcggatagcgggcaaacagctccacctctacacattgcccactggcaacctgcgtcggcactggcaaaacccgattaagcaccgtcgcataacgggttagtaccgttttgctggtgccactgccagtaacccacagcggtgtaccatcggttaaccagccagcaaaaccaccctgacggatttcctgtttatcatcggcaaaccagctccaggttttcacccgtacccgactaccgagcatggatgcgacaccgattttcgcctcgtccagcaccacatccagtaagacttcctgagctttgttttgcgcgggtaacgtcgctaatgaatcaagcagcgatttaaccgttaccgaggtttctggcttcagcgtagtcagagacgctaaccacgcaggtgcctgacgctgttgccagtattgcccccacacatctgcgccaatatgcaaccgctgcggcgcaaaatagagcccacaggaacgtaccagcgcggtatcgcgcgttatgctctccccagcctgacaacaataaacctcttccggggagtttccgcgacactggtagggctgctccggttgatgggtatcctccagccaggcgtaaacatacagtttccacaaactccctaacggcgtggtgagcgagtcaggtaatgctgagactttggtcacgcctgatgacgacagctgatacagttgatcgtgctgcgcaccgcgcagcaccagttgtaacggcgtctcctccgcaagtgttggcagagtaaccaacgccaatagccagacgattctgcgccagttcacttatttcacctgcatcccggtccattcactccctgccgcaacactttgctgcgcaggtgcataggaacgcacataacgagcaggaggcagaacgaattgccctttttgcgagaagcgcagcaaatggcggaaagtgaccgttcccgtcagttctttcaccggcaccatataggccagttcgcccatttcatttcgcgctttttccagcaattgcccctgctgtttcgcggcgttgggtttattgaccgaaatgccccatgttgtgcgctcaacgtcggctcccggtggcagcggtacttccacctgaccgtagcgcagaactgcatcctgctcgctggtaagcgtgatttcatcgagatacagcgcatcgctgtcaatctcattgctggtcaccggttgcagaataaagctcatctcttcttcaccagggataagccgatacaactggcgttcaacggtcaccggaatgttactttgttgagccatttttgccggctcacgtcagcggacctgcacattttgcggcgataattcgtcaccaaaagagagaatgtccggcacgccctgaccaacccaacgccagtcttcgccccctccagttaacttatgtttagcccatgcgcccgcaggcgcaggcaaaacaactggaggcattgtcgccatatatttcgccagccagttcatggccagcgcgcgctcaatagtggattgctcagcggtcaaaccacttaaaatagcggccgtctgggtagcgtcgccaccgctattaagcagcacaaccgtgtgcgccagcggctgattgctgtttgccgctttatcccacgcatattgctgaacctgtggcatcaccgtggacttcaactgcgcttttttcagcaacgtcatggttaagacgtttgccaccgcatctgccagtggagactccggtgtatcgaggatcaggctatcattgatatcgcgggtgtcttcctcagagaaatcttcagttttagttccgcgccgggcgatagcttcatccaaccctttcaacaacgttttgcacggcaaattcatctcctgcgcccatgccagcaccagcgcccgatgcaataacggcatgttatctgcctgctccgcgtagctgtcgagcatatgctgccagtattccggttgttgcgttacgccgatcgcctggctggcctgccagtcggcgtaccatgcccatgccgtaaggaaggcgtcaccattgccatcttcaccccaccaggtaaagcgcgctccgggccccgccagttgcatcagccgcagacggttatcctgaatcatctgacgaatgtcgttagcggcggcactttgatgatcggcaagcgaacgccaggcgagactgagcgggatcagacggctaccggtgttgattacgccaccccacggttcatcgactaacgcatcaagattgttgcggaaaatctcctgcggcgtttcactactttgtagccggatattgctcgcctgctcgggcaacatcagcgcgttatcgccaccaccgagcatgacatttttctgctgttcaacgggccagctgttatccacaaaagacagttttgtgctaatgctgtcctgcacttgcccattttgttgcagttctgcacttaacaagccagattgctgaatattctgcgtcagcgaaatataattcgcccctttgtgcagcgtcagcgtctggcgcatctcagcgcctgcaaatttagtcaccagcgccaccggttcgttatcctgctgactgaagataaacagtcctgccgccggtttgtcgcccacgcgatacaccgttggcatactccacttcatgtagagatttttttccgaacgcagataagcacgcccctgcccgaccagcccgtcgccgttcatcccacgcgcggtgatacgccagcgggttaacgaatcaggcatcaggaacgtgaaatacgctttgccttgtttatcggttgtgagtgacggcatccatgccgcggtatccacctcttcacgccgtggacgttcaagcatttttactcgccgctcgctgcggttagttgcgccaggcgcaaccggctcgctggagagcgcctggtcgtagctgataaacgacagactggagctggtacgcacattgttacgccccagcggatagaaaaatttgccgatattcggcgcgatttctggttgcagcgcgtagatcatttcatcgaccacgcctaccgttagctgcgcagaaacaggtttacctttcagcgacgaggttaattcgacattgaccagttcaccaggctggtaatgggttttgtccgttttcacccggatatccagctggggaacggcaactttgatcccggcgttctgaaaactgtactgaccgttacgggtatacagcaccgaaaaagtgatgttaggcgcaaaggaattgctcactggaacccgggcttcatactgggtatcgtttaaacgttgtagcgttagccagtttgccggatgcgaaagcagcgactgctgttccacgcgatcgcgttccagcgtcaataatgcttcatcaattggctccggaaaggtaatcagcatcttcgcggtttcgcctggctggtacagcgttttatccgccacgatatctaccgtaccagtatgcgccgtgctgcccttaccgctgacggcatgacttaacccagcgagaattaagccgtctttatcgcgtaatgtcagattgtagttgccaggtttagcgaaattgacggtaaaggatttgccgcctgacggtagctctccgctatggctcgtgcggtcttcgagacgcaaccattcatacgtaacaggaacctgttttgaagattccagcgcggcataacggaacacaaccgactcgccgctattactgtattgtgcggcagtacttaatgagtaatgcgccagaccgcgttcaatgaggatctctttggtggtggtgacgcgatacgccgcgccgtcactggcggagacggttaacaaatagcggctcggtttatcggcggcggggagatttaacgccacatgaccgctggcgtcggacaccgtttcgctgccttccagcgacacggggaaacgtccggcataacgcaaatcgttaccgaccattgataattgctgagcgcgcaaacttaactgcacgcgggcattttttaccggctcgccatccgggtagagcagttgcagtttgccgctgaccgcttcgccagttttgaactcttttttggcgagagctaaaccaatctcgaaatgtggcttgatgtagtttgccacgcgaaaactgctgctatagacctgattgcggtaagcaagacgtaactcataacctccggctacggcattttctggcaggcggaaacttccctgcccgccattgcgcgcatccagcgtgacattgacggtttgcaacagactgccgttggcgtccagcaccgaaagcttcgccggggcgctgacgatgggggatgaatgcaacggatcgtggaactcgcggccgatcactttaacatcgacacgatcgcctgcgcgatatagcgggcgatcggtaaaaatatacaagcgggtgttgtagatttcgctttcgtagaagaagttctcggagacaaaaacgccgccttcagcatccttacccagaatgtatgaacgttctggcgatatatgttgtaactgcaaggtaccgctgtcatcggtcacaccgcgggtcatcacgccaagaccgtcagtccacaagatctctgagccgggcttcgcttcaccctgttttttacccgcggtccacaccagaagctctttgcctgacactttgctaagcgccacggtatcggaaacaaacaccaccgtcgtcgcccgatacccaccaaccatcgcctcgacgaggtacagtcccggctcttgttggccgagaggaatataaatgttacccggctgcggcgagatgaaattgctggatgcgccttccagttttaccccttgctgcggctcgaacggtttagcctgccatagtggataacggaactgtttcaccaggggatattttttcagcggggaaaactggttgttctgtacataacgggaaggtttaataatggcattgccgagctgtaattcgggtaacgcctgagtcacattctgccgtgactgagaagagaaagtacgctgcatcacgcggcgagatttgccgtaccagttatcccacagccaggttagcgtattgttcagcccgtcgcccagatattgcggttgcaccacaatgcgatgcaggtttttctgctggcgcaaaaatgccatcgggtcaggaatacgatacaggcgaacgtccacgccgccgtactcttccatctgatagcgccgataatcacgccccggcgcttccagtcgcactttcgcctcttcactgctgctaaaactgctgtcagcaagcaaaaagaatgttcccccggcaggcggcgcatagttgctggaaggaagcgaatcatcagcattagcaagccctgttcccacaagagacagggacaagcacgctgctatcgcgccagaaaatttaaacgataaatgccaatgaaattgggattggaatcgttgggtatccatcgggtgtccttccatgtcataagttgttgcagactgactgcgcgcattccgttgtcagttttcgtggcgcttccggtgtggtagatgacgtaacgccccatccagaccattaagtgctgggcatcgccctgatcgaaaaaaatcatatcgccaggcagcgcctggtttatgtcctggccaataaactggctgttgtactgaatcaaattaatcgcggtcacataggggccggttttcccgttcccctgattccagttttgcgccagttgacgctgttcaggtgttagcgtcatctctggcggcaaatactggctagataaaccgttactttttagccatttactgtcgtgaactttcagcgtctcgttcgccgcaaatcgcaccaggcccgcacaatcctgctgataccagcgtggacttggcccctggcggagctgttcttgtgcaatgcgtacaaaccaggcgcgaaacagcccggattgttcgacattcagcatttcgctatgggcaacaacacaacacagccagcaaatcagcgccagcagcccgtgcctcatagcggctgccaggttatgggtagccactgccaggcggcaccgggttccatctgggccagcttcatgacataacgcggttgttgagataaagcgtccagcttcggcattaataaagtttgtgcggcgttataaaaaaccggttcgagattcttcggcagactggtcaacgtttcgttacgcagcagtttcgctattccttgtggattgatatagagcggaacgatgccatcagtgggtattacatccaccattgccgggcgggttttattcagtgtttgcagcgcgttattaaccagcgtgtcatcgagggagaaaagcagcgttttgttttgcatcgccagcgacacacggaaaaaataatccgacattaattgatcgggttgcgccgcctgcgctttcggatactggccgtatcgggaactcacttcgcgacgccagatttgcgcttcgccctgctgagtctggcttaccggcaaaacaccttctggcgctttgctttcgtgcgcaccaatattttgcgtaaacagtttccctggcaattgcgcctgttcggcagtgccatcaaactgaccgacaaacagcggggtttgcaattttgagtcttcataccagcacagccccgcggcaccgtctaacgccccattcagcttgtcgttttcctggctgatgtgcgaaagcatctcttcggcaataccgtgtgaatacggcaccgccacacagaagctggctccggcaggcatactgttccataccggcgtaaaatcgaaactggcatctacgctggcggattcatcatttaacgccacaaaactgtgccagccgtcgttacccatttcgaagcgtacgccagcaaaagaaggcattaaccgctggtagccaaaccccagccacctggcgctgactacgatgcgctggcgtactggcgttttttcggcagtacgctcttccaggccaaagcttgcttgccagcgttttttgccgctcaacaaatcacctgcgatcgccgtggcttcggtatcctgctgatcatctttaaacaacatatccgtgctggaaaacaccagcatcttgtcctgataagtcgcgaacatcagggcgttattgccgttatagcgcaactgataaacaggaacagtttcactatttatcttgatgctactgatttccgttttgcttaactggctgtcgctggtagcggcaaacaacaatggctccagcagtttgcttaaaccactgcgctggatcagcaccatataatgtgaaagatggccttgtttatcgtgccacagcgctgcctgcgcgggctgatctaagagtgacgaaaagagcttatctttcagcgtgagatcgtgttcatagacaatacgacgaatgctgccttcaatgcccagacgatcggcatgattctgataatagaaaacgaaatcttcgctcagaacatcgtggagaaacggaatggtgaggagatctttgggaagctggctcagagagtcgctgtcgagaaagaggtccggctcattgagatcgatttgcagattgttgtgcaccaccagcggcgacaacgttttttctggcccactgccagcatattgcaacgcccagacgccagcggaaagcagtgctattgcgccaaaacctacaagaccatagaaccgccagcctttcgcctttttttcaccactcattgccacattccttgtgtatagccagccattttttacgggcacagccaaactttaccgtgccctaatacgacaaaagcccagactttgcagcctggacttttcaattcaaacaagggagatagctcccttttggcatgaagaagtaaaattattcttcttctggctcgtcgtcaacgtccacttccggagcgatttcatcgtccccttccgcggcactgccgtcgatggtatccagatcttcctcgtcaaccggttcagcaacacgttgcagacccactacgttttcatcttccgcagtacggatgaggatcacgccctgggtgttacggcccacgatgctgatttccgaaacgcgagtacgtaccagcgtaccggcatcggtgatcatcatgatctggtcgcagtcatctacctgtaccgcgccaacaactaaaccgttacgttcggtaaccttgatggagataacccctttcgtcgcacgcgacttggttgggtattccgccactgcggtacgtttaccgtaaccgttttgcgttgcggtgaggattgcgccatcgccacgaggcacgatcagagagacgactttatcgccttcacctaagcgaataccgcgaacaccggtggtgttgcagcccatcgcacggacagaagactctttaaagcgcaccactttaccttcagcggagaacagcattacttcgtcttcgccgctggtcaggtcaacgccgatcagctcatcgccgtcaaccagtttgatcgccactttaccggcggtacgcagacggttgaactcggtgaggacagttttcttcacggtaccgttagcggtcgccatgaagactttcacgccttcttcaaactcggtcactggcaggatcgcagtgatacgttcgtcctgctccagcggcagcaggttgacgatcggacgaccgcgcgcgccacgagtggcttccggcaactgataaactttcatcgaatagacgcgaccacggctggagaagcacagaatatggtcgtgagtgttcgccaccagcagtcggtcgataaagtcttcttctttaatacgtgcggcagatttacctttcccgccacgacgctgcgcttcgtattcagaaagcggctgatacttaacgtagccctggtgagagagcgtcacgaccacatcttcctgggtgatcagatcttccaggttgatgtctgcgctgttggcggtgatttcagtacgacgtttgtcaccgaactgttcacgaaccagctccagctcttcacggatcacttccatcagacgatcggcgctaccaagaatacgcaacagttccgcgatctgatccagcagctctttgtattcgtcgagcagtttttcgtgctcaagaccggtcagtttctgcaaacgcagatccagaatcgcctgagcttgctgttcggtcaggtagtacagaccatcacgcacgccgaactctggctccagccattccggacgcgcagcatcgtcgccagcacgttcgagcatcgcggcaacgttgcccagctgccacggattagcaaccagcgcagttttcgcttctgcaggcgtcggcgcatgacggatcagttcgatgatcgggtcgatgttcgccagcgccacggctaatgcttcaaggatatgagcacgatcgcgagctttacgcagttcgaaaatagtacgacgggtcaccacttcacggcggtgacgaacaaacgccgcgatgatgtctttcaggttcatgatcttcggctgaccatggtgcaatgccaccatgttgataccgaaagaaacctgcaactgggtctgggagtagaggttgttgagcacaacttcaccgaccgcatcgcgtttcacttcaatcacgatgcgcataccgtctttgtcagactcgtcacgcagcgcgctgatgccttccacgcgtttttcttttaccagttccgcaatcttctcgatcaggcgcgctttgtttacctgatacggaatttcgtggacgataatggtttcacgaccggttttggcgtcaacttccacttctgcgcgagcgcggatatacaccttgccgcgaccggtacggtaagcttcttcaataccgcgacgaccgttaatgattgccgccgtcgggaagtccggccccgggatgtgttccatcagcccttcaatgctgatgtcttcatcatcaatatacgccagacaaccgttgatgacttccgtcaggttgtgcggcgggatgttggttgccatacctacggcgataccggaagaaccgttcaccagcaggttaggaattttggttggcatgacgtccggaattttttccgtgccgtcatagttatcaacgaaatcgaccgtctctttttcgagatcggccatcagttcatgggcaattttcgccagacggatttccgtataacgcattgccgccgcagagtcgccgtcgatagaaccgaagttaccctgaccgtctaccagcatataacgcagcgagaatggctgcgccatgcggacgatcgtgtcatagaccgccgagtcaccatggggatggtatttaccgattacgtcaccaacgacacgggcagattttttataggctttgttccagtcattgcctagtacgttcatggcgtaaagtacgcgacggtgtaccggcttcaggccatctcggacatctggcagcgcacggccaacaatgaccgacatcgcataatccagataggagctcttcagctcttcctcaatgttgaccggtgtaatttctctcgcaaggtcgctcatctaaccgctatccctctactgtatcccggattcaaaggtcgcaaattataacacagccgcgcagtttgaggtaaacctatacgctttattcacatccaatgcctgatatactcgtttgtcttgccaattacggagtagaagtgccaatgaatgccgaaaaatcgccggtaaaccataacgtagaccacgaagagatcgctaaatttgaagccgtcgcctcccgctggtgggatctggaaggtgagttcaaaccgctgcaccgcattaacccgctgcgtctgggctatattgccgagcgtgctggcggtttatttggcaaaaaggtgctcgatgtcggttgtggcggcggcattctggccgagagtatggcgcgcgaaggcgcgacggtgaccggtctggatatgggctttgagccattgcaggtggcaaaactgcacgcactggaaagcggcattcaggtggattacgtgcaggaaaccgtggaagagcacgcggcaaaacatgccgggcagtatgatgtggtgacctgcatggagatgctggagcacgtccccgatccgcagtcagtggtcagagcctgtgcgcaactggtgaaaccaggcggcgatgtctttttctcgacacttaaccgcaacggcaagtcatggctgatggcggtggttggtgcggaatatattttgcgcatggtgcccaaaggcacgcatgatgtgaagaagtttattaaaccggcagaattgctgggctgggtggatcagaccagtttaaaagagcggcatatcactgggctgcattacaacccgatcactaatacttttaaactcggccccggcgtggatgtgaactatatgctgcacacgcagaataagtgaggttgatgtttggccgcgccaatgcctgatgcgacgcttgccgcgtcttatcaggcctacaaatgctccccgtaggccggataaggcgtttacgccgcatccggcaaccgtgccgactagacagtgattaccatttcaccgtcatcgacaaaaaccctgccgtctgggcaaaatcatcactccctttctgccacgccacgctgccgcgcagggacactcgctgactgatattgcccgtgactcccacttttatttcaccccgttgcttcaccgcatcgtcactgatagtgctgccatcctcttcaatttccgtcgaatggggatcgtgataataattcagatctaatgttggtatgacatgaacagcggtacgccattcgctgtgtaaacccagccgcgtctgaatatcatcaccctgcgattgtgacacgcgcgcacggttagcggcggtaaaatcatcctgctgcacgccctgataaatcacctgcgcctgcggttcaatcaccacaccacgccccggtaaccactgataccccgcctccagcgaggcgataatccccgacgagtggtaatgatctgtgccatcttcttgttcggaaacatcattgctaaaccacgcgtattgcagccagctatccagccaggccccttgcttctgattaccgtgctgaaaccagcttgatgtcagcccaacggcataaccgtggttctggttatcggcgcgagttccggtcatattcgagcggctgtcgccctggttatcgctgtagccaccaacaatcccaagcatccactcgccatccgtgccccagcgcccgctaaacagatcgccgctaagttgcaccgtagaagtgtcttcatgttgagccagttgccccgctgctgtgtaatgataatctccgccgataacacgtaaattcagcgtctgaccatcgccacctgcgtgatcgcgtcgctccatcataaacgcctgatttgccgcccgcaggttattaagataaccgccaactttggcattcaacaccggctggtaagcaggcgtaggttccgggtcgggtgttggatcaggatccggcgtgggatcaggatcgggagtcgggtctggatcaggtggcgatggcggcgttacttcttgcgatcgcagataccagtcgttgttatcttccaccagcgtgtagtcatacgctcccatattgacgtagccgctgcctgccagactgaactgcgcattgttttgaaactgcgtgggatcagctgcgaaatcaaccactttaatgcctgtcgatgtcggctcaccaatccctgtaatggagttaaccaccacagttgtgttgccagcagtattaccgttcatcaccaattgatcgcttaccgagtcatcgccgtttaattcgctatcgagcagtagcgtaccgccgccggtataatcaccgtttaccgtcagcgtatcgccagcgacgccattttgcaggctaaccgcaccggacgtattggtcagattgccattaaccgtcacgttggaaagataagtcaggctgtcagtttcaaggttggtattaagctcacctgtcaacgtcacaccatcggtggcattcaccagcgtcccatcgccgttaaatagtgaggcattaagggcgacggaagtatcctgcccggtcaggcgcaaaaccgtaccatcgctgatgtcgatagtgccgctggaaatagcatcaattgactgaatatcctgatccgcgccagtaacgaacgttgccccatcaccaacccacagtgacgaagcataaggaaggatatcagcaacatcacctttcagggtgccttcttcgacacgtaccgccgactgcgttgtaccgctggcggtcagctccagtgtaccagcccccgttttagtcaatgtgctaccctcatcctgatgctgcccgctgctgtcagccatcagtgcgccccactgcgtgtctacccccgcatcaactgccacttcaccgtcggcgcgcatttcaatatcacgtccgtggcctgccgcatctgaacgcgtgtcaacgtcggaggtaatctccatcacgctttcttgttgcttatcggtaaagataacctggcggttatagtgggtatctccaagctgcgagttgtcgctcaccatcagcgtaccggaggcgatttgtgttgtgcccaaataactattattgtttgccagacttacctgcccgtcgctcgcatcgaccaccacgtagacgccatctttcccgtcgccgccgatatgcaaattgtcgccacctgcaagatctaccacatcctgactgccgataaccgttccgctgctgccactgacttcaaggccatcgttgtatgatgtgccgctctgccaggtggagaaatcagagagatcgagcacaccgccgtttaacacgatcgactgcggatcgtcctggagagcggtaagatctgccgcgtcgccttccagcgaaagcaccgcaccatcatcaacgactatatcgccggttagcgccatcgactgcgcccctgccagcacgtagctgccgttttgcgcaatggtgagctgaccagcaccttcgatgatgccagcaaaactgccctgattaacagtaacgttgccaccagcatcgatatttaaagtgccattctgaaagcccgtcaatgcgtgcacaaaagtttgttgggtcgagccaacgtttagctcagcctgattctgatactgatcaatactccctatcgtcagaccgtagcagtcttgcggatcgtcctggcaatgcgtatcgccgacattcatcagggagttgctgcggcccagggtaacttcaccgttttcaatctgcatctcaccagtaaagtcattgttatctgcattaagtaccagatcgccggaacctgttttggtgattaacccggtaccagcaatagagtcaacagctccgtcattctctgtattgccaataaccagcgtttttccgtcggcaatatcaaaggtaacttcacttaagccgagatacataaagccacccgccgcagaggaaggaccatctccatagcctgctgcgctattgttctcatcgactaacacgcctccgttctggctgtagctgtcatcaacagaaatatcaataagatagggagccgtcacgctattggtatatatcgccccgccataaccttcggcagtgttatttgtaaaggcagtgttatttactatcgtataacctgaaggatgcttgctgtcgctattattatcggtaacatcgattgccccgccatcgccatcactgtaacttgttgatgtatatgcctggttgttatcaaaaataacatcacttaaataaacgtcattattaatggtataaattgcgccacctttgccatcattagcgatgttattgcgaaacatggcgttagtgacacgtaaatcgacggcaccagtatcgttagtaccagaagaatagattgcgccaccatagccgcctgcgacgttaccggaaaaaataacatcagtaagattcagcgttgagttttctttagcaaatatggccccgccgttattatattctcctgtaacggtgttattggcaaacagagtcattccagtttcattttctggtaatagtgaaaattccgctccttgttgcaaaaatacggccccaccgctggcgttattggtcatatccgaaaaaaccagccattgcccatcagcgatactccagtcctgcgtaatgcctgaaaggctttgcctgctggcctgacaactcgctttgacatcatatccctggcatgaatcagtgaccgccgcgacaccgttagcagagaaaagagatgcaatcattgacgggagtaaagataaatactccttgcgtagaaagataatccgcatattaatctaaccatcattttctataagacggcgtatttaatcgcattatacgatatggaatatctttcttttgtaaattgttcaacccggtgcaatggctattttgttattatttgatgaataatatcagtgcgtcataattcaagttaataaccttcagggatatcagttatatttaaactaaattaaagtcatgaataattttcttataatataaggtaaattaacaaaatggcttagcatttaacaataaccgaatagaaaacaaccatttcgccatcaacaatctcttacattcgcttatatattgaccacaactgatacatcagattatgtgatgactcgtgcttagatcaatttttgcaatcattagcaaaaagattaataagccatctatatcaatttatctaacctattatgccgttcaagaaatcgccgaacagttatttttaacaaatttttctcttcccattgactttcccggacaccttgtctgacctaaggtgcgcgaaagccactttttccttcctgagttatccacaaagttatgcacttgcaagagggtcattttcacactatcttgcagtgaatcccaaacataccccctatatatagtgttctaagcagcttcccgtactacaggtagtctgcatgaaactattgcggaaagaattccaaaaacaggtacgacatacatgaatcagaatctgctggtgacaaagcgcgacggtagcacagagcgcatcaatctcgacaaaatccatcgcgttctggattgggcggcagaaggactgcataacgtttcgatttcccaggtcgagctgcgctcccacattcagttttatgacggtatcaagacctctgacatccacgaaaccattatcaaggctgccgcagacctgatctcccgtgatgcgccggattatcagtatctcgccgcgcgcctggcgatcttccacctgcgtaaaaaagcctacggccagtttgagccgcctgcgctgtacgaccacgtggtgaaaatggtcgagatgggcaaatacgataatcatctgctggaagactacacggaagaagagttcaagcagatggacacctttatcgatcacgaccgtgatatgaccttctcttatgctgccgttaagcagctggaaggcaaatatctggtacagaaccgcgtgaccggcgaaatctatgagagcgcccagttcctttatattctagttgccgcgtgcttgttctcgaactacccgcgtgaaacgcgcctgcaatatgtgaagcgtttttacgacgcggtttccacatttaaaatttcgctgccgacgccaatcatgtccggcgtgcgtaccccgactcgtcagttcagctcctgcgtactgatcgagtgcggtgacagcctggattccatcaacgccacctccagcgcgattgttaaatacgtttcccagcgtgccgggatcggcatcaacgccgggcgtattcgtgcgctgggtagcccgattcgcggtggtgaagcgttccataccggctgcattccgttctacaaacatttccagacagcggtgaaatcctgctctcagggcggtgtgcgcggcggtgcggcaacgctgttctacccgatgtggcatctggaagtggaaagcctgctggtgttgaaaaacaaccgtggtgtggaaggcaaccgcgtgcgtcatatggactacggggtacaaatcaacaaactgatgtatacccgtctgctgaaaggtgaagatatcaccctgttcagcccgtccgacgtaccggggctgtacgacgcgttcttcgccgatcaggaagagtttgaacgtctgtataccaaatatgagaaagacgacagcatccgcaagcagcgtgtgaaagccgttgagctgttctcgctgatgatgcaggaacgtgcgtctaccggtcgtatctatattcagaacgttgaccactgcaatacccatagcccgtttgatccggccatcgcgccagtgcgtcagtctaacctgtgcctggagatagccctgccgaccaaaccgctgaacgacgtcaacgacgagaacggtgaaatcgcgctgtgtacgctgtctgctttcaacctgggcgcaattaataacctggatgaactggaagagctggcaattctggcggttcgtgcacttgacgcgctgctggattatcaggattacccgatcccggccgccaaacgtggagcgatgggtcgtcgtacgctgggtattggtgtgatcaacttcgcttactacctggcgaagcacggtaaacgctactccgacggcagcgccaacaacctgacgcataaaaccttcgaagccattcagtattacctgctgaaagcctctaatgagctggcgaaagagcaaggcgcgtgcccgtggtttaacgaaaccacttacgcgaaagggatcctgccgatcgatacctataagaaagatctggataccatcgctaatgagccgctgcattacgactgggaagctctgcgtgagtcaatcaaaacgcacggtctgcgtaactccacgctttctgctctgatgccgtccgagacttcttcgcagatctctaacgccactaacggtattgaaccgccgcgcggttacgtcagcatcaaagcgtcgaaagacggtattttgcgccaggtggtgccggactacgagcacctgcacgacgcctatgagctgctgtgggaaatgccgggtaacgatggttatctgcaactggtgggtatcatgcagaaatttatcgatcagtcgatctctgccaacaccaactacgatccgtcacgcttcccgtcaggaaaagtgccgatgcagcagttgctgaaagacctgctcaccgcctacaaattcggggtcaaaacactgtattatcagaacacccgtgacggcgctgaagacgcacaagacgatctggtgccgtcaatccaggacgatggctgcgaaagcggcgcatgtaagatctgatattgagatgccggatgcggcgtaaacgccttatccggcctacggctcggtttgtaggcctgataagacgcgccagcgtcgcatcaggctccgggtgccggatgcagcgtgaacgccttatccggcctacggctcggatttgtaggcctgataagacgcgccagcgtcgcatcaggcacaggatgcggcgtaaaatgccttatccggcattaaactcccaacaggacacactcatggcatataccaccttttcacagacgaaaaatgatcagctcaaagaaccgatgttctttggtcagccggtcaacgtggctcgctacgatcagcaaaaatatgacatcttcgaaaagctgatcgaaaagcagctctctttcttctggcgtccggaagaagttgacgtctcccgcgaccgtatagattaccaggcgctgccggagcacgaaaaacacatctttatcagcaacctgaaatatcagacgctgctggattccattcagggtcgtagcccgaacgtggcgctattgccgcttatttctattccggaactggaaacctgggtcgaaacctgggcgttctcagaaacgattcattcccgttcctatactcatatcattcgtaatatcgttaacgatccgtctgttgtgtttgacgatatcgtcaccaacgagcagatccagaaacgtgcggaagggatctccagctattacgatgagctgatcgaaatgaccagctactggcatctgctgggcgaaggtacccacaccgttaacggtaaaactgtgaccgttagcctgcgcgagctgaagaaaaaactgtatctctgcctgatgagcgttaacgcgctggaagcgattcgtttctacgtcagctttgcttgttccttcgcatttgcagaacgcgaattgatggaaggcaacgccaaaattattcgcctgattgcccgcgacgaagccctgcacctgaccggcacccagcatatgctgaatctgctgcgcagcggcgcggacgatcctgagatggcggaaattgccgaagagtgtaagcaggagtgctatgacctgtttgttcaggcagctcaacaggagaaagactgggcggattatctgttccgcgacggttcgatgattggtctgaataaagacattctctgccagtacgttgaatacatcaccaatatccgtatgcaggcagtcggtttggatctgccgttccagacgcgctccaacccgatcccgtggatcaacacttggctggtgtctgataacgtgcaggttgctccgcaggaagtggaagtcagttcttatctggtcgggcagattgactcggaagtggacaccgacgatttgagtaacttccagctctgatggcccgcgttaccctgcgcatcactggcacacaactgctgtgccaggatgaacacccttcccttctggcggcgctggaatcccacaatgtggcggttgagtaccagtgtcgcgaaggttactgcggctcctgtcgcacacgcctggttgcaggtcaagttgactggattgccgaaccgttagcctttattcagccgggggaaattttgccctgttgttgccgggcaaaaggcgatattgaaatcgagatgtgaattggttgtagtgccagatacaacgcttatgcgtcttatctggcctacaacgattacatggcgtagtaatacgctttcacctgctcccagtccgctttggggattggctccagatatttttccagctggcggaagtcatgattaatcgctttatcgcgacgcaagcggcgacgacttttctccaggtcaagaaaaccagcttctgcattaccttctgttttcacatagatatggcgaacataacaacagccatgctgacgattaatgctatgcattttcttaaacgccagcgccactgctttcaacatggcttgccgtacttcgtcagaataaggcgatactgcatgctgggcataccagtcagcaatgctgatgaaccccgccatatcttcagtcaccagcaacgctcgccattcaccctcaattttcaccgcttcaccaaaaacgatcttcggcacgatgacaccggcccgttccagttctttaattaccgcaacctcacggacaatcgttggtcggccgaacggataacgtacggaatgaaacagatgatgcgtcatgcgctttacatacagctttttgccgttgcgctcgacgcattgcaccccgctcataccattacggcgatagttaggctcttcaacccagtcgccctctgttgcccaccagtgattaaattcgtcgtactttgctgaaactgccataccctatcgcctgtcatttttattaacgacaatgactataggtggttacctgaggaaaatcttaatgaaacgtgtcgtattaatgaatttcttttgccactactagcttgacaccgcttttacccttcatttgcagcgcatagattccaccagccactaccactaatagtgcgcccagcagataaaatgtgaatttaatcaggcggatacagcgatgaattttattcgacagggattaggcatcgccttacaaccagagttaacgctgaaaagcattgcaggtgaattgtgttccgttcctctcgaaccaactttctatcgacagatttcgttgctggctaaagaaaagccggtagaaggcagtccactgtttttactacaaatgtgcatggaacaattagtggcgattggaaaaatttgatatgagacaggatggcgcatgaacgccatcctgcagtaacattactctttattaagaaattttactgccttatcagggaaatcagtaaacagcccatttacacccgctttgttatacagagcatcatataactgattcacatcaggagtgtattcaggcagtttatctgaccgcacggtataaggatgcactaccagtttattctgctgagcatcttgcaccatgccagtgagtttgatattacccggctgcgatgtctcctcaatcaacatatggtaatccggaccaataccatctgcatattccgccacctgtttcatggcacccggcttaaacatccagtcgtagttgtaattaacccagcttccatccggctgtttctgctgcgtttcattccagtcggtataggcaatcagctgtaccagattgagctccatgcccattttgggttccagctcattcttaatacgcttcagctcatcagcatcaaaacattgcaaataaactttatcgtctttaccggtgtaaccatatttcttcagcacttccagcgtttttgccgcaatatccttcccttcctgatgatggaaccacggcgctttgatttctggataaataccgatatttttcccggtagagtgatttaacccctgaacaaattcaatctcttcttcaaaggtgtgcacccggaagtcggacttacccattgggaaacgccccggataagtctgcacttttttaccgttttcaatatcgaaaccttcggtaaatttcaacgacttaatttcatccagcgtgaaatctatcgcgtagtaacgaccgtctttgcgcgcccgatccgggaaacgatcggcaacatcagtaacacgatcgaggtaatggtcatgcagaacaaccagattgtcgtctttggtcatcaccaaatcctgttccagataatccgctccctgcgcatacgccatcgcttttgctggcagcgtatgctccggcaaatatccactggcaccgcgatgggcgatgactattttttcgttgctgtccgccgccattgcactgcttcccatgactatagtgctcatcatgatcgccatgctaaggtttttcagcgtcaatttcatgccattagcctccgttgcgttcttgcagtaattgttcatggcgacgtttttcgccaatcatcacaacaatcaacaagataaccgccagaatgctgccgccaatcattaccataaagccgccatcccagccgaagaagtccacggtgtagccaacaatcgcgctcgccgccaccgaaccgcccaggtaaccaaacagcccggtaaagcccgctgccgtacctgccgcttttttcggtgccagttccagcgcatgcagaccgatcagcatcacaggaccgtagatcaggaagccgataacaatcatacaaatcatatcgacggttgggttacctgccgggttcatccagtaaacgatagtcgcgatggtcaccagtgtcataaagaaaacgccggttgccccacggttgccacggaagactttatccgacatccagccgcacagcagagtgcccggaatacctgcatattcataaaggaagtaggcccaggaggatttatctagcgcgaaatgcttaacctctttcagataagtcggtgaccagtcgaggatgccgtaacgcagcagataaacgaacacgttggcgatggcgatataccacagcagtttgttcggcagtacgtactgcatgaagatttgcttcgccgtcagctcctgttccgctttttcgttatagtcgtccggataatcatttttgtactcttcgatcggcggcaagccacaggattgcggggtatcgcgcatcatcgcaaaggcgaataatgccaccagaatggcgcagaaagcaggcatatagagcgccgcatgccagtcattgaaccaggccatccccagcaggaacagcagcggcggaataccaccaccgacgttgtgcgcacagttccacactgacacaatgccgccacgttctttctgcgaccaccagtgcaccatagtacgaccacacggcggccaccccatcccctggaaccaaccgcagaggaacaacagtacaaacatcaccgcaatgctcgacgtcgcccatggcacaaagcccataaacaacatcactgccgccgccagaatcaaacctgcgggcaggaaaacgcgcggattcgagcgatccgataccgaacccatgatgaatttcgaaaatccataagcaatcgagatccccgaaagggcaaaacctaaatcaccgcgtgagaatccctgctcaaccagataaggcatagcaagcgcaaagttcttacgaaccaaatagtaagccgcatagccaaagaatatccccaggaaaatttgccagcgcaatcgacgataagtcggatcgatctccgcggcaggtaagcgcgctttgtgtggcgctggtttaaaaatactcaacattgatagcctccgtggcccgtggtcttatttatgattaacagcctgattcagtgagagaacctgccgtttcttgagttgccgcgatgttaagaaaacattcataaattaaatgtgaattgccgcacacattattaaataagatttacaaaatgttcaaaatgacgcatgaaatcacgtttcactttcgaattatgagcgaatatgcgcgaaatcaaacaattcatgtttttactatggctaaatggtaaaaaacgaacttcagagggataacaatgaaaactcgcgactcgcaatcaagtgacgtgattatcattggcggcggcgcaacgggagccgggattgcccgcgactgtgccctgcgcgggctgcgcgtgattttggttgagcgccacgacatcgcaaccggtgccaccgggcgtaaccacggcctgctgcacagcggtgcgcgctatgcggtaaccgatgcggaatcggcccgcgaatgcattagtgaaaaccagatcctgaaacgcattgcacgtcactgcgttgaaccaaccaacggcctgtttatcaccctgccggaagatgacctctccttccaggccacttttattcgcgcctgcgaagaagcagggatcagcgcagaagctatagacccgcagcaagcgcgcattatcgaacctgccgttaacccggcactgattggcgcggtgaaagttccggatggcaccgttgatccatttcgtctgaccgcagcaaacatgctggatgccaaagaacacggtgccgttatccttaccgctcatgaagtcacggggctgattcgtgaaggcgcgacggtgtgcggtgttcgtgtacgtaaccatctcaccggcgaaactcaggcccttcatgcacctgtcgtggttaatgccgctgggatctgggggcaacacattgccgaatatgccgatctgcgcattcgcatgttcccggcgaaaggatcgctgctgatcatggatcaccgcattaaccagcatgtgatcaaccgctgccgtaaaccttccgacgccgatattctggtgcctggcgataccatttcgctgattggtaccacctctttacgtattgattacaacgagattgacgataatcgagtgacggcagaagaggttgatattctgctgcgtgaaggggaaaaactggcccccgtgatggcgaaaacgcgcattttgcgggcctattctggcgtgcgcccgctggttgccagcgatgacgacccgagcggacgtaacgtcagccgtggcatcgtgctgctcgaccatgctgaacgcgatggtctggacggatttatcaccatcaccggtggcaaactgatgacctatcggctgatggctgaatgggctaccgacgcggtatgccgcaaactgggcaacacgcgcccctgtacgactgccgatctggcactgcctggttcacaagaacccgctgaagttaccttgcgtaaagtcatctccctgcctgccccgctgcgcggttctgcggtttatcgtcatggcgatcgcacgcctgcctggctgagcgaaggccgtctgcaccgtagcctggtatgtgagtgcgaagcggtaactgcgggtgaagtgcagtacgcggtagaaaatttaaacgttaatagcctgctggatttacgccgtcgtacccgtgtggggatgggcacctgccagggcgaactctgcgcctgccgcgctgccggactgctgcaacgttttaacgtcacgacgtccgcgcaatctatcgagcaactttccaccttccttaacgaacgctggaaaggcgtgcaacccatcgcctggggagatgcactgcgcgaaagcgaatttacccgctgggtttatcagggattgtgtggtctggagaaggagcagaaagatgcgctttgatactgtcattatgggcggcggcctcgccggattactctgtggcctgcaactgcaaaaacacggcctgcgctgtgccattgtcactcgtggtcaaagcgcactgcatttctcatccggatcgctggatttgctgagccatctgccagatggtcaaccggtgacagacattcacagtggactggaatctttgcgtcagcaggcaccagcccatccttactcccttctcgagccacaacgcgtgctcgatctcgcttgccaggcgcaggcattaatcgctgaaagcggtgcgcaattgcagggcagcgtagaacttgctcaccagcgggttacgccgctcggcactctgcgctctacctggctaagttcgccagaagtccccgtctggccgctgcccgcgaagaaaatatgtgtagtgggaattagcggcctgatggattttcaggcgcaccttgcggcagcttcgttgcgtgaactcggccttgccgttgaaaccgcagaaatagagctgccggaactggatgtgctgcgcaataacgccaccgaatttcgcgcggtgaatatcgcccgtttccttgataatgaagaaaactggccgctgttacttgatgcgcttattcctgtcgccaatacctgcgaaatgatcctgatgcccgcctgcttcggtctggccgatgacaaactgtggcgttggttgaatgaaaaactaccttgttcactgatgcttttgccaacgctgccgccttccgtgctgggcattcgtctgcaaaaccagttacagcgccagtttgtgcgccagggtggcgtgtggatgccgggcgatgaagtgaaaaaagtgacctgtaaaaatggcgtagtgaacgaaatctggacccgcaatcacgccgatattccgctacgtccacgtttcgcggttctcgccagcggcagtttctttagtggcggactggtagcggaacgtaacggcattcgagagccgattctcggccttgatgtgctacaaaccgccacgcggggtgaatggtataagggagatttttttgcgccgcaaccgtggcagcagttcggtgtaaccactgatgagacgctacgcccgtcacaggcagggcaaaccattgaaaacctgtttgccatcggttcggtgctgggcggatttgatcccatcgcccagggatgcggcggcggtgtttgtgccgtcagtgctttacatgccgctcaacagattgcccaacgcgcaggaggccaacaatgaatgacaccagcttcgaaaactgcattaagtgcaccgtctgcaccaccgcctgcccggtgagccgggtgaatcccggttatccagggccaaaacaagccgggccggatggcgagcgtctgcgtttgaaagatggcgcactgtatgacgaggcgctgaaatattgcatcaactgcaaacgttgtgaagtcgcctgcccgtccgatgtgaagattggcgatattatccagcgcgcgcgggcgaaatatgacaccacgcgcccgtcgctgcgtaattttgtgttgagtcataccgacctgatgggtagcgtttccacgccgttcgcaccaatcgtcaacaccgctacctcgctgaaaccggtgcggcagctgcttgatgcggcgttaaaaatcgatcatcgccgcacgctaccgaaatactccttcggcacgttccgtcgctggtatcgcagcgtggcggctcagcaagcacaatataaagaccaggtcgctttctttcacggctgcttcgttaactacaaccatccgcagttaggtaaagatttaattaaagtgctcaacgcaatgggtaccggtgtacaactgctcagcaaagaaaaatgctgcggcgtaccgctaatcgccaacggctttaccgataaagcacgcaaacaggcaattacgaatgtagagtcgatccgcgaagctgtgggagtaaaaggcattccggtgattgccacctcctcaacctgtacatttgccctgcgcgacgaatacccggaagtgctgaatgtcgacaacaaaggcttgcgcgatcatatcgaactggcaacccgctggctgtggcgcaagctggacgaaggcaaaacgttaccgctgaaaccgctgccgctgaaagtggtttatcacactccgtgccatatggaaaaaatgggctggacgctctacaccctggagctgttgcgtaacatcccggggcttgagttaacggtgctggattcccagtgctgcggtattgcgggtacttacggtttcaaaaaagagaactaccccacctcacaagccatcggcgcaccactgttccgccagatagaagaaagcggcgcagatctggtggtcaccgactgcgaaacctgtaaatggcagattgagatgtccacaagtcttcgctgcgaacatccgattacgctactggcccaggcgctggcttaaactcctttctgatgcccggtaagcatgtggttaccgggcatttttgcgtacacgattccgtgcccaatgtatgcgttgcaacgcagtgaaaattcctctgaaaacgtctcgcaaaggctgaaactggcagatgtcaaaggcctgggataaccgtaatgtcgcgtcatcataaatatcaggtgacggacaaccatgaccgaatcaacaacctcctccccgcatgatgcggtatttaaaacctttatgttcacacccgaaaccgcacgggattttctcgaaatacatttaccagaaccactgcgcaagctttgcaacctgcaaaccttacgcctggaacccactagttttattgaaaaaagtttacgcgcttactactcggatgttttgtggtccgtggaaaccagcgacggtgacggctatatctactgcgtgattgaacatcaaagctctgcagaaaagaatatggcttttcggctaatgcgctatgccactgccgccatgcagcgtcaccaggacaaaggctatgacagagtcccgctggtggtgccgttgctgttttatcatggcgaaacctcgccttacccgtactcactcaactggctggatgagtttgacgatccgcaacttgcccggcagttgtacaccgaagcttttctgttggtggatatcaccatcgtacctgacgatgagatcatgcaacatcggcgtatagctctgctggaactgattcaaaagcatattcgcgaccgcgatttaatcggcatggtcgacaggatcaccacgcttttggttagaggcttcactaatgacagccagctacaaacactgtttaattatctgctgcaatgcggcgatacctcccgtttcacccgttttattgaggagattgccgaacgttcaccactacaaaaggagagattaatgactattgctgaacggctacggcaggaagggcatcaaattggctggcaggaaggtatgcatgaacaagccattaaaattgctttgcgcatgctggagcagggctttgaacgtgagattgtgctggcgacaacccaactcactgatgctgatattccgaactgtcattaaaaggagagattaatgactattgctgaacggctgcggcaggaaggacatcaaattggctggcaggaaggtaaattagaaggtttgcatgaacaagccattaaaattgctttgcgcatgctggaacagggctttgatcgtgaccaggtgctcgcggccacccagctaagcgaagccgatctggcagcgaataaccactaattaacacaggcccacagccgatccccatgggcctttgatatcaataactaccttttatgcgtggcccatttttgcctgatttaaacatcgccagtcgttgatccagggcatcgctgtagagcatcgtgtcaacgccaacagcgacaaagttcgctccccacgccaggcattgctgcgccatatcaggagccacagccagaaaaccagccgctttacccgcagcacggatccgccgaatactggtttcaataattcgctgcacttccgggtgcccggcgttatccgggtagcccaacgacgcagaaagatccgcaggtccaataaacacgccatcaatcccttcgacgtcgaggatttcgtccaggttatccagtgccgttttactttccacctgcaccaacagacaaagcgaatcgttaacttgcgccatgtaattctcaatgcgtccccagcgcgcagcccgtgccacactggccccgacaccacgctcaccgtagggaggatagcgcgtggcagacaccacctgacgtgcctgttcggcagtatcgaccatcgggatcagtagagtttgcgcgccaatatccaggacttgtttaatcagcggtttactgccttccaccggacggatcacgggttggctggcatagggcgctaccgcctgtagctgatgataaagatcctgaatggtgtttggcgcgtgctccccgtcaatcagcaaccagtcataaccagaagtggcggcaatttctgccatataggcagtcgttgagcttaaccacagaccaatttgcacttcgcccttgcgtaaacgttctttaaagggattgcttaataatgcgttcatcgtgttccttaacctatttaatgatgtgccacgtcggtctgcgcaacagtgcgatttacacgcagagtgaaaataatcagcgaaccgatgaccgccaccgctgccagcgtcagtaatcccgccgcatcgctggcaaataacgtttctgctttcacgcgcaggatcggggcaataaacccgcccactgcaccaaacaggtttacaaaaccaattcccgcagccagcgccgtaccggaaagcagttgtgtcggcatcgtccagaacactggctgcacggcaataaacccgatagctgcaacacacagcgctacgatcgccattactggagaaagcagcccggacagaccaataccaatgcccgccgccagtaatgtcagcgctgcgacattacgccgttcgccggttttatcggaatagcgcggaataagccaggtcccaaacaaggccgcaacccacggaatggcggtgaccaccgacgctgtaaagcccacttttgttcccagcaatgccgcaacctgggtcggcaggaagaaaattaatccgtaaaccgccacctgaatggtcaggtagataatcgctagttgccagactcggccattacgcagcgcatcgctcagccgagaagtcactttctgttgttcttcacttgccagttgattgataagcaacgttttttcttgtttactcagaaaacgtgcctgctccggtgtgtcatcaagccaaaagaatgtgaataccccagcaccgactgccaacaatccttcaatcacaaacatccagaaccagccgggatgccccataaatccatgcatctccaacagcgcgccggaaagcggtgatcccagtgttaacgccagcggtgcgcccatatagaacagccccataatgctggcgcgattacgctgcggaaaccattgcgaggtgagataaatcataccagggaaaaatccggcctccgcagcacgaagcagagtgcgaactatcagaaatttcgcttcagtatcggcccatgccatggctgccgaaagaaatccccacagcagtgttgtcgtaccaatccaggttctggcccccagtttgcgcatcaaaagattcgccggaacacccagaaacgcatataccacaaagaaaatgcctgctcccagcgcataagcttcattactcaacccggtatcaatctggtaggtctgtttggcaaaaccgatattcgaacggtcgagaaacgccagcacatacagcgccaacataaacggaattaaacgcacacggtttttcttcaccacggcgtcaagcaaagcggtgctcataaaaagctccttagaatatgtgggcgttaccgttgtcacagcaacgcccggagtgattagtggctgtaggggcgtttcaaattgcagtcacgattgagttcgacgccaaaaccgggtttatcaagcactgatttatgaatacgaccattcaccggaaccggctcattgagcagaatcgggtcaaactgcggacgcatcgttgaacaatccgggctggtcatcaggaattcgctgaatggcgtattggtgaaggtgatcaccgcatggtgagagtaaacagacgaaccgtgcggcaccaccagttgccccctggatttggcgattgcggcaatttccaccagcgtggttaaaccaccgcaccagccaacatccggctgcataatgtcgataccggtttctgaaagcgtacgaaaagattgcagtgtgccgtggtgctcaccgctggtgaccatcattccgactggcgcgttgcgtttcagttcgcgataactttcatactgctgtggcggcaggcactcttcgatccatttcaggttatagggcgcgcaagcgtgggccagtttggtcgcatagttcacgtcctgactcatccagcagtcgagcattaaccagaaatcctcaccgcatttttcacgcatatccgcgaccatagcggcatctttgcggatccccgcatcgccatcatgtggcccccagtgcgtcggcattttgccaccgataaagcccatctcttttgccagatccggacgcgcacctgtggcgtagaactgaatctcatcacgaacagcgccgcctaaaagtttataaaccggaagcccgaccactttgccgaacagatcccacagagccagatcgacacaagaaatcgtattcatcaccaggccaccagagccggagtaatacagggtggcactgagcatttgatcgtggatcagtttgatatcactgacacatttaccctcaatgaaacggttaagatgtttttcgacaataaaacagcccatttcaccggctgtcgaaacggcgaatccggtctggccgttttctgcttcgacttcaacaaccaacgtgccaagaacgttaatgccaaatgactggcgtgactgctcgtaatcgcggtatttactcatcggggtggcaatatgatcgtctatccagtgattcgccccctggtcgtgataatcaccgccgccagcgcctttttctgctgtcgcaccgccagtaaaccaggcgcgaacctgtttaatttttggtagggtcatgatgttctccattgttatgaggcttgtaagtcaaagggacttttccatcccaacagacgtgaaatatccctggcgcaggcaatggccttgcccgccagataatcacggtattcttcattgatttgtaagcgggtaccgaccaccgagatcgcagcggtaagctcgttattggcgttaaacaccggcgcagcgacacaacggacatcggcgtaatcttcgccgttgtcatagctccagccctgacggcgaatacgcgccagttcttcgtgaagttgctgtggatgagtaatcgttgtgggtgtcgcctgctcccagaccagcccttcgataatactttgctgtaccgctgcaggttgccaggcaagcaggcatttacctattccggagcgataaagcgaaaggctttttccttcatgggaacgcacgctgatagtggctgatgactccactttcaaaatgtaataagcgctgccgttatcaataatccccaggtgacataacagcccggtggtatccatcagttgcgtcaaacgcggtcgagccagttcccggagatccatcttgcttaacgcatgaccggaaagctccaccagcctggtccacaaacaaaaattttcctggtgatcaaggctaagaaaacgctgacgcctgagttcattaagcagcaaataggccgtgcttttagggattcccaatgtgtcaatgatcgtcgcagcactacaggggccaatgcgggcaatcaaattgagaatatcaatagcccgtgtcagggcgggaactttgcttgattccaacatactggactccagtcttagatactggaatcagtctcgttgctcagggggagtaaaattgtgaagcgcatcaaatcccgctcctcgtccagcagactggagaaattacgcacaaatttgtgaatcagcgcacggattttttcttattgagtacaacaggttggacaaattttgccggagggggaatgtgccggtgcagtaaaccggcacagagtggcggaatcagacagataaggtcatggactcaacaacctcaatccagccatgctcactggcgatatcctggccgtttaaccaacggcgcagcatattcagtgccatcattgcgcacacttcctgacggatagccaggctgtagcgcgtagtgctgaaacgcacacgcagagcgaaagtgccgtctggcgtggctagcgcaaagttgagatgctcgttctcgaaacccgaaacagccagtgccagcccggcaaaatggttggcccgccgttctgtaatccagtgcgcagtttgcgccagggtttcctcctgtgaaggaaccacttcacacgccagcaatggagcacctgcgcgagaaagttgcaaagccaataaaccaccggtgaattgctcgctcaacgtcaggctgaactggcggttttgcaattcgcgactgatctgcgcgggcagtccttcagtgccttcgaaaatcacgctctgtccggcaacacgtttaacatccagccacagtttttccatcgcctgttgctcgcttgccggtccggtgagtttcagttcgatgataggcattgaggagcgatagcccattgttacgcccggcggcagttgtagagtgtccaggctttgtgccagatcgctttccgaacgaccaaaagtagtcaaacgcagacaaaccggcggctgcggtaaagaaaaacgctcgcgcaggcgcggcaggatttcgtgctcgaccatcaccttaaattctgacggtacgccgggagtaaagaacatcaggcaacgattaagctgcacggcaaaaccacaggcggtgcctaccgggttattgataaattcagcactggcaggcagctccgcttgtttacggttgctcggtgccattactcgtccacgttcgtggaaatagcgttccatctctttgagccaggcttcatgcagcaccaggccttcaccttttgctgtcgcagcggcgagtgcgcttaaatcatcgctggtcggtcccagcccgccgttaacgatcagcacatcggcgtgctgactacgttcgcgaagaatggtgactaagtcatcaaggttatcccccaccgtattgcggcgagataatggcaacccctgatgaaagaaaaaatcggccagccaggcagcgttagtgtcaacgatttgcccgtgtaacacttcatccccggtggataacatttccacttttaacatggttatctcctgcttttgttatcgaatcactataacgcaaagggagataaggcgtagtaagaaactgaatggcgcgacagaatgccgcgccggaagggatcagaaactggcgttaaccccaacatacgggccgtcagccacggcgttgtcgcggttaccgtctttacccgacagattcaggtagcgataacccgcctcaatactgactggacgcataatggtgtaacgcgcgccagcattcgcttcttcataactttgaataccgctggagagcgaatccggagagtagtaatactcgccaaacaaacggaagctgttgccaattttccactgcaaaccacctcctaccgctgcggcataaccttcatcgccgtaattcgggttggtgtaaacgccttttccgccaacggtcgccattaacggcccgagaggcagattcaaccccagccccacgccagcgacatcaccgtcgtcgtcgttatgtgtccagttaccgcttaacgccaggcccgtcgtttcagtcccaaaaccgacaccaatattggtgtattctttacccgcctgaccgctgatgctcattgcattgaccgatgcagaaaccaacagcattccggccagacctgctagcgcaatttttttcattatcccctttcccacaagcaattaatcaaaattcccaaagctgcgggattgtactgcctggcacagaggattcaatgagcgaaaaaaaggatctagtcacttattgtaactaaatacttcttaaataattaaatgccgaaaaaataaacacactttatcgatacacacaaaaataataataagtacagttatcatcgcaaaagagattactgtcactttcacatatttgtgagttaccgtattctcatggtttctttttatttataaggaatatccctgtgcgacaacggactattgtatgccctttgattcaaaatgatggtgcttatttgctgtgtaaaatggccgacgatcgcggcgttttccccggtcaatgggcgatttcgggtggcggcgtggagcctggcgaacgaattgaagaggcactacgccgcgaaattcgcgaagaactgggagaacagctgcttttgacagaaatcacgccgtggaccttcagcgatgatattcgcaccaagacgtatgcagatggtcgcaaggaagagatttatatgatttacctgatttttgactgcgtttctgccaaccgagaagtgaaaataaacgaagagtttcaggactacgcgtgggtaaaacctgaagatctggtgcattatgatttgaatgtcgccacccgaaaaacgttacgtttgaaaggtcttctgtaacaatgatgacagccattactggctgtcagattgaaaatttagtggttaacgaattccccatccagataaactttgcctttttccacatgcatgactaaaccatccagataatcaggtttaaatgtcgcgtcacgcttatctttagcaatatatgtcaggcaatgattatgggtgaaaataacgatatttttatcaggcgctttgctttgtaagtccttaattgcactataaatctcattaccgcactgaagaagtcgtttatctaccgtcaattttttacccgctgaaaaccaggtagccgactgaatggtccggacggtattactggaataaagatcgaaatcagggatatcagcactaaaagcgttgcccagttcacgggcatcctgggtacctttaaccgtaatacctgttttatctgacaagcattgattggttgaacggtcgcaacgttcagcatgacgaaacaaaacgacaaccgggtgctgctgtgccagtctggccagtgttttattgtcgatacgtggcaaaccattgctactccaggcggcatgagtacccagtccggcaattgcagcgagcgccagtaaaatgatgatatatttttttgacttcaacgaagagcggcaaaaagctaacacgtaaactccacctatagacaagcgcaaccagacaattaccgtgaaattgagctacatttctggcgataattcgcagttggtgtaatattaaaaatcctacgatgtcggcaaaatgcctcaaaattttgccaaatgcaaagcctaaataagaaaaaatataaaaatttcaatatttacgtctaatattagtttcttaaggttaagttaatattctatccttaaaatttcgctccaaatggcaaaatatacacaacactctttatagcaaatataagtggacaggtattcaatggcggaaggaaaagcaatgtcagaatttttgcctttttcgcgaccagcaatgggcgtggaggaactcgctgcagttaaagaggttctcgaatccggttggatcacaaccggtccgaagaatcaggcgcttgagcaagctttttgccagttgacgggaaatcagcatgccatcgcggtcagttcagccaccgccggaatgcatatcacgctaatggcgttgaaaattggcaagggcgatgaagtgattacgccttccctgacctgggtttcaaccctcaatatgatttccttgttgggtgcaacgccggtaatggtggatgtcgaccgcgatacgctgatggtcacgcctgaagctatcgagtcagccattacgccacgcactaaagccatcattccggtgcattatgccggtgcgccagcagatattgacgccattcgcgccattggcgaacgttacggcatcgcagttatcgaagatgctgcccatgccgtcggtacgtattacaaagggcgacatattggcgcaaaaggtaccgctattttttcatttcatgccattaaaaatattacctgtgctgaaggtggcctgattgtaactgataatgaaaaccttgcccgccagctacggatgctgaaatttcacggtctgggtgtcgatgcctatgacagacaaacctggggccgtgcaccgcaggctgaagtcttaacaccgggctataagtacaatctgaccgatattaacgccgcgattgccctgacacagttagtcaaattagagcacctcaacacccgtcggcgcgaaattgcccagcaatatcagcaagcactggcagctctcccctttcagccattaagccttcccgcctggccgcacgttcacgcctggcatctgtttattattcgtgtcgatgaacaacgttgtggtatcagtcgcgatgcgttgatggaagcgttaaaagaaagaggcattggtaccgggttacatttccgcgccgctcacacacaaaaatattatcgcgagcgttttcccacgctgtcgttaccgaataccgaatggaatagcgaacgcatctgttctttgccgctgttcccggatatgactaccgccgatgccgaccatgtcatcacagcccttcagcaactcgcaggacaataagccatgtttgaaatccaccctgttaagaaagtctcggtggttattcccgtttataacgagcaggaaagcttaccggaattaatcaggcgcaccaccacagcctgtgaatcgttggggaaagagtatgagatcctgctgattgatgacggcagtagcgataattccgcgcatatgctggtcgaagcctcacaagcggagaacagccatattgtgtctattttgcttaaccgcaattacgggcaacattcagcgattatggcgggattcagtcacgttactggcgacttaattattacccttgatgccgatctccagaatccgccagaagaaatcccccgcctggtggcaaaagccgatgaaggttacgacgtggtagggactgtacgccagaaccgccaggacagctggtttcgtaaaaccgcttcgaagatgattaaccggcttattcagcgcaccactggcaaagcgatgggtgattacggttgtatgctgcgcgcctatcgccgtcatattgtcgatgcgatgttgcactgccatgaacgcagcacctttatcccgattctggcgaatatcttcgcccgccgtgccattgaaattccagtacatcatgccgagcgtgagtttggtgaatccaaatacagttttatgcgcctgattaatttgatgtacgacctggtgacctgccttaccacaacgccgctacgtatgctgagtctgctcggcagcattattgcgattggaggttttagcattgcggtgctgctggtgattttacgcctgaccttcggaccacaatgggcggcagaaggcgtctttatgctatttgccgtgctgtttacttttattggcgctcagtttatcggcatgggattactcggtgaatatatcggcaggatctacaccgatgtccgcgcccgcccccgctattttgttcagcaagttatccgtccatccagcaaggaaaatgaataatgaaaaccgtcgtttttgcctaccacgatatgggatgcctcggtattgaagccctgctggctgccggttacgaaattagcgccatttttacccatactgataatcccggtgaaaaagccttttatggttcggtggctcgtctggcggcggaaagaggcattccggtttatgcgccggataacgttaatcatccgctgtgggtggaacgcattgcccaactgtcgccagatgtgattttctctttttattatcgccatcttatttacgacgaaattttgcagctcgctcccgcaggtgcatttaatctgcatggttcgctgttaccaaaatatcgtggtcgcgcgccgctgaactgggtgctggtcaacggtgaaacggaaactggcgttacattgcaccgaatggtgaaacgtgccgatgccggggccattgtggcgcaactgcgcattgccattgcgccagacgatatcgctattacgctgcatcataaattgtgccatgccgcgcgccagctactggaacagacattacccgccattaaacacggtaatattctggaaatcgcccagcgcgaaaacgaagccacctgttttggtcgcagaacgccggatgacagtttccttgaatggcataaaccggcatccgtactgcacaacatggtacgtgccgttgccgatccgtggccgggtgccttcagctatgttggcaatcagaaattcaccgtctggtcgtcgcgtgttcatcctcatgccagcaaagcacagccggggagcgtgatttctgttgcgccactgctgattgcctgtggcgatggcgcgctggaaatcgtcaccggacaggcgggcgacggcattactatgcagggctcgcaattagcgcagacgctgggcctggtgcaaggttcacgcttgaatagccagcctgcctgcaccgcccgacgccgtacccgggtactcatcctcggggtgaatggctttattggcaaccatctgacagaacgcctgctgcgcgaagatcattatgaagtttacggtctggatattggcagcgatgcgataagccgttttctgaatcatccgcattttcactttgttgaaggcgatatcagtattcattccgaatggattgagtatcatgtcaaaaaatgtgatgtcgtcttgccgctggtggcgatagccacgccgattgaatatacccgcaacccgctgcgcgtatttgaactcgattttgaagagaatctgcgcattatccgctactgcgtgaagtaccgtaagcgaatcatcttcccgtcaacttcagaagtttatgggatgtgtagcgataaatacttcgatgaggaccattctaatttaatcgtcggcccggtgaataaaccacgctggatttattcggtatcaaaacaattacttgatcgggtgatctgggcctatggcgaaaaagagggtttacagttcaccctcttccgcccgtttaactggatgggaccacgactggataaccttaatgcagcgcgaattggcagctcccgcgctattacgcaactcattctcaatctggtagaaggttcaccgattaagctgattgatggcggaaaacaaaaacgctgctttactgatattcgcgatggtatcgaggcgttataccgcattatcgaaaatgcgggaaatcgctgcgacggtgaaattatcaacattggcaatcctgagaacgaagcgagcattgaggaactgggcgagatgctgctggcgagcttcgaaaaacatccgctgcgccatcatttcccaccgtttgcgggctttcgcgttgtcgaaagtagcagctactacggcaaaggatatcaggacgtagagcatcgtaaaccgagcatccgcaatgcccaccgctgcctggactgggagccgaaaattgatatgcaggaaaccatcgacgaaacgctggatttcttcctgcgcaccgttgatcttacggataaaccatcatgaccaaagtaggcttacgcattgatgtcgatacctttcgtggcacccgtgaaggcgtgccgcgtctgctggaaatcttgagtaagcataatattcaggccagcatttttttcagcgtcggcccggacaatatgggccgccatctctggcgactggtgaagccacagtttttgtggaagatgctgcgctcaaacgcggcatcgctttatggctgggatattttactggcaggtacggcctggccaggtaaagagattggtcatgccaatgccgatatcattcgtgaagcggctaaacatcacgaagtcggcctgcacgcctgggatcaccatgcctggcaagcccgtagcggtaactgggatcggcaaacaatgatcgacgatattgcacgcggtcttcgcactctggaagagattatcggtcaaccggtaacctgttctgccgctgcgggctggcgtgccgaccagaaggtgatcgaagcaaaagaagcgttccatttgcgctacaacagcgattgtcgtggggccatgccgttccgtccattgctcgaatcaggaaaccctggcactgcgcaaattccggtgaccttacccacctgggatgaagtgattggtcgggatgtgaaagcagaagattttaacggttggttactcaaccgcatcctgcgagataaaggcacgccggtttataccattcatgcagaagttgaaggctgcgcttatcagcataattttgtggatctcctcaaacgcgcagctcaggaaggcgtgacattttgccctttaagcgaactgttatcagagacgttgccgctcggacaagttgttcgcggaaatattgccggacgtgaaggctggctgggttgccaacaaattgcgggtagtcgctgatgaaatcggtacgttaccttatcggcctcttcgcgtttattgcctgctattacctgttaccgatcagcacgcgtctgctctggcaacccgatgaaacgcgttatgcggaaatcagtcgagaaatgctggcatccggcgactggattgtgccccatctgttagggctacgttatttcgaaaaacccattgccggatactggattaacagcattgggcaatggctatttggcgcgaataactttggtgtgcgggcaggcgttatctttgcgaccctgttaactgccgcgctggtgacctggtttactctgcgcttatggcgcgataaacgtctggctctactcgccacagtaatttatctctcattgtttattgtctatgccatcggcacttatgccgtgctcgatccgtttattgcattctggctggtggcgggaatgtgcagcttctggctggcaatgcaggcacagacgtggaaaggcaaaagcgcaggatttttactgctgggaatcacctgcggcatgggggtgatgaccaaaggttttctcgcccttgccgtgccggtattaagcgtgctgccatgggtagcgacgcaaaaacgctggaaagatctctttatttacggctggctggcggttatcagttgcgtactgacggttctcccttggggactggcgatagcgcagcgggagcctaacttctggcactattttttctgggttgagcatattcaacgctttgcactggatgatgcccaacatagagctccgttctggtactacgtgccggtcatcattgccggtagcctgccgtggctgggattactccccggtgcactgtacacaggctggaaaaaccgcaagcattccgcaaccgtctatttgttgagctggacgataatgccgctgctgtttttctccgtcgctaaaggtaaattgcccacctatattctttcctgctttgcatctctggcaatgctgatggcgcattacgctttgctggcagcaaaaaataatcctctggcgctgcggattaatggctggattaacatcgcttttggcgtcactggcattattgccacatttgtggtctccccgtggggaccaatgaacacgccggtgtggcaaaccttcgagagctataaagtcttttgtgcctggtcgattttttcgctatgggcatttttcggctggtacaccttaacaaacgtcgaaaagacctggccttttgccgcgctttgcccgctggggctggcgttgctggtaggattttcaattcctgacagagttatggaaggaaaacatccgcaattttttgtcgagatgacacaagaatcacttcagccaagccgctatattcttactgatagcgtcggtgttgccgcaggtctggcatggagcctgcaacgcgatgacatcatcatgtatcgccagacaggtgagttgaaatacggccttaattatccggatgcgaaagggagatttgtcagcggtgatgagttcgcaaactggcttaatcaacatcgtcaggaggggattattactctcgtgctttcggttgaccgcgatgaagatatcaacagtctcgccattccgcccgcagatgccatcgatcgtcaggagcgtctggtgctgattcagtatcgtcccaaatgatctggctaacattagtctttgccagcttgcttagcgttgccgggcagttgtgtcagaaacaggcaacctgctttgtggcgataaacaaacggcgcaaacatatcgtgctgtggctgggactggcgctggcttgtcttggtcttgccatggtgctctggctgctggtcttgcagaacgtaccggtaggcattgcttacccgatgttaagtctgaattttgtctgggtgacgctggctgcagtaaaactgtggcacgaaccggtatcgccgcgtcactggtgtggggtggcgttcattattggcggcattgtgatcctcgggagtacggtgtaatgggcctgatgtggggattattcagcgtcattattgcctcagttgcgcaattaagcctgggttttgcggcgagtcatctgccgccgatgacgcacttatgggattttatcgcggctctgttagcttttggcctggatgcccggatactgttactcgggctgctgggttatctgctttccgttttttgttggtataaaacgcttcataaacttgcgctaagcaaagcctatgccttgctcagtatgagttatgtgctggtatggattgcttcaatggtacttcccggctgggaagggactttttcgctgaaagcactactgggagtagcctgtattatgagcgggttgatgctgattttcctgcccacgacaaaacaacgttactgagttttccctgccactttacactgccgttcccactcatcggggctataactgcttgccgagaggactttcaccgtatgcagcttttcacgattaatacaataaagcgcattctgcaaaggcgagagtaaatcccccactttcacggcgaagtcactcttcacttcggcgatcatttttatcgcgccgccagcatcgcagagcataagtacatgtctgttatcttgtttattgcagcacgattttttgaccagccattccattgcattatcctgtttgctaagagttttcacatcaatttacagattaacagataaactctttatcaacggcaatggaatggcagaaatgagaagtgaaacggagggttaattattgctgacgttgcacccactcttttagcgcctgacgtgaaattttaataccgccgtttttcagctccggcggcagagttagccagcgcaccggttgttgaaaacgggccagcttatctttcacccattcactaagatcaacgctctcgtggtcatactccatcaccgccaccggtcgatgaccaaactccttgtcggcaacggggacgataaacacctgcaaaaccgcaggatgtgcagcaattacgcgctcgacttcttccggctgaataccctctccgccactgaagaatagattgtctaaacgtccgacaatggtcagcttgccattatgcatctcaccgcgatcgcgcgtagcgtaccagccttcgtcattaaccagtgaaaccagttgcccgttacgccagtaaccttctgccatactggcagcccgcagccacacttcattattaacgattttcacttcccgacccggcagcggcgaaccaacgtctgccaggccgtcggcttctttcgcacacaccgtggaggcaaactcggtcagaccatagccgcaaaagcaacgaatcccctgctcgcgcgcctgttccgtcaactcgaccgggatagccgcgccgccaagtaacaccgctttcagggaaacggaactacggttaaccagcaaacgccagagttgtgttggcaccagtgaagcgtgagtacagcctgccagcatttgctccaatggctgtttatcacgtaccgtcatccgcgcaccagcgtataaccagcgccacataattccctgaccggagacgtgaaacagcggtaaagagagcaaccaatcatcgtgatcgccaaacggaatcagcgataacacaccttgcgcactggcaagatgggcctgataagtatggacagcggctttcggcaaaccggtagaacccgaggtcaacgtcattgagcacagacgcgtcggctgccacgtagcggcatgtgcgccttcaaccagctgaatgtgcagcgacgttaatgccggaaacgtgttttccccatccggcaccagagcaaattgcagcgtcagattgggcagcaattcttcaagcaacggttgcggcagctgagggttcacgggcaacacccgcgccccgcattgcagtaacgccagccaggcgagcagcgtttgcggcgtattccacgcccgcaacatcacgccgctgccctcaaccaccccctgcaccgcaaatccggaggctaattcatcgacgcgagcacaaagctcgcgccagttgagttgctcgtcattaagacgtaaggcgatggtttctccccgcacttgccgccagtgacgccacggccagtcagagaagatcataacaaccgctccagtgcatcaacttccacgacaggcagcgtgctacccggccagcgacgtacctgctgcgcctgcatcagatccagcgtgtccagccctggaatggtgtccggcgttaaccaggcggcaatccgcgccagttgcgttaagcctaagctcgattcaatggaagaactgatcaccgccgtcagccccagcgcgtgcgccgcctgtacctgctcgcgtactttttccagactgcccgtgagcgtgggtttgataactaccgcgcgcacgccctcttcagccacaaaggcaaaatccggctcgcgcaggctttcatcccaggcaatggcaatgccggtttcacgggcaaacgctcgcgaatcatcgcgggttttgcacggctcttcgagaaacgcgatgcggtcgcgataatccgggttaacgtatttggcaaactgctgacctttcagcggtgtccaggcgcgatttgcgtcaagacgcaaatgcagatccggaattgcctccagcaacagattcaccaccatgccgtcgcgcaccgcttcgtacaatcccactttgaccttcgccactttctcgcctggcatatctgcaagtttgaggatcagatcgtccggatcgccattacacagcggtgccgcacggtagttggctgcttgcggcaacgtatctgtcagttctgccaatgcacagcttacgccaaaggccacggaaggcatctgcggtagctcgcaatcgcctgccagccagttatttacccaggcaagcagcacactttgcgcctcttcccaggtttcctgactgaagcccggcagtggggagatctccccccacccttcgcgctcgccttcacgcaggcaaacatacagcccgtcgcgggtttttaaccgcctgtcgcgcagaaccacccccgcgtccatggggatctgccagcggtatacctgcgcgctacgcattacggattccgtttgaatttgctgaagtcaggctgacgtttctggttgaaggcgttgcgaccttcctgaccttcttccgtcatgtagaacagcatggtggcgttgcccgccagctcctgcagccccgcctgcccgtcacagtcggcgttcagtgcagctttcaggcagcgcagcgccatcgggctgttttgcagcatttcgcggcaccaacggacggtttctttttccagatccgccagcggtaccacggtgttcacaaggcccatatccagcgcctgttttgcgtcgtactgacggcacaggaaccagatttcacgcgcttttttctgcccgacgatgcgagccatgtaggaagcgccccagccgccgtcgaaggaaccgactttcgggccagtctgaccgaagatggcattatctgccgcgatagtcaggtcgcacatcatgtgcagaacgtgaccgccgccgatggagtagccagccaccatcgcgacaaccggtttcggacaggtacggatctgacgctggaagtccagcacattcaggtgatgtacgccggaatcatctttatagccgccgtaatcaccacgcactttctggtcaccaccggagcagaacgctttatcgcctgcaccagtcagaatgatcacgccgatgttgtcgtcataacgcgcatctgccagcgcctggatcatctcttttaccgtcagaggacggaaggcattgcgcacctgcggacgattaatggtgatttttgcgataccgtcggtggatttttcataacgaatgtcctcgaaaccttcggagcagtcgtgccattcaaccggtgcgtaaagcattgcttcatcaggataaatcatattgtgtcctttagtcagaaacgcaagatctgcgccagacttgcgattacgccagcgggattttcccgatgcgcgttatgtccggcgcgaggaatgacatggcagtcggcagccagttccgccgccagggcgcggaatttgctgtcacgttcaccacataaataataaaacgcaaatgtgcgggcgctaaggttagcacgtaaatcaggctggacggcgagagaagtcgcctccagcatggcggcaagcgttgcgccattattgttgctgcgcagcgccaccagctcccggcgttgatcgtcattgagtgaggcaaaaacaggctgttgataccagtcggcaaataccgccgttaacggttctgtgagaaaacgctgcacccattggcgatcggaacgctgacgttccgcacgttgttcagcattttgcagccccggatgcccgccttcgacaataaccccacaaagccccgccagcccctggcaagccgccatcatcgccacccgtccaccaagcgagtaccccaccagccagaagtcaaggatgttgtaactaaccaaggttttacgcagtaagtcggtgacatcatcaaatccatcgacgctaatcgccgccgaaccaccgtgacctgggagatcaacatacaaccgtgagtagtcggcaaacgcctcgcccacttcttgccattcgtggcaatcgccggaaaaaccgtgcaaaaacaccagccagggtaaacctggttttccgtgttttgcctgcgcgtgcaggatcataaatggcttacctgcgccagaagttgctggagcgtttgcgcaccatcggtgtcgttaaccaccatttcaatcaccgtggtggttggcgtgcgccaggcgtcggcaaatgccgtttcaagttcctgccagttttgcggacgatgatatttcagctcgaacatcgcggcggcgtgctcaaaatggacgttttgcggcatcagatagaaacgctcacgctcgctttgcggcgttggcaacagcgagaaaatttgcccgccgttgttgttcaccacaattaataccagcggcgcagaaacctgacgcaataacgccagcgcgttgagatcgtaaagtgcggagagatcgcccacaatcgccagcgtcggtttgccgcttgcccgctgaacgccggcggcggtcgaaagcagcccgtcgataccgctggccccacggttgctgtacaccgggtaacctgccggaagttgcgaaagcgcatcaatcagacgtaccaccaggctgttaccaacaaacaattgcccctgttcaggcagatagtcgcagatgcgatgcgccagttgcgcttcgccaaacgcatcacggcgggcaataaccgcctgcattgcctgttccgccaggcgcgggatttcaacgcaccagggctggcgtttttctgccggatgcagctccagccagtcggcaatattggcaattaagcgacgtccgcgatggtgtgccggatcaagtcgcccttcaatgtcatcaacaatccagtactcttctggttcacagcttgcctgccattgcaggagccgtttccccgtcaggctgcttcccagttgcaccacaatttgcgcctgctgcagctcgctggtcgctttggcattgcctaaccaaagatcggcacacggcagcggctgcccggtttgtgacagcacatcgccaatcagcggccagccaagagtttgcgcccacagggcaacttttttgccctcttccgcactcatgcgcccggcaaccaccacgccgcgcttttgtcgccagaagaaccagtcgcgctgtttttcactttccagacgaggcgcttcacgcagccacggtttgtcgtcctgccaccagtcacccagacgctgttgccagctaagcccggtatcgtccatttcgccatacagcggttcagcaaacgggcagttgatatggactccccccgcatgaagcgtaccgagagcgtggtcgatggtagaaaccagccaacgtgcggggatatcctgggtcgggcgcggcaatgaaatactgtgcgtggggtgagaggcgaacattcccggctggcgaattgcctgattcgcgccgcagtcaattagctccggcgggcgatcggcggttaagagaatcagtttttctccggttaacccggcttcaatcagtgccggatagagatttgccaccgccgtgccggaggtcacaatcaccgccaccggctgcttgctgactttcgccagccccagcgccagatgccccaacccacgctcatcgaaatgggtgtggtgaatgaatgcggaattctccgccgccgctaacgttaacggtgtagaacgcgagcctggggcgatacagatgtgtctgacgccgtgacgcgttaatgcttccagaatgaccgccgcccagcgtcggttaaatgcgcttactgacatgagtttgtccggtatcaatattgcggctaagtataaggagctacaaaaatagattattgatatgaatcggtaatgatgcgactcattactattccatttgtaataaagtacgcagccctgccgctttgttgtcgatttcctgccactcttgctcggggtcggaaccacggacaatgcccgcgccagcatataatcgcacgacattgccgctaatttttgctgagcgcagggaaacgcagaattcgctttgttgtaatgagagatagcccgcagaaccggcgtaccattctcgggtgaacggttcgtgacgggcgataaactgtcgcgccagatcgcgcggtaagccagcaactgctgccgttggctgcaactgatgtaaacagatcacatcatccgctttgttgagtgaagtccagatacagcggcgaagatgctgcactttacgcagacgcagtacctgcggcggtaaaacatccagcgtctgggtatcggcctgtaatcgttgacagatatcttccaccaccagcatgttctcgcgctggtttttatcatccgccatcagccactctcctaactgctgcgcctgcttatcatcaggattatttgctactgttcccgccagcgcttcagtacgcagcgctttgtcacgccgccgccataaccgttccggtgaagagccaagaaaagcattttcgccatcaaaggccatgtaaaaatggtagcaattcagattcagtcgacgactggcagccatcatcgccgccgcgttgaccggacttgcgaaatgcaggtcagttgcccgagcgagcaccactttgtcgagctcaccttcggcgatggttttcgttgccagttcgattaattgcgtccagcccgttttgtccggccagtgttgttctcgcgtggtggttaaatgtaacccaggcaagggcttgatactcaccagtgtggcgataaattcttttgcctgaatcgcatcgtgctgaagggagctttcgctgaatagcgtcagccgcagcgtggctttaccgccacagcgtcgccattccaggcggggtaaaagtaaattgccctgcgacgggtcaaaagcattcagcccccaaatgcgtaagtcggcgtgttccgggtgctggcgaagaaaacgttgtgcctggtccaacgacgtaaaacgggtaatcgcgcccaggacgacagcttcttcatcaccattacgttgttgccagtagaattgcgggtatgtttgctgactggccagccagctcaaggcatcaaaagcgtctttgagagggaaaggaatatcgataacccgaatgccgggtgtcgccggaatctcttgcgacaaatggcgcagtagattttccagcgccgtagtaagtgattgcacgcggacctctccctgttaaaagcctcacattatacggggtactacaaaaaaaatgcagtaccccggtgtagggaggttttaacggcgtgccagcaacagtcctagtaccagcccaacggccgcgcccacaccaattccttgccagggtttttcgtggacgtagtcatcagcacgataaactgcctgcttcgcccgatagtaataactgtctgaagcctggctaacccgttttttcacatcatccagcgctttttctgcacgcgctttcagctcaacatatttctgatcggcgggatcgccagaggagcggagcacctcttccagtgtttcactaagcagcgtcaggtcgtcatcgatacgtgtatcaccaaactgattagacattctcgttctccatttgcgtaaaacctgtcactaactatagacaagggttgttgattacgcctgaattacctcgcgtgccatcccaatgtgtgggataccatcttcttcatagacctccgtcacagggataaaaccgaaactctggtagaagttttgcagatgcgcctgcgccccgaggtaaacaggcttatcaggccagtgatgcgtacatgtttcgagtgttttactcatcagctgctgccccactttttcgccacgcaacgcttcactgacaatcacccgacctataacgaccggctcaagatcatcatcacttttcagaatcctcgcatacgccaccagttcatcatttttccaaccgagaatatggcgattatcccccgtcaaatcatcaccatcgatatcctgataagggcaattctgctcgacaacaaacaccgcgcaacgcagttgtaataaggcataaagctgggaaaccgataattcagagtgatgcagatcttgccattcaatcataatgctctccttttagatgtatgccttatactagccggaatattttttgaaacgtgatgaactcatggaattaatttttttaggtacttcagccggtgtgccaacccgcacgcgcaatgtcacggcaatattgcttaacctgcaacatccgacccagagcggactttggttgtttgactgcggtgaaggcacccagcatcagctactgcataccgcctttaaccctggaaaactggacaagatttttatcagtcaccttcatggcgatcatctttttggtttacccggcttgctgtgcagtcgttctatgtcaggcattatccaacccttaacgatttatggtccgcaaggtatccgtgaatttgtggaaaccgcgctgcggattagcggctcatggaccgattatccgctggaaattgtcgaaattggcgctggcgaaattctcgatgatggcctgcgcaaagtaaccgcttatccgctggaacacccactggaatgttatggctatcgtattgaagaacatgataaaccgggtgcattaaatgcccaggcattaaaagctgctggcgtgccgcctggcccactgtttcaggaattaaaagcgggcaaaacaatcacgctggaagatggaaggcagattaacggcgcagattacttagctgctccagtgccaggtaaagcgctcgctattttcggcgataccggcccctgcgatgccgcacttgacctggctaaaggtgtcgatgtcatggtgcacgaagcgacgctggatataaccatggaagccaaagccaatagtcgcggccatagctctacacgccaggctgcgacactagcccgtgaggctggagtcggcaagctaatcattacccacgtcagctcgcgctatgatgacaaaggttgtcagcacctgttacgtgaatgcaggtcaattttcccggcgactgaactggcgaatgatttcaccgtgtttaacgtttaactctgcttattattaaaaacagggcgaaacttgccctgttatcgcaacccgcgctacatatatccacccacacaggcatattgagcgatttttgatatttattcatctccttacgcactatattcagagcaataagttgcctcttttcatcttgattcagcacaacctttgcaactaaaaggagcccatgatggttacagttgtcagcaattattgtcaattatctcaaacgcaactcagtcagacatttgcagaaaaatttactgtgaccgaggaattactgcagtctttaaaaaaaacagcgttatccggagatgaagaaagcattgagttactgcataatattgcgttaggttatgataaatttgggaaagaagctgaagatattctttaccatattgttagaaccccaacaaatgagaccctatcgattatccgacttatcaaaaatgcttgtttaaaattatataatctggcacatatcgcaaccaactcccccctcaaatcacatgattcagatgatctcctgttcaaaaaactattctccccttcgaaattaatgacaattatcggtgatgaaattcctcttatatctgaaaaacagtcgctttcaaaggtgcttttaaatgatgagaataatgaactgagtgatggtacaaacttctgggataaaaatcgtcaattaaccacagatgaaatagcttgctatcttcagaagatcgccgctaatgcaaaaaatactcaagtcaattatcctactggtctctacgtcccctactccaccagaactcacctggaagacgctctcaatgaaaatattaagagcgatccatcatggccgaatgaagtccagttattccccataaatactggcggacactggatattagtttcgctacagaaaatagtaaataaaaaaaataataaactacaaataaaatgcgtcatattcaactcattgcgtgcactaggctatgataaagaaaattcacttaagcgtgtcattaatagttttaattctgaactcatgggagaaatgtcgaataataatataaaagttcatttaaatgaaccagagataatatttttacatgccgatcttcagcaatacttaagccaaagttgcggtgcatttgtgtgcatggcagcccaggaagtgattgaacaaagggaaagcaattctgacagcgccccctatacgttattaaaaaaccatgctgacagatttaaaaaatattcagcagaagagcagtacgaaattgattttcaacatcgactggcaaacagaaattgttatttagataaatatggcgatgcaaatatcaatcattattatagaaacttagaaataaaacactcacaacccaaaaatagagcatccggcaaaagagtgagttaacatcattgttaattaattcgaccagtcagcaaatatgctgactggtcgaacatagtttgctaaacagtcatcactgactgatgtcagtcacaccatccgccagttcaatcaggcgaataaattccgccctgtaaccctgtggatcttccccttttgcctgctgagcccactgtttgatctgctgccaggaggtattgttcaggtattcagaaccgcgtaacttttgcccatatgcagctactgctgcgcgaaaacgcatatcttcagagggcgcgtttattgttggccccagcgggaattcaactaactgactttcttttccctgcgggtatttccagcgaatttttaaccaggccagttctttcgttttgtccgatttcgctaatttgttatccggggcatagcgtaacttatcaattgatgctttttgcccgttcagcgttaattcgaataacaacgttatatgtttgcctgcgcctatatcccctgcatcaacgttgtcgttattaaaatgttccacccgaagttggcgcttttcataaccaatctgacggtattccgttacccacgcggggttaaactcaatttgcgctttgacatcttttgctacggtaatcaacatctgccgcatttcactattcaatactttctgcgcttcagagagggtatcaatgtagctgtagttgccgttaccaacatcggcaattcgcaccatcattgcctcgttgtaattgctattccccacgccaaacgtcgacagagtaacaccagactcccgctgttttttgaccattgattcaatcgattttggatcgtcaatgccaacgttaaagtcaccgtcagtggctaataaaatgcgattgatgccgcccttaataaaccccttcgtcgcctgctgataagccagttccagcccggcaccgccattggtactgccttcggcatccagcgaatcaattgcggcattaatttccgccttatgactcccggagatagaaggcaatgcaatacgggagtcgccagcgtaggtcacgatggcaatgttatcctgctcacgaagttctttgaccaataatttcaacgaagactggataagtggcaaacgttcatcagaaatcattgaaccagaagtgtcgataagaaagaccagattagaagctggtaactcttcacttttgcgatctttcgccaggatatcaactttcagcaatgttcgctgttcattccatggtgcaggtgccaattcgtagcgcatagcgaaaggtattggcttagaggccggaatagattgtttgtctttgatatcccaatcagacgggaaataattgactatctcctccacccgcacagcgtctggcggaggtaacagcccttgattgaggaaacgccttacattcgcataactgccagtgtcaacgtcaagactaaacgtcgccaacggattttgcgctacctgcttaaccggattatcatcgaactgctggtagcgagcggttcctggatttgcgatatgtgtagcttttgctttagccgctcttgcaaatgttggcgcttcctgcaatcgcccctgtaaagcctgtttgtctgaatattgttgcacttcttgctgggccaaggctttcgcggcggcggcgctttgctcagcctcttttattgcagcttgctgcgcggcaagcacttgctgctctgtgggagtactgggttgttgttgctgactttccttattctcaggttgcggcccacatcctgacaaaatcaaactactcataagcaacatgattatatttttatttcgcatataaaatccttttaaataaactcaggcaccagacataaaatatactctttgtataatcctgctaatcttaataaaatacaatatcgaaacccatagcaaataatgattcaacaacgcaacccattaataatttgcatatgaaaaaaataatctttgcttttattatattatttgtgtttttactccctatgattattttttaccaaccctgggtcaatgcattaccgtcaacgccccgacacgcaagtcctgagcaattagaaaaaacagttcgttatcttacacaaactgtgcatccacgtagtgccgacaatattgataatctgaataggtccgcagaatatataaaagaggtctttgtcagtagcggtgccagagttacctcgcaggacgtccccattacgggtggcccctacaaaaacattgttgctgattatggtcctgccgatggaccgctgattattattggtgcgcattatgactctgccagcagttatgaaaacgatcaattgacctatacgccgggcgcggatgataacgccagcggtgtggcaggattactcgaactggcacgtttgttacatcagcaagtaccgaaaacaggcgtgcagctggtcgcctatgcgtcggaagaaccgcccttctttcgtagcgatgaaatggggagcgcggtgcatgcagcttcgcttgagcgtccagtgaaattaatgatagcactggagatgattggctattacgactctgcgcctggaagccagaattacccttacccggcaatgtcctggctttatcccgatcggggagactttattgccgtggtcggcagaatacaggatatcaacgccgttcgtcaggtaaaagcggcattgttgtcatctcaggatttatctgtttattctatgaataccccagggtttattcccggtattgatttctctgaccacctgaattattggcaacacgatattcccgccataatgattactgacaccgctttttatcgtaataaacaataccacttgcccggtgataccgcagacagattgaattatcagaaaatggctcaggtagtggatggtgttataactttgttatacaacagtaaataataaaaatttctcgaggcgggtccagaaaaagcgacatgcacattttattttccctcatctgttttaagatgcgaaacatgaaattcaacggaggaaaaataaatgggaatgattggctattttgcagaaattgactcagaaaagattaaccaactgcttgagtctactgaaaaacctttgatggataatatacatgacacgctttcaggattacgccgactggatattgataaacgctgggattttttacactttgggctgacaggcacctctgcttttgatcccgcgaagaatgatccgctgagtcgtgccgtgcttggtgaacacagcctcgaagatggcatagatggcttccttggattgacctggaatcaggagttagccgcgacaatcgaccgactggaatcactggatcgaaatgaactgcgtaaacagttttccattaagcgactcaatgaaatggagatttatccgggagtgaccttttcagaagagttagaggggcaactctttgcctcgatcatgcttgatatggaaaagctgattagcgcgtatcgacgtatgctgcgacaagggaatcatgcgctgacggttattgttgggtgatatagcttgatgcctgggggagaaagacccattagttaagatttacgccaggatcatcttgaaaaaatctttaaccatggtccggtttttatccccttgtataaatattactaaatgcttgcttagtcgcattgttaaatgcaataccgtatattcggtatgtaacagcgatatcctctgtgctggcaacgatctgtcatgcttgatgaaaacggaattgaacctgtcattaccaggtagataaaaagcctgttcaattttgggattattttttataactcgtgtctgttatggcgacacgggaaaacatcaatattgtccttcacaaattgcagtaatatagaatcaacctctcttgcaagttggtcacaatgtattataagcattttgaatatgtcatcctctgtaatctcgtgaaaattttcggccttgtcttttagctcatcatatcggattcttgcagtaaccattttttgggcgagttctaataaccccaaagcttgcaattgctggtgagtatgatcactttcaaaaaatatcccacactccattccttcccaaccaacatattcatgccattcataaaccagcataaatgtttgtaaaactggcggtaataattggatatctgcaaaaccaaaccaaaacttacgcttgagatcccactcatattcaatcgccaatgctatattgtttaaggcatctccggcatccttatttttacgcaaaatcaattccgtcagtgtatagcgttgttcatcaatacgccgaagagcttctgcaatatcatagtttgtagccaacaaaacattctctgcttcctgatgagtgacgtctgcttttgccgtcaatatattgatttggtcaatatgaaacaacttgatggcttcatcaacatcaccgccagtcctctctaacaaacgtctggcaacctggataccgacaggtacgttcttccgaagtttacgaatttcacttaaccattccatgtcaaacccctttaaatatttatgatattaaatataacaacgtctggataacgacccggcctgactgaatatctcacgttttcctgcttaacattcatgttatgatgctcttgaaactaataatacgtatggaattgtcactatttatctgctaatgaattcaaacaatgtcattcgtttgatgaatatattatttcagggaataattatgacacctttagaacgcattacccaacttgttaatatcaatggtgatgttaataatcctgatactcctcgtccattgttatctcttgaggatttttttattgacaataatatccatggttcaatatgttgcaatgtgattccagaacaatctccgcaagctatctatcaccattttctgaaaatacgtgagcgtaacaatgttagtgatgttttggtagaaattacgatgttcgatgacccagactggccctttagtgaaagtattttagttatcaccactgcttcaccagaagaagttcagagctggtttgtagaagaaattgcccctgatgagtgctgggaaggatggtcagaagatacggagcatggatgggttgaagtccctgtgggtatgcatccggttacttgttggtgggattaaaacatttatataaacagataagcggatgtttacataaatttttatgtgaaggaacatgatgaaacttattcctcgcagtagtgatatttcacctggcattgatggaatttgcccggggccttttcctccgaacggatttaccgtacttacagatgcagcatatggtaacggagactgtttcggtttgtactggcctattggtcaggagcataaactacctatagtgtgcgaaacgtaccatgacgaatggcgaatcgtacctgccttttccagcattaagaagttcgaagaatggctggaagtgaatgatgatgatccccatgaaaatggcatcagcatcgaagatcaagactttgcagcaaatctcttccgtgttgctcggaaatgtctttcaacgggaaggcttgatgacgcactgccactgttacagcgagcaacagaacaattgcctgaagtcagcgaatattggttagcactggcaatccagtatcgccgatgtaaaaaaacagaagctgcagcacaggctgcgcttaatgcttatcttggcaattgggcatttggtgttcctgacaataaagtcattcatttgctgtcacaggccgcagatgtcccgaatttccaggatgatcctgtgattcagtgcattaaagaacaaggattagatcttagctttggaggaacaaaggaaaataataattaccccttgatgcagatgtgtgttgatacttattttgcgcagagaaaaccgcttcaggcattaaccctgttacataattatgcctggataatgtccagtgaaacgactgcatttcaggaacgctatgattttaatatcgatgaatggcgggcaaaattcaggcagttatgtttagagtattttggcgatagtcgtacacagttcacttaacgctctgcgtctatctactatcccttctttttcagaaaaaccgccgagcatgtcggcggctttctgacttacaaagtaacagattacatcagcggcattgccaaacgcacaatgctaatcagcggttgtggccatacacccagcaccagtaccaacagtgcagagatcagcacaacgataccgcccgcgctgtactgccagtttgatggtgcatcgcgacccggttgttccggggcgtgaagatacaggctcaccgccacgcgcaggtagtagtagaggccgattgccgaaccgacaaccacggcacccaccagccaccacaagtgtgcctggacaccgaccgccagcacgtagaacttaccgataaagcccagcgtcatcgggataccggccagagacagcatcatcaccgtcatcactgccgcgaggatcggacgatgccagaacagaccgcggtaagagaacagggaatcagcatccgggccacgatacgggctggacatcaggctgaccacgccgaacgcgccgaggctgctgaacagataaccggccaggtaaacccctaccgcttccatcgacatctcgccggtttgcagcgcaatcagcgctaccagcagatagccgaggtgagagatagatgagtaaccgagcagacgtttgatattggtctggctcagcgccatcaggttaccgaagatgatggaggcaaaggcgataatcgccagcaccacgcgaatcgcttcgctgtcacccaccggtgcgtagaggaacagacgcatcaccacaccgaagatagcgattttgctcgccgtcgccaggaaagtggaaaccggcgcaggcgcgccctggtatacgtctggcgtccacaggtggaacggcaccagagagagtttgaagccgaggccaacaatcatcaggccgaaacctgccagcaacagcggctcgttgagcataccgtcgccaaggtttttacccaacgcgacaaacgacaggtcgccagactgcgcatacaccagcgccataccaaacagcaggaaagaagacgctgcggcagaaaggatggtgtatttgatactggcttccagtgaacgtttctggcggaaagcgtaaccgaccaggccaaacagcggcaaagagatcagttcgataccgaggaacagagacgccagatggttggcattcgccagcaggatcccgcccagcgcggcaattaacaccaacaggtagaactcatccttgttgtcgttatagccttcaagccacgggtaggcgaaagtacaggtggcgaggctcgccaacaataccagcccggtgtaaagcatggcgaaaccatcaacgcgcatcagcggcgtaacgtccatagcgcccgcctggccaacaaaccagagcgaaaccagcgccgcgttaagcccaataaccgagagcgtagcgttgaggaaatgattgcgtcgccacgcaatggagagcatcacaaccaccaccgtcaagccgacgatcagcaacggtagcagtgcgatcaggttttgtggagttattgtcatggcgatttacggccttgtagtagtaacggaattaacaaaccactgctggatattgccaatcgcggagtgcgaggtatccagaatcggctgcggatagaagcccagcagtaccagcagcaccaccagcaacaggatcataaacagctcacgcagcgacatccctggcagttcctggctggcaatctggcttttcgctttaccgaagtaagcgcgatgtaacatcgccagcgaataaacagatgcaaagaccagcccaaaggtagagataacggtaatcaccggtacaacctggaagctgccgaacagaatcataaattcgccgacgaagttaccggtgccaggcatcccaagcgttgccaccgcaaagaacagcgacagtgctggcagccatttcatcttgctccacagaccgcccatcatgcgcatgtcgcgggtatggatacgttcataaagctgaccacaaagaataaacagacccgccgccgacaaaccgtgcgcaatcatctggattaccgcgccctggtaggccaactggctgccggtgtagatagcaatcagcacgaagcccatgtgggaaaccgaggtgtaggcgatcagacgtttgatatcggtctgggcgaaggccatccacgcaccgtagaagatgccgataacacccagccacatagcaattggcgcgaactctgccgacgcgttcgggaacagcggcagggagaaacgcagcaaaccgtaagcggcagttttcagcaagatccccgcgaggtcaacggaaccggcggtcggagcctgggagtgcgcatccggcagccagccatgcagcggaaccaccggcattttgactgcgaaggcgatgaagaagcccagcattaacaggtattccacaccactggacattggcgtattcagcagctcttcatagttgaaggtccagacgccggtcgcattgtagtgaacaaaaaccagcgccaggatggcaatcaacatcaccaggccactcgcctgggtgtaaatgaagaacttggttgccgccgtgatacgcgttttaccgtcagaggctttatgcccccacagtgcgatcaggaagtacatcggcaccagcatcatttcccagaagaagaagaacaggaacatgtcgatggcaaggaacacgccgataacgccgcccaggatccacatcaggttgaggtggaagaagccctgatatttttcgatctctttccacgaacatagtaccgccagcacaccgagcagaccggtcagcacgaccatcagcagcgacagcccgtcaatggcgagatgaatagagataccaaaacgcgggatccacggcatgtcgaattcagactgccactgcggaattccggcggattgcgtcagtgaataaccgccctgcaaccacagttgcagcgacagcgccagcgtcaatcccatggtgatcagcgcgatccagcgtggcaccttgacgccaaagcgttcggtctgccagcacaggaagccgccaataaagggaattaatattagccagggtagtaacatggcgatctttattccttgtaaaagtcccgtcaggaccggattttcaacgaattctcacgacagaaaattctcttcggactgggggtagtgtcggatgcaccgcgaaggcggcttatccgacctacgttcttatatgcccaggggcaatcccacaatccttaactcaacgcagtaccatcaacagtgccagcaccacgaccgcaccgatgctcatggatgccacataccagcgcagatagccgttctcacttaacagcagacctttacctgcaaagcgggaaaggacagccgggatgttcatcattgagttcagcggatcgcgtttcagcaaccaggcaatacccaggaacggcttgacgaacactttgtcatacagccagtcaaatccccaggcgttgtaccaccaggtgcccagcagacggcccggcgcactgttggcgatggaggtcaccagagtacgtttacccagccacagccaggctgccagcagaatgccgaccaccgcgaccacgccagaggtaatttccagggtcaacatgctgccgtgcgccagttccgtcgtttgcggaagcacgccctgcagcggcggtacaatcagtgcgccaacgaaggtggaaaggatcagcagcacaatcagcggcaggctgtgagttacccctttcacggcgtgagcgtgaatttgttcttttccgtggaagacgatgaaaatcatacggaaggtgtagagcgaggtcataaacgcaccgaccagacctgccaccatcagattgatatgaccattcgccatcgcacccgcgaggatctcatccttactgaagaagcccgcagtgaccagcggtagtgccgacagtgctgcgccgcccaccaggaagcagagataaaccagcggaatagatttacgcagaccgcccatcttgaagatgttctgttcgtgatggcaggccagaatgacggaaccggatgccaggaacagcagcgctttaaagaacgcgtgggtcatcaagtggaaaatcgccgcatcccatgcctgcacgccaagcgcgaggaacatgtagccaatctggctcatggtagagtaagcgagaacacgtttgatgtcggtctgtaccagcgcggcaaaaccggccagcagcagcgtaaccgccccgacaatacccaccagatgcagaacttccggcgtcatcaggaacaggccgtgggtacgggcgatcaggtagacacccgcggttaccatggttgcggcgtggatcagcgcggagacaggcgtcgggcccgccatcgcgtcggcaagccatgtctgcaacggcaactgcgcagatttaccgaccgcaccgcccagcagcatcagcgtcgcccacatcagcatgttattgccgtcagcaaagtgcgctggtgccagttccaccatttcgcggaagttcagggtgcccagttcgttgtaaagaatgaacagtgcgaaagcgaggaacacgtcacccacacgggtcacgacgaacgctttcattgccgctgcgccattcttcggatcggtgtaatagaacccgatcagcagataggagcacaggcccacgccttcccagccgaggtacatcagcagcaggttgtcggcaagcaccagaaccaccatgctggcgatgaacaggttggtgtaagcgaagaagcgagagtagccctcttcaccgcgcatataccaggaggcgtacatgtgaataaggaaacccacaccagtgaccaccgagagcatggtcagcgacaggccgtccagcaccaggttaaaaccgatgttaaagtcgcctaccgacatccacgtccacagcggctggctgtatgtctgctcgccgttagcgaagaaatcaacgccgataaaggcggttaccagcgccgccaggcccacagagcctacgccgacgatcgccgagacgttttcagaccagcgcccacgggagaatgccagcaggacgaagccaatcaatggcaaaataatggttaaggcaagcatgttcatccgcgcatctcacttactgaatcgatgttcaggttctggcgacgacggtgaagttgcagcagcagcgcaaggccgatactcgcttctgccgccgcgaggctgatggcgagaatgtacatcacctgaccgtcggtctggccccagtagcttccggcgaccacgaaggccagcgcggaggcgttaatcatgatttccagaccaatcaacataaacagcagattgcgacggataaccagaccggttaagccaagaacgaataagattgccgcgaggatcagtccatgttgtaaggggatcatgcgtgctcctccgtttttcttttcgcgctgtcgtctttacgattgctcagcacttcacccgcacgctcttcacgaccgacgtggaaggccacaaccagacctgcgagcagcagcatagaagccagttccaccgccagtacgtaaggcccgaacagcgtaatacccactgctttagcactgattggcgtaccgtcgataccctgatcgttaacaccgaggatggcgtaaacaatcaccaccagcatgatggccgacaaaattgccggaccaatccacacctgcggtttcagccactggcgttcctgttcgatttctgaaccgcccaggttgagcatcatcaccacgaacacgaacagcaccataatggcacccgcgtagacgataatttccagcgcaccggcgaagtaagcgcccagtgagaagaacaccccggaaatcgccagcagcgaaataatcaggtacagcagtgcgtgtaccggattggtatgggtgatcactcgcaaggtcgcaagtatggctatcaggccacagatataaaaagcgaactccattgcccctctccttacggtaacaggctcttgacgtcgataggcttggcttcgttctctgcttcgcccttatctttgccgtcgattgccatacctgccatccggtagaagttatattccgggtatttgcccggaccggagatcagcagatcctctttctcgtaaaccagatcctggcgcttgtattcccccatttcgaaatccggggttaactgaatcgccgtggtcggacaggcttcttcgcacagaccacagaaaatgcagcgtgagaagttgatgcggaaaaattccgggtaccagcgaccgtctttggtttctgctttttgcagcgagatacagccgaccgggcaggctaccgcgcagaggttacaggctacgcaacgctcttcgccgtccgggtcgcgggtcagaacgatacgaccacgataacggggcggcagatagaccggctcttccgggtacattcgcgtttcgcgtttggcgaacgcgtgcaggccgatcatccagatactacgaacctgggtgccgaaacctactaacaattcttttaaggtcatggtcttattgccccttattgcgcctgccagagaatgacagccgccgttaccagcaagttgatcagcgtcagcggcaggcagattttccagccgaaggacattacctggtcataacgcggacgcggtaacgacgcacgaatcaaaatgaacatcatcataaagaacgcggttttcagcgcgaaccagatgaatggcggtaacaacgggccttgccagccaccgaagaacagcgtcaccatcaatgcagagatggtcacaatcccgatgtactcacccacgaagaacagaccgaacttcataccggaatattcaatgtggtaaccatccgccagttcctgctcggcttccggctggtcaaacgggtgacggtgacataccgccacgcccgcgatggcaaaggtaataaaaccaaagaattgcgggataacgttccacacatgcgcctggctgttgacgatgtcggtcatgttgaatgaaccggcctgcgccaccacgcccatcaaggaaagcccgaggaacacttcgtagctcagggtctgcgcagaagcacgcatcgcacccagcaacgagtatttgttgttacttgaccagcccgcaaacagcaccgcgtaaaccgccagacctgccatcatcaggaagaacaaaatcccgatgttcaggtcggcaaccacccaacccggactgactggcacaatcgcaaaggccagcagcagcgaggtaaaggcaatcatcggtgccagggtaaagatgacgcgatccgagaatttcgggatccagtcttctttaaagaacattttgatcatgtccgcaaccagctggagcgaaccgccccagccaacacggttaggtccgtaacggttctggaacagacccagcaggcgacgttcgccaaagctcatgaatgccccgcaggtgacaaccaccagcaggatcaccaccgctttgaggatggtcagcaggatctcaatcagttccggtgatatccaactcattgttgtgcctccttgagatcctcaagatgcgcgccagccagcaccggagcaatgccggacatacccatcggcaagcccacctgccctgccgtcagtccttcggcgatttcaaccggcagcgtgaccgtgttgccatcgtaactaaaggagacgcgtgtacctgcgttcacacccaacttcgcggcatccgctgggttgagtttgatgtacggctgcggcatacggctctggaagaccggagcacgctgtgacaattcatcgctgccaaacaggtggtaatacggcgcgatacgccatttcccgtcctgcggctggaagcgtgccggtacgctggtgaagtaatccagaccattttcgctggtttcaaacagacgcacgcccggatcgccaaagcgcagtttgccgcccacttcgtcctggaatttgttccacgcctgcggggagttccagcccggcgcccaggcaaacggcacttgcgaacggtgcgcagtcggctggttgttaccttccatcgagaaggtgaacatggtgtcaatatcctgcggctgacgcggctcatgaacgctgatattggcgcgcatggcggtacgaccgctgtaacggtgcggttcacgggccagtttctgcccacgaatacggaatgtcgcatccggcgcagcatctttgatacctgccagttccgggattttcgccacaacagcgtcaatcacatggtcgagctgcgtccagtccacttcacggctcagcagggtgctgtgcagcgagtgtaaccagcgccagctttccagcatgacagttttgctgtcgtaataagcaggatcgtaaacctggaagaaacgttgggcgcggccttcgttgttgatcaccgtaccgtcgctttcagcaaagctggcagcagaaagtaccagatgggcgttttccataatcgctgtgcgttgatgatcaaccaccatcaccagcggtgctttagccagcgcagcattcacgcggatagcagaagcgtgacgatgcagatcgttttccaacaccaccaccgcgtcggcgcgtccggtttccagttcggttaacgcttcttcaagcgaaccgccacccataatgcccagccccatgctgttgacggaacgggcaatcatggtgataccgacgtcagcgccgcgacctttcagggctttcgcgacgttagccgccgcctgaatcacctctaagctaccggcgttcgtcccggagataatcaacggtttcttcgcacctgccagtgcctgcacgatgacgtcgattttgctttgcagctcaggttcgataccgtcaaccgctggtgcagagttatccagcgcatgggcgatggcaaaacctaaacgcgcctgatcttcaaccggtgcgcggtaagtccacgccgcgatatcatccagacgggtgtcatcaacgttggtaacaaacagcggatgcttcgcacgttgaccgatgttgaggattgccgcaatctgccagtcagccactttctgtgctgccgccatttcgcgcgctttacctttcacagcctgacgcactgccagcgcgacgcgcgcgccggtctgggtaacgtcttcgcccagcaccagtaccgcatcgtaagattcgatttcgcgcagagccggagtataaatgccgccttcacgcagcactttcagcgccagttgcagacgttcctgctcaccgtgagcgataccggtgtagaagttttcttcgcccaccagttcacgcagcgcaaagttgctttccacgctggcacgcggagaaccaataccgatcactttcttcgactgacgcagaatatctgccgcgccctgcattgcctgttcggcgttgagggtaatgaaatcatcgccacgacgctgtactggctgacgcggacgatccttcaggttgacgtaaccgtaaccgaaacgaccacggtcgcagaggaagtagtggtttaccgtaccgttgtaacggttttcgatacgacgcagttcgccgtaacgttcaccggggctgatgttacagccgatggaacattgctggcagatgctcggcgcaaactgcatatcccatttacggttgtaacgctcggagtgcgttttgtcggtaaatacgccggtcgggcaaatttcgaccaggttaccggaaaattcgctttccagcgtgccgtcttccgggcgaccgaagtagacgttgtcgtgcgcaccgtaaacgcccagatctgtaccgtcagcgtaatctttgtagtaacgcacacagcggtagcaggcgatgcagcggttcatttcgtgagagatgaatggccccaaatcctgattacggtgggtacgtttggtgaaacggtagcgacggaagctgtgtccggtcatcacagtcatatcctgaagatggcagttaccgccctcttcacataccggacagtcgtgcgggtggttggtcatcaaccactcgaccacgctttcacggaactgtttcgcttcttcgtcgtcaatggaaataaaggtgccatcggaagccggtgtcatacaggacatcaccaggcgaccacgcgtgtcttccgcgttttggtattgcttcaccgcacactggcggcaagcaccgacacttcccagcgccggatgccagcaaaagtaaggaatatcaaggcccagagacagacaagcttccagcaggttgtccgctccgttgacctcgtattctttgccgtctacatgaattgtagccattagcatgcttccagttttctcagtcagagactgagcgttaatcgaaattcggttaccagcgctctttcagcaggttcggctgaatcccattaatcaaatgggtattgctgaacggctgtttgattcccgcctcaaattcttcgcggaaatatttgatggcgctctgtaacggctccactgcaccaggtgcgtgggcacagaaagttttacccgggcctaagaatcgacacagttgctcaagtgtttcgatatcgcccggctgaccttcaccacgctccagcgcacgcagaattttcacgctccacggcagaccgtcgcggcacggcgtacaccagccgcaggactcacgggcgaaaaactcttccaggttacgcaccagcgacaccatgttgatctcatggtcaaccgccatcgccagcgccgtacccagacggctgcccgctttaccgatactttcgaattccatcggcagatcaaggtgcgcttcggtcaggaagtcagtccccgcgccgcctggctgccaggctttaaatttcagaccatcacgcataccaccggcgtaatcttcgaggatctcgcgtgcggtggtgccgaacggcagttcccacagtcccggatttttcacccgaccggagaagcccatcagcttggtgccagcatctttacttttcgagatgttctgataccactccacgccgttagcgaggatcgccggaacgttacacagggtttcgacgttgttgacacaggtcggtttaccccatgcgccggaggttgccgggaagggtggcttcgagcgtgggttagcacgacgtccttccagggagttgattaacgctgtttcttccccgcagatgtagcgccctgccccggtatggacgaacagttcgaaatcgaaacctgttcccataatgtttttgccaagcagacccgcttcggtggcttcggcaatggcacggcgcagattaactgccgcttcgatatattcgccacgcaggaagatgtagccacggtaagctttcagcgcaaacgcggagatgagcataccttccaccagcaggtgcggcagttgctccatcaacaggcggtctttataggtgcccggctccatttcatcggcattacacagcaggtaacggatgttcatggattcgtctttcggcatcaggctccatttcaggccagtcgagaagcccgcgccgccgcgccctttcagaccagcgtcttttacctgattaacgatttcgtccggagacagcccggtcagcgccttacgcgcgccttcgtaaccgtttttgctgcggtattcgtccagccacactggctgtttgtcatcgcgcagacgccaggtcagcggatgcgtttcgggagtacggataatgtttttcatttataccgctccagcagttcagggatcgcttccggggtcagatgcgcgtgagtgtcctcatcgatcatcatgtttggccctttatcacagttccccaggcagcaagttggcagcagcgtaaagcggccatcaaatgtcgtttgccctggtttgatgttcagctttttctcgagcgccgcctgaataccctgataaccgttgatatgacagaccacgctgtcacaataacggatcacatggcgaccaaccggctggcggaagatctgactgtagaacgttgccacaccttcgacgtcgcttgccggaatacccagcacatcggcgatcgcgtggatcgcaccatccggcacccagccacgctgcttctgaacgattttcagcgcttcaatggacgccgcacgcgggtcttcgtagtggtgcatctcgtgctcgatcgcttcacgctctgccgcactcagctcaaaagcctcggtttgtggttgttgattctcgtgcataattagcggtccacatctgacataacaaaatcgatactgcccagataaacaatcaggtcagacaccaggctgccgcggatcgccgccggaatttgctgcaaatgcgcaaagctcggggtacgaacacgggtgcggtaactcatggtgctgccgtcgctggtcaggtagtaactgttgatccctttggtcgcctcaatcatctggaaagattcattggcaggcatcaccggaccccacgacacttgcaggaagtgggtgatcagggtttcgatatgttgcagcgtgcgctctttcggcggcggcgtggtcagcgggtgatccgctttgaacgggccttccggcatgttgttgaggcactgctcaagaatgcgcagactctggcgcagctcttccactttaagcattacgcgggtgtagcagtcagaaacgccaccacccaccgggatttcaaagtcgaagttttcatagccagaataaggacgcgccttacgcacgtcgaagtcgatcccggtagcacgcaggcccgcgccagtggtgccccactccagcgcctctttcgcgccataggcggcaacgccctgggaacgacctttcagaatggtgttttgcagcgccgctttctcgtaagacgccagacgtttcggcatccagtcgaggaactcacgcagcaggcgatcccagccgcgcggcaggtcgtgcgctacgccgccaatacggaaccacgccgggtgcatacggaaaccagtgattgcttccaccagatcgtaaattttctgacgatcggtaaaggcgaagaacactggcgtcattgcgccgacgtcctgaataaaggtcgagatatacagcaggtgactgttgatgcggaacagttcggagagcataacgcgaatgacgttaacgcgatccggcacggtgatcccggccagtttctctaccgccagcacgtaaggcatttcgttaacgcagccgccgaggtattcgatacggtcagtatacggaatgtagctgtgccaggactggcgttcgcccattttctccgcaccacggtggtggtaaccgatgtctggtacgcagtcgacaatctcttcgccatcgagttgcaaaacgatacggaaagccccgtgcgccgacgggtggttcggaccgaggttgaggaacatgaagtcctcgttttcggtgccgcgcttcatcccccactcttccggtttgaaggtcagggcttccatctccagatcctgtttggctttggtcagctcaaacggcgagaattcggtagcgcgcgccggataatctttacgcagcgggtgacctttccaggtttgcggcatcatgatgcgtcgcaggttcgggtgaccgtcgaaagtaatgccaaacagatcccaggtttcacgctcataccagttagcgttcgggaacagtttggtgaaggtcggtacgtgcaggtcgttttctgccagcgccaccttcagcatgatgtcgcggttacgatcgatagaaatcagatggtagaaaacggaaaaatccgcggcaggtaacccttcgcggtgtgtgcgcagacgttcgtccatgccgtgtaagtcaaacagcatgacgtaaggtttcggcagtttctttaagaaatcgccaacttccagtaattgttcacgcttgatccacacaacgggaaccccggtgcgagtcgcctgaacagtaaaggcatccggcccaaaacggttgcgcagttcgccaatcaccggatcatcaagatgatcgcgggtctgccaggcgggttcttgcgcggttaagtcggtcatattgttcaccattgcaaatggtccgtggtgactgtcggcgcagtaagcttcgcgaaatagatttaggaataagcgaagaaaaatccctttgccgacaggcgcaaattaaatctcgtcaggtgtacgcaggttagttacggcaatgcgttcaccgcgcttgcgttcgcgctctgattgcatattggcgcgataaacgccctgatcgccaaccacccaggagagcggacgacgttctttgccgatagattcctgcaacagcatcagtgcctgcatgtacgcttcaggacgcggcgggcagcccgggatatacacatcaaccgggatgaatttatcgacgccctgcacaacggaataaatatcgtacataccaccagagttggcacaggcacccattgagataacccattttggttccagcatctggtcatacagacgctgaataaccggtgccattttggtaaagcaggttcctgcaaccaccatcaggtcagcctgacgcggcgaagcacgcaatacttctgcgccaaaacgcgccacgtcatgcaccgcggtaaacgaagtcaccatctcaacgtaacagcaggaaagaccgaagttatacggccaaattgagtttttacgaccccagttaaccatgtcattgagcttgcccataaacacgtttttgttaacttcttgctccagagggtcggttacgatctcctgcttttgcagggggtaacggtcgttctcaccgttgggatctatgcgggtgagcgtataatccatcttaatgcctcgcggttagcgttgacgattagcgatactgttcgtttccgggttcatacgctcgcggcgtgaacgcgcgggcgtccagtccagcgcgccaatacgcaccagataaaccagacctgccagtaacacaaaaataaaaattgcagcttccacaaagcctacccagccgctttcgcggatagaggttgaccatgcgaacagatacagcgcttcaacgtcgaagataacgaagaacatggccaccagataaaacttggcggacaggcgtaagcgggcggagccgaccgagtcgataccggattcaaacggcacgtttttcgacctcgcgcgtgcgcgaccgcctaaaaaccaaccgcctaccagcatcaggcaacacaggccaatggcaacgataagaaagatagcgaatgcccagtgatgagcgatgacttcagtggatgttgacatactcattgcttactcatcaaaagtagcgccagattcactgctcttcacggcagatggacgccacatcgattcatggggaggaataaaaaaaaccttacaatcactgtagaaattcttttatacagctaattgatgtggttttttactcctttctataaccttttgtcaactttaacaaaagtttcttcacattagtttacataatatcaacaccattagcatttaatgccctttcaccccagatccttgacgactccaggataattagatgttgttgaatcgtgtccgttgtgaagcaatggaaaaaatacgggtctattttgacaggaatttgtgtcgattcctccccccaaaagagagtattttcttgatctgtgacacgcttttgtcattccataacaaaaacgcagcaacaaatttacgtattttttaacatcattgtagcaggtgatttttttcaggcgattatttgtgcgttcgggacgtgaatctctggtggttgaaaaatgaacagttttgtacgttctgcactatgcgatgaaggatttttactaaaaaaaagccgctggggtttaaaacacccccagcggctcgttttttacactattgtctcaggaattatctatcgtccgtcgattactcgatatccctttcaatcaacaatgaatcatccccttccggagcagacattgggctgtattgccacggattatggtagctctccatcgcctgatagatcacctgggccagctcattattactggacggatcatagcacagcaaatattcggtatcaggtagcggcggtaagccatctactccactcagcacacgcaggtccgggctcatcatctcaaccggccttgccgtcacgccaagaccggctttcactgccgcacgaacggccggaagcgtcgaggcgacataagccagtcgccatggaatatctgctttattaagcgtcgccagcaccatatcgcgaaacgggctaggatcatccagcaatacaagagggatcggctcgcctttttgcaatatgtattccgctgcgcagtaccagtgtgttggcgaggtacgcaggttcaatgccttaaacgctgaaggacgatgggtggttaccatcaaatccacttcctgggattccagcatttctgccatataggcattacgtttaacgcggacatccagcgctaatttcggataaaccgaactcacgcgatttaacaggaaaggtaagatcgtatcggcagattcatctgaagcaccgatagttaatacgccctgaagattactgaacattaatgatgagcaggcctcatcattaaaacgcaggattttcctggcgtaaccaagaagttgaatgccatgttcagttaacagtttgttgcgaccgtgacgagcgaacagttctttcccaacgagttgttccagacgctgcatttgctgacttacggcggactgagtacgacacacagcggcagctgcggcagcaaaagtgttcagatcggcaacagcaacaaatgttctcagcagatcgaggtcgaggttaattatcggacgatttgcacttatcatatattatcacttactggcggctcatactgagctggttaatgctgtgcacacacaaacaagcaattccatttgtaatgtgcctccctggcagtttcatccggaacccggacgaaagtaaaaatgcatatgagttgcactaaaaaagcgactcacattgttccgttataatgcctgaagtagatcacagaatatatcttcagggatcgcatatctattaagttactcactcttttctatttatgacatgcgcgtgtttgtataaatgtaaatgtgagtccttgttccactctcgtgcagcatcgctggtcatacgcgaacacgtaccaacagcaatggtgaggcggcatcaagagcagggatccgtcatttatccgagcattttaccccaaaaaccttttatttataagggtcattgcgaattatctgatgcaaagttatgttatgttaggcaaagtaatcttctattattaataagcacatcaaaacctttttgaatattaaataataattaattagcatcatcctcattcattaattccgcttaacaatagtttcacaccttgcccccattgcgacacctcggaaatcatcacgcagttaaactctccgtaatgaggaaatatcatcatcgcgtttcattagtgaattcttaaatgaggcattttcacacaattatcttacagataaaaaaaccagacttacaattaagaatcagaacaattcactatataacattgcatgtaaagcatatacacctcattattttgtcattattaagttattaacagcacaatcgagccttcccctctggcaaaatcttattctgcagaccttcaaaacaccgtcctgggggagtacattgttctaagctgacttccacggcagggagtggcgataacagcaaaaaaggtcaagattcatgtcccccattgaaaaatccagcaaattagagaatgtctgttatgacatccgtggtccggtgctgaaagaagcaaaacgcctggaagaagaaggtaacaaggtactgaaactgaacatcggcaacccagccccgttcggttttgacgcgccagatgaaatcctcgttgacgtgatacgcaacctgcctaccgctcaagggtattgcgattccaaaggtctttactccgcgcgtaaagccatcatgcagcactaccaggctcgtggcatgcgtgatgttaccgtggaagatatttacatcggcaatggtgtatcggagcttatcgttcaggcaatgcaggcattgctgaacagcggggacgaaatgttggttcctgcaccagattacccactctggaccgcggcggtttcgctttccagcggtaaagcggtgcattatctttgcgatgaatcctctgactggttcccggacctcgatgatattcgcgctaaaattacgcctcgtacgcgtgggatcgttattatcaacccaaataacccaaccggcgcggtatattccaaagagcttttaatggagattgtggagattgcacgtcagcataatctcattatcttcgccgatgaaatttatgacaaaattctctacgacgacgctgagcatcactcaattgcgccgctggcacctgacctgctgaccattacctttaacggactgtcgaaaacgtaccgcgttgcaggcttccgtcaggggtggatggtgttgaacgggccgaaaaaacacgccaaaggctacatcgaaggtctggaaatgctggcttcaatgcgcctgtgtgctaacgttcctgcgcaacacgccattcagaccgcgctaggtggttatcagagcatcagtgaatttattacccctggcggtcgtctttatgagcagcgtaaccgcgcgtgggaactgatcaacgatattccgggcgtttcctgcgtgaaacctcgtggtgcgctgtatatgttcccgaaaatcgacgccaaacgctttaacattcacgacgatcagaaaatggtgttggatttcctgttgcaggaaaaagttctgttggtgcaagggacggcattcaactggccgtggccggatcacttccgcattgtcacgctaccgcgtgtcgatgatatcgagctgtctttgagcaagttcgcgcgtttcctttctggttatcatcagctgtaatcttaatttcactgccggagattgcatccggcagcgttatcccgccacaatgacctgatgatgtcatcatacgtaaggtcactatgaaacagagccatttttttgcccatctctcccgcctgaaactcattaaccgctggccgctcatgcgcaacgtgcggacggaaaatgtgtccgaacacagtttgcaggtagcgatggtcgcccatgcgctggcagctatcaaaaatcgaaaatttggcggtaatgtcaacgccgaacgtatcgctttactggcgatgtaccacgatgcctcagaagtgctcaccggcgatctccctactccggtgaaatacttcaattcgcaaatcgctcaggagtacaaggctattgaaaaaatcgctcagcaaaaactggtcgatatggttccggaagagctgcgggatatctttgcgccgttaattgacgagcatgcatatagcgatgaagaaaaatcgctggtgaaacaggcagatgcactgtgtgcatatctgaaatgtctggaagaactcgcggccggaaataatgaattcttgctggcaaaaacgcgactggaagcgacgcttgaagcgcgtcgcagccaggagatggactacttcatggaaatatttgttcccagcttccatctttcgctcgatgagattagccaggattcaccgctgtaagcagccggagtctgcgtcgcatcaggcaataagcgccggatgcgacatcaggctcttgtcaaaacggaaacagcatcgggatcatcaccacacaaaccgccatcacgataatggtgaacggtacccccaacttcacaaagtcactgaagctgtaatttcccggacctaaaaccagtgtgttaacaggtgaagaaaccggtgtcataaaggcggcggatgctgccatcgccacgaccatcgcgaatggataaggcgacacccccatcgttttggcagcagccagcgcaatcggagccatcaacaccgccgtcgcggtattagagataaatagcccaataaccgccgacaagacaaacaaacaccccagcatcatatgtggcccgtaaccaccgccaatgtccatcagccctttcaccgccagcgcgacacctcccgttttctgtaatgccacagcaaacggcatcatcccaacgatcaaaataatgctcggccagtgaatggatttataggcgctttcagcatctatacagcggaatttccccatcagcaggcaggcgatgatagcggcaacaggattaggaatttcatctgtcagcattaacgccaccattagcaccagacagaaaatggcatggggtgcctggctgtgcgcgggtgatgcttcactcacctcttccggtaagttcagcgctacgaagtcgcggccctgtttggccagcataccgatcagtttccagttacccacaaccaggatgatatcgcccagcagcagaggctcatccgccagcgaaccttccagcgccacgccattgcgctttagccccaccacattcagtccgtagcgggtacgaaaaccaatttcgcgcaccgatttaccaatcagttctgactcaggaattaatgaaatctctgccatgcccacatcaagggcctggtcagaaaaatactcgccgcgcagtaccatcggctccagcaattgctcactacaaaattgccggagatcgacatcagccgcagacatatcaataagcaaaacgtcacgcgcgcgaaattcagaaaccccattaacgttcacgataacgcgacgaaaacgccgccagcgttcaacaccgatgacgttagcgccataacgctcacgtaatttgagatcatccagccgttgaccaatcattggcgatccggggcgaatagccagacgtcgcgcacgcccggtcagtcgatattcacggataagatcgcgaaaggttcgacgcgtccagccttcgcgctgcggggtctgggtatcccctttcagcatgaaacgcatcactaacatatacaaaatacccagcaccagcacgaccaggccaataggtgttacgctaaagaaactgaagccgtgatagccttcacgcagcaattcactgttgactaccaggttcggcggcgtcgccaccagcgtcatcatgccgctaatcagcccggcaaaacttaacggcatcatcagacgtgacggcgacgtttgcatacgcatggcaacgcttaacaccacgggaataaagatagcgacaacgccggttgaactcataaacgcgccaagccccgcgacggtcagcatcaacaaaaccaacattttgatttcactattgcccgcaactttgaccagccatgttcccattacggtggcaacaccggtacggaccaaaccatcgccaataataaacaaggcggcaatcaggacaacgttaggatcagaaaagccggaaaatacttctgggactgtcagcgttccgcttaatgcaaacgcgacaataacaaacaaagcgaccgcatccatacgcactctgcccgtcgcaaacaagacgatggcaacggccagtaatgaaagaacccaaatcaattcaccgttcacaacttatccttgttaattgagggggatgacttgattctgccataaaaaagccccgacgagacggggctaaatcatgatcaggtgtttcactgaataataacatcgccatttggctgtttggtcacagtaatttgctccagactgtggaggaccaaatcgacctcattcaggcgcggggtatctgccggagcgttaaccgcaatgacatgacaacccgccgccaggccagaaagcacgccagcgggagcatcttccaccaccacacactcctgcggcgcaagccccagcagctgcgcgcctaacagatacgcatcaggttctggttttccgcgcttcactcgctcagcggttacaaacacctctggtgcgggaagcccagctattttatggcgcgctcgcgctaccggcatggagccagaagtcacaatggcccacggaatacctgctttattcaaatgactgagtaaggcgattgcccccggaagcgcggtaataccttcggtttccgtggcctcgatgtgctccagacgcgtaaactcggcggcaatatcagcctcggatttgcccgccataaaatggcgcagagaggtgatcgcctgtttaccgtgaatgaaagccagcacctcttccggcgctaacccatgacgtctggcccagttgctccacgcccgttctaccgcaggcagggaatccaccagcgttccatcaagatcaaacagaaaacctttgcaccgcacgcgggcctcctcaggcattgataatttgattaatttcgttggcgctcaaatggtactgacgcgggcaggcatgccacacattaagcatgcgctgatatttttcccacattggcgtctgggcgttaaaaccgtgagttccggcgtcaaaatgggtatagcgcccttccacattaaccataaagcggacataaccgaggtaacgtgcttcagtggcggcgtcaaagccgaggaaggtgacacgacgttcatcgatggattgctggtcctgcaaattagaccaggaaacatgcaacgcatgatacatctccataatgtcgatgatagtgcggcaggtttcttctttcagctcgccaaactcgcgatccaattcacgcatctgtaatccgtaaccacgctcaataattgtttgcaggcgacggtaacgttcagcatttgccggatcgagcatagtcatcatcttgtactgattagacaaaataagacgttgcgcgttggtcatttccattgttgactcctgtatcactctactacggtgaaaaaaaagaaggctgagtatgccttcttttatatgcgtaatcaggggtcaattacaaatcatcaaggaaagttttatccagttgtttgaaggcgcgcttaagcgtgtcagctaatgcctggtaatcaggcttgccttcaacgggtgccaacacctgtccagactcctgcaatttaccgcgaacttcataaaaccagttaaggattgcagggggtaatggcgtgacagaacgcttgcccagccaccacaatccctgcatgggtaaacttaaggcgaacagggcagtggcaactgccggcccaagctgaccgcccagggcaatctgccagcagagagtaaatacggcgatcggcggcataaaacggatcgcataacgcgtcatcttgataacgcgattttcgacaaagaccggggcaaggcgtttttccagcggccacgtctttgagtaatgctgtccccggcgaaacaagctaaaaaaattaacagaacgattatccggcgttgacatgcttcacctcaacttcacatataaagattcaaaaatttgtgcaaattcacaactcagcgggacaacgttcaaaacattttgtcttccatacccactatcaggtatcctttagcagcctgaaggcctaagtagtacatattcattgagtcgtcaaattcatatacattatgccattggctgaaaattacgcaaaatggcatagactcaagatatttcttccatcatgcaaaaaaaatttgcagtgcatgatgttaatcataaatgtcggtgtcatcatgcgctacgctctatggctccctgacgtttttttagccacgtatcaattataggtacttccatgtcgagtaagttagtactggttctgaactgcggtagttcttcactgaaatttgccatcatcgatgcagtaaatggtgaagagtacctttctggtttagccgaatgtttccacctgcccgaagcacgtatcaaatggaaaatggacggcaataaacaggaagcggctttaggtgcaggcgccgctcacagcgaagcgctcaactttatcgttaatactattctggcacaaaaaccagaactgtctgcgcagctgactgctatcggtcaccgtatcgtacacggcggcgaaaagtataccagctccgtagtgatcgatgagtctgttattcagggtatcaaagatgcagcttcttttgcaccgctgcacaacccggctcacctgatcggtatcgaagaagctctgaaatctttcccacagctgaaagacaaaaacgttgctgtatttgacaccgcgttccaccagactatgccggaagagtcttacctctacgccctgccttacaacctgtacaaagagcacggcatccgtcgttacggcgcgcacggcaccagccacttctatgtaacccaggaagcggcaaaaatgctgaacaaaccggtagaagaactgaacatcatcacctgccacctgggcaacggtggttccgtttctgctatccgcaacggtaaatgcgttgacacctctatgggcctgaccccgctggaaggtctggtcatgggtacccgttctggtgatatcgatccggcgatcatcttccacctgcacgacaccctgggcatgagcgttgacgcaatcaacaaactgctgaccaaagagtctggcctgctgggtctgaccgaagtgaccagcgactgccgctatgttgaagacaactacgcgacgaaagaagacgcgaagcgcgcaatggacgtttactgccaccgcctggcgaaatacatcggtgcctacactgcgctgatggatggtcgtctggacgctgttgtattcactggtggtatcggtgaaaatgccgcaatggttcgtgaactgtctctgggcaaactgggcgtgctgggctttgaagttgatcatgaacgcaacctggctgcacgtttcggcaaatctggtttcatcaacaaagaaggtacccgtcctgcggtggttatcccaaccaacgaagaactggttatcgcgcaagacgcgagccgcctgactgcctgatttcacaccgccagctcagctggcggtgctgttttgtaacccgccaaatcggcggtaacgaaagaggataaaccgtgtcccgtattattatgctgatccctaccggaaccagcgtcggtctgaccagcgtcagccttggcgtgatccgtgcaatggaacgcaaaggcgttcgtctgagcgttttcaaacctatcgctcagccgcgtaccggtggcgatgcgcccgatcagactacgactatcgtgcgtgcgaactcttccaccacgacggccgctgaaccgctgaaaatgagctacgttgaaggtctgctttccagcaatcagaaagatgtgctgatggaagagatcgtcgcaaactaccacgctaacaccaaagacgctgaagtcgttctggttgaaggtctggtcccgacacgtaagcaccagtttgcccagtctctgaactacgaaatcgctaaaacgctgaatgcggaaatcgtcttcgttatgtctcagggcactgacaccccggaacagctgaaagagcgtatcgaactgacccgcaacagcttcggcggtgccaaaaacaccaacatcaccggcgttatcgttaacaaactgaacgcaccggttgatgaacagggtcgtactcgcccggatctgtccgagattttcgacgactcttccaaagctaaagtaaacaatgttgatccggcgaagctgcaagaatccagcccgctgccggttctcggcgctgtgccgtggagctttgacctgatcgcgactcgtgcgatcgatatggctcgccacctgaatgcgaccatcatcaacgaaggcgacatcaatactcgccgcgttaaatccgtcactttctgcgcacgcagcattccgcacatgctggagcacttccgtgccggttctctgctggtgacttccgcagaccgtcctgacgtgctggtggccgcttgcctggcagccatgaacggcgtagaaatcggtgccctgctgctgactggcggttacgaaatggacgcgcgcatttctaaactgtgcgaacgtgctttcgctaccggcctgccggtatttatggtgaacaccaacacctggcagacctctctgagcctgcagagcttcaacctggaagttccggttgacgatcacgaacgtatcgagaaagttcaggaatacgttgctaactacatcaacgctgactggatcgaatctctgactgccacttctgagcgcagccgtcgtctgtctccgcctgcgttccgttatcagctgactgaacttgcgcgcaaagcgggcaaacgtatcgtactgccggaaggtgacgaaccgcgtaccgttaaagcagccgctatctgtgctgaacgtggtatcgcaacttgcgtactgctgggtaatccggcagagatcaaccgtgttgcagcgtctcagggtgtagaactgggtgcagggattgaaatcgttgatccagaagtggttcgcgaaagctatgttggtcgtctggtcgaactgcgtaagaacaaaggcatgaccgaaaccgttgcccgcgaacagctggaagacaacgtggtgctcggtacgctgatgctggaacaggatgaagttgatggtctggtttccggtgctgttcacactaccgcaaacaccatccgtccgccgctgcagctgatcaaaactgcaccgggcagctccctggtatcttccgtgttcttcatgctgctgccggaacaggtttacgtttacggtgactgtgcgatcaacccggatccgaccgctgaacagctggcagaaatcgcgattcagtccgctgattccgctgcggccttcggtatcgaaccgcgcgttgctatgctctcctactccaccggtacttctggtgcaggtagcgacgtagaaaaagttcgcgaagcaactcgtctggcgcaggaaaaacgtcctgacctgatgatcgacggtccgctgcagtacgacgctgcggtaatggctgacgttgcgaaatccaaagcgccgaactctccggttgcaggtcgcgctaccgtgttcatcttcccggatctgaacaccggtaacaccacctacaaagcggtacagcgttctgccgacctgatctccatcgggccgatgctgcagggtatgcgcaagccggttaacgacctgtcccgtggcgcactggttgacgatatcgtctacaccatcgcgctgactgcgattcagtctgcacagcagcagtaatctcgtcatcatccgcagctttgcgctgcggatatctgaaccggaaataatcactatttccggttttttattctcttaatttgcattaatcctttctgattatcttgcttaactgcgctgcatcaatgaattgcgccatcccactttgcatacttaccactttgttttgtgcaagggaatatttgcgctatgtccgcaatcactgaatccaaaccaacaagaagatgggcaatgcccgatacgttggtgattatcttttttgttgctattttaaccagccttgccacctgggtagttccggtggggatgtttgacagtcaggaagtgcagtatcaggttgatggtcaaacaaaaacacgcaaagtcgtagatccacactcatttcgcattctgactaacgaagcaggcgaacctgagtatcaccgcgtacagctgttcacgacgggcgatgaacgcccgggcctgatgaacttcccgtttgaaggattaacctcaggatcgaaatacgggacagccgttggcatcatcatgtttatgctggtgattggcggcgcgtttggcattgtgatgcgtacaggaaccattgataacggtatcctggcgcttattcgccatacccgcgggaatgaaattctctttattcctgcgctgtttattctgttttcacttggcggcgcggtatttggtatgggagaagaggccgtcgcctttgccattatcatcgcaccgctaatggtccggctgggctatgacagtattaccaccgtcctggtgacctatattgccacgcaaatcggttttgccagttcgtggatgaacccgttttgtgtggtcgttgctcaggggattgccggcgttccggtgctttctggctccgggttgcgcatcgtggtgtgggttatcgccactctgattggcctgatctttaccatggtgtacgcctcacgagtgaaaaagaatcctcttctgtcacgcgtgcatgagtccgaccgcttctttcgtgaaaagcaggctgatgttgaacaacgtccgtttacctttggtgactggctggtattgattgtcctgaccgccgtaatggtctgggtgatttggggcgtgatcgttaatgcctggtttattccagaaattgccagccagttcttcaccatgggtctggtgattggcatcatcggcgttgttttccgccttaacggcatgacggttaataccatggcttcatcctttaccgaaggggcgcgaatgatgatcgcccctgccctgctggtgggtttcgccaaagggattttgctgctggtcggtaatggtgaagcgggtgatgccagcgtgttaaataccatcctcaacagcattgccaatgccattagcggtctggacaacgcggtcgcggcctggtttatgttgctcttccaggcggtatttaatttcttcgtgacgtccggttctggtcaggcggcgttaaccatgccgttactggcaccgcttggcgatctggtcggtgttaaccgtcaggttaccgtgctggcgttccagtttggtgatggcttcagtcacatcatttacccaacctcagcgtcgttaatggcaacgctcggtgtgtgcagggtggacttccgtaactggctgaaggtgggcgcgaccctacttggactgctgtttattatgtccagcgtcgtagtgatcggcgctcagttgatgggctaccactaaaaatgttaagagccgcaattgcggctcttttttcattctgccgtttcagtctctacggcttcatttttggcattgcgcttcatccacaacgctagcgctttcagcgagtctggagtgaactcatcgcagcgtgcggtgatttcttccggcgtcagccagcaaacttcactgacttcatcttcctgtagtgcgaagggaccgtgagagacgcagctgaacaatgcgccccagacacggcaatttttatcttcgaaatagaactgcccgtgctcggcaaaggggacaccggcaatgcccaactcttcttccgcttcgcgacgcgcggattccagcagttgctcatcggcctggactacaccgcctgcggtcgcatctaacatgccgggtaaaaagtcttttgtctcggtacgacgctggaccagaattttgcccatgccatcatgcacgacgatgtaagttgcacgatgacgcagacactgtgcccgcatttgttcccggctggcttgtgcaatgacttcgttctcttcattgacaatatccacccattcagtacttgccaaacgacgctgttccattatcaggaaaccttctttttctggcgctcttacggcgcattttgagttgtgggtaaattacggattaatcgcgacctgcgcaatgatactttgatcattgagtgcgattacactaagtacgtcattatccagcatgccataactcgccggattaccgcctttcggaatactcaccgagccggggttgaagtggaaaatctccccccgctgttctgccactggcagatgggtatgaccgtacaccagcacatcgttctggtttaaagcaggcagattttccgggccaaaaagatgaccatgcgtcaaaaacagacgttgtttttccagtaatacctgttgccacggcgcggttatcgggaaatgcagcagcatttgatccacttcgctgtcgcagttgccgcgcacagcgataaccttatgtgccacttcattaagccgttcagcgactttggctggcgcgtaaccctccggtaaagcattacgcgggccgtgattcaacacgtcgccaaggatcaccagccactgggcaccgctttgggcaaacaactccagaacacgttccgtcgccggtaacgacccatgaatgtccgatgcaaacatcagtttcatcactcactcctcgtcgaaaaaacgtaagctatgatactggattctgtcgttgctatcagccagattgcttcgccgaaagtgcaataaaacgctggacagacgctcgctgccactggaatgttgcataatccaccaggcgttctggcacctcatcgccatgtagtaccaggcggttaatcattagcgccagatcagtatcagcaatgcaccattcaccaaataaattcggctgacccagtactaacaaatgttctgccatcgcgaacagtttctctgcactggcttttccctcggccgttagtggcgcttttttcgcccccgcaaagacaacatccgtcggacgctcttcgcggatgggcatcagatcgctgcgcagccaggcctgaatctgtcgtgcacgcgcacgattttctaaatcaagcggataaatacgttcccaggtcggtggcgcaaatcgatcttccagatactccgcaatggcagaagattcactcaactcaaaatcatcgatttgtaataacggcacacggcgtgtctgaccgtaaccttgccacgtcggctgcaaatgttcaccgctgtcgaggtcgatggtcttgatatgaaacgacaggcctttttcctgcaacgccacccaggcggataacacataaggggagaaaaagtgggcatctgaccaaagcgtgatagcgggtttactcattatgtcctcggcaataaagggggctggctatcaaactatagagcctttttgtcactgtcacgtgacgaatactcacgtaagtcgccgcgctttctatacttgtggtgttcagatgattaaacaaccggagctgcaatgatcgatctctatttcgccccgacacccaatggtcacaaaattacgctgtttctcgaagaagcagagctggattatcgcttgattaaggtagacctggggaaaggcggtcagtttcgtccggaatttttgcgcatttcgcccaacaacaaaattccggcaattgttgatcattctcctgccgatggcggcgaaccgctaagcctctttgagtctggtgccattttgttgtatctggctgagaaaacaggactctttttgagtcatgaaacgcgtgagcgcgccgccacattacagtggttattctggcaggtaggcggactggggccgatgcttgggcaaaatcatcattttaatcacgcagccccccaaaccattccttacgctattgaacgttatcaggttgaaactcagcgtctttaccatgtactgaacaagcggctggaaaactcgccctggctgggaggcgagaactacagcattgcggatattgcctgctggccgtgggttaatgcctggactcgccagcgaattgacctagcaatgtatccggcagtcaagaactggcatgagcggatccgttcgcgccctgccaccgggcaggcactgctaaaagcacaactcggtgatgagcgttcggatagttaacagaaacaggttctcgtgtattatttcatcctaagtaaaacaacggagaacctgcaatggcacaacctgccgctattattcgtataaagaaccttcgtttgcgtacgtttatcggaattaaggaagaagaaattaacaaccgtcaggatattgttatcaatgtgacgatccactaccccgccgataaagcgcgcactagcgaagatatcaacgatgcgctgaattatcgcaccgtaacgaaaaacattattcagcatgtagagaataaccgtttctctttgctggaaaaattaactcaggatgtgctcgatatcgcacgtgaacatcactgggtgacgtatgctgaagtggagatcgataaactgcacgcgctgcgctacgccgattcggtatccatgaccttaagctggcagcgttaatcgccatatcgggaggctgcatgaacatagtgatcaccggagggacaggattaattggtcgccatttgattccgcgtttgctggagctgggccatcaaattacggtagtgacgcgtaacccgcagaaagccagttccgttctcggccctcgggtgacactatggcaagggcttgccgatcaaagcaacctcaacggcgttgatgcggtaatcaacctggccggagaaccgattgctgataaacgctggactcacgagcaaaaagagcgtctctgccaaagccgctggaatatcacgcaaaaactggtcgatttgattaatgccagcgacacgccaccgtcggtactcatttccggctcggcaacgggctattatggtgacttaggtgaagtggtggttaccgaagaggaaccgccgcataacgaatttacccataaactctgcgctcgctgggaagaaattgcctgccgggcgcaaagtgacaaaacgcgagtgtgcctgctgcgtaccggtgtagtgctggcaccggatggcggtattctcggtaaaatgctgccgccgtttcgtcttggcctgggcgggccgattggctctggtcggcagtatctggcctggattcatattgatgatatggtcaacggtattctctggctgctggataacgagctgcgcgggccatttaatatggtttcgccctacccggtacgcaatgaacaatttgcccatgcgctcggtcatgcgctgcatcgcccggccattttgcgcgtccccgcgaccgccattcgactgttaatgggcgaatcttcagtactggtattaggtggacaacgcgcgctgcctaaacggctggaagaagcgggttttgcgtttcgctggtacgatttagaagaggcgctggcggatgtcgttcgctgatgtggtttacagcaaacatccgccagttaactcccggtgttacaggattagtggctttgcgcgataagatcgtctggtgaaagtcgggtcaccatcataactaactctctgtctaaacctctatccagcatctcctgagcaatacgcagggcttcttcgtgtttgccctgcattgcgccttcttcacgtaatctgtcagcaatggtcatcagtttctccttttcttgtggtgcgcgttccgctatctcaccaataaatgcacgaaaacgctgggcatcccctgtttgtaatacgtaattaaacagggcttttagctgtctgtcattagtgttccctgtaactagcagcgaaacaatttggtcgactaatcccaacagatcgcgctgacgaatatgtttctgaattaactccaacagcgccattttgcggtgttgcataatctcgtcatccggcaccacggtaatatccaccaacggaaaagccgatgaatatattttgcgggctatagcaggctcggcaaattcatcaagccagcagagtgaataaggataaggacttctgcaaccatgataaaacagcatcgggagcaccaatggaagctctttatagcccgcatcaagatggttttgcattgccgcaatggaataacgcatcatgcgaaaagccattaattcttccggcttactttggtgctctatcactacataaatataacccactccctcctgcgttttcacagaccacaagaggtcggaataatattgccgcaggtcttcatcaataaaactgtttggttccagtttaagcgtcgttaaatcacacagtttgcgcagcggcgcgggaagatgaatatcaataaaatcccgcgcggtgtctggatggcgtaaaaaagatttaaataccgcatcatgcggcgtggaagttgtcgatattgtcatggcgttccgtcacccctcaaatttaagatgacgcgacaataaccacgattaacacccaatgcagcaggcagtttttatctttggacagcgaattcagaagtatttttagcggactgtaacttttacatttcagcggaagctgactcgcaaattccccatgaaaatactccggcagcgttagccaccggagaggaaattatttcagcgatcccttaaggaaccgttgcagacgagggctttgcgggttgccaaataactgctccggcgcgccctcttcttctattttcccctgatggaggaaaatgacatgagtagaaacatggcgagcaaagcccatttcgtgagtcactaccaccatggttttcccctcttctgccagttgctgcataatacgcaacacttcgcctaccagttcaggatcgagcgccgaggtaggttcatcaaacagtaaaacttccggttccatcgccagcgcccgcgcgatagaaacacgctgttgctgaccgccggaaagatgcaccggatatttcccctgcgcacgttcgtctatcccgacttttgccagatacttcaccgcccgctcgcgcgcttcctgcttgctcaggcccaacacctgaatcggcgcttccatgacgttttccagcaccgtcatatggctccagagattgaagtgctggaataccatcgtcaggcgtgtgcgcagtaagcgcagttgatttttatcggcgactttgagttgaccgtctttgtcgcgcaccagattgatcgtctggccattgaccacgatcgacccttcactcggtttttcgaggaagttaatgcagcgcagaaaggtacttttccccgatcccgacgatccgatgatgcttattacatctccggcattcgcttgcagtgatacccctttcagcacttcatgttcgccgtagcgtttgtgcaaatcgataacgtttaatttattctcggacatcgtattctcagtgcgttgaagaaggtttcacatgctgcaaccagcgtttttccgctctgcgaaagaggctgatcaggacataagagatgattaaatagagcaccgcggcaatgccgaaggcggtaaaaggttgatacgtggcggcgttaatatcgcgggctattttcagcagatccggcaccgtggcagtaaatgccaacgcagtagagtgcagcatcaggatcacttcgttgctgtatgccggtaacgcaatacgcagcgcagaaggcaaaataatgcagcgatacattttaaaagtcgagaagccataggctctggcggcttcaatttccccatgcggaaccgaacggattgccccagcaaaaatctcggtagtgtaagcgcaggtgttaagcgtcagcgccagcacggtacagttcaggccactgcggaagaaagcgttaaggaattcggttcccttaacaatctcaagcgtgtacatgccggaatagaacaccagcaactgaacatacagcggcgtaccgcgaaaaatataggtaaataaccagattggaaactggatgtatttattactggagacacgaccaatcgccagaaacagcgccaggactccgcctatcactaccgacaaaataagcagccacagagtgatcgccacaccagtaaagcgataaccgtcggtccacagcagcggtttccagtattcatgtaagatttcgatcacaggtcagccctcttcacacccacggagtagcggcgctcaaggaacagcagcacaccattggaaacagtggtgaaaaccaggtaaatcacgccacagacgatggcgaaatagaacggttcccaggtacttttgcctgccagttgggtggctttgaccacatcttccaggccgagtaacgaaaccagtgcggtagatttgaggatcacctgccagttgttgccaatgcctggcagggcgtaacgcatcatcgacggaaacatgatccgccgaaacacttgcccacgagtaaaaccgaacgccgtcgccgcctctatatgtcctttcggcactgccataaaagcaccacggaacgtttcggtaaaataagcaccgtagataaaaccgagagtgataataccagcgaccatcggatcgatatcaatctgcccgacgcccatcgcctccgtcaccgtgtttagcgcaatctgcaaaccgtagaaaatcagcagcatcaacactaagtccggcacgccacgaatcagcgtggtgtacccttcgaaaatcagccccgaaagccgattttgcgagagcttaccgccagcgccaattaaaccgatgattacagcgagcactacagagctgatagccagctccagcgtgacgagcgcaccctgtaaaataacacctgaaaacccatacaacatgctgcctgtcctgtcgtgtgtggtgaattaccgcctcttgtctccctccggttacccgaagggagcgggctttctttcaccgatggcgattagccaccataaacatcaaaatcgaagtactttttcgctaatttctcgtaagtaccgtcagcgcgcatttcggcaaaggctttgttcagtgcttcgcgcagttcgttatcttctttacgcaggcccatgccggtccctacgccaaacagtttttcatctttaacagacgggccaccgaatttgtaatctttaccgacaggttgtttgaggaaaccttcgctggcagcgacctcatcctggaacgcggcatcaatacgtccggcagtcaggtcagaataaatgttgtcctgcccctgatacgagacgatttcaatgccttttggtgcccaatgttcattaccgaacgtctcctgggtggtgccctgcaatacgcctacccgtttgcctttcagcgactcgactgtcggctgaatgtcagaatttttcgccaccaccaaacgagaatcggcagcgtacagtttgtcggtgaaggctatttcttgctgacgtttttccgtaatggaaagcgatgacatgatggcgtcaatcttcttcgcttttaaggacgggattaacgcatccagcggattttcgacaaacgtacattgcgtattgatgcgtttgcataattcctttgccagatcgatatcgaagccaaccagttcgccttgtgaattttttgattcaaatggcgcataggtcgggtcggtaccgatgcggatgttttgcggaatcgcagcaaacgccgcagttgcgctggagaaggccagaaccagagagagcgatagcaccagttttttcataatgtcctcaactgacagtctttttatagggaatatttacaggtttgttacacttatcgtgccataaaattgaccatcaaggcaaaatatcccgccccgttagacgtattatttttcattaaaaatgcttaagtatgcatttcaatgcaccacgatagtgcaacaaacctggcgtgcaccatgatgatcattccatcaggtacagcttcccagcgacgtatcagtcaccgtagacattaaagtcgaaatactttttcgccatcttgtcgtaggtgccgtcctgacgcagctcgccaagcgccttattgaaggcagccgtcagttcagcatcatctttacgtagccctacaccggtgccatcaccgaagtattttttgtcttttactgatgagccagcaaaggcgaaatctttaccagcaggttgcttgaggaatccttcgctggcagcaacttcatcttgtaacgcagcatccagacgtcctgcagccagatcggaatagaccaaatcctggttggcataggccaccacatccacgcctttactacgccaggtctcgttagcgtaagcttcctgggttgatccctgcagcacaccaacatgtttacctttcagtgaatccagcgttggctgaatcggtgaacctttggccgcaatcaaacgagaatctgcggcgtacagcttgtcggagaaggcaatctcctgctgacgtttatcggtaatggaaagcgacgaaataatagcgtcgatttttttcgctttcagtgaggggatcagcgcgtcaaagtcactggcaacccaggtacatttcacctgcatccgtttgcacatctcgttaccgagatcgatatcaaagccaacaaaatcacctttagcatctttcgatgagaacggtgcgtaggtggtatcggttccgatacgtaccgtctccggtagcgccgcatagctggaagccgctgtggagagaccgactaacaaagacagagcgagaatcgacttcttcatacataaccctcaagtgaaaatggcttttttatgttgtgtattgtgttgtgtgtttgcaggctctttcatgcaggtcttatgccatcttgacgacaacagtaacattcaacgttaaatatgttaataagacgttgcattattgtcctgaagttgaagatagcaggtatagcggttgaatcgcagcgtttcgattgaatggcagaaacaaaatgtcgaggatttgatcgcggttgcaaaattgccctgaaacagggcaacagcggagttatgcgccctgccagcgggcaaagagatcttcaggaagggttatcgcaaactggtcaagaacacgattaaccgtctgatttatcacatcatcaagggattgcgggcgatgataaaacgccggaacgggaggcataatcaccgcaccgatttctgccgcctgagtcattaaacgcagatggcctaagtgcaatggtgtttcacgcacgcagagcaccaacgggcgacgctctttcagcaccacatctgccgcacgggtcagtaagccatcagtatagctatggacaatgccggaaagggttttgattgaacagggtaaaatcaccatccccagcgtctggaaagaaccggaagagatgctggcggcaatatcgcgcgcatcgtgcgtgacatcggctaatgcctgcacttcgcgcagagaaaaatccgtttcgagggataaggtctggcgcgctgcctggctcatcaccagatgcgtttcgatatctgtgacatcgcgcagaacctgtaataagcgcacgccataaatcgcgccgctggcaccgctgatgcctacaatgagtcgtttcataaatagttgccctgtcagacttgcaggcagactttgcaggatttcggcgggagttgcaagtcagggtgccagaccggcaccctcagcgaaggcatcatccttcgttatgcatttcgagattttccacttcgttctgacgttgcactgctttggcgtcatcattacgtaacgtatcgaggaaatcgaggtagccctgatcaacatctttggtgacgtagacgccgttgaacaccgagcattcaaactgctggatatccggattttcagcgcgaacggcgtcgatcagatcgttcagatcctggaaaatcaacccgtcagcaccgatgatctggcgaatttcatcaacttcgcgaccgtgagcgatcagttccgtggcgctcggcatatcaataccataaacgttcgggaagcgaatttccggtgccgcagaagcgaggtacactttcttcgctccggcttcgcgtgccatctcgataatctgctcagaagtggtgccacggacgatggagtcgtcgaccagcaggacgtttttatcgcggaactcggcgcggttggcattcagtttacggcgcacggacttacgacgcagctgctggcccggcatgataaaggtgcggccaacatagcggtttttaacgaagccctggcggtacggtttgcccagaatacgagcaatttccagcgcgatatcacacgaggtttctgggatcgggatcaccacgtcgatatccagatcttcccattcgcgggcaattttctcgcccagtttcgtgcccatattcacacgcgcgctgtaaacggaaattttgtcgataaacgagtccgggcgggcaaagtatacatactcaaacaggcacggattgctgaccggattgtcagcacattgacgggtaaacaactgcccttcttcagtgatgtaaatcgcttcgcccggcgcgacgtcacgcaggaaatcaaagcccagcgtatcgagcgctacgctttcggaagcgaccatatattctgtacggttctcgtcaatatcacgttttcccagtaccagcggacgaatcccgtttggatcgcggaaagcaaccataccgtggccgataatcatcgccacacaggcatacgcgccgcggattaagcggtttgtggcagcaatggcagcgaaaatattgtcggcttccagcgggtagtggcggaagttgtccagctcgctggcgaagatattaagcagaatttccgagtcggaagtggtgttgatgtggcggcgtttttcttcaaacagttttttacgcaactcgtgagcgttggtcagattgccgttgtgggcaagcgtaatgccatacggggagttaacgtaaaacggctgcgcttcagaggcgctggagctgccagccgtggggtaacgcacatgaccaatgcccatattgccctgcaaacgctgcatatggcgagcttcaaatacatcgctcaccagcccgttcgctttacgcaaacggaagcagttattggcatctatggtgatgatgccggcggcatcctgaccgcgatgctgaagcaccgttaaggcatcataaatcgactggttaaccggcataacaccggcgataccgacaataccgcacatacgtctttttcctcgttaagccacatctcagagcacttacgctctgggcaagaaacttgacgagctttgcagataatcaaaaaaacatctgatgataaaactgaattgcgggatcagctgtgatttgctccagtcttcgcttttcgacaccccggtaaaggagtcgagaaagaagagaatggcagcaacaatcaacacaccgcgcaacgcaccgaaacagacgcccagcacccgatcggtgcctgacaaccccgttttctccaccaactggcctatcacgaagttcacgatagcaccaacgatcagggtagcgataaacagtaccgcgatggcaatcccatttcgaaccagttcgtcttcaaagcccgtaaaccagactgacaggtaagtgtagtaatgactggcaacaaagaaagcacaaccccatgtcaccagcgataacgcttcacgaacaaagccgcggatcaggctaaccagagaggaaaaagcaatcaccgcgattatggcgtaatcaatccagaccatatgtgtcccacgattttacgccctgtcatcctgttcggggcgcattctaacagaaaaagaaaacgtttgcgtagggatttccttcccgcgcatcaataaaaatggcgctgaaaaaatattcaacgccatcgactttttatgcctttgcggcatcgggcaatgcgtgtcggatgcggcgtaaacgccttatccgacctacggttctacccctgcgtaggcctgataagacgcgccagcgtcgcatcaggcaagaccgtattaattcggcgtatagcccattaccacgccacttaagccagaaagttgcttcaactcacccagcgaacctttcagcttatctttcgaggcatccggcccaaccagaatacgggtaattttaccctgcactggcgtggatggcgacgtataaacccgataaccggcaccgcgcagcttaccgacaatctcattcactttatcggcatttttcagcgcacccagttgcacaacataggctttacccgtcggtgcagctttttcttccacgaccggcttcggttctggcttcggcgcaggtggtgcttcaacctttggtttaggcggctccaccggtttcggcttcggtggggcgaccggtgcaggttccggttcaaactcggtgttattggctgcaatagtggccggatcgagcgacggtgctgcggcatcacctgcccgcacctcttccgctgcgccttccggcggctgcgtcggtaacgcctgggtggcggctggcatcatatcaggctcatcacgatcgcccgctttcggcaccagcgggatagccgcgaactcatcctgataatgttttttctgcccgtccagcagccctggaagtacaatcacccccagcgccaccagcacgatcgtgcccactaaccgattctgaaacttacttgccaccgcttctcctcgcgtcaatcacttccatgacatgtgcgaccgtgtggaaagaaccacacaccagcacggtgtcttccgctttagcgtccgccattgcggcatcccatgcctgcgcaacgctatcaaatgatttgccgttacccaaatgctcaagcagttgttctgccgtggcaccgcgcggcccttccagtggcgcacaataccagtcatcaaccacgcttttcaaccaggccagagttccggcaatatctttatcatgtagcataccgataaccgccagcacgcgcccgtttttcggtagcgctttcatacgcccggtgagatattccgccgcatgtggattatgcgcgacatcaaaaataacgcgtggcgactcgctcacaatctggaaacgtcccggcaaaattgcgctggcaatcccgtcgcgaatggcattttcactgacttccagcccgctggcacgcagtgccgccagcgctgttgcggcattcggttgcgggacaagcggcaacggcagattttccagcgtgccgtgagcatcgctaaacgcccagtcatgatcggtgacggaatagttccactcaacgccccgacgttgtaacagtgcacctttttcctgcgccacatcagcaatggtagaaggcatttccggctcaccgacaattgccggtttttcgctgcggaagatgcctgctttctcgcgaccaatactttcgcgatctggacccagccagtcggtatgatccagcgcaatactggttactaccgcgacatcggcgtcgacaatattggttgcgtccagacgaccgcccagccctacttccagaatcaccacgtcaagttgtgcctgcttgaacagccacaacgccgacagcgtaccgtactcgaaataggtcagggaaatatcaccgcgtgccgattcaatctccgcaaaagaggcggtgtgggccgattccggcaattcctggccctgcacacgtacgcgctcggtataacgcaccagatgaggcgaactgtagacgcccactttgtaccctgccgccatcagaatcgactccagcgtacggcaggtggtgcctttgccattcgtacccgcaacggtaaacacaaatggcgctggtttcaggacgccaagacgcgccgcgaccaggctcacgcgctcaaggccgagatcgatagttttactgtgcaggttttccagataagaaagccacgaagccagaggcgacgcggcttgaggagtgcgtttgataatcatggtatccgctgattcgttacggtgagaatagcaaaagggcagagccagtggccctgcccttatcagttatcaggcctcaggttcctgatccggtaccgggggtaccactacgccttcacgcggcgcttcaggattcggcgctggcagattcatcaacttcgccagaatgctcgccagtttcaggcgcatttccggacgacggacgatcatgtcgatcgcgcctttctcgatcaggaattcactgcgctggaatccaggcggcagtttttcgcgaacggtctgttcgataacacgcggaccggcaaagccgattaacgctttcggttcagcgatgttgagatcgcccagcatggcgaaacttgcagaaacaccgcccatcgtcgggtcggtcagcacggagatgtacggcaagccgcgctcctgcatttttgccagtgccgcagaggttttcgccatctgcatcagcgacatcagtgcttcctgcatacgtgcgccaccagaggcggagaagcagatcagcgggcagttatcttccagcgcctgctcaacggcacgcacgaaacgtgcacccacaacagaccccattgaaccgcccataaaggcgaactcgaatgccgcagcgacaaccggcattccatacagagtgcctttcatcaccaccagcgcatctttttcgccggtttctttctgcgcagatgccagacggtctttatacttcttggagtcacgaaacttcagcacatctttcggctcaagctcgctacccagctccacaaggcttccttcatctaacaggctatgcaggcgattacgcgctgtcatacgcatgtgatggtcacacttcggacagacctcaagattacgttccagctcagcgcggtataaaacctgaccgcagctatcacacttagtccacaccccttcaggaatgctcgccttgcgggtgggagtaatgttgcttttaattcgttcaatccagctcattagggacctttctgtctgaacctggttcgatgccagttttatctttggggacgcataatgccatttttgcccccaacagaccatgaatgttgcacattaaaacataacagcccgaaactttggataaaaaagtggtcgaaccgcggagttactttttattttgcggcgcgtgccgcagcgcgtttgtgacggattatttcgatgacgcccggcaaaatagaaaccacaataatcccgacgatcagcagcttaaggttatcctgaaccatcgggattgtaccgaagaaatagcctgcgtaggtaaaaagcagtacccacaacagtgcgccgatcacgttataagcggcgaaatgacggtacgacatgtggcccattcccgcaacaaacggggcgaacgttctgacgatcggcacaaaacgggcgagaataatcgttttgccgccatgtttctcataaaactgatgggttttgtcgagataactgcgacggaaaattttcgaattgggattactgaacaacttttcaccgaacaaccgcccgatagtgtaattgaccgcgtcacccacaatcgcggcgatcagcatcagcaccaccatcatatggacgttgagatcgttggtttccagtgatgccaacgctccggcaacaaacagcaatgaatcacccggtaaaaacggcgttaccaccagaccggtttcacagaacaaaattaagaacaaaatggcataaacccagacgccgtactccgcgaccagctctgccagatgcacgtcaatgtgcaggataaaatcgatgaggaaataaatcaggtccatatttgcctatgccttgtactcgtcatctttcaggctgtaactacgttggctacagcctgaaatgttccgagcattattctcgttagtccgccagaaatagcgggcccattggcggttttggaagatcataccggtcagggtaatccaccgcgaccagatacagcccttccgcttttgccgttgctgccgccagcgttctgtcctttgccgccagcaactctgctatccagctctccggctggttgtgggcaccgacttccatcaggctgccgacaatattcctgaccatatgatgtacaaaagcattcgctttaatatctaccaccacataaggaccgtgacgcgtgacattaatatgcataacgttgcgccacggggttcgggactggcactgcaccgcacggaacgaggtgaaatcattctcgcccagcaagcattgcgcagcccgatgcatccgttcagcgtccagcggttcgtaaaaatgggttacccctttactcagtaccgccgggcgcagccgatgattgtagatgatgtagcgataacggcgagccgtggcgctaaatcgggcatgaaaatcatcaggtacagttttaacccaacgcacagcgatgtcaccaggtaaattcgcatttacgcccaaggtccacgccgcgtctttgcgcagcgcggttgtttcgaaatgcacaacctgcccggtaccgtgtacccctgcgtcagtacgcccggcgcagaagacggtgatgggttcgttcgccacctgggagagcgccttttccagcttctcctgcacactgcggacttcgttctgccgttgccagccgtaatacttactgccgtcgtactcaatgcccagcgcaattttataaactggcggttgttgctggtcggacattagtacagatactcctgcaccagtttctcggcgatttttactgccatcagcgcgccgccaaagcgaacgttatcggccaccgaccagaactggacttgctccggcataccgtagtcattacgcacgcagccaacagaaagatgcggcgtacccgaagcatcacctacctgagttgggaattcgttctcttcagagagcacaatatcttcgccttgaacaaacgcatcacgcgcttcttctgctgccagtggacgcagagcttcaaagttgaccatctgggcatgaccgtagaataccggtgcctggacgacgctagccgaaatcatcagcccttcgtcctgcaggattttgcgtacttcgtcaacgatacgacgttcttcacgcacgctaccttcgctatccggcagtaacggcagcatgttgaacgccagctgacgcccgaagaaatcttcttcgtcaatcggaatgccgttgagcaatttcgcactctgccccgctaacgcatcgaccgcttttttgccctgggcggaggctgaaatcaggctggtaacgctgatacgtgataaaccgccctgatcgattaacggtttcagtgccgccagcagctggctggtcagactgtctggtacggcgatgacattccggttccggtaatctgtcagtacaaacgggtttacttccggcaccaccagcggtacgtcgggttcgagagcaaacaatccactgctgtcgatcaccaggcaacctgagttggtcgcttcttcaacccaggcagcggtagcttctttgcctgcgacaaaaaatgccagctgcgcctgcgtccagtcgaattcagcggcatcctgcacggtgattgtcttaccaccaaagcgcagttgttcgcctgcgctttcgttacgtgccagtgcataaatttccccaaccgggaactgacgttcagccagcgtttcaagcagggcttcgcccacagcgccagttgcgcccaggacggcaatgttccagccttcagacatggtggtttactccagaaatagcaaagctccctgccaatgttacagcagagagcatgaagaagagattaacgtgccggatgatgaacggcgttaaaacccagtttacacagcaatgatgccgcactggcgtcatcacaaattacatacagagatgaccattcacggcgctcaagatagtttttgcgcagtttatcgaactcacccggtatcccggcgactttacgcagcggtgcgtcatcgcggcgcacatcatacaccaaatgcaccagccttttcagcgtcggttgatcgagcgggccatgcagcgtaatgcgaccaaactctggcgcaggcagtaatgtatccagcgcaacgtgctgttcatgcccaataaacttgctataagcttcaaacacttgcgtagtaccgcgtgctttaccttccagggtatagcctgcgatatgcgacgtgccgatatccacttttttcagcagctcgacgttgagttccggttcgccttcccagacatccagcactacgcttaacttctggccttcattcaggcaggtcagcaacgcagtattatcgacgactgcgccacggcaggcgttaatcagaatcgctccgggcttcaggctacggatcagtttttcatccgccagatgtagcgttttgtacggaccatctttaaagagtggcgtatggaaagtcagaatatccgcgcgctggactaactcatccagcgagcggaaatcaccctcatccccacggtcggcgcgaggcggatcgcaaagtaaggttttaatccctaacgcttccagtcgcgcctgcaatcgacgtccaacgttaccaacgcccacgatccccaccgtacggtcgtacagtgaaaatccatcgcgttcggcaagcatcagcagggaggagaaaacatattccaccaccgcaatcgcattacagccaggtgcagcggaaaaaccaattcccgcctgcttcaaccatgcttcatcgacatggtcggtccccgcagtggcagtgccaacaaatttaatgggttttcctgccagcaaagattcattcactttcgtgaccgaacgcaccatcagcgcatccgcgtctgccagttgagcgacggggattggacgcccgggaaccgcggtcacctcacccaaacggctaaataagtcgcgggcataaggcatattttcatcaacaaggattttcacgtttgtgttacctgtatgagacgagagttaaccggacaagtgtgccataatctcgcggccaggcatacttgcgaagatttcaggtataaggatacgtaatgatacaacctatttccggccctcctcctgggcaaccaccaggtcagggagataatctgccgtctggcacgggcaatcagcctttatccagtcagcaacgtacttcgctggaaagcttaatgacgaaagtgacctcactgacgcaacagcaaagagcagaactgtgggcgggtatcaggcacgatattggtctgtcgggagattcaccgctgctttcgcgtcacttccctgccgctgagcataatctggcgcaacgtctgctggccgcgcaaaaaagccattctgcccgccagcttttagcgcaattaggggagtatttacgtctggggaataatcgtcaggcggtcacggattatatccgtcataactttggtcagacgccgctgaatcagctctcaccggagcaattaaaaaccattctcaccctgttgcaggaagggaagatggttattccgcaaccacagcagcgcgaggcgaccgaccgtcctttattaccggcggagcacaatgcgctaaaacagctggtgaccaaacttgcggcggcaacgggggaacccagcaaacagatctggcaatcgatgctggaactttccggggtgaaagatggcgagttaattccagcgaaactgtttaaccatctggtgacctggctacaggcgcgtcagacgctaagccagcaaaatacgccgacgctggaatcactacagatgacgctaaaacaacctttagatgccagtgaactggcggcgttatcggcatatatccagcaaaaatatggtctttctgcgcaatcatcgctttcttctgcccaggccgaggatattcttaatcagctttatcaacggcgggttaaagggattgatccgcgtgttatgcaaccgctgcttaatccttttccaccgatgatggacacgttgcaaaatatggcaacgcgtcccgcgctgtggatactgttagtcgcgattatcctgatgctggtctggctggttcgttaaccccgacgaaatgacagtatcgtgacaataatacccagcaccgcagagatcgccccggcaagaaataccgaagagtaaccaaacgtggtcgccagcattcccgccagcggcccggagacgccgagggcgatatcctgaaacgcggcgtaaccgcccagtgcggtgccgcgaacttgtgaggggacgcgtttaaccacctccacgcccagcgcaggaaagataagcgaacatccggctccggttaacgccgcgcccgctaatgcgacccatgcacctggggcttgccagagcagcaacaagcccaccgtttctacaagcagagagacaatcgccactttcacgccgccaaaacggtccggcatccagccaaacatgacgcgcatcacgacaaatgcgccgccaaacgcggtaagagtaaagcccgccatcgcccatcctttgctggcaaagtagagcgaaacgaaagtcccgataacagcaaaaccaacgccttgtagtgccagacctaaccctggtttccagataagcccgacaacgctccacagcgatggacgttctcccgccagggccggtactttgcgcactgtgccgttacaggcccacgccagtacgggtaataccattgtggtgatcgccagtgcggcaaaaccgtaatggctatgaatcaacaggccaagcggagcaccaacagcgagggcaccgtaaatcgccattccgttccatgacatcactttgccagagtgttttggccctacgatgcctagtccccaggtcagagcgcctgtcagtaactggctttcaccaaagccaagaatcaaacgcccgacgaccaacagagcaaatttgaacggtgcggagacaggcaaaatcgccgccagcagcaacgcgccgccagccagaccacaagctaacattccctgaagcgccgaacgttttgcaccatattgatcggccagtcgcccggcgtaaccacgcgtcagcaccgtagccagaaactgaatcccgacggcaatgccgaccatggtattgccatagcccagttcatgatgaacaaacagcgggataaccggcaacggcaaccctacggtcatgtaggtgagaaaaaccgcaaaagcgatgcggaagagcgaaaaattggcagaagatcgtgtttcggtttggcttacagcagtcatgcattactccagaatgcagcgcaaggcgaggagtatccccgtctcatctctctggtttcagggttacggtgcgttggcaggatttaacgcgtacgtcttttcagaaggaaatcgacaaagcgggaagtttgcctggaactggcggcgattgtcaatgatgtgaaaaagggaaccatcaggttcccttttgcgttagtgccggaggccgcattggcgcgtaacgtcggatgcgacgctggcgcgtctactccgacctactgcgaattaatctttcagcttgcgcattaccagcgtggcgttggtgccgccgaagccgaagctgttagacataacggtggtcagttcgcgatcggtcgtttcggtcacgatgttcagacccgcagcctgctcgtccagctcttcaatgttgatgctcggggcgataaagccgtgttccagcatcagcagagagtagatagcttcctgtacgccagcagcgcccagagagtgaccggtcatggctttggttgcagaaatcgccgggctcttatcgccgaacacttcacggatagctgccagctctttcacgtcgccaaccggagtcgaagtaccgtgggagttcaggtaatcgattggggtatcaacgccatgcatcgccatcttcatgcagcgtactgcgccttcgccagacggagcaaccatgtctgcaccatcagaggttgcgccgtagccaacgatttcagcatagatgtgagcaccacgcgccagcgcgtgttccagctcttcaaccactaccataccgccgccgccagcgataacgaaaccgtcacggtgagcgtcgtaagtacgggaggctttttccggggtgtcgttgtatttagtagacagcgcacccattgcgtcgaattcgcaagccatttcccagcacagctcttcgccgccgccagcaaacacgatgtcctgtttgcccagttggatctgctctactgcgttaccgatacagtgtgcggaagtcgcacacgcggagctgatggagtagttaacgccatgaattttaaacggggtggcgaggcaggcagaaacgccggatgccatcgctttggtgaccacatacgggccaaccgctttcaggccgcgcgggccgcgcattgcgtcagcgccgaacacctggaaacgcggggagccgccgccggaacctgcaatcaggccaacgcgcgggttattctggtaagcttccggagagaggcccgcatcagcgattgcctgctccatagaaaggaatgcataaatggatgcgtcgctcataaagcgcacaactttgcggtcaatgaggccagtggtatccagttttacgttgccccagacgtggctacgcatgccggaatccttcagctcctgagagaaagtgatccctgaacgtccttcacgcagagatgccaggacttcctgctggttattaccgatgctggaaacaatgcccaggccagtaatcactgcacgtttcattcaatacctctgtaagtcgcacatagagtaagtttcgaatgcacaatagcgtacacttgtacgccgaacaagtccgatcagccatttaatagagaaatttgcgcagccttacacacatcgctaagatcgagccaccgcctgtaagacgagtaacttacgtgaaacactactccatacaacctgccaacctcgaatttaatgctgagggtacacctgtttcccgagattttgacgatgtctatttttccaacgataacgggctggaagagacgcgttatgtttttctgggaggcaaccaattagaggtacgctttcctgagcatccacatcctctgtttgtggtagcagagagcggcttcggcaccggattaaacttcctgacgctatggcaggcatttgatcagtttcgcgaagcgcatccgcaagcgcaattacaacgcttacatttcattagttttgagaaatttcccctcacccgtgcggatttagccttagcgcatcaacactggccggaactggctccgtgggcagaacaacttcaggcgcagtggccaatgcccttgcccggttgccatcgtttattgctcgatgaaggccgcgtgacgctggatttatggtttggcgatattaacgaactgaccagccaactggacgattcgctaaatcaaaaagtagatgcctggtttctggacggctttgcgccagcgaaaaacccggatatgtggacgcaaaatctgtttaacgccatggcaaggttggcgcgtccgggcggcacgctggcgacatttacgtctgccggttttgtccgccgcggtttgcaggacgccggattcacgatgcaaaaacgtaagggctttgggcgcaaacgggaaatgctttgcggggtgatggaacagacattaccgctcccctgctccgcgccgtggtttaaccgcacgggcagcagcaaacgggaagcggcgattatcggcggtggtattgccagcgcgttgttgtcgctggcgctattacggcgcggctggcaggtaacgctttattgcgcggatgaggcccccgcactgggtgcttccggcaatcgccagggggcgctgtatccgttattaagcaaacacgatgaggcgctaaaccgctttttctctaatgcgtttacttttgctcgtcggttttacgaccaattacccgttaaatttgatcatgactggtgcggcgtcacgcagttaggctgggatgagaaaagccagcataaaatcgcacagatgttgtcaatggatttacccgcagaactggctgtagccgttgaggcaaatgcggttgaacaaattacgggcgttgcgacaaattgcagcggcattacttatccgcaaggtggttggctgtgcccagcagaactgacccgtaatgtgctggaactggcgcaacagcagggtttgcagatttattatcaatatcagttacagaatttatcccgtaaggatgactgttggttgttgaattttgcaggagatcagcaagcaacacacagcgtagtggtactggcgaacgggcatcaaatcagccgattcagccaaacgtcgactctcccggtgtattcggttgccgggcaggtcagccatattccgacaacgccggaattggcagagctgaagcaggtgctgtgctatgacggttatctcacgccacaaaatccggcgaatcaacatcattgtattggtgccagttatcatcgcggcagcgaagatacggcgtacagtgaggacgatcagcagcagaatcgccagcggttgattgattgtttcccgcaggcacagtgggcaaaagaggttgatgtcagtgataaagaggcgcgctgcggtgtgcgttgtgccacccgcgatcatctgccaatggtaggcaatgttcccgattatgaggcaacactcgtggaatatgcgtcgttggcggagcagaaagatgaggcggtaagcgcgccggtttttgacgatctctttatgtttgcggctttaggttctcgcggtttgtgttctgccccgctgtgtgccgagattctggcggcgcagatgagcgacgaaccgattccgatggatgccagtacgctggcggcgttaaacccgaatcggttatgggtgcggaaattgttgaagggtaaagcggttaaggcggggtaatctgctctcgcagtgtttgccggatgcggcgtgaacgccttatccgacctacgtgtgacgtgtaggcctgataagacgcgataagcgtcgcatcaggcatgctgctccagacgccgcaacttactgctgtgacgcctgctgaaacaggttttcccacatatcggtcaccagcgcctggtcacgcggcgacaattcaccagcaccaatggctttttccagactctggctaacggtcgtatgcaccgcctgagcggagtggtcatcaccactttccagttctgcgatggctaatgtcaggtggccacgcaaatacccactggcaaacaactcatcatcactggcatggtcaaccataccgtcgattaatgccagaatgcgtgattcaaactccgcgatcatcttctttcctcattgtaaaacgtggcgctggcttcagttgagcgcttccggccacgggaactgttccgccgtaagttccggcgtgtgataataattttgtagtgctttaatgaagcgtgccggacgttccggaatgccatttgtcagataatccatcacctgcgcatgtactcgccgttgaaacaccacacgatccggttcgaaatccccttccagattgtcgcaactgacgttaaacggatatcccgccgccacacagaacaaccagtcgagcgcctgcggcttcacttcaacatcttcaaactggctttgcgtttgggcatcgcgtccgtccgggcaataccagtagccgaaatcaaccagctcacggcgcgctttcccggcaatacaccagtgcgaaatctcatgaattgcgctggcataaaagccatgagcaaagacgattcggttatacggtacttccgcatcagcaggaagatagatcggttcgtcgtcgcctttaatcagacgggtattaaaatcatcggcaaagcagctattaaaaatttcaatcaactgctcgtagtggtgtgtactgttcattagttcatccccaaccagtggaggatctcctgtccgtggctgtcgtaaagtaatttggcactcatcaccgccgagacgataacaatcatcgggcggatcagcttttgtcctttgctcaacaccagtcgtgaacccatgcgcgcgccgaggaactgccccaccagcatgacaaagcccgtcgcccaaatcactttgccgccgagaataaacagcagtaaaccgccgatgtttgacgttgcgttgagtaatttggcgtgagccgtggctttggcgaggttaaatccgcacagcgtaacgaaggccagcgcgtaaaacgacccggcagccgggccaaagaatccatcataaaaaccgacgcagccaccggctattaacgcgaagggtaaaccgtacatccggcgctggcggtcttcttcacctagctttggcatcagcaagaaatagaggccgatacaaattaccagaatgggcaaaatctgccgtaagacatcagcctgaacgtattgcaccagcagtgcgccgctcattgagccgacaaaggtcatggcgatattgagtttctgatcgcttaaactaaccactttgcggcgaataaagtagatagtagcggaaatagagccgccgcaggcttgcagtttattggttgccagcgcattagcgggagacatccccgctgccatcaatgccggaatggtgagtaacccaccgccaccggcaatcgagtcgataaatcccgccagcatggcgacaaaaaagagaactcccagcaacagcggggaaaccataaacaggctattaaacgtttccattagatcacgtgctcatccagtagcgcctggcaggaaggcggcaacggaggcggtgtcttcttctcaggctttgttgttcccggttttggaggttcaaaccagctttgcagttctgccccgcaaccatcgcctgatggcggtaaaggttgatcttcacactccagactatcggcagggcaacgtaatcgtacatgcatatgcgcgcgatgctggaaccagggtcgcactttgcgcaaccagtcgcgatcggtgcccgcatcaaggcaaagttgttgtttaatcgccggattaacaaaaatgcgcgtgacgtctttgtcctgggcggcgagtttgatcaagctgaaaatttctggcttccacagcgtggagacaacgtgtttaccgtcgcgggaaactaagtccagtgcttgcgggcgcaagagctgcgcggaggtccagcgagttttcggcagttgcagaaagatatcgacatccagtccggtctggtggctggcatgaccgccgttgaaacgcccaccagcgggcatccccatatcgccaatcagcaccgtacccatgcccagattgctcacctggctactcagacgctggataaacatcaccagatccgggtgaccgaaatagcgacgctgatcggtacgcatgacctgataatgttcggactgtatcggcagcgtgtcagcgccgacaatacagccattagaaaaactgcctatcgattgtgcgctacccggcacaggttgggttattttttgccacggcgtcgctgccaggctggcgctactggcaagcagagccagcagcgcaatcgcggttttattcattttttaccagcgtggaatatcagtcttcacatcggcattttgcgcccgttgccgtaacaggtgatccattaaaacgatcgccagcatcgcttctgcgatcggcactgcgcggatcccgacacagggatcgtgacggcctttggtgatcatctcaacttcttcgccaaagcggttaatggtacgacccggcacggtaatgctggaggtcggtttcagcgccatatgggcaatgatttgctgcccgctgctgataccgccgagaatgccgcccgcatggttgctctggaaaccgtctttggtgatttcatcgcggttctggctgccgcgcagcgccaccacgtcaaagccgtcgccaatttccacgcctttcaccgcgttgatgctcatcagcgcatgggcgatgtcagcatccaggcggtcaaagaccggctcgccaagtccggcaggaacgccactggcaacaacggtgactttagcgccgatggagtcgccctcttttttcagcgcacgcatcaactcgtctaacgcgtcgattttgtcggggtccgggcaaaaaaacggattttgctcgacctgcgaccagtctttgatatccagcggaatgtcgcccatctgggtcaggcagccacggatttcaataccaaatttctcggcgagatattttttggcaatagctcctgccgccacgcgcatggcggtttcgcgggcggaagaacgtccaccgccgcgataatcgcgcagaccgtatttttgttcgtaggtgtaatcggcatggcctggacggaaaacgtccttaatcgcactgtaatcctgagagcgctggtcagtgttttcgatcaacaagccaatgctggtgccggtagtaacgccttcaaaaacaccggagagaattttgacctgatccggctcgcggcgctgggtggtatagcgcgatgtcccagggcgacgacggtcgaggtcatgttgcaggtccgcttccgtcagcggaatgcctggcggaacaccatcgacgatgcagccgagcgccagcccgtgcgattcgccgaaggtggttacgcgaaagagttgtccaattgtgtttccagccatcacggctccgttattgttgtgtttgcgtgtttacttaatctttataaatcgcgaaatgttctcgtgcggcaataagctgctctttggtgagcataaacacaccatcgccgccgttatcaaactccagccaggtgaacggaacatccggatattgttccataagatgtaccatgctgttgccgacttcacaaatcaacacgccatcatcagcaaggtaatctgccgcgttaccgagaatgcgacgcgtcagtttcaggccgtcagtgccagatgccaggcccagttccggctcgtggcggtattcgtttggcaggtcggacatatcttccgcatcgacatacggcgggttagtgacaatcaggtcgtactgcactttcggcaagtcgcggaacagatcggaacgaatcggaatgacgttgtggatcagaccgtgttcttcgatgttctgttcagcaaccgccagcgcgtctggagagatatccaccgcgtcgacttctgcatccgggaaggcataagcacaggcaatggcgatgcagccgctaccagtacacatatctaaaatatgctgcggttgcttgctgataagtccggcaaatttattgttgatcagttcaccaatcggcgagcgcggcaccagcacgcgttcatcgacgtaaaattcatggccgcagaaccacgctttgttggtcaggtaagccaccggaatgcgttcattgacgcggcggatcacgcgttcaacaatacggtgtttttcgctggaggtcagacgcgcggtgcgcatatcttccggaatatccagcggcaggtagagcgaaggcaacaccagctgtacggcttcatcccacgggttatcggtaccgtgaccgtaccagatatttgccgcgctgaagcggctcaccgaccagcgcaacatgtcctgaatggtttgcagctcatttactgcttcatcaacgaaaattttatccacgtattcctccagggcatgatcgcaataatttcggcggctagtttgccatgaagatgacgataaatcagcattcacgcgcggtgagtgaggaaaaatacgtttaaaacgatcgattgcgctacgagtcgggtaaactgtaggaaaattagaaatagagacagataaatgaaaaagaaaacaacacttagcgaggaggaccaggctctgtttcgccagttgatggcggggactcgcaagattaagcaggacacgattgtccaccgaccgcagcgtaaaaaaatcagcgaagtgccggtgaaacgcttgatccaggagcaggctgatgccagccattatttctccgatgagtttcagccgttattaaataccgaaggtccggtgaaatatgttcgcccggatgtcagccattttgaggcgaagaaactgcgccgtggcgattattcgccggagttgtttttggatttacacggtctgacgcagctgcaggccaagcaggaactgggggcgttgattgccgcctgccgccgtgaacatgtgttttgcgcctgcgtgatgcatgggcacgggaagcatattttgaagcaacaaacaccgctgtggctggcacaacatccgcatgtgatggcctttcatcaggcaccaaaagagtatggcggtgatgcggcgttgttggtgttgattgaagtcgaagagtggctgccgccggagttgccctgaggagttgagcgcgttgcgccaggtacgggtaatggcaggggcgaatgcccctgcctggtgtatctaagggctacaactcattcagtatgtactggaaccggcaagtagaatcgattggctgcatactgctggtatcaacacgcacgaccatatcgtgtaactgtttgtccgttatagggtgtcgatttggcgtgaccgagacttccgccttgtcacatcccgacgcggtaaaagttatcatctgtgcaacccagcggcagtaaccacctgtttcattcatctgcgtactgtcgcacaacttcccatctttcatcaaatacgttgaaagcgttttctcaaccacaccgcccgtcgactgcagggtgagcagttttgacttactgacataattctcattccatgaaacgtcataaggttgaacagaaacggatggacaaatcgtgtcgtgactatcaggcccctgatacgtcacgccccctggagaggcttcagagtcattcataataaccaaccatggacaagaaaagtaagattcaatctctgcagagacaataacctcaaatgtataatacccgcagttccacccagacggtaatccaggacaacttgctttgttgatattttgatggtagccaatcagcttaaccgaaggggcaggaggaggaccactccagctcacattttgcaatatttccccagtcatgagccattgactacttttatattcaccaacgtacactgcggatggcatcattatttttaaattaaaagtcgcaatattacgcgaatcaccgttgtaaccgtagtaaacgtcaacgctatgcccggcagccatagcttctgtagtagcaataagcatgaccagagcgaacaaccatcgtagtattttcattttaaatatactcaaatgtcgcagttaaagaggcggtaaattcaccgatcgtcacatcacggccgcttttcgcctgtagccaggctctgaaattgatatcgttattgccattggttagcgcaaaggtcgccccatttgtattgttgatggcaacctgcattccgtcggttttttccatgccaattcccactccctgagcggttgatgacgtatccagtgccagaaaaccgggttgttcgctgtcttctacccccgtgagcgtgacttttacgttgtatcccgccggccctttgcaatctttcagcttaaagactacgggtacacgagcggactggcctgcaacgttcaaatcctgacgactgaccgtgggaaagcgcacctctgccagatattggccatccaccaccagcgcacaggatttacttaataaattaccggagaaatgcagattattatctgccgcgaataacgtgctactcattgccaatatcagccccgctaacaggacgtaaccaccggactgaatcattgatttattcattgataatccacccgtaatgttgcgtaagccgaaaaattcgtatcgcttaacacagcatcactcgcttttaccggtacggcctccagcttcggcttttgcgtaaaatcagtggcgttgatagcaagcggagtattgagtttaaaacgctgaccatcgtgctgaagctcgataccaaaaccgggtacatcagtttcaattgctgcatcattaaaactggtttgtgtaccagtccaggtgagggtcatctcccaatctggatgacgggtcgtcgagtcacaagtgagttcatatggcacctctttacgaccatagttgccgttgatgtcgtcgataatgagatcgcgaaattcgacttcaatggttttaccaccgctgatgctacaggttggcggtgacaataatgtcccgtgaaaggtgatgtcttcatcagcagcatgagctatggcgctactgacacaaagcagggttaagaaagtctttctcattgatagtccaccaccatggtcaaactggcgttaaactcgcccgcagcaagttgcgccccgcttgccttcacaggtacagccttcaactgtggctggttattgatattaaatggcgtccagctattttcaccgacggcaaacaatgagttatcggcgctattttctatccgaatgcccagcccggtgatattggtactgagtaccgtttcgccgttaatcgttgaggtattgcccttaagttgcatccgcaagtcgttagcaagactgtttgtgcagttcaacgtgtatttcgcatcttgccgataattggtgccatcaacgttatcagcaatcatattgccgaactctacctggctgcccttgattgaacagggtggcggagcatcgaccaacacgcgcagaattaaatccacgggtttactaccagccatagcagataaactacagacactgcataccagcagccctgcgcccactacaaacttttgactcataactccccccgtcatcagcctttgcggctctgctcttcatccacctggcagctgttgccattgcactggaagaacagcggcatccgtgcgccaaagtcgttgacgtaagtcagcaccggtacgctatccattttcacattcagcggtaccgtggttttcggctcaatgaccagaggcgagaaccctgcagctggattaccgtttttctgcgcactggcgttgctgataatcacgtagtacggcgttgggttattgacggtaaatgcctgaccgctgcgggtgagcgtcaccttgtgctgccacggacttttcatactgaccttttccagcgcctttggtcgccagaacaacttgatacgcgtttgcagcgcgatttgcagggtattgggtttgtttgattttggcgggatctcgcgcacgttaaagtagaacatgctttcacgatcggctggcaatttgttgatatccggcattccctgcacttttacctgcccgttcatcattgaatcgatgcgttgcactggcggcagcacagttaacggcgaggtgatcttgttacccttttcatcttcaatccagctttgagccagataagggagtttcggatcgttattacgcagcgtcacgctgattgatttgtcgctttcattaaatatcaaacgggtacgatctggcgttacagacgccagggcagacaaactggtagcgctaagcagtaacgccagcgtcatagcacccaatttggcagagcaaagtaaatcagacatggatcattccttaatcacgttattggttagctgaaacagaaacagggggatcggtgggtgtcacctgttgcgtctgctcctgaatgacaggctttatgtcatcaggaacaaccggcgcgacgttgcctttatgctggcatggcagtaacaagccgttaaacagatcggcaggcagcgggtccggcaggttgatatcgcaatgcgcaacaccactccagaacacactcatatgttcgccaggtttcaccccagccagatagacactaccgtcatcatcgacaaggcccactgtctgctcgttatcattttttacttctgcgccaaacggtggatggctgccatcttgtaaacgcagcaccgccatcgctttttgaccactgatgacggcaaatttgcggtagccaatggctccttcagttagcgtggcttgcaccaccgactgggttgcttcggcgttttccggcaatttgttgaggtcgatatacgcctgattgcgataataattgttaacgtcagaaacgacggctttaccaaacatattggtataaacagcagccccgttaccttccaccggaacatcggcaacgccatcggcatcaatcagcaggcgtgtcccgcccatattctgggtacggtgaagtgcgccgccgtgggtagtaagcgttgcgccgccctgtaacgacaagcccgcagaggtgtattgcccttcatggtagttcgcactgaggtcaacctgcgccagcgaaccatcatggctgtagtagccatcaacgctggtgtgtttgtcactggtgccgatgttcaactgatagtgagtcgcgtcatcgacacggctaaaataaccgacctggctgctgtccgtcccactgccatagttgccgttatagctaacggtactgttgtcgccccacggcatactgagcgaaatctacatgcccttatccgcccggttgtcatactcgtagcggtagccagtcagggaaacgctcatattacgaatgctgcccatattgaaatagtgggagagcatgatgttgtagtttgtctgctcctcacgatcccagtaggtatggcgggtatagttgagataaaccgaaacacccgcatcgcggaagttctggttataagtggcggtgtacatctctttgtcgttgcccgtacggaccatttcgctgtcactggcatccagatactcgctcatggtcataaagttctcttccgagaagcgatatccagcgaaagtgacgcggctgttgagctggtcaaagtctttggaataactcacacggaaggagttaccgtccagcgaacctttgccataagcggtgtctttatccagtttggtatgcgaatgagtaacatcaaacgcgaccgcgccgaaggtagacaaatcgcgaccgacgcccagcgccgcagactgatagttttcatcacccagcgcaccgccatataacgaccagccgttagcgatgccccaggaggcttcagcaccagagaaaaatcccccctcgacatggtggccccactcttgcggacgtcccatcatgatcttatagcgaacctggcctgggcgagtgaggtatggcatcgaggcggtgctgatgtcatattcctgcacctggccgttctgttcttcaatgcgaatatgcaacgtaccggagacggaatcaccaagatcctgaatacgaaacggtccagccggaacctgcgtttcgtaaatcacacgccccatctggctgacggtcacttttgctgtggtgtgtgccacgccggaaatgtctggcgcgtagccgcgcagattgggaggcaacatttgatcgtcagtgctgacactgccaccaacataattaaaaccgtcgaaaatatcggaattgaggtaatcttcgcccagcgccagtttggcttttaatgacggtaacgcccgccaggcataatagcgactccactcccattttttttgtgtgtcatcgccgccaaattcatcgtcatcatcattactgcgcgtatgttgatagttggtctgccagtcagcgcgcatacgccatggccccaggttaaccccgaccgtcccgttgccgctgatctcgttactgtcatcgccgccattttcttcgtgtcgtgtttgcgcagtgatgctgtagtccgcaatgatcccggagatgccatcatcccaacgagaaggtggatcccagtcgggccaggtatattcgaggtaagcctgcggtagtgaaatgactaatgcggactggcttaaatcagccttaatttccacgccttccagttgaccgggcttcaggcatttaccatcgtggctccattgcagatttttcgccacgtcttcttttaaaccaaactgcgccaccagttccggtgtcagacaagcatagcttttgctaacgtcatcttcaccagcataccagtaaatatcgtactcttccgccaatggctgtttatttagttgaacctgtaaattgtattttccgggctcaacatacccctggctggaaaaacgcttcagatcaatttttgtgtcgccttttaattccagaaaacgggaatcaaactgaatgtcgtcttcagcccagacactgctataactccctgacattgccagcgcaatgcaccacggaagaatccgtaatcgaaaaagagaatggtcaggcatacacgtttttatccgtttttattcttgttcggtcaaaatccatttaaataccccatagcagtgtcgctatgggggtatgccttacaggtaagtaatctggaaggtggtatttgcttcgaaattacccagatctggcgcatcagctgcgccgaccagccaggctttaaagttcagagtctgcttcgctttgcctttattagtggcagtatctttcacgattttctggtcaatacccatgccgcttttgtaagaggtacccagagagtcaccgatcgccaggctaacattgttaaatgccgcaccggtatcggtattgaaaatggtgtaataattgccgctatttgcagaagaaacggtaccagtaaaggtagtggtcattgtttcctgagtatcaaatacgcaatcttgcaggcgaatctggaaatttttcggcgtggtggtgccgttatttttcagtttttcggcaccgatatcacccatatcaacttccagtttgtgatcgtccggaacgatagaacacactgagtcttcaatggtgccgtaaaaacgtgcagtaccgttgttacccgcagcgattgttgccgtagaggtgaacgcgcccatcaccattgccgcagcaatagctgttttaacaaacttactcattatttgtccttaaactataaataattaaaatataaacattgcaatacattgattcagtcaatagccaatgtttatacccagccattgaatacggcatgcgatccaaaaaaacaggtcgtaaaaaatgtattcgttggtgtggggtcgaatagtgatgttttcactcccctgattcaatttaattttactaatgagtaaatgtagatttaattaatatattgataggggaaagattatcttaaggatcttctaaaaaaacacgaaatatatatttagaaaaaacaggaagcatatcaacaatgaatgccaatagcttaaaaaacaaacaatgaacatataatgcgattggcattaacccgcttttgtcgatataatatataaacactatagccagaatttaatcaagtttcaattacgtcctgcctgattattcaactctattttctccattatctgtattaataaatgataatgagtgtcaaacagacattattcatttcaacatgtaactttgggcaaaatcaagatacgcgcagaagaatactttccgaatgaaagttaaaggtgttttatttatagatggggagagtcttcgatagtagtgaggttgacagatatccgctgcctgatgagcaattatgcccaatgaatctacctcattgggcataatttggaactcatcagatagcttttgccatcttcagattacacgggctcatctgccagttgaatgtgccgtttccgctttcatcaagcgttacgctggcaatggccgaggtggtaaacataggcggcgtttcgcccggacataactcggcaaccagatacccgactaacggtaagtgagagatcaccagtaccgaagcaacaccttcattggtcaacgcctgcaaataggcactgaccagaccaacatcgccgcagggcgttaactccggcagaacttctgcactggaaggcaggttcagacaatcccctacttcttccagtgtttgctcggctcgcaggaacgggctcaccagaacgcgttcgatttccactttttgacctttcagccagttcgccatcaggcgagattcgtcacaaccattagtggtcagaggacgaacggaatcactggcggcatcgagggctgcgtcgccgtgacgcatgataaaaacttgcatattgcaccgcttttgttaaccagattcgcccgttttctttcatctgaaaccagagaaagaaaacggtggccggcattgtgccttatccattcaccgaatgaaacgctgttttttacctcaatggcgtaagtatagtcaatatgcgtttacattttgaccaacactccgccattcagcgcggattcatatagctttgaccttcttattgcaggtcagttgcagttgttttccaaaaactttccccacgcgcgcccatctcgaccaaacgctcgcaaggggtaaaacgggaaccatactgcgtggcaagtcgttgcattattgcaaccacttcgcccgcgccgagagaatcgatatagcggaacggtccaccgagaaatggcggaaaaccaatgccaaataccgcgccaatatccccgtcacgcacgctacggataacctgctcatcaacacaacgtactgcttcattcagcatcaacatcacacaccgttcagcaacctgcggtgcggagattcgcccctgcccttgtgtgccaatcagcgggtaaatggcgggatcgacctgttttttgcttttacgccctttctgaccataaagatagaaaccccggccattttttctgcctttgcgatcgtcgttcaaaattgaagaaacaacatttgcaggcgcgctaaaacgttctccataagcggcttccagtacaggaataattttagtcccggtgtcgattcctacctcatccaaaagttggattgggcctaccggaaaaccaaatttcactagcgcggcatcaatgtgctctacccgttcaccttgggtcaacatgcggatagcttcattaatgtaaggcgctaagatgcgattgacgtaaaaaccggctttgtcacgcacgacaattggcgttttaccctgttttttcgccagttttactgtggtagcgatggtttgcgccgatgtccccgcatgaggaataatctccaccagcggcattttttccaccggactgaagaaatgcaggccgataacttgctcaggtcgcgtggcgtgagcggcgatatcaccaatcggtaaagatgacgtattcgaagcaaagatggtatgagcggcgcaattttgctcaacttccgccaccatctgttgtttcaattcgagattttcaaacaccgcttcaataatcagatcgcgatgggcaaagccgcgatagtccgtcgttccggagattaatgccagctgtttgtcacgttcgctggctttgagatgacgacggcgaactttgccctccagctgatcccaactgtacttcagcgcatgatttatgccctgcgggttgatatctttaattctgaccggaatccccgctttacaagcagtgacataagcaataccgccgcccatcaagccaccacctaaaatccccacgctgtttaatggcgcaggcggcgcatcactgccgggatctttcttcacgtccgtactggcaaaaaagatactacgcagcgcctgcgattgtggcgtcatcgccagttcgccaaacgcccgagcttcggcgtcataaccgctgctggtgccctgcgctaatcccgtttcaacaacctccaggatgcgttctgtcgccggataattgccttgagttttgtgttctgttttcttgccgaccattttgaacagcagcgcacgacctaacggccccgccagaatacgctcgcgtacaggtagagggcgggaagatgggcgctccttctttgccagctcaacagcggcttccagcagaatggagtgcggaacaacgtcatccaccagccccagctttaatgcctgtttcgcccgaagttgttttccggtgaggatcatctctaatgctgtgctgacgcctatcagacgcggtaaacgctgggtgccgcctgaaccgggtaacaatccaagttgtacttcaggcaaaccgagcaccgttttaggatcgtcagtacaaacgcgaccgtggcacgccagcgccaactccagcccaccacccaggcaagcgccatgaatagccgcgataacctgaatgggcaaagcatgaatctccgccatcaactgttggccctgccgcgccagagcttccgcttcttgcgccgttttgcagttgccgatcatgttgatgtctgcgccagcaatgaagttgtccggtttagcggagacaaacaccacgcctcgcaactctttgttttcacggagttgcttaataatggcgcgcacctgcgaggcaaactccgccttcagggtattcattttctcacccggtacgtcgatggtgataacggcaatgttgtccagacgaacattaagggtaaacgctgatgtcatttccattattccgcctccagaaccattgccgcgccaagcccaccggcagcacaggcggtaactaaaccaaatccaccgccgcgacggcgaagttcatgcaatgtctgggtaatcatccgcgcgccggtcgccgcgaagggatgcccgtaagcaatcgaaccgccaagcacgttaaatttgctatcgtccacttcgccagtggcatgtgcacgccccagtgcttcacgagcaaaacgttcactacccagcaactgaatattcgccagcgtctgagctgcaaaggcttcgtgcatatcgatcaatgtcagatcgctcatcgtcaaaccggcacgctccagcgccagcggtgttgaccaggctggaccgagcaacatgtcctgccagacatcaatcgcagtaaatgcgtagctgcgcagataccccagcggcaccagccctaattctttcgcccgggattcagtcatcaggatcaccgctgccgcgccatcggtcagcggcgtactgtttgccgccgttaccgttccgtgtttgcgatcaaacgccgggcgcagctttgcgtaatcggcaagcgaggaattaccgcgaatattgttgtcttcgacaagcggttgtttataaggagggataaaggcagtcatcacctcttctttgagttttccgtctgaccatgcctgagcggcacgctgatgcgaacggtgcgctaatgcatcttgctgttctcgggtgatgccgtaggttttcgccatttgctctgcggtgtcgcccatccgcaagccggtagaatattctgctaccgcaggtggtacgggcattaagtcgcgcaaacgcaggcgagagaagagtttcagtcgctggctcatggtacgagctttgttgacatcaaccagcacgcgcgccagttttttactgacgccaattggcaataccgaagaggaatctgccccaccggcaatccccgctcgaatagttcccgccatcaggctttctgcgacgtttgcaactgcctggaaactggtagcgcaagcgcggctgacgctgtaagcatcggtatgtacattcattcccgtaccgagaacaatttcacgcgcaatgttgggggcttcaggcatttgtacgacctgaccaaagaccagttgttcaatcacttcggcggggatctcgctgcgtgccagcagttcgcctaccaccatcttccctaaatcaaccgcgggaatgccatgaaaagccgtcgcctgacgggcaaaaggcgtacgtaaaccgctaacaatggcgatacgatcgccctggcgggtaaccagcggtaaaacctgacccataacactcccctgtaaaaaaataaataaagtggtctgacctgatcatagtcttaaccatttttttacatttagccaagtggagaaaagggaaagtgggagctatgacacagagagaaaagaagaagagaaaagaaaacgcccctgccagcaactgacaggggcgtacgtacccgagaggaattaacgcagacccagctggaaaatcagcatttcagcttcgcaggcaaaagtgaaatcgatatccaggcgcacaccgtcagactcttcagtgaaagtcggggtgattttgcaaggttcagattccacgctacgggctttttcagtcagcgccgccagcgtttgctctgcttctgcgcggtttgcaaacacgcggctgtaagacgcggtgcagtcggagttgtccataatggtgccaacatccatacagcagcaaaccggggtttcatcagcactacatttactcatcgttgatttcctctgtatgtgcacccaaggtgccagataaacgttgtggatattttacgcttccggaaagtgctgctccagttgttaattctgcaaaatcggataagtgaccgaaatcacacttaaaaatgatctaaaacaaaattcacccgaatccatgagtgcgccacctccaaattttgccagctggatcgcgtttcttagatcatatttgaaaaaagatagaaacatacttgcaacattccagctggtccgacctatactctcgccactggtctgatttctaagatgtacctcagaccctacacttcgcgctcctgttacagcacgtaacatagtttgtataaaaataaatcattgaggttatggtcatgagccagaaaaccctgtttacaaagtctgctctcgcagtcgcagtggcacttatctccacccaggcctggtcggcaggctttcagttaaacgaattttcttcctctggcctgggccgggcttattcaggggaaggcgcaattgccgatgatgcaggtaacgtcagccgtaaccccgcattgattactatgtttgaccgcccgacattttctgcgggtgcggtttatattgacccggatgtaaatatcagcggaacgtctccatctggtcgtagcctgaaagccgataacatcgcgcctacggcatgggttccgaacatgcactttgttgcaccgattaacgaccaatttggttggggcgcttctattacctctaactatggtctggctacagagtttaacgatacttatgcaggcggctctgtcgggggtacaaccgaccttgaaaccatgaacctgaacttaagcggtgcgtatcgcttaaataatgcatggagctttggtcttggtttcaacgccgtctacgctcgcgcgaaaattgaacgtttcgcaggcgatctggggcagttggttgctggccaaattatgcaatctcctgctggccaaactcagcaagggcaagcattggcagctaccgccaacggtattgacagtaataccaaaatcgctcatctgaacggtaaccagtggggctttggctggaacgccggaatcctgtatgaactggataaaaataaccgctatgcactgacctaccgttctgaagtgaaaattgacttcaaaggtaactacagcagcgatcttaatcgtgcgtttaataactacggtttgccaattcctaccgcgacaggtggcgcaacgcaatcgggttatctgacgctgaacctgcctgaaatgtgggaagtgtcaggttataaccgtgttgatccacagtgggcgattcactatagcctggcttacaccagctggagtcagttccagcagctgaaagcgacctcaaccagtggcgacacgctgttccagaaacatgaaggctttaaagatgcttaccgcatcgcgttgggtaccacttattactacgatgataactggaccttccgtaccggtatcgcctttgatgacagcccagttcctgcacagaatcgttctatctccattccggaccaggaccgtttctggctgagtgcaggtacgacttacgcatttaataaagatgcttcagtcgacgttggtgtttcttatatgcacggtcagagcgtgaaaattaacgaaggcccataccagttcgagtctgaaggtaaagcctggctgttcggtactaactttaactacgcgttctgataacgcgttcgcctggataaagtcacctgcatagcaggtgactttaactcccccacttcaccgaaagtagtgtcctcattgcttacctcctgagttttgcaaacagcctgttggcagcttgccctttcaaatcaataagcggtatccacagacaaacctgaagggaaaggcatattttcaggcgttctgctcgtccttctcaaagagtttacttttctgcatttccaggatactccccccccctggctattgtgcgctcatacactcaaattaaagataggttctaaataaatgagcgttttttgatagtctatttcattaggtaatatatatttgtaacaaatcaatcaaaatggaataaaatcatgctaccatctatttcaatcaacaataccagcgcagcttacccagaatccatcaatgaaaataacaatgatgaagttaatggattagtacaagagttcaaaaacctttttaatggtaaggaaggaataagcacctgtattaaacatctacttgagcttataaaaaacgccatacgagtaaacgacgatccttatagatttaatattaataattcctcagttacttatattgatattgactccaatgatacagaccatattactattggtatcgacaaccaagaaccaatagaattacctgcgaactataaagacaaagaactcgtccgtactatcattaatgacaacatagttgagaagactcatgatatcaataacaaggaaatgatcttcagcgcattaaaagaaatatatgatggagatcctggttttatcttcgataagatatcacacaaactcagacatacggtaacggaatttgatgagagcgggaaaagcgaaccaacggacttatttacctggtacggtaaagataaaaaaggcgactctctcgctattgtaattaaaaataaaaacggaaatgattacttatctctcggttactacgatcaggacgactaccacattcaaagaggaattcgtattaatggtgatagtctcacccaatattgtagtgaaaacgccaggagtgcttcagcgtggtttgaaagcagtaaagctatcatggcagaatcatttgcaactggttccgatcatcaggttgtaaacgagctcaacggggaaagactgagagaaccaaacgacgtttttaaacgttatggtcgagcaataagatatgattttcaagtggacgatgcaaaatataaatgcgaccatctaaaagaaatagtttctactttagtcggtaacaaaattaacgttggccattctcaaaaaatatataagcattttaaggatctcgaaggtaaaattgaagaaaggcttcaaaatcgccaggctgaatatcaaaatgaaattaatcaaccatctgcgccaggtgttaattttgatgatatttaaaattatttttccagttttttgatttttcaacagctgaatatcggaaatagtcagtgacgaacatcagtatttttacataattacgtctaggtcattgtcggtttatctccttttacttgtggtaattgagggataacaacaaaaaaggtgagttttgcgactcaccttttttatttgtttcttattcagaatcaatatcttttaaatcatcctgaatcgcttgtgcgttcggattttcctgcggtttgagttcgccgccattagcgatgaaatcatgacgctggaagtacgcttcgcgcaccataatataaggatcggacgactgacgcagcagaccatcggaatccagcagctgagcgcgggtttcgatcccttcaagcgtccatttacccacagacatcggccaggtcagccaggaaagaaccgggtaaaaaccatccgccatatcaccaccgtcatcacgcagcgtgaagctaccgtagaacggtaactgaacgtaaggcccataacccacgccataatgaccaagcgtactaccgaagcggtgaggttcagtccgttgcagtttcgggttcgccatccctgcaacatcaataaaaccgcccatccccaaaatggtgttcaggaaaaagcgggtaaagtggaccatcccctgataagggtcgccctgcaagaagtagttaaccatcaccgcaggttcttcaaggttgccagtaaagttgctcaaaccgttacgcgccggttgcggaacataatcacgccaggcgacagcgaccggtcgaacaatatacgggtctaatacattgaagttgaagttgtacatggtgcggttgaacccttctaacgggtcagaacgcccttgctgatctgtaccggaactcgcacaccccaccagaagcgtagttcccagagcaagcgccgacaggcgaagcttcataaatgtctccctgtttttttatggcttatgcagtttgccatccatgacggaacgataccgtatccgcctgtttaggtgtgggcgattgtaacagcacgtcaactgatgtccagacgccctgatttgctgatttgatcatagcctggtaatcgccgccctgtaggctacttgattctatagaaacagaaaaaggcaaacgcagccttttctacattttcagagtaactcccgtcagttgcgagcaaaaaagccgctacgctttagctatacgtgctaattcaagagaagagaccatggacaacgacaaaattgatcaacacagcgacgaaattgaagttgagagcgaagaaaaagagcgcggcaaaaaaatagaaatagatgaagaccgactcccctcccgggcgatggcaattcatgagcatatccgccaggatggtgaaaaagagctggaacgcgacgcaatggcgctactgtggtcagccattgcggcgggtctgtcgatgggcgcttcgttactggcaaaagggatatttcaagtcgaactggaaggtgtgccgggcagcttcttgctggagaatctcggttatacctttggttttattatcgtcattatggcccgccagcaattatttaccgaaaataccgtgactgcggtactacccgtcatgcaaaaaccgacaatgagcaacgtcggcttacttatacggttatggggcgtcgtgctgctgggtaatattctcgggacaggtattgcggcgtgggcatttgaatatatgcctatcttcaatgaagaaactcgcgatgcatttgtcaaaatcggcatggatgtgatgaagaacacccccagcgagatgtttgccaacgcgatcatttccggctggctgatcgccactatggtttggatgtttcctgcagcgggtgcggcaaagattgtggtgattatattgatgacctggcttattgccctgggtgacaccacccatatcgtggtcggttctgttgaaatcctctatctggtgtttaacggtacgctgcactggagcgatttcatctggcccttcgcactacctactttagcggggaacatctgcggcggcacctttatcttcgcgttaatgagtcatgcacagattcgtaacgacatgagcaataagcgtaaagcagaagcacgccaaaaagcagaacgtgcggaaaacattaagaaaaattataaaaacccggcataaatggcgagggtttaagcaatcgagcggcagcgtacttaccccgcactccattagcgggtatactcatgccgcattgtcctcttagttaaatggatataacgagcccctcctaagggctaattgcaggttcgattcctgcaggggacaccatttatcagttcgctcccatccgtaccagtccgcaaaatcccctgaatatcaagcattccgtagatttacagttcgtcatggttcgcttcagatcgttgacagccgcactccatgacgggtaaaaagtggataaaataattttacccaccggatttttacccatgctcaccgttaagcagattgaagcagcaaagccgaaagaaaaaccataccgccttctcgatggtaatggcctgtacctttatgtccctgtgtcagggaaaaaggtatggcagcttcgctacaagattgacggtaaggagaaaatcctgaccgtcggaaaatatccgcttatgactttgcaggaggcaagggataaagcatggactgcgaggaaagacatctcggttggcatcgatcctgtaaaggcgaaaaaggcttcgtctaacaacaattcctttagtgcgatttacaaggaatggtacgagcacaagaagcaagtatggtcagtagggtatgcaactgaacttgccaaaatgtttgacgacgacattttacctatcattggcggccttgaaattcaggatattgagccgatgcaactgctggaagtaatccgcaggtttgaagatcgcggtgcaatggaacgagccaacaaagcacgcagaagatgcggcgaggttttccgttacgctattgtcaccggaagggctaaatataacccggcacctgaccttgctgacgccatgaagggataccgcaagaagaacttcccgtttcttcctgcagaccagatcccggcattcaacaaagcactggcaacattttcaggaagtatcgtatcgctcattgcgaccaaagttttacgctacacagccctaagaacgaaagagcttcgttccatgctatggaagaacgtcgattttgaaaataggattatcaccatcgacgccagtgtgatgaaaggacgcaaaattcatgtggttcctatgtcagaccaggtagttgaacttctcactacgctaagctccatcaccaaaccagtctcagagtttgtttttgccgggcgcaacgataagaagaagccaatctgcgagaacgcggtactgcttgtgatcaaacaaatcggctatgagggtctggaaagcggtcacggattcaggcatgaattcagcacgattatgaacgagcacgaatggcctgctgacgctattgaagtgcaactggcacatgcaaacggcggatctgtgcgtgggatttacaaccatgctcagtatctcgataaacgcagagaaatgatgcaatggtgggcggactggcttgatgagaaggtggagtgagcgaccttaacaactatcgaatagcacaaagtcttgcaatccagtgcaaagctttgtgtgtataagttttgtctcatcaaccacagcaagtatcgatcgattaagacttggatgatagacttcattcctttgattattagctgatagaagaaatgttaaagctatttgcaaagtacacctctattggtgtgctgaacacccttatacactgggtggtttttggtgtttgtatctatgtcgcgcatacaaaccaagctcttgcaaacttcgcaggtttcgttgtggctgtgagctttagcttcttcgcgaatgcaaaattcacattcaaggcatcgactacaacgatgcgctacatgctatatgttgggttcatggggacactgagtgctactgttggatgggctgctgatagatgcgcacttcccccgatgataactcttgtcaccttctccgccatcagcctggtgtgcggtttcgtctattcaaagttcattgtctttagggatgcgaaatgaagatatctcttgtagttcctgtcttcaatgaagaagaagcgataccaattttttataaaacggtacgtgaattcgaagaattgaagtcatatgaagtggaaatcgttttcataaatgacggcagcaaagacgctacggagtcaatcattaatgctctggctgtttcagatcctctagttgttccgctgtcatttacacgcaactttggtaaagaaccagcattgtttgcagggttagaccatgcaaccggggatgcgataatcccaattgatgttgacctgcaagacccgattgaggttattcctcatcttattgaaaaatggcaagcaggtgctgatatggttcttgctaaaagatctgaccgctcaactgatggacgcctgaagcgaaaaacggctgagtggttctataagctccacaataaaataagcaatcctaaaattgaagagaatgttggtgatttcaggctgatgagccgtgatgttgtcgaaaatattaaacttatgccagaacgaaaccttttcatgaaaggtattctgagctgggtaggaggaaagacagatattgttgaatacgtgcgagcggaaagaattgctggagatacaaaatttaatggatggaaactttggaatttagcacttgagggtattacaagcttttccacattccctcttcgcatctggacatacatagggttagtggtagccagtgtagcatttatttatggggcgtggatgattttagatactatcatatttggaaatgctgttaggggatatccttcactacttgtttcaatactgtttttaggtggaattcagatgattggaataggagtattaggtgaatatattggacgcacatacattgaaaccaaaaaacgcccgaaatacatcatcaagagagtcaaaaaatgaataaagcaataaaagtatcattgtatatatcttttgttttgattatttgcgccttatctaaaaacataatgatgttaaatacatctgatttcggaagagccattaagccattaattgaagacataccagcatttacatatgacttacctttattgtataaattgaaaggtcatattgattcaattgatagctatgagtatataagttcatatagttatattttgtatacatacgtcctgtttattagcatttttactgaatatcttgatgctagggtgttatcgttatttctaaaagtaatatatatttattcattatatgcgatatttacttcatatataaaaacagaaaggtatgtaactttatttacattctttattttagcttttcttatgtgttcttcatcaacactgtcaatgtttgcatcattctatcaagagcaaatagttataattttccttccatttttggtgtattcattaacatgcaaaaacaataaatctatgcttttgctatttttttcgttgctaataatatctactgctaaaaatcaatttatattaaccccactaatagtgtattcatattatattttttttgatagacacaaactaattattaaatctgtaatatgcgtggtgtgcttgcttgcgtcaatatttgcaatatcttattcaaaaggtgttgttgaattaaataagtaccatgcaacatacttcggtagttatctttatatgaaaaacaacgggtataaaatgccatcgtatgttgatgataagtgtgttgggttagatgcctggggtaataaattcgacatatcatttggcgcaaccccaacagaagttggaacggaatgtttcgaatctcataaagatgaaacgttttcgaatgcactctttttattggttagcaaaccaagcaccatcttcaaacttccatttgatgatggtgtgatgtctcagtataaagaaaattatttccatgtatataaaaaactacacgtaatatatggagaatcaaacatactaacgactattactaacataaaagacaatatatttaaaaacattagatttatatcattgttattattttttattgcttctatttttattagaaataataaaataaaggcatctttatttgtagtatctctttttggaatatctcaattttatgtgtcatttttcggggaaggatatagagatttaagcaagcatttatttggaatgtatttttcgttcgacctttgcttatacataacagtcgtttttttaatttataaaataattcaaagaaatcaagacaatagcgatgtaaagcactaagtttaaattgcgcgccaatcatggcgcgcacaagctataataccaacctaatttctcctcctcttagagtgactatatctcctgatagaattgcggtattgactatcaaatgccctgattcgttgtttattgtaatatctcctctatctgcagacgataacttaaatgcatcattgcccacaacaaaccccctccagaaccaagtgctgatattatcatcaacagtgatagatacatatactaactgattatcgttataagtgattcctgtcttatacttaacataaggacttccactttgattctcgatagacacataacatccaggggttatgtttgtatgcgtcccgcgactatcgccccattaacgccatacgataaatgggatggtgagaaatgggtgacggataccgaggcacagcatagcgtcgcagtagatgcagcagaagcacagcgccagtcgctgattgatactgcaatggcttccattagtctgattcaactgaaattacaggctgggcggaagctgatgcaggcagagacctcccgacttaacactgtgctggattacattgacgcggtgacggcaacagataccagcaccgcgccggatgtcatctggcctgaactgccggaggagtaggccattcaatatctggcgcactggaagtatcgaccagctccagtgcgtccagataatccagccacaaattatattgcgccagttcctcacctttcagacgaccaatagccgctttaccagcccattgtttactgttcatataatcgttggcctgattaatcaattgctgctttttcagttcggctgcagcaatctgttcctcatgtgttggtggtggaatttcagaccatgcaggaaaaccattttctccagcgatacggatttttcctttcggcggtaatccggaaaactcaatatacacttgctcatcaacttcaacagcatcatctggccatgagccagcttgcgtgtaatcctctttcatctccaagggatagaaagagtttgtagtcgcggaatatatgtaattcatttttcactccataaagttaaaagaaattaacaccctaatgcgaaaaatgaagcaccgataccgggtacgcctgctctggaaataaatttcaccgggtcctggttataaccggcacaagctatatagccaacatttgcactgccgggagtgtaatcctgagtcgcaaatacccgcagacatctattcggaaatgcaatcggaaaataggttactgtgtcctgagacgtcagcggaacatcaattggcccccattgaataattaaaccggatggcaatttttgatatccaggaactgaagcagaaagcataaaactacccatatcaggtatctgattcgcccctgtccctacatttcttttagccgcttctcccaaaccaaggttttcgagagccttttgcaccgtgccgtccaatttgatatcgccaaacggattcttgcggcttaacagcagcgcacgaagcgcggtaagcagctggtcatgccgccccttctccaggctggcaccggaggcctccacaacgctgcaaagctcctcctgcaacatgtcaaagtagtcatcatccagatcggtggcaggcgtgccggtctgggggttaccacgggtacgggggattaccaaaggcagcacctttaagctccgcaagacgttctgaccagtcatgcgccagcgcgttgtcttccgcagtgtaatacgcggcacatttggcgttatcaccatcagtaaacagatccagaacaaacgggccaaacagggtgttaattccccagaaaatgttgtccggcgtgcgccactgatcgcccacttccttcagttcatgggctggtttgttccgcagctccaccagcgcctggcaatatttattactcattaagcccccacgtaattccctgagagataccactcttcacctgatgcagcccgcttactgcttttccgtaaacaccgttcacgacgcgccagaaaattgtttcgttctggctgggagtggctttcacggaatgccgccatccacaccgttgcagcacgacggtataagcccctggactccagttcttccgcctggcgggtcaggcacaaaatcacccgcgggtcgttagtgccgacatagaaattgcgcacaggtctggtttcacgaactggttgtggttccggatcctgcgctctctcagtcaggcgcgggaaatgtctgtgtgtatctccttcacaacggtgagccacacgcccactctgacgtaacttgcttgctgactgcagaacgcgctgccgtgagtaacctgcaaaagcatccgcaatgtctccggaagtacagcccggatgggcttcaatgaatttctgaacgtcattcaaaagactcatgctcaccccctgaatcctgccgggatctggctgtagtccacattgtcgtaactggctttgaagtacgggtcttcgcgtttttctgtgtacgtgctgacggacggcgataagcgcagggaaagctcatcccatttttcccgcagcttcgacgggctgagcacgttacggcaccagaacggatcgcggctgacgcggctgtacatctcgcagatttgtttgtgagtacgaccatcctgcacacacatcaggcgaatttcgtttgcccaggctgtccagttcggttctttgggacgaaccacctcgccgtcacattcggcggcctgctcgtacagggcgatgatttttttccagagccactgtgcgcaggtcaaatcatcctgcgttccccactggcgctttttagggctgaatacaaccgcatcaggatggcgagttaaaaaatcctgttcatccgtctgcgtgtccggttgcgaagcgtccggacgagaaggttttttatctgacggatcatgttttgattttactgacggatccccgccagattctgacgggtgaaaacccgattttttgccagatttcgacgcatcaaattttgacgggtcagattttgatgcgtcagattttgacgggtcagagtctgacagttgagaaaatgccgctgcctgaagcttcgcaacgttaagctgataaacattcgacgcattgcggttatgatgaggagcagcaaaatggctagcgaacgcagtactgatgtgcaggcatttatcggggagctggacggcggcgtatttgaaaccaaaatcggcgcagttctcagtgaagtcgcttccggtgtgatgaacacgaaaaccaaaggtaaggtctcactcaacctggaaatcgaaccatttgatgagaaccgtctgaaaatcaaacacaaactctcatatgttcgcccgactaaccgtgggaaaatttccgaagaagacaccaccgaaacgccgatgtatgtcaatcgcggtggtcgcctgactattctgcaggaagaccagggacaattactgactcttgccggtgagcctgacggaaaactccgcgcagcaggtcattaatatcattcttaattaactaattatttatctcatcactgaatatcttaatatagtgaggacttattatgtctcagaacttagacgcaaccgcaattaatcaaatccatgcccttatttctgctcagggtgttaatgaaattatcagtaagattggtgccgatgctgtggcattgcctgagaatttccgcattcatgatctggaaaaatttaatttaaatcgcttccgtttccgtggtgcgctttccactgccagcatcgatgactttacccgttattctaaagatcttgcagatgaaggcacccgctgctttatcgatgctgataatatgcgtgccgtcagtgtgcttaacctgggtactattgatgaaccaggtcacgcagataacaccgccactctcaaactgaaaaagacagcaccgttctctgccctgttgtctgttaacggcgagcgtaactcccagaaatcactggcagaatggattgaagactgggccgactaccttgtgggctttgatgctaatggtgacgccattcaggcaacaaaagcggctgcggcaatccgtaaaatcacgattgaagcaaaccagaccgctgattttgaagataatgacttcagcggcaaacgctccctgatggaatctgtcgaagcgaagaccaaagacattatgccagtggcatttgaatttaaatgcgttccgtttgaaggtctgaaagaacgtccgtttaaattacgcctcagcattatcactggcgatcgtcctgtactggttctgcgcattattcagctggaagcggtgcaggaagatatggctaacgaatttcgtgatctgcttgttgagaaattcaaagacagcaaagtagaaacctttattggtactttcaccgcctgatttcattactgcaaatgcccctgcgggggcatttatggaaacgtaattaactcaataatcaccggatggtgagggcttccttttacccaaactcagcgcggtgcagcgcatatacgtggagaacaaaatgtcatttattaaaactttttccgggaagcatttttattatgacaagataaataaagacgacatcgtgattaacgatatcgcggtttccctttcaaatatctgccgctttgccggtcatctttctcacttctacagtgtcgcccaacatgcggtgctttgcagccagctggtgccgcaggaatttgcttttgaagcattaatgcatgatgcaacagaagcgtattgccaggacatccccgcaccactgaaacgccttcttcctgactataaacggatggaagaaaaaatagatgcagtaatccgtgagaaatacgggttacctcctgttatgagcacgccagtgaaatatgccgatctcattatgctggcaaccgaacgccgtgatctcgggcttgatgatggctctttctggcctgtactggaaggcatcccggcaacagagatgttcaacgtgattccactggcaccgggtcatgcctacgggatgtttatggaacgttttaacgatttatcggagttacgcaaatgcgcatgaatgttttcgaaatggaagggtttcttcgcgggaaatgtgtaccgcgagatctgaaagtgaacgaaacaaatgctgagtacctggtacgtaaattcgacgcgcttgaagctaaatgtgcggcactggaaaacaaaataataccagtgtcagctgaactgccaccagcaaatgaaagtgttctgttatttgatgctaacggagaaggctggctgattggctggcgttctctctggtacacctggggacaaaaagaaaccggagaatggcagtggacatttcaggttggggaccttgaaaacgtcaatatcactcactgggcagtaatgccaaaagcaccggaggctggagcataatgaccacatttaccaataaagaactgattaaagaaatcaaagaacgaatcagcagcctagaggttcgagacgatattgagcgccgtgcttatgaaatcgcactcgtatctctggaagtagagccagatgaacgcgaagcctatgaattattcatggaaaagcgtttcggtgacttagtagatcgtcggagagcaaaaaacggcgataacgaatacatggcatgggatatgactctcggttggatcatctggcagcaacgagctggtatccatttttcaacaatgtcacaacaagaggtgaaataatagagccatacagcctcacactcgatgaggcctgtcagtttcttaaaatatcctgatctaccatcgccgtcatagagcgtatttttattacctgatttgcaggttcgattccctattcggagatagcactcatgcaacacgaactacagcctgattcactggttgatttgaaattcatcatggctgatactggctttggtaaaaccttcatctatgaccggattaagtcaggcgacctgccaaaagccaaagttatccacgggcgagcaagatggttatatcgtgaccattgtgaattcaaaaataagctcttaagccgcgccaatgggtaaaatagcgggtaaaatatttctcacatctaaaaaacaccattccaatcaatcccctgctgcttcaagtagatgtctgcaggggacaccatccttgtgtttatccctaaaaccacataaaaaccgtaaattaaattcgaactagcaggccgaataaggcacaccaggaactcgtggttttattcattatgaagtggtttttacctgttctcttagccagataataaacgcttcaatttttggccactgcctgcccggtaatgtggtgatgtaataatgctgatggcatttcaccgtcatatcgccaaacggcgcgacgagctcaccactggcaagccttttttgtaccaggcgttttcttcccatcgccaccccaatatgattcatcgcggcaataacagctaaatcagaacgatcaaagccaattccagaagatgtcggcaaattaaccgcataatgttgcgcccaactatgccattcatccgtaccggagtcgttgctccatgcctgtctgtcatggagcaacgtacagtgacacaggttaattaccgtgttggttaaagcatgtctttgagcgtattccgggctacatactggcaggatttcttcatccatcagaaagtgatgagtgagttgcgctgacggcgcatcatcaaagtagatcgccaaatcgattccggcacgttgcagattgacgttgtcattaccagtgagcacggtgagcgaaatagacggataccggcgtgtaaagtcacctaatgcgggcaccaaccagcattgggcgatagagggccgggaatacagagttaacgttcccgataactcctgatttttgatatcaagaatttcctggttcagggtatccagcgacgattttagcgcccaataaacacgtttcccctcgtgcgttaattccactttgcgatgggaacgaacaaacaactgaatgcccaattcttcttccagctgattgatacggtgacttaccgcactggggctcagcgacaattcctctgccgccagggcgaaggactgatgcctggcagccacttcaaaagtatgcatttttgataattgccagccgttaagcagccgatttcttatttcacgaaggggttccataatcacctcatttttcgcttaagtgtaaaaaaatagcggcaaaatttcagctatgagatgagctaaagtgaaccatatctcaattcaccttcatttttagatgtaaatcactccattgatgcaatttacctcatgtgaaaggcaaattttatcgtttgtcagcctgcgttgtttttttgtccaatatcatcaggttaatcacaggggaaggtgagatatgcactctcaaatctgggttgtgagcacgctgcttatcagcatcgtgttaattgtactgaccatcgtgaagttcaaattccacccgtttctggcgctgttgctggccagcttcttcgtgggaacgatgatgggcatggggccactggatatggtaaatgctattgaaagtggaattggcggaacgctggggttcctcgcagcggttatcggccttggcacgatactgggaaaaatgatggaagtatccggggccgcagaaagaattggtctgacacttcaacgctgccgctggctttcagttgatgtcattatggtgctggttggcctgatttgtggcatcacgctgtttgttgaagtgggcgtcgtgctattgattcctctggctttttcaattgccaaaaaaaccaatacctcattattaaagcttgccattccgctatgtaccgcattgatggcagtgcactgcgtggttcctccacatccggctgctttatatgttgccaataagctgggcgcagatatcggttcggtgatcgtctacggtttgctggttgggctgatggcatcactgatcggtggcccacttttccttaaatttctgggtcaacgactgccctttaaacctgtacccacagagtttgcagatctcaaagttcgcgatgaaaaaacactaccgtcattaggcgcaacgttattcaccatactgctacccattgcgctgatgttggttaaaacgattgccgaattgaatatggcgcgtgagagtggtttgtatatcttggttgagtttattggcaaccctatcactgccatgtttatcgccgtgtttgtcgcctattatgtgttgggtatacgccagcatatgagcatggggacgatgctcacacatacggaaaatggcttcggttctattgctaatattttgctgattatcggggccggaggcgcattcaacgccattttaaaaagcagcagtctcgctgatacgctggcagttattctctccaatatgcatatgcacccgattcttctggcctggttagtggctcttattctgcatgcggcagtgggctccgctaccgtggcaatgatgggggcaacggcaattgttgcacccatgctgccgctgtatcccgacatcagcccggaaattattgcgattgctatcggttcaggtgcaattggctgcactatcgttacggactcgcttttctggctagtgaagcaatattgcggcgctacgctcaatgaaacatttaaatactatacgacagcgacatttatcgcttcagtcgtcgctctggcgggcacattcctgctgtcatttatcatctaagcgcaaagagacgtactatggaaaacgctaaaatgaactcgctcatcgcccagtatccgttggtaaaggatctggttgctcttaaagaaaccacctggtttaatcctggcacgacctcattggctgaaggtttaccttatgttggcctgaccgaacaggatgttcaggacgcccatgcgcgcttatcccgttttgcaccctatctggcaaaagcatttcctgaaactgctgccactggggggattattgaatcagaactggttgccattccagctatgcaaaaacggctggaaaaagaatatcagcaaccgatcagcgggcaactgttactgaaaaaagatagccatttgcccatttccggctccataaaagcacgcggcgggatttatgaagtcctggcacacgcagaaaaactggctctggaagcggggttgctgacgcttgatgatgactacagcaaactgctttctccggagtttaaacagttctttagccaatacagcattgctgtgggctcaaccggaaatctggggttatcaatcggcattatgagcgcccgcattggctttaaggtgacagttcatatgtctgctgatgcccgggcatggaaaaaagcgaaactgcgcagccatggcgttacggtcgtggaatatgagcaagattatggtgttgccgtcgaggaaggacgtaaagcagcgcagtctgacccgaactgtttctttattgatgacgaaaattcccgcacgttgttccttgggtattccgtcgctggccagcgtcttaaagcgcaatttgcccagcaaggccgtatcgtcgatgctgataaccctctgtttgtctatctgccgtgtggtgttggcggtggtcctggtggcgtcgcattcgggcttaaactggcgtttggcgatcatgttcactgcttttttgccgaaccaacgcactccccttgtatgttgttaggcgtccatacaggattacacgatcagatttctgttcaggatattggtatcgacaaccttaccgcagcggatggccttgcagttggtcgcgcatcaggctttgtcgggcgggcaatggagcgtctgctggatggcttctatacccttagcgatcaaaccatgtatgacatgcttggctggctggcgcaggaagaaggtattcgtcttgaaccttcggcactggcgggtatggccggacctcagcgcgtgtgtgcatcagtaagttaccaacagatgcacggtttcagcgcagaacaactgcgtaataccactcatctggtgtgggcgacgggaggtggaatggtgccggaagaagagatgaatcaatatctggcaaaaggccgttaataacgtttcaacgcagcatcgcaatcctttccctgggtgagcgatgctgccgatggcgcagacttaagatccccggtcttacccgctataaccccctccttttatcatcacccaacgcctttcgctgtaaacggcggtttcgcaaaccaaaccaaaaccgtaagtaagataaaagcaatagccgccatacggaaaatctcatttgcagaaatagaaagtgactgctgggttatttcattattaatttcattaagaactcctgaaagcgaaccataatatttatccataatttgtgacgatgaattaaacacggggttaaattgatcgatggttgctgtcaactgactatggtgtaacgattcgcgtcgtccccacagcgtcattgtcaacgacgtaccaactgatcctgacaaggtacgaaaaaaattactcatactcgaggcattggcaaatttattatctggcaagcctgaaaacgaaatcgttgttaagggtaaaaagaaacaggcaacggcgaatccctgaaaaaactgcggcaaaatgatgcctgtaaaatcaatcgttggcataaatgtcacagaacgccagtaatagcaaaccgcatacatcaaaaaactaaatgtcactaacaaccgcatgtctattttgttgccataacgtcctatcaaaggtgaaattaatagtggcatgatgccgatgggcgcataagcaagtccggcccatatcgcattataccccatcgtttcctggagtaactgcggcataaggacgatcgctccagagtaaaataaatacgcgcatgtgatactcacaataccaatggtgaagttacgggacttaaacaaactgagatcaagaatcgggttctctgaggtcgactcccaaatgactaaagagatcagagaaataactgatactactgttaatattattattgtactcgagttgaaccaatccagatcgcgccctttatcaagcataatttgcaagccaccaacaccgagcactaacagggtcagtcctggtagattcattttgaccggtgaagtctcagtttctcttcctttaagtaaggttaagcataatgtcaggacgataatccccatagggacattgattaaaaatatccaaccccagctaaagttatcacaaatataaccgcccaatatcggcccacatatcggagcgataatcacggtcattgaccataatgccagagcaaatgttcttttttctggcggataattccttaataataaactctgtgacagtggaattaacggccccgccattaacccctgaacgactctaaaaaatatcagcacatcaagattggtcgataggctacacattaatgaagacagcgaaaaaaaagtgactgaaagtaaaaataatcttaattcgcctattctttgtgccaacctgccagtaacagggatcgcaatggcatttgctacaccaaacgaggtgataacccaggtgccttcgtctgttgatgctcccagaaagccagatattgtcggtattgcgacgttagaaatagtggaatccaacatttgcataaatgtcgctaatgacaatgcaatagtgacgcaccataacgtcccaccggttaatggtgccggagttgatttagtgattgccattaaagttgtccattatgcgaaataatgttgctaatttctttttctatcggactggtatcgataactaaagccttactggtataagccggcatggaggtcacggttgaagccagctcaggcatctcggcaatgtcttcgttcttcgtatcaatagttgctgtcatcgataaaccaatacgcaaggggtgttccatgagttcttttggatcaagagaaacttcaaccggtacacgctgaacgattttgatccagttccctgtcgcattttgtgcaggtaataaggagaacgcattgccggttcccatattgatccctgtcacccgaccatgaaacacaacattttcaccataaagatcgctgataatattgaccgattgaccaatccgtacatccgtgagttgtgtttctttaaagttggcattaacccacatttgacgtgccggtacgacagccattaacgattgtccggggctcactgtttcgccgacctgaacacttctctgggcaatatagccggtaaccggactcttaatatccgtacgtttaagcgccaaccaggcttctttagttgcatccgccgcttcaacgacttgtggctgacggtttaatggtgtgttcattactaaagctttattcgctttataagcctggatagcggcattcaatgccgctttgctacttattaacgtatctttggtatgctccagcgtttcttttgaaataaccccctgcttcgctaacggcactcgacggttataatcttctaaagattgttgatactgaatacgtgctgaagcgacttcggcactgtattgtttatcctgtaagtatagtttattcgtttgccgaacaatatttgccagattatttttagctttattgagtgcgatagtggcatcagttttatccagtgaaactaaaatgtcaccttgtcgaacgtagttcgtatctttatgattaacgacagtgacactacctgagacttgtgcagaaattggatctgcattccccgtgacataggcgtcatctgtactaatcatgtcttctaattccattgaccaataggcataggcacctgaaaacgcaataaataaaactaccgccaataaagaaaagtattttcttctgttagaatgttttttatttgaattaatctgttccactattatctctcatttctcatagatgaaatttatgaattgaatgaaaagagcattcattcttcatatcaaacacagtgcatgtgttgcacattatcccaggaacgttggaggcctaatttaaatgaggtgcaaaaaaaacaacagaggactaaaccgtggcttttgcaatacaattcttacgcctgtaggattagtaagaagacttatagtgccaacttgaaactataaatcatcggtacaatccctgattttattgttgacatttcatttatgccgactatttatatggtatacttgtcgaattatcttaaaggaagctcagattttcttatttttattgagaaaatgagatgacgccttatgtctgtattactacagggagaagggagatgcttcattgcaaagggaataatctatgaacgcaataattattgatgaccatcctcttgctatcgcagcaattcgtaatttattgatcaaaaacgatattgaaatcttagcagagttgactgaaggcggaagtgccgttcagcgggtggaaacacttaagcctgatatcgtcatcattgatgtcgatatccccggagttaacggtatccaggtgttagaaacgctgaggaagcgccaatatagcggaattattattatcgtctccgctaaaaatgaccatttttacgggaaacattgtgctgatgctggcgctaatggtttcgtgagtaaaaaagaaggcatgaacaatatcattgcggctattgaagctgcaaaaaatggctactgctatttccccttctctctcaaccggtttgttggaagtttaacgtccgaccagcaaaaactcgactccttatcgaaacaagaaattagtgtcatgcggtatattcttgatggcaaggataataatgacattgctgaaaaaatgttcatcagcaacaaaactgtcagcacttataaaagtcgcctgatggaaaaattagaatgtaaatcactgatggatctttacacattcgcacaacgtaacaaaatcggctaaccacatgaagtttttaccctatatttttcttctctgttgtggtctttggtcgaccataagtttcgcagacgaagattacatcgaatatcgtggcatcagtagtaacaaccgtgtcacacttgatccactacgtctgagcaacaaggaattacgttggttagcgagcaaaaaaaatcttgtgattgcagtacataagtcccaaacggctacgttgttgcataccgattcgcagcaacgggttcgtggtattaatgctgattatttaaatcttttaaaaagagcgttaaatatcaaattaacactccgggaatacgcagatcatcaaaaagcaatggacgcgcttgcagaaggtgaagtcgatatagtgttatcacatttagttacttcgccgcctcttaataatgacattgctgcaaccaaaccattgataattacctttccggcgctggtaaccacccttcacgactcaatgcgaccgcttacctcaccaaaaccagtaaatattgctcgggtagcaaattaccccccagacgaggtaattcatcaatcatttccaaaagcaacaattatctcttttacaaatttatatcaggcattagcatccgtctcagctgggcacaatgattactttattggtagtaacatcattaccagcagtatgatttcccgctatttcactcactccttaaatgtagtgaaatattataactcgccgcgtcaatataattttttcttgaccagaaaagaatctgtcattcttaatgaagtactcaatagatttgttgatgctttaacaaatgaagttcgctatgaagtatcacaaaattggcttgatacaggaaacctggcctttctgaacaaaccattagaactcactgaacatgaaaaacagtggattaagcagcatcccaatttaaaggtgctggaaaatccttactcgcccccctattctatgacggatgaaaatggctcggttcggggcgttatgggggacattcttaatattattaccttgcaaacaggtttaaatttttctccgatcaccgtttcacacaatatccatgctggaacacagcttagccccggaggatgggatataatacctggcgctatttatagtgaagatcgagaaaataatgttttatttgctgaagccttcataacaacgccttacgtttttgtcatgcaaaaagcgcctgacagtgaacaaacattaaaaaaaggaatgaaagttgccattccatattattatgagctgcattcgcaattaaaagagatgtatccggaggttgaatggatacaggtcgataatgccagcgctgcatttcacaaggttaaggaaggtgaacttgatgctctggtcgcgacacagctaaattcgcgttacatgatcgatcattactatcctaatgaactttatcattttcttattcctggcgttccgaatgcatcgctttcgttcgcttttcctcgcggagaaccggaacttaaggatattattaataaagcactgaatgcaattcccccaagcgaagttctgcgcctgacggaaaaatggattaaaatgcccaatgtgaccattgacacatgggacctatatagcgagcaattttatattgttacgacattatccgttttattagttggcagtagccttttatggggattctacctgttacgctcagttcgtcgtcgtaaagtcattcagggtgatttagaaaaccaaatatcattccgaaaagcactctcggattccttaccgaatccaacttatgttgtaaactggcaaggtaatgtcattagtcataatagtgcttttgaacattatttcactgcggattactacaaaaatgcaatgttaccattagaaaacagtgactcaccctttaaagatgttttttctaatgcgcatgaagtcacagcagaaacgaaagaaaatcgaacaatatacacacaggtatttgaaattgataatggcatcgagaaaagatgcattaatcactggcatacattatgcaatcttcctgcaagtgacaatgcagtatatatttgtggttggcaagatattactgaaacgcgtgatctaattaatgcactcgaggtagaaaaaaataaagcgataaaggctaccgtagcaaaaagtcagtttctggcaacgatgagtcacgaaataagaacaccaataagctctattatgggcttcctggaacttctgtcgggttctggtcttagcaaggagcaacgggtggaggcgatttcacttgcctacgccaccggacaatcactcctcggcttaattggtgaaatccttgatgtcgacaaaattgaatcgggtaactatcaacttcaaccacaatgggtcgatatccctactttagtccagaacacttgtcactctttcggtgcgattgctgcaagcaaatcgatcgcattaagttgcagcagtacgtttcctgaacattacctggttaagatcgaccctcaggcgtttaagcaggtcttatcaaatttactgagtaatgctctcaaatttaccaccgagggggcagtaaaaattacgacctccctgggtcacattgatgacaaccacgctgttatcaaaatgacgattatggattctggaagtggattatcgcaggaagaacaacaacaactgtttaaacgctacagccaaacaagtgcaggtcgtcagcaaacaggttctggtttaggcttaatgatctgcaaagaattaattaaaaatatgcagggcgatttgtcattagaaagtcatccaggcataggaacaacatttacgatcacaatcccggtagaaattagccagcaagtggcgactgtcgaggcaaaagcagaacaacccatcacactacctgaaaagttgagcatattaatcgcggatgatcatccgaccaacaggctattactcaaacgccagctaaatctattaggatatgatgttgatgaagccactgatggtgtgcaagcgctacacaaagtcagtatgcaacattatgatctgcttattactgacgttaatatgccgaatatggatggttttgagttgactcgcaaactccgtgagcaaaattcttccttacccatctgggggcttacagccaacgcacaggctaacgaacgtgaaaaagggttaagttgcggcatgaacttatgtttgttcaaaccgttgaccctggatgtactgaaaacacatttaagtcagttacaccaagttgcgcatattgcacctcagtatcgccaccttgatatcgaagccctgaaaaataatacggcgaacgatctacaactgatgcaggagattctcatgactttccagcatgaaacgcataaagatctacccgctgcgtttcaagcactagaagctggcgataacagaactttccatcagtgtattcatcgcatccacggtgcggctaacatcctgaatttgcaaaagttgattaatattagccatcagttagaaataacacctgtttcagatgacagtaagcctgaaattcttcagttgctgaactctgtaaaagaacacattgcagagctggaccaggagattgctgttttctgtcagaaaaatgactaaatagcggctcccacaatgttcaaatgtgggagctatttaccagcacatcttacatttatgatgagaactcctggcgaatttgttccccatgctggtcgagcgttgccgctcccggcataacatgcgggtccgcgcagccgctgatttttatcggattacccggcatcattattcccccggcttcaatcaacatatttctcgcctgagtttgtggcaatttaatggcctcagccacacttaataacggcgcgacgggtacaccaacttcatgtattctggctaaccaaacttcagctgcctgcgtttttaacgtccgctcaatatattgtttaagaatagcctggttttgtacgcgtaaaatattgctgctaaatcggggatcattaaccagttccgtaagctccagtgcctggcataacgcagaaaaaagcttgtcattaccacaacaaatcgtaatcggcttatcctgagtattgaaaacatcaaaaggtgccatgtagggatggcgatttcccagacgttgtggtgacttcccagttgcgatatatgccatcagaccatgctccagaaaactcagcgtggcatcaaacatcgctatatcgacatgcgcccctctctggctcttttcgcggccataaagtgcactcactattccgctgaataaatagacaccgccgcatagatccgcaagagatgtaccaacgcgcactggcggagcatcaggatatcctgtttccatcattatcccgctcattgcctgaatgatggtatcgtaggcaggagcatcttttagcggaccggtatgtccgaaacctgacgatgaagcatatatgaggcgcgggttgatttcttgaagcgtttcccatgaaaaccccagtttttccattgtacctgggcgaaaattctcagctaatacatcagcttgtttgagcatatttataaatatacttttatcgtgatcattctttaaatcaagaaccacactctctttgccatgattaataaaactgtaatagagtgactgtccatccacatagggaccaaatgtgcgggtatcatcaccatgacccggcggctcaactttaattacccttgcgcccatattacaaagaagttgagttccgaaaggtccattaaggacatgtgtcatatcgataactaataagccttcaaacggccctttgctttcattatttgtcatttgcttatgccttgaaaaaagccgaaggtgaaaagacacttcggcatttatgtaaaatcaataacatgattaattatgaaaccagtcgactgacataaatccacaagggagccgtgacgacaaagcccagtacgctcacagccaatgacgctgtaccagtacgggtgtagacattaaaccggctggcaataatgattccggagaatgccggcggtaatgcgcctgccagtaccatcatctgcagatgttcgctgttcaaatgacatgccataccaacgagaagcagtgccagtggcatcagaatcagcttcaggaaggtgttataagcaatttcggcactgaactcgaatttatgtgcagccagagtcaaccccgcagcgaataccgctacccctgagttagccttcgcaatcagattaaaggttgggtcccatgctgccggaatttttaccccaaccaacaccaggatcgttgccagaacaggtgcccatactactggctcctttgccgcagaaattaatgcgctcagattactattcttcttaccatccgctcctgaagaaggattcagcaaatacagaccaataggaatagtaattgcgttaacaataatagaaataattgctaccactaaacctgttgatacggaatcaccataaataggatcgagaactgcaaaccccaggaatccaatggtaggtgaacctgcaattaatgcacatacagctgcttctgcatgggtacgtttaaaaaatttgtagcaaccgaaccaggagaaaaagaaacatccgacaataaccacaagtgatacaagggtcagacgagtgtccgcaaaaatcatttccctgtttgcccgagtaatagatacaaatagagccgcaggaagcgcgtagtttaataccagtttattaaatgcccgagcttgatcttctgaaaatgtttctcgtctgccgctaaaataacccaacagcatgattacgataataggcaataaatcgccaataaaaaatgttagcataatagtatttccgataagggtcccctcaccatcgcataatgagttggcaagaggagacgatgtcagtatttaattaccagcgacttgttttgggttaagtttggtaatatggccactttcagttcctgctgcagggtcgatgaccacattaataatggtcggtttgcgcgactgaataccggtggttaaagcatgacgaagttcatctgtcgtggtgacgttatagccaacgccacgaaacgcatccattaatttgtcataccttgcatggtgcaacagatccgttggtgatggtgcaccagcgccactgagatcaacaccgtctcctctgtagatgccgccattattaaaaataacgatcgtcaccggcaggttatatcgacaaatcgtttcaatttccatcccactgaaaccaaaagcactatcaccttcaatggcgacaaccggagaaccagaagtcacgctagcaccgatggcatagcccataccgatgcccatgacaccccaggtaccacaatccagacgacgacgtggtttatacatatcaataatatttcgtgcattatccagggtatttgcaccttcattaactaaataaatatcctggttctcgcgcaatacgtcgcgcacagcacttaatgcattaaagtaatttaatggttgagtatctgtacttaatttttcatgcattttttgtgcattttgctgcttgtggatatttaaaatatcgcgccataccagtggagtcgtaaatgtgttttgtttcagttctgccagcataccttgcatactggatgcaatatcaccaacgactggcacagcaatggggcggttgctgtcaatttcctgcggttcaatatccagttgaataaactgtgtatctgccgcccatccttttttaccgtgtgccaataaccaattcagtcgtgcaccaacaagcatgacaacgtcagcatttgccagggcaaacgaacgcgcagctgccgcagaaagtggatgcgtatcttcaaggatccctttcgccatagacattggcaggaatggaatctgagcactttcaataaattcacgaagctgttcatcagcttgtgaatacgccgcgcctttgccaaggataattaatggccgttcagcttttgctaaaagcgaaattgcgctagtgactgacttcgggcatggcaataatgctggcgacggattttcaactttaacaatcgtggttaacgcttcgtctttttccatcgtcgcggccaggacatttgctggcaaatcaagataaactccgccagggcgacccgatacagagacccggatagcgcgtgccaatgcaatgccaagatcctgcggctgattaacgcgaaatgctgctttggcatacggttttgccgcattcatttggtccagctcttcataatcaccttgctgtaggtcgacgatcgcgcggtcgctggagccgctaatcatgatcatcggaaaaccatttaccgttgcgttggccaatgcggtcaaaccattgaggaatcctggcgcagaaactgtcaggcagatccccggtttttgggtaagaaaaccgcttgccgcagcggcatagcctgccgactgctcatgacgaaaaccaatataacgaatgccttccgcctgggcatggcgtgccatatccgtcacaggaatacctacaacaccataaatagtgtcaatattattctgttttaatgcttcaacgatgatatgcataccatctgtcatttgaagttgatctgacatgattaataacctcgaaatttttataaattgggagccagaagcccccgttaatatcagatggcgtggttttgcttcattgcagcaatttcatcgtcgctataacccagctcctgcaatacagcagcggtatgttcacctaatagcggcgcagctttaatatccggcgtaaaggcagagaatttcattggacaaccaacggtcagatattttccacgcaacggttgttccacttcaacaacactgccactttggcgcaaagagggatcaagtgaaatttctttcatacttaaaaccggtgcacaaggaatatcaaactgagtcaaataggccaccgcttcatgtttatcaatagtgacagtgtatttttcgatttcagcaaaaatatcgaaaatatgtggctgtcgtgcatgggctgtactgtatgccggatcggtaatccattctggtttgccgatggctttacaggtgttttcccagttttgctcctgaatagtgaaataaatataggcgttaggatcggtttcccagcctttacatttcaggatccagccaggctgaccgccaccacctgcattaccaccgcggggaactgcatcaccaaatgtaccattcggatactgcgggtattcttccagataacccaatttatcgagacgctgctggtcacgtaatttcacgcggcaaaggttcaatacggcatcctgcattgacatggtgactcgttgcccacgccccgttttttcgcgatgcagcaaagcagcaagtaaaccgatcagcaaatgcattccggtgttgctgtcacccaacgctgcagcgcttaccagcggcggaccatcccaaaaacccgtagtggatgccgcgccacccgctgcctgagcaacgttttcataggcttttacattcacataaggcgaacactcatcaaaccctttgatcgaaccaaaaatcagacgtggattgatttcttgaatatgctcccaggtgaagcccatgtgatcaatggcccctggatgaaagttctcgactaagatatcagcttcgcggatcagcttttccattacctctttgccttccgctgttttggtatttaactcaatagaacgtttgttactgttaagcatggtgaagtaaagcgcatcgatatcaggaatatctcgcagctggtgacgcgttacgtcaccaacgccgggacgttcaattttaataacgtcagcgccaaaccaggccagcatttgagtacaagatgggccagattgcacaccggtgaaatcgagaactttaattccttgaagtggagttgacatagcaatacctattagttaattaaatatgtgttaatttagcgtttatttaaggcgtaatatcttctataaataacccgcaaaatatcgtcgtagctgcactcgatatttttaaaatcctgtatcaagtgctgaaaatcatttcatcgccacttccaattcctttctgcatggtaagtagtgaggacgaaaagaagaatatgataaatattgattcgtggtaatcagagagagtcgcgacatttgtgatgttattcttacaactgtaagaagcgccggtgatttacaagcaagggtatgattacgctttttaaagcgtaccataaaacataacataataaatgatttgtgatgacacgggattattgcggtttactttgaggaatataaaatgcgagtttatagcaccgcgagcgccaaataattttatgaccacaacctgtcgtattgtggtcataaaaaattgtcggctggagggagttaaatcctttacctcaatatactgcctgtcagcattagttcacaaacagtgcttcgctatcgacgatgattccatcttccgcacctttaagcgccaggtttgcctcgtagtattgctttttatcaagcagtttctgcgcatcagcaagtgcattacgagtctgtttaagtggcatcagatattggttttccattacgccaacaccggccaggcgaagctcttccattgcgccctttttatcccctttcgccattttttcattggcaatttttatcgcggcttctttttcgggagttgctacataactctcagaaattccgacagatgcattaatgacaatatattggtcatcattgagattggtctttttacctggcttagcgaactttgcccattcggtactgtcatctgacagcaaagcggaagcttcattggtcagttcttttgccttttctggatcgccatgaaacagagccaggcgcgctacctgcacgtcacgcatcgcatataaaccttgttcagagatacgctctgctgccgctgccgttttctgggtttgctgaacttgctgagtttgctgttgtgccgctaccggagcattatcagcagcccatacagttgaagatgccagaattgctgtgaccatcgtggccataattaaacgtttcatacttacctcattctttaacagttttagaaaacgccgccatcatattgggtgagcatgaaatgagaaatcagagagcaacggtcattttgaaagggttatcttacagttgtagttattatcgcaagaagtattttagtcttacaattgtaggaatatgcttcctgtcgcagagaactattcttatataccacaaagagatgtcatttattatatcgatgtaaatactgattaattaaatgtaaatacagccataacatcgtaggttctcagtgaaccattttcaggataactttctatgaaagtaaacttaatacttttcagcttatttttattggtctctattatggcatgcaatgtttttgcattttccatttcgggtggtggaagtgagaggagctataaagagactgaaaaaacatcagcgatgacgaccacacactctacaaaacttcagccatcacaggcgattttgtttaagatgagagaagatgcgccaccattaaacctcacagaagaaatgccgcccccttttccgacaaaggcgaattatcttattcatcctgtgcgatagcgtctttcacatggcaggtgaacaatcatgtctgatgctgatgtgaacacctgcccaaatgagccatcctgacccactaccgcctgccataccccaccataaagcgaatcatcaagccacaagccggggcaagaaacataaatatccccgtcactagttcattaccgccagttaaccacatggtgaagtaataaatgagtgcagcgaggatcaccatgccgaagaaagaagagaccgccgataccacgttcagtacctgaccgatgtagccgcttacgcagacaatacacagggcgagaaacatccataaattaatcatagctcaacctcctgccgcgctaaaaaacctgtaacttcagtcactttaatagtaagacaatccttaacctctggcaatttttgctaagcatcaatgaaaacagcatgttaaatgcaagactgttgtgtacggaaaaatatttactttgcacgattaataatcagtagctgaaagcagtcagcgagtgataaagtacagataccgcattcatgctcctcgtggttatgtcctgactagtctttacactctttacaggaaccattgtcgtacatgatggcccaaccaattgagtgtaccgctgtcgacatggaatcttctgcgatacaacaattcgtatctacagaaggtaactatgtttccacaatgcaaattttcccgcgagtttctacatcctcgctactggctcacatggtttgggcttggtgtactctggctttgggtacagcttccttatcctgttctctgctttctcggcacgcgtattggcgcaatggcgcgaccattcctgaaacgtcgtgaatctatcgcccgtaaaaacctggaactttgtttcccgcagcattctgcggaagaacgcgagaagatgattgccgaaaactttcgttcactcggcatggcgctggtagaaaccggcatggcatggttctggcccgacagtcgcgtacgtaaatggtttgatgttgaagggttggataaccttaaacgcgcacaaatgcaaaatcgcggcgtaatggttgtcggcgtccattttatgtcgctggaactgggcggccgcgtgatgggactgtgccaaccaatgatggctacctatcgtccacataataatcagctgatggaatgggtgcagacccgtgggcgcatgcgctctaacaaagcgatgatcggcagaaataatctgcgcggcattgtcggtgcactgaagaaaggtgaagcggtatggtttgctcccgatcaggattatggtcgtaaaggcagctccttcgcgccgttctttgcggtggaaaatgtcgccacaaccaatggcacctatgttctctcccgtctctctggcgcagccatgttgaccgtaacgatggtaagaaaagcggattacagcggatatcgtttgttcatcaccccagagatggaaggctacccgacagatgaaaatcaagccgctgcctatatgaacaagattatcgagaaagagatcatgcgcgcaccggagcagtacctctggatccaccgtcgctttaaaacgcgcccggtgggagaatcgtcgttgtacatttaacaaactgctcttactctttccctcctcaaatcggccataataacctcatggtttttatggcttttttcttaaggttttttccttcgctgaatatctaattattaccgtcagaaattaaactgtcgccgatatgagacacttgtaagttactaaaagtaaataagaaaatgcctcttgtctcgtttcagttttaggcgtacattagcgccgtctcgagcagtttagctcagaattctggggtgatgcccacggtaaaatacagggcttttaaggtcgctttgcccggtgtcaactcactgtatcaggtgtaatgaagtcattcaggcgtaacagtaattacgcggagagatgtaaagtgaaatatttctttatgggcatttcttttatggtcatcgtttgggccggtacttttgccctgatgatctaaaagcaaactgtgcaatgaaaaacaggagccatcaggctcctgtttgcatttctgacgacggtgtttattccgcgttttcgtgaatatgtttgctgctggcgggtagtaaaccgtcggcacggaacatcgctttaatccctctgatggcctgacgaatacggtcgcggttttcaatcagtgcaaagcgaacatgcgtatcaccatagtcgccaaagccaatccccggcgagacacaaaccttcgcttcgttaaggagcttcttggcaaattccagcgatcccatggccgcatatggttccgggattttcgcccagacatacatcgaagccttcggcatttcaaccatccagcccgcttcatgcagccctttaaccaatacatcacggcggcgtttgtactgttcggcaatgtcgcgcacgcactgttgatcgccctccagcgccgcaatcgccgccacctgcaacggcgtaaaggtgccgtaatcgtgatagcttttaatacgagccagggcgctgaccagcgttttgttgccaaccataaagccgatacgccagcccgccatgttgtagcttttcgacagcgtaaagaactcgactgccacatcgcgtgcacccggtacctgcataattgacggcgctttccagccatcgtagacgatatcggcataggccaggtcatggaccaccagcacatcgtagcgtttcgccagcgccactactttttcgaagaactccagttccacgcattgcgcggttgggtttgacgggaagccgaggatcatcatcttcggtttcggataactttcacgaatggctcgctccagttcgttgaagaaatcgacaccttccaccagcggcactgagcgtacctgcgccccggcaatcaccgcgccataaatatggatcgggtaacttggattcggcaccagcaccgtgtcaccatgatccagcgtcgccagcatcagatgcgccaggccctctttcgaaccaatagtgacgatggcttctgattccgggtcgatttcaacgtcgtagcgatcctgataccagcgggaaatggcgcgacgtaaccgcggaatgccgcgtgaagtggagtaaccatgcgtgtccgggcgctgggccacagtacataatttttcgacgatatgcggcggagtcgcaccgtccgggttacccatgctgaaatcgataatatcttcgccgcgccgacgcgcagccattttcagttcagcggtgatgttaaaaacgtagggcgggagacgatcaatgcgcgtaaagcgacgttcagggcgagtgtcagccataatttcctcagattaacgttagcgcccggaccgtccgagcgacgctgccacgatggtggctgttttgaaaatagcctgattaatttctgtctgtccagcgttttagaacattttattaatgacgttaaatgaggaactctgctttaaaaacaggaaatttatctgcgctaacaagaaaattaccactcattttattaacataataatttcaataaatttactaaccagaagtgcattatcaagagatgcattgctaatacaccatttatctatcaatccccttttaaaattgtggtttttcctcaaaaacggcctgctggtcatcagccttcaggttacctatcatagaggtttaatccttattcagagtcacccgtgcacgaaatattcaacatgctgctggcggtcttcgatcgggcagcgttaatgcttatctgcctgttctttctcatccgtatccgcctgtttcgcgaactgttgcacaagtcggcgcactccccaaaagaattgctcgccgttaccgccattttctcgctgttcgccctgttcagcacctggtccggcgttcccgtagaaggctcgctggtgaacgtacgtattatcgcggtgatgtccggcgggattctgtttggcccgtgggtaggcatcattaccggcgtgattgcgggtattcaccggtatttaattgatatcggcggcgtgacggcgatcccctgctttatcaccagcattctggcgggttgtatatcgggctggatcaacctgaaaatccccaaagcacagcgctggcgcgtcggtattctcggcggcatgttgtgtgagacgttgaccatgattctggtaattgtctgggcaccaactaccgcgttggggatcgatatcgtctctaaaatcggcattccaatgatcctcggtagcgtctgtatcggctttattgtgcttctggtgcaaagcgttgagggcgaaaaagaggccagcgccgcgcggcaggccaagctggcgctggatatcgccaacaaaacgctaccgctgtttcgccatgtcaatagcgagtcattacgcaaggtctgcgaaattatccgcgatgacattcacgccgatgcggtggcgattactaataccgatcatgtgctggcctatgttggcgtgggtgaacataactatcagaatggcgatgacttcattagcccgactacccgtcaggcgatgaattacggaaaaatcatcattaaaaacaatgatgaagcccaccgcacaccagagattcattccatgctggtgatcccattgtgggagaaaggggtcgtgaccggaacgctgaaaatttactactgccacgcgcatcagatcacctcgtcattacaggaaatggcggtcggtctgtcgcaaatcatctccacgcaactggaggtttcacgcgccgagcagctacgtgaaatggcaaataaggcagagcttcgcgccctgcaaagcaaaattaatccccattttctgtttaacgctctgaacgctatttcatcgtcaatccgtctgaatccggataccgctcgccagttgatctttaatctgtcgcgttatctgcgctataacattgaattaaaagacgatgagcaaatcgatatcaaaaaagagctgtatcaaattaaagactatattgccattgagcaggcccgctttggtgacaagctgacggttatctatgatattgatgaagaggtgaattgctgcattcccagcctgctgatccagccgttggtggagaacgccattgtccacggtattcagccttgcaaaggtaaaggcgttgtcaccatcagcgttgcagagtgcggaaatcgggtacgcattgcggtgcgagataccgggcacggcatcgatccaaaggtgattgagcgggtcgaagcgaatgaaatgccgggcaataaaattggcctgctgaatgtccatcatcgcgtgaagttattgtatggcgaggggctgcatatccgccgcctggagccggggacggaaattgcgttttacattcctaaccaacgcaccccagtcgcctcacaggctacgttattgctttgagccggagtgatattgtgaaagtcatcattgttgaagacgaattcctggcacaacaggaactgagctggctaattaaagagcacagccagatggagattgtcggcacctttgacgacggtctggacgtgttgaagtttttgcagcataaccgcgtcgacgccatttttctggatatcaatattccgtcgctggatggcgtgttgctggcgcaaaacatcagccagttcgcccataaaccgtttattgtgttcatcaccgcgtggaaagaacatgcggtagaagcgtttgaactggaggcgtttgactacattctcaaaccgtatcaggagtcacgtattaccgggatgctgcaaaaactggaagcggcctggcaacaacagcagaccagcagtacgcctgccgcgacggtaacgcgtgagaatgacaccattaatctggtgaaagatgagcgaataatcgtcacgccaattaacgatatctattacgccgaagcgcacgagaaaatgacctttgtctatacgcggcgtgaatcctacgtaatgccgatgaacattaccgaattttgcagcaaactgccgccgtcgcattttttccgctgccatcgctcattttgtgtcaatctgaacaaaatacgcgaaatcgaaccgtggtttaataacacctacattctgcgactgaaagatctggattttgaagtgccggtcagccgcagcaaagtgaaagaatttcgccagttaatgcatctttaatcgggaactttcatgaaagcaccaggcttgcccgccgatcaacaatttttcgccgatctgttcagcggcctggtgcttaacccgcaactactggggcgcgtctggtttgccagccagcctgcctcgttgccggtgggcagtttatgtattgattttccccgtctggatatcgtgctgcgcggcgaatacggcaatctgctggaagcaaagcagcaacgtttggtggaaggagaaatgctgtttattccggcgcgcgcggctaatttaccggtcaacaacaaaccggtgatgctgttaagcctggtgttcgctccgacctggcttgggttatcgttttacgatagccgcaccacgtcgttgttgcatcctgctcgccagatccagcttcccagcctgcaacgcggtgaaggtgaagcgatgcttaccgccctcacccatcttagccgttcgccgctggagcaaaatatcattcagccgctggtgttaagtttgctgcatctttgccgtagcgtggtgaatatgccgccgggcaattcgcagccgcgcggcgattttctctatcacagcatttgtaactgggttcaggataattatgcccagccgctcacccgcgagagcgtggcgcagttttttaatatcacgcccaatcatctgtcaaaactgtttgctcagcatggaacgatgcgttttatcgagtatgtgcgttgggtgcgaatggcgaaggcgaggatgattttgcagaaatatcatctgtcaattcatgaagtggcacagcgttgcggttttccggatagcgactatttttgtcgcgttttccggcgtcagtttggtctgacgccgggagagtacagcgcccgttttcagggctaacgtcagaaggttaattctgtttccagcagcgtcaggatactttgtgcatcttgcgcggcaaacaacgactggcggaagtttttattcaccagtttacgcgccagctgcgagaagactttcacatgattcatcccttcgttagcacccagcgtcagcatgatcaccagttcgacttcgcccatttctgactgccagccaatcggtttcgccagccgggcaatgctgatactggaatgacggatccactgagatttggtgtgcgggatcgctacgccaaaaccaacgccggtggtaacaatctcttcccgctgccagacatcttcttccagctcaaacggatgttcagtgcgcccgttaacgccgaggttgccgcacaggaactggatcgcctgctctttattgctaaaatcctgatcaacaaagatattctccagcgccagcagtgggcgaacgtcttcttccggcgtaaaggcggtgagtaacgcttcaatttcctgcgcactgcggcattcacatgcctgacgcgccagttcccgacacgcctcgctatccagttgacgaagctggcttttcaccgccggaatacgcgggctactcatactcagctcatccaggcccagcccaagcagtagcggcagataacggctttcaccgcccagttcaccgcaaatgcctacccatttgccccgctgatgcgcagtggtaactatttgctgcaacatgcgcaggaacgatggcgtaatcgggttatatagcggcgatacgcgcgggttattacgatcgaccgcatacagatactgggtcatatcgttggagccgatactgaagaaatcgacctcatcgcagaagtggtcgatgatgtagcacaccgacggaacttccaccatgatcccaagcgtaatcgtctctgcatgacgcaggccatcgcgcttaagctcaacgatcgctttttggatctcgcctttcacccataagatctgatcgaggctgtgaaccatcgggatcatcaactgggcgttgccgaaactggcggcgcgcaaaatggcccgcagttgagtgcggaacaggccagcaaattccgggtaaatacgtaccgcgcgatagccgaggaacgggttctcttcctggggaatattcagataaggaatgcttttatcgccgccgatgtccatcgtgcggaagataatcggcttgtcgcccgccgccagtagcacctgctggtaggcttcaaattgctcctgctcgtccggcgcgctgtcgcgatccatatagagcatttcggtacggaacagcccgacaccttccgcgccgttggcaaacgcgcctggcgcttccagagcggtgccgatattcgccgcaatatcaatacgcttgttatcacgggaataggccagctgcgcggcagcctgcgcctgttgtttttggcgtttatccgccagcgtctgcgcgacctgataataaccgctcaccgcgtcattcgggttaatcgccagcacgccgcactgggcgtcaagcactgcaggttgcccggcataacgggcaatcgcatccagcggcaagccactcagtaccgggatcgccgaggcacgggccagaatcagtgtatgcgaggtgcgcccggttttctccagaatcatgcccgcaagatttttcaaatcaaggctcaaaaactggcttggggttaaatcttcagccaccagaatggtcggtttttcaagcaccagcttgttgcgcggcttcagttccggccaggtgatatgcagcaactgttcgctgatatcgcgaatgtcgctaacacgttcgcgcagataatcgctggcagaggcagaaagtttggcgcaaacctgctccatattgctgatgatcgccgcccccagcccctgatgctgttctgtcatcaggcgacggatattgcctgcaaattcatcatcctgaatcagcgacaaatgggcgctgaggatagttttgctttcgccgtcacgctcacgcaattgctggttcagttgctcggcaagcgttgccaggctgtgctccagccgggtggaatcttgcgcactggcggggattgcccgataactgtcgaggctgtcgctttgtaacagggtcagcgtacccacgccgacgccgcttgccagcacattgccgtacagtaaatccgggttaaggcggcttaatgaacgcggcagcggatgcgccgtcagttctgcctgcgtaggctgaacgctgtcgctgtcgataaagcgcacctggatgtactcttccagcacgcgccgcgcctgctcttcatcgctgccgctaatgttcaggctgcaactgtcattaaatagggtgccggtgccaatcagcgccagcgagcttttcgcatctgcctttgcgttctggcgatggttaataaaagtgatttcgctttgccactggctgcactgttctttaagttcccacgccggacgagcatgtagaccgttaggcaaaggacagagaaattgaatcgttaacataaccgctccgggttaatcaggagatcatctgaaatccgtcagttgaacaaccgtctcacgcgtaagacgttgaataagggcagataaaagttgctgcatctgcaaaatgtcgcggcaatcggcaatcgatgcggcgcaatgtccatggcgggttgctggccccatcaccactgtgggcacgccggtgccggttaagtgcaccgccccgccgtccgtgccgccgttgctgaacatatctgcctgcaacggcacgccaatttctgccgccacggtttcgacccaggcggtaagttttggcggcgcaatcagcgacttgtcgcttaacaccagcatcggcccgttaccaatctggcgatggttagccgcgccataatcaaagtttttcgcccagcaggcggtatcaagcacaatggcgacgtccggcgacaccgcgcgggtggcagtttgcccgccgcgtaatcccacctcttcgctggaacttgccaccagccacacttccgcaggtagttcggcgtcgtgcagttcgcgcagtaacgtcaccagcagatagcaaccgaggcggtcatcaaaggctttccccatcactcgctggtgagggagaacctgaaaagtggtatcaaacgtgacgcgatcgccgggacgaattcccgcctgcatcacttcgtcataggagcgcgcaccaatgtccacgcgcatggcgctgacgtcattcccctgccggtcgccgtcaagcaggcctggaattttgcactcttcacgggtggtgatgcgcaccggctgcagctggcgggcagccatgcgtacgttgccaaccggcagcacatcaatcgccccttcgcgggagatgctgcgcaccataaatcccacttcgtccatatgcgcacagatcatcaccttcggacctgtcgattcattcaggcggatcagcaccgatcccagaccatcaaatcgcacttctttttgcaggcgatccgcttcttccagcaggatctgccgcacttcctgttccgaggaggcgatcgcatctgcctcgctcaacgcttttaatagcgataaatccattatgcctctcccgtgagcaacactgttttcggcatggcgtagagcacttctgcgccttgcggggtaaccagcacaacatcttcgatgcgcacgcccccttgccctggcaaataaatccccggctccacggtcagtaacatgcctggctgtagcgtcgtggtgtcccgcggtgaaaaacgcggatcttcatgaacttcaatgccgatagcgtgaccggtgttatgaccgaaatagtcgccataacctgcttctgtaatgacccggcgcgcggcatcgtcaacctgctggcagcgcacgccggggcgaatcgcggagattgctgcgagctgtgcctgcaggacaatttgatagacgttaaacagcaggtgagattcggcgctcaccccttcgccattcaccagcaaggtgcgcgtcatatcagagcagtagccctgatacagcgcaccgaaatcgagagtgacaaactcgcccgctgcaacaatcttgtcgctggctttgccgtgcggcagcgccccacgccagccactggcgacaatggtgtcaaaagaggctttttctgcgccctgctggcgcataaaccactccagttcagcggctatctcgcgctcgctcatccccgcctgaataaagcggcgaatatgctctgcaccgcgatcagcaatcccacaggcgaggcggattttctccacctcctctggcgttttgatttgccgcagcacatccggcgtggcgctaaccagtttcgcattgagttcagactgccagcggtgcgcggtttcccaactcacctgctggccctcaaaaccgagcgtttgcaactgttcatcggcaatgatttgattgacgatagtggtaagcgtgttcgtcgcgtcaagcaaatgcagctggtagccttgcgcacgggcttccacctcaacgtaatagcgcgaatccaccagaatgtgcgcactttcacggctaatcaccacataacctgatccggtggagatccccagatgcggctgtttgttctgccgtgaggagagaagcactgcatccagttgttgcgccttaagccagtcgcgcagcgaagcgagtaatgtcatctggattttccttcttacaggctatcgattaacaatttgcctttacggaacatcatcagacgcaggaacaccaccatcagcgcagttatgactgcccccagcgcgatccccgccatatagacgcccaggttagtgaccagcggccatgcccagatagcggactccgggaaccattgcactgcgcccagccagacagcggcggttgagccgacaatagcgccgaccatatacgacggaatggcggtgatggggctttccagcgcaaacggaatcgcaccctcactgatccccataaacgccaggaacatggcggtcttaccctgcggataaagttgagcgttgaacaggcgtttgccggttaaacgacggtcgataatggtcgccagccccagaccaatcggcggaataacgatagcgatagaacgagcggtgaccggtaatacgtggtcagtggtaaagctgaaggcaacaaaacctgcggctttgttgatcgggccaccaaggtcgattgctgtcgccgcggcgatccccattgcgtacatcagcgcgcccttctcacctgcggcagtcagcacagtacggataccgccgttgatccagccaccaaagggggtgatgacgtagtacatcgccagcatgacaaaaatggcggaaagaatcgggagcaaaaatgtggttttgaacgctaacaggaaatccggtaactggattttctggttcatccacttcacaaggtaaccggcaacgatagaaataatcagcgcaccaatgaaggtggacggcaccggcgaagaggtcgcccattgcatagtgctgggatcgaagttcagcagttgcgtcggctgggtagacatcaacccgccgataaaaccagccgggaacgccagtttgccaccgatagagttcgccacaaaagcagcaaacatcggaatggcaaaaccaaacaacacgccgccgaaggactgcgacagccaggcaaatttaagtaaggagaggtcgaaaccggagaatttcccgctattaagagcatccatgatgccgatctcagcaggaattttaagccagctataagcaatcagctggctgaaagcgaggatcacaccgcccataattaaggtcggcaccatgcgtgaaatccctgacatcacatgctgcgggagttcaccccagaagctggttttagaggcctgcggattcttaactgccgctgccgcaccggatgcgccaggcacaacggttgcactgcgttttttaatggccataacaattatccctgtcgaatattactgttgttcagaggcaatcatctcttcgatttctttgatgatgcccgcagcgtttttaattgcgtcctgcaaagtgatttcataaacgtcgcgtgattcgaaacgttcgttatcttccggggtaactgccacggagtggatgatgatggtcgcttcggcgatatcctgcgccgtcaggcgattctggataccgtccgcgccctgggtttcaattttcacttcataaccggcttctaccgccgcttcttccagcgcctgagcggccataaaggtgtgagccaggcccatcgggcaggcacataaggcaatcagtttcttactcatcgttaattcctcgttcagtgatagttgacgagtgaaattatgaacgtgcaaaacaaatcgccgttaccagacaaataatgcatttactggagaattaatcccgctgtacggaagtgtgacgcaggtcgaccttgtgaggggacacaaagaaaaattgaataaactgtatgatttaaaagattatcgggagagttacctcccgatataaaaggaaggatttacagaatgtgacctaaggtctggcgtaaatgtgcaccggaaccgagaaggcccggattgtcatggacgatgagatacaccggaatatcatggacatattctttaaagcgccctttatcttcaaatgcggcacggaaaccggaggctttgaagaactcaaggaagcgcggcacgataccgcccgcaataaacacgccgccaaatgtcccgagattgagcgccagattgccgccaaaacggcccataatgacgcaaaacagcgacaatgcgcggcggcaatcggtgcagctgtcagccagcgcgcgttcggtaatatcttttggcttgagattttctggcaggcggttgtcagctttcacaattgcgcgatacaaattcaccagcccagggccagaaagcacgcgctccgccgaaacatgaccaatttccgcacgcaatatttcgaggataatggcctcttcttcactattcggcgcaaaatcaacgtgaccgccttcgcctggcaagcttacccaacgcttatcgacatggaccagatgcgcaaccccaagccccgttccggcaccgtaaaccgcaataggcttaccttcgaccggttctgcgccaccaaactgaatcagatgctcttttttcagcatcgggatcgccatcgatacagcggtaaaatcgttaataatttccagatggctaaaaccgagattctttttcatttcggcaattgagaacgcccaggtatggttggtcatcgccacccagtcaccggtaattgggcaagcgatggcaatacagccgtctttcacctcgaccttatgttcttcaagataaacgcgaatgaccgcttcgaggctggggtaatcaagccctgaataggtcttagcctgcgagatttcaccactggcaatatcacacagagcaagacgtgcgttggtgccgcccacatcaccgactaatgcatactttgtcattcttcaactgctccgctaaagtcaaaataattctttctcacactgtaaatacctgggggcataacaacaacgccggaaaggcaggctccctgtaaatatcgatctgggtcacacaattactttatcgtttcagcaccaattgcagcgatgcctttttgcaagctgggcaaactaagtatctgaccccgcataaggaatagaacatgctccatccgcgagccagaaccatgttgttattatcgctccccgccgtggcaattgggattgcgtccagtcttattctgattgtggtgatgaaaatcgcctcggtattacagaatttgctctggcaacgactgccgggaactctggggatagcccaggattcacccctctggatcatcggtgtattaacgctaacgggtattgcggtggggttggttatccgtttcagccagggtcatgccggaccagaccccgcctgtgaaccgctgatcggcgcaccggttccgccctctgcgctacctggacttatcgtagcattaattctcggtcttgctggcggcgtcagcctggggccggaacatccgatcatgaccgtcaatatcgcccttgcggttgccattggcgctcgtctgttaccgcgcgtcaaccgaatggagtggactattttagcctctgccggaaccatcggcgcactgtttggcactcctgttgcggcggcgttgatattttcgcaaaccttaaatggcagtagtgaagttccgctatgggatcgtctctttgcgccgttaatggcggcagcagctggtgcacttactaccggattatttttccatcctcatttttcactgcccattgctcattacggacagatggaaatgaccgatattctcagcggtgcaattgtcgcggcgattgccatcgcagcagggatggtcgccgtatggtgcttaccacggttgcacgcgatgatgcatcaaatgaaaaatccggtgctcgtgctgggtattggcggatttattctcggtattctgggggttattggtggaccagtttcgctgtttaaagggctggatgagatgcagcagatggtggcaaatcaggctttcagcaccagcgattactttttgctggcggtaattaaacttgccgccctggtcgttgctgccgccagtggctttcgcggtgggcgaatcttcccggcagtgtttgtcggcgtggcattagggttgatgctgcatgagcacgttcccgccgtaccagcggcaataaccgtttcttgcgctattctcggcatcgtgctggtggtaacacgcgatggctggttaagtctttttatggcggcagtcgttgtacccaataccacattgctaccgctgctctgtatcgtcatgcttccggcatggctgttattagcaggtaagccgatgatgatggtcaatcgtccgaagcaacagccaccccacgataacgtttagcaaaaaatgctctcctttatgatttaagagttatggcgatgatacggggctttacctccccgtaatattgcgttaacaggccgctgacggcttcgagcgtgaaggagaataacaatgttcaggtcactgtttctggcggccgccctgatggcatttaccccgcttgcagcaaacgcaggtgaaatcaccctactgccatcaatcaaattacaaattggcgatcgcgatcattacggtaattactgggacggtggtcactggcgcgaccgtgactactggcatcgcaattatgagtggcgcaaaaaccgttggtggcgtcatgataatggctaccaccgtggctgggataagcgtaaagcgtatgagcgtggctatcgtgaaggctggcgcgatcgtgacgatcatcgcggaaaaggccggggtcatgggcaccgccattaaacgcgtccgccaatggagcacaatgcctgatgcgacgctagtgcgtcttatcaggcctacaaaccggctctttaacgcgtagggcggataaggcgtttacgccgcatccgccaatagtgccagatgcgacgctcattcaactacaatcccagcgccgtccccaccaacaaccagatattcagcgccacgaccagcaccacaatcacccagcctgtctgttttacgcgtttgctgttcaccagatcgcccatcaacttgctgtcactggtgaaaatcagcagtggaaccagcgccagagcgataccaaaacttaacagtacctgactcataaccagaatccgtgtcggatctaatcccatcagaatgacaataaatgacggcaacatggtgactgtacgacgcacccacagcgggatatgaaagcgaatgaagccctgcatcaccacctgccccgccagtgtccccaccaccgttgaagacagccccgcagcaaccaggcttaatccaaagaccgttgccgcagcgtggcttaacagcggttgcagcgtcagataagcctcatcaagatcggcaacaccagtatgaccggaaaagtggaacgccgccgcagctgtagccatcatcgccagattgacaaaaccggcaatagtcatggcgatagccacatcccatttggtggcggaataacgttgttgacgcgaaccgccatgtaaatgctgagtgagcgaggagtgcaaataaatcacatgcggcataatcgtcgcccctaacacgcctgctgccaggaagaccgcttccgaagtaggtaaactcgggatcaccattcctttacccagctgcgccaggttaggctgggagaaaatcaactcgacaatgtaagccgcggcaacaaacaacagtaacccgccaatcactttctccagcggtttttgcccgcgacgttgcagcattaaaatcaggaaagtcgcgatccccgtcagcaccgcgccctgcaacaacgaaacaccaagaatgagtttaaaaccgatcgccgcaccaataaattccgccaggtcggttgccatcgcaataatttctgcctgaacccaatagaaccacactacgggacgcggatagtgatcgcgaatctgctccgccagatttttaccggtggcaatccctagtttggcagagaggatctgaatcagcatcgccatcaggttggcccaaacgacaacccacagtagctgatagccgaagctagcacccgcctgaatattggtcgcaaagttaccgggatcgatataaccaatcgccgcaatgaacgcaggtcccattaatgcgagcctcatcttgcgcgccgcccgtccgctgctactctcaacgcgatagttcgtcatcttgtgcctctaaaacatagcctttgctatgtttcatgctatgccaaacgagaatgattatcaaattcatttaaatggattgtggtgatttctctgatagaccaggattatgactacgaaaagattgatgacttgaatgttatggttatgtttaatgttagcacatttacataactttcagcttccatacacaacatagcagaaatgtatgacagatcactatttttgaagcctgtcacaggacgtcattatagtgtgtgtcagatctcgttttccttaaccatgttacatagaatgtgcacggaaatttaacctgcctcatatttggagcaaatatggaccgcgtccttcattttgtactggcacttgccgttgttgcgattctcgcactgctggtaagcagcgaccgcaaaaaaattcgtatccgttatgttattcaactgcttgttatcgaagtgttactggcgtggttcttcctgaactccgacgttggtttaggcttcgtgaaaggcttctccgaaatgttcgaaaaactgctcggatttgccaacgaagggactaacttcgtctttggtagcatgaatgatcaaggcctggcattcttcttcctgaaagtgctgtgcccaatcgtctttatctctgcactgatcggtattctccagcacattcgcgtgttgccggtgatcatccgcgcaattggtttcctgctctccaaagtcaacggcatgggcaaactggaatcctttaacgccgtcagctccctgattctgggtcagtctgaaaactttattgcctataaagatatcctcggcaaaatctcccgtaatcgtatgtacaccatggctgccacggcaatgtccaccgtgtcgatgtccatcgttggtgcatacatgaccatgctggaaccgaaatacgtcgttgctgcgctggtactgaacatgttcagcacctttatcgtgctgtcgctgatcaatccttaccgtgttgatgccagtgaagaaaacatccagatgtccaacctgcacgaaggtcagagcttcttcgaaatgctgggtgaatacattctggcaggtttcaaagttgccattatcgttgccgcgatgctgattggctttatcgccctgatcgccgcgctgaacgcactgtttgccaccgttactggctggtttggctacagcatctccttccagggcatcctgggctacatcttctatccgattgcatgggtgatgggtgttccttccagtgaagcactgcaagtgggcagtatcatggcgaccaaactggtttccaacgagttcgttgcgatgatggatctgcagaaaattgcttccacgctctctccgcgtgctgaaggcatcatctctgtgttcctggtttccttcgctaacttctcttcaatcgggattatcgcaggtgcagttaaaggcctgaatgaagagcaaggtaacgtggtttctcgcttcggtctgaagctggtttacggctctaccctggtgagtgtgctgtctgcgtcaatcgcagcactggtgctgtaagaccatacataaaaaagccggggataattcccataagcgctaacttaagggttgtggtattacgcctgatatgatttaacgtgccgatgaattactctcacgataactggtcagcaattctggcccatattggtaagcccgaagaactggatacttcggcacgtaatgccggggctctaacccgccgccgcgaaattcgtgatgctgcaactctgctacgtctggggctggcttacggccccggggggatgtcattacgtgaagtcactgcatgggctcagctccatgacgttgcaacattatctgacgtggctctcctgaagcggctgcggaatgccgccgactggtttggcatacttgccgcacaaacacttgctgtacgcgccgcagttacgggttgtacaagcggaaagagattgcgtcttgtcgatggaacagcaatcagtgcgcccgggggcggcagcgctgaatggcgactacatatgggatatgatcctcatacctgtcagttcactgattttgagctaaccgacagcagagacgctgaacggctggaccgatttgcgcaaacggcagacgagatacgcattgctgaccggggattcggttcgcgtcccgaatgtatccgctcacttgcttttggagaagctgattatatcgtccgggttcactggcgaggattgcgctggttaactgcagaaggaatgcgctttgacatgatgggttttctgcgcgggctggattgcggtaagaacggtgaaaccactgtaatgataggcaattcaggtaataaaaaagccggagctccctttccggcacgtctcattgccgtatcacttcctcccgaaaaagcattaatcagtaaaacccgactgctcagcgagaatcgtcgaaaaggacgagtagttcaggcggaaacgctggaagcagcgggccatgtgctattgctaacatcattaccggaagatgaatattcagcagagcaagtggctgattgttaccgtctgcgatggcaaattgaactggcttttaagcggctcaaaagtttgctgcacctggatgctttgcgtgcaaaggaacctgaactcgcgaaagcgtggatatttgctaatctactcgccgcatttttaattgacgacataatccagccatcgctggatttcccccccagaagtgccggatccgaaaagaagaactaactcgttgtggagaataacaaaaatggtcatctggagcttacaggtggccattcgtgggacagtatccctgacagcctacaaaacgcaattgaagaacgcgaggcatcgtcttaacgaggcaccgaggcgtcgcattcttcagatggttcaacccttaagttagcgcttatgggataattccccggtttttttacgcctgttaatcagctaatggctgcgggcgaccaatcaaatacccttgcagatattgcaccccgagcttatgcaatagcgcctgctgctgttgcgtctcgacaaactccgcgaccacactcaatgacttcgctttcgccagatcggtaattgatctcacaatcatcgcatccagcgtgttcgtgacaatatctttcacaaagacgccatcaattttgatgatatcagcctgcaaacgctttaaccgttcgtagttggcatatccggtgccaaagtcatcaatcgcaatccggaaaccaaacttatgcagctgctcgatgttgtacatgctgctttctgcgttagaaaacgcctgctcctcggtgatctcaagaatgaccgcctgcggggagatgtgataacgcttaaacagacgaataatccgcccggcaatattcttttgcagcagcgtgagcggcattaaattgactgaaaagcgcggtccttttttgtcgcaagggtgtgttgccagccacttcaacaaggattccagcacttgcaaatcaaaacgcgcgctaaggttaaactgagcaataaggggcagaaacttatccggggtcataatgccgccgtcatatttcagtcgcgcgaggatctcatcataaccttcaccctctttgttgcgaattggctgggcgtagagcagcaaatcaccctgatctaacgccgtgcgaatggtattcagcaatagcacctgtttagtggtctgcccggaaaccatctcctctctgctatccagcgccagcacatgatgatgtgcgcaggattgctccgccagccagcttaactgccccaacaagggttgcagggtttcctgatttccatcaaaacgcccccaggcagcaccatagcccatatccagcccggtattgttccagtgaatttgccgactattcaggatgttaaccatatgctggagtcgcccttccgtttccggcccgctcagcactaacagcagttcactacccggcaattgatacaacttttcgttttcctgcatcaacggcagcagcgtacggcaaattgagcggatacagtgaacgcgcatcattaagccgtaatgacgactcataaactcaagattatcaatgcgcaggcagcaaaaactcttgcccgcctcttgctccggcgcttgttccaacgcacgaaagttgggtaggagcgttaacggatctgtcagcgcctgcaaatgccagcggcgattaagccattcactgcgatgataaatgcgcaccatatagagcaggcaaacgctaaaggaaatcagcaccgcaagaataaatgccagcgaatattcggtttccaccccttgcaaaaagttctggttgtaattcagaaggcaaagcgttgaaacagcccaggtgagatttaaaaacggatagcgaagcttaccgaccccgagggtaaagatgatgaagaaaacgggtaccaggtaaccggcaataaagtcgttttcataaggtgtgcacaacagaagtagcagcacgcttaacgctgccagccagcttaaggtaaatgcgcgtttctctttgcccaacgacggagcgatatccctgcgccacaatatctgcgcaaagtggggacttacaatcatgcgagtgagatagtagaaaagcatgttgtaaatcagcacagcggtgaaaaggcttagcaaatcaacgaccgtgaaaatggcatccgcatcgccgaaaaaggtggatatctttagcgggaaatcaaagaagctccccacaagatacatgctgcatttgatgccgatcggcgtcaccaaaccaagccagaacagacgttgccagacatatcggctggtcaatccataacgccaacgcgtccccagctgccagcgtaatattgcgcaggcacacaacacgacaaacgtctggctaccgagcatgaccgcagtctgtaaaaaagagagatgaaagttccacagattggtgcaaaacatcccgcataaaacgggaacgacaccgcgccagccaaagataaacaagattgacagcattacgcacagtggcatccacgccagaaagatataactggaatggataatggcaagtggcgaaataaaacgggatagctgaataagtaccacggtgagcgtaaacgctagtgtgaatatcttgatattttttatcaggttatgctccacaaacatgagtacactactctcactgatcggggttttcaggcacacaaataataagtttattcgcatcgcgaagcaaacagggggccagcctgttgccgatttttcatccaatgatgctttcaccaggcggcactaacccggacgtagactgtattacaaaagcggcaaaaagcagagacaaaaaacccccgctttgcagcgagggttggaaatttggtggagctaagcgggatcgaaccgctgacctcttgcatgccatgcaagcgctctcccagctgagctatagccccacgatgcgtttacgtaccaagtttgctgggtgcaaaatttggtggagctaagcgggatcgaaccgctgacctcttgcatgccatgcaagcgctctcccagctgagctatagccccgtcacgtaaagcttgtcgagttgacgggcggcatcatatgaattccgcccgaatgtgtcaacggcaaattgcaacgtgtagtttcaatcgctgaaaaatcaggcaaatgaacaattttggaaaaccgctcgcattcagtagttattcatgtcacggtttcctgtaaagtggtgttataaaatgaactactaatagacccacatacattcagggaattgttatgttcaaggagaggatgacaccagatgaacttgccagactgaccggctatagccgccagaccattaataaatgggtacgcaaggaaggctggacaacgtcaccaaaacctggcgtccagggtggcaaagcccgactggttcacgtcaatgaacaggttcgtgaatatattcgcaatgctgaacgtccagaaggtcagggagaagcgcctgccctttctggtgatgcgccgcttgaagtattgctggtgacactggcgaaagagatgacgccagttgaacaaaaacagtttacatccttgcttctgcgggaagggattatcggattgttacaacgcttagggattcgcgatagcaaataatatgaaaagattacgcaataaaatgaccaccgaagaactggctgaatgcctcggtgtggctaaacaaactgttaaccgttggatcagagaaaaaggctggaaaacggaaaaatttcccggcgtgaaaggcggtcgtgccagacttattctggtcgatacgcaagtttgcgagtttattcagaacacgccagccttccataacacaccaatgttgatggaagctgaagagagaattgctgaatacgctcctggagcacgcgccccggcgtatcgacaaatcatcaacgcgatagataatatgacagacattgagcaggaaaaagtcgcgcaatttttgtcacgtgaaggaattcgcaatttcctcgcccgtctcgatattgacgaatcagcataaataaaaaacggcaggatattatctcctgccgtttatctttttacacgctaattactgctgattttcgcgttcagcaataaaatccagcgctttgttgatacgctcgatactgcgggtcttaccaattgcgtgaacggtaacatccagtgctggagactgccccgcaccggttacggcgacacgcagcggcataccaactttacccatacccacttccagctcatccgccgtcgcctgaatagcgtgatgaacgttttcagcggtccagtcagtaatcgcggccagtttgtcacgaaccacttccagcggctgacgcgctaccggacgcagatgttttttcgcggcgtcggcatcgaactcagcaaaatcttcgtagaaataacggcagctctgtgccatctctttcagcgtcttgcagcgttcgcccagcagtttcaccagatcagccagctgcgggccgttacgggtatcgatattttcctgctcaatgtgccactgtaagtgagtagcaacatactccggcggcagcgcgttaatgtagtgatggttcagccacagcagcttgtcggtgttgaacgcactggcagatttgctgacggcattcaaagtgaagtatttgatcatctcttcacgagtgaagatttcctgatcgccgtgggaccagcccagacgcaccagatagttcagcagtgcttctggcaaataaccgtcatcacgatactgcattacgctgactgccccgtgacgtttggacagttttttaccgtcatcgccattgatcatagaaacgtgcgcgtaaaccggcaccggcgctttcagggccttaagaatgttgatctggcgtggcgtgttgttgatatggtcttcgccacggataacgtgggtgatttccatatcccagtcatcgacaaccacacagaagttataggttggggaaccatcggtacggcggataataagatcgtccagttcctggttgctgaactcgatcggaccacggatctgatcgtcaaaaacaacagaaccttcctgcgggttagcaaaacgtacaacacacggttcatcatcagcatgatgctcatggctgtggcggcagcgaccgtcataacgcggcttctcacctttcgccatttgctcttcgcgcagcgcttccaggcgctctttagagcaatagcatttataagcagtgccctcttccagcatctgatcgatcaccgcgttgtagcgatcaaaacgtttggtctggtagtacggaccttcatcccactccaggctcagccagttcatgccatccataatggcttcgatagcttccggcgtggaacgctcaagatcggtgtcttcaatacgcagcacgaactcaccgccgtggttacgtgcaaaaagccaggagtaaagagcagtacgcgcgccgccaacgtgcagatagcctgttgggcttggcgcgaagcgagttttgattttcatgaaatggccttacgtttagaaagatgccgacaaccggcaaatcctggaaaaattaagtgggcgatattctatcactcccgcctgattcctcaatgtagttcgggtttctaccttacgcattattgttttcgttgacaaattgcgcaacacggtctgttttgcgatcatcttgcttaaatttacgacgaacgaacaatttctttagaaaatgcgttgactcattttgaactctccctataatgcgactccacacagcgggggtgattagctcagctgggagagcacctcccttacaaggagggggtcggcggttcgatcccgtcatcacccaccaactactttatgtagtctccgccgtgtagcaagaaattgagaagtgggtgattagctcagctgggagagcacctcccttacaaggagggggtcggcggttcgatcccgtcatcacccaccactttctcgccagctaaatttcttgtaaaaatgtgaagtaccgaagtgggtgattagctcagctgggagagcacctcccttacaaggagggggtcggcggttcgatcccgtcatcacccaccacttcgggtcgttagctcagttggtagagcagttgacttttaatcaattggtcgcaggttcgaatcctgcacgacccaccaatgtaaaaaagcgccctaaaggcgcttttttactatctgcgatactcaaagattcgaacctgcagcaggtttgagttgagcgcagcgaaacaacggagccgctcgcggcgacggcccgaagggcgagcgaagcgagtcatcctgcacgacccaccaatgtaaaaaagcgccctaaaggcgcttttttgctatctgcgatttgcgaaattgcctgatgcgcttcacttagcagactactatttccggcaattcctgtctcctcacctactgtgtcaatgcagccaacagcttaaccatcgcgggcgtcacctgctgtgtttcataaacaatatataaatctgcagggatgcgctgtttgagcggacggaaaatgacacctggccagttcatttgtgcgtagctgtccgctatcaatgtgataccaatgcccatactgaccatagcgagtaccgtttgcggttcattaacttcgcgaataacaaccggtgaaaatcccacctgctggcaaactcgctgcaaaaaatcccagtcagtgtaaacgggcggcattgtaacaaaatactcgtcacgtagcgcttccagcgggacggtggaaaatgatgagagatgatgctcttcaggcatcgccaccagaaacgccgattcatgcaaccgtaagctggtaaaaccagtcggtggttctgtcgccattcgccagatcccggcatcaagttcgcggcgttccagcaaggccatttgcatcgcgggcatcttttcgcgaaaaagaacgtcaacgttaggattttccctgaggaatcgccgcataaccgggcgcatccgtccccacattgccgttcccactacgccgagttcaatccgccctgcttctccccgacctatttgttcaatccgagccaatacattattagcattcaccagcaatcgacgcgattcttccatcaagattttgcccgcgtgtgtcagtacgacgctgcgcgaatggcgaataaaaagctgcgtgccgagttgattttccagctctttaatatgaatgctgagcggaggctgagacatatttaaacgcgctgctgcgcggccaaaatgcaactcttccgctacggcaagaaaataacggagcaacttaagatctgttctgtatacgcgttccataattaagtgctccatataataaatacatcgtattaaattatcatggcataaagtatttcaccaccagatatccgacatacataaacacaatggataatatacccggtaatacatttggtacaggaataggcaagcgcacgattgtaaacaaagcaccaataccaaaaccaacgccggaagaaaataaaatatctttcactaattaacctttatcataaaagcagctctgaagagcagagccgcgaatccttttaatgagtcaccgctcgatgctttatcttttcagggtcatgattatatttaaacccaaagaaaaatatcactgcgagaaaaagagcatatcctgcaaacaccagccagatagtttgccagtcttttacgccatccaccgaaaagtaatctactgccatgccactcagaatcgagccaacccatgcgccgacaccatttaccatggtcataaagagcccctgcgcgctggcacgaatgctggaatcaacttcctgttcgacaaataccgaaccagaaatattgaagaaatcgaatgcacagccataaacaatcatcgacagcagcagcaaaataaatccggttgttgacggatcgccataggcgaagaagccaaagcgcagcgtccaggccaccatactcatcagcatgacggttttaatgccaaatcgctttaaaaagaatgggatagtcagtataaagcccacttctgccatctgtgaaactgacagtaaaatggagggatatttcaccacaaaactgtcagcaaactccgggttacgggcgaaatcatgtaggaacggattaccaaaaacgttggtaatttgcagtaccgcacccagcatcatggcaaagaggaaaaagatggccatgcgtggatttttaaacagcacgaaggcatccagacccagcttgctggcaagcgatgtggtcgcttttttctccgcaaccggaatcttcggcaaagtcagcgcataagccgacagcagcaatgacgcaccggacgcgatatacagctgcagactactcaattccagatgcagcaggcttactgcccacatcgcgacaatgaaccccaccgtaccaaaaacgcgaatgggcgggaaagcggtcaccgggtcaagccctgcctgggcaagacaggaataagagacgctgttcgataacgcaatagtcggcataaacgccatcgcattgactaacatcacccaaaacatcatatccggatcagttacggatgccgcataaaaaagtacgcccgcacacaccaggtgacacagcatgtatgcacgttctgcgcgcagccatttgtctgcgatgatccccattataccaggcataataatcgcggcgatccctttggaactgtaaaccatgccaacattagcgccggtgaaatgaagagtattaatcatgtaagagccgagggtaaccagccagctcccccagataaaatattgcaaaaaggacattacctttaagcgcatcgcgatgctcataatcgtttccttgtcgcatcatttggcctcacccgcgaggccgtttcttattgtttttctcaggcaattttgcgcagaaagccacaaataaggttgatgaagttctgcttagagagctccgcagccgccagcgtttgcgcatgtgacaatttcacatcgcttaaaccttccgccatattggtaatcgcagagaccgcaacgactttaaggtcgcaatggcgagctgaaataacctcaggcaccacagacataccaacaacatccccaccaataatttgcatcatgcgaatttccgccgcagtctcgaaattcggccccggatacgagacgaacacgccctccgtcagagggaaaccctcttctttcgccactttttgtaacagtgcgcggtattccgcatcgtaggcatttgccagtgagaagaagcgctctccaaaacgatcatcgttaagacccaccatcggcgtaccgggcatggtgttgatatgatctttcaatgcgaccaggctgcctgcccccacttccggacgcagcgagcctgccgcattggtgcagaacagtagctcgcagcccagcagcttaaaggtacgaattgcgtcagtcataatggtcattccacgaccttcgtagaaatgtccgcgacctttcatacataccaccggtacgccctggagatggcccagcactaactcccccgcatgaccatgtaccgtacttaccgggaagcccggcagcttttcgtaggaaattgcgacagcgttctcaatctgatcggccagcgcgccgagcccggaacctaaaataaaggccactcgtggcgtgaaatcaggtttataagtcttgataatatctatgcaaaacagcgggttatgagaaaattgaacctgagacatacatatcctttttctgtagggtggaatctaacgcctttttatagcgaggttgtcccggctcttaccaatacacttttctcacgcattcaatagcgattcgatatcgatggatttatatcttttctctattaatccacggtaaaaactgtattggcgatattaattcctttgcattaacaatatgtcgtttttagcaaaccactttattaagcaatctactaataacgatcggcatagggaattatgctatgaaaaaacatcttttaactctgacactttcctctatattagcgatacctgttgtatctcatgcagaatttaaaggcggttttgcagatatcggcgtgcattatctggactggaccagccggactaccgaaaaatcgtcgaccaaatcacacaaagatgattttggttatcttgaatttgaaggtggcgctaactttagttggggagaaatgtacgggttcttcgactgggaaaacttctataacggtcgccataataaaccaggtagcgagcagcgttatacctttaaaaataccaaccgtatttacctgggtgacaccggatttaatctctacttgcatgcgtatggcacctacggttctgcgaatcgcgtgaatttccacgacgatatgttcctgtacggtatcggctacaatttcaccggcagcggttggtggttcaaaccgttctttgctaagcgttatacagatcaaacctattacactggcgacaacggctatgtcgccggctgggttgcaggttacaactttatgctgggcagcgagaaattcactcttaccaactggaacgagtacgagtttgaccgtgacgctacctatgcagcgggtaatggcggtaaagaagggctgaatggcgcagttgcactgtggtggaatgcaacatcacacattactacggggattcagtatcgatatgcggatgacaaactgggcgaagatttttaccaggatgcgataatctactccatcaaatttaacttctgattgattactgccggggctcccggcagtatgaattcactctatatctgatacaacggatccccttcccgcccagccattagcgcattgccctggtctcgtaccacgtcccataaagcttcagcggcggtggaaagtgaacggttcttcctgcgcaccagcatcaactggcgttcaacaaccggcgtaatgcgctttaccaccagtgggctaccttcaggcaatggtagcgccagtgcgggaagaatactgatgccgatgcctgcggctaccatcgggaacagcgtcgccggatgtccaatctcctgcacaatattcgcctgaataccattgcgcgccagcgctgcgtcaatcagcggtcggctgcctgacgcgtaatcctgcaacaccaatttcgctccctgtaatgcctgccagggtacataatcttccacggccaaagcgctatcgcgatggcaaagcagaaagaaaggctcggaaagaatcgcttcacattgcagatcgcccactgggcctggatcgatgacgatgccaaaatcgacatctccctggcgaatactttccattacccactgctgcggacgatcgtgcaggacaaactgaatatctggatagcggcgatggctttcagcaatgcattgcggaataagatgcgcggaaatggtctggctggcagcgacccgaacttttccgctcagttgttgccccatacgcccggtatcgcgcaacgtgctgttcagttcatccagcagtcgctcaagacgcaaagccagctgctgccctgcatctgtaagcaccacttcacgcgtggttctgtccagcaggcgaacaccagtatgattttccagttccttcacactgtgactcactgccgactggctcaggccgatacgctctcctgcacgactaaaacttttctcctgcgctactgtgacgaaaacctttaattgttttaaagaataattcatctgttttcttcatgaatggatgcaataaatcaattttatttctcaaactggaagaagcacaatagaaccatcgatcatctggagtctttatgaaactttttcgtatcctcgatcctttcaccttaaccctgatcacggtggtgttgctggcctctttctttccggccagaggcgatttcgtccccttctttgaaaatctgaccaccgcagctattgccctgctgttctttatgcacggcgcgaagttgtcgcgtgaggcgattattgctggcggtggtcactggcgactgcatttgtgggtaatgtgcagcaccttcgtgctgtttccgattctgggtgtactgtttgcctggtggaaaccggtaaatgtcgacccgatgctctactccggttttctctacttgtgcattctcccggctaccgtgcagtctgcaatcgccttcacgtcaatggcgggcggtaacgtcgcggcagcggtttgttctgcgtcggcatccagcctgctggggattttcctttcaccattgctggttggtctggtgatgaatgttcacggtgcagggggcagccttgagcaggtcggtaaaattatgctgcaactgctgctgccgtttgtgttggggcatctttcccggccgtggattggtgactgggtgtcgcgcaataaaaaatggattgcgaaaactgaccagacgtccattctgttggtggtttatacagcgttcagcgaagccgtcgttaatggtatctggcataaagttggctggggatcattgctgtttatcgtggtggtcagctgcgttcttctggctatcgtgattgtagttaacgtctttatggcacgccgactgagcttcaataaggcagatgaaattactatcgtcttttgtggttcgaaaaagagtctggcaaatggcatcccgatggcaaacattctgttccccacatcggtgatcggtatgatggtgctgcccctgatgattttccatcagatccaattgatggtctgtgcggtgctggcgcgtcgatacaaacgccagaccgaacagttacaggcgcagcaggaaagcagcgccgataaagcttaaagcggacgcttcaggggctggaccagttgcgtcagcccctcggttttaatcagcagcgtgatttgcattagctcaccgagcttccctgccgggaactcatctttgcgggcaaaccacagcagatactcctccggcaggtcgattaagcgacgccctttgtatttgccaaacggcattatcgtattggctatttcaatcagctgctctttttccatctcagctacccagcaaacgcagcatttccgcttcgtcgatgacttcaatgcccagttcctgcgccttcgccagtttagatcctgcagcttcacccgctatcaccagatcggttttcttcgacacgctgcccgcgactttcgcgcccagttcgaccagtcgagctttagcgtcatcacgcgacatctggcttaagctgcccgtaagcaccacggttttaccagcaaacgggctgtcaatctcttccgcgttgataacgatcggcgcaggccagtgaacaccttccgccaacagctcgctgatgacattgcggttgctttcttcggcaaagaagttgtgaacgtgggatgcaacgacaatgccaacatcaggcaccttttgcagctcttcaatcgaagcggcttccagcgcttccagcgtgccgaaatatgccgccagacctgctgcggtggcctcgccgacttcacggatgccaagtgcatagaggaagcgagcaaaggtggtttctttcgctttttccagcgcgttaaccacgttttgtgccgattttggccccatacgctccagtccggtcagtttgcctgcggtgagtttgaacagatctgccggagtatggacatattctttttcaaccagctgatcgatgattttgtcgcccattccgtcaacatccatcgcacggcgggaaacaaagtgtttcagcgactctttacgctgcgcaccgcaaatcaggccaccggtacagcgggcaaccgcttcaccttccacacgctcaacgtcagaaccacataccggacaatgcgtcgggaatacaacctcacgggtatcttccgggcgttcagaaagcacgacgttaaccacctgcgggatcacgtcgccagcgcggcgaatcaccactttatcgccaatgcgtaaaccaagacgttcgatttcatccgcattgtgtaaggttgcgttactcaccagcacgcctgcaacatggacaggttccagacgcgcaacaggcgtaatcgcgccagtacgcccaacctgaaactcgacgtcacgcacaaaggtcatctgctcctgcgccgggaatttaaacgctaccgcccagcgcggggcacgcgcgacaaagccaagctgctcctgctgtgccagtgagttgaccttaatcaccacgccgtcgatatcaaagcccagcgtcgggcggtcttcttccactttgtgatagaacgccagcacttcttccgccgattcacaaagcgttacccgatcgctgaccggcaacccccactttttaaattgcagtaaacggccaagatgagtatccggcagctcgccaccttccagaacaccaacgccatagcagaaaaaagtgagcggtcgcttcgctgtaatacgcggatcaagctgacgcagtgaaccagctgccgcattacgtgggttagcaaacactttcccgcccgtgcgtcgcgcatcttcgttaatcttttcgaaccccgcctgcggcaggaacacttcaccacgcacttccagacgcgccgggatattctctccgtgcagcttcagcggaatggcgcgaatagtacgcacattagacgtgatatcttccccggtggtgccatcgccacgggtcgcggcactgactaaaacgccattttcatacagaatactgacggcaagaccatccagcttcagctcacagcaccaggtgactttctcgttgtttttcagacggtcctgcacacgtttgttgaaagcaagaaagctttcttcatcaaaaacgttatccagtgacagcattggtacttcatggcgtatctggctgaaagccgccagcggcgcagcgcctacacgttgagtaggcgaatcaggcgtaatcagttctggatgtttggtttccagctcgcgcagttcgcgcatcagcctgtcgtattcagcgtcgggaatttccggcgcatccatcacatgataaagatattcatgatggcgaagcgtcgttcgcagttctgtcagttgttgttcgattgattccatatcgcaccatcaatgctaaaaacccccgacaagcgggggttcgaagaggagttaatttgccttaagtgtatcaggcgttggcgtctttgacttcgcggatgatgtcctggtactcgcgcaatttctgcggagtcatcatacggcgctgatcgtcaagcacgacaccgcccacttcatcggcaatatgctgcgcagattgcagcatcagcttgaagttctgcagctcgtcaccgtaagacggtacctgcataaagatagtgacacccggagtagtgaaatccttcatttcaggatcaaaggttcccggtttcaccatattcgccaggctgaataacgccgggccgctgccatccgggctaagatgacgatggtaaatattcatatcgccaaaaatgaagcccgcttgttgaatgctgttaagaagcagttcaccgtttagctcgctaccgtgatgcgccgcgacgttcatgataatcaccgcttctttgcgcttcggtttatccataactggagcaggttccgctacaggctcaggctgtggtgccgctacgggttctgcaggctggaaagcctgttgtgccggttgcggtgctgaatgcacaggctgcggcgctggcgcgacctgtggcgaaactggctgctgcaacggctgttcaggctgcggctgataggcaggctgctgcaccggctgcgctggatgcggagcatgttgcggcggtacctgcgcttcaggcggctgctggaccggttgacgcggctgcgcagacgcataaggcggttggtactggtgttgcggcgacggacgagcagcctcatgctcctgagcgttagccggggcatgattcacgcggtgaacacgaacctcaccaacgccctcatcatcttcgacatcctcgtcataagaatcgtcgtcacgttttgacttcattcgttttaatggccgatcgcggaacatagaagatcgttctttacggctggtccagaaaccatgtaccagtaaagcgattatggcgatcgcgccaacaatgattaatatcagacgcaaatcctgcatcattatattctctgttgttctaacaccttgccaccacggcaaacatttactcactaagagtatttgccgattacctcaagtgcaagtgcactattaactttcacagcacaaagatagatgaaatcgtgctttttgctgttttttcgaacatatcctaactgtccattgcgcaattacccggtaaaatacgcagaattttcctgggattggtcaaaaggagctcatcctgattatggtttcatcattcacatctgccccacgcagcggtttttactattttgcgcaaggctggaagctcgtctcgcaacctgggattcggcgtttcgttattttaccgctgctggtcaatattttgttgatggggggcgcattctggtggctctttacacagctcgatgtctggatcccgactctcatgagttacgttccggactggctacaatggctgagttatctgttgtggcctctggctgtcatctctgtgctgttagtgtttggctatttcttctccacgattgctaactggattgccgctccgtttaacggtttattggctgaacaactggaagcacgattgactggcgctacaccgccagataccgggattttcggtatcatgaaagatgtgccgcgaatcatgaaacgcgaatggcaaaaatttgcctggtatctgccgcgcgcaattgtattactaattctttacttcatccctggtattgggcaaaccgtcgcgccggtactgtggttcctgtttagcgcctggatgttagccatccagtattgcgattaccccttcgataaccacaaagtgccgtttaaagagatgcgcaccgccctgcgcacacgcaaaatcaccaatatgcagtttggtgctttaaccagcctgtttacgatgatcccgctgcttaatctgttcatcatgcccgttgccgtttgtggcgcgacggcgatgtgggtcgattgctatcgcgataaacacgcgatgtggcggtaacaatctaccggttattttgtaaaccgtttgtgtgaaacaggggtggcttatgccgccccttattccatcttgcatgtcattatttcccttctgtatatagatatgctaaatccttacttccgcatattctctgagcgggtatgctacctgttgtatcccaatttcatacagttaaggacaggccatgagtaagatttttgaagataactcgctgactatcggtcacacgccgctggttcgcctgaatcgcatcggtaacggacgcattctggcgaaggtggaatctcgtaaccccagcttcagcgttaagtgccgtatcggtgccaacatgatttgggatgccgaaaagcgcggcgtgctgaaaccaggcgttgaactggttgaaccgaccagcggtaataccgggattgcactggcctatgtagctgccgctcgcggttacaaactcaccctgaccatgccagaaaccatgagtattgaacgccgcaagctgctgaaagcgttaggtgcaaacctggtgctgacggaaggtgctaaaggcatgaaaggcgcaatccaaaaagcagaagaaattgtcgccagcaatccagagaaatacctgctgctgcaacaattcagcaatccggcaaaccctgaaattcacgaaaagaccaccggtccggagatatgggaagataccgacggtcaggttgatgtatttattgctggcgttgggactggcggtacgctgactggcgtcagccgctacattaaaggcaccaaaggcaagaccgatcttatctctgtcgccgttgagccaaccgattctccagttatcgcccaggcgctggcaggtgaagagattaaacctggcccgcataaaattcagggtattggcgctggttttatcccggctaacctcgatctcaagctggtcgataaagtcattggcatcaccaatgaagaagcgatttctaccgcgcgtcgtctgatggaagaagaaggtattcttgcaggtatctcttctggagcagctgttgccgcggcgttgaaactacaagaagatgaaagctttaccaacaagaatattgtggttattctaccatcatcgggtgagcgttatttaagcaccgcattgtttgccgatctcttcactgagaaagaattgcaacagtaatgccagcttgttaaaaatgcgtaaaaaagcacctttttaggtgcttttttgtggcctgcttcaaactttcgcccctcctggcattgattcagcctgtcggaactggtatttaaccagactaattattttgatgcgcgaaattaatcgttacaggaaaagccaaagctgaatcgattttatgatttggttcaattcttcctttagcggcataatgtttaatgacgtacgaaacgtcagcggtcaacacccgccagcaatggactgtattgcgctcttcgtgcgtcgcgtctgttaaaaactggcgctaacaatacaggctaaagtcgaaccgccaggctagactttagttccacaacactaaacctataagttggggaaatacaatgttccagcaagaagttaccattaccgctccgaacggtctgcacacccgccctgctgcccagtttgtaaaagaagctaagggcttcacttctgaaattactgtgacttccaacggcaaaagcgccagcgcgaaaagcctgtttaaactgcagactctgggcctgactcaaggtaccgttgtgactatctccgcagaaggcgaagacgagcagaaagcggttgaacatctggttaaactgatggcggaactcgagtaatttcccgggttcttttaaaaatcagtcacaagtaaggtagggttatgatttcaggcattttagcatccccgggtatcgctttcggtaaagctctgcttctgaaagaagacgaaattgtcattgaccggaaaaaaatttctgccgaccaggttgatcaggaagttgaacgttttctgagcggtcgtgccaaggcatcagcccagctggaaacgatcaaaacgaaagctggtgaaacgttcggtgaagaaaaagaagccatctttgaagggcatattatgctgctcgaagatgaggagctggagcaggaaatcatagccctgattaaagataagcacatgacagctgacgcagctgctcatgaagttatcgaaggtcaggcttctgccctggaagagctggatgatgaatacctgaaagaacgtgcggctgacgtacgtgatatcggtaagcgcctgctgcgcaacatcctgggcctgaagattatcgacctgagcgccattcaggatgaagtcattctggttgccgctgacctgacgccgtccgaaaccgcacagctgaacctgaagaaggtgctgggtttcatcaccgacgcgggtggccgtacttcccacacctctatcatggcgcgttctctggaactacctgctatcgtgggtaccggtagcgtcacctctcaggtgaaaaatgacgactatctgattctggatgccgtaaataatcaggtttacgtcaatccaaccaacgaagttattgataaaatgcgcgctgttcaggagcaagtggcttctgaaaaagcagagcttgctaaactgaaagatctgccagctattacgctggacggtcaccaggtagaagtatgcgctaacattggtacggttcgtgacgttgaaggtgcagagcgtaacggcgctgaaggcgttggtctgtatcgtactgagttcctgttcatggaccgcgacgcactgcccactgaagaagaacagtttgctgcttacaaagcagtggctgaagcgtgtggctcgcaagcggttatcgttcgtaccatggacatcggcggcgacaaagagctgccatacatgaacttcccgaaagaagagaacccgttcctcggctggcgcgctatccgtatcgcgatggatcgtagagagatcctgcgcgatcagctccgcgctatcctgcgtgcctcggctttcggtaaattgcgcattatgttcccgatgatcatctctgttgaagaagtgcgtgcactgcgcaaagagatcgaaatctacaaacaggaactgcgcgacgaaggtaaagcgtttgacgagtcaattgaaatcggcgtaatggtggaaacaccggctgccgcaacaattgcacgtcatttagccaaagaagttgatttctttagtatcggcaccaatgatttaacgcagtacactctggcagttgaccgtggtaatgatatgatttcacacctttaccagccaatgtcaccgtccgtgctgaacttgatcaagcaagttattgatgcttctcatgctgaaggcaaatggactggcatgtgtggtgagcttgctggcgatgaacgtgctacacttctgttgctggggatgggtctggacgaattctctatgagcgccatttctatcccgcgcattaagaagattatccgtaacacgaacttcgaagatgcgaaggtgttagcagagcaggctcttgctcaaccgacaacggacgagttaatgacgctggttaacaagttcattgaagaaaaaacaatctgctaatccacgagatgcggcccaatttactgcttaggagaagatcatgggtttgttcgataaactgaaatctctggtttccgacgacaagaaggataccggaactattgagatcattgctccgctctctggcgagatcgtcaatatcgaagacgtgccggatgtcgtttttgcggaaaaaatcgttggtgatggtattgctatcaaaccaacgggtaacaaaatggtcgcgccagtagacggcaccattggtaaaatctttgaaaccaaccacgcattctctatcgaatctgatagcggcgttgaactgttcgtccacttcggtatcgacaccgttgaactgaaaggcgaaggcttcaagcgtattgctgaagaaggtcagcgcgtgaaagttggcgatactgtcattgaatttgatctgccgctgctggaagagaaagccaagtctaccctgactccggttgttatctccaacatggacgaaatcaaagaactgatcaaactgtccggtagcgtaaccgtgggtgaaaccccggttatccgcatcaagaagtaattcttgccgcagtgaaaaatggcgcccatcggcgccatttttttatgcttccgccagcggcggcaaaatcaattcatcgctctcatgctgctgggtgtagcgcatcacttccagtacgcgcaaccccgctcggtgcactgcatcggttaacgccttccctttcagcaagccactgatgagctgagcacaaaacaggtcgccagtccctttcaggtcggtttttacccgtgaatgggaaatgacattcacgctgtcggcagtgaccaccacaacctgcatctcctgattttcttcattaccggaggcgctggtaaccaccacccattttaatgtgtctgaaagcagactttttgcggcagcaatggcactgtcgagatcgcggcaatttttaccggtcaggatttccaactcaaagatattgggggtaattccctgcgccagcggcagtaaatattgtcgatacgcttcgggaaggtcaggtttgacataaattccgctatcaatatcgccaatcaccggatcgaccatgatcaataggtcaggatggtctttgcgtagcgcagtcagccactcggcaaggattttgatttgcgatgccgttcccatatagcccgtggttacagcacgaagttggcgcagcgcatcacgctcctgaagcgcacgcaaatagccgctaaaccattcgtccggaatcgcaccaccgtagaaagtgtcataatgcggcgtattgctcagcaataccgtcggcacggcaaagacattcaggccgttctgtttgatagcaggcacggcaatgctgttgcccacgctgccgtaaaccacctgcgactgcacggcgacgatatccgcctgcagtgccctactcttatcgttaaacaacaacaaactactcatttaattttttctccttgccgatgatcctcatcgtaatccaaccgaaactttacctgattctggcagtcaaatcggctatcacaaaacaaggataaggtaattcaatgaagaaaatcatttgtctggtcattacactactaatgacactccccgtttacgcgaagttaactgcccatgaagaagcccgcatcaacgccatgctggagggattagcacagaaaaaggatttgatatttgtgcgcaacggtgatgaacatacctgctatgaagcggtttctcatctgcgtctgaagctcggcaatacccgtaaccgcattgacactgccgagcagtttattgataaggttgcttcgtcgtcatcgattactgggaagccgtatattgtgaagatccccggtaagagcgatgagaacgcacagccttttttacatgcgttaattgcgcagacggataaaacggtgcctgcggaaggaaattaatccgctttgggaaggcatttacaggaggtaacatgaaaaaacgctttatttatcacgatgaaaaatcgaataaattttggtggatagattacgaaggggatagtttagctgtcaactatggcaaggtaggtagtattggtaaattccagacaaaagagttcgataatgaagaacagtgtctgaaagaagccagtaaattgattgccgcaaaaatgaagaaaggctatcaagaagatccaaagtttaacttcatggatcgctactattttgatgatgaagaaattgggttacatgttaaaacgtcacacccaaacttccagtgccattttactgatccactttatatgtgttgctgggatgaagaatctccttttggcagcgatgaaggtgctgatgctctaaacgttcttgaaaatagcctccgtaaagagccggatctggactgtgctgatttccctcaaatgttaattgaaactatgtggggtatgaaatacatcgctatggacagtattcttgaagaggatgttcgtgcgcaattactagtcgatgaaatgagcactatccagagcaatatgattacctacgcaactgcattcggtcagattaaagtcatgggtaaaatctcccataaacttaaaaagatgggactcaatgcactagcgcgtcatcagcttaccgcaaaaattcttcaatggggtgacggtcaggactcaccaatacttcaaaaaatgattgatgaccttacggcgtttcctcacgaaaattaaatactgcatttgtcggcagcaacaactgttaaaaaagtgcgctttgtttatgccggatgcggcgtaaacgccttatccggcctacaaaatcgtgctaattcaatatattgcagaaaccttgtaggcctgataagcgtagcgcatcaggcagttttgcgtttgtcatcagtctccgatgctattaatccttaaatccccgccccctggctaaaatgctcttccccaaacaccccggtagaaaggtagcgatcgccacgatcgcagatgatcgccaccaccaccgcgtcagggttagcttttgccacccgcagtgctccggcaaccgcgccgccggagctgacgccacagaatattccttcccgcaccgccagttcgcgcatggtgttttccgcatcgcgctgatgaatatccagcacctcatccaccagagaagcgttgaaaatccccggcagatattccgtaggccagcggcgaatgccgggaatgctgctgccctcttccggttgcaggccgacaatggtcaccggtttggattgttcgcgcataaagcgtgagacgccggtgatagtgccggtcgtccccatgctggagacaaaatgagtgatgcgcccgccggtttgctgccagatttccggcccagtggtggtgtaatgcgcataagggttatcgggattattgaactgatcgagcagctttccttcgccacgattcgccatctccagcgccagatcgcgcgcaccttccatgccctgctctttggtgacaagaatcagttccgcaccataagcacgcatcgccgcacggcgttcctggctcatgttgtcgggcatcagcaatttcatgcgatagcctttcagcgcggcaatcattgccagcgcaatgccggtgttaccactggtggcttcgattaagacatcacccggtttaatttccccgcgcttttccgcctcgacgatcatcgaaagtgccgcacgatctttcaccgaacctgccgggttattgccttccagttttaaccacacttcactgccgttatccggccccattcgctgcaacttcaccagaggcgtattgcctattgtttgttctaatgtactcacgatctctatccatacgtggtgttgcctgatgcgacgcttgcgcgtcttatcaggtctacaggttacaaaccttgccattaaaaagcccggatcgcgggaagcgcctccgggcgtttaacattcactcaacctatcaggcgctttgtgcgagagcaagttcctcatcgcgggtttcgatacgctcgtcgccgttatacagccgcgcatgttgcagaccaacgaataaacgctcgccacgctgcggggcatcgtcgccatgcatcacgaccgtcagcggttcgttgtaccaccccagcggctgcaccactaattgggtgtagtgacctttcgggctggcttccagtacctgtaccggcagcggcgaatcgaggctggtacggcggctgatatccacttcccaagggcgcaggaagagatccaccggcccctgatacgcaggtgtgtagcccagcggccagcgatgcgcgccaacatggaactgcccgccgcgaatggttccctgcaggcggttcacttcgcccataaattcgagcacaaaacgggtcgccggttcgcgccatacctgatccggcgcgtcagcctgttcaatattgccctggctcatcacaactacacgatcagctacttcggtcgcttcttcctgatcgtgggtcacaaaaacgctggtgaattttagttcttcatggagttgacgcagccagcgacgcagctctttacgcacctgcgcatccagcgcgccaaacggttcatcaagcagcagaatttgcggttccacagccagcgcgcgcgccagcgccacgcgctgtttctggccgccggaaagctgcgccggataacgatccgccagatgggcaagctggaccatttccagcaattttgtcactttcgctttgatggctgcggcattcgggcgctcgcgacgcggcagcaccgtcaggccaaaagcgatattgtcgaacaccgtcatatggcggaacagcgcgtaatgctggaacacgaaaccgactttacgatcacgtgcgtgcaggcggctcacgtcggtgccgtggaagcgaatatgcccgctggtttgatgctccagcccggcgataatgcgcagcagcgtggttttcccggaaccggacggccccagcaacgcgaccatctgacctgaaggaatatccagtgagatatcgttcagcacctgggtgcgaccaaacgacttcttaatattggcaatctcaatgctcatgatgttcctcctgctgtgcgcgtttttcctgattctccaggcgccactgcaacatactttttaaaaacagggtgataatcgccatcagcgttaacagcgccgcagcggtaaaggagccgacggtgttgtagtcctgctccagcaattcaatctgtaacggcagcgacagggtttcgccgcgaatcgagccggaaaccaccgacaccgcgccaaactcgccaattgcgcgggcgttggtcaacaccacgccataaagcagcgcccagcggatgttcggtaatgtgacgcgacggaacatctgccagccggacgcgccaagcaaaatcgccgcttcgtcttcctggctgccctggcttaacatcaccggcaccagttcgcgcaccacaaacggacacgtcacgaagatggtgaccagcaccattcccggccaggagaacataatttgcaggttatgctcgtcgagccaaccgccgagcgggccgttagagccgtagaacagcaaatacaccagaccggcaaccaccggcgatacggcaaacggaatgtccagtagcgtcagcagtaactggcgtccagggaagttaaagcgcgtcaccagccaggccagcagaatgccgaacaccaggtttaccggtacggcaatcagcgcgatcatcaccgtcagccagatggcgtgcagcatgtccggatcggccagattctgtaaaaccggcatcagccccttgctgaatgcctgcacgaagatgtaaatcatcggcaccagcaggatgaacgccgaaaccagcatcccgatgccaatcagaaaccatttgccccagttaatcgggcgcgcgtcataacgcttcaattgggtaacttccgccattaatgacctaccacacgccgaccaaagcgactttgcagagtgttaattgagaacagcagcagcagagatgccgcgaggatcaccgaagcaatcgcgctcgctgccgggtaatcaaactcctgtaagcgcacaaaaatcatcagcgacgtcacttccgtcttccacgcgatatttccggcgataaaaatcaccgcgccaaattcaccaagactacgggtaaacgacagcgccacgcccgccaccagcgccggagaaagctccggcagcaccactttgcagaaactctgccagcgcgttgcaccaagcgtttccgccgcttcttcatattccgggcctaactcttccagcaccggctgcacggtacgcaccacaaacggaatgctggtaaaggccatagccaccgcaatccccagccatgtataggtgactttgatatcaaacttcgccagccattcaccgtaaaaaccgtttacggaaaagagcgaggccagcgttaaaccggcgacagccgttggcagcgcaaagggtaaatccatcagcgcatcaagcagcgtgcggcctgggaagcgatagcgggttaggatccacgccatcagcagaccgaaaacgccgttaaaaatcgatgccacaaacgccgacagcagcgttactttgtaggccgcgaccacctgcgggttggtgatcacctcccagtactgcgcccagctcatctgggccagttgcatcaccagcgcggagagcggcagcagcaaaatcaggcacacaaacagcagactggtgccgaggcttaaggtaaagcccggcagcacgcgtctggaggagacagcaaacatcagttacgccccgccgctaacagcttgtctaactcgccgccgctggtgaagtgggttttcatcacttccggccaggagccaaatttgtcttccacgcggaacagctcggtctgcgggaatttgtctttcagtttgtccatcacctccgggttattcacgcggtagtaatagtcggtgatgatggtttgcgcctgcgggctatagagccagttcagataggctttggcggctttttccgtaccgttggcctgcacgtttttatcaacccacgccaccgggaattccgccagaatgttggttttcggaatcaccacttcaaagccctgcgcttcatactgtttacggatgttgttcacttccgattcgaagctaatcagcacatcgcccaggccgcgctcggcaaaagtggtggtcgcgccacgaccgccagtatcgaacacttcaacgtttttcaggaactgggtcataaactgttcggttttgcctttgtcaccaccgtcagctttatccgctgcgccccatgccgccagataggtataacgcgcgttacccgacgttttcgggttcgggaaaatcagcttcacgtcggagcgcaccaggtcgttccaatcgtggatattcttcgggttacccttacgcaccaggaagcccatggtggagtagaacggcgagctattattcggcaggcgcgactgccagtcggccgggatcagcttgcctttatcgtgcaggatttgtacgtcggtcacctggttataagtgacaacgtcggcttttaagccctgtaaaatcgccagcgcctgttttgatgacccggcatgagattgttttatcgtcagtttgtcgccgccgttatcttttgcccattgttgctcaaacggcggattcagggcggcaaacagctcgcgggagacgtcataagaactgttcagcagttccgttgcctgtacatggcccgccagcagcagagaagcgaccagcgcgagtgagttctttttcagtaagttaacggccattgcgcacccttataaatttaatgactttctaatagccatcatatttataacggacgtgaaaggagtaacggttttatataccgtttggtgatttggaagttgaaaagggaataagaacttggttcaacaggcgtaattgttgcagtcagtttggacacgaacagcgcggagaaaccggagcgtacacatagtacgtgaggatttcgagcactgcccggggccaaaatgacaaataaaatagcctggtgaacttagttcaagacgaaatcctccccacaaatgcagggaggaaacagaggtgaatcagataccgacgctaaccgtctccggcagtgtgctgccgccatcaatcacattctgtgtaccggttaaatagctggattcatccgatgcgaggaaggccgccagttcgccgacttccagcggatcggcgaggcgacgcatcgggattgctttcgccatttcagtcagcaccgactctggatcttccgggttcgactggcgggcaatgctttccgccattggtgtgcgcacgtatcccgggcaaatggcgttaacgcgaataccagactgcgcgtactccaccgccagcgattttgtcaggccaacaatcgccgctttcgttaaggcgtacgccgtttcgccaggatcggccaccatatcaccagtgactgaagacatcatcacaatgcgaccatctttgcgggcaatcatctccggcagcaccgccttcgtgacgttccatacgcctttaatattgatgtcaatatggaaatcgcgatcgtcatcgctcatatcgaggaaactgcccagacgacaaacgcctgcgttattcaccaggatatcaatgcgcccttctttttccttcgcgcgtttgatagctgcggctaccgacgccgggtcacgcacatcggcgacaaccgccgtacagcgatgaccacgaccacacagttcgtccgccagcttttcgatctcaggggagatatccagcaagattaggttcgcgccatgacgtgcaaaagttctggcaattccttcgccaattccctgcaatgcgcccgtaatcagtgctgtcttgcccgtgagtttacccattttaatgctctccttgttaatacagagcgttacactccattccctctgaaaatacaggataaacaaaatattgctgcggatcagctcactaattcaggaaaatctcaatccagtcgctgctttatgcatcatttcaggcgttgtgttagctcactgctgcgctgaatcattttcaatgactccacatcattgagttgcacaaggccaacaaacagtaaatcggtaacagaattttgcgccgtgcgggtagacatcgacgagctacgccattcggtttctccggaaacggtatcgagggtgaaatgcgccagccgccgcagcggagagtcagtcagagaagtaatggcaatcaccgttgccccctgctttcgtgccgcttctgcgcacaagacaatctcttttttactgccgctgtaagagatagcgatttgtacatcgccttttttcaacgcctgagaaacggtggcttgtacgtgcgtgtcggcttcgcaggccacgcgatagccaattttcatcagtttgaacgacagatcgcgccccaccagcgccgatccgcccaggcccgttatctggataaacggtgctttactgatgacctcaatgattttttgcagccgcgcgtaatcgagcaacgcgcaggtttgctccagcgccagctctttttcgcgattcagtttgcgcgcgatcacttccagcgaatcatcactggtaatcgaactgtgcaggtgcagtgccgtggcattcgttttctcccggctggcactgtattcgcctattaacgccatacgcaattcagtaaatccttgcgcgccgagtttttgggcaaatttcactatgctcgactggctaatgccgagctgtttcgccatctgccgtgaagaaacggattgcagctcactcacgttggcctgcagaaagtcagcgattttttgctcgttttcggtgaattcactccccgcattgcttattttcgtcaggtacaacatcttccactctcctgggctggcagcataaattccgcttaagttcttatgacgctcttcacactctgcgagtgtagactcaatgattcctttaagcctgtcaattcgggatatatgattccatacatctgcaattatttgatcgtaaatagtaaggtcaccaccgatgcaatttgaaaagatgattactgaaggctcgaacaccgcctcggctgaaattgaccgcgtatcgacgctggaaatgtgccggattatcaacgatgaagataaaaccgtaccgcttgccgttgagcgcgtactgccggatatcgccgcggcgatcgatgttatccacgcccaggtaagcggcggcgggcgtctgatttacctcggtgcgggaacatccggtcgtctggggattctggatgccagcgaatgtccgcccacctacggcgtgaaaccgggtctggtggttggtttgattgctggcggcgaatatgccattcagcacgcggtggaaggcgcggaagatagccgggaaggcggtgttaatgatctgaaaaatattaatttaacggcacaggatgtggtggttggcattgctgccagcggtcgcacgccgtatgtgattgccggactggaatacgcacgccagctcggctgccgcacagtgggaatttcctgtaatccggggagcgccgtttcaaccaccgctgagtttgccattacaccgattgtaggtgccgaagttgttaccggttcttcgcggatgaaagcaggtacagcgcagaaactggtgctcaatatgctttccaccgggctgatgattaaatccggcaaagtgttcggcaacctgatggtcgatgtggtcgccaccaacgaaaaactgcatgtgcgacaggtcaatattgttaaaaacgccaccggatgtagcgcagagcaagcggaagcggcgttaattgcttgcgagcgcaactgtaaaacggccattgtgatggtgctgaaaaatctcgatgccgcagaagctaaaaaacgcctggatcaacacggcggctttattcgtcaggttttagacaaggaataacccatggccaaagagatcagcagtgaacttctgaacaccattcttacccgtgtcggcggaccgggaaatatcgccagttgtggtaactgtatgacgcgcctgcgtctgggtgtacatgacagttcactggttgatcccaatatcaaaacgctggaaggcgtgaagggcgtcattttgaccagcgaccaggtgcaggtcgtttttgggcctggtaaagcgcatcgtgccgcaaaagcgatgagcgagctgctgggagaagcaccggtacaggatgccgcagaaatcgccgcccagaacaaacgtcagttaaaagccaaacaaacctccggcgtgcaacaatttctcgccaaattcgccaccatcttcacgccgctgatccccggttttattgccgccggtctgctgctggggatagcgacgttaattgccacggtgatgcacgttccggcagatgctcagggaacactacccgatgcgctgaattttatgaaggtgttcagcaaaggtttgttcactttcctggtgattctggtgggctataacgccgcccaggcatttggcggcacgggcgtaaatggcgcaattatcgccgcgctctttttgctcggttataaccccgcagcgaccaccggttactacgccggttttcacgatttctttggtctgcccatcgatccgcgcggcaatattatcggcgtgctgattgccgcgtgggcctgcgcccgcattgaaggcatggtgcgccgctttatgccggacgatctcgacatgctgctgacctcgttaatcaccctgctgatcaccgctacgcttgcgtacctgatcattatgccgctgggtggctggttattcgaaggtatgtcatggctgtttatgcacctgaacagtaatccgttcggttgtgcggttttagccgggctgttcctgatcgccgtggtatttggcgtgcatcagggctttattcctgtttacctcgcgttaatggacagccagggattcaacagcttatttcccatcctttcaatggcaggcgcgggccaggtgggcgcggcgctggcactctactggcgggcgcaaccgcacagtgcgctacgcagtcaggtacgcggggcgattattcccggcctgctgggcgttggtgaaccgctgatttacggtgtcaccctgccccgcatgaagccgtttgttaccgcctgtttaggcggcgcggcgggcggtttgtttatcggcctgatagcctggtggggtctgccgatgggcttaaacagcgcctttgggccgtctggtctggtagcgctgccgctgatgacttccgcacaaggcatccttccggccatggcggtttatgctggcgggattctggtggcatgggtttgcgggtttattttcaccacgctctttggctgccgtaacgtcaatctggactgatatcatgaaacggacaatgctctatctttctctgctggctgttagttgtagcgtcagcgccgcaaaataccctgttctgacagaaagctcgccagagaaagcagggtttaacgtcgaacggcttaaccagatggatcgctggattagccagcaagttgatgtcggttatcccagcgtaaacctgctgatcattaaagataatcagattgtgtatcgcaaagcctggggagcggcgaaaaagtacgatggcagcgtgttgatggaacagcctgtcaaagccaccaccgggacgctgtatgacctggcctcaaacaccaaaatgtacgccacgaacttcgccctgcaaaagctgatgagcgaaggcaaactgcatcctgacgatcggattgcgaaatatattccggggtttgccgatagtccaaatgacaccattaaaggcaaaaacaccctgcggatttctgacctgctgcatcacagcggcggtttcccggcagatccgcaatacccgaataaagcggtcgcgggcgcgttatattcccaggataaaggccagacgctggagatgatcaagcgcacgccgctggaatatcagcccggcagcaaacatatctacagcgatgtcgattatatgctgcttggatttatcgtcgagtcggttaccggtcagccgcttgaccgctatgttgaagagtcgatttatcgcccgctcggcctgacacatacggtatttaacccgctgctgaaaggctttaaaccgcaacaaattgccgccacggaattgaacggcaatacccgcgatggcgtgatccatttcccgaatatccgcacctccactctctggggtcaggtgcacgatgaaaaagccttttattcgatgggcggcgtttccgggcacgcaggtttgttttccaataccggcgatattgcggtgttaatgcaaacgatgctgaacggcgggggctatggtgatgtgcagctgttcaatgcggaaacggtgaagatgttcaccaccagctctaaggaagatgccacttttggcctcggctggcgcgtgaatggtaatgccaccatgacgccgacgtttggcacgctggcaagcccgcaaacctacggtcacactggctggaccggaacggtgaccgttatcgatccggtgaatcatatgacgattgtgatgttaagcaacaagccacattcgccggttgccgatccgcaaaagaatcccaatatgttcgaaagcggtcagttgccgattgcaacttatggttgggtagttgatcaggtgtatgcggcgttaaagcagaagtaataaaaaggccagtcagtaatgttactggctggtctgagagtgctgacaaacgcaaaactgcctgatgcgctacgcttatcaggcctacgtggagcccacaatatattgaattagcacgatttcgtaggccggataaggcgttcacgccgcatccggcgtgtacaacgcgcacttggtcaacaatctgaggccagtcagtaatgttactgcctggcctttaatcaatgaatcagaaacgcttacagcgccatcaacttgtccagcgacggtgcgaaataatagccgccggttaccggtttggtgaaacgcaacatcgcatcacgcttaccatcggtatcgccaaacatgctcagcagttgctgctcaatgttatgcagacgcgcgcagtaggcgcagaagtacagaccgtgagtgccactggcagtgccgtacggcaggctctggcgaacaatcttcagccctttgccatcttctttcagatcaacgcgggtgaggtgagaggtttccggacgttcgtcgccgtcgatctcttcgttggcctctttggtgcgcccgatcaccatctcctgatcgtgaacgctcatccggttgagctgcttcaggttgtgttcccaacgctggacaaacacatagctgccgcccgcatccacgccgtctttgataaccgccacttcgcgacgcgtctcttcacccgccgggttttccgtaccgtcaacaaagccgctcaggtcacgctcttcaacccaacggaagccgtggatctcttctttcacttcaatgcagtcaccaaaggcttccatcgccgcctgggcgacagagaagtttacgtcgtgacgcagagaaagaatgtggatcaacacatcgaactgggtcgtcggcgcaaggcctttaccgtagcccggaaaatctttcagctcttctgccccaacgccgccgctcagagcgcgccaggtgttgttaccaaaggcaaccaccgcaccaagatgcgcgtccgggaatttcgcttcaaaagttgccagtttgtcggcaaatgttttactggccgcacgcagggcgtcaacttcccctttcacgttggcttcgatccaaatcgccgcgcggcaatgttctggcaaaatgccactctgaacctgagacattgttcctcctgaaaataataatgccacgcaatccgtggcattgttgagcgctattttacgtgttttttcgcggcggcggtttgttcagacgcaaattaacgccgccagataattttactgactttccagtttttcagggtatcgtccgaaggcattaacccttcaggaccacgccattccccgctgaactggtagctaatatgttgactgccttcggctttacattcgacggcacgattatcatcaccatcagctttttggcaattgccaaatgctttgctgtaaaggtcgctaaacggtgtaccgattttaacaccggtgtcagcaggaatatcgctatccagcacgtcaatgcgactgatcgtgccttgatcgccgttaatcaccatcgccacgttgtcgcccttcatcacttcaaaaaagcgcaccacgttgccgttcgcggttttcattccgctgcgcaggcgataatcgccatcaagcgcatcggcaatggcttgttcttgcagtggtgtggacgccgttaattcacccacgccctgctcgctcactttggtggacgacccaaaccagttccacgggttagcggcagaccagttaactgacgacatcgtggaacagccggtcagcatcaatggcatagcgcataacattaaacgcagcgatttcatgtcacttcctttggttattcaataacgttgcttggagtgcaaattcaccaaaaagtgccgttattcttttacttcataaaaacaagcgcgtaaacgtcgattggtcagcagccagattaacgccacaatatccgccactaccagcgccagaccgataccgctaacggattcaccgttcagccacagccacggttgccagcaaagtaaaaccacctgcgccaacagcaacagaaaatagagtacacgccaggtgcgaggaaacgtagcccgccgaccgctcaacaaaaacgccagcaccgccggaatgccaggaatcagccccagccagaaattatcgtgatcgggataaaacagatttagcagcgcagtaccctgctcgcgcgacgcaccggcaatgacaaacagcacccaggttcgcgcctgaagcaatagcacaagccagaagagcaagggtaaacgcaggcgaccgtgcgcatcataatggacaggatgaaactcagtactcttcatcttcaatcaaacgcttacccagactcagcacgtcggcgtgttcatatcccaggcgttcatacattccgagcaccatgtcgttatcttccggcacattgatctgaattttcgggcagccacgagcaatcagctttttctccagccgattaagcaacgcattggcaatcccacgcccacgaaactctggatgcacgccaagataataagcagacccgcgatgcccgtcataaccgcccatcaccgttccgaccacgtcaccgtttacctcagcgaccaaaaacaaactgacgtcatggttcatcttacgctcgatgtccatttccggatcgttccacggacgcagcaagtcgcaacgctcccaaagggtgatgacctcttcgaaatcttcctggcgaaatacgcgtatctccatggtattcgttacctttttgcgggttaaaaggctgattatggcgtgaacggtcgaattagccaatatctgacgaaaatcggttgaaaaagtggcataatggggagttgtcaactattgaaatgaaaagtaaaacaattctcaacagcaaaccgtcgtaacggattacgcgatacgatataacatctggaactttattattacaactcaggccgtatgagcacttttaaaccactaaaaacactcacttcgcgccgccaggtgctgaaagccggtttggctgccctgacgttgtcaggaatgtcgcaagccatcgccaaagacgaacttttaaaaaccagcaacggacacagcaagccgaaagccaaaaaatctggcggcaaacgtgtcgttgttctcgatccaggtcacggcggaattgataccggagcgatcggacgcaacggttcgaaagaaaaacatgtggtgctggcgattgctaaaaacgtccgttccattttgcgtaatcatgggattgatgcgcgtttaacgcgttctggcgatacgtttatcccactttacgatcgcgttgaaatcgcccataaacatggcgcagatctgtttatgtcaattcatgccgatggctttaccaacccgaaagctgccggtgcttcggtatttgccctctctaaccgtggggcaagtagcgcaatggcgaaatacctgtctgaacgcgaaaaccgcgccgatgaagttgccggtaaaaaggcgactgacaaggatcacctattgcaacaagtgctgtttgatctggtgcaaacagataccattaaaaatagtctgacgctcggctcgcatattctgaagaagattaagccggtgcataaactgcacagccgcaacaccgaacaagcggcatttgtggtgttgaaatcaccgtcggttccttcggtgctggtggaaacctcgtttatcaccaacccggaagaagaacggctgttaggcacggcggcgtttcgtcagaaaatcgccacagcgattgctgaaggcgtgatcagttatttccactggttcgacaaccagaaagcacattcgaaaaagcgataagttatgaaacccgacgcacaccaggttaaacagtttctgctcaaccttcaggatacgatttgtcagcagctgaccgccgtcgatggcgcagaatttgtcgaagatagttggcagcgcgaagctggcggcggcgggcgtagtcgggtgttgcgtaatggtggtgttttcgaacaggcaggcgtcaacttttcgcatgtccacggtgaggcgatgcctgcttccgccaccgctcatcgcccggaacttgccgggcgcagtttcgaggcgatgggcgtttcactggtagtgcatccgcataacccgtatgttcccaccagccacgcgaatgtgcggttttttattgccgaaaaaccgggtgccgatcccgtctggtggtttggcggtggcttcgacttaaccccattctatggttttgaagaagatgctattcactggcatcgcaccgcccgtgacctgtgcctgccatttggcgaagacgtttatccccgttacaaaaagtggtgcgacgaatacttctacctcaaacatcgcaacgaacagcgcggtattggcgggctgttctttgatgacctgaacacgccagatttcgaccgctgttttgcctttatgcaggcggtaggcaaaggctacaccgacgcttatttaccaattgtcgagcgacggaaagcgatggcctacggcgagcgcgagcgcaatttccagttatatcgtcgcggtcgttatgtcgagttcaatctggtctgggatcgcggcacgctgtttggcctgcaaactggcgggcgcaccgagtctatcctgatgtcaatgccgccactggtacgctgggaatatgattatcagccaaaagatggcagcccagaagcggcgttaagtgagtttattaaggtcagggattgggtgtaactccctcacccccactcccgcatccgctgatgcagcgtcagtgacggcttctcggaaaacagctgctggtaatccgtggcaaattgccccagatgccagaatccccactgcatggcggcgtcttttaccgtcatactttgcgaccacggacttatcagttcgcggcgtacggcgttcaggcgaatgcgtttcagccacgcgttcgggccaatgcctaaaatagcgtgaaacgcgttttgtagcgtgcggcggctgacatgcagttgattacacaaatccagcaccgtcaccggttcggacatgttttccagcacatattcacgggcgcgggaaagcaatcgacggtaactctgatgactgatgctttccgccgtcaccattggttgcgcttcttccagcatggcccccatcgccattagcaaattatcccccagcacttttcgcactgcaggctgatggagattttccggattctcgcaaaacgtcgccagcgcctgttggacaaagccccacagcgcggctttatgctgctctttcacttccagcgccgactggttacgcaacatatgtaatacccgatccgggttatgcaaaaagttagcctgccgggtgatgacatcttcagaaagcaccacgcccaggatcgtgtaatcatccggcgtgctcagttcaaattcagtgccaccagggcgggtggcgatttccgcgcttcccagacattgcgaaccgataaatccctgctcaccgcgcgtcgccggaatgccaaaccagaacgagttcggccagaccaggcacgactgacgcagcgccagaccggtgtattcacgaaaaacctgaatatcatcgagtagaatttccgtaaattcaccatgaaacttgcccggatgcagctgatcgtaaatctgctgccaggcggtaatcgttaaagcatgttcatagacatccgttgtctgtcgttgatgaacattatccacttcgaccttcggcgtgagcttcaggttttcgggtaagggttcatgataaagatggtgcaaattggctgtacgggtctttttcatgatgttaatgccgggtgttgtaggacacccggcacctccgacaggttaatggggcttgagacgataacgactactgcgtttacgtaacgtcccggcagaaaagagctgttcgagcgcatttctggctttttccagcggccagccaaagtgggcagccacttctcctgccgtcattccctgacgtactgatgttaacagcgccaacaactcgtcagcagattccgcgacgataactggcgcgtcgggttcccttacgggttgcttcggctggcggttaaagccagtaaccagccactgggtgtcatcgtctggccgaccgatctccttgcggctgatgacacgcccggtacgcatcgcggcagcacaacctgcgtccagcgccgcacgacacgccgccagatcgccttccaccaccagcgttaagcgaccagggtcaagcacttcgtgactgagcagacgaacgttagctgctttgagcatggcatccgctgcatctatcgcggcgaccatgccgtccacttccagcaatcccagtgcattgatcatcggcaacctccgttacgcacgctggattggattacgcgcgatttccagcactgcatcggtaaaggcgttacaggctgctttacacgctgcctggctaccggttaaaaatgctgccgagtagttggtttcagacggtggcgggacataggtcgccagctgtacgtcggcagacttcagggctgcatcaatgccataggtcgcttccagcggcggtgccaccagatacgccatcggatcgccaagcgtgatcccggcggttgatgagagataagaaccggtacgcgaaactacatgtgccaggaatgccgtatcttgcgcgtcattagcccactggaaagctgcgccattttcaatatgcgcaatcatcgcatccagacctgcacgcacttccgccgggtttggcccaccaagcataatcagcacttcaccggcagtcggtgacgggccgtgtgcagcgcccgcatatagcgagcggccatacaccacttccaccatcgcctgcttggtcgcttcatcagcggcaatgtaggtgacgtcatcggagtcggcagaaatcagaccgaggctacgaatatgcggcggcaatttcagttcacgcgcaaaatcggcgttaacggaggcaatcacccgcatagcggtgacagacggtcgaatcaaatctaaagctggcatgatgcctccttatcgggtcatgttgatgccggatgctttctgctccagcatacgtttcgccaaatccacaatgacggctgcggcttcaaccggcggcgtgccgccctggtgaatgttagagatacaggtgcgatcggcctcaacggtggtcgccatacgcggcgagtaaacggcgtagcaggagaggctttctgactgacccaaccccggacgttcgcccaccagcaggatcactactttcgcgccgaggatctcaccgatctgatcttcaatcttcacgcgaccataacgaacaaagaatggtgtaccgactttcagcccggcctgtttcaggcccgccatcagcggtggcaggatctcttcgtagttcacggtgatcgcatcagttgacaggccatcagaaataacgacctgtacgtccggattggcaacacactgcgctttcagcgcttcaacagcttctgcacacaggcggcggcccatatccgggcgagtcaggtagagatttttgtcgctaatttcagagcgtacttccagcaagccctgcgctttcacccactcttccggcacttctttcagtacggtatctttcgaacgagagtgatcggccaggaaacgcagcagcgcctgcgtacgtggacgcggaccggcacgaccggtacaaacgcgggccacggtgctgcggcgcagttctgttaatacgtctgcgcgatgcggattttcaacaccaatccacgcttttgcttcagcggaacctaaatccagcgcacagctttccgaggtcaccggtgccgcacagttggtggtggcgcactttgcttctgacggcgcgggggccgcttgtcccattgacgccatcacgctgcgtacaatttcttcaatctgtttttgatccatgatatgttatctccgcgtcatcagaagaacagtgacggatcgcccgcccgtttggtcaggcgaccgtttgccataatgcccatgctttccagccagcgttcaaactccggtgacgggcgcaggttgagtaactgacgcacagtggcggtatcgtggaatgcggtggtctggtagttgagcatgatgtcatcacccagcggcatccccatgatgtagttgcagcctgcggtggcgagcaggatcatcaggttttcgttgaggttctggtcagcgtcagcgtggttggtataacagcagtcacagcccatagagatgccgctcagcttgcccataaagtgatcttctaagccagcacggataatctggcggtcgttgtagagatactccggcccaataaagccgaccacggtgttgacgataaacggatcgtaatgacgcgccagcccgtagttacgtgcttccatcgttacctggtctgcgccgaagttagcgccagcggatagcgcagagccttgtccggtttcgaagtagaggcagttttccccggcgatacggttgaactccgcgcccactgcgcgcgcttcgtcgagcatcgccagctccacgccaaactctttcagccctttttcgctgccacagatactctggaaaatcagcccgcccggtgcgccacgacggatcgcttcgatctgggtggtgacgtgcgccagtacacagccctgagttgggatgttgaatttgtcgatcacgccatagatggtatccaacacgcggcttaagttttccacgtcgtcagtcaccgggttaacgccgatcaccgcatcgcccaccccgaaggaaagcccttcgtagatttgcgcggcgatactttgcacgtcgtcacgggtgtcatttggctgcaaacgggcgctaaaggtgcccggaataccgatggtggtattggcctttttgattaccggcattttcttcgcgccgtagatcaggtccgcgttggagcaaatcttcgctaccgccgcgaccacttccgaggtcagccctttgcgggtaaaggcaatgtcgtccacgctggtttcatcgctcagcacatactcacgcagttcgctgatgctccagtttttaatctggttgtaggccgtttcgttaacatcgtcctgaatcagccgcgtcacgcagtcatcttcataggcaatcaccggattattgcggatgtccgctacggtcatttccgacaacacctgctttgccgccacgcgctcctgtgagcttgccgctgcgacgcccgccagcacatcccccgaacgcagttcgttggctttagccagcacctcttttacatccttaaactgatatacattgccgaacaatgtggtctttagtttcataagtcgttccctcaggaagaatcgatgattggcatttttcacagcattctaacaatcacgtttcatcgtcagcccttgtcgtgtaaggtggttgcctaaacacgcccgttattcatcacgccgaacgcgccggatacatgatcggggttatccagtcgttaaatcaaggtatccggttttgagcaagacaccactcacagcaaaggccatagacgccgcacagccgcaggacaagccctataaactcaccgattcactgacgccggggctgtttttgctggtgcatcccaacggttcgaaatactggcgattcaggtattggctgaataaacgagagtttttgcaggccattggagtttacccgctaatcacactcaaagaagcacgcaggcgcgccacggagagcagatcccttattgccaatggaattaacccagtggaacaagcccgcaaggaaaaagccattgatgcgctcaacatggcggcaggatttaagaaggtggcggaagactggtttgctaccagggttggagggtggtcggaatcctatgcaaaacaggtcagatcggcactagaaaaagacgtctatccggtacttggcaagcggtcgattgtcgatataaccgcccgtgacgtgctggcattactccagaagaaagaacgtaccgcaccggagcaggcccgcaagctacgccggcgcatcggtgagatcttcaagtttgccgttatcaccgaactggtaacgaggaatccggttgcagatcttgatacggcactgaaggcccgccgacctggtcacaacgcgtggataccgattagtgaaattccggccttctacaaagcccttgagagggccgggagcgtccagattcagacggcaatacgtttgcttatattaacggcattaaggaccgcagaactgcgtttgtgccgttgggaatggataaacctggaggacgcaacaatcacattgcccgctgaagtcatgaaggcccgccgcccgcatgtggtcccgctatcacggcaggcggtcgagctattgcaggaccagttcacacgcagcggatacagtgctttcgtctttccaggccgattcatggataaacccttgtcagccagcgcgatacttaaagcgcttgagcgtatcgggtacaagtcgatagccacaggccacggctggcgcacaacgttcagcaccgcacttaacgaatcaggcagatactcgccggattggattgagatccaactagcccacgtcccgaagggaataaggggcgtttataaccaggctgcctacctgaagcaacggcgagcaatgatgcaggattacgccgacgctattgattcaatattggcaggtaacggcaatcctctagaaccggaatgaataattaagcggcttttttgcaaagcgcaattttgcattttgtataagtatttgttttgtgtggtttaactatcacctgataagaaacctgtattcaatttgccggattcgtccggcttttctttttcgctaattattccattattccaattaagtggaataaattattcaatatcaagaacttaaatccatgtttgcaacgaaagatccagagttcgaaaataggatcaacacaaataaaagcccccggaatgctgcaacatgccgggggcggtatgagaaacaagctaaaggagaatttctcatgtctgatatgctagcagtagaacaagaaacaaacaatgatgttcgtcaatttttaaacaaaattaacgagttacggaataaagcacccaaaaacgaagagactaaacacgaagaacacacgccagataatcacgaggaaacagatcatcacgaggcaaaacagcaggagcaagcctggcgtggcaacctgcgctacctggacacattaaaccgacttgatgaagtattgccccgcaaactgtacgaaagatgggagaaagaacatacagtcaacgacgaggctgtgctacgtgctctttgttacttcgctggtactggcaaaaactcacagttgggatggtgcagggttggtaggggaacaatcgacaaacgagccaggctatcaaaaaacacggttaaaaaatgcctcgatcgtctggtcaaccacttcaaacttgttgagcgtactgaaggctatataccaggatcggcagaaagggagtgcaacgaataccagttattattcaagccgtacaacatgaaataacggaatcaggcgggcaatgttcccgccttttctttgccttaattccatgaattcaggtgggtcaaaagttgccgttagtggtgggtcaaaagttgccgttaaggtgggtcaaaagttgccgttaaggtgggtcaaaagttgccgagtaagaattctactattaagaattctaggcgacgggagttttttagcctcccggtcggtcatagagagtcgcctagagttaaacagaagaattatttcgccgcctgataggtcggctggttgcgagcattaaccatgctgattagcgcaatcatttccagcaagctggaaacgcccattcactcacgcacaacctgaacagcagaccaacaaaccatcatggcattcgttcatggggagcgcggtatatctcaaagggtgatttcttattggtgggccttcggaaggcttcgagcaattgccagcttaaaagacgggcttagcagtgatggttatccgccacgaatgtccgtcatattgcattgcgcagaaacgcgtggcactgagggagttttccgaattagttttggggaccctttccctgcttctggagcaaaagacgaacggcaaatgcagtgcttccttgtacgactgcagcgaagaagaaaagctgtttgttaagcgcctgaagttaatcaaagcggatatccacgcccagctgaaggcctgtgattgcgatatttctgaatgacaggtggaatcatgaaacacgtttttaaatatcttgattttgcagaagaccgcgaacacgcagaatcagtggcgaccaaagagttaaaactggaccacgtagaaaaattcgctatccgcgatctagccaatgatatcaaagagcgtgggtgtgttgagcttgtccagcctggtggattcgatgagctggttcagatctatgaggccggaggcgatggaatagagccactcaattgtggaatcgaatcaaggaaggtggcaattgctgccctgcttcgcgtcatgcgtgaaccagactttcaatgcctggaaatggttcacgaaatcataagaattgctagagatttggaagcgccagttgacgctccgttagattgctaacgccaaaattagcgctgaattaatgggtaattattgcggtttttgtcaattttcaacctcaattcttgcgaaaaatggcaaaaataacggtatttttcatcatttattgggggttttatggaaggcgaactgatagaaaacaatgggttagacatttatgacaccagcgaaacaccgaaaaagcgcggtcggccagctaaatataatgaaaaaatagcaacgcaaatcgtcctattggtaagcgaaggttatagtttgcgcaagatcagcatgatgccagggatgccgagccaccgtcagatgatgcgctggcaactggagcatatggacttcagggaagggatagcctggatgtcgtggctatggtgcgctgaagctggccgacgtgccgtcgagataatcgacgaggttgatataaacgcagaggatgggccgaagcagttgcgcaaagcagaagcaaaggcaaaggcactactggcagcagccaagctgaatagtttgaaacattcaccatttggagatgacaaacaatgagcctgatccgcactgaaaccagagacacaaaacgcgcagctgacccactgcacgacctgcgtagcaagccgttttctgagtggggcgaagatgaaatcaggcgttttaatctgatagacgcgcttcttgagtttgtctacacagacacatccagcccgttcggtatcggcatgaccttcgattacacggagtgctgggaaattggtgttcgtgacgactgcctggtaatgacacgcgttaagccggtgcatccagaatatgcgaagcactggaacatgaaaggcgtcatgaatgacaaaacccgcttccacgccgacaagtgggtagggtacagcaaggtgcttgcctgggtgagcttatcgcacaaagacaccttcacgggtgcgaaacggtttcaatacttccaaacgatgtacgacatggaacggcaaatcaacgcaaacctgccggttggcggccttcccaacgttgacacagagcgaactggcaaactgttccaacgcgatgacttttctgaggatagccatgccaacgatccgaagttggttggtgatgattacgtcccccaggcaccggagcaaatcaactgaattttcggacaaacgcgcgcgtagccgacgtcagcggcaagactggcggtcatttccccgctcctacgcgaaaaatccctcacaactaccctgcaaattttccagatttcacgtacacgcgccaaaaataaaggcccaggcagttagcaacctacccgggcctttctcacaatccccgctgacattatatcacccatctttccgttttcaggtgggagactgatggccgccgacgttgcacaattgattaatttctgaacattcaaatcaactcccaccaaagccaacaagatgggaggtgaattttgtgatgcagatcgctttttcccttcaggcatttttgtttaattcaatcaacgaaaggcagttcccaacaacaaaataaagatgggaggtaaaaatgaaacggtgggaagtggctttactggtgatggtaatgttggtttgctgtattgaactgtgaaggaggacgccatgaaacttttaatcgcaatcatcctgatggtgctgactggtgtttgctttgcagatgttggtgattacaggctgaacggggaggataacgcaagaattgaatcagtcgttactgataactgtgaaaaaacagccgtattggtaggcggtgacaggcttgcgagggttgagatcgaatatatagcgacattgtgcaagccggtggctttggtgattatttacgacagatttgacgatatagcggcaatccctcttaaggtgacgttgaaaaaggtattgaaagagaatagcgatgaaaagattaacctattgaacaagatgggggatctggctggtcgtatcgttgcagagcagtatttaggcatgagttttgagtaaggaggcaatcatgaaagtgttaggtaatattttatggtgggcttttgttggtttcatggcttacgccactttgattaagccggacaacactgatccagctgttgtgaactatgaagagcctttgcctatggagcttgccaactatggcgaaccaggtgaaggggcgaaaatcatgaatgccgcaaaaataatgggtcgcgactacgcatggaaacatgtaaaagaagacaggttgccatgtctgtttgccgccggggttgttgctgataacatcctggtaaaataccatttcagcaatgaaactgagttcaaacttaaagcggcagcggtcagagaatgcgccaacgtagcagaaaacaacggctttgttttggtaggtagagtatttgaaaaacgtaattgattgcgaatagcaacaactaaacaaccaatacacccggcccctcgccgggttttttgtgatctgcgtcaatattcccttccgttacgcttaccctccaccaatacgcgtgttaacctcccaatggattctatgagatgggagataaaaatcatgagttacgaaatcaaaatttgcgacatcctcaaaggcgctgcgatggaaggacaatataagggcgctcaacgtggggccaaatgcgaggagatcgcaaacgagttaactcgccggggagttaaaaacaacaagggagaggttattactaagggcggcgttagccattggctggaaggtagacgggagccaaatttcgacactctggctgaactgtgcgacatgttcggcgtttatgccctgatgccgatgcgtggcggtaaatggattcgagttcacccggaagaccgtggagaaatggaattacgcgaggctgtagctgaacgagatgctattatcgacgacctgaaggcccgtatcgctgagcttgaggcggcactagcaaataaacaagtcccagcagaagcggaagagatgggaggtgaaaaagtggaagaagtggcagcagagcaagcgcccaacgatgaaaaagagatgggagctaaggagtgggttaacccgaacccgaaaaaatacagcgtcggcatgttgtgtcaggtactggctgcaatgggcggcgaatacctgggcaacaacgcagggttacagcagaagatcactgtgttggataacgacggcaaccggaagccaatcagtaacggcgcgttttatcgactgattgagcaggccaaagggagaggattgattagcgttgaacaggaaatcaaacacaagaaagacgaaaacggcaaccagatcggcaaaggcaagaaaggtgacaagctgataactttgcttcccaactggattgataagctgggagacgaataaaccagccttcaaccccatctcatcaatcaacgcccggccccgctgccgggtttttgctatgcaccacaattaccccaaccggatacacagccggatacaattccaccagcacccagccacccagcgccaccgctggcgaataccgcattcaggaaggaaatgcgagtgatttcaccgtcaccggcacaaccgatccgccaaaaagaggcgtaccaatgtcgatatagtcccccgcgcggacaatcacttcgtcaatgactgccaacgggagttgttgtagctgtgggcgcaacaacatgcccagagctttaccaaagtcctgcccggccaccaccagcaggggatgcggattcggaaaacgcgcgacgaaatcgaccaacgcgttgatgaccgtcagtaccgcggcgtaacgcacaggcagcgaggcgggaagcgccagcacgtacgcgtcagttttgggatcaagatccagctgaatcagcgcctgttgccaggcccccaccagatccgtttcatcaatcgggatcgccaccggcaaattgcgcagcggcagttgtacgccctcaagccagattgtgctgccagagagcgaaagggtatgcgcgcccgcgccaatcaccgtggcgcgcacggtttgcgccggaaactgtacgttcatctcacgcaggcgcggatggtcatgcagcgcagttgccagcagcgggccaatatcggcaaaacagaacgggtcggcgggctggtggcgataacattcgcccacgccgccagaaagcgtaatgatttcgggcgtaacacctgcgggcagcaaaccggtttgcatcaatgcctgcgcgagcggtgagagcgttccgtcaatcacttcgacaatcagttctgccatccgccgggtcacctgcaccagctgcgcgccggtcagcgaacgggcgtcggtgcctgcaccgaagcactcatccacaatcatctgccccggtttatgagcgtaaaccacgcgcccgtggctgtcggtttccagcaggcgaccaccgacgttgaggcaggcagtgccgctgatttttccggcatcgaacagggcgtagttcgcggtgccaccgccgatgtcgatattcagtacccgacacagccgttgttcagaaagggtttgtgccccggctccgtgaccggcgatcacggattcgaggtgcggcccggcgctggcaacgacaaaatcgcccagcgactgagagagcgccatcaccgccgggcgagcattgcgggttttcgcgctttcaccggtgatgatgatggcaccagaatcaacgctttccggctcaatacccgcagcatgatattgctcgagtattaaggttttcagttccgcttcttttaaaccgccctgtttatcgacaggggtaaagaacaccggactttgccagctaatttcgcgtttaatgaattcgtagcgcggcacctgcgacaccgccgcacggttaaccagctccagccgggagaaaatcacctgggtggtggtggtgccgatatcgataccgacgctcaatagctggcgagtgttcacgattgtgcctccgcttcggttttagtcgcggtcgcgtcttcttttggcaccagcatcatcgccacgccaatcgccgttacgccgccgatcaacttgccgacaatcatcgggaagatcatggcgttcatgttggcagcggcgaagcctaagtggtcgcccagggcgaaagcagcggaaacggcgaaggcgcagttgatgactttgccgcgggtatccatctgcttcatcatgccgaacatcgggatgttgttggcaagcgttgccaccatgccggctgccgcgatgttgttcatattcagtactttaccgacgctcatcagcggtttttcaaaccagcgagtcagcagcagcaccatcggatacgcccctaacagaacgcaggagatagaaccgataacttcaatggcgcgcatcacctcaccgggtttatcgccaggggccataaagataggatccagaccggggatcagttcccagccaagcaggaatttcactaccgcagcggcaagaccgagggtgatcaatgcaacgaggaatttggcgaagatctggaagccgttgatcattttttccgggatgaatttcagccccagcgccaccagaatcgcaacaatgatcaccgggatcatgttcatcaggatcagggcgaaagtgaattccaccggctggccgttgatctgcacaccggagtacatagcaaccagaccaccagcgatacaaccaatcggaatggtcacaatgcccgccagcacgccgagcgccagataacgacggtcagaaggttcgataatgccgagcgccaccggaatggaaaacacaatcgttggccccatcatcgacccgagaattaacccagagtatagccacgcggctacgtcgccgcccgccagctctttggcgaggaagaagccgcccatatcgcacgccagcagtgttccggcgaacatcgatgggttagcgccgagcatttcgtaaaccggaataattaccggcccgagaacgtgagccagtaccggtgccagcgcggtcataccgaccatcgccaggcccagtgcgcccattgccataaagccttcttcgaactgaccgcctgatccttcgatacttttaccgaacttaccgaggaaacgagcagaaccgccgaactgcgacaggatcctgtctacggcagctatcagcataaagaacatcatgatgtacatgatgatttcgttaattcccatcgcctttactccctgttagttgttatttattggcggatgcggcgtaaacgccttatccgccctacatgtgcaatcccgtaggctggataagacgcggcaagcgtcgcatccggcaattgcaccgcgccactggcggatgcggcgtgaacgccttatccgccctacatgtgcaatcccgtaggctggataagatgcggcaagcgtcgcatccggcatttattgcgccgctgcgtacaggccgacaatctgctccaggctggcggtacgcgggttactgcgcagacaaatatcttccagcgcggcctgcgcccatgcgccgtaatgcgcagatgtcgcaccaacatcgcccagtcgtttaccaatcccaacttccgcaatcagctcacttaccgcgttaatagcgtcacgatcgtcggattttttagttcgcagtgcccgaccaatctgactaaagcgttcacgacaaaccatccggttaaattccatcaccgttggcagcaacatggcgttcgcgagaccgtgcggaatatgcagcgccgcgcccggctgatgcgccatcgcgtggcacaacccaagacccgcactggaaaacgccattcccgccatacatgaagccagcaacatgctctcgcgcgcggcaaggtcgtgaccgtagcccaccgctttcggcagcgatttgccaatcatcgcaatggcaccaatcgccagactgtcggtaaacggtgtagcgttcagggcgctgtatgcttcaatggcatgggttaacgcatcaatgccggtcatcgccgtgacatgcgacggcacaccttcggtcaatgcggcgtcgaggatcgccacatccggcatcagcgaggcatgggctaacacctgcttgcgcccgctcaccgcgtcgataatcaccgttacattggtggtttcagagccggttccggcggtagttggaatggcaatcagcggcaagcgcggttgcagaacgctggtttctgacatctctgccagcgtgctatccgggttcgtcaccagcaacgtcacggctttcgccgcatccagcaccgagccgccgccaaacgcgatcaccccatcacagcctgactcacgcaactgcgccacggctgcacacacgtcggtaatgcacggttcgcccaccggacatggccagagcgtcatggcgatacctttaacggtcaggctacgcgtcagcccggcggtcatccctgcctgatgcaaaaagctgtctgccatcacgaacagatgtttcagcccacgcgtttgcgcttgctgtccgcaactgctcaccgagcccggaccgcaaagcgtcaccggtggaacgctaaatgtttttacccgttgcagattcagggtatcgaacgcctgaaagagcgcggtctgcaattcattttgcatatagcccctccgctttctctcgcccactactggcgatcgccagcggggtcataaacaaactgtgctgcggtaaatgcacctgtaacgccgggaattgtttgcgaaacagttccgccacgcccggttgcatacaagagccgcccgccagccataaatcagtaatgccctgcccttcaatatgccgggcgacaatgtccgccattttttcgtacaccggtttcaccgcaggccaaatctcttcaccgtgaccgcgcttgtactgctccgcctcttccagcgaaatacggcgatttccggcgagagtcagagagatgtgatgtccgccggtggcttcatccgccgagtacgtcaccttgccctttttcacgatggcaatgccggtagtgccgccgccgatatccactacaccggcgttgtccagttgcagcagatccgcaactgcggttggctcatccagcacatggctcacttccagtccggcagattccagcacgttgatggaaatacgcgggtccgtacctggaggaaatgaagtcgccgcatggctaaaacgacgaccgaattgctgctcgagcgtgtcgagatggcgacgaacaatggtgacagcgccgaagaaatcccagacgatgccgtcgcgaaccacatcggcccagtcgaggcataccgccactggctgaccgtcgcggtcgacaaccatcgacaccacatcgcaggtgcccagatccacccccagccacagcggagattccgtcgcggcgggcgtctggttacacagcgttgccgccgtttgcagacgtggggtgagccattgttcgtcgtgcgccatctgttactccttaaacaatgcgaaacgcatcgactaatacacagcgacgcagacggacaaacgtacgcgcgctggttaccccttcaccggttggcgtggtgatggtcatggtggtccagccttccccgcccagccccagcccggcaatgcacggtccgttcttaacgaaaatgctggtatcaatagcattcgccatctggttcatgttttcgatgttgcgcgagtgcattgccgccgtgtggtggcaaccgccttccagtttcaccgctagcgcaatggcatccgccacgttggcgacgcgcacgacgggcaacaccggcatcatcagttcagtcacggcaaacggatgttctgcggtggtttccacaaacagcaggcgcgtttcttgcggaactttaaggccgattgccgccgcgattttgcctgcgtcgcgaccaacccagtcacggctgacggtgccttttccgcgctcgtcgatatttttcagcaacaccggttgcagctgctgcgcctgttctgcggtcagtttcaccgcgtgctggccttccatcagacgcatcagttcatcggctacgctatcaacaacaatcagtaccttttcgtcggcacaaatgatgttgttatcgaaagaagcgcctttgacgatggactgagcggcacgggcgaggtcggcggtttcatccaccactaccggcgggttgccagcgcctgcggcaatcagacgtttattggtgtgtttacgcgccgcttctactaccgcttcgccgccggttaccaccagcaggccgatacccggaaacttgaacaagcgttgcgcggtttcgatatccggatttgccacagtaaccagtaagttttccggcccacctgcggcaacaatcgcctggttgagcagcgtaatcgcccgctgggagacttttttcgccgccggatgcggggcaaaaatgacgctgttgcccgcggcaatcaggctgatggcgttgttaattacggttgccgccgggttagtggaaggcgtcaccgaagccaccacgccccagggtgcgttttcaattagggtcaggccgttgtcgccagtcagcacttgcggagagaggcactcaacgcctggtgtgccgcgcgcctgagcgacgttttttgcaaatttatcttcaacgcgccccatgccggtttcactgacggcaagttccgctaaatctctggcgtgtttttcgcctgcttcacgaatggcagcaatggctaactggcgcattgccacgctttttaacccttgctgggcgactttggctgccgcaacggcgtcatccagggacgcgaaaacgcccatctcatgaacggcggcggacggcgtgtcactgctttgcattttcagcagtaccgctttcaccacctgttcaatatcctgttgattcatgatgttctgccttatttgtggaaaattacctgaccgccagacaccacctcatcgacaatgccaatcacgcacagatcgaccggtgacgtttcgcttttatgcgcctggcgggcggaactgccactcaccagtaacacccactccccggttcccgcgccaatattgtcgatggcgacggcgcattgcccgtcaggattaccttgtggatcaatcatttccaccatcagcaatttgtcatgcgccagtccgtgatggcgtacggtacaaacaatttgtccagtgacgactgccagtttcatacccgcctccgtggcgtatttcaggtaaaagctccccctaccctccgcagaaggtaaaatgaaaaaggagagagcgtgacgcccgaatcgacgtcacacagggtgattacaggttgctgctatcgcctttcaggccgatcgggaagacttcttccaggtcgccgtgcggacgcgggataacgtgtacagataccagctcgccgatacgctgtgccgctgcggcacctgcatcggtcgcggctttacaggctgcaacatcaccacgaaccatggcagtacacaggccgccgccaatctgcttaacaccaaccagcttgacgcgcgcagctttcaccatcgcgtcagaagcctcaatcagtgcaaccaggccccgggtttcgatcattcctaatgcttccattgtgctttcctctttatcagggtccagaacgggaccgttcattcaaccagtgtttgtaaactgctttcgcggttcacttctgtctgacgcggcacagctgccaccagcgccagctcgataatttcctgcacgctacaaccacgagagagatcgtgcatcggcgcggcaagtccttgtatcagtggcccgacggcacgatatccgccgagtcgttgtgcgattttgtaaccaatatttccggcttccagcgacggaaaaaccatcacattggccttgccctgtagcgggctggcaggcgctttttgcgccgccacttccggcacgaaggcggcgtcaaactgtaactcgccatccaccaccagctttggtgcgcgctcacggacgatttctgtcgcctgctggacgttagcaacacaggggtgacgggcgctaccattgctggaaaacgacagcatcgccacgcgcggctcttctccggtgatggcgcgccaggtttcggcactggcaagcgcgatatccgccagctgcgccgccgtcggctgtggcaccacgctgcaatcggcaaagcccaacgccgggccgctgtactgtggcaacatcaggaaaatggaagagagcgttttacagcctggctgcaagccgataatgcgtaatccggcacgcagcacatttgccgtggaagagaggttgcccgcgatacagacatccgctttaccggcgctgaccattgctgcggcgaacatcagagggtcggtaagtttttccagcgcatccggcggcgttttttcgcccgcgcgggccagccagcgatgagcaaattcttcccgcattgcgaggttgccatgcggatcaatcacctgtagcccgtccatcgccacgccgtgactgagcgcaaactgacgaagttcaaacggattggcgaccagaatgggcgttgccagaccttgttgatgtaaatattgcgcggctttcagcacacgttggtctaacgcatccggaaaaaccactctggcgggcgctcgcaacgccagttcacgacaacgttcaataatcattgcgtttcccccagtcgttgttggatctgcttcaccgttagcggctgcttcgttacgctcaggatcatcatcacgtagaccgtgctcgaaaggcggttcagcgcctgcaaaatgtccgggcgtaatacttcaaagctgcgggtgataaagacctgcgccgctacggtttcggtttcccgcactttggtgcgtagcagattgagcaacgcagcatcgcgcccgtggctggcttccggcaccagatgatcgtggtcgagatagcgcagcggctgatgagaaagccgatgcagatcttcgtcagaaagcccgacaatcgcctggcagcccagcggttcccccagcgcatcggcgcgcataatgttgccaagacgcgaacggatatccgccagccacggctgccacggttccgccagttcaatttgcagccacactgccagcgcaatggtgctgtcgagaaccgcgcgaaaacccagacgcggatcgcttttggcgaccattttttccgccgacaggtgagtcagcgtatccggcttttttgccaccggctggcgacacagttcgcagcacgcctgcggatgttcatcgctactggtcagcccatgaacgggctgcggctgctgctgttcatcgtcaacaaacaggcggccctgctcgtcaataaacttgatgcgcagatggcggctttccagcaactcccgggcagagggcgtcaggcgactgtccgcagggagatggatctctgcgccttcgctgagcgtatggttcgctcttagccatgcttcggtgatgaaatctttcatagggattgccagttagccggccaggcgacatacaggaatttcacgctggatgtcgtaccaaattcgatgctggagcctttcgggataaacatcacgtcgcctgctttggcgatcatggtttggccttcgtggcgaacatgcagctccccttccagcaccatgtcgatttcgtcgtagttcagggtccacgggaagaatgcgttctcccactgcataaaaccggcggccatgctgctgccgtcgtctccggtcacaagatcagtcaagcccacgcaatgcggctctgcgccgtcgaaacgaccaaacttgacgctactgccatcaatcactttgatgccgcctttgccggtcaccgatttgaagctcggctgcattgcgccctgctccagcgactgtttttccttcatcactttttccatcagctgtgcgaccaggctttcggtaaactggccttccggcagctgggcaatgatggtttcgcggatgcgctggctttcggttttgtcggctggcacgctggcgggcacggacgccgttaccgggatcgattcatcacattcggtgatggtaaaacccagtagatccgccacttcacgggcttccggggtaataatgctggcgcgcagaaccacggacattgcctgttcgccgcgcgcgtgtgcttcacgaatatcattcgctgtgatgagttttttcacctgcttcctcctgtttggtgagagatgccagataatccaccagttgctgcacgctttgcgggtcgtggctgtttagctcgaacatcggctcttcgaaacccgtctcaagcaataactttcgcgttgcggcgacgtcagcatctggcatgtccgttttactgatgacggcgatttgccgtttgctgacgccaatatccagcaacccggcaggcaaccgactttccgggtcatttgcgccatggacatagatcagcatgtctacatcctgtagcgtggtaattaaggcgtgataccagcggggatggttaaaatattcacccggcgtatcaatatcgcccttatcattaaattccacggcctgtgtttttctggcgagggtataattcccctgcaacgcattaaataacgttgtttttcctgccccgacgctacccacaaacgcaattcgtttcatgaatgcctcgtattaacttttggtcatttcacaaagcgtataatttaataagcgacctaaaccgctgacggtttgtgataacgcttcttctactgcgcccaccgagccataaatcaccaatgcaccgctgaatcggtcgagaaaaccgatatgcacatcagcggctttcagcgctaaatcaccggcgatcatcgccgtttcgccgggagttagcgtcataatgccaattgcgcccgcatccggaacgccgattttcttcgccagttcctcaccgggatgcgcgatgagatgcgccagtgtgacctgtttgccgggcacaaattcctgaatgatgcgttctttatccatgagtcgccgcctgtgaaaaactttcgtgtatcgtgacaatttttcgtcagagtaaataacaaaattcggcaagcgcgtttaaaaggtgaggtagatcactaagaatggagagatattcgctgtggtgcataaactttcatatgcaacgcatgaatataaataaaataatatcgagatattatatagactgcttttttttattattcgcaaactcagtaataagctttactaatatattgcagctaaactgcttaccctgaatattcagggtaagcgtgagagttaaaaaaaattacagcggttgggtttgcgcttctaccacggccagcgccaccatgttgacgatacgacgcaccgatgcgatcggcgttaacacgtgaaccggtttcgccacacccatcagcaccgggccgacagtcacaccttccgagctggaaacacgcagtaagttgtaactaatgcgggcagcttccatgttcggcatcaccagaatattggcggaacctttcaaagagctgtccggcatacggtcgttgcgaatcgcttccaccagcgctgcatcgccgtgcatttcaccatcaatcatcagttctggtgcacgttccctgaccagttccagcgcctgacgcattttgctcgacgacgggcagtcagaagaaccaaagttggagtgcgacaacaaagcaacgcgcggctcaataccaaaacgacggacagtttctgccgccatcaaggtgatctccgccagctcttctgcatccggttcatcattaacatatgtatcggcaataaaggtgttaccactcggcagcagcagcgcgttcatggcacctgcggtgtgaacgccatcgcgataaccaaagacatttttcaccacgctaaaatgttcatgataatcacccaccgtaccgcaaatcattgcatcggcttccccacgctgaaccatgatcgcgccgatcactgtcgggttactgatcagcgcccgctgcgcctgttcctgagtgacgccgcgacgcttcatgatctggaagtattcggtccagtactctttaaagcgcggatcggattcgttattgacgatctcaaaatcaacgcccgctttgatctgcaagcccagtttctgaatgcgcatttcgatcacgttcggacgaccgataaggatcggtttcgccagtcccagcgttaccagttcctgagtggcatgcagaacgcgcgcctcttccccttccggcagaacaacgcgcttcggcgctttgcgagcctgggagaaaatcggcttcataaacaggttggttttgtaaacgaactcagtcagcttgtcgatgtagacgtcgaaatcagcaatcggacgagtcgccacgcccgactccatcgcggctttagcgaccgcaggagcgatcttaacgatcaagcgcggatcaaacggttttggaatgatgtattccggaccaaagctcagatcctgatcgccatacgctgaagccaccacttcgctctgttccgcatgggcgagttctgcaatcgcacgtaccgccgccagtttcatctcttcgttgatggcggttgcgccaacgtccagcgcgccacggaagatgaacgggaagcacaggacgttgttcacctggttcggatagtcagaacgaccggtgcaaatgatggcatccggacgcacttctttcgccagcggcggcagaatttccggttccgggttcgccagcgccaggatcattggcgcacgagccattttcttcaccatttcctgggtcagcactttcgggccggaacagcccaggaaaatatccgcgccttcaatcacatcatcgagggtacgtttgccgtcatccaccaccgcatatgcggctttggtttccgccatgtttggctcacggccctgatagataacgccttttgaatcgcaaaccacgatgttatgtttttgcagacccagcgctaccagcaggttcatacaggcgattgctgcggcacccgcgccggaaaccaccatccgcacgtcggagatgtttttctccaccacgcgcaagccgttgaggatggcggcagtgctgataattgccgtgccgtgctgatcgtcgtggaataccggaatattcatccgctcgcgcagtttctgttcaatatagaaacattctggcgctttaatgtcttcgaggttgatgccgccgaaggttggttcgagcgcggcgacaacttcaataaatttgtccgggtcgagttcgtcaacttcaatgtcaaatacatcaatcccggcgaatttcttaaacagaacgcccttgccttccatcaccggtttgcctgccagcgcgccaatgttgcctaaccccagcaccgccgtaccgttagagatcaccgccaccaggttacctcgggcggtatatttgtaggcttttaacgggtctttttcgatttcaagacaaggtgcggcaacgcctggtgagtaggccagcgccagatcgcgctgtgttgccagaggcttggttggagaaacctggattttccctggaactggaaattcatggaaatcaagtgcactttgttttaactggtcatccatttggttgttcctttcacgtaacgttcacaaataaagtgtgtgggcaacagcccctgcccacaacgtggcgcacattattaccctgccggagtctacagactttgagcaagtccaaactctcaccattaatataatgttttggtaataatcctataacactgatgttacctgcttaatccagcaataccatgcctgtctgctatgcttttttgatgcgtttagcgaaatttctcagaagtgtgaattaacgcactcatctaacactttacttttcaaggagtatttcctatgaacgagttagacggcatcaaacagttcaccactgtcgtggcagacagcggcgatattgagtccattcgccattatcatccccaggatgccaccaccaatccttcgctgttactcaaagctgccggattatcacaatatgagcatttaatagacgatgctatcgcctggggtaaaaaaaatggcaagacccaggaacaacaggtggtcgcagcgtgtgacaaactggcggtcaatttcggtgctgaaatcctcaaaatcgtacccggtcgcgtgtcaacagaagttgatgcacgcctctcttttgataaagaaaagagtattgagaaggcgcgccatctggtggacttgtatcagcaacaaggcgttgagaaatcacgcattctgatcaagctggcttcgacctgggaaggaattcgcgcggcagaagagctggaaaaagaaggtattaactgcaacctgacgctgctgttttcttttgcacaggcacgggcctgtgcggaagcaggcgtttttctgatttcgccgtttgtcgggcgtatttatgactggtatcaggcacgcaagccgatggacccgtatgtggtggaagaagatccgggcgttaaatcggtgcgcaatatctacgactactataagcaacaccactatgaaaccattgtgatgggcgcgagcttccgtcgcaccgaacaaatcctcgccttaaccggctgcgatcgactgactatcgcaccgaatttactgaaggagctgcaggaaaaagtttcgccagtggtacgtaaattaatcccaccttctcagacgttcccacgcccagctcccatgagcgaagcggagttccgttgggagcacaatcaggatgcgatggcggtagaaaaactgtctgaaggcattcgtctgttcgccgttgatcaacgcaaactggaagatcttcttgccgccaaactataaaccagccacggagtgttatatgtcccgaaaagaccttgccaatgcgattcgcgcactcagtatggatgcggtacaaaaagccaactctggtcatcccggcgcgccgatgggcatggctgatattgccgaagtgctgtggaacgattttcttaaacataaccctaccgacccaacctggtatgatcgcgaccgctttattctttccaacggtcacgcgtcgatgctgctctacagtttgctacatctgaccggttacgacctgccgctggaagaactgaagaacttccgtcagttgcattcgaaaaccccaggccacccggagattggctatacgccaggcgttgaaaccaccaccggcccgcttggacaaggtttggcgaacgccgtcgggctggcgatagcagagcgtacactggcggcgcagtttaaccagccagaccatgagatcgtcgatcacttcacctatgtgtttatgggcgacggctgcctgatggaaggtatttcccacgaagtctgttcgctggcaggcacgctgggactgggcaagctgattggtttttacgatcacaacggtatttccatcgacggtgaaacagaaggctggtttaccgacgatacggcaaaacgttttgaagcctatcactggcatgtgatccatgaaatcgacggtcacgatccgcaggcggtgaaggaagcgatccttgaagcgcaaagcgtgaaagataagccgtcgctgattatctgccgtacggtgattggctttggttcgccgaataaagcaggtaaggaagaggcgcacggcgcaccactgggggaagaagaagtggcgctggcacggcaaaaactgggctggcaccatccgccatttgagatccctaaagagatttatcacgcctgggatgcccgtgaaaaaggcgaaaaagcgcagcagagctggaatgagaagtttgccgcctataaaaaggctcatccgcaactggcagaagagtttacccgacggatgagcggtggtttaccgaaggactgggagaaaacgactcagaaatatatcaatgagttacaggcaaatccggcgaaaatcgctacccgtaaggcttcgcaaaatacgcttaacgcttacgggccgatgctgcctgagttgctcggcggttcggcggatctggctcccagcaacctgaccatctggaaaggttctgtttcgctgaaggaagatccagcgggcaactacattcactacggggtgcgtgaatttggcatgaccgctatcgccaacggcatcgcgcaccacggcggctttgtgccgtataccgcgacgttcctgatgtttgttgaatacgcccgtaacgccgcgcggatggcggcactgatgaaagcgcggcagattatggtttatacccacgactcaattggcctgggcgaagatggtccgacgcaccaggctgttgagcaactggccagcctgcgcttaacgccaaatttcagcacctggcgaccgtgcgatcaggtggaagcggcggtgggctggaagctggcggttgagcgccacaacggaccgacggcactgatcctctcaaggcagaatctggcccaggtggaacgtacgccggatcaggttaaagagattgctcgtggcggttatgtgctgaaagacagcggcggtaagccagatattattctgattgccaccggttcagagatggaaattaccctgcaagcggcagagaaattagcaggagaaggtcgcaatgtacgcgtagtttccctgccctcgaccgatattttcgacgcccaggatgaggaatatcgggagtcggtgttgccttctaacgttgcggctcgcgtggcggtggaagcaggtattgccgattactggtacaagtatgttggtctgaaaggggcaattgtcgggatgacgggttacggggaatctgctccggcggataagctgttcccgttctttggctttaccgccgagaatattgtggcaaaagcgcataaggtgctgggagtgaaaggtgcctgatggtgattgccggatgctgattgccggatgcgacgctgacgcgtcttatccggcctacagcgtcttatccggcctacatgtcccgccattttgtttaacgggtgatccacaacgtgggccaggcgtctggcccatgccagttatcgcaggtgggttctgcggcgtaacgcaccaggcgaaaacgctgaccgtcaaagcgccagcgcgcctgaatgccacaatcgcttaatccgcgccctttcgctaaggtcaccagttcacgcgatttctcatcaaatgttgcgttcatcagttccagttcattcgtctcctgaccgttgttgaacggcaaacgcaaccgaaccgggcgcgaagctagtggctttttacgcgacacaatccatgccaaatcaatggtgttataggcccctgcctcacagctaatcatcatcagcgctttatcatcagtcagcgcagtgacattcacctcacgacgcaatggatcaagcgagcagcgcagaccattcatccgccagtttccataatccagcaaatcgttgcgttcttcgagtgagagtggcgtcggcgttgggttaaccaccgcgacctctttcagcgcaggcgcgggcggtacgctgagcggcggttcgtcccctttcttgatccacgcggtttcactgccaacgcgcttttgctgagcatcaataaacaacaacgctgcttttaagccactcagagaaatggtctgatcgccatcgcgtaaggtgattgccttcccttcctgaatcatctgcaaaaacgcggtgatggttgccgtatcatcggttactaataaccatggtgaaatccgccacttgtcaccacttaacgccaacggctcgccatctaacagcagccgtggcgctatctccccttctgacgcctccggcgacttcaatccgccgcgctcaatacgtaaaacggcatcggtatgcgccccggcgctgcggctcagggtcatcaccagtccattatgatcgcccgtattacgcgccacgcagaaattttggttattacaggtgacctgccagtcggaaaacgcccgttgcgctggtgccgcccacaccaaagacgtcggcaacaaagcgaaaaaaaagagaaggaaaatgcgatagcgcatggacggtacgaccccagaagttcaaacaaacagcacaagtcgtatcttcgttgcgcaggtagcgcggctcaatcggatttgtcggattgagccaataataaacaacgaaatattattgttatttttcagtccattaaatgtgacgtttgcaaatagttaagcaataacaccgtcttaccgtcacgtatctcgccggttttgatcatctccagcgcctggctgaacggcagctcgagcacttcaatatcttcatcttcgacaccgccaccggcgttagcgcgctgattgtcactgtattcggcgataaaaaagtggattagctcagtcacaccgcctggcgacatatacagttcaaataatttgcgcacttcacccacttcatagcccgtctcttcaatcgcttctttgcgaatacacacttccggttcgtcgttatccagcagcccggcgcagctttcaatcagctgcccgctttcattgccattaacccaggtagcgacacggaactgacgaatcagaaccacggtctttttcttcgtgttgtacaggaggatcgtcgcaccattgccgcgatcgtacacttcacgtttatggcggataacttcgccgtctttgcgcgtgagatcgtaagtaatgttgtgcagggtgaaatagttatcggagagaattttgtctttaatgagggtgatttgttgcgtcataccgactccacagcgcgaaatgaacaattatcttacgctgtgaagtcgggtttgtctgcgcaggctatcagtgagatttgactgattttacccccagccagtcaataatcccctgtgccgcatgacgtccttctgccattgcggtaaccaccagatccgcaccacgcacggcgtcaccaccagcgaagattttcggattggtggtctggtaacggtactggctttccacatccgcgatgatgcggccccatttgtctaccgttacaccgtgcgactccagccacggcatcccgtgcggattgaagccaaacgccataatcaccgcgtcggctggcatgacaaattcactgccttccaccggcactggacgccgacgcccctgggcatccggctctccaagacgcgtgcgcaggaaacgaatcccgcagacgtgaccttgttcattcagctcaagcgccaccggctggacgttaaattcgaagttggccccctcttcgcgggcgttcttcacttctttcttcgagcctggcatgttagcttcatcacgacgataagcgcaggtgacgttactcgcgccgtggcgcagtgcggtacgcacacagtccatcgcggtgtcgccgccgcccagtaccacgacgttaagtccggcggtattgataaacggctcttccggtagctcttcgagccccatcacctgtttagtgttggcaatgaggaacggcagcgcgtcataaacgcccggcgcatcttcattgggtaaacccgctttcatggaacggtaagtgcctacgccaacgaagaccgcgtcgtattgttccaaaagcgaatccaaagagacatctttacccacttcacaattgagttcgaagtgaatccccatcgcgctgaagatttcccgacggcgtgccagcagggatttatccagtttgaaagaaggaatgccgaaagtgagcaagccaccgatttctggatggcgatcgtacaccgtcacccccacgccattgcgggtcagaacatccgcacaggccagccctgccggacctgcaccgataatcgccacccgcttgtccactttggtgacatggcttaagtcaggacgccaacctttcgccaacgcctgatctgaaatgtagcgttcaatgttgccgatagttaccgcgccgtgctcatcgcgaatagtacaggcaccttcacacaaacggtcttgcggacaaacgcgtccggtaatttccggcagggtgttggtctggtgagaaagctcgacggcggcgtcgatgtttccggctttcaccagttcaatccactgcggtatatggttatgcagcgggcaggtccattcacaaacgctgtgctcgccgcacttaaggcagcgcgaggcttcccgttgtgcctggtcggcgcgaaatggcagataaatttcatcaaaaccggttttgcgcgcttcaatcgccagtttatccggctcgccacgcgcgggcgttgcctgcatttgttcgactttactcattaccggcatttcttgcgccgcggtactggcatgccacggttgatgttcctgacgcgcggtgcgcaagcggcgggatttcgccatgccggagagtgcgacgtcagtgaccagttgcagcgcgtccgccgggcaattctcaacacaggcaggaccgttttcgcgccccgcacaaaggtcgcatttatgcgccgtggcttttacttttcctgccgcgacgggtgtcaggacgatttgcatcgtaccaaaaggacaggccaccacgcaggatttacagccaatacacttttgctgattgacctgaatgctgtcatcaacgtggctgattgcgccattagggcagctacgggcgcagggcgcatcttcacaatggtgacaggtcactgcactacgttgctgttgatgtttgataaccgtaattcggggatgaaaatggtgttggctcaggacatgttgctcatcattgtgagccatgacacaggcgatttcacaagcatgacaacccagacattgctgactgttggccataataaaacgattcataacgaccttcttttttggttgtaaaaaccttattctttatatgagtgttgttattacccgacttacaggggaatcggcaatgttcatgtgcccagaataagtaactatttcgctataaactgtggcagatcaaataatcccatcactgactaaattgcgtttcagcgaactggaacattaatgattttttgtggagaagacgcgtgtgattgttaaacgacccgtctcggccagtctggcccgggcctttttttacattgtgctgctgtcgattctttccacgggtatcgctctgctaactctggcgagcagtttgcgcgacgctgaggctatcaatattgccggatcgctgcgtatgcagagttaccgcctgggctacgacttgcaaagtggcagtccacaactcaatgcacatcgccagttatttcagcaggcactgcattcaccggtattaaccaacctcaacgtctggtatgtgccagaagcagtaaaaactcgctatgcgcatctgaatgccaactggctggagatgaataatcggctcagcaagggcgatttgccgtggtatcaggccaatattaataattatgttaatcagatagacctgttcgtactggctttacagcactacgctgaacgcaaaatgctgctggtggtggcgatttccctggctggcggcatcggtattttcacgctggtcttttttactttgcgccgcatacgccatcaggtggttgccccgctgaatcagctggttaccgccagtcagcgtattgaacacgggcagttcgactcgccgccgctggataccaacctgccgaatgagcttggtctgcttgcaaaaacctttaaccagatgtcgagcgagctgcataaattgtaccgttcgctggaagcgtcagtagaagaaaagacccgcgatctccacgaggccaagcgtcgtctggaggtgttgtatcagtgttcgcaggcgctgaacactagccagattgatgtgcattgtttccgccatattttgcagattgttcgcgacaatgaagcggctgaatatctggagttaaatgtcggtgaaaactggcggattagcgaagggcaaccaaacccggaattgccgatgcagattttaccggtgacaatgcaagagacggtttacggcgaactgcactggcaaaatagtcacgtttcatcatcagaaccgctgcttaacagcgtttcgtcgatgctgggacgcggtttgtactttaatcaggcgcagaagcattttcagcaattattgttgatggaagaacgtgcgaccatcgcccgcgaattgcacgactcgctggctcaggtactttcttacttacgtatccagttgacgttactgaagcgttcgataccggaagataacgccaccgcacaaagtatcatggccgatttttcccaggcgttgaatgatgcttatcggcagttacgcgagctgttgactactttccgcctgacgctgcagcaggcggatctcccctccgcattgagggaaatgctggatacgttacaaaatcaaaccagcgccaaactgaccctcgactgccgtctgccaaccctggcactggatgcgcaaatgcaggtgcatttgttgcaaattattcgcgaagcggtgctgaatgcgatgaagcacgccaacgccagcgaaatcgccgtcagttgcgtcaccgcgccggacggcaatcacacggtttatatccgtgataacgggattggtatcggtgaaccgaaagaacccgaaggtcattatggtctgaatatcatgcgcgaacgcgcggaacggctaggtgggacgctgactttttcacaaccttccggcggcggcacgttagtgagtattagctttcgctctgcggagggtgaggaaagtcagttaatgtaatgcctcctactgaccaaagaatacttgcacttaaggttcagtataaaagggcatgataatttacattaactcctttttttctccacgattggctcgtaccttgccgctacagtgaagcaagtcaagcctacaacgatacgcagaaacacgaggtcctcttttaatggcgaatttctttattgatcgccccatttttgcctgggtgctggcaatcctgttgtgtctgacaggtaccctggcgattttttcattgcccgttgaacaataccccgatctcgcgccaccgaatgtgcgagtgaccgctaactatcccggcgcatcggcccagacgctggaaaacaccgtgacccaggttatcgagcaaaatatgaccggcctcgataatctcatgtatatgtcatctcagagcagtggcaccggtcaggcatctgtcactttaagttttaaagcaggcaccgatccggacgaagccgtgcagcaagtacaaaaccagctgcaatcagccatgcgaaagttaccgcaggcggtgcaaaatcagggcgtgacggtgcgtaaaaccggcgataccaacattctgaccattgccttcgtctctaccgatggttcgatggataaacaggatattgctgattatgttgccagtaatattcaggacccgttaagccgcgtgaatggcgtcggggatatcgatgcctatggttcgcaatattccatgcgtatctggctggacccggcgaaactcaacagtttccagatgacggctaaagatgtcactgatgccattgagtcacagaacgcgcagattgcggttgggcaacttggtggtacaccttccgtcgataagcaggcgctcaacgccaccattaacgcccagtcactgctgcaaacaccagaacagttccgcgatatcaccttgcgggtcaatcaggacggctcagaggtaaggctgggcgatgtcgccaccgtcgaaatgggggcggagaaatacgattatcttagccgcttcaatggtaagccagcctccgggctgggggtaaaactggcctccggcgctaacgaaatggcgacagcggagctggtgctcaatcgtctcgacgagctggcgcagtatttcccgcatggactggaatacaaggtggcgtatgaaaccacctcgtttgttaaagcctccattgaagacgtggtgaaaacgctgctggaagctatcgctctggttttcctcgttatgtatctgttcctgcaaaacttccgcgccacgctgatacccactatcgccgtgccggtggtgttgatgggaaccttctccgtactttacgccttcggttacagcgtcaacaccttaaccatgttcgcgatggtgctggcgatcggtctgctggtggatgacgccatcgtggtggtggaaaacgtcgaacgtattatgagtgaggaaggactcactcctcgcgaagccacacgtaaatcgatggggcagatccagggggcactggtcgggattgcgatggttctttcggcggtatttgtaccaatggccttcttcggcggcaccaccggtgccatctatcgccagttctctattaccattgttgcggcgatggtgctgtcagtactggtagcgatgatcctcactccggctctgtgtgccacactacttaagccactgaaaaaaggtgagcatcatgggcaaaaaggcttttttgcctggtttaaccagatgtttaaccgcaacgccgaacgctacgaaaaaggggtggcgaaaattctccaccgtagcctgcgctggattgtgatttatgtcctgctgcttggcggcatggtgttcctgttcctgcgtttgccgacgtcgttcttaccgctggaagaccgtggcatgtttactacctcggtacagttgcccagcggttcaacgcaacaacagaccctgaaagtcgttgagcaaatcgagaaatactacttcacccatgaaaaagacaacatcatgtcggtgtttgccaccgttggttctggccctgggggtaacgggcaaaacgtggcgcgaatgtttatccgcctgaaagactggagcgaacgcgacagtaagaccggcacctcgtttgccattatcgagcgtgcaacgaaggcgtttaaccaaattaaagaagctcgcgttatcgccagcagcccgccagcaattagcggtcttggtagttctgcaggttttgatatggagttgcaggaccacgctggagcgggtcacgatgcgctgatggcagcacgtaatcagttgctggcgctggcggcggaaaacccggagctaacccgtgtgcgccataacggcctcgacgacagtccgcagttgcagattgatatcgaccagcgtaaagctcaggcgctgggcgttgctatcgacgatattaacgacacactgcaaaccgcctggggttcgagctatgtgaatgactttatggatcgcggtcgcgtgaagaaagtctatgtgcaggcagctgcgccgtatcgcatgctgccagatgacatcaatctctggtatgtccgaaataaagatggcggcatggtgcccttctctgctttcgcgacctcacgctgggaaacaggctcgccgcgtctggaacgctataacggttattctgcggttgagattgttggggaagccgcaccgggggtcagtaccggtacggcgatggatattatggaatcgttagtgaagcagctgccaaacggctttggtctggagtggacggcgatgtcgtatcaggagcggctttccggcgcgcaggctccggcgctgtacgccatttccttgctggtggtattcctgtgtctggctgcgttgtatgaaagctggtcggtgccgttctcggtaatgctggtcgtgccgctgggggtaatcggcgcgctgctggcaacctggatgcgcgggctggaaaacgacgtttacttccaggtgggcctgttaacggtcattggtttatcggcgaaaaacgccatcctgatcgtcgagtttgctaacgagatgaaccaaaaaggccacgacctgtttgaagcgacgctccacgcctgccgtcagcgtttacgcccgattctgatgacctcgctggcatttatcttcggcgtattgccaatggcaaccagcacgggtgccggttccggtggtcagcatgcggtgggtactggcgtaatgggcgggatgatttcggccactattctggctatttacttcgtgccgctgttctttgtgctggtgcgccgccgcttcccgctgaagccgcgcccggaataagcaataaaaaaggcgacatgccaatgtgtcgcctttttcaactttccgattaagaacctgctcagcgggttcttgctgtttgtactttgtctcaggaattacttacgaagcataacttcgataaagtctttccagttccccagttcacgttcaatcataacaacctctcttataattatgggtattctacggaaacaatataccgtggtgaagctaatttactcgattgctgcgatgactacctccgggggacaaatcttatgtaaatactatggtcctgcggtgatgatttgtatgtgatacacagcaacatttcgagatattcatacggcatctaatactgatttaattctggttaaaatacagacagataacaagatgaatattcttaatgtttacgttaaaaatgtttaatattatttaatagttgttaatttgaatacttcgataatgttatatttcctgataatcatttgcaggcaaaatgttttcacccttaaatgagtatttattctcataaatcgaaaaaggattcattatggttacactttacggtatcaaaaattgtgacaccattaaaaaggctcgccgttggctggaagccaataacatcgactatcgttttcatgattaccgcgtcgatgggctggacagcgaattattgaacgattttatcaacgaattaggctgggaagcgttactcaacacccgtggtacaacctggcgtaaactggacgaaaccacccgcaataaaatcaccgatgcggcctctgcggcggcattaatgactgaaatgcctgcaattatcaaacgtccattgctctgcgtgcccggtaagcctatgctgctgggtttcagtgattccagttatcagcaatttttccatgaggtgtagtctatgtcgtgcccggttattgagctgacacaacagcttattcgccgcccttccctgagtcctgatgatgcaggatgccaggctttgttgattgaacgtttgcaggcgatcggttttaccgttgaacgcatggactttgccgatacgcagaatttttgggcatggcgtgggcagggtgaaacgttagcctttgccgggcataccgacgtggtgccgcctggcgacgccgatcgttggatcaatcccccgtttgaacccaccattcgtgacggcatgttattcgggcgcggtgcggcagatatgaaaggctcgctggcggcgatggtggtggcggcagaacgttttgtcgcacaacatcccaaccatacggggcgactggcatttctgatcacctctgatgaagaagccagtgcccacaacggtacggtaaaagtcgtcgaagcgttaatggcacgtaatgagcgtctcgattactgcctggttggcgaaccgtcgagtatcgaagtggtaggtgatgtggtgaaaaatggtcgtcgcggatcattaacctgcaaccttaccattcatggcgttcaggggcatgttgcctacccacatctggctgacaatccggtacatcgcgcagcacctttccttaatgaattagtggctattgagtgggatcagggcaatgaattcttcccggcgaccagtatgcagattgccaatattcaggcgggaacgggcagtaacaacgttattccgggtgaactgtttgtgcagtttaacttccgcttcagcaccgaactgactgatgagatgatcaaagcgcaggtgcttgccctgcttgaaaaacatcaactgcgctatacggtggattggtggctttccgggcagccatttttgaccgcgcgcggtaaactggtggatgcggtcgttaacgcggttgagcactataatgaaattaaaccgcagctactgaccacaggcggaacgtccgacgggcgctttattgcccgcatgggggcgcaggtggtggaactcgggccggtcaatgccactattcataaaattaatgaatgtgtgaacgctgccgacctgcagctacttgcccgtatgtatcaacgtatcatggaacagctcgtcgcctgatgagtggttctgcaagaggaaataagcatggactggctggctaaatattggtggattctggtgattgtctttttggtaggcgtcctgctgaacgtgattaaagatctcaagcgcgtcgaccataagaaatttctcgccaacaagccggagcttcccccgcatcgtgatttcaacgataagtgggacgatgacgacgactggccgaaaaaggatcaaccgaagaagtaagctgagtgctcaaccgtaggccggataaggcgttaacgccgcatccggcaatggtgaacgatgcctgatgcgacgctcacgcgtcttatcaggccaggtaatctgtcttttacatcatttcaatcacatcatcatcgccaggcttaccgccacttagcgcttcgtcgaaataatgtttcggaatggtataacgcaagtgatccagggcaaattgcatactgcgattgtcgatcgcatggcctaaatcctccacgatatccagcgtcacgtcaccaccggcactgattaacgcttcctgcgccgcaaccgcatgcgccagatcgataaccggatcttcaccgccatgaatcaggtgaattgtcgtggctgtagacgcagtttccggcaggctcgcatagcgtccgttaaaagcaatgacgcgtgaagcaaggcccggttcggctttaatgctctccagcaccataatcgcgccttgagagaaaccgatgagcgccgtggcgttagcccctactccgctctgtttctgccagtagcgcaccgtttcaataaacgtcggcatgatcgcatccacacgcgcctggcgattatcttccgtaataccctgcaccgaaaaccactgacgccccgccggattaccgctcggctccgcgccaccgacactcaccaccagcgcatcaggaaacagcggtgcaaaccagttgcctatttcccccattgccaccgggttatccccgacaccgtggaaaagcagtaacaactgttgcgcaggtttatccgggctttgaacaacaaaatggtcatgtttcatggcgaactccttaactgatgtcattaattttacgccgctgactcacaatgaccatgagataaaattgaaggagtcagtgaaataattgccattgcgttatgcgatcgcgcagacgctcagtgcgaacatcattaagtgcgaacagcgcctgcgcggcctcttcccgctgacggaccagtaacatcttgcggcctgaaagtttaagtgtggtacataactgcgcatcactggcgtttttctgtaaacgcccacgcagcgccggtaatgccagttcactggtttgtaacagacgcaataagcaacctaacgacgttaatagcggacgatgagcgaaagcaaaaccggccagttcaagccagtcgtcgtcagaaaggacggcatcgtttagtggatcaacaggaagcgtttcgccattccactgcgcgagagcttgcgcatcgcgacgtaaacggtaatgctcacgttcagccagctgtttacccgcatcactcatcggtaacagcgccatcgccgtatagcaaccgctgctggcttcccgatgattacccatccgcaccagcacaaaaccgcagcgttgccagaaacgccataactccccggtgtaaccaaaactcaccgaaagatagtcgaggtcttgcgtatattgcaaagcaccagcaataagttgccgccctgtgccttcccgctgacgagccggatgaactgctatccggctgacccgccgtccacgcaatgtcgccgccagtggattgttgccgtgcgccgccagcgactgggccaccagattaccccgcgggcgacgaaaacctgcccataccgcctgactgagttgttgagataatccaccctcatccaccagccacagcgccccggcaatctcgttttcgccagccgcctgtaaaaaatgttgccctggtgcatccatcatccggcgtaaatccagcggcgaagtccgatagtgcgcaccagacaagagctgataaacctttaacggcgtttctggatcgctttgccataacgtctgttcaaatgcggaaatgacaatattgccttgtggtgtatgggtgaagttttcatcgtcaaaaaccagtgcctcgctgaccattttttccagcgggcatccctgcgcccagcggatcggctgttgcagttcaaaacggtgtaaatgcggaaagcgagcgcaaaatttcagcaaaaaaccacgtccggtgccttcgtagccctgcaccgtagtggttaacaacgttcgaggaaaacgcgataccagttgatgcaacaatggcgcaggtatggctgcggcttcatcgaccaccagccagtcggcttgctcatcgctggctaacaaggcatccggcgcaataaagcgaaacttctcgcccgcaaattgtgccagtacatccgttgacgcttttgcgggcgcggtgacaatcgctctgcccgcaatacgagaaatgagttgccctgccaacgccgacttaccgcgcccacgcgcagccgttaccgctgccacgcccggcggcatggtcattagctgctttaagagttgctgttgttctggttgtggtgcgccagtcgcggggtaccagtcagtacggggagtaaaatgcgccaacgagaatggctggttttgccgccagaggatagcctcgttatccgccgtaagtacgcgtttgagatgctggacaaaatgcggcgtcgcaatagggtcagggcaatcactccagcgcagcgagtcggcatcaggttggttttcccactcttcccatacagggagtaacaaaaccagccagcttcccgctttcaacgttccgctaagtgcggcaaaggcagcggcatcaaagccgtggcgggcgtcgaataccgcatgccggaactcgcgcccaagtaaagtttgtagtgccgagggagaacagtggttttcagcatctggccgcggcgaaatccacagccagtcgccaggtaaggcatcacgcaacttaagagtatgctcaaaacaccaaccctcttccccgctcaacaccagcaagcggcggatcccttcacgtttcatttgcgctgttaatgtgtgaagcgcagtcagttcagccatccctgccccggaagttaaatgcttttaccaaaagtattgcattgtgccggatcgccgctgtcgaaaccacgtttaaaccagctgtagcgttgctgagaagtgccatgagtgaaactgtctggtactactcgcccctgactttgctgttgtaaacggtcatcgccgatggcctgcgccgcgttcagcgcctcttccagatcgccggtttccagaacgccttgctgctgcatactatgcccccagacaccggcaaaacagtcggcctggagttccatacgcacagataagcggtttacttccgcctgcgtcgcgttttgttgcagttgacgaactttcggctcgatgcctaacagtttctgcacatgatgaccgacttcatgggcgataacgtacccctgggcaaaatcgccatccgcgccaagtttgtctttcatgtcatcatagaaggagagatcgatataaaccgtgccatccgccgggcaatagaacggccccattatggactggcccgccccgcagccggtacgcgtcattccacggtacatgaccagcttcggttgctgataggtcttacccatcttctcgaactgttgtccccaggtgtcttccgtggttgccagaatcaccgaggtgaattttgcggcttcgtcttcatttgggctaattgaccgcgttgattgttgttgggaaaccggctgcccggtcatcaacccggttaaatcaacaccatagtagcctgcaaccagcacgactatcagtaaaatcagcccgcctttaccgcttggcaggcgaaaaccgggaccgcccatagatggaccaccagagctgttgcgcctgtcttcaacattgtcactttcacgtcgcccttgccaacgcatagatacctcaacaatatattcattatagaaatgatcgtaggtggttcagaggaagattaccacaggaaagcgggatgaaatggcggaggaatgagcgttcaatgcatatattccgagagcggttgtcttgccgtgccagctgcacggcaagatgatgaacagaaaaatcagtccagctgtacacccaggcggcgggcgacggcttcataggcttcgatcaggccaccgaggctctggcggaaacggtctttgtccattttctccagcgtttctttgtcccacaggcggctaccgtccggggagaactcatcacccagtaccacttcgcctttgtacagaccaaattccagcttgaagtcgaccagaatcagaccagcatcatcgaacagttttttcagcacgtcgttcgctttgtaggtcagctctttcatacgcgccaggttctctttgctcacccagccaaaggtttcgcagtaagattcgttgaccatcggatcgtgcatggcgtcgtttttcaggaacagatcgaacagcggcgggttcagctcaataccttcttcgattccaagacgtttcaccagagagccagcagcacggttacgcacgacacactcaaccggcaccatatccagctttttcaccagacattcggtatcggagagcagacgctccatttgagtcgggatacccgcttcagccagtttgctcataatgaagtagttgaacttgttgttcaccatacctttgcgatcaaactgctcaatgcgcgcgccatcccctgctgacgtatcattgcggaattcgagcaccaacaggtccgggttttccgtgctgtatacggttttcgctttaccacgatacaactcagcttgcttttgcatctttatcactcctgggtgtgaattaacgttttaaaatcttttgctgtctggtgtgccggatgttttgtcggatgcggcgtgaacgccttatccgaactacgtccgacaaacaaatttcgtgcgaattaccgctaaaatcgcgttttcctgcagacgcacacgtttgcgtatcatatcagaaaaaagggccggatgattccagccctgtatttttacttgctaaacgcagcctggaagacagctaccagcgcgtcgttctgactctgagtcagagtatgacctttcggatcgatgaactgtaggctgctgcggttatctaaatcgccaacctgcagtttatagtcaccggatgccaggcctggatcgctcgcgcccagttcctgccagtcgctgtcagacagcggcttataagttacggccatgttgccctgcgaacgggtgctgtcggtcactttcatgcccactttttccagcgccgctggcagacgttgccaaaccacattgaacggcccgcgtacgaccagcattggtaaaccggtgtcatcagctgcactttgtacgtccatagtggtggaggcacgattttgcgcagcgttcgcggcgtcagtggcagatttatccagaccggcggaaataacgttcatcatctccgtgctgtaacgctgcatggaagccgcgtctgcaaccggtttgcccgcctgttccaggttcagcagtttaaccgtaaccgcctgctgataaccctgcggcttaacagagatttgataacgaccacgatactgctcgtcttcgtccagacggttccattgtacccaatcggtggtcagtgtctgaccagcatcatcacgttgggtgatggtgtagtttttcgcctgcagcacgctaaccacctgcggccacagagtattgccacgaccattttccaccagcaatgaagcggtatcgcccgtgaactgggtacgcgcgccagaaaccagtgccagcggctgggctggtggacgaatgtccagcgccttaccgacagcaccactaccgttggtcaccgggattgcataatcaccggaggtcaccggcaaaatcattccagccggggcatgaagctccgcaagcggtgccgcttccaggtaggcttcatcaccactgacctgacgcttatagcgtgagtcagaactacaggcagcgagtaataaaacaagcgaaacacccgcaacctttgccaggcgcgacttttgaacagagtaagccatcaaatctccctaaactttacagcaaaccggcatgcttaagcgccgctctgaccgtctcacgaccactgtcggtgattggtgtcattggcaggcgcagcgtatcggtcgccacaagacccagttccttacatgcccatttcaccgggattggattgggttcgacaaatagtttgttgtgtaatggcatcagacgctgattaataacgcgtgcctcggcaaaatgcccttctgctgccagtttgcacatctgggccatatcacgcgctgcgacgttagccgtaacggaaataaccccatgaccgcccaattgcatgaagtccagcgcgctcgcatcatcgccgctcagcagaacaaaatcatctgaaaccagctctttgatctggtttacacgcgttaagttccctgttgcctctttgattccgataatattttttactttcgccagacggcccaccgtttccgggagcagatcgcagccagtacgggacggcacattatacagaatttgcggcaggtcagtatgctcagcgatggctttgaaatgctgatacaaaccttcttgcgacggacgattgtagtaaggggttaccgtcaggcagccgacgataccactgtcattgaagcgctgcgtcaggctaatggcttccgcagtagcgttagcgccggtcccggcaattaccggaatgcgcccatcagccagatccagcgtcatcatcaccacatcagcatgttcgtcatgatttaaggtagcggactcgccagtggtgccaacagaaacgatcgccgaagtaccgctggcgacatgataatcaatcagttttttcaagctagcccgacagacattacctttttcatccatcggagtaacaatcgcgacaatacttcccgtgaacatgggccatcctctgtgcaaacaagtgtctcaatggtacgtttggtatggcattaaaagcaagcagacagaaccgttctgattgttgtatgcatgttttttttatgctttccttaagaacaactcaccccttaaaggaataaccagtttgacactgtcatcgcaacattatctggtgatcactgcgttgggtgccgatcgccctggaattgtgaacaccatcacccgtcatgtcagtagttgcggctgtaatattgaagacagtcgcctggcgatgctgggagaagagttcacgtttattatgctgctttccggttcatggaatgccattactctgattgaatcaacgttaccgttgaaaggtgccgaactggatcttttaatcgtgatgaagcgcacgacggcgcgtccgcgtccgccaatgccagcatctgtctgggttcaggtcgatgtggcagactccccgcatttaattgaacgcttcacagcacttttcgacgcgcatcatatgaacattgcggagctggtgtcgcgcacgcaacctgctgaaaatgaacgggctgcgcagttgcatattcagataaccgcccacagccccgcatctgcggacgcagcaaatattgagcaagcgttcaaagccctatgtacagaactcaatgcacaaggcagtattaacgtcgtcaattattcccaacatgatgaacaggatggagttaagtaatgaatccactgaaagccggtgatatcgcaccgaaatttagcttgccggatcaagacggagaacaagttaatttgaccgacttccagggacagcgtgttctggtttatttctacccgaaagccatgacccccggctgtaccgtacaggcctgcggcttacgcgataacatggatgagttgaaaaaagcgggcgttgatgtgctgggtatcagcaccgataaacccgaaaaactctcccgttttgcggaaaaagagctgcttaactttacgctcctgtctgatgaggaccaccaggtgtgcgaacaattcggcgtctggggtgaaaagtccttcatgggcaaaacctacgatggcattcatcgcatcagcttcctgattgacgctgatggcaaaatcgaacatgtctttgacgatttcaaaaccagcaatcaccacgacgttgtgctgaactggctgaaagaacacgcctgattactttgctccattccgtgctggctgcgcttgcggccagcatacctcacttctcgtgatcaagatcacattctcgctttcccctgcgacacgggtgtcgaatccattttttgctgaacgttaatgaccatcatttttgtaccgttcagaatccagttaatacataacttattgaatatattgagttaatcagaatggcatcctttatgcaatatgaaatgcaatgtttcatatcattttcaaggagccgacatgaaccgctttgtggtggccgaaccactgtggtgtacaggatgtaatacctgtctcgctgcctgttcggacgtgcataaaacgcaaggtttacagcaacacccgcgcctggccctggcgaagacgtcaacaatcactgcccctgtcgtgtgtcatcactgtgaggaagccccttgcctgcaggtctgcccggtcaatgccatctctcagagggatgatgcgatccaactcaacgaaagcctctgtattggctgcaagctttgcgccgtggtctgcccatttggcgcaatcagcgcttcaggaagccgtccggtgaatgcccatgcgcaatatgtttttcaggctgaaggctcactcaaagacggcgaagaaaacgcgccaacacaacatgctttgctgcgctgggaacctggtgtccagaccgtcgcggtgaaatgcgacctgtgtgatttcttgccagaaggtccggcctgcgttcgcgcttgcccgaatcaggcgttacggctgatcaccggtgatagcctgcaacgtcagatgaaagaaaaacagcgccttgccgcaagctggtttgccaatggcggggaggatcccctttccctcactcaggagcaacgctaatggatgccctgcaattattaacctggtcgctgattctctatctgtttgctagtctggcttcgctgtttttactcggtctggacagactggctattaagctttccggcatcacatcgctggtgggcggcgtgattggcatcatcagcggaattacgcaattacatgctggtgtaactttagtcgcccgttttgcccccccttttgaatttgccgatttaaccctgcgaatggatagcctctcggcatttatggtgctggttatctccttgctggtggtggtttgttctctctattcattgacttatatgcgcgaatacgagggcaaaggcgcggcggcgatgggcttctttatgaatattttcatcgcatcgatggttgccctgctggtgatggacaacgctttttggttcatcgtgctgtttgaaatgatgtcgctgtcttcctggtttctggtcattgccaggcaggataaaacgtcgatcaacgctggcatgctctacttttttatcgcccacgccggatcggtgctgataatgatcgccttcttgctgatggggcgcgaaagcggcagcctcgattttgccagtttccgcacgctttcactttctccggggctggcgtcggcggtgttcctgctggcctttttcggttttggcgcgaaagccgggatgatgccgttgcacagctggttgccgcgcgctcaccctgccgcaccatcgcacgcttcggcgttgatgtctggcgtaatggtcaaaataggtattttcggcatcctgaaagtagcgatggatctgctggcgcaaacgggtttgcctctgtggtggggcattctggtgatggcgatcggcgcaatctccgcgctcctgggcgtgctatatgcgctggcggaacaggatatcaaacggctgctggcctggagtaccgtcgaaaacgtcggcattattttgctggcagtcggtgtggcgatggtcggtctgtcactgcacgacccgctgctcaccgtggttggactgctcggcgcactgtttcatctgctcaaccatgcgctgttcaaagggctgctatttctcggcgcgggagcgattatttcgcgtttgcatacccacgacatggaaaaaatgggggcactagcgaaacggatgccgtggacagccgcagcatgcctgattggttgcctcgcgatatcagccattcctccgctgaatggttttatcagcgaatggtacacctggcagtcgctgttctcactaagtcgtgtggaagccgtagcgctacaacttgcgggtcctattgctatggtaatgctggcagtcactggtgggctggcagtaatgtgcttcgtaaaaatgtacggtattactttctgtggtgcgccgcgcagtacacacgctgaagaggcacaggaagtgccaaatacgatgatcgtcgccatgctactgctcgcggcactctgcgtattaattgcgcttagtgccagttggctggcaccgaagataatgcatattgcccatgcgtttaccaatacccctcccgccactgtcgccagcggaatagcacttgtacccggcacgtttcatacacaggtcaccccctcattactgttgctgttactactggcgatgcctttgctgcctggcctttactggctgtggtgtcgttcgcgccgcgcagcgtttcgtcgcacaggagatgcctgggcatgcggctacggctgggaaaatgcgatggccccgtcaggcaatggcgtgatgcagccgctgcgtgtggtcttttctgcgctatttcgtctacgacaacagctcgaccctacgctgaggctaaataaaggtcttgcgcacgtcaccgccagggctcagagcacagaacccttctgggatgagcgggtgatccgccccatcgtgagcgccacccaacggctggccaaagaaatacagcatctgcaaagcggcgactttcgtctctattgcctgtatgtggtcgccgcactggttgtgctgctaatcgctattgccgtctaaggaaatcaccatgagacaaactctttgcgacggatatctggtcatttttgcgttagcacaggccgtgattctgctgatgctaaccccactttttacgggtatttcccggcagatacgcgcgcgtatgcactcccgccgcgggccggggatctggcaggattatcgcgatatccacaaactgtttaaacgccaggaagttgcgccgacatcttcaggtctgatgttccgcctgatgccgtgggtattaatcagcagcatgctggtgctggcgatggccttaccactgtttattaccgtttccccttttgcgggcggcggcgatctgatcacccttatctatcttcttgccctgtttcgttttttctttgctctttccgggctggataccggaagtccgtttgcgggagtcggtgccagtcgcgagttgacgctcggcattctggtcgaaccaatgcttattctctcactgctggtattggcgctgatagcaggttccacgcatatcgagatgatcagcaatacgctggcgatgggctggaactcgccgctaaccaccgtactggcgttactggcctgtggttttgcctgcttcattgagatgggaaaaattccctttgatgttgctgaagcagaacaggaattacaggaaggcccgctgaccgaatattccggtgccgggctggcgctagcgaaatgggggctggggctgaaacaggtcgtgatggcatcactgtttgtggccctgtttctgccctttgggcgcgcgcaagaactttctctcgcctgcctgctgacttcacttgtcgttacgctgctcaaggttttgctgatttttgtactggcctcaatcgcagaaaacacgctggcacgcgggcgttttttactcattcaccatgtgacctggcttggcttcagccttgctgcgcttgcatgggtcttctggttaaccggtctgtaaggagcactgacggaatatggaaaatcttgctctgacgacgttattgctgccttttatcggcgcactggtcgtttcgttttcgccacaacgtcgggccgccgaatggggggttttgttcgccgcgctgaccacgctgtgcatgttgtcactgatctccgcgttttatcaggccgataaagttgccgtcacgttgacgttggtcaacgtgggggatgtggcgttgtttggcctggtcattgatcgcgtgagtacgctgattctgtttgtggtggtgtttctcggtttgctggtcacgatctactccacgggttatctgacggataaaaatcgcgaacacccgcataacggcacgaatcgttattacgcatttttactggtgtttatcggcgcgatggcgggactggtactctcctcgacgctgctcggtcagttgttgttttttgaaattacaggcggctgctcctgggcgttgatcagttattaccagagcgataaagcgcagcgttcagcactaaaagcgttacttatcactcatatcggctcgttggggttgtatcttgccgccgccacgctgtttttgcagaccggaacgtttgcgcttagcgcgatgagcgagttacacggcgacgcacgttatctggtttatggcggcatcctgtttgccgcgtgggggaaatcggcccagctaccgatgcaagcgtggctaccggacgcaatggaagcgccaacaccgatcagcgcctatctccacgccgcatcgatggtgaaagtgggcgtttacatttttgcccgcgctattatcgacggcggcaatatcccgcatgtgattggcggcgttggcatggtcatggcactggtcaccattctttatggctttctgatgtatttgccacagcaggatatgaagcggttgctagcctggtcgaccatcactcaacttggctggatgttcttcggcttgtcgctctccatcttcggctcgcggctggcgctggagggcagcatcgcctacatcgtcaaccacgcgttcgctaaaagcctgtttttccttgtagcaggtgcgctgagttacagctgcggcacgcgcttgttgccgcgtctgcgtggcgtattgcacaccctgccgttgccaggcgtgggtttctgcgtggcagcgctggcgattaccggcgtgccgccgttcaacggcttcttcagtaaattcccgctgtttgctgccggttttgcgttgtcagtggagtactggatcctgctgcccgccatgattcttctgatgattgaatcggtcgccagtttcgcctggtttattcgctggtttggtcgcgttgtgcctggcaaaccgagcgaggccgtcgccgatgccgcaccgctgccaggatcaatgcgcctggtgttgattgtactgattgtgatgtcgctgatttccagcgtaatcgccgcgacctggttgcagtaaggagatgatgaatgaccggttctatgatcgtaaataatctggcgggactgatgatgctgacatcgctgtttgtgattagcgtcaaaagctatcgcctgtcatgcggattttacgcctgccagtcactggtgctggtgtctattttcgccactctctcgtgcctgttcgccgcagagcaactgctgatctggtccgccagcgcctttatcaccaaagtgctgctggtaccgttaatcatgacttacgctgcacgaaatattccccagaacatcccggaaaaagcgttattcggtccggcaatgatggcactgctcgcggcgttaattgtcctgctttgcgcatttgtcgttcagcccgtgaagctaccgatggctaccgggctgaaaccggcgctggcggtagcgttaggtcattttctgcttggcctgctgtgcattgtcagccagcgcaatatcctgcggcaaatttttggttactgcctgatggaaaacggctcccatctggtgctggcgcttcttgcctggcgagcaccggaactggtggaaataggtatcgctaccgacgccatcttcgccgtcattgtgatggtgttactggcaagaaaaatatggcgtacccacggcacgctggacgtgaacaacttgaccgcgctgaagggataatgagatgagttattctgtgatgttcgctttactcctgctcacgccgctgcttttttcgctgctctgttttgcctgccggaaacggagactttctgcgactcgcacggtgaccgtattacatagcttagggatcacactgctgctgattctggcactctgggtggtccaaactgccgctgatgcaggagaaatattcgctgcgggactgtggcttcatattgatggtctgggcggtttgttcctcgccattcttggtgtgattggctttctcaccggtatttactcgattggctacatgcgtcatgaagtggcacacggcgagctttcacccgttacgctgtgcgattactacggtttcttccatctgtttttgttcaccatgctgctggttgttaccagcaataacctgattgtgatgtgggcggcgatcgaagccaccaccttaagctcggcgtttctggtaggcatttacggtcagcgttcatcgctggaagctgcatggaagtacatcattatttgtactgttggtgtcgcttttggtctgttcggtaccgtgctggtatacgccaacgccgccagcgttatgccgcaggcagaaatggcgatattctggagcgaggttcttaagcaatcgtccttgcttgacccaacattaatgctgttggcctttgtgtttttgctaattggctttggtaccaaaaccgggctatttcccatgcacgcctggctgccggatgctcacagtgaagcgccgagtccggtcagcgccctgctctccgccgtattgctgaactgcgcgctgttggtgctgattcgctattacatcattatttgccaagccatcggcagcgatttccccaaccggttgttgctcatcttcggcatgttgtcggttgccgtggcggcatttttcattctggtacagcgggacattaagcgtctgctggcgtactccagcgtggagaacatggggctggtcgcggtggagctaggcattggcgggccgctgggaatttttgccgcgctgctgcacatcttaaaccacagtctggcaaaaacgctgctgttctgcggttccggcaatgtactgctcaagtacggcacgcgcgatctcaacgtcgtctgtgggatgctcaaaatcatgccatttaccgccgtgctgtttggcggcggtgcgctggcgctggcagggatgccgcccttcaacatttttcttagcgaatttatgaccattaccgccggactggcacgtaatcacctgctgattatcgtcctgctgttattgctgttaacgctggtgctggcgggcctggtacggatggctgcgcgggtgttaatggcgaaaccgccgcaggccgttaaccggggtgatctcggctggttgaccacctcgccaatggtgattctgctggtcatgatgctggcgatgggaacgcatattccacaacctgtcatcaggatcctggcgggcgcttccactatagtcctctcagggacgcacgatctgcctgcacaacgtagcacctggcatgattttttgccttcaggcaccgcatctgtttcggagaaacacagtgaacgttaattcatcgtcaaatcgtggcgaagcgattctcgccgccctgaaaacgcagttccccggcgcggtgctggatgaagagcgacaaacgcctgaacaggtcaccattacggtgaaaatcaatctgctgcctgacgttgtacagtatctttattatcaacatgatggctggcttccggtcctgtttggcaacgacgagcggacacttaacggtcattacgcggtttattatgccctttcaatggaaggggccgaaaaatgctggattgtggtgaaggcgctggtcgatgccgacagtcgggagtttccgtcagtcacaccgcgcgtccctgccgcggtctggggcgagcgagaaattcgcgatatgtacgggctgattccggttggcctgccggatcagcgtcgcctggtgttgcccgatgactggccggaagatatgcatccgctgcgcaaagatgcgatggattatcgactgcgccctgaaccgacgactgattccgaaacgtatccgtttatcaatgagggcaacagcgatgcgcgggtgatccctgtcggcccgctgcatatcacctccgatgaaccgggtcacttccgcttgtttgtggatggcgagcaaattgtcgatgctgattaccgcctgttttatgtccatcgcggcatggagaaactggcagaaacgcggatgggctacaacgaagtgaccttcttatcggaccgcgtgtgtgggatttgcggttttgcccacagtgtggcctataccaattcggttgaaaatgcactggggattgaggtgccgcaacgagcacatactattcgctcgattctgctggaagtcgaacggctacacagtcatttgcttaaccttggcctctcctgccatttcgttggttttgataccggctttatgcaatttttccgcgtgcgggaaaagtcgatgacgatggcggaattgctgatcgggtcgcgtaaaacctacggtctgaatctgattggtggtgttcgccgcgatattctcaaagagcaacgtctgcaaacgctgaaactggtgcgcgagatgcgcgccgacgtgtcggagctggtagagatgctgcttgctacgccgaatatggaacaacgcactcagggcattggcattctcgaccgacaaatcgcccgtgatttgcgctttgatcacccctacgccgactacggcaatattccaaaaacactgtttacctttaccggcggcgatgttttctcccgcgtgatggtccgtgtcaaagagacgtttgattcgctggcaatgctggaatttgccctcgacaacatgccggataccccactgctgaccgaaggctttagctataaacctcacgcattcgcgctgggctttgttgaagcgccacgcggtgaagacgtgcactggagcatgctcggtgataaccaaaaattgttccgctggcgctgccgtgccgccacctacgccaactggccggtgttgcgttacatgctgcgcggcaataccgtttctgacgcaccgctgattatcggtagccttgatccctgctactcctgtaccgaccgtgtgacgctggtagatgtgcgcaagcgccagtcaaaaaccgtgccgtataaagagatcgaacgctacggcattgatcgtaaccgttcgccgctgaagtaaggacagaagatgctgaagttactgaaaactattatgcgcgccggaaccgcgacggtgaaatatcccttcgcgccactggaggtcagccctggctttcgcggaaaaccggacctgatgcccagccaatgtattgcctgcggtgcctgcgcctgtgcttgtccggcaaatgcgctgactatccagaccgacgaccagcaaaattcgcgcacctggcagctctatctggggcgttgtatttactgcggacgttgtgaagaagtgtgcccgaccagagccatccagcttaccaataactttgaactgaccgtcaccaataaagccgatctctatacccgcgcgacgttccatctacaacgttgcagccgttgcgaacgcccgtttgccccgcaaaaaaccatcgcactggctgctgaattgttagcacagcaacaaaatgcgccacaaaaccgcgaaatgttgtgggcgcaagcgagcgtctgcccggaatgcaaacaacgcgcgacgctgatcaacgacgatacagatgtactgctggtggctaaggagcagctatgagtccagtgcttacacaacatgtcagccagcccatcacgctggacgagcaaacgcaaaagatgaagcggcatttgctacaggatatccgtcgctcggcttacgtttatcgcgtcgattgcggcggctgcaacgcctgtgaaatcgaaatttttgctgccattacaccagtattcgacgcagaacgttttggcattaaggttgtttcatcaccgcgtcacgccgatattttgttatttactggcgcagtcacccgggcgatgcgtatgcctgcacttcgggcgtatgagtctgcccccgatcataaaatttgtgtttcctacggcgcgtgcggtgtcggcggcggtattttccacgatctctacagcgtctggggcggtagcgacaccattgtccccattgatgtttggatccccggctgcccgccaacaccggccgccaccattcacggtttcgccgtggcgctcggtttgctgcaacagaagattcacgctgtggattatcgcgatcccaccggggtgactatgcaaccgttgtggccgcagatcccgccatcacagcgtatcgccattgagcgagaagcgcggcggctggcgggctatcgtcaggggcgagaaatttgcgatcggctcctgcgccatttaagcgacgatcctacaggaaatcgggttaacacctggttgcgcgatgccgacgatccacgtctcaatagtatcgttcagcaactctttcgcgtactccgggggttacatgactgaagagtgcggggaaattgttttctggacgctgcgaaaaaagtttgtcgccagtagcgacgagatgccggaacacagctctcaggtaatgtattactcgctagctatcggccatcacgttggcgtgattgattgtctgaatgtcgccttccgctgcccactgacggaatacgaagattggcttgcactggtcgaagaggagcaagcccgacgtaagatgctgggggtgatgacttttggtgagattgttattgacgccagccacaccgccctgttgacccgggcattcgcgccactggcggatgacgcgacgtctgtgtggcaggcgcgtagcattcaattcattcatctgttggatgaaattgtgcaggaaccggccatctatctgatggccagaaaaattgcgtgagaaggatttctcattaataaggactgttgatggctatgtcagacgaggcgatgtttgccccgccacaaggaataacaattgaagcggtaaacggaatgctcgcggagcggttagcacagaaacacggcaaggcgtctttattacgcgccttcatcccgctgccgccgccgttcagcccggtacaacttattgaactgcatgttctcaaaagcaacttctattaccgctaccatgatgatggcagcgatgtgacggcaacaacagagtatcagggcgagatggtcgattattcgcgtcacgccgtccttctcggcagtagtggaatggcggagctacgctttattcgcacccacggcagtcgttttacttcccaggattgcacactgtttaactggctggcgcggataatcaccccggttctgcaatcatggctcaatgatgaagaacagcaggtggcgctgcgtttgctggagaaagatcgcgatcatcatcgggtactggttgatattactaatgcagtgctgtcacatcttgatctcgacgatctgatcgctgacgtcgctcgtgagatccatcattttttcggtctggcttcagtcagtatggtactgggcgatcatcgaaagaacgagaagttcagcctgtggtgcagcgatctttctgcctcacattgtgcgtgtctgccacgctgtatgcctggcgaaagtgtattgctgacacaaacgctacaaacccgacaaccgaccttgacgcaccgtgcagatgatctgtttctctggcaacgcgacccgttattactcttacttgcatctaacggctgcgaatctgcgctccttataccgcttacctttggcaaccatacaccgggtgcattgttgctggcgcatacctcttccactctctttagtgaggaaaactgccagctactacaacacatagccgatcgcatcgctattgccgttggcaatgccgatgcctggcgtagcatgaccgatttgcaggaaagtttgcagcaagaaaaccaccagcttagcgagcagctcctttcgaatctgggcatcggtgacattatctatcaaagccaggcaatggaagacctgctccagcaggtagatattgtggcgaagagcgacagtacggtgttgatttgtggtgaaaccggaactggcaaagaggtgatcgccagagcgatccatcaacttagcccgcgacgcgacaagccgctggtcaaaatcaactgcgctgccatccccgccagtcttctggaaagtgagttattcggtcatgacaaaggggcgtttactggtgcgattaatacccatcgtggtcgttttgaaattgccgatggcggcacgttgtttctcgatgaaattggcgatctgccgttagaacttcagcctaaactgctgcgcgtattgcaggagcgggagattgagcgtctcggcgggagtagaacgatcccggtgaatgtcagagtcattgccgccaccaaccgtgatttgtggcaaatggttgaagatcgccagtttcgcagcgatctcttttatcgcctgaatgtcttcccactggaattgccgccgctacgcgaccgtccggaagatatccctcttttagcaaaacatttcacgcaaaaaatggcgcgccatatgaatcgcgcaattgacgccatcccgaccgaggcactacgccagttgatgtcgtgggattggccgggcaacgtgcgcgagctggaaaacgtgattgagcgggcggtactgttgactcgtggtaacagtctgaatttacatctaaatgtccgacaaagccgtttactgccgacgctaaatgaagattcagcgcttcgcagttcaatggcgcagttactgcacccgacgacgccagagaatgacgaagaagaacgtcagcgcattgttcaggtattgcgagaaaccaatggcattgttgccgggccccgtggcgcagcgacgcgattagggatgaagcgcaccacgctgctgtcacgaatgcagcggctggggatctcggttcgcgaggtgttgtaatctgcttttgcaggagtatgcatgagaaacaaactctctttcgacttgcagttgagcgccagaaaagcggcaatcgctgaacggattgccgcccataaaattgcccgcagtaaagtgtcggtctttttaatggcgatgtccgctggcgtgtttatggcgatcggatttactttttacctttccgttatcgccgatgccccgtcttcacaggcattaacccatctggtgggcggcctttgctttacactcggctttattttgctggcggtttgcggcaccagcctgttcacctcgtcggtaatgacggtgatggcaaaaagtcggggcgttattagttggcgaacttggctgattaacgcacttctggtggcctgcggtaatctggcaggtattgcctgtttcagtttgttaatctggttttccgggctggtgatgagtgaaaacgcgatgtggggagtcgcggttttacactgcgccgagggcaaaatgcatcatacatttactgaatctgtcagcctcggcattatgtgcaatctgatggtttgcctggcgctgtggatgagttattgcgggcgttcgttatgcgacaaaatcgtcgccatgattttgcccatcaccctgtttgtcgccagtggctttgagcactgtatcgccaatttgtttgtgattccgttcgccattgccattcgccatttcgcccctccccccttctggcagctggcgcacagtagcgcagacaattttccggcactgacggtcagccattttattaccgccaatctgctcccggtgatgctgggtaatattatcggcggtgcggtgctggtgagtatgtgttatcgggctatttatttacgtcaggaaccctgaaaaatcagcccggcgaaacagttcgtcgggctgaagattattcttgcgcgatttgcccatcgggccaggcatgaatcacggctttgatcagcgtcgccaacggaatggcgaagaatacgccccagaatccccacaaaccaccgaagatcaccaccgataaaataatcaccagcggatgcaggttaaccgcttcggagaacaacaccggcactaacaggttgccgtccagcgcctgaataatcagatacaccgcgaagcagctccagaattcagtacctgcgccaaactggaatagcgccacgccaaccaccggaatggtcaccacaaatgcgccaatgtacggaataagaaccgagaagccgaccagcactgccagcagcagcgaatagttcagcccgaagagcaagaaccccagccaggtggcgatccccaccacgatcatctccagcactttgccgcggatatagttggtgatttgttgattcatctccttccacacctgtcctgccagcccacggttacgcggcagcacccggcgaacggcgttcagcatctgctctttgtctttcagcaggaagaagaccatcaatggcaccagcaccagatagacggctatggtcagcaaaccgaccagcgaggcgagggaaattttcaccaccgaatcgcccatggtcagcatccgactgcgcatattttcggccattgcatcaataatgcccgcgtccattaacgccggatagcggcgcggcaacgtggcggcaaagtcagaaagcttattgagcatccccggcatatcgcggattaagtagatgccctgttgccaggcgataggcagtaccacgaacgccatcagtagcaatataccgacgaaaaccaccaatacaatcgacgtcgcccagcggcgggagcagccaatagattgcagacgcacggttggccattccagcaaataggccagcacaatagccaccagcaacggagcaagcaggccactaaagaaaaagataatgccaaatccggcaactaaaataaccagcaaggcaatcgcttccgggtcgctaaaacggcggcgataccattgcatcaacatttcgagcataaagaccttccctgaacctcaagagcgggattgcgatccgcaattgtatcgaaatgtcacaaaaaagacttcgctttttatgacggattcaggaaactgaaaagtcatttgagtgggctaatcttcgccgttacactcaaaggcggcgcggtgggaacgatatttcacagtatcggtcaaatgactatctccagaaatacaggatagaggttatgttcaggcagttgaaaaaaaacctggttgcaaccctcattgctgctatgaccattggtcaggtagccccggcgtttgccgacagcgcagacaccttgccggatatgggaacctccgcaggaagcacgctttccattggtcaggaaatgcagatgggcgactattatgtccgccagctacgcggcagcgcgccgttaattaatgacccgctgttaacgcaatatattaattcgctggggatgcgtctggtttcgcatgccaattcggttaagacaccgtttcatttttttctgatcaacaacgacgaaattaacgcctttgctttctttggcggcaacgtggtgctgcactctgccctgttccgttattccgataacgaaagtcaactggcttcagttatggcgcacgaaatctcccacgtcacccaacgtcacctggcgcgagcgatggaagatcagcagcgcagcgcgccgctgacctgggtcggcgcgttaggttctattttactggcgatggccagtccgcaggcggggatggcggcgctgaccggtacactggcgggaacgcgtcaggggatgatcagtttcacccagcaaaatgaacaggaagcggaccgcattggtattcaggtgctgcaacgctcgggattcgatccgcaggcgatgccaaccttcctcgaaaaattactcgatcaggcgcgttactcctcgcgcccgccggaaattttattgactcacccgttgccggaaagtcgtctggcagatgcccgcaaccgtgctaatcagatgcgcccgatggtggtgcagtcgtcggaagatttctatctggcgaaagcgcgcacactggggatgtataattccggacgtaaccagctcaccagtgatttgctggatgaatgggcgaaaggaaacgttcgtcagcaacgagcagcacaatatggtcgtgctttacaggcgatggaagccaataaatacgacgaggcgcgtaaaacgctgcaaccgttactggcggcagaacctggcaacgcatggtatctcgatctggctactgatatcgatcttgggcaaaacaaagccaatgaggcgatcaatcgtctgaaaaatgcccgcgatttacgcaccaatccggtgttgcagctcaacctggcgaacgcttatttgcaaggcggtcaaccacaagaagcggccaatattctgaatcgctacacctttaataataaagatgacagcaacggctgggatttgctggcacaggcggaagccgcgctaaataaccgcgatcaggagctggctgcgcgagcagaaggttatgcgctcgccggacgactcgatcaggccatttcgctgttgagtagcgccagttcgcaggtgaaattaggcagcctgcaacaagcgcgttacgatgcgcgcatcgaccagttgcgccagctgcaggaacgctttaagccttataccaagatgtaattcgcattaaaggaagaacaatgaccaaacaggtaaaaatctaccataacccacgctgttcaaagagccgggaaacgctgaacctgctgaaagaaaacggcgtggagccagaagtggtgctctaccttgagacacccgccgatgcggcaacgctgcgcgatttgctgaaaatactggggatgaatagcgcccgtgaattgatgcgccagaaagaggatctttataaagaactgaacctggctgacagttcgcttagcgaagaggcgctgattcaggcaatggtggataatccgaagctgatggagcgcccgattgtggtcgcgaatggcaaagcgcggattggtcgtccaccggagcaggtactggaaatcgtgggttaagatgtgctccatcgctagttgaagcacattgccggatgcgacgcttgccacgtcttatccggcctacgaatactatggattaacttcgcgtagttcggataaggcgttcgcgccgcatccgacaataaacaccttatctacaacttcagaatttctttcacaaacggaatggtcagcttacgttgcgcggtaatcgacgcacgatccaactgatccaacgtcataaatagcgtgcgcatttctctgtcgagccgcttcagcaagaaacgccccacatcttccggcagttcaaaaccacgcaaacgcgcgcgtaactgtagcgcctgcaacttatcttcatcagaaagtggctgcaatttgtagatctgcccccagtcgagtcgcgacgcgagatccggtaatcccagattcaactgccgcggtggacgatcgccggtgatcaacaaccgtgttttgcccgattccagaattcgattgtagagatcgaaaatcgccatctcccacaactcatcgcctgcaatacactcaatgttgtcgatacagaccagcgacaaatgctccataccgtcgagcacttccggaacaaaccaggtgcgtttatccagcgggacatagcccaccgcatcgccacgctgcgacaattccgcgcaagccgcgtgcagcagatggctgcgccccgcgccttcgcgtgcccagagatagatgtaaccgctatgttcctgacgcagcacgttttgcagcgcggccagtaaagaggagttatcccccggccagaaacttgcaaaggtttcgtcgtcaggaagataaagtggcaaagagagctgtgccggtgtgttcagagatacctcaaccaggatttcacaaaatcgcgagaagtttaccacagaatcccatgatgtttgaaccgggcagcaacactgcccggtcggtacattatttgtctgttatatccgcgtcttctgcgtccagcaccacttcttcagggcgcagcacactgatcagtttgaagatcaaacttaagccgataccgacgatggtcgccagcgccataccttttaactccgccgcgccgatgtttaccttcgcgccactgacgccgatgatcaaaatcacggaagtcaggatcaggttctgtgctttgttgtaatccactttcgattcgatcaaaacacgaataccggaagcaccgatgacaccataaagcagcagcgaaacgccgcccatcaccggcaatgggatcatctggatagcggcagccagtttaccgacgcaggaaagcaggatagcgaaaatcgccgccccgccgataacccaggtactgtaaacacgggtgatcgccatcacgccaatgttttctccgtaagtagtatttggcgtagagccaaagaagccggaaatcacggtcgacaagccattagcaaacatcgaacggtgcagacctggatcgcgcagcagatcttttttgacgatattagccgttactaccaggtgccctacgtgttcggcaataaccactaacgccgctggcagaatagtcagaatggcaaaccactcgaagcgcggcgtatagagggttggcagcgcaaaccagtgagcattaataatcggcgtggtatcgacaattcccattgcgaaagagagcgcgtaccccaccagcacgccaattaaaatcgggataattgccaggaaaccacgaaacagcacggaacctaaaaccgtgaccgccagggtggtaatagagatgatgatggttttggagtctggcgtttgcccttcagccgggagtaaacccgccataccggcagctacgcccgccagctccagaccgatgacggcaacgattgcgcccattgccgcaggtggaaacagcacgtccagccagccggtccccgctttcttcacgataaaagaaaccaggcagaacagcacgccgcacataataaagccgcccagcgcgacttcataccctaacggcaacagtaacaataccggtgaaataaaggcaaagctggaaccaagataagccggaattttccctttacagatgaagagatacagcagcgttccaataccgttaaataacagtacagtcgccgggttaatatgaaataagacgggcaccaggacggttgcaccaaacatggcgaacaaatgttgcaaactaagcgggattgtctgtaaaagtggcggtctttcactcaccccgatagcacggcgcgtcatagtattatcctctgtattatgtgttataggcgctttactcaaaaaaaagccgactcttaaagtcggctttaattatttttattctttatttcgtaccaaagattttgtcaccggcatcgccgaggcccggaataatgtatccgtgctcgttcagtccctgatcaatcgatgcggtatacagttcgacgtccgggtgcgctttttccagcgcagcgataccttctggcgcagctaccagcaccagaactttgatgctgctgcagcccgcttttttcagcaggtcgatggtcgcgataacggaaccaccggttgccagcattgggtcaacgatcagcgccatacgctcatcgatgttagaaaccagtttctggaagtacggtaccggctccagcgtttcttcattacggtacataccgacaacgctgatgcgcgcgctcggaacgttttccagcacaccgtccatcataccaagacccgcacgcagaattggcacaacggtaattttcttacctttgatctggtcgatttctaccgggccgttccagccttcgatagttactttttccgtttcgaggtcggcggtcgcttcgtaagtcagcaggctacccacttcggaagcgagttcgcgaaagcgcttggtgctgatatcttgctcacgcatcagtcccagcttgtgtttgacgagtgggtgtttgacttccacgatcttcatactctttctcctttgaggggcagccacaaaaaaaatcgacggattatacctcctttcttcaaggcggcaatattcttttcgttgactttagtcaaaatgataacggtttgagataaagttattttatattcagatggttatgaaagaagattattccatccgaaaactaacctttaccctggcacaagtcttctttcgccgcgcgcctggggaaaagacgtgcaaaaaggttgtgtaaagcagtctcgcaaacgtttgctttccctgttagaattgcgccgaattttatttttctaccgcaagtaacgcgtggggacccaagcagtgaccgataaaacctctcttagctacaaagatgccggtgttgatattgacgcgggtaatgctctggttggaagaatcaaaggcgtagtgaagaaaacgcgtcgtccggaagtgatgggcggtctgggcggcttcggtgcgctgtgtgcattgccgcaaaaatatcgtgaacccgtgctggtttctggcactgacggcgtaggtaccaagctgcgtctggcaatggacttaaaacgtcacgacaccattggtattgatctggtcgccatgtgcgttaatgacctggtggtgcaaggtgcagagccgctgtttttcctcgactattacgcaaccggaaaactggatgttgataccgcttcagcggtgatcagcggcattgcggaaggttgtctgcaatcaggctgttcactggtgggtggcgaaacggcagaaatgccggggatgtatcacggtgaggattacgatgtcgcgggtttctgcgttggcgtggtagaaaaatcagaaatcatcgacggctctaaagtcagcgacggcgatgtgctgattgcactcggttccagcggtccacactcgaacggctattcgctggtgcgcaaaattcttgaagtcagcggttgtgatccgcaaaccaccgaacttgatggtaagccattagccgatcatctgctggcaccgacccgcatttacgtgaagtcagtgctggagttgattgaaaaggtcgatgtgcatgccattgcgcacctgaccggcggcggcttctgggaaaacattccgcgcgtattgccagataatactcaggcagtgattgatgaatcttcctggcagtggccggaagtgttcaactggctgcaaacggcaggtaacgttgagcaccatgaaatgtatcgcaccttcaactgcggcgtcgggatgattattgccctgcctgctccggaagtggacaaagccctcgccctgctcaatgccaacggtgaaaacgcgtggaaaatcggtatcatcaaagcctctgattccgaacaacgcgtggttatcgaataatgaatattgtggtgcttatttccggcaacggaagtaatttacaggcaattattgacgcctgtaaaaccaacaaaattaaaggcaccgtacgggcagttttcagcaataaggccgacgcgttcggccttgaacgcgcccgccaggcgggtattgcaacgcatacgctcatcgccagcgcgtttgacagtcgtgaagcctatgaccgggagttgattcatgaaatcgacatgtacgcacccgatgtggtcgtgctggctggttttatgcgcattctcagcccggcgtttgtctcccactatgccgggcgtttgctgaacattcacccttctctgctgccgaaatatcccggattacacacccatcgtcaggcgctggaaaatggcgatgaagagcacggtacatcggtgcatttcgtcaccgatgaactggacggtggcccggttattttacaggcgaaagtcccggtatttgctggtgattcggaagatgacatcaccgcccgcgtgcaaacccaggaacacgccatttatccactggtgattagctggtttgccgatggtcgtctgaaaatgcacgaaaacgccgcgtggctggatggtcaacgtctgccgccgcagggctacgctgccgacgagtaatacccccgtaattaaagcgccagctctgccgctggcgtttttcaattcacctgtaaatcgcaagctccagcagtttttttcccccttttctggcatagttggacatctgccaatattgctcgccataatatccaggcagtgtcccgtgaataaaacggagtaaaagtggtaatgggtcaggaaaagctatacatcgaaaaagagctcagttggttatcgttcaatgaacgcgtgcttcaggaagcggcggacaaatctaacccgctgattgaaaggatgcgtttcctggggatctattccaataaccttgatgagttctataaagtccgcttcgctgaactgaagcgacgcatcattattagcgaagaacaaggctccaactctcattcccgccatttactgggcaaaattcagtcccgggtgctgaaagccgatcaggaattcgacggcctctacaacgagctattgctggagatggcgcgcaaccagatcttcctgattaatgaacgccagctctccgtcaatcaacaaaactggctgcgtcattattttaagcagtatctgcgtcagcacattacgccgattttaatcaatcctgacactgacttagtgcagttcctgaaagatgattacacctatctggcggtggaaattatccgtggcgataccatccgttacgcgctgctggagatcccatcagataaagtgccgcgctttgtgaatttaccgccagaagcgccgcgtcgacgcaagccgatgattcttctggataacattctgcgttactgccttgatgatattttcaaaggcttctttgattatgacgcgctgaatgcctattcaatgaagatgacccgcgatgccgaatacgatttagtgcatgagatggaagccagcctgatggagttgatgtcttccagtctcaagcagcgtttaactgctgagccggtgcgttttgtttatcagcgcgatatgcccaatgcgctggttgaagtgttacgcgaaaaactgactatttcccgctacgactccatcgtccccggcggtcgttatcataattttaaagactttattaatttccccaatgtcggcaaagccaatctggtgaacaaaccactgccgcgtttacgccatatttggtttgataaagcccagttccgcaatggttttgatgccattcgcgaacgcgatgtgttgctctattatccttatcacacctttgagcatgtgctggaactgctgcgtcaggcttcgttcgacccgagcgtactggcgattaaaattaacatttaccgcgtggcgaaagattcacgcatcatcgactcgatgatccacgccgcacataacggtaagaaagtcaccgtggtggttgagttacaggcgcgtttcgacgaagaagccaacattcactgggcgaagcgcctgaccgaagcaggcgtgcacgttatcttctctgcgccggggctgaaaattcacgccaaactgttcctgatttcacgtaaagaaaacggtgaagtggtgcgttatgcacacatcgggaccgggaactttaacgaaaaaaccgcgcgtctttatactgactattcgttgctgaccgccgatgcgcgcatcaccaacgaagtacggcgggtatttaactttattgaaaacccataccgtccggtgacatttgattatttaatggtatcgccgcaaaactcccgccgcctattgtatgaaatggtggaccgcgagatcgccaacgcgcagcaagggctgcccagtggtatcaccctgaagctaaataaccttgtcgataaaggcctggttgatcgtctgtatgcggcctccagctccggcgtaccggttaatctgctggttcgcggaatgtgttcgctgatccccaatctggaaggcattagcgacaacattcgtgccatcagtattgttgaccgttaccttgaacatgaccgggtttatatttttgaaaatggcggcgataaaaaggtctacctttcttccgccgactggatgacgcgcaatattgattatcgtattgaagtggcgacgccgctgctcgatccgcgcctgaagcagcgggtactggacatcatcgacatattgttcagcgatacggtcaaagcacgttatatcgataaagaactcagtaatcgctacgttccccgcggcaatcgccgcaaagtacgggcgcagttggcgatttatgactacatcaaatcactcgaacaacctgaataaccctatgccaatacacgataaatcccctcgtccgcaggagtttgctgcggtcgatcttggttcaaacagttttcacatggtcatagcccgtgtggtagatggtgccatgcagattattggccgcctgaaacagcgggtgcatctggcggacggcctggggccagataatatgttgagtgaagaggcaatgacgcgcggtttaaactgtctgtcgctgtttgccgaacggctacaagggttttctcctgccagcgtctgtatagttggtacccatacgctgcgtcaggcgctgaacgccactgactttctgaaacgcgcggaaaaggtcattccctacccgattgaaattatttccggtaatgaagaagcccgtctgatttttatgggcgtggaacatacccaaccggaaaaaggtcgcaaactggttattgatattggcggcggatctacggaactggtgattggtgaaaatttcgaacctattctcgttgaaagccgccggatgggttgtgtcagctttgcccagctttattttcctggcggggtcatcaataaagagaattttcagcgcgctcgcatggcggcagcacaaaaactggaaactttaacctggcaattccgtattcagggctggaacgttgcaatgggcgcttccggtaccataaaagccgcccatgaagtgttaatggaaatgggcgagaaagacgggataattaccccggaacgtctggaaaaactggtaaaagaagttttacgtcaccgtaatttcgcatcgctgagtttaccgggtctttccgaagagcggaaaacagtcttcgttccgggactggcgattttatgcggtgtgtttgatgctttagccatccgtgaactgcgcctttctgacggggcgttacgcgaaggcgtactgtatgaaatggaaggacgtttccgtcatcaggatgtgcgtagtcgcaccgccagcagcctcgccaaccagtatcacatcgacagcgaacaggcccgacgggtgctggataccactatgcaaatgtacgaacagtggcgggaacagcaaccgaagctggcgcatccgcaactggaggcgctactgcgatgggccgccatgctgcatgaggtcgggttgaatatcaaccacagcggtttgcatcgccactccgcttatattctgcaaaacagtgacttgccgggttttaatcaggaacagcagctgatgatggcgacactggtgcgctatcaccgtaaagcgattaagctcgacgatctaccgcgctttaccttgtttaagaagaaacagttcctgccactgatacagctattgcgccttggcgtattactcaacaatcaacgtcaggcaaccaccacaccgccaacattgacgctgattactgatgacagtcactggacactgcgtttcccgcatgactggtttagtcagaatgcgctggtactgcttgatctggaaaaggagcaagaatactgggaaggcgtggctggctggcggttgaaaattgaagaagaaagtacaccagaaatcgccgcttaatactttgcgggccgacgagaaatgtcggcccgcattattcaggcactttcgcgaatgggttcgatttcattcagcgtatcaattaacggctgcggcttaccaataagataaccctgcatataatcgatccccaaagagagcaccgcctcgcggatctcttcgttttcaacgtactctgccactaccagcattttcttcattcgcgccaggtggcaaatcgatgccactatctgataatccagactatttgacacaatattgcggataaaactgccgtcaattttaagcagatcggcattcacatttttaagccgcgcatagctggcgtagccggtgccgaaatcatcaatcgcaatctggcagcctaattcctgaagatgctgcaaggtgatttgcgcctgcttaacattggtcagagcattactttcggtgacttcaaaaataagttgccacgcttcaatctgatatttagccagcaactgactgacttcaacaggaaaacgagcctgacataccgaggttggagacagattaatagcaaaacggtgagcgggcatcttcgctctgttttcagccataaattgcagcgtatgctcaatgacccacatgtcgatactcgacgataaaccaaattcgtgcgcgaccggcaagaagctatcggggctgatcagttcatcattctcacctttcatgcgcagaagaatttcatggtaaacatcaccacgcataccggtaatcggctgggccatcaggaaaaaatggttgtgttccagcgcctgctgtagtcgattcatcatcgcgactttatctttcaattcgcgttgcaaatacattgccccgcgacgctgcatattttccggggcgttggtcacgatggaaagttcggcgaccgtatttagctctcccagcagcaggtagatatgattcactggcgagcgcacatagcagtaactgacgccaatctgcggttgcatcggcatgccatcccaaaagaaacgaaattgcttgagatggctatccagtgcggtaatgcgctcctggtgcgattctgtattcagtcgcagcgcgagatcgttacccgaaagctgataaacatcttcacccggttccagcaagggtgacagccagtgagaaagtttttgcttgtattgaatccgcagcatgatgccatagttcttaaccagcatttccatgccagggatgcgtaaataacaaagcgcagaccagggggcatcacgcaacgcgcgattcagggcgcgaacatttggcagatgaaccaccgggtccacatacgcaagccgctgaatgcgtctgactaccgctctctgacgggttgccagtacagccatataattgacaataaaagagaataccagataactggaggaggttatggtcagctgcgtggtatagccaggataaatgggaatgtaattttgatagctgtggatgctgatcatcaacacgaccgcccagagcagcgaaatcagcttataaccatagcgcatcgctccccacatcatcaggggcagcaataatgacaaggtataattggtgctaaaaattgtgcttttttcatttaacggcatgcataacagcaacaataaagcacctaatgccagtagccagagcgcgaactcttttttggtgactttggcatcaacctgctgttttaattgcgaataatagctacgtaaataaaatggatttcgcactacccgaatgatgaagtagcacagcgggacaccgatcagattacccaccagtaaggcctgataattgattaaagtcccgaggttaaaaggcatgacaccgaccagattttctctgctcgccagtaatcctacaaatgcagcaaactggaaaagtatcagaaacagcgttgcaggaaacacaatctgccagaatatacgctgggaaattaaacgggtatcaccatgtgaaacgttgttacgccggggagtaaagaccctgtaaccgccccaacagagaatgataatgataataaaattagccgttaatgatagcgtttcgtaaaaacccagctctgcatatttgcggacaaaaatccctaaggcgatccctggcaatgccgcccagctgaaaaacatcatcatgctgatcatcagtgccagaggcagataaaagagaaaaacctcaccggaagaaatatgcgcgaaagtattaatgtgggcgaaaatgggcaagattaaagaaggcaggaacagcggaagcccccaccatttatcacgtatttttatataagttgcattcagtttcatagatgctcagcagaatcccccacatcctgaaggaggtgtattcagacaggcatcccacctgacttcgaatgatgattattcatcactatagagagcattgattctaagtgtcatatgaaagtaccaattgatatatatcaaacaaaataaccctgattaatgaattattacgtttatcatgttaattcatcattattacatcatcattgtaaataattaaattaacttccataacattaaaatatgtatccactgacgcttttttacataacgaagaattgaccattttgtcctgttgtgccttaatgtaagtaccgtccacagcgtgggacatacttcaaggaaccttttgtgagtcaggcaaccagtatgcgaaaacgacaccgatttaacagtcgcatgacccgtatcgtactgctcatcagctttatcttcttctttggccgttttatctactcgtccgtcggtgcctggcagcaccatcagagcaaaaaagaagctcagcaatccacactctccgtcgaatcaccggtacaacgttagcggttaccttctccactttcacagaacataacggcacttcgctgtcggatgcttttgctgtttgggattatcaaagcggcagatattctttcatcttaaattttacgtctttatcctgactgatgtttatcctgtttggctgcgaaataaatataaaattaatatatatgttgtaatgatatatttttataaattattccctgcgtgaattttaataaatttaatctatccctttatacgcaatacatttactttcctcttttgatgatcttaaatgtcttatttttcgtaatgtgtataacaaggaatagtgatgaaatttaaaaaatgtcttctgcctgtggcaatgttagcgtcattcactctggcaggatgccagtcaaatgctgacgatcatgctgccgatgtttatcaaaccgatcaactgaataccaaacaagaaactaaaaccgttaatattatttccattcttcccgcaaaagttgccgtagacaactcccaaaataaacggaacgcacaagccttcggcgcgcttattggcgcagtcgctggcggtgttatcggccacaacgtcgggtctggcagcaattccggaacgacggcaggtgcagttggcggcggagctgtaggcgcggcagcgggttctatggtgaatgataaaaccttagtggaaggtgtttctttaacctataaggaaggcaccaaagtgtatacctctacccaggtgggtaaagagtgccagtttacgacaggtttagccgttgttattaccacgacgtataacgaaacgcgtattcagccaaataccaaatgtcctgaaaagagctaataatcaggaggagtcatgaagaaagtttttctttgcgccatcttagcctccttaagctatccggctatcgcctcatcattgcaggatcaactctctgctgtcgcagaagcggaacagcaaggtaaaaatgaagagcaaaggcagcatgacgaatgggtcgcggagcgcaacagggaaatccagcaagagaagcaacgtcgcgcaaatgcccaggccgccgctaacaaaagagcggcaacggcagcggcaaataagaaagctcgtcaggataaactggacgccgaagcctctgcggacaaaaaacgcgatcaaagttatgaagatgagctacgcagcttagagattcagaaacaaaaactggcgctggcgaaagaagaagcccgcgttaagcgagaaaacgaatttatcgatcaggaactgaagcacaaagctgcgcaaaccgatgtggtgcaatctgaagctgacgccaacagaaatatgactgaaggcggtcgcgatctgatgaaaagcgtgggcaaagcagaagagaacaaatcggacagctggtttaattaatcgatgttagtaacttcaatcctataattcttgaagataaaaaaccctctgtagtaacagagggttttgttcattcatagtgcagggtcaaatcattcccactcaatggtagctggcggcttgccgctgatgtcatacaccacgcgggaaataccgttcacttcattgataatgcggttggaaacgcgaccgaggaaatcgtacggcagatgcgcccagtgtgcggtcataaagtcgatggtttcgacagcacgcagagagacaacccagtcatacttacgaccatcgcccattacgccaacggaacgtaccggcaggaacacagtgaacgcctggctgactttgtcgtacaggtccgctttacgcagttcttcaatgaagatggcgtcagcacggcgcagcaggtcacagtactctttcttcacttcacccagaacacgaacgccaaggcctggtcccgggaacgggtgacggtacagcatgtcgtacggcaggcccagctccagaccaatcttacgcacttcgtctttgaacagctctttcagcggttcaaccaggcccatcttcatctctttcggcaggccgcccacgttgtggtgagatttgatgacgtgtgctttaccggttgcagacgccgcagattcgataacgtcagggtagatggtgccctgcgccagccacttcacgtcttccagtttcagcgcttcttcatcgaatacttcaacgaaaacgcgaccgatgattttacgttttgcttccggatcgttttcgccagccagcgctgacaggaagcgatcttctgccggtacgtgaacaatgttaagaccaaagtgatcgccaaacatatccagaacctgctctgcttcgttgaggcgcagcaggccgttgtcgacgaatacgcaagtcaggtttttaccgatagcgcggtgcagcagcattgcggttacggaggaatccacaccaccagagaggccgaggatgactttatcgtcgcctacctgctcgcggatgcgagctacagcatcgtcgataattttcgctggcgtccacagggcttcacactggcagatatcacgcacaaaacgctccagcatgcgcataccctggcgggtatgagtcacttccgggtggaactgtacgccatagaagcgtttttcttcgttagccataatggcaaacgggcagctttcggtgctggctacggtgatgaagtcggacggaatagcggtaactttatcgccgtggctcatccagacatcgagcagcggtttaccgtctgcggtcagcgcatcttcgataccgcgaaccagtgcgctgtcgtttacgacttcaacctgcgcgtagccaaattcacgttcgttagaggcttcaacgtgaccgcccaactgcattgccatggtctgcatgccatagcaaacgccgaataccggtacgcctgcttcaaagacatactgcggcgcacgcggactgttttcttcagtagtactttccgggccgccggaaagaataatgccgcttggattgaagtcacgaatttgtgcttctgtcacatcccacgcccacagttcgcagtaaacacccagctcacgcacgcggcgcgcaaccagttgagtgtactgagaaccgaagtccagaatgaggatgcgatgcttatgaatgttttccgtcattgacgcttattccgaggcaagtgaaacagataatataaatcgcccgacatgaagtcgggcgaagagaatcaggagcccagacggtagttcggggactctttagtaatggtcacgtcgtgaacgtggctttcctgaatgcccgcaccgctgatacgtacaaactccgctttagtacgcagttcgtcgatagtaccacagccggtcagacccatacaggagcgcaggccgcccatctgctggtgaatgatctctttcaggcgacctttataggctacgcgaccttcgataccttccggcaccagtttgtcggcagcgttatcgctctggaaataacggtcagaggaacctttggacatcgcgcccagggaacccataccacggtaagatttgtaagaacggccctggtagagttcgatttcacccggagattcttcagtacccgccagcatggaacctaccatcaccgcgcttgcgccagcggcgatagctttggcgatgtcgccggagaagcgaataccgccatcagcgataaccggaataccggtgccttccagggcttctactgcgtcagcaacagcggtaatctgcggaacaccgacgccagtcacgatacgagttgtacagatagagccagggccaatgccgactttaaccgcactgcaaccagcttctgccagagcgcgtgcacctgcagctgttgccacgttgccgccgataatttgcagatccggatatttagcacgggtttcacggatacgttgcagtacaccttctgagtgaccgtgggaggagtcgatcagcagaacgtcaacgcctgcggcaaccagcgcgtcaacacgctcttcgttacccgcacctgcgccaaccgctgcaccaacacgcagacggccttgctcgtctttacaggcgttcggtttacgttccgctttctggaagtctttcacggtgatcatgccgatcaggtggaattcgtcatcaaccaccagcgctttttcaacgcgtttttcgtgcatttttgccagcaccacttcacgggcttcaccttcacgcacggtgaccagacgctctttcggcgtcatgtaaacgctaaccggctggttcaggtcggtaacaaaacgcacgtcacgaccggtgataatacccaccagttcgttttcttcggtaacgaccggatagcccgcaaaaccgttacgctcggtcagttctttcacttcgcgcagcgtcgtggttggcagaacagtctgcggatcagtcaccacaccagattcgtgttttttcacacggcgaacttcttctgcctggcgttcaatggacatgtttttgtggataaagccgataccgccttcctgagccagagcaatagccaggcgcgcttccgttacggtatccattgctgcggaaagcatagggatattcagacgaatagttttcgtcagctgggtgctgaggtcagcagtattcggcagaacggtagagtgagcaggaacgaggagaacgtcgtcaaacgtcagagcttctttagcgatacgtagcatgggcaatatctcgaccagagtggttaataaatattgccgcggcattatacagagcgtaaccgattgcatctacccctttttgcaaaaaatgcttgctatccccgaagggcgggttactatcgactgaataacctgctgatttagaatttgatctcgctcacatgttaccttctcaatcccctgcaatttttaccgttagtcgcctgaatcaaacggttcgtctgctgcttgagcatgagatgggacaggtttggatcagcggcgaaatttctaatttcacgcaaccagcttccggtcactggtactttacactcaaagacgacaccgcccaggtacgctgcgcgatgttccgcaacagcaaccgccgggtgaccttccgcccacagcatgggcaacaagttttagttcgcgccaatattacgctctacgagccgcgcggcgactaccagataatcgttgagagtatgcagccggccggtgaagggctgctgcaacagaagtacgaacagctcaaagcgaagttgcaggctgaaggtttgttcgatcagcaatacaaaaaaccacttccctcccctgcgcattgcgttggtgtgatcacctcaaaaaccggtgctgcgctacatgatattttgcatgtgttaaaacgtcgcgatccttctctgccggtgatcatctaccctgccgccgttcagggcgatgacgcgccggggcaaattgttcgcgccattgaactggcgaatcagcgcaatgagtgcgacgtattgatcgtcgggcgcggcggcggttcgctggaagatttatggagttttaacgacgaacgcgtagcgcgggcgatttttaccagccgcattccggttgtcagcgccgtcgggcatgagacggatgtgaccattgccgattttgttgccgatctgcgtgcgccaacgccgtctgccgccgctgaagtagtgagccgtaatcagcaagagttactgcgccaggtgcaatcgacccgtcaacggctggagatggcgatggattattatctcgccaaccgcacacgtcgctttacgcaaattcatcaccgattacagcaacagcatccgcagctccggctggcacgccagcaaaccatgcttgagcgcctgcaaaagcgaatgagctttgcgctggaaaatcaacttaagcgtaccgggcaacagcagcagcggttaacacagcggctgaatcagcaaaatccacagccgaagattcatcgcgcgcaaacgcgcattcagcaactggaatatcgtttagcagaaaccctgcgcgcacagcttagcgccacgcgtgaacgtttcggtaatgcagtaacgcacctcgaagccgtaagcccactgtcaacgctggcgcgtggatacagcgttactactgctactgacggcaatgtactgaaaaaagtgaagcaagttaaagcgggtgaaatgctaaccacacgtctggaagacggctggatagaaagtgaagtaaaaaacatccagccagtaaaaaaatcgcgtaaaaaggtgcattaagccagcacgaattcaacgcgttttttcgatatcaagccatgcccgtgctgacagaagtaatctactgcaccacaggcttttaacacctgcaacggttgatggcagtctggacaaagagctttcatttcaataaattccccgcaggatcggcaacgcgcatggccgttatcctgatcaagcacatgctgacattgtggacaatgcagttccatatgaattcctccggtagccattccctctacattcatagagggaatggcagataaaatacttacggataattatttatttttcttgatgtgcttcatcagacgcttacgtttacgcatctgggttggcgtcagggtgttacgcttattcgcatacgggttttccccttctttgaactgaatacgaatcggcgatcccattacgtccagcgatttgcggaagtagttcatcaagtagcgcttgtaggaatcaggcaggtctttcacctgattaccgtgaatcaccacaatcggcgggttataaccaccggcgtgggcatatttcagcttcacacgacgaccgcgtaccagcggcggttggtgatcttcaacagccatcgtcatgatgcgcgtcagcatagaggtccccacacgacgggtggagctgtcatacgcttcacgtactgattcaaacaagttaccaacaccactgccgtgcaaggcagagataaagtgcacacgagcaaaatcgataaagcccagacggaagtccagcgtttctttcacctgctctttcacttcctgactcaggccatcccacttattcaccacaatgacaagtgagcgcccactattgagaataaagcccagcagcgagagatcctgatcggaaataccttcgcgcgcatcaatcactaacatcaccacgttggcgtcttcaatggcctgcaacgttttgattacggagaatttctctacagcatcggtgattttgccgcgtttacgtacgccagcggtgtcaatgagcacatactcacgtccatcgcgttccattgggatgtagatgctgtcacgcgtcgtgccaggcatgtcgtaaacaacaacgcgctcttcaccaagaatacggttagtgagtgtagacttacctacgttcggacgacccacaatcgccagtttgatcggcagactttgcgggtcgaagtcgtcttcctcttcttcttcgccgttctcttccgcttcaaattgcgcccagtattcagcgtcttcgtcgacttcctcttgcggtgcgagatcttccatccacggcagcagcacatgctccagcagacttaatacgccacgaccgtgagacgcggcgatcgggtagatttcacctaaaccaagcgagtagaaatcaaccactgcctgatcgggatccagaccgtcagttttgtttgccaccaggaaggtcggtttttcacgggagcgcagatgtttggcaatcgcttcatctgccggcatcaggcccgcgcgcgcatccaccataaacagtacgacgtccgcttcttcaatcgccagcagcgactgttccgccatgcgggtttctacaccgtcttctgtgccatcaatcccgccggtatcaatacagataaactcacggccttcaatttccgcacgaccgtacttacggtcacgagtcagacccgggaaatccgcaaccagcgcatctcgggtgcgagttagacggttaaataacgtggattttcctacgttagggcgcccgacaagcgcgaccacaggtaccatgtttaaagcctcatttttataaatcatcagacaacgcacgctatattcgcgtcgttgttaaaaacaggaaaacggcccctgtccaggagccgttttcaaagtgaacgacagagacgattaacgtgtaatagagtacacggttccgtcttttgcctggatcagcagtttgccgtcagcggcaaccggttcagtctggaaaccggaactatcaactttttgctgggcaacgaaacgaccatcttcgacgttaatccagtgcagataaccttcactgtcaccgaccaccaggttgccattatacagcaccggagaagtcagcaggcgatgcagcagatcgctttgtgtccacagcgtaacgccgccatcaatggtcaacgccatcacccggtcattttgatcgaccagatagatgcgattgccgtcgacgatgaaatcattcaccgaacccagttcgcgtttccacataatctgaccactgcgcagatcaagcgccgtcaggttaccattataggccagcgcgaaaacaacgccgttaacaacgacgggagtcgtgtcaacatcgctcagacggtcaatttcggtagaaccggtcgcctgggaaatacgctgctgccaaatcatctggccctgttccatcagcactgcgctgacgcgaccattatcgccccccacgacggccgcaccaaaagccgttgtcggcgcagactcgccacgcaaagagagcgaaggcatatcgaggttaactgtccatttgacagcgccgtcagcttcgttcagcgcttgtaactgaccgttactggtgtggattaacaccagaccgtcgctgaccaccgggcgcgaaagtgcttcacccgcgactttagtttgccatgccacagtaccatcgctggtattcagcgcgtaaacctgcgccttttcgctgccaatgtagacatgcccaccagacacggtcacaccgccagaaagtaatgcaggctctttagagaaccagccatctttctcggccaggctgacagaccagatttctttgccatcatccgcattcagcgcttttactaaaccagcgcggtccgctgcatagacaacgttgtccgccagtgccggatgaagattggaatagaagttgccaatgccgctaccaacggaagtgctccacgccgtggtcggcgtaaactggttttcaacggttggcaatggggacatctttaccacatcttcttcgctgttaaacagcgaacagccgcttaaaagggtaacggaaagcagtcctggcagcagtaatttacgcaattgcatcgggtccctctcagatggacaaattattaattttcatctgcatcatttcgctcagtgccggagtaacatcgcttttcacgcctgcttcccatgcactacgcgcaccttgcttatcacctttgctcagcaatgcttcaccacgcaggtcggcaacaatggcagcccacccttcacctttgatggtatcaagggttttcagcgcggcatcagcctgcttgagctgtacctgaacgcgagcaagacgcagatttatcacggctttgagattttcatcgctcgtgtctgccagcccctgttgtaactgggcggcagctttctctagttcatttttgtcaacaaattgctgcgcaagttccaaagaagccagcgcaccataagtatttttattttcagcagcaaatttttccgccgccgggatgctatccggtttgccttcgctcactgcggtaaccgcattttgataggcaagagaagcggagcgtgcagaatcaacctgatggctgttccagtagcgccagccaatcagtgcgccaacgcccaaaatcaccccaacagccagtgctttgccattttcagcaaaaaagcgtttaaccgcttctacctggtcgttttcgttctcgtaaatttccacgctgtccttctccttccttaacccagtaacgtgcgcaaatgcgcggctacgctatcctgcgcaactgccgtttgctcaccagagcgcaaatccttcactactgctgtgccgttagccacttcagactcacccagcaccacagcaacgcgggcaccccatttatcagcacgggcaaactgtttcttaaagttgccgccgccgtggttggtcatcaatttcacgcccggtaattcatcacgcagacgctcagctaatgccatagccgcagattgtgtatcagcacctgaagccaccaggtatatatcgacaacaggatcggctttaaattccggattaacggcctgtactaacaatacaagacgttcgaggcccatagcaaaaccgacagccggtgttgcacgaccgcccagttgttccacaagaccgtcataacgaccgcctgcacacacggtgccctgggagccgagactgttagtcacccactcgaaaacggtacggttgtagtaatccagaccacgcaccagacgctggtttacggtgtaagcgatccccgcgctctccagcagtttgcacagaccggcaaaatgctcacgagattcctcgtccagatagtcacctaatgccggagcgtcgttgagaagcgcctgcacttccggattttttgaatccagcacgcgcagcgggttagtgtacatgcggcgtttgcagtcttcgtccagcttttctttatgctgctcaaggaatgccaccagcgcatcgcggtaattggcgcgtgcttccagcgaaccgatagagttcagctcaagagttacgtgctcggaaatacccagcgcgcgccaccagcgggcagtgagcataatcagttcagcgtcgatatccggaccttgcagaccgaaaacttcgcagcccaactgatggaactgacgataacgccctttctgcggacgctcgtgacggaacatcggcccgatataccacagacgctgttcctgattgtacagaagaccatgctcgatgccggcgcgtacacagcccgccgtcccttcagggcgcagagtcaggctgtcgccattgcgatcctcaaaggtgtacatctctttttcaaccacgtcggtgacttcaccaatcgcacgtttgaatagcggggtctgctctacaatcggcaagcggatttcactgtaaccgtagctgccgagcacgtttttcagtgtgccttcaatgcgctgccagatggccgtttcgccaggcaggtaatcgttcatgccgcgaatggcttgaatgttttttgccacgtttattctctttctgaatataaaaatgaaccctcaacgcttccctcaatgtttcgggagccatgcgggttcaatcatacacgggaagcgaggcgcttcccatcacgttattatttttcaacctgctgaacgtcaattcgacgcgcttcgtccagctgactggctttcgcacgaatgcgtgcttccagctggtcgatcatatcgttgttgtccagacggtctttgcgcacgccatcttcatagaggccgcttttcttgttgccgccggtgacgccgagtgtagaaaccagcgcctcacctgggccattcaccacgcagccgataatcgaaacgtccatcggagtgatgatatcttccaggcgttgctccagcgcgttaaccgtaccgataacatcaaattcctgacgcgaacaggtcgggcaggcgatgaagttgatccctcgcgaacggatacgcagcgatttcaaaatatcgaaaccgactttgatctcttcgaccggatcggccgccagcgatacgcgcagcgtgtcgccgatgccttcagacagcagcagacctaaaccaatggcggattttactgccccgctgcgcgcaccaccggcttcggtgatccccagatgcaacggctgatcgatctgttttgccagcaaacgataagactcaacagcgaggaagacgtcagacgctttcacgctgactttgaactgatcgaagttcaggcgatcgagatgatcaacatgacgcatggcagattccagcaacgcctgcggcgtcggttcgccatacttttcttgcagatctttttccagcgatccggcgttaacgccaatacggatcggaatgtttttatcgcgcgcacagtcaaccaccatgcgaatacgctcttcattaccgatattgccagggttaatacgcagacaatcgacgccgtattccgctactttcagcgcaatgcgatagtcgaagtggatgtcagccaccagcggcacgttaacctgctgtttgatgagtttgaacgcttctgccgcgtccatcgtcggtacggatacacggacgatatcagcgccaacgcgttccagcgccttgatttgattgaccgttgcttcgacgtctgtcgtacgcgtattggtcatggactgtacggcgatgggagcaccatcgccaatcggcacattcccaacgtaaatacgtgttgattttctacgttgaattggagcctggttatgcatgaaaaatctcccgcgttacccgtctgttactgcgccggtgattgttcggcattgagggtcagacgcgcaacctggttagttctgataaaacgactcagatcgacaggtttcccttgatactggatctgtactgcggctggcgcaccaattttcagtttgtacggtgcctggccggttaagttcaaattaccgtctttacgctgcataccgctaaacaattttttaccggtagcatcagtgacctccagccagcaatcggcagtaaagttcatcaccagcgcattcggatcagccaccggcgtggtcacgccagcctgatcggttggcaacggcgcagcaccatctggcgttgttgctgccgttggtgccggggtcgcggcggtatcaacatttgcctgcgaaggcgaaacaaccgcattctgttgcggatcaacagctggtgctggcgcagttacggcaggtgtttgcgtgttggttgcggtagtatccacagacgctggcggcgtggacgttgtagccgggtctgtagttgtcgacgtatttaatggaacactctgcccctgctcgctattactgctcagttccgccgaagattgatcggccatagtggtgatctcttcctgctgagctttgcggtcttgccaccaccaggcaccgctcaggccgataaccacaaacaacaccagccaagtgaaggtcatcagccagccgtcgcgttttttgcggcgtttaccgagggaaaaactctgcatcggcgcaacttttgcagcccgaagtggagcctgcttttccagccctggcagcagttcttcttctggaatatgtaccagacgcgcataagagcggatatatccgcgcaggaatgttgaagcaagatcggcgggtgccttatcttcttcaatgtcgcgtaccgtggaaaccttcaggcaaagtcgctcggcaacggcctgctgactaagtcctagttgttcgcgagcattacgcaggcgagcgccggtagtaagtgcttcattttggtcgtgcgtggcttcagtattcattcgctgcaggtacgtttaaatgagaattgagatgccggtgaaccatcatgctcacccacaccgcgaaacatccgttaagttaaccgttatcatacagtataagaccgtctgtgtgctcgtgacaaagcccacattcactaaggctaacttactgttgcatcgttacatactgccttaaagtcagcaaaaacgcaccgttaatattgaccagacaattgcaacttaatacttcattcataaaacattacgccacggtacataaagtaaccgtggcgtaatggctatcagaccgctttaatgtcgatggcttcaccctgcatccgtttacgcagggtacgtttcgtacggtcgataacatcgcccgccaactgaccacaggcagcatcgatatcatcaccacgagttttacgcacaatagtggtgaaaccgtagctcatcagcacttttgagaaacggtcgatacggctgttcgagctgcgtccatacggcgcacccgggaacgggttccacgggatcaggttgatcttacacggcgtatctttcagcagttccgccagttggtgcgcgtgttcagtgccgtcgttaacgtggtcaagcatcacgtattcaatagtgactcggccctgattggcgttggatttctccagataacggcgcaccgcagcaaggaacgtttcgatattgtactttttgttgatcggcacaatttcgtcacgaatttcgtcgttcggcgcgtgcagggaaattgccagtgcaacgtcgatcatatcgcccagtttatccagcgccggaactacaccggaagtggaaagcgtgacgcgacgtttagacaggccaaaaccgaaatcatcaagcatgatttccatcgccggaacgacgttgttcaggttgagcagcggctcgcccatgcccatcatcactacgttagtgatcggacgctgaccggtgacttttgctgcgccgacgattttcgccgcacgccacacctggccgataatttccgacacccgcaggttgcggttaaagccctgctgggcggtggaacagaatttacactccagcgcacaccccacctgcgaagagacgcagagcgtggcacggtcgtcttccgggatatacaccgtttcgacgcgctgatcgccaacggcgatcgcccatttaatggtgccgtcagatgaacgctgttcttcaaccacttccggtgcgcggatttccgccacctctttcagtttgccgcgcaacactttgttgatgtcggtcatctcatcaaagttgtcgcagcaatagtgatacatccacttcatcacctgatcggcgcggaagggtttttcacctaaatctttaaaaaactcccgcatctgctgacggttgagatccagcaggttgatttttccatctttcgtggtgacgttttcaggtgtgactaattgttcagacatatgctattccggcctcgttattacacgttatggcccctggagggttgaaaaaagaaacgccccggtgagcggctgctcgtccgggggcgctgcattgtacaaattctggcgcacggatgccacgtttgcacgcggcatttacgaaattattaacgggtgcgcgggcacacttcgccttcgccaaagaaataagcgatttcgcgagcggcagattcgacggaatcagaaccgtgggtaccgttttcggtcaggctgtcagcgtaatcagcgcgcagagtaccagccagtgcgtttgccggattggtcgcgcccagcagatcgcggtgacgctgaacggcgttttcaccttccagcacggaaaccacgatcgggccagaggtcatgaattcaaccagaccatcaaagaacggttttccatcgtgttcagcataaaagccacgtgcctgttcaacggtcaggtgcagcattttggtgccaacaattttgaaccctgcagcttcaaagcgcgcaaagatattaccaatgacgttttttgctaccgcgttcggtttgatgatggaaaaagtacgttcaatagccatttttacctctgtaaattgttctgttgttgtctgtaccagcgtacgagatggcgcggattataatgagcaacagggccgttgactattgatgaaggtaacatttttttaaaataaaatgagttttagcaacaatcagggacaaaacagactattgcatgacaaatttcactgtcgcgatttgccccacgtcatccatcaccagcaattgataatcacctttatccgtcaaatgcagggtcacgttgcgcccgcgttcagttaacggttcgccattcagaaaccaccagcgttcacctgcccctccacttgattgcaacggcaaagtcgcttccgctgcgcccggtaaacgtttaataatcgcgccatcgcgaacgcctgtcagctgcagcgggagctgggcatcgtgaccgtatggcgggcaacttgtcgaggccggtggtaagcgcacagcgcgacgttctgatgcgggcagccagggttccagcggtagcggccagacatttatcatttcttgtcgcgcttgcgggcaatcagcggcaacacgtttgccattttcatccagccagatggggaaacgaatgccattaatgccttcctgctccggcagtaatagagttggcggctgactcccgtccagcagccaggttgccaggcggcggcgacagttaccgtcaccttccggcaaagactgtccgcccggccagcagataacgccacgagtgactgagttcgggcgcgggtcttccggcagattcgcactgcgcgacagtaagatattattgacctgattcaacaatggtacggcactggcaaagccaaactgaccaacaacgggcgtgccgtccggtctgccagtccagatcccaatgacatagcgagcgttaaccccaatcgcccaggcgtcacgatagccatagctggtgcccgttttccatgccagtggggcgacgcgcggcaaggcactatccggcaagggttgcgcttcatcagccataatccggcgaatgatccacgccgcccccgacgacattaaaggccgttcaagcagcggatcgtcaggctgtaagcgcaatttgcctgccttgccgtggcgagcaaacgcggtatacgctgccgccatatcttccagttttgcaccagcgccgccgagaatgagtgaaagattcggcgcagcaccgttgggcaaatataacggcaatccaacattgcgtaactttgccgcaaaccgtttcggtccataggcttccagcacctgcacagcaggtaagttcagcgagcgcaccagcgcctcgctcatgctgatcgggccatgaaaaccgctatcaaagttacctggtcgataatcaccggtgcgccgggggacgtcttgcagcagtgatgccgggtggatcaagccttcatccagcgccagaccataaacaaacggtttgagcactgatcctggcgatcggatcgaattgaccatatcaacatgaccaaagcgtgaatcatcgttgagatcaaccgatcccacccagccgcgaacacgcatatcggtatgatcaaccacgatcatcgccagtgagctgcgcggtggcaaccgccctttccagttttgcgccagttcttccagacgtcgttgaagaccggcatccaacgtagtagtgattttgtcgcttttgcttttaccgagcatcatgcgcgaaaacagcggtgccagttgcggcatttgtcggggggccagccagatgggttcttcccttgactcttttacctgctcacgggaccacacaccttgcacggccatccgttcgagcactttattacgcgcggcttcggcacgctccggccaacgatccgggcgaagacggctgggcgcttgcggcaaaaccgccagcattgccgcctcggaatagcttaaattcgcaggcgattttccgagataagcccaacttgccgcaccgatcccctgcaacgtaccgccaaacggagcgcggttaagatacaaggtcagaatttcacgcttagacagatgccattccagttgcaacgcgcgccagagctggcgaattttgccgccaaatgttttggggtgaggatcaagcagacgagcaacctgcatagtgagcgtgctgccaccggaaataacccgtcccgaagtgagatcttgccatgctgcgcgcgccaccgagaatggattcacccccggatgcttccagaaccagcgatcttcataattgatcagcgcttcaaggtaacgtggagaaacatcttcgattgttaccggataacgccagatgccgtcagcatcggcgaagcgccagagcggcgtaccatcctgcgccacgaccactcgtgcgggattgacttcatgcagcggtagaggccagagtttatctgctccccacgctgcaagaaaaaggagaaagggcgcggctgccaacgttatccagcagccgcgtttggttaacaagcgaggcatttacggtctgacaatcagcagatcttcagccgcgccggtcgcccgccattggggaacatacattgattccaccatcggttgcggtacctgatacgttcccggcgtcaccgcccgcgccagatacaccagcgttaccggttggtattcatcaacggcaaccgccgccacaaagcgatcgtcacggaactcaatgtgcttaatgctcgcctgctgcatctggttcagtaagttctgcacttcgccaccactttgctccaggctggcgctaccgttcgccagattctggttttccagttccagacccgcaggcagcagatccacgactaacgcatccggcacgctgttactggcttttacctgcaaccacaccagcaccagatcgccgctacgtaacgagtccagcgatttgctcttaccatcagtaccaagaatatgacgctcgatttgcagcacattgttcgccggtaaaggtgcggattgcggataaccgctggcatccatacgcaaccataacggctgatcgccactgttgctcacctgcaaggtgacaagttgatcgctattcagattgctgttttgcgctttctcgcctgtcagctgctcagctgagaaagaggtttgcgcctgccatttaccgggtaaatcctgaatcgtacgggcagccaggaacaacgcgttactttcctgcgtcgatagccagcgttcaccaaacgcctgctgcgaaagtgtgttcagcaaagtgtactgctcatcgggtagcagtttattttcttccagcaaggagagcattaacgcgttgtcgcgcagtgaactaccgtaatcacccagccatatccgctcatcactattacgcggcgttttcagcgccagcgcaatcgcttcttcaccacgcgtcgcatcacccatggttttcagcgcaacgccaagttgcagcagcggtaaaccagaagcggcatctgcacgatgctcccagatttcacgcagcgcacccagcggagccttttgctgacgggccaacaccagcgcagcgtaagactgtacggcgaatttactggctttgagattatccgcgtacgggatcgacatcatgcccggatcttgtaaatagcgcagcagacgctcattaccccggttaatggcgtctgtcggcacgctgtaaccctgttcgcctgcgcggaccaggaaatccatcacgtaagccgtcagccagtactcttcgtcaccgtttttatcccacagcgcaaagccgccgttatcacgttgcatttgcagcaaacgggaaatgccgatatcgaccgatgcacggcgtttctcatcactgtcgcctttgatgcccaacgcctgcagttgggctgcgttggtataaagtgacggaaacaggccgctggcggtttgctcaagacagccgtacggatacgcttttaactctttgatataacgtgcgatgttcagcggtggtttgccgctcaacaacaattgcccttccagcgtaacaggcgagaagttttgcaatccatccgccggaatcgcccatgtctcaccaggctgtaacgccgtaccgtaattaaccgtttgtgccgggaacgccggacggacgccgattttccactgcttatgctgatcggcaacggtttcacccggtaacgctaacccgctaatggtggcctgaatttctccatcgccataacccggcaatgctcgcaccgggataaacagcgtagtacgcacacctggcgctaattcaacggctgcgggtgaatcgctgaccagttcaagcaaaccactggcggtcagggcaacgttcagtttttgcggtttatcggtaagattagtgatatccagcgtcagacgcgaggtatcgccactcgccataaagcgcggcatgttcagttcagcaatcaccggtgcggcaactatcactttactttcgttgctaccgaagtcatctgccgtccaggcttgcgccatgacgcgcaattcaccgttaaaatcgccaatcggcagtgtaaccgagccttcgccctgttcgttgagcgttaccggcagcgcctgctgcacgacaatattgacgtgattgaccggcggtttaccaccacgtttcagctcatcaccatcgccaccgaaacgcagagctgccagacgcccctgaccttcaataacctgaccgtaaatatcgtaaatgtctgcgccatagcgtttctgaccaaagaacgcctgccacggatctggcgtgacgtagtcagtaatattcagcacaccactatcaacggcagacaccagcacattcacctgtttaggcttctcgccatttttagtgctggctttaattttcacggttaatggttgattgggacgcatttttgctggtgtttccagcgccagatcgaggcgacggttttcatcgccaagcggcagatgcaacacaccaaccgcgcgttttggcgtcgcggagcgagatttatcgccaggacgtaccaccagcgtacttaaatacagatcatgacgattccaggttttatcgaccggaatcgtcagatccagcccttgagcccgaacatcaatctcttgccaccacagcggcccttcactggactcgaccatcgcataacctttacccgccgttggcgcggcgatatgcaacttaatggtgtcgccagggcgataactggctttatccagtttcagcgtgacacggtcgggtcgcactgcgccgctaccgtcgctgttgtcctgccagctatagccagcccagaaacgaacactactgaccgcttcattcggcgctttgacttccagacgataagcgccccactctaccggaaaactgaccttgccggtttcgtccgctttcagatccagagtttgttcattttcgatcagatctttttgatcaaactgtgactgccagccttcatcttctgaccagttccagtagtaatcgcggcgttcgcgaatcaggcgcacctgcaagcccgacacggcttttttcacgccttgcgcatcgctataaacgatgtcaaaagcggcgttactgccttcatcaacaatgggctgtttcaccgtgctgtcagtacgataatcgtaaaccgatttcgaggcgaactgcggacggatccccggcaatgcatcggcaggccagatagcctgctcagcgcggcgcgtcaccgggcgaccgcccgattccagcaaactaccctggaaaataacctgtaatggggaatgcgtttccttccactggctttctgtagaaacttcgccgcgccctttatcatccagcgtcaactgaacttcatccagcgtgcgggaaagattttcggcagctatatcgccgaattcaaaaccaggtaaggctgacacagcttcacgcagtgggcgcaggaaaagttgcccttgcaaagtattaccattagcaggtgcaccatacaggtagtaccccaccacggagaatttcacttcatctttcggcgttagcggggttttctcaccggtcagattcagcgccatgcgctctggcataaaatcttcgacgtggaaatcccacatccgatactgattatcgcccgtgttagcgcgaatatgccacataccggttgccgcattgctatcgagtggccaggtaaagtggtagaggccattctccggctgactaacgacgctcctgagtacctgcccatcgggtttaatcacgtctaacttgatgggttgattgggcaacgctttaccgtctgcatcacgcagcaaaccattgaggattaccgtttcacctgggcgataaagatcgcgtgggccaaacatgaaaaactgtttgctatagcctggcgcgccagcaatgttaaattctgctaagtccagcgccggaagttttaaatcgagtagcgttgtctgaccgtctttacgcgccaacagtaatgccgcgtttttatcattttccagctgcacatgcccctgagcgtcactggttgcctgagtcagagtctgccctttctcatttaataaagagacttcaattccttgctgggccgcgccgttttccagactttgggtaaagatatccagacgattgtgataacggtgagctgaaacgccgatatcacttaacgtaaacagcgtcgcgggattactgtaatcgtaacgtccagcctgattcatcacagccagatacacgcccgcctgctgaagcggtttgatatcgcccagcggcagcaataatttttcacgggtgttacgcgcaggattgagatcaaaccgtccggtgtagaccagatccgccatctgcagcagtttgtctgactgccagttcgccagcgaattgcggtattcccattggctaatgaatgctggcagagattctggcttaacgcggaagaagttaacatcgacattattaacgttgagcgccattaccggcagcccttcaacgactttgccaggcagcagcgaaccacggctggcaaaaccgacgctgggttggatgtcgcgggtagttatagttttttcgtaatctttactgaaggttgcgttgttgagtgctttgacctccttgccaatagtaacgatcaaatcacgtttcggttcgaggtggcgtaaacgtaactctttaagattatctgacagctcccaggcaccatccactttgccgctttttttatcgacgacatgaataacgcgtgagaaatcctgatccgggtcgagagggatggagaacgtcagcaccagcgtggctgcaccatcaagttggacttcagagagatccagcaatgtcagcaccttaccggcactctgttgggccagtttttgtctctccggcacggagagttttgctgaactcgcgttttctgaagaggccgctttagtaacttcagaaggcgcatcttttttcaccgctgttggcgcgttatcgttgttgtcgcaccctgccagcgccagcattagcatgcaggcggctacgcgtaactttttcatttttcatccctgccacaatggcccgttagcaacgtcgaataattattatgcgtgagaatttacgttatgtaattcagtatcacgcccatacaatccgaattttagtgagaattgtggctcagacagccaaatcagcctcttttgcttgtcgcttttcactaaacatccgacaatttagcctaaccccggcaaaaatggagatgcctatgtccacgacatggtttgtaggagccgactggctcgccgaacatattgatgacccggaaattcagattatcgatgcccgcatggcgtcgcctggacaggaggatcgtaacgttgctcaggagtatctgaatggacatattcccggcgcagtgttttttgatatcgaagcgctttctgatcacacttccccgcttccgcacatgctgccgcgcccggaaacgttcgccgtggcgatgcgtgaattaggcgttaaccaggataagcacctgattgtctatgacgaaggtaatcttttctcagccccacgagcatggtggatgctgcgcacctttggtgtagagaaagtgtcgattctggggggtggacttgcaggctggcagcgcgatgatctgctgttagaagaaggtgcagtagagctgccggaaggagagtttaacgccgcgtttaatcctgaagccgtggtgaaagtaaccgatgtattattggcaagccatgaaaatacggcgcaaattattgatgcccgcccggctgcacgttttaacgcagaagttgatgaacctcgcccaggtttacgtcgcggacatattcccggagcactgaatgttccgtggacggaactggtgcgcgaaggcgaactaaaaacgaccgatgaactggatgcgatattttttggtcgcggcgtcagctacgacaaaccaattatcgtcagctgcggctctggtgtaacggcagccgtggttttgttagcactcgcgacgctggatgtgccaaacgtgaaactgtacgacggcgcatggagtgaatggggcgcgcgggcagatttaccggttgagccagtgaaataagtattttacaggcaataaaaaaccgccgaatttggcggttttttattgctagtctggttcgcggcctttccagcaggttgacttgtgttacatgagcaacgcaggtgcttcacagcaaaacaatactcaccagtaactctctttttgtcaagcaaaagagagtaattattgtttatttagcgtattatcgacaccggccctttccgccgtgttcggtaataaaataacctggcttattagtccgaattcagacaaatataaataaatcctgctcaaaattaaaaattctaaccggtaaaagatattacttaaacatgtaaattcactttcctttaaaaaacaaaaaaccgccaaaatcaggcggttttttgttgctggtccggttcgcggcctttccagcaggttgtattaccgtagtaatgcaagcgcgtctcagcggagacaatactcgccagtaactctctttttgtcaagcaaaagagagttattattgttctgttagtgtattatccactgcggccctttccgccgtctcgcaaacgggcgctggctttaggaaaggatgttccgtggccgtaaatgcaggtgtttcacagcgcttgctatcgcggcaatatcgccagtggtgctgtcgtgatgcggtcttcgcatggaccgcacaatgaagatacggtgcttttgtatcgtacttattgtttctggtgcgctgttaaccgaggtaaataataaccggagtctctccggcgacaatttactggtggttaacaaccttcagagcagcaagtaagcccgaatgccgccctttgggcggcatattttagattatccgattctgtttaaagtcacgcaaaaaaccaccccagcgacgttcatagaatggcgcaatatgttcggtaataaagtggctaattcctttttccccttttttcacctgacaaatatcgattggttcatcgccaggtaatgtatcggtcgctacacttcccgtcgcctgaataatttcttcgatatcaccatcggcttcaatgccaataagtaaattaggctgtgcctcttcgttctctttaattgaacaaataaaagcacgcttcaccggcttaatggttttaaataaggtggtgagtgaatcaatcatttgtgctggcggctctgcgacttccgataatatcagcgattcaccgccttccaggatttcctggctgctcagcggatttccctcttcaccaatcaacaaactgatttcacgcggcataaattctttaccggttggcagtttggcattaaggaagagcgtttcgccaagtgtcatctcaaacagcgtgcgaacgggcattacgacaaatgcctgttcgtcttcaaccgcctgttgaagtgcttctaacgaggtgaaaaaaggaatgacgctggtgccgtcttctttttcccagtgctgtaaatcaagcgcgctatcttcaaccacagcctcgccctgcgccgccgtaccaggcacccagacggtggattccagtagagtacggaaaaaggccgggcggtgcgccggttcagttgctgctttttccagcaggtcttcaagttcgttttttgtttcggacataagaaccacaattcattcaacgttcggggcgcaaatgcctgatgcgctacgcttatcaggcctacaagggattcgcaatttgttgaatttgcagaatttgtaggccggataaggcgtttacgccgcatccggcatattagtttacgccgttaacagattagctatcgtgcgcacaccaagtcccgtagcgcccgcagaccactgttcaaccggcgctttacggtaagtcgccgagcagtcgatatgcagccagccttgctgatagttctcaacaaagtgcgacaggaagcccgccgccgtgctcgcgcctgccggatacgccgcgcttccggtattgttcagttcggcaaagttagacggcagctggctgcggtggaactccgccagcggcagacgccagaacggttcgttctcctgcgcggcactcgccagcaagcgaccggccagcgcatcgtcaaaactgaacagcgcgtgataatcattacccagcgcagttttcgccgccccggtgagggtcgccgcatcaatgatcatttccggtttctgcgcactggcatcaatcagaccatcggcaagcaccagacgcccttcggcatcagtgttcatcacttcaacttttttaccgttgcgataggtgatgatatcgcccagcttgaacgcattgccgctaatcaggttatccgcacagcagaggaacagcttcacgcgcttgttcagtccgcgcgtaatggcaaatgccagcgccccggtaaccgttgccgcgccgcccatgtccgacttcatcgagtccataaacgcagtctgtttgatgctgtagccgccggagtcaaaagtgatacctttacctaccaggcacgcgtacactggcgcttctttatcgccagttgggttgtaatccagcgccagcaataccggagaacgttctgaaccgcgtccgactgtgtgcagccccatataaccttgctcacgcagatcttcgcctttggtgatccgataagtcacacgatcgcccgcgacgttgctgatcagatcaacagcacgctgtgccagttgcgatggtcccaattcttctgccggtgcgttgatggtgtcacgcacccagtcgatgatcatcaggcggttatccagttcctggcgctgggcatcgtccagatccggccacaccactttacgcgtgcctttcggggctttgtaaccttgccagaatgcccagcagcgatccgcatcccagccttcaccgcttaactgaacatgcttgatgcccagaccgtcaatcttgcgcgccgcacgctggatcagccccagatcgtctgccccgttcaaatgcagggtaatgccgtcattattaatgctgtaagttgctttttctccccagcgcgcgtcggcaggttgggtagagagggtaatcttcatcgcttctgtcattttagttatccttctttgtaaaagggccgccagttggcagccccaggatttttccgctaaatgattcgcgttgcaggaaggcggcaagtgagtgaagccccaggagcatagataactatgtgactggggtgaacgagcgcagccaacgcatctgcggcgtgaagcatgacgcggaaattattcggcctcgtccagccagactaacaaaatcgcttcgaggattttctcgttggatgcctgcgggtcgtcgtcgaaatcttccagatcgcaaatccactgatgcatatcggtgaatcgaaccgttttcggatcaagatcgggatacgcatcgtacagtgcttcgccaatttcgcggctatcggtccacttaagtcccatactaacctctgttaatgctcacgcgcatggttgatagtgtaacgcgggatttcgactactaaatcttcgtcggtaacgcgcgcctggcagcttaaacggctttccggctccagtccccaggctttgtccagcatgtcgtcttcctgctctgagctttccggcagtgagtcaaaaccttcacgaacgatgcagtggcaggtggtgcaagcacaggatttttcacaggcgtgttcaatctcgataccgttacgcagagctgcgtcgagaatggtttcaccgctattagcttccagaacagcgccatcagggcagagatcctgatgaggcaaaataacaatctttggcatattaaacctcgtccacggaatggcctttcagcgcacgacgaaccgactggtccatgcggcgagcggcgaaatcctgggtttgtttgtctacgtttttaatcgcttgttcgatggcgtcaacatcatcgccctgcgccacttcactcaggtgagcggcagcatcgtcaatgacctgacgttctgcggcgcttaacagcgcggcatcagcagccagcgcgccgtgcagactttccagcacacgcgccgcttctactttttgttctgccagcattcgggcttttacgtcctgctcggcatagctcattgagtctttgatcatcgaagcgatttcgctatcggtcagaccgtaagacggtttgacctgaatagacgcctcaacgccggtggatttctccatcgccgtcacgctcaaaagaccgtcggcatcgacctggaacgtcacgcgaatatgcgcaccgccagccggtagcgccggaataccacgcagcgcaaaacgcgccagtgagcggcagtcctgcaccagttcgcgctcaccctgcattacatggatagacatcgccgtctgaccatctttaaaggtggtgaaatcctgagcgcgggccaccggaatagtggtattacgcggaatcactttctccaccaggccgcccatcgtttcgaggcccagcgacagtgggatcacatcaagcaacagcatttcgctgtctggcttgttacccaccagaatatccgcctgaatcgccgcgccaatagcgacgactttatccgggtcgatggaagtcagcggtggacgaccgaaaaattcgcctacccgttcacgcaccagcggcacgcgagtagaaccgcccaccatcaccacttccagcacttcatcagcttctacacccgcgtctttcagcgcgcgacgacaagccagtaaggttcgttttaccagtggcgcgatcagttcattgaattgttcacggctgatttcgccctgccagcccgcaacgttaacggtcacggagtccgcatcgctcagcgcgattttggctgcaatggcggcatccagcagttcacgctgaacgcggttatcgctacgatcaggaatgcccgcctgctcgcgaatgtaatccgccagcagatggtcgaaatcatcgccgccgagcgcggaatcaccgccggttgccagcacttcaaacacgccgcgacttaagcgcagaatggaaatatcaaacgtcccgccaccgaggtcataaacggcgatcacgccttcctgaccggaatccagcccgtaggcgatagccgcagcggtcggttcgttaagtaagcgcaggacgtgaaggcccgccagacgcgccgcgtctttggtgccctgacgctgggcatcgtcaaagtacgccggaacggtgataactacaccatccagctcgcctgccagggcttcagttgcccgcgccgccagtgctttgaggatgtccgcagaaacgcgcaccgggttcagcagccccgccgccgtttcaatcatcggcaggccgttttcgctggcctggaattgataaggcagatgcggatagcgttgctggatatcagccagcgagcgtcccatcaggcgtttaacagaactaattgtgttggcggtatcgagcgctgcattagtacgcgcgtcataacccaccgaatgcccttgctgttgatagtgaacaacagatggcagcaggtgacggccttcatgatcggctaacgtttcggcctgaccgctgcgcactgtcgccaccagcgagttggttgtgcccaggtcaataccggccgccagacgacgctgatgcggcgcagcactcaaaccaggttcactaatttgtaataaggccatgtttagcttccagaaattaaaaatcgagcagtttttcttcgagttgttcggcactgcttcgcagtttatcgagaaaacgcagcttacgcacggtatccgccgccgcgtcccacgtctcgttgtctaactgttcaaccatcaactgatggcgggtatcaaacatctttttcacacgtttgataaagctttccagccgcgcttcatctttcgcctgttcgatctcgtccagctcttcgcgcagctccaactgttccatcaggaacgcggtgtcgcgcacagtatgctgctcgctggcgagatcaaagccgtgcaaagaaagcaaatattccgcgcgcattaacggatgacgcagcgtttgccaggcctggttaatggttgcagattgctgtacggcggcgagttgttccgcctggcttccgctggcgaatttatcaggatgatactgacgttgtagatcctgaaaacgcaggctcagcgcctgggtatcgagttgatagcgggcaggcaagccaaagagggtgaagtaatccataacattctcagggctgcgatccgccgcgataacggcgaatcaggtaaaacaaaccccacgcgcaggcgaccacggtggggttatcggtatgcgcatcaaacgtggaagctttcgccgcaaccacactcatctttgacgttcgggttggtgaatttaaacccttcgttcaggccttcttttacgaagtccagctgcgtaccgtccagaaattgcaggctcttgccatcgaccacgactttcacgcctttgtcttcaaacacgatgtcttccggcgtcggttcgtcaacaaattccagtacataagccatacctgaacacccggaggttctcacgcccagacgcaggccaaaccctttaccgcggttagccagaaaggtatttactcgcgctgctgcactgtcgctcagtgtaatcgacataaccaaacctcaactcttattttgcttcacgtttgcttttatagtccgcaatggcggctttgatcgcgtcttctgccagaatagaacagtgaattttcaccggcggcagttcaagttcttcagcaatatcggtgtttttgatcgcctgcgcttcgtcgagagacttccctttcacccattcggtgaccagggagctggaagcgatagcggaaccgcagccgtaagttttaaaacgcgcgtcttcaatgataccttcatcgttgactttaatctgcaacttcatcacgtcgccacaggccggtgcccccaccatgccgctgccgacgttctcgtcgttgttgtcaaaggaacccacgttacgcggattctcgtaatggtcgataactttttcgctgtaagccattataaattctcctgattccgataccgattaatgatgagcccattcgatgctgttcagatccacgccctgcttgtacatttcccacagcggagaaaggtcacgcagacgaccgatggatttacgaactaactcgatggtgtagtcgatctcttcttcagtagtaaaacgacctaaagagaaacggatagagctatgtgccagctcgtcgttcagccccagcgcgcgcagcacgtaggacggttcgaggcttgctgacgtacaggcggaacctgaagaaactgcgaggtctttcagcgccataatcagcgactcaccttcaacgtagttgaagctgacgttgagaatgttcggcgcaccgtgttccaggtcaccgttcaggtaaacttcttcgatatctttgatgccgttccacagacggttacgcaggccgcgcagacgttccatctcggtcgccatctcttcttttgcgatgcgataggcctcgcccattccgacgatctggtgaacaggcagagtgccggaacgcataccgcgctcgtgaccgccgccgtgcatttgcgcttcgatgcgtacgcgcggtttacgacgtacatacagcgcaccgatacctttcgggccatagattttgtgaccggagaaagacatcaggtcaactttcaactggctcaggtcgataggcagtttacccacgctctgggttgcatcaacgtgatagataatgccacgagcacggcacatttcgccgatagccgcgatatcctgcaccacgccgatttcgttatttacgtgcatgatggacacgaggatggtgtcgtcacgcatcgctgcttcaagttctttcaggtcgataatgccgttacgctgcggtgccaggtaggtgacttcaaaaccttcgcgctccagctgacggcaggtatccagtaccgctttgtgttcggttttgctggtgatgatgtgcttgccttttttctgataaaagttggctgcacctttgatcgccaggttgtcagattcggttgcaccagaggtaaagacgatttcacgcggatcagcgccgaccagatcggcaatctgattacgggcgatatctaccgcttcttcagcctgccagccgaaacggtgagaacgggaggccgggttaccaaaggttccgtccatcgtcataaactgcatcattttctcggcaacacgcgggtccaccggcgtggttgcggagtagtcgagataaatcggtaatttcattgctctataaactccgtacatcactcaatgcaaggaatcaggctaccggctggatgtacgaccgtgtttacggagtatttagcactccggcctgattctgaattctttttattaagcgcgtaacttaacgtcgatcgcgtcttgtgtgcgggtgcgtggcgcgtcgtgagtatgctgacgaccagacacatccagcacttcctggttattaaccagttcgcctaaagtaatgttgttgagaaaaccggtgagacggtcgctcaaatcacgccacagcgcgtgggtcaggcatttatcgccgccctggcagccgcctttaccctgacaacgggtggcatctacagattcgtcaacggcgctaattacttcgccaacggcgatgctgctggcatctttgcctaacagataaccaccgcctggtccacgtacgctggaaaccagaccatttttacgcagacgggaaaacagttgttccagataagaaagggaaattccctgacgttcggaaatatcagccaacggtaccgggcccgcttcagagttgagcgcaacgtcaagcattgcggtcacggcatagcgccctttagatgtcagtctcatgtcttacttcacctcaaactcgcccctgcccggggttttttattgtaaaagtgggggtattgcatagcagggtcaagtctgacattcccgagtaaattggtcaactatttacttgactgatttagtcgggtatttaaccttcagtgccatttttttatcgtggcgtttgtacctgttgtcggatgcggcgtgaacgccatatccgccctggggttctgtacactgtaggcctgataagacgcattacgcgtcgcatcaggcaacggctgtcggatgcggcgtgaacgccttatccgacctacggttctgttcactgtaggcctgataagacgcattacgcgtcgcatcaggcaacggctgtcggatgcggcgtgaacgccttatccgacctacggttctgttcactgtaggcctgataagacgcattacgcgtcgcatcaggcaacggctgttattcggccttgttacctttattctgctgctcaatagaagccagaatcccgcgcaggatattcaactcctggctttccgggcgcgcacgggtaaacagacggcgcaatttattcatcacctgccccggatggttttcacggataaaaccggttgccagcagcgtttgttccagatgaccataaaaacgctccagatcatcgaccagcggatacggcgtctcttcatgctcgacctgctcgccgttttcctgagttgccagccaggccatgcgcacttcataggcaataacctgaaccgccatcgccaggttcagcgagctgtattccgggttagccgcaatcgcgacatgataatggcatttctgcaactcttcattggtcaagccgacgcgctcgcgaccaaacaccagcgccaccggggtatttgccgcttcagcgacgcttttcaggccgcattcgcgcgggtcgagcatcggccatggcagcgtgcgggaacgtgcgctggtgcccaccaccaggctacaaccggctaacgcttcgtcgagcgtatcgacgatgtgagcattaccaatcacatcgctggcccctgctgccagggcaatcgcctgggagtcgggtttcaccagtggattaaccagccacagattggttaatcccattgttttcatggcacgggcaacagaacccatattgccggtgtgtgacgtctccaccagcacaattcgaatattttgcagcattgtctttcttcatctaaagattattcacgcatcttatcataaaacgaagacagatgccgatctcgctgctatactctgcgccgttttcccgttctttaacatccagtgagagagaccgatgcatccgatgctgaacatcgccgtgcgcgcagcgcgcaaggcgggtaatttaattgccaaaaactatgaaaccccggacgctgtagaagcgagccagaaaggcagtaacgatttcgtgaccaacgtagataaagctgccgaagcggtgattatcgacacgattcgtaaatcttacccacagcacaccatcatcaccgaagaaagcggtgaacttgaaggtactgatcaggatgttcaatgggttatcgatccactggatggcactaccaactttatcaaacgtctgccgcacttcgcggtatctatcgctgttcgtatcaaaggccgcaccgaagttgctgtggtatacgatcctatgcgtaacgaactgttcaccgccactcgcggtcagggcgcacagctgaacggctaccgactgcgcggcagcaccgctcgcgatctcgacggtactattctggcgaccggcttcccgttcaaagcaaaacagtacgccactacctacatcaacatcgtcggcaaactgttcaacgaatgtgcagacttccgtcgtaccggttctgcggcgctggatctggcttacgtcgctgcgggtcgtgttgacggtttctttgaaatcggtctgcgcccgtgggacttcgccgcaggcgagctgctggttcgtgaagcgggcggcatcgtcagcgacttcaccggtggtcataactacatgctgaccggtaacatcgttgctggtaacccgcgcgttgttaaagccatgctggcgaacatgcgtgacgagttaagcgacgctctgaagcgttaatgactcaggcgggtgatatcactcacccgccctcgcctttcaggcgctattccgaaatacttcctcactgctttactttctttcgtcactctcccaccatctttccccgattaatggatgataaagaagtcgcaaggaaaggttatggcactgccagtgaacaaacgcgttcccaaaattctgtttattctctttgttgttgccttctgcgtttatttagtgccgcgcgttgccatcaacttcttctattatcccgacgataaaatttacggtcccgatccctggtcggcggaatccgtcgaatttacggctaaggacggtactcgtctgcaaggctggtttatcccttcttcgacgggccctgctgacaacgccatcgcaaccatcattcatgctcacggcaatgccggaaatatgtccgcccactggccgctggtcagttggttacccgagcgtaatttcaacgtttttatgtttgattatcgcgggtttggtaaatcaaaaggcacgccgtcccaggccggattgctggacgatacgcaaagtgccatcaatgtggtgcgccatcgcagtgatgtaaacccacaacgtctggtgctgttcgggcagagtattggcggggcgaatattctggatgttattggtcggggtgatcgtgaaggcatacgtgcggtgatcctcgactccacatttgcctcttatgcaaccatcgccaaccaaatgatccccggcagtggctacttacttgatgagagttacagcggcgaaaattatatcgccagcgtcagcccgatcccgcttttactcattcacggtaaagctgatcacgttatcccatggcagcacagcgaaaagttgtatagcctggcaaaagagccaaaacggttgatcctaatcccggatggcgaacacattgatgctttttccgatcgtcacggcgatgtttatcgcgaacagatggtggactttatccttagcgcgttgaatccgcagaactaacccatgatcgctagcacgataatcattcacaaaaccaccttaagacatgctaatccactggtcagaacagtttaagatgagaaaaattctgtgacgcttgccaacatttctgatgattagcattcccttcgccatttccttgagcaaactttagctattcttatcaattatgcttatgggagatctacagatgatgcctacgcttgctccaccatctgtcctttcggctccccagcgccgctgccagatcttgctgacgctctttcagccggggttgaccgccaccatggcaaccttcagcgagcttaatggtgtggatgatgatattgccagtcttgatatcagcgaaacaggacgggagatcctgcgctatcatcaactcacactgacgactggttatgacggtagctaccgggttgaaggtacagtgcttaaccaacgtttgtgtttatttcactggctacgacgtggtttccgtctgtgtccgtcatttattaccagccaattcacccccgccctgaagagtgaactgaagcggcgcggaattgcgcgtaacttttacgacgataccaatctacaagcgttagtgaatctctgctcccgacggctgcaaaaacgctttgaatcgcgcgatattcatttcctgtgtctgtatctgcaatattgtttgctgcagcaccacgctggaattacgcctcagtttaatccgctccaacgtcgctgggcggaatcctgccttgaatttcaggtagcgcaggaaattggacgccactggcagcgtcgggcgctccagcctgtaccacctgatgagccactgtttatggcactacttttttccatgttgcgggttcccgatccattgcgggatgcgcatcagcgggacagacaattgcgtcagtctatcaaacgtctggtaaaccattttcgtgagctgggaaatgttcgtttttatgatgaacaggggttatgtgatcagctttatacccacctcgcccaggcgttaaatcgcagtttgtttgccatcggtattgataataccctgccggaagagttcgccagactgtacccacgcctggtgcgcaccacccgcgcggcgctggccggatttgaaagtgaatacggcgtccatctttctgatgaggaaagtggtctggtcgcggtgattttcggtgcctggctaatgcaggaaaacgatctgcatgaaaaacagattattcttcttaccgggaatgatagcgagcgagaagcgcagattgagcagcagttacgcgaactaacgttactgccgctcaacattaagcatatgtcggtaaaggcatttttgcagacaggcgctccgcgtggcgcggcactgattattgcgccttataccatgccattaccgctcttttcaccaccgctgatctatacggacctgacgctgacaacacatcaacaggagcagatccgcaaaatgctcgaatcagcatgagggaacaactttcgggcgcaaaaacattgccggaagcgccaccagcgccattacccagaacacgccgtggcccagatattgatacaggaaaccggcgaaaacggtcatgatagcgatactgccgcccatcgcgacggcagagtaaaccgcctgtaaacggatgacttcgctaccctggcgagcagcaatataacgcatggcggccaggtggcagaccgtgaaggtgccgcaatgcagaatttgcaccactatcaaccacggcaacgccgtagttgctcccataatgccccagcgcactacgccgcaaatcgccgagatcaacagcatatcgcgtgcactacaacggcggaaaagtttattactcagcgcaaagataatgacttccgccaccacgcccagcgaccacaaataccccaccgccgaggccgagtagccagctgcctgccagtaaatggcgctaaaaccgtaataggccgcatgtgccccctgcaataaacaaacgcaggccagaaagcgccagttctggcgaaccagcgccaaccacgcagaccaaccggtgctctcctgctggcgacttgccccttgtggctgaatcgtcggacggatgagaaagccgagcagcatggatgccacgcccaacgtcaacagcgcgaggatcacccgataatcaaacatagtgaccagtttgcccgtcagcgccgagccaatgacaaacgccaccgagccccacagtcgcactttgccgtaatcaagcgggaactgcttttgccacgtattcgccagtgcatcggtcaacggtaccagtggtgagaaaaagaggttaaagccaatcatcaccagcatcagccacgctacgtgcgcccccgcccagaaggcgacagcaaagagaagtgtcagcagtgccagcacgcgcaaggcggaaatcaggcgggaaggatcgctgacgcggggcgcgatgagcaaactcccgaggaaacgggcaaccagacctgcccccaataacaggccgatggtttctggcgttaaaccaatccctttaagccagacgctccagaaaggtagaaaaatgccgtaactaaaaaagtatgtgaaatagccgagcgccaaccagcgcgtggattgcaaaaccatgagtccctcccgtcaggaggcgttagtctggggttaatcgaatgttggtgcaagttgaaaaataagaatattcgagcctgcttcccgatgtctgtaacgccagttcacaagcactaaaaaactgagatccgcgacgcatgttgcaaaaataatgcgtaattatgccgttacgcttgccaaacgttcctgcacaatggcgatgaaatcgcgtaatgccggcttcatctcccctttcttccacgccatcagtaaagcaatggaaggcacatttccggcaatgggacgaaaaacaacctgtccggtattaaaattattcatataaccgggtatcaaagtgacgcccagccccatgcccaccagattcatggtcaccagaatattcgttgccacctggacgatatttggctggctgttttcttgcgcaaaccacgctttaacgatcggcgcaagcgaaccggaatacaccggatcggtactgacgaaattcacgccatccagttgcgcggcggtgatctctttttcatgtgctaaagggtgatcaaccggtaacacaaccactaatggttcgtcaaaaagctccagataatcaatctccgggctataaacaggatggcgcattaagccgacgtcgagttcaccacggcgaattttttcctcctgttgcgtggtgattaaactcaccagctcaatcaaggtgtctggctgtctgagacgaaacatcggtaatacttttggcagtaaattcacttccgccgatggcacaaagccaatggttaattgtctgtcttcctgaacaattttccgcgcccgtaatttggcattttccgcttgttcgaggattgccagcgcgtcctggagaaaacattctcccgccgccgtcaacgcgactttgcgcttatccctcaccagtaacggaacaccgacacagttttcaagatcgcggatctggctgcttaacgaaggctgtgaggtatgcagtttttccgccgcacgggtaaagttcagtgcctgcgccactgcgacgaaatagcgtaaatgccgtagttccatcaccttccccttgttatcgaaaaaacgtctcagctggtagaaattaactatttcacatattagcaaccaaccagcaacatccttatggcacaaaaatagaaggtcaatacatcttatctttcaggattaaaaaatatgaccacaccctcagatttgaacatttaccaactgattgacacccaaaatggtcgggtcactccgcgtatttataccgacccggatatttaccaactggagcttgagcgtattttcggtcgttgctggctatttctcgcccacgaaagccagatcccaaaacccggtgatttctttaacacctacatgggagaagatgcggttgtcgtagtgcgtcagaaagacggcagcatcaaggcgtttctcaaccaatgccgccaccgggccatgcgtgtgagttatgcagattgcggcaacactcgcgcctttacctgcccgtatcacggctggtcttatggcattaacggcgagttgatcgatgtaccgctggaacctcgcgcctacccacaagggttgtgtaaatcccactggggactaaacgaagttccttgtgtggagagttataaagggctaatttttggcaactgggataccagcgcaccgggcctgcgtgattacctgggtgacattgcctggtatctggatggcatgctggatcgtcgcgaaggcggcaccgaaattgtcggcggcgtacaaaagtgggtgatcaactgtaactggaaattcccggcagagcagttcgccagtgaccagtatcatgctctgttcagccatgcttctgccgttcaggtattaggggcgaaagatgatggcagcgataagcgcctcggtgatggacaaaccgcccgcccggtgtgggaaaccgccaaagatgcgctgcaatttggtcaggacggtcacggtagcggtttcttctttactgaaaaaccggatgctaatgtctgggtcgatggcgcagtttcaagctattaccgcgaaacctatgccgaagcagaacaacgtttaggtgaagttcgcgccctgcgcctggcgggtcataacaatattttccccacgctttcatggctaaacggcactgccacactccgcgtctggcatccgcgcggccctgatcaagttgaagtgtgggcgttctgtattactgacaaagccgcctccgatgaagttaaagccgcttttgaaaacagcgccactcgtgcttttggtcctgctggttttctcgagcaggatgactcggagaactggtgtgaaatccagaaattgcttaaaggccaccgcgcccgcaacagcaaactgtgtctggaaatggggcttggtcaggaaaagcgccgcgacgacggcattcctggcattactaactatatcttttcagaaactgccgctcgtggaatgtaccaacgctgggccgatcttctgagtagcgaaagctggcaggaagtgctcgataaaaccgccgcttaccagcaggaggtgatgaaatgagtgcgcaagtttcactagagttacatcaccgcattagccagtttctctttcacgaagccagcttactggacgactggaaatttcgtgactggctggcgcagctcgacgaagagattcgttacaccatgcgcaccacagttaacgcgcaaacacgcgaccgccgcaaaggcgtccagccaccgacaacctggatttttaatgacaccaaagaccagctggagcggcgaatcgcccgtctggaaacgggcatggcctgggcagaagagccgccgtcacgcacccgtcacttaatcagcaactgccagataagcgaaaccgacatcccaaacgtatttgctgtgcgggtaaattatctgctttatcgggcacaaaaagagcgcgatgaaacattctatgttggaacgcgtttcgacaaagttcgccgtctggaagatgacaactggcgcttgctggaacgggatatcgtcctggatcaagcggtaatcacttcccataacctgagtgtactgttctgatgaatcgaatttatgcgtgtcccgttgcggatgtgccggagggtgaggctctccggatcgatacctcgcccgtcatcgccctgttcaacgttggcggcgagttttatgccattaacgatcgttgcagccatggtaatgcgtcaatgtcagaagggtatctggaagatgacgccacggtggagtgcccgctacacgccgccagtttttgcctgaaaacggggaaagcgttatgcctgcccgccaccgatccgctcaccacttatccagtacacgttgaaggtggtgacattttcatcgacttaccggaggcgcagccatgagcgatctgcataacgagtccatttttattaccggcggcggatcgggattagggctggcgctggtcgagcgatttatcgaagaaggcgcgcaggttgccacgctggaactgtcggcggcaaaagtcgccagtctgcgtcagcgatttggcgaacatattctggcggtggaaggtaacgtgacctgttatgccgattatcaacgcgcggtcgatcagatcctgactcgttccggcaagctggattgttttatcggcaatgcaggcatctgggatcacaatgcctcactggttaatactcccgcagagacgctcgaaaccggcttccacgagctgtttaacgtcaatgttctcggttacctgctgggcgcaaaagcctgcgctccggcgttaatcgccagtgaaggcagcatgattttcacactgtcaaatgccgcctggtatcctggcggcggtggcccgctgtacaccgccagtaaacatgccgcaaccggacttattcgccaactggcttatgaactggcaccgaaagtgcgggtgaatggcgtcggcccgtgtggtatggccagcgacctgcgcggcccacaggcgctcgggcaaagtgaaacctcgataatgcagtctctgacgccggagaaaattgccgccattttaccgctgcaatttttcccgcaaccggcggattttacggggccgtatgtgatgttgacatcgcggcgcaataatcgcgcattaagcggtgtgatgatcaacgctgatgcgggtttagcgattcgcggcattcgccacgtagcggctgggctggatctttaaggaagcacgatgaaagaaaaaacgatcattattgtcggtggcgggcaagcggcggcaatggctgcggcctcgctacgccagcaagggttcaccggtgagctgcatctgttttccgatgagcgacatcttccttatgaacgacctccactctcgaaatccatgttgctggaagattccccgcagttacagcaggtgttacccgctaactggtggcaggaaaacaatgttcatctgcattccggtgtaaccatcaaaacgctgggtcgcgacacacgagagttagtgttaaccaacggcgaaagctggcactgggatcagctttttatagcaaccggcgcggcagctcgaccgctgccgttgcttgatgcactgggagaacgctgctttaccctacgccatgccggtgatgccgccagactgcgagaagttctgcagcccgaacggtcagtcgtgattatcggtgccggaactattggtctggaactggctgccagcgccacgcagcgcagatgtaaggtgacagtgattgaactggcggcaaccgtcatgggccgtaatgcaccaccgcccgtgcaacgctatcttttacagcgccaccagcaggctggtgtgcgcattctgctcaataatgccattgaacatgtggtcgatggtgaaaaagtagaactgacgctgcaaagtggggaaacgcttcaggctgatgtggtgatttacggtattggtatcagcgccaacgagcaactggctcgcgaggccaaccttgatactgccaatggcattgtcattgatgaggcttgccgcacctgcgatcccgcgatctttgccggtggcgatgtggcaatcactcgtcttgataatggtgcactacaccgctgcgaaagctgggaaaacgccaataaccaggcgcaaattgccgctgccgcaatgttagggctaccgctaccgctactgccgccgccgtggttctggagcgatcagtacagtgataacttacagtttattggcgatatgcgtggcgatgactggctttgtcgtggcaacccggaaactcagaaggcgatttggtttaatctgcaaaacggcgtgcttatcggtgcggtcacgctgaatcaggggcgtgagattcgcccaattcgcaaatggatccagagcggcaaaacgtttgatgcgaaactgctgatagatgagaacatcgcgcttaaatcactgtaaccaggataattagcgaatatctcaatgcctggggcgtggcgaggtgcaagagtgtgtattacgtttaaatcacattatcttgcaaagggattggttatgaacacactacgttattttgattttggagctgcccgccccgttttgttattaattgcccgtatcgccgtggtcttaattttcattatttttggttttcccaaaatgatgggctttgacggtacggtccaatatatggcctcgttgggcgcgccaatgccgatgctggcagcgattattgcggtagttatggaagtgcccgccgcgatattaatcgtgcttggctttttcacccgtccgctggcggtgctgtttattttctacacgctgggtacggcggtgattggtcaccattactgggatatgaccggcgatgcggttgggccaaatatgattaatttctggaagaatgtcagtatcgctggcgcgttcttgctattggcaattaccgggccgggggcaatttctctcgatcggcgttaggaaagatgccggatgcggcgtgaacgccttatccggcatttaataaattacagccactctacccgcaacgacatctctgaagttgttgattcccctggtgctagcgcaatgagatcacccccttccgggcgatgatgatcatccggcgcatggctcatcggttccagacagaagaaatcaaacgcatatcctttatcaaacgcagggtcggaaacaaagatgaaataacacggtgcaggtggcgtcgtttccatgatgatggcataaccttcctgcggctgctcgatgcgggcctgaccattccatccggcaaaaccattgttcacccactggcgcggcaacggcgcgggctggttaaaatccagttcctgcggtagctgctcgcaaaactcacccgccagccactgctcccgctccagccagtaaccgctcgcctgtgcctgaatccgcgtttgcggcgacaacggaaaataaggatgccagccggtaccaaatggcagcgtctctgccccttgattggtgacagagagcgtcaccgtcagcgtatccgccgttaaatgaaacgcctgacttacccgatagtgatagacaccgctgcgatgttcatacaccagacacaaactatcatcgctgtgcgagacacattgccactcgcccagccagccatcgccgtgtagatagtgcgcatcccactcaacattcggttgcagttgatactcacgcccctgccagacaaaacgattgccgctcacccggtttgcaaatggcaccagcggaaaacatgaggcatcggttgccacaccgctttttttaccaggacgtaagagcggcgtcgtatcgcgccagaagccttcgattacgccgccctggtcagaaacgtccagctttagcgacccgtgggataaggtatagatggtcatccgctaactccttaatccgggaagttaatcacaactttcccgcatttgccgctcgccatcagcgcataggcatcacctgcctgttccagcgagaagcgatgggtaatggcgttacgcggccacagcttccagtccgtcagatcatgggcgcatttttccatatggaacagactggtcacccaggagccgataatccgccgttgatggtgcatcagatcggcgctgacctcgaattccacttttccggtttcaccaatgtaaaccacccgtccccagtcagcggtggattgcagtgccagcaagcgacctgcggcattaccggaacaatcgagcgcaacatccgcgccaccgtgggtgagttcggcgataatctgcggcagaccttcggtggttgctaaatagccgtgatccatcacccctaactgttttgccatcgccagacgttccggcagcatatcaacgccgatgatccgttttgcaccgcgacctttcgccagcatcatcgccatcatgccgactggccccagaccgaccaccagcacgttatcactgccggaaacttcgccgcgcaaaattccttcatacgctgtaccaacgccgcaactgataaacgcaccatcttcgtagctcagcgcatccggcaggaggatcagatctttttcttccgccagcaagtattcggcatgaccgccgtcacgctgccagccgtaagccgcttttccttcgccagtacaagaaataggaaaaccgcgacggcagttcgggcaaaaaccacagccagaaatgtgatacaccagcacgcggtcgccctctttaaaatggcggcagccttgccccatcgccacaatctgcccgcacggttcatgaccgttgataaagccctggtataacggtttatcgggtgccgccgctgtggcacggtgttgatgatagatatagtggacatcgcttccgcaaatcccggaggatttcattttgatcagtacctggttaatccccggcgtcggcaccgcaacttcccgcagatcgacggtcgaatttcctggtaaataagctgccagcatcgttttcataaatccctcattaacaatacgattaattttcatccctgccgcacccgcgccaggggcgttaaggtttagcgtttcgctttactgcttcgctgggtcagcaagatattcgccagcaccgccaccacgatgatgacgccgcgtaccacctgctggaaaaaggagttaataccgagcagcaccagaccgttaccgattagcgtaatcaccagcacaccaagcaatgtaccgaacagggaaccgcgaccgccggaaagtgccgtaccgccgaccacgaccgcggcgatgacgtcaaactccagaccgtttgcggcacctgcgttaccagaaccgaggcgcgccgccaacaaaatgccggtcaccgccgctaataatcccgaaagggtaaagataagaatgcgcacccgacgaacgttgatgccgcacaactgcgccgccgtagcattaccgccaacggcaaaaaccgagcgcccgaaggcggttttgcggctgatgaacacaaacagcgcaaacaacacaatcatgatcagcgcggataccggcacaccgagaaattgtccgcccagccagtccagcacctcgttttcatcaatcggcactggcagtgcgttcgtcataaacagccccattccgcgcagggcgctccacagccccagtgtggcaacgaaacttggtacattaaacacgccgcgcagcaccccggccagcgttcccatcagcgcgcctaacagcaacaccagcaggcacgccaccgccagcggaacttcaaattgcagcaaaaatgccaggcacaccgagacaaaagccaccatcggcccaacgctgacatcaatttcaccggagataataatcagcgtcatcgcccaggcggcaatcccaatggtggcggcatcgcgcagcacgttcatctggttattcaatgagataaagccaggcgcgttcagggagaagaccagataaagaatggcaatcaccaccagcaaaccgatctcattaatatggcgactgacaaattgtttgagcgagacgctcttgccctgcggcaatggtaatgacgaagcagacatcttcaggttcctcggtaaaattcatcagtgcacagacagaatggcggacatcagctcatccacattgaccggagcgtgaaactcctgcgagaacgtgccgtgctgtaataacaggatgcggtcacacaccagcggcaactcctccacttcactggagataaacaccacgctttttccttcggcagccagctcacggacaatacggtaaatctgctgtttggcttcgatatcgacgccgcgcgttggctcgtcgagcaacaaaatctggctggcagcatagacccaacgaccgatcaccactttttgctgattgccaccagaaagcgtgccgatgggtgtttcgctactggcggccttgaccgtcatccgctgcatcacctcttcggtcaggcggcggatggtggaccattgcagcacaccgttggcgctgattttttgccgattggtcagcactgtattttcgtcaacgcccaaccagggaatgatccccgcttctttgcggttttctggcgtatagccaatgccgcgtttcagcatgtcgccgtaatcggggcgcgtgattttctcgccgttgataacaatttcgccctgttcatactcctccagcccaacaatcgccttcagcaattcactgcgccctgcccccagcagaccagcaatgccgagcacttcgccacgacgtagcgtaaaactgatatcctccagcttgggcttatggcgtaacgcacggacttccagcacggcctgatccacaatttcctgaggggctaccggcgcaatatcaacgtgatcgcgcccgagcatcagcgacacaatatgatgcgtggaggtgttttcgagcatcacatcgcccgccacctgaccatcgcgcataacggtggcacaggaggcaatgcggcgaatttcttccatccggtggctgacataaatcaccgccacgcccagtgccgacatctttttcaccgcgctgatcaccagttcaacttccgcactcgcaagcgaactggtaggttcatcaagaatgaccacgcgcggctcgcccttcatcacccgcgcaatttccaccagctgcttttgcgccgggcttagcgttgaaacaagttgttcaggactaacgtcaacgcccagcgcctgtaagcaacgttgggcatcctgcgccatttgcaggtaatcaatcatgccgttgcggcggggccactgaccgaggcagaggttttccgccactgtcagcccttccaccagacttaactcctgataaaccgcgcgcacccccagttcagcggcacggcgagtcagcgtagcttcgtcaccttccagtcgcgtctcgccaatccagatatcaccgctatccgggcgttcgctgccggtaagcattcgaatgagagtcgatttgcccgcgccgtttttacctaacagcgcacgaacttcgcctttattgagcgtgaagttaacgttatccagcgcaacgacgccgggataacgcttatttcctgccaccacttttgctaccgggactgcctctgttgccgtgaacatagggacctctgcgaatcagcgattagggcagaccatcaacgtgcgttgccagccactgtttaccgtcttccgttttggtatagagatcgataggcacctgaatcactttttcaccgtcggcttgtttattgataaccttcaatgtttgcgcgaaaacagcattgcccattttcttaccggaaatatccactaccgctttcagcacctgattgttttccagctcctgagcaatttcggttgtcatatccgaaccgaaaacagcaatttttccggcctgattttgattacgtaccgcttttaccgcgccgagtgtcgcaccgcccgattcccccataatggcgttgagatccggcgtggagataattagtttttcaccaacggaaatcgctttatctaaaacagtcccttcctgattagcgacaatttgcgcgccgggaacgcgggattttaaaacttcttcaaatcctttacgtcgctgcacacaaacttcaaaggcttcgcaattgatgacggcaattttcggctggtcaattttattggcaataaaataatcagcggcagcgttacccagttttttaccaaattccagcggatcgccgaccagatacgccgagacatatttatcgacccccttttgattaatacaggtgttgtagcaaatcaccggaatgcccgcttcactggcgcgacgaacggtacggctactgccattttcagacactgccgataaaataatggcatcgacattacgcgccacgagggtatcaacaaaggtactttctttcgaaatatcaccctgggcgttagtttctattaactgaacttgtactgaggaatcttttgccgcatcctgaacgccctgacgcactccagcgtagtatccctgagtatcaaggtatattgcgccaatggtcatttctttttccgcagccctggcaaatagtgcgctacctaatagcgtagccattaataatagattacgggttgttctcatttttgtaggcatagagcctcctgtagggtttttattaacaacggcttattctaattattttgtgatgagcggcagcgcgtgccgctcaaatattacagttaatagggtttagtgaacgcggttaaaaataaaaggcatcacggtggtgaataatgccgctttcggccaagccggattaatcgccgtcaattcagcgcgagcagactcatattgcgcaacctccccgagtcccgcggacgccagcatcgccaccatcaggcatttttctttatgctgctgttgtaaatcgccatacagcgacaacaagtcaggttgcgagacggcaaagaaatccgcttcgatactggttttcgccatctcttgcgcccactgtttcatttcactaaacagttgctgtgcggtttgttgttcgcccagcagtcgcagcgccatcccttgccagaagagataatcaaccggctgatcgttgtaataactgtgaatgttaatagtgcgatcgccggtcgccgccagacgtaaacaacgcgtcgcttcagtttcatcgccctgcgcgttggcgcatatcgcctgccagaaccagatgtcgttatcagtttgccccggtaaacggccttcgcttaaattctccggataatgcagcgcggcatgaagcagttcgcaggcctgctgcggctgtctggcatcaagatgctgccaggcgcgtaataactggttgaggataaactgactggtgaccttcccttccccgccttcccacgggtggaatttgcgcgtggcgagaatgtccgccgctttgtctgcctgacccgtgagatgccacaaattgagcagttctgcggtcatgtcgtcgcgtttcagcgcaatttccagattattttccagacgcgccagtcgtttctccggtgtggctccacttaacttatccagcaaatcccgttcgaaaagcagacgtgcatcctgcggcgcaagctgataagcattatcaagataacgcgcggccagctcataatcgtgttgcttattccacgcatggatcgctaacccgcgccagccgtcggcaaactccggcgacatctctacgcaacgttgccaaaaggcaatggctttgttgtagctacgtttgttgtagtagaagcaagctagtaaatggcgagcaaaccagcactcttcaatactctccagcgccgccacttcttccagcgtattcgggaaacggacaaactgcgggaagacatcaatggcttttgcgaccagttcgccacgttcggctttcggcagcaagctggcttgcaggtaaagcggcagcgtgcgctggcagtccagtgcgttcagcatctctgccgccagggtgggcattccccagttaatcagttgcccggcggtcatcagggcgttaacgtcgcgtccctgacacagaccgcgccactgcgcgagagctgattcgctacgaccatcgaaccagttcagccaccacagagtggcgttcagcggataatcgcgcagcagtttctcgcgctgcacacgcgcgttgtcctgacgaccacttaacaccagcagcagattatgcaggcaaagcacttcctgattggttgggcaggcgcgaagactttgttggcaaaaatccagaccagcgtcgaagttaccattacgcgccgccagtcgtgccaggccataatagccaccggctttgctgttgccgctccagaccgcacgccagaaatcctcttcggcttgttgatattgtccctgacgttcgtaagcactggcgcgaatcaaactcgcctgtccgcactgcggatttttgttcagcgcatgtgcgcgtttcagagcctgagtggcatacgccaccgcttgcgggaaatctgcgcggttatattccagcatcgccagcgccaggttacagcgataatccagcgggtccagcgccacgccgcgcaggtagtaatcgaacggtgaacggctggcgtgatgatattgctccagatgctgaccgataaaccaggcttcatctgtactggtaatgtcttgtgctgccagtggcgctttggcgacgtccggtaacggcaacgcttgcggctgatgttcctgataactcagtacaatattgccgtcggcatcggagagctcaatggtcagcctttcaggattgataccgtgcaacacgccctggatggcggtcgcaggcatcagtgccacggcatcatcaagtaacgcgttgcatttaccgatttcgcggatcgccaggcggtatccgttcaacggagagatggcatacagcccccactcaatcccccgcttactacgctggagttttatcaccgcatcgcgggaggcattttgcaccatgcccaaagaatgataaggcaggaaatactgctcaaaacgcttctcttcgtaagcatcaagccaggtaaaatcgggctggttatcggcaaaaataccggtcatcagttcgatatacgggccgttattgtcggtcagactcttatcccacgcctggccaaattcactgtgtccccaactccactgttttttacctggcgcaatatggtggttggcaacgtgcagcaaaccgccatcttcatcgtgacaccacgcgccgacaaaatcgtactgcgatttttcggccatatatgaggttggaacaggcacatttttatagcgagaaatgtccactccagcggagtagtccactttgtagtaagtgccggtagcgatggggaaagcggagacggcccgtttgccgtgatcaaacaccgccgttacatccggcgggaagacgctctgatgcccttccccccctttcactgccgggttggcccaccacaagaaatgacgcggcgtggcgttcccgttatagacgcggctggcgatttccagcgccgcccggtcagggcgcagggtgaaacctgtcatcacctgtaaaccatgcatcggctccgtttcgcctacccacaccgtctgtgcaccgtcttcatgggcttcgagggtgaaatcaacgggcataaaggtggtcgggcgatgatgttgcggccagttaaactcaatcccaccggaaatccacggccccagcagccccaccagcgcaggtttaatgacttcattgtgataaacaaaatcgcgctgtttcactttatcccacgcgcgatgcacccgaccgcccagttccggcaggatcatcactttgatgtagtcgttttccagccacaccgcctgccaggatttcagggttttctgctcgctcagcgtatcggtcacgccgtagggataaaccgcgccggacgatccctgataaacgcgattttccaggaacatgggatgtatatcctgcggcccggtttcataggtcgggatctcaacgcgctcttgccacacttttactggagtcatggtgccctcaatattaacaagacatactgaattaaaagatttgtggcagtgtattgaacaatctggcaatgttttcgcggaataatcacgcaattaactaaacaaggtttagtgaagatgagagcctgcattaataatcaacagattcgccaccataacaaatgcgtgattctggaactgctgtaccggcaaaagcgcgccaataaatcaacgctggcccggctggcgcaaatttcgattccggcagtcagtaatattttgcaggaactggaaagcgaaaaacgggtggtgaatattgacgatgaaagccagacgcgcgggcatagtagcggtacatggctgattgcgccggaaggtgactggacgctgtgcctgaacgtgacgcccaccagtattgagtgtcaggttgctaatgcttgtttaagtccgaaaggtgaatttgagtatttacagattgatgcaccgacgccgcaggcgctgctgtccgaaatcgaaaaatgctggcatcgccaccgtaaattgtggccggaccataccatcaacctggcgttggcaatccacggtcaggttgatcctgtgaccggcgtgtcgcaaaccatgccgcaagcgccgtggacaacgccggtggaggtgaaatatctgctggaagagaagctcggcattcgggtgatggtcgataatgactgcgtgatgctggcgctggcggagaaatggcaaaataattcgcaggaacgggatttctgcgtgatcaacgttgattacggcattggctcgtcgttcgtgattaacgagcaaatttatcgcggcagtttgtatggtagcggacagattggtcacaccatcgttaatccggatggcgtcgtctgcgactgtggacgttatggctgcctggaaactgtcgcctcgttaagcgcattaaaaaaacaggcgcgggtatggctaaaatcacaaccggttagtactcaacttgatcctgaaaaactgactacagcgcagttaatcgctgcctggcaaagtggagaaccgtggatcaccagctgggttgatcgctctgccaatgccattggtttgagtctgtataacttcctcaacatcctcaatattaatcagatttggttgtacggtcgcagttgtgcctttggtgagaactggcttaatactattattcgccagacaggatttaacccgttcgaccgcgacgaaggaccgagcgtgaaagcgacgcaaattggctttgggcaattaagccgcgcacaacaggtgctgggaattggctatttgtatgttgaggcgcagttacgacagatttgatggcgcgataacgtagaaaggcttcccgaaggaagccttgatgatcataaacgaaaaattgcctgatgcgctacgcttatcaggcctacacggagattgcaatatattgaatttgcaaagttttgtaggccggataaggcgttcacgccgcatccggcatgaacaacgagcacattgacagcaaatcaccgtttcgcttatgcgtaaaccgggtaacgtgcgcagatgtcgagaactttacctttgatgcgctcgataacggcttcatcattgatgctgtccagcacgtcacacatccagccagccagttctttcgcttcggcttctttaaagccgcgacgggtaatcgccggagtacctacacgaataccggaggtcacaaacgggctcttcggatcgttcggtacgctgtttttgttgacggtgatgttagcacggcccagagcggcgtctgcttctttaccggtcaggtttttatcaaccagatcaaccaggaacaggtggttatcagtgccgccggaaaccactttgtagccgcgctcgaggaacacttctaccatcgctttagcgtttttagcgacctgctgctggtaagttttgaactcaggctccatcgcttctttcagagcaaccgctttaccggcgattacgtgcatcaacggaccgccctgaccaccagggaaaacggcagagttcagttttttgtacagctcttcgctaccacctttcgccaggatcaggccgccgcgcggacccgccagggttttgtgagtggtggtagtaacaacgtgagcatgaggaaccgggttcgggtagacgccagcagcaaccaggcccgcaacgtgcgccatatcaacgaacaggtaagcaccgatgctgtcagcgatttcacgcattttcgcccagtccaccacgccggaatatgcagagaaaccaccgataatcattttcggcttgtgttctttggcttgtttttccagatcggcgtagtcgatatgaccggtagcatcgataccgtaaggaacgatgttgtacagtttaccggagaagttaaccggagaaccgtgagtcaggtgaccgccatgcgccaggttcatacccagaacggtatcacctggttccagcagcgcggtgtagaccgcaaagttagcctgggagccggagtgcggctggacgttagcgtagtcagcgccgaacagttctttcgcacgatcgatcgccagttgttcaacgatatcaacatactcgcaaccgccgtagtagcgtttgcccggataaccttcagcatatttgttggtcagctgagaaccctgcgcctgcattacgcgcgggctggtgtagttttcggaggcgatcagttcgatgtgctcttcctgacgtactttttcctgctccatagcctgccacagttcggcatcataatcggcaatgttcatttcacgctttaacatccgcatctcctgactcagctaacaataaaatttttggcctttataggcggtcctgttggacaacggcgaacagtataaccgaatcattgtgcgataacaggtcttgacaaaggaatttacgcaaacgattaccttcaggctacgcaaggctttggagaataaagagcttgcaaccggaaacggatttcttttcaggtttgtgatgcaaatttttcacttcatcacattctttctgaaaaacaccaaagaaccatttacattgcagggctattttttataagatgcatttgagatacatcaattaagatgcaaaaaaaggaagaccatatgcttgacgctcaaaccatcgctacagtaaaagccaccatccctttactggtggaaacggggccaaagttaaccgcccatttctacgaccgtatgtttactcataacccagaactcaaagaaatttttaacatgagtaaccagcgtaatggcgatcaacgtgaagccctgtttaacgctattgccgcctacgccagtaatattgaaaacctgcctgcgctgctgccagcggtagaaaaaatcgcgcagaagcacaccagcttccagatcaaaccggaacagtacaacatcgtcggtgaacacctgttggcaacgctggacgaaatgttcagcccggggcaggaagtgctggacgcgtggggtaaagcctatggtgtactggctaatgtatttatcaatcgcgaggcggaaatctataacgaaaacgccagcaaagccggtggttgggaaggtactcgcgatttccgcattgtggctaaaacaccgcgcagcgcgcttatcaccagcttcgaactggagccggtcgacggtggcgcagtggcagaataccgtccggggcaatatctcggcgtctggctgaagccggaaggtttcccacatcaggaaattcgtcagtactctttgactcgcaaaccggatggcaaaggctatcgtattgcggtgaaacgcgaagagggtgggcaggtatccaactggttgcacaatcacgccaatgttggcgatgtcgtgaaactggtcgctccggcaggtgatttctttatggctgtcgcagatgacacaccagtgacgttaatctctgccggtgttggtcaaacgccaatgctggcaatgctcgacacgctggcaaaagcaggccacacagcacaagtgaactggttccatgcggcagaaaatggcgatgttcacgcctttgccgatgaagttaaggaactggggcagtcactgccgcgctttaccgcgcacacctggtatcgtcagccgagcgaagccgatcgcgctaaaggtcagtttgatagcgaaggtctgatggatttgagcaaactggaaggtgcgttcagcgatccgacaatgcagttctatctctgcggcccggttggcttcatgcagtttaccgcgaaacagttagtggatctgggcgtgaagcaggaaaacattcattacgaatgctttggcccgcataaggtgctgtaatttgatgttgccggatggaaacatccggcaacccttgacgcggtttaaattgccgcgtcgtcctcttcaccggtacggatgcgaatgacccgtgccacgtcaaagacgaagattttaccgtcaccgattttgccggtttgcgccgtgcgaataatggtatcgacacaggtatcgacaatgtcgtccggtacgacaatctcaattttcactttcggcagaaaatccaccatatactccgcgccgcggtacagctcggtatggcctttctggcgaccaaagcctttcacttcggtcaccgtcatgccggtaataccgacttcggccagtgcttcgcggacatcgtccagcttgaagggttttataatcgcatcaatctttttcatgctattccttgaaaaggtcgcctgtcttttgatctgctaaacgtaacacataacgccaattcattccttgaaatcgtttgcatccagctcgtgtcgggaaagcagtttataaaattctgtccggttgcgccccgccattctcgccgcgtgggtgacgttgcctttggtgatttgcagcagcttacgcaaatagttgagttcaaactgattacgtgcctcaacaaaggttggcagcgccgtattttcaccctccagcgcctgctccaccagcgcatcactaatcaccggagatgaggtcagcgccacgcactgttcaatcacgttgaccaactggcgcacattacccggccagctcgcggtcatcaggcgtttcatcgcatcggtagagaacgcgcggacaaacggtttatgtcgctctgccgcctggcgcaacaggtgatttgccagtagcggaatgtcttctgtgcgctccgccagtgccggaattttcaggctgacaacgttgaggcggtaatagagatcttcgcggaattccccgcgcgccatcgcttttggcagatcacggtgagtggcagaaataatccgcacattgatatcaatatcgcggttactgcccagcgggcgcactttacgctcctgcaacacgcgcagcagtttgacctgtaacggcgcaggcatatcgccaatttcatcgagaaatagcgttccgccttccgccgcctggaataaaccttcgcgattgctgacagcgccagtaaacgcgccacgcgcatgaccaaacagctccgactccagcaattgctcgggcaatgcgccacagttaatagcaataaatggtttgctgttgcgcgggctggcgttgtggatagcctgggcgaaaatctctttcccggtgccgctctgaccgttaatcaaaacgctgacgtctgattgcgccaccagccgcgcctgttccagcaaacgcagcatcagcgggctgcgggtgacaattgcctcgcgccagcgttcatcggtggctggcgcggattgctccagcgcatcgtcaattgcctgatatagcgcgtctttgtcgacaggcttggtgaggaaactaaaaacgccctgctgtgttgcagcaacggcatcgggaatagaaccatgcgcggtaagaataattaccggcattcccggctgcactttctggatttcagcaaacagctgcataccgtccatttcatccatccgcaggtcgctgatgactaaatctactttttcgcgattcagtacccgtaatccttcagcgccactttccgccgtgaccacactgtagccttcgctggtcaggcgcaggccaagcagtttcagcaatcccggatcgtcatcgaccaataataaatgcgcaggtttatggctcatcaggagtgacctcatgggtggatggcgcgggcttttcactctcgtgcggcgtatccggcgagaaatttccagccggtttgcgggtcgagagctggcgttcaatatcggtcaggttttccagcttgcgggtggtgagttccagttgctgctgtagaacgtgatgttgctggcgcaatgtatccagctcgctgtcgctggactgctggagtttactgtaacgttggcgctcttccgccagttgcagttgcagcgcctgaccatcgcgccagagttgatacagtgggcgaacctgtgccgggatctcggtacttaacgcttcaatacgcgcgaccagctggcggcgctcatacggcgtaattttggcgtcggcgagcaaaatcccttgtttaaaggtattttgccagctgccgtcgtcatattggcgagcttgctgacgcgactgcgcaggcattaaacgatcagcacaatccatcgcccgcagccagtaaagcggattggtttcggttgatttaccttgcagcgcccagatgtcgctacattcagtagaaagatagtcagccagttgataaaccggaattttttcttctgctggcgtatcaatggctggcttattgtgattctgcacgcaacccagcaatgccagacatggcagccctgccagccacagccgtcggggcaataatcgttgaaaaatgtgtcgcatattcaccagacttaaagcctatcccagtgggcgtaattgttgcagacagtctggacatggacagcgcggagaaaccggagcgtacatatcgtacgtgaagatttcgagcactgcccggggccgaactgacaaataaaatagcctgataggataggctgttagcattatttcgtgtttttcgacgacggtaattcaatgcggaaacaaacgtcttgcccgctctcgtcgaccagatacagttccccttgcatacggcgaatacaatccctggcaatgcttaatcccagaccgctgcccttcaccgccccttttcgctggtggcttccctgaaaaaagggttcgaagatcatggcgcgttcctcttgcggaatgggcgtgcctgtattgatgacatcaatataaacccgcgcaccatgtaaactgctgcgaaggcaaatgttaccggattcagccccgtagtgcaccgcattggagtaaagattatccagtacgctcatcagcagcattggctccgccaggcaagctgttgctttgagatcgacgtcggtatgcatcattttagcccgtgcgggcaggctatgagcagaaaccactgtctccaccagcggtgctaactcaacattctccagttccaccgcactgtccgcctgtttacggttgtaatcaagcagttgttcgatcagtttttgcaaattgcggctgctgctatcaagaatgctcaccacctctttttgctctggcgtaagcggcccgacaacctggtcagccagtaattcagtgccctcgcgcatactcgccagtggcgtttttaattcatgagataaatgtcttaaaaattgatggcgttgggattccagccatgacaggcgctcacttaaccaaagaatacgttgcccaaccgagcgtaactcgctcggtccactgaacgagacgctattgcccagagaacgcccttcccccagacggttgatcatgcgctcgatatttttcaccggcccgataatcatccgcgtgaaaagcagtaccattaccagactcaccagaaatagcaccagcgattgccaaccaaaatattgcccacgttcggcgatttcacgctgaagctgctgcccacgagagaacaccactgtgcgcgtggcctgtaccatttcggtattggcactggcaaaggcttcaagacgtgcggcggcggcagcatcgggaccgctgttgttacactgaagttgagccagattgtgcaaatcctgacgtaatgcctggtagagtttatcgtccggcagcacgcctgcgtgggcatcgagcatttcgctgtaacgcttgcgctggctttgataaaccttcgccagggttgggtcgtccagcacgcaatactgacggtaactacgctccatctccagcgccgcgttggtcatcgcttcactgcgccgggcatcaataagcgtagtgcggttaaccagcgccgcctgatcgctaagcgcattcaggctttgccaggcttgccatgccagcaccaacaggggcagcagaatcagcaaaaatgccagcattaccagttgtcgtaatgagcggggaaaaacgggccagcgtttcaaggtgttactctcgtcagacgcgaatagcctgatgctaaccgaggggaagttcagatacaacaaagccgggaattacccggctttgttatggaataaggcggtgcctaactcgacgtttcgcccgatggttgatatagctacgctgatatcagaagttggacggcaggcaccttgttgtgcgtcattcgtattttatgtagcacgtcccgaaggggctgacataagtcggtgaatgagccactggttactattatgcagtaactgtgccaataaagaaaatagtttggtaacgtactgattatacgttgctttgaggggtttatgtctcctccgctgtttgaatgtaaatcagccactgtgtcgctaaaaagagacaacttaagataaacttattagataatattaaaatcaatgagttaagtgtcgccagaaagcgacacggcaaaccacccattgtcgtgatttacagacacaaaaaagctcccggagttgggagcttatgatagtggttggtgcttaatgccgcatccgggctgcaaaaccaatgggctgacgacttaccccaactgcttacgcgcattgcggaaaatgcgcatccatgggccatcctcgccccagttttccggatgccaggagttgctgacagtacggaaaacacgttccgggtgcggcatcataatggtgactcgaccactttcagtcgtgactgccgtaataccgttcggtgaaccgttcgggttagccgggtaggtttcagtgactttgccgaagttatcgacatagcgcagtgccaccagccctttgctttccagtgccgccagatgcgccgcatcacgcacttccacgcgcccttcaccatgagagacagcaatcggcatttgcgagcccaccatcccctgcaacagcagagacgggctttgggttacttcaaccaggctgaaacgcgcttcaaagcgatcggaggtattgcgcacaaaacgtggccacaactcactacctgggatcagttcacgcagattagacatcatctggcaaccgttacatacccccagcgccagcgtttgcggacggtggaagaaggttgcaaactcatcgcgtacacggtcattgaacaggattgacttcgcccaaccttcaccggcacccagcacatcaccgtaggagaaaccaccgcacgcgaccagggcgtggaaatcttccaggcccgtgcgtccggtcagcaggtcactcatatgcacgtcgatagcatcaaagcctgcacggtggaaagctgccgccatttcaacatgcgagttcacgccctgctcacgcagtacggcaactttcggacgtgcgccagtggcaatatacggtgctgccacatcttcgttgatatcgaacgacagttttacattcaggcccggatcggcgtcgttagatttcgcctgatgctcctgatcggcacactccgggttgtcacgcaggcgctgcatctgccaggtagtttctgcccaccagacacgcaacgtggtgcggctttcgctgaatacagtctgcccgttggcggtaatcacaaaacggtcaccggaaaccgcctgccctacataatggacacaatcagcaagcccatgctgtgccagtacggactcgaccgcttcacggtcagcggcacgaacctgaatcaccgcacccagttcttcgttaaacaacgccgccaggcgatcgtcacccagagtggcgatatccgcgtcaatgccacaatgaccagcaaaggccatttccgccagcgttaccagcaggccgccatcagagcggtcgtgatacgccagcagcttacgctgtgcaaccagcgcctgaatcgcgtcatagaagcctttcagttgcgcgacatcgcgtacatctgccggtttgtcgccaagctgacgataaacctgcgccagcgccgttgcgcccagcgcgttattgcctttgcccaaatcaatcagcagcagtgcgttatcttcggtagaaagctgcggcgtgatggtgtgacgtacatcttccacgcgggcaaatgcagaaatcaccagcgacagcggcgacgtcatttcgcgctcttcgttaccttcctgccagcgggttttcatcgacatggagtctttacccaccgggatcgtcaggcccagcgccggacaaagctcttcgcccacggctttaacggcttcatacaggcccgcatcttcaccagggtggcctgccgccgccatccagttggcggaaagtttgatgcgtttgatatcgccaatttgtgttgcggcgatgttggttaacgcttcaccgaccgccagacgggcagaggcggcgaaatccagcagcgcaaccggcgcacgctcgccaatcgccatcgcttcaccgtagtagctgtcgaggctggcggtagtgaccgcgcagttagcgaccggcacctgccacggccccaccatctgatcgcgcgctaccatgccggttacgctgcggtcgccaatggtcaccaggaaggttttttccgccacagtcggcagatgcagcacacgtttcaccgcgtctgcaatggtgatcccttcacgggccagcgcgtcgcctttcgctttcagcgtttgtacatcgcgggtcatcttcggcgttttaccaagcaggacgtccagcggcagatcgatcggctgattatcaaaatgacgatcgtgcagagaaagatgcagttcttcggtcgcttcaccaatcaccgcgtagggtgcgcgctcacgcttacacagttcgtcaaacagcggtaattgatcggcagcaaccgccagcacgtagcgttcctgggattcgttacaccagatttccagcgggctcatgcccggttcgtcgcttagaatctcgcgcagttcaaatttaccgccgcgcccgccgtcgctcaccagttccggcatggcgttagaaagaccgccagcgccaacgtcgtggataaacaggattgggttggcatcaccaagctgccagcaacggtcgatcacttcctggcagcgacgctccatctccgggttgtcgcgctgtacggaagcaaagtcgaggtcggcatcagactgaccagacgccatagaagacgctgcaccaccgccaagaccgatgttcattgccgggccgccgagaacgaccagcttcgcaccgacgttgatctcgcctttttgtacgtgatcggcgcgaatgttgccgatcccgcccgccagcatgatcggtttgtgataaccgcgcagctcttcgccgttgtggctgttcactttttcttcataagtacggaagtagccgttcagtgccggacgaccaaattcgttgttaaacgccgcgccgcccagcgggccttcggtcatgatgtccagcgcggtgacaatgcgctcaggcttaccgaaatcttcttcccacggctgttcgaagccaggaattcgcaggttggaaacggagaaaccaaccagacccgctttcggctttgcgccgcgcccggtggcaccttcatcgcggatttcaccgccggaaccggtcgccgcgcccggccacggagaaatcgccgtcgggtggttgtgagtttcgactttcatcagaatatgcgccggttcctgatggaaatcgtagcggcccgtttcgtggtcagcaaagtagcggcccacttcagaaccttccattacggcggcgttatctttataagcagagagaacgtgatctggcgtggtttcgaaagtatttttgatcatcttgaacagcgatttcggctgctgttcaccatcgataacccagtcggcgttaaaaattttgtggcggcagtgctcggagttcgcctgggcaaacatatacagttcgatgtcgttcgggttacgaccaagctttgtgaaagcatcctgcagatagtcaatttcatcttccgccagagccaagccaagacgcaggttagcgtcgatcagcgcctgacggccctgccccagcaaatcaacgctggtaaccggagtcggttgatggtgggcaaacaactgctctgcatcatctaaagcaaaaaagaccgtttccatcatgcggtcgtgcagttcagcggtaacctgctgccattgttcattggtcagcgtaccggcttctatatagtaagcaacgccgcgctcaaggcggtttacctgttgtagcccgcagttatgggcaatatcggtcgctttcgaagaccagggagagatggtgccaggacgcggggtcaccagcaggagtttgccttgcggggcgtggctggcgagtgccgggccatatttcagcaggcgttcaagttgtgcgtgctcatcatcgtttaacggcgcattgaggtcagcaaaatggacatactcggcgtaaatattgtgaaccgggagcctggcagcctgaaaacgtgccagcagtttgttgattcggaatgccgacagtgcaggcgaaccacgcagaatttccatcataagtctctcgtcttctaagctttcggtgtacccaagggggggaaacgggcgtcattataaagaatctgatgcgctgacgaaaccgtttgcgtggaaataaaatcaccatcgtgaattagcaacgcgtgccgccaatggctgtaataagttgccatctggcgcaggtttacgcaaaatgccgctcatttatgagtaaacctttcactattattacgttttttcaagctgggacgcgcacgacacagagaattaactaattgaaaaaattaaagattaattatctgttcatcggcattctggcactgctgctcgcggtcgctctctggccatccattccctggtttggtaaagccgacaaccgtatcgccgccattcaagcgcggggagagttgcgtgtgagcaccattcatactcccctgacttataacgaaatcaacgggaaaccttttggcctggattacgaactggcgaaacagtttgccgattacctcggcgtaaaactgaaagtgaccgtgcggcagaatatcagccagctgtttgacgaccttgataatggtaacgccgacctgctggcggcaggacttgtctataacagtgagcgggtaaaaaattatcagcctggccctacctattattccgtgtcacaacaactggtttataaagtgggtcagtatcgcccacgtacgctgggcaacctgacggcggagcaactcaccgttgcaccgggtcatgtggtggttaacgatctccagaccctgaaagaaacaaaattcccggaattaagctggaaggtagacgacaaaaaaggctctgcggaattaatggaagatgtcatcgaaggaaaactcgattacaccattgctgattctgtcgccatcagcctgtttcagcgcgttcacccggagctcgccgtagcgctcgatatcaccgatgaacaaccggtgacttggtttagcccgttagatggcgataataccctttccgccgccctgctcgacttcttcaacgaaatgaatgaagacggtacgctggcacgcattgaagagaaatacctggggcatggcgatgattttgattacgtcgatacgcgcacatttttacgcgccgtcgatgcggtactgccgcagttaaagcccctgtttgagaaatacgccgaagaaattgactggcgtttgctggccgctattgcttatcaggaatcgcactgggatgcacaggccacttcaccgacgggtgtgcgcggcatgatgatgttaaccaaaaataccgcgcaaagcctcggcattacggatcgtaccgatgccgaacagagcatcagcggtggcgtgcgttatttgcaggatatgatgagtaaagtgccggaaagtgtgccggagaacgagcggatctggtttgccctcgctgcgtacaatatgggctatgcgcatatgctggatgcccgcgccctgacggcaaaaaccaaagggaatcctgacagttgggctgacgtaaaacagcgtctgcctttacttagccagaaaccctattacagcaagctgacttacggctacgctcgtggacatgaagcctacgcttatgtcgaaaatattcgtaagtatcagattagcctggtgggttatctgcaagagaaagagaagcaggctacagaagcggcgatgcaactggcgcaggattatccggcggtatcgcctacggagttgggcaaagagaaatttccttttctctcgtttctttcccagtcgtcatcaaactatttgacccattctccctctctgctgttttccaggaaagggagtgaagagaaacaaaattaatccgtcgaggattgcgcttttttctgcgctttaatttcctggcggcgcatgcgaaagaagtcactgagcaacgccgcgcactcatccgccagtattccttccgtaatttccactcggtgattcatacccggatgatgcagcacatccattaaagatcccgcagcgccagttttcgcgtcacgcgcaccaaagaccacgcgaccaatgcgactgtggatcatcgctccggcacacattacacatggttcaagcgtgacatacaacgtggcgtcgatcagacgataattttgcatcaccagaccaccctgccgcagggccatgatttctgcatgtgcggtgggatcatggcgaccaatcgggcggttccagccttcgccgattacccgattgttatgcactaataccgcgccgaccggcacttcccgctcatcccaggcacgtttcgccagcgtcagcgcgtgacgcatccagtattcgtggctaaattcgacttcagacaaaaagaaaactccggttataaaagcgcggcgcattatacacggacgctatgctttactctattccagttgctggagttcaccgcgcggggttactcgccaacgatgctgacagaaataaagcagcggattgtcctgattactgtcgctatagccactgtacagccgcagcggagtgccgattttgcgctccagttgtgcgaccttttcatgtcccagacaacgcatcgtcaatacccaaccaccatagccacgctgaatttggctggcgataagattaacccgcggcagccagggcgtatcgaaataaaccgcttcaaccagcggctgcggagagccggtaatcaaccagatatcagcatcggaacttaacaggtaggtggttaatcgctcctgaaccagcggaaaggcggtaacattgtcgcgaaaccagcgcacgaaatcggcctgcaacgtctgtaaacgtgcttcgctgtgaccaaaagtgcacccccacagaagcagactcatcggccagcgtgccgcacgaccttttatcaataacgcaatggctataatcggtaacaacggcaggacaagtaacgcattcagcggttggcgacgtagtaaatagcgcagaaaactgccgaacatatcctgctgatgcaatgttccatctaagtcaaaaaacaccacacgacgctcgtgagttgccaaaccatactcctctggactgaaacatcctgattaattttcgctactacatagcctaacagatagatcatcacttttccggcaacaatcgaccgcatcatggctaactggaatttttaattcatggcaattagcggcaatggaatataaaattcactcgcgtgtgtctcatattgcctgttgtcgccactatttcatcgcgaggaaagatatgaacggcttacttcgtatccgtcagcgttaccaggggcttgcccagagtgataaaaaactggcggattatctgctgctacaacctgatacggcgcgccatttaagctctcagcaactggccaacgaagccggagtcagtcagtccagcgtcgtgaagttcgcgcaaaaactcggctataaaggttttccggcgcttaagttggcgttgagtgaagcgctggcaagccagccggaatcaccctccgtgcccattcataaccaaatccgcggtgatgatccgttacggctggtcggcgaaaaactgattaaagaaaatactgccgctatgtacgcaacgctaaacgttaatagtgaagagaaactgcatgaatgcgtaacaatgttgcgctctgcgcggcggataattctgaccggtattggcgcttcgggtctggtggcgcaaaactttgcctggaagctgatgaagattggcttcaatgctgccgcagtgcgcgatatgcatgcgctactcgcaacagtacaggcgtcgtcccctgacgatctgttattagccatttcctacaccggtgtacgacgcgagttaaacctggcggcagatgagatgctgcgagtgggcggaaaagtgctggcgattaccggctttactccgaatgccctgcaacagcgtgcttctcattgcctgtataccattgccgaagaacaagcgacaaacagtgcttcaatctctgcttgtcacgctcagggaatgttaacggatttgctgttcattgcgctgattcagcaggatctggaactggcaccagaacgtattcgtcatagtgaagcgctggtgaaaaaactggtctgagtaaagaatgcgcgtataatgcccgcccggtttgtgttgttttgagagtttccttatggcgttgttaatcactaaaaaatgcatcaattgtgatatgtgtgaacccgaatgcccgaatgaggcgatttcaatgggagatcatatctacgagattaacagcgataagtgtaccgaatgcgtagggcactacgagacaccaacctgccagaaggtgtgcccgatccccaatactattgtgaaagatccggcgcatgtcgagacagaagaacagttgtgggataaatttgtgctgatgcaccacgcggataaaatttaatattctactctggaagtagagtattaattatattactgggaagccttaacgccattatatttatttaattgatgacattagcataatcattcactaagttaatttatatagtatctgcccagacacttatttatagttattaaaggtgcgtccgactggttcaccggacgcaccttaagtacgtttccttgtgttataagaacagaaggatcagctgtaaaacagcaatgatgattttgatgacccgtttaatcaggtatcggcaatcagtcattcgtttttccttaaacaaggaatgcagccattcagattagcccttacatctccccaaaactgaacgtgcgagttattgagggtgcatgctgcactccacaccagagctttgacgacaccactcgtttcaatgggggaattctgtggcatggtgtaaagcacagcaaaatcttcaataacgaagccaattttaatgtacttacgaattggcggtcacgttaatctttccatcaatattgctttcttcgtaaaggctcgagtttttatgctaaagattgcaagttgcttgtaaaagataagtacactgatccataatcgctgttgttgagggtgcatgctgcacaaaattaaagttaaaaagtaaaacccccgttccttaccagttcgggggttttactttttaaagagaacggtattatttttaactttcaataattaccgtggcacaagcatagtgccgctcatctgccagcgttacatgcatatttgcaacgcccagcttttccgccagttttaatgcctcgccccatagccgtagccgtggtttgccgagctcatcattgaatacttcaaattgattaaacgccagaccattgcggatcccggtgccaaacgcttttgctgcggcttctttcacagcaaaacgcttcgccagaaaacgcaccggctggtggtgcgttttccagatagcccattcgttatcgcttaatacgcggcgtgccaggcgatcaccggatcgggcgatcaccgcttcgatgcgagcgatctccacaatatccgtgcctaaacctaatattgccattagccacgcgcttccagcatcagacgcttcatttctgccaccgcatctttcagtccggtcatcactgcacgaccaataatggcatgaccgatattcagttcatgcatctcagggatggcggcaatggctttcacgttgtgataggtcagaccgtgtccggcgttaactttcagaccgaggcttgcggcaaaggtcgcggctttggcgatacgcgccagctcttgcgcctgttcggcgtcagttttggcatcagcatagcaaccggtgtggatctcgataaacggtgcgccaacctctgccgcagctttgatctgctcttcatcggcgtcaataaacagagaaacctgaatcccggcatctgccagacgtttgcaggcatcgcgcattttgtcacgctgccctgcgacatccaggccgccttcggttgttacttcctgacgcttttccggtaccaggcagcaaaaatgtggcttcgtctcaacggcgatcgccagcatctcttcggtcaccgccatctccagattcatgcgggtatccagcgtctgacgcaggatgcgcacgtcgcggtcagtaatgtgacggcgatcttcacgtaaatgcacggtaatgccgtccgctcccgcctgctcggcaataaacgcggcctgcaccggatccgggtaagcggtaccgcgcgcgttgcgcagcgtagcgatatggtcaatgttgacgcctaacagtaattcagccatgacaatcctcatcattcataatgtgttttcaccgttcgcttaggcataaactgccggaacagttccctgctctttaaaggtttaccgccaagatacggcttaagcgccatgcgggtaaagcgtttcgcggcgcgcagtgtgtctgcgtcaggaaattcccgtgcgtttaacgcttttaactgccttccggtgaacgttttattgtcgataacgacgcttgcgataaaccctttttcttcgcgataacgatacgtcatggtgtcatctaccggctcgccgctacccgcacaatgggtaaaattgacgccataacccagatgcccgagcagtgccagttcaaagcggcgcagcgcgggttctggcgtaccagtgacccctgcaagagactgaatgcagtgcaagtaatcgaaaaaaagttcagagaagcgcgtctcgtattccagtacgcgggagagaagttcgttgatgtacagaccgctgtaaagcgtgataccgcttaatggcagcgccagcgagacggcttcagcactgcgcagcgttttgacttcgccacgcccgccaaaacgtagcaagagaggggtgaaaggctgtaatgcacctttcagggtagagcgtttagagcgtgcgcctttggcaaccagacgcacgcgccccgattcctccgtgaagacgtccagcatcaggctggtttcgctccacgggcgactatgcaggacaaatgcgcgctgccagccttccatcggagttactcttaaagatcgtcaacgtaaccgagactgcgcagtgcgcgttcgtcgtcggcccaaccggatttcacttttacccacagttcaaggtgaacaggcgcttcgaacatttcctgcatgtctttacgcgcttcaatcccgatggttttgatcttggcccctttgttgccaatgaccatcttcttctgcccttcacgctcaacgagaatcaaaccgttgatgtcataaccaccgcgttcgttagagacgaaacgttcgatctccacggtcacggagtacggcagttcagcgccgaggaaacgcatcagtttttcgcggatgatttcagacgccataaaacgctgtgagcgatcggtgatgtaatcttccgggaagtgatgagtcgcttcaggtagatgcttacgcacgattgccgcaatagtgtcaacattcagcccggtttcggcagagattggcacgatatcgaggaagttcatctggcttgccaggaactgcaggtgcggcagcagatcggctttctcctgcacgttgtccactttgttcaccgcgaggattaccggcgctttgccttcgcgcagtttgttgagcaccatttcgtcgtccggcgtccagcgggtgccttcaacgacaaaaatcaccagctcaacatcgccaatagagctgctcgccgctttgttcatcaggcggttaatggcgcgtttttcttccatatgcaggcccggtgtatcgacgtagatcgcctgatacgcgccttcagtatggatccccacaatgcggtgacgagttgtctgcgccttgcgggaagtgatggagattttctgccccagcagtttgttcaacaatgtggatttgccaacgttcggacgtccgacgatggcaataaatccgcagtaacttttatcgatgctcattccagctccagttttttcaacgcctgttcggcggcagcctgctcagccttacgacggcttgaacctgtgccaaccaccggttcactcaggccgctgacctggcagtggatagtaaattcctgatcgtgcgcttcgccacgtacctggactaccagataagtcggcagcggcagatggcgaccctgcaaatattcttgcaagcgcgttttcggatctttttgtttatcgcctgggctaatttcgtccaaacgagtttgataccagttgaggattaatttctcgacggtttgaatatcactgtcgaggaatacgccaccaattaatgcttcgacggtgtcggcgagaattgactcacgacgaaatccaccgcttttaagttcacctggccctaaacgtaagcactcgcctaactcaaattcgcgcgccagttccgccagcgtattgccacggaccagcgtggcgcgcatccggctcatatcgccttcatccacacgagggaaacggtgataaagcgcattggcgataacgtagctcagaatagagtcgcctaaaaattctaaacgctcgttatgtttactgctggcactacgatgagttaatgcctgctgcaacagttcctgatgattaaaagtgtagcccagcttccgttgaagccgattaattacgatggggttcatgcgataccaataaataaatgcgtcaacaattcagcacacgaaacagacctgatatacatggttctgctaactgcttcgctgcagtttcagtttaccggtatatggggaccaacgctgtttcgtgtgccgtggcaacctggaggtgccaaccttaaacttcgggggaatattctatacacaacgacgggggatgtcgttagccacgggagatttatctcataaataattcacgttgtcgccataacggcgacaacgtgaacgaagatggctattaatggatgccgccaatgcgacttaagcgcagaccagtcggccattcgccttcttgcttatcgaagctcatccagatagccgttgcccgaccgaccagattcgcttccggcacaaagccccagtaacggctgtccgcgctgttgtcgcggttgtcgcccatcatgaagtattgtcccggaggaacaatccaggttgccagttgttgccctggctgctggtaatacatccccacctgatcctgcgcaatcggcactgtcagaatgcggtgcgtcacatcacccagtgtctctttacgctcggaaagacgaattccattttctttggtttcgtttttcggcacttcaaagaatccgctggtcgcttccccaccattacggcgtgagaaggtctgaacgaaatcgctcggttccacgtttgagtaggtgaccggcagcgcgttttcacacgcctggccggaactgcatcccggttgaatcgtcagctcttttgagaccggatcgtaagtgactttatcgcccggtaaacccaccgcgcgcttgatgtaatcaagctttggatcttccggatatttaaagaccacgatatcgccgcgtttcggatgaccggtttcgatcagcgttttctggtagataggatctttaatgccataagcaaacttctctaccagaataaaatcaccaattaacagagtcggcatcatcgaacctgacgggatctggaacggttcataaataaacgaacgcacaatcaatacgatagccagtaccggaaaaacagaagcaccggtttccagccagccaggcttcggcgcaacctttttcaacgttgctttatccagtgagtccccggcagccgcctgcgccgctgcctgacgttcccgccgtttaggtgcgaaaaagaatttatccacgcaccataaaatgcccgtcaccagtgtggcaatcaccagaatcagggcaaacatattcgccatgccaactcctaagggttatttgttgtctttgccgacgtgcagaatggcgaggaacgcttcctgcggcagctcgacgttaccgatctgcttcatgcgtttcttaccttctttctgcttctgcagcagctttttcttacggctgatatcgccgccataacatttagccagtacgtttttacgcagctgtttcacggtggatcgcgcaatgatgtgcgtaccaatcgctgcctgaatggcgatatcaaactgctggcgtgggatcagatctttcatcttctccaccaactcgcgaccgcggttttgcgaattatcacggtgggtgatcaacgccagcgcatcaacacgttcaccgttgattaatacgtctacacgtaccatgtcggacgcctggaagcgcttgaagttgtaatccagagacgcataaccacgcgaggtagatttcaggcgatcgaagaagtcgagcaccacttccgccatcgggatctcgtacgtcagcgccacctgattaccgtggtaaaccatattggtctgcacgccgcgtttttctacgcacaacgtaataacgttgccgagatatgcctgcggcagcagcatgtgacactctgcaatcggctcgcgcagttcgtagatgttatttaccgcaggcagcttggatgggctgtcgacgtagataacttctcttgacgtggtttcaacttcatacactacggtcggcgcagtggtgatcagatccagatcgtattcacgttccagacgttcctggatgatctccatgtgcagcaggccgaggaagccgcagcggaaaccaaagcccagcgcgctggagctttccggctcatagaacagtgaggcatcgttcaggctgagtttacccagcgcgtcacggaaggcttcatagtcgtcggaacttaccgggaacagaccggcgtatacctgcggtttgactttcttaaagccaggcagcgccttttctgccggattacgcgccagcgttaaggtatcgccgactggagcgccgtggatatctttaatcgcacatacgagccagcctacttcgccacatttcagttcagtgcggtcaacctgtttcggcgtgaagatgcccagacggtcggcgttataggtctgcccggtactcatgactttcactttgtcgcccttacgcagggtgccgtttttaatacggataagtgaaacaacgcccaggtagttgtcgaaccatgagtcgataattagtgcctgcaacgggccttccggatcgccttccggcggcggaatgtcgcgcaccagacgttcgagaacgtcctgcacaccaacgccggttttcgctgaacagcgcaccgcgtcggtggcgtcgatgccgacgatatcttcaatttcttccgccacgcgttcaggatcggctgccggcaggtcaatcttgttcagtaccggcacaacttcgagatccatttccatggcggtgtagcagtttgccagggtttgcgcttctacgccctgcccggcgtcgaccaccagcaatgcaccttcacaggcagccagcgaacgggaaacttcataggagaagtctacgtggcccggggtgtcgataaagttaagctgataggtttcgccgtcagacgctttgtagtccagcgtcacgctttgcgctttgatggtaatgccacgctcacgctcaagatccatggaatcgagaacctgcgcctccatttcacggtcagacaggccaccgcagatctggataatacggtcagacagcgtcgatttaccgtggtcaatgtgagctatgatcgaaaagttacgtatattcttcataaagtatgattattgtgccttaatgcccggttaaccaggcttttagaagtcgctgttctgagcttaacgtctgtattaatagaaacgccgcattctacactacaacattgaggcgaggaaatgttcataccgtatggattgtggtatctggaaacgtcctcgcatttgttatgcaaaatgcaacaaagccagtgaaatcactggctcgcgtcttccgaagatgtttcaaatcgcacaaggccaggcggcaatgccacgcttaagatgatcggttgccattctgcccgggcagcaaacttacgcgagtagccgcgcgcaatcaggaacccgccaataccaccgaggatcgcaccacataatgctgcgacgtcagaagcaaagagtagctgaaatagcgaagcgataaggaataatcccaccagcggcgacatataaaccagtaatgcggagctaagcaggctgccttcggcgatccccaattccactttttgccccggcactaacggctcatcacagggtacgacaatggtatgcgtggtttgcgggccaagtttatttaacacgcggctaccgcaaccggcgcgtgaagcgcagctgctgcatgaagctttaacatcacaactgaccagcgcctgcccgttttgccaggagacgacggtagcccactctttgatcattgcgctgccccgaacttaatattctcggcaatgcgtttcgccgtttgcggcggcagttcaccgacaatggtgatttcggcgttatcacgtacgcttgtactgacggttctgcgtccggtgcgcaacatctgatcggtgctcgatggcgtagcgcggttaacgtttaccgagaagctgaataatccgtcggaatagagacgtgattcgataggcatgttgtccatcgtcggtagcggacgtcgactactggaaacttcgctaaaaccctgtggcaaccaggttggcgtccagctgaatttagctttttcacctacaggaacagaaagcaacggcggcaaatttgccttcgccagcgtctgcatactgctgctgatatcctgattgacgttaaaagcaatcacgcgaaattgttccagcgtttcaccatcgcgatcaaggagatcaacccgcatcggtaatttcgattcggtgtccatccacacgatgtagctgtagcgtgtaccatctcgggcaaccacgcgaatgacttcgcaaagacgatcagcaatacgcgtgcgcccgacggagataaagtcgtagtaaggagaaaggcgtttgaaatcggtatagataagcgatggcagagaatcaacaatgtaatcgccattaagcgtgaacggttcaagtcccggttcaaaatagctgatttcattgccgcgctgtaccacttcccggcgcgggccatccatttgcaacaattgtgcaagaggacggttatcgaggcgtgcatgtcgataacgcagagactcaacaccctgtttattgatgctgatgaatgacagctcgtaattcagtgactgactggccaggttcatctgctgtaataacgccccggacgcgggagtggccgaggcgttagcagagaataacaggctacctgtcactaatgacatggcaaaccaaagttgcttcattactgcgattgcgttcctaaagtttgaattcctggcacctgtacagcggcttgctgggtttgcgcctgctcaaactgaagctgttcagagtggagtcggcgttgcagttcgtaatcctgcaacattgcattaatgcgacgacgctgctcctgtacctgctgctgttgaccattgtttgcggtcgcttcagaaggtactcccaggcttaccgggctggctttacccatcatcggcagtgtattaaataccggcgtttcgggctgctgggacgtttcagattgtccattatagtgctggacgccaacgataactgcaagcgatacgcatgcggctacgcccatttgggtaagctgtgccgcccacggacgtactttctgccagaatggcattttctgccattgatgcggcgcaggctgggcttccgggatcaatgtcgccggttgacgtactggctcttcttcaatggcggccatcacgcgtgaagagatatcgaaatggagcacctcgggagtatcaccccgcattgagtcacggattaagtgatagctttcccaggttttctgcatttctgggttatgagccagttcgttaagcagctcactatccagcgtttcgccatccattaaagcggaaagttgttctttctgcatgcctaatacccttatccagtatcccgctatcgtcaacgcctgataagcggttgaactttgttatcaatagcttccctcgctcggaagatacgtgaacgcaccgtacctaccggacaatccatgatagcggctatctcttcatagctcaggccatccagctcccgcaaggttattgccatgcgtaaatcttccgggagggactcaatagttcggaaaactatctgtctcagttcttctgacaacattaagttctcagggttcgaaatttctttcaacgcgccgccactttcgaagttttcagcttcaatggcatccacatcactggaaggtggacgacgcccctgagcaaccaggtaatttttcgctgtatttacagcaatccgatacagccatgtataaaaagcgctatctccccggaacgaatccagcgcacgataggctttaataaaagcttcttgtaccacatcgggaacatcacccgacggcacatagcgggaaaccagactcgccactttatgctgatagcgcactaccagtaagttaaaggctttctgatctcccttctggacccgttcaaccaggacctggtccgttaactgctcgctcatccgaggtaaagtctccccaaaccaaatttccacgcgctatcgaaacgccactccattagctgcaatttgagcaagcaaagggttagagtgtctcgtttttgtaaagttccgtaacgcatctgtttttgtttgtcatgctgtagacggatcattatctatcattataagtctacagaatctgaacatcgcattatctgtgtagaaatgcccatttaactgcctgaagagtaacccaacggcctttttatttcaccacctaatcctccaccagccagtaacttctctttttctcgccgccctgcgtcagcgtgtttagcaactgtaacaaatattaaaatagcaggtgtttatccgcacaacatgatgctatgctgaccaaaccatgtttagtaaattaaacaaagaaaatgaatactctccctgaacattcatgtgacgtgttgattatcggtagcggcgcagccggactttcactggcgctacgcctggctgaccagcatcaggtcatcgttctaagtaaaggcccggtaacggaaggttcaacattttatgcccagggcggtattgccgccgtgtttgatgaaactgacagcattgactcgcatgtggaagacacattgattgccggggctggtatttgcgatcgccatgcagttgaatttgtcgccagcaatgcacgatcctgtgtgcaatggctaatcgaccagggggtgttgtttgatacccacattcaaccgaatggcgaagaaagttaccatctgacccgtgaaggtggacatagtcaccgtcgtattcttcatgccgccgacgccaccggtagagaagtagaaaccacgctggtgagcaaggcgctgaaccatccgaatattcgcgtgctggagcgcagcaacgcggttgatctgattgtttctgacaaaattggcctgccgggcacgcgacgggttgttggcgcgtgggtatggaaccgtaataaagaaacggtggaaacctgccacgcaaaagcggtggtgctggcaaccggcggtgcgtcgaaggtttatcagtacaccaccaatccggatatttcttctggcgatggcattgctatggcgtggcgcgcaggctgccgggttgccaatctcgaatttaatcagttccaccctaccgcgctatatcacccacaggcacgcaatttcctgttaacagaagcactgcgcggcgaaggcgcttatctcaagcgcccggatggtacgcgttttatgcccgattttgatgagcgcggcgaactggccccgcgcgatattgtcgcccgcgccattgaccatgaaatgaaacgcctcggcgcagattgtatgttccttgatatcagccataagcccgccgattttattcgccagcatttcccgatgatttatgaaaagctgctcgggctggggattgatctcacacaagaaccggtaccgattgtgcctgctgcacattatacctgcggtggtgtaatggttgatgatcatgggcgtacggacgtcgagggcttgtatgccattggcgaggtgagttataccggcttacacggcgctaaccgcatggcctcgaattcattgctggagtgtctggtctatggctggtcggcggcggaagatatcaccagacgtatgccttatgcccacgacatcagtacgttaccgccgtgggatgaaagccgcgttgagaaccctgacgaacgggtagtaattcagcataactggcacgagctacgtctgtttatgtgggattacgttggcattgtgcgcacaacgaagcgcctggaacgcgccctgcggcggataaccatgctccaacaagaaatagacgaatattacgcccatttccgcgtctcaaataatttgctggagctgcgtaatctggtacaggttgccgagttgattgttcgctgtgcaatgatgcgtaaagagagtcgggggttgcatttcacgctggattatccggaactgctcacccattccggtccgtcgatcctttcccccggcaatcattacataaacagataaaaagcctgggtcagcgccgtatacgcttcggaatagttctggtctggcccacgaatgactaagcgatcgctaaagcattctcccgcctgcggggagaatgccagcagcacccgatgcggcagtcgcgcttcgttttccgccacatccgtccgcaaacgtaaatgccagcccatgcttaatgccagctccgtaaaaccattaccaatctgctctggcagcactacgcagaaaaatccctcttcggtaatgcactccgccgcacaggtcagcaacgatgggtgatcaagcgtagtggtatagcgagcctgttcccgttgaggtgtcgagcactctactccctgctgatagtaaggtgggttactgatgattaaatcgaagcgtactgtctgctgtgtgatccactgctgaatatccgccgtatggacgttaatccgctctgcccacggggactggttgatattttcctgcgcctgcgcggcagcttcactttccagttcaactgcatcaatcatcacgctgtcatcggttcgctgcgccagcattaatgccagcaacccgctacccgcgccgatatcaaggcaacgttttaccccagccaccggtgcccatgcgcccaataaaataccatccgttcccactttcatcgcacagcgatcgtgagcaacaaaaaactgtttaaaagtaaatccattacgacgaagcacggatgtagactgtgacatgaaaataaaaccttgcaggaaaaacggcgatagcaccgggtgagaacaatacccgagaagcgatatccatacaaacagatgaagattgcagccgtaacgtctataatcagcgccccacacagaggtagaacatgactgtaacgactttttccgaacttgaactcgacgaaagcctgctggaagccctccaggataaaggtttcactcgcccgaccgccattcaggctgccgccattccgcctgcgctcgatggccgtgatgtactcggttctgcgccgacaggcaccggtaaaacggcggcgtatctgctgccagcgttgcagcacctgctcgatttcccgcgtaagaaatccggtccgccgcgtattttgatcctcaccccaactcgcgagctggcgatgcaggtgtccgatcatgcccgcgaactggcgaaacatacgcatctggatatcgccaccatcaccggcggcgtagcctatatgaaccacgcggaagtgttcagcgaaaatcaggacatcgtggtcgccacgaccggacgtctgctgcaatacataaaagaagagaacttcgattgccgcgcggttgaaacgctgatcctcgacgaagcagaccgtatgctggatatgggcttcgctcaggatatcgaacatattgctggcgaaacgcgctggcgtaaacagaccctgctcttttcggcaacgctggaaggcgatgcgattcaggactttgccgagcgtctgctggaagatccggtggaagtttctgccaatccctccacccgtgagcgcaaaaaaattcatcagtggtattaccgcgccgatgatcttgagcataaaaccgcgttgctggtgcatctgttaaaacagccggaagcgacccgctcaattgtgtttgtgcgtaagcgtgagcgtgtgcatgagctggcaaactggctgcgcgaagcgggcatcaacaactgctatctcgaaggtgagatggtacagggcaagcgtaacgaagcgatcaagcgtttgaccgaaggtcgcgtaaacgtactggtcgcaaccgatgttgccgcgcgcggtatcgacattcctgacgtcagccacgtctttaacttcgatatgccgcgcagtggcgatacttatttgcaccgtatcggacgtaccgcgcgcgccggtcgtaaaggcaccgcaatttcgctggtggaagcccatgaccatctgctgctgggtaaagtaggccgctatattgaagagccaattaaagctcgcgttattgatgagttacgcccgaaaacgcgtgcgccaagcgaaaagcagaccggcaagccatcgaagaaagtactggctaaacgtgctgagaagaaaaaagctaaagagaaagagaagccgcgggtgaaaaaacgccatcgcgacaccaaaaatattggtaagcgccgtaaaccaagcggaacgggcgtgccaccgcaaacgacagaagagtaatctcaatgccaggtttaagcctggtattaaaagtgctggcaaacgcaaaactgcctgatgcgctacgcttatcaggcctacgtggctcatgcaatatattgaatttgcacgatcttgtaggccggataaggcgttcacgccgcatccggcatgaataaagcgcactttgtcgacaagttaaatgccgggtttaatcccgacattatttttatccagccacaaaactctcttcaacacactgaataaaagtgtgcatcgccgggctaaccgcttttccagcatgatgtgcgcacatggccgtaatggtctgcgactgttcgccaaaaggcaattcaattaattctccgcactccaactcttttgccaccgcaaagcgcggtaggtagctgaccccgatattcgccgcgacacaacgcttgatgctttcgatacttataagctcaatggtgttttccaccgtgatccgccgctgacgcagcgtgctctcaaatatctgccggaagacacattgcggttcgttgataataaagctacaggcgttatgtcttcccggctcagtaaaatcgacatctgcaatttgcggtgaagccaccagcaccagtgattgttcacccaactctcgtcgattcagagcatcatcattccctacacgataaaagacgccaacatcggcctcatcattcagtagcgcatcacggatcacgtaacagttcagcgactgcaacgataaacgcacttttggggcgcgttgccgaaaacgctgcaacacctgcggcattcggtaagagagcaacgtttcgcccgaaacaacgcgtagttccccgtccggatctgactcctttttggcagcctcacgaagcgtatccatcactcgggtaagttcataaatgtgcggcagcaacttttttccttcgcgggtaaggcacatccgtcggccaattttctcaaataactggactgaaaactcctgctcaagctgctgaatatgaaaagtcaccgtcgattgtgtacagcacaatttttgcgaagctcgcaaaaaggaaccctcttccaccacggttttaagcgtaataaaacggcgcagatccataaccccaaacctatcgaaaatatcgaatctagaatataaaaacattcatttttttaaatgttccgtgtcgggtactgtctaccaaaacagaggagataacaagtgacaccgacccttttaagtgctttttggacttacaccctgattaccgctatgacgccaggaccgaacaatattctcgcccttagctctgctacgtcgcatggatttcgtcaaagtacccgcgtgctggcagggatgagtctgggatttttgattgtgatgttactgtgtgcgggcatttcattttcactggcagtgattgacccggcagcggtacaccttttgagttgggcgggggcggcatatattgtctggctggcgtggaaaatcgccaccagcccaacaaaggaagacggacttcaggcaaaaccaatcagcttttgggccagctttgctttgcagtttgtgaacgtcaaaatcattttgtacggtgttacggcactgtcgacgtttgttctgccgcaaacacaggcgttaagctgggtagttggcgtcagcgttttgctggcgatgattgggacgtttggcaatgtgtgctgggcgctggcggggcatctgtttcagcgattgtttcgccagtatggtcgccagttaaatatcgtgcttgccctgttgctggtctattgcgcggtacgcattttctattaacgaaaaaaagcggaagaggtcgccctcttccgcttagtaacttgctacttaagccttacaggctttcagtaaaggtacgagcgataacgtcgcgctgctgttccggagtcagagagttaaagcgaactgcataaccggatacacggatggtcagctgcggatatttttccggatgcttaactgcatcttccagagtttcgcgacgcagaacgttaacgttcaggtgttgaccaccttcaacgcgaacttctggtttcacttctactggaacttcacggtattcaatgtcacccagtttgcttactgcaaccacttcatcttctgcataacctgcttttgcaacgatgcaacgcgcttcgcctttttcgctgtccagcagccagaaagagttcagcagatcgtcgttagcggctttagtaatctggatacctgtaatcatgtgatgcctccccggcaaaattatttgatttgttcagcctgtcgcggccaattggtaaaaccattgttgcttgagtgtatatatactcctcaaacacccttgaatctttgatttaaatcaataaaaaccacacatcaagtatggtcgcaaatggattttattgttttacatcaacttatgcgggtgtgaaattttaccaatttacatttttttgcactcgtttaagtctaaaaaatgagcatgattttgttctgtagaaagaagcagttaagctaggcggattgaagattcgcaggagagcgagatggctaacgaattaacctggcatgacgtgctggctgaagagaagcagcaaccctattttcttaatacccttcagaccgtcgccagcgagcggcagtccggcgtcactatctacccaccacaaaaagatgtctttaacgcgttccgctttacagagttgggtgacgttaaagtggtgattctcggccaggatccttatcacggaccgggacaggcgcatggtctggcattttccgttcgtcccggcattgccattcctccgtcattattgaatatgtataaagagctggaaaatactattccgggcttcacccgccctaatcatggttatcttgaaagctgggcgcgtcagggcgttctgctactcaatactgtgttgacggtacgcgcaggtcaggcgcattcccacgccagcctcggctgggaaaccttcaccgataaagtgatcagcctgattaaccagcatcgcgaaggcgtggtgtttttgttgtggggatcgcatgcgcaaaagaaaggggcgattatagataagcaacgccatcatgtactgaaagcaccgcatccgtcgccgctttcggcgcatcgtggattctttggctgcaaccattttgtgctggcaaatcagtggctggaacaacgtggcgagacgccgattgactggatgccagtattaccggcagagagtgagtaaatttgcggggaaatgccggatggcagagttgccacccggctgatttatcaggctttattctgacgccaccattcaccaagcaaaacgccggttgcgacagagatattcagcccggcaacgttgcccgtaccgtcaatcttcacgcgcagatcgttcggatcgcgtgcggcatccggtaacccttcatattcctgacccagcaccagtaccattttcgctggcagactagttttgaacagcggtttaccctgctcgctggaagtggtcactacggtgtaacctgcctgacggaaatcatccagcacgttaacaatgttgtcgccagtaatcggctgaacgtgctctgcgccgccttctgcggtacggatagccgcccccgactccagcagtgccgcatcctgcaccacgacacctttcacgccgaagtgcgcgcagctgcgcatcatgccacccaggttatgcgggttagattcgttttccagtgccagaacgcaatcctgcgcgcctgcctggcttacccactgctgcacggttgtaccgttacgctttttgatcaagaagcaaacgccgccgtgatgttccgtgcctgacgcttttgtcaattccgcttcatccaccacatggtacgctttgcggtttgctgccatccagcgcaaagcttctttaaaacgcggcgttacactctggataaaccaggcgcgaacaatcgcttccggacggctctggaaaagtgcctgacatgcattttcgccgtagacgcgggtttcttccgcacgctgacgacgcaacacttccggatcaataaaacttttaccactgatgccaccgtgatcggccttttccggcgtctcatcacccggcgcgcgggaaaccgtgcgccacggcgaatcttcccacttgcggtcacggggctgactctgtttgtcatcgcgggcggggcgacggccaccgtcagcacgagattttcctggacgcccgccccctttcccggtacgcgggttgtgggtacgtttatcagaatcatcatcactgcggacatacatcactttgaccttgccgcttttacctttcatttcatcgttcatgcttttctccaccagcgctgcgcgaagcgcgcagattacccgaagtccgcgcggttcgccatgatttcgtaccaaagcctgcgactatcatacctattgaataaaacagattgttgtctggaacaatgtccccgataatatgtaacatattagaaacataccggcgtcgttgccgataagtctccttactcatcccgaggttagttatgaataccgtttgtacccattgtcaggccatcaatcgcattcccgacgatcggatcgaagatgcggcaaaatgcggacgctgcggtcacgacttgtttgacggagaggtgattaatgcgaccggtgaaacactcgacaaattgctgaaggatgatctacctgtggtgatcgacttctgggcaccgtggtgcggcccctgccgtaatttcgcaccaatttttgaagatgtcgcgcaagagcgtagcggtaaagtgcgctttgtgaaagtgaataccgaagctgaacgtgaattgagcagtcgctttggaattcgtagtataccgacgatcatgattttcaaaaacggtcaggttgtcgacatgcttaatggcgcagtaccgaaagcgccgttcgatagctggctgaacgaatctctttaatcttaccggggcgcatcttgtgccccgttttctcctctgcgacaatggcgttttttcgacgctctcttatgaccgaaaacgctgttctccagttacgcgccgagcgtattgcgcgcgcaacacgtccttttcttgcccgcggtaatcgcgttcgtcgctgccaacgctgtcttttgccagagaaattatgtctctgttcgacaattaccccagcacaagcaaaaagtcgcttctgtttgctgatgttcgacaccgagccaatgaagcccagtaataccgggcgtctcattgctgatattttgcctgataccgttgcgtttcaatggtcgcgtaccgaaccctcgcaggatttgctggagttggtgcaaaacccggactatcagccaatggtggtctttcccgcttcgtatgctgatgagcaacgggaagtgatcttcacaccacctgccggtaagccaccgctgtttatcatgctcgatggtacctggccggaagctcgcaagatgtttcgtaaaagtccgtatctggataatcttcccgtcatttccgtcgatctttcccggctttctgcctatcgcctgcgtgaagcccaggctgaaggccaatattgtactgccgaggtagccatcgcactgttagatatggccggcgataccggggcggcggcagggttaggcgagcattttacccgctttaaaacacgctatctggcaggaaaaacgcaacatctgggtagcatcacagcagaacagttagaaagcgtttaaaatcattcggtcacttctgcgggagaccggtatgagtcagcgaggactggaagcactactgcgaccaaaatcgatagcggtaattggcgcgtcgatgaaacccaatcgcgcaggttacctgatgatgcgtaacctgctggcgggaggctttaacggaccggtactcccggtgacgccagcctggaaagcggtgttgggtgtgttggcctggccggatattgccagcttgccctttacacccgaccttgcggttttatgtaccaatgccagccgtaatcttgctcttctggaagagctcggcgagaaaggctgtaaaacctgcattattctttccgccccggcatcgcaacacgaagatctccgcgcctgcgccctgcgccataacatgcgcctgcttggaccaaacagtctgggtttactggctccctggcaaggtctgaatgccagcttttcgcctgtgccgattaaacgcggcaagctggcgtttatttcgcaatcggctgccgtctccaacaccatcctcgactgggcgcaacagcgtaagatgggcttttcctactttattgcgctcggcgacagcctggatatcgacgttgatgaattgcttgactatctggcacgcgacagtaaaaccagcgccatcctgctctatctcgaacagttaagcgacgcgcgacgctttgtttcggcggcccgtagtgcctcgcgtaataaaccgattctggtgattaaaagcggacgtagcccggcggcacagcgactgctcaacacgacggcaggaatggacccggcatgggatgcggctattcagcgtgccggtttgttgcgggtacaggacacccacgagctgttttcggcggtggaaacccttagccatatgcgcccgctacgtggcgaccggctgatgattatcagcaacggtgctgcgcctgccgcgctggcgctggatgccttatggtcacgcaatggcaagctggcaacgctaagcgaagaaacctgccagaaactgcgcgatgcactgccagaacatgtggcaatatctaacccgctcgatctacgcgatgacgccagcagtgagcactatattaaaacgctggatattctgctccacagccaggattttgacgcgctgatggttattcattcgcccagcgccgctgctcccgcaacagaaagcgcgcaagtattaattgaagcggtaaagcatcatccccgcagcaaatatgtctctttgctgacgaactggtgcggcgagcactcctcgcaagaggcacgacgtttattcagcgaagccgggctgccgacctaccgtaccccggaaggaaccatcactgcttttatgcatatggtggagtaccggcgtaatcagaagcaactacgcgaaacgccggcgttgcccagcaatctgacttccaataccgcagaagcgcatcttctgttgcaacaggcgattgccgaaggggctacgtcgctcgatacccatgaagttcagcccatcctgcaagcgtatggcatgaacacgctccctacctggattgccagcgatagcaccgaagcggtgcatattgccgaacagattggttatccggtggcgctgaaattgcgttcgccggatattccacataaatcggaagttcagggcgtcatgctttacctgcgtacagccaatgaagtccagcaagcggcgaacgctattttcgatcgcgtaaaaatggcctggccacaggcgcgggtccacggcctgttggtgcaaagtatggctaaccgtgctggcgctcaggagttgcgggttgtggttgagcacgatccggttttcgggccgttgatcatgctgggtgaaggcggtgtggagtggcgtcctgaagatcaagccgtcgtcgcactgccgccgctgaacatgaacctggcccgctatctggttattcaggggatcaaaagtaaaaagattcgtgcgcgcagtgcgctacgcccattggatgttgcaggcttgagccagcttctggtgcaggtttccaacttgattgtcgattgcccggaaattcagcgtctggatattcatcctttgctggcttctggcagtgaatttaccgcgctggatgtcacgctggatatctcgccgtttgaaggcgataacgagagtcggctggcagtgcgcccttatccgcatcagctggaagaatgggtagaattgaaaaacggtgaacgctgcttgttccgcccgattttgccagaagatgagccacaacttcagcaattcatttcgcgagtcaccaaagaagatctttattaccgctactttagcgagatcaacgaatttacccatgaagatttagccaacatgacacagatcgactacgatcgggaaatggcgtttgtagcggtacgacgtattgatcaaacggaagagatcctcggcgtcacgcgtgcgatttccgatcctgataacatcgatgccgaatttgctgtactggttcgctcggatctcaaagggttaggcttaggtcgacgcttaatggaaaagttgattacctatacgcgagatcacggactacaacgtctgaatggtattacgatgccaaacaatcgtggcatggtggcgctagcccgcaagctcgggtttaacgttgatatccagctcgaagaggggatcgttgggcttacgctaaatcttgcccagcgcgaggaatcatgagtaaggtactggaaatgttgaccacttaatcgggactggtgttattattgcccgcttatgtcgtctgcattgcacagaggacccttcaatgaacagagaagaaatgcactgtgatgttgtcaaaatttaagcgtaataaacatcaacaacaccttgcccaactacccaagatttctcaatcagttgatgatgtcgatttcttttacgctcccgccgacttccgggagacgctgctggaaaaaatagccagcgcgaagcagcgcatttgcattgtcgccctgtatctcgaacaggatgacggtggcaaaggcattctgaacgcgttgtatgaggctaaaaggcagcgtccggaactggatgtgcgggtgctggtcgactggcatcgtgcacaacgtggacgcattggcgctgcggcatctaacactaacgctgactggtactgccgcatggcgcaggaaaatccgggcgtagatgttccggtttatggcgttccaatcaatactcgtgaagcccttggtgttctgcactttaaaggctttatcatcgacgatagcgtactttatagcggtgccagcctgaacgatgtttacctgcatcagcacgataaatatcgctacgaccgttatcatctgatccgtaaccgtaagatgtcagacattatgtttgaatgggttacacagaatattatgaatggccgcggcgttaatcgtctggatgatgttaatcggccaaaaagcccggaaatcaagaacgatattcgtctgttccgccaggagctgcgtgatgccgcttatcatttccagggcgatgccgacaacgatcagctttctgtaacgccgctagtggggctggggaaatcgagtctgttgaacaagaccattttccatcttatgccttgtgccgagcagaaactaaccatctgtacgccatacttcaacctgccagcaatccttgtgcgcaatattatccagttgctgcgcgaagggaaaaaggtcgaaattattgttggtgataaaaccgcgaatgacttctacattccggaagatgaacctttcaagataattggcgcattgccttatctctatgagatcaatctgcgtcgtttcctgagccgtttgcagtattacgtcaatactgaccagctagtggttcggttatggaaagatgacgacaacacctatcacctgaaagggatgtgggttgatgataagtggatgttgatcaccggtaataacctgaacccgcgcgcctggcgtctggatctggaaaacgccattttgatccacgatccgcaacttgagctggcgccacagcgagagaaagaactggagctgatccgcgagcataccaccatcgttaagcactatcgcgatctgcaaagtattgccgattatccggtgaaggttcgtaaactcatccgccgtttgcgccgtatccgcatcgaccgattaattagccgcatcctgtaatcacaaccccgtcctgtacggggtttgttttttggaggccacgttttgcgtattctttttgtctgttcgctattgttactttctggatgcagccatatggctaacgatagctggagcgggcaggataaagctcaacactttatcgcctcggcgatgctttccgccgccggaaatgaatattcacagcatcaggggatgagccgggatcgcagtgccatgtttggattgatgttctctgtcagtttgggggcgtcaaaagagctttgggatagccgccccgaagggagcggctggagctggaaggatttggcctgggatgtcgccggtgcaagcaccggctataccgtctggcaactgacccgtcactaaagacgcatccccttccctttgcgatgtagcatcaaagaaaccagaaacgccaccacggccatcaaggtcacataccagaagaaggctgtttccattcctattgatttcagcgacaacgctacgtactccgccgaaccaccaaatatagcattagcgaccgcatatgacagaccaacgcctaatgcgcgaacctgtgccgggaacatctcagccttcagtattccactgattgatgtataaaaactcactatcagcagggcacacatcaccagaccaaaagcggcataaggcgaggaaacgttttgcaatgctgagagaataggaacggtaaaaatggctgccagcgaaccgaaacataacattgaggtacggcgaccaatcttatccgacagcgcgccaatgagtggttgaataagcatgaatacaaacaatgcggcagtcataatgccactcgccacgttggcatgcattcccgcagtatttaccagatacttctgcatataagtagtgaaggtatagaaacaaagggagcccgcagcggtaaaaccgagaaccatgatgaatgcacggcgattgcgccataatcctttcagagatccagcttcttttaaagcgcgcgtttcttgttgcgaagtttcatctaactgacgacgtaaccacaacgccacaacagctaacacagctcctaacgcgaaaggaatacgccatccccactctctgagtgcagcgtcttccatggtgtgttgtaaaaccacgacaaccagtagggctagcagttgtccgccgatcaacgtcacatactgaaatgatgcgtaaaaacctttgcgcccttcaacggcaacttcactcatataggtggcgctggtgccatattctccgccaacagataatccctgaaataaacgagcgagaagcaataatgccggagcccacgtacctatagtttcataacctgggaggcaggcgataaccagcgatccgaaacacatcatacacaccgataacagcatcgattttttgcgaccatgtttatcggctatgcggccaaatagccaaccgcctattgggcgcatcaggaatcccgcagcaaaaacacctgctgtttgtagtagttgagtcgtcgtgttcccggaagggaagaagatgtgggcaaagtagagtgaacagaacgagtagacatagaaatcgaaccactcgaccagattacctgaagaggcccccacaatcgcccaaatgcggcgacgagtatcactacttgtcagtttgctgtctgccgttacagtactttcagccatgccattatgtctcctgccgtaatccgatgcttttgtcggtcgcttttgtttattttttttgtaaaggaaatattatacatttgttgcatatcattatgcaaccttaaccatgaatttagttagcaggaaaatggttattgaggagcttaaggataaatttctggtaaggaggacacgtatggaagtgggcaagttggggaagccgtatccgttgctgaatctggcatatgtgggagtataagacgcgcagcgtcgcatcaggcatttttttctgcgccaatgcaaaaaggccatccgtcaggatggcctttcgcataatttgatgcctggcagttccctactctcgcatggggagaccccacactaccatcggcgctacggcgtttcacttctgagttcggcatggggtcaggtgggaccaccgcgctacggccgccaggcaaattctgttttatcagaccgcttctgcgttctgatttaatctgtatcaggctgaaaatcttctctcatccgccaaaacagcttcggcgttgtaaggttaagcctcacggttcattagtaccggttagctcaacgcatcgctgcgcttacacacccggcctatcaacgtcgtcgtcttcaacgttccttcaggacccttaaagggtcagggagaactcatctcggggcaagtttcgtgcttagatgctttcagcacttatctcttccgcatttagctaccgggcagtgccattggcatgacaacccgaacaccagtgatgcgtccactccggtcctctcgtactaggagcagcccccctcagttctccagcgcccacggcagatagggaccgaactgtctcacgacgttctaaacccagctcgcgtaccactttaaatggcgaacagccatacccttgggacctacttcagccccaggatgtgatgagccgacatcgaggtgccaaacaccgccgtcgatatgaactcttgggcggtatcagcctgttatccccggagtaccttttatccgttgagcgatggcccttccattcagaaccaccggatcactatgacctgctttcgcacctgctcgcgccgtcacgctcgcagtcaagctggcttatgccattgcactaacctcctgatgtccgaccaggattagccaaccttcgtgctcctccgttactctttaggaggagaccgccccagtcaaactacccaccagacactgtccgcaacccggattacgggtcaacgttagaacatcaaacattaaagggtggtatttcaaggtcggctccatgcagactggcgtccacacttcaaagcctcccacctatcctacacatcaaggctcaatgttcagtgtcaagctatagtaaaggttcacggggtctttccgtcttgccgcgggtacactgcatcttcacagcgagttcaatttcactgagtctcgggtggagacagcctggccatcattacgccattcgtgcaggtcggaacttacccgacaaggaatttcgctaccttaggaccgttatagttacggccgccgtttaccggggcttcgatcaagagcttcgcttgcgctaaccccatcaattaaccttccggcaccgggcaggcgtcacaccgtatacgtccactttcgtgtttgcacagtgctgtgtttttaataaacagttgcagccagctggtatcttcgactgatttcagctccatccgcgagggacctcacctacatatcagcgtgccttctcccgaagttacggcaccattttgcctagttccttcacccgagttctctcaagcgccttggtattctctacctgaccacctgtgtcggtttggggtacgatttgatgttacctgatgcttagaggcttttcctggaagcagggcatttgttgcttcagcaccgtagtgcctcgtcatcacgcctcagccttgattttccggatttgcctggaaaaccagcctacacgcttaaaccgggacaaccgtcgcccggccaacatagccttctccgtccccccttcgcagtaacaccaagtacaggaatattaacctgtttcccatcgactacgcctttcggcctcgccttaggggtcgactcaccctgccccgattaacgttggacaggaacccttggtcttccggcgagcgggcttttcacccgctttatcgttacttatgtcagcattcgcacttctgatacctccagcatgcctcacagcacaccttcgcaggcttacagaacgctcccctacccaacaacgcataagcgtcgctgccgcagcttcggtgcatggtttagccccgttacatcttccgcgcaggccgactcgaccagtgagctattacgctttctttaaatgatggctgcttctaagccaacatcctggctgtctgggccttcccacatcgtttcccacttaaccatgactttgggaccttagctggcggtctgggttgtttccctcttcacgacggacgttagcacccgccgtgtgtctcccgtgataacattctccggtattcgcagtttgcatcgggttggtaagtcgggatgacccccttgccgaaacagtgctctacccccggagatgaattcacgaggcgctacctaaatagctttcggggagaaccagctatctcccggtttgattggcctttcacccccagccacaagtcatccgctaatttttcaacattagtcggttcggtcctccagttagtgttacccaaccttcaacctgcccatggctagatcaccgggtttcgggtctataccctgcaacttaacgcccagttaagactcggtttcccttcggctcccctattcggttaaccttgctacagaatataagtcgctgacccattatacaaaaggtacgcagtcacacgcctaagcgtgctcccactgcttgtacgtacacggtttcaggttctttttcactcccctcgccggggttcttttcgcctttccctcacggtactggttcactatcggtcagtcaggagtatttagccttggaggatggtccccccatattcagacaggataccacgtgtcccgccctactcatcgagctcacagcatgtgcatttttgtgtacggggctgtcaccctgtatcgcgcgcctttccagacgcttccactaacacacacactgattcaggctctgggctgctccccgttcgctcgccgctactgggggaatctcggttgatttcttttcctcggggtacttagatgtttcagttcccccggttcgcctcattaacctatggattcagttaatgatagtgtgtcgaaacacactgggtttccccattcggaaatcgccggttataacggttcatatcaccttaccgacgcttatcgcagattagcacgtccttcatcgcctctgactgccagggcatccaccgtgtacgcttagtcgcttaacctcacaacccgaagatgtttcacttcagagttgcgaaaatttgagagactcacgaacaactttcattgttcagtgtttcaattttcagcttgatccagatttttaaagagcaaatatatcaaacaagacttaacagtctgttttgagatattgaggtcggcgactttcactcacaaaccagcaagtggcgtcccctaggggattcgaacccctgttaccgccgtgaaagggcggtgtcctgggcctctagacgaaggggacacgaaaattgcttatcacgcgttgcgtgatattttcgtgtagggtgagctttcattaatagaaagcgaacggccttattctcttcagcctcactcccaacgcgtaaacgccttgctattcacttttcatcagacaatctgtgtgagcactgcaaagtacgcttctttaaggtaaggaggtgatccaaccgcaggttcccctacggttaccttgttacgacttcaccccagtcatgaatcacaaagtggtaagcgccctcccgaaggttaagctacctacttcttttgcaacccactcccatggtgtgacgggcggtgtgtacaaggcccgggaacgtattcaccgtggcattctgatccacgattactagcgattccgacttcatggagtcgagttgcagactccaatccggactacgacgcactttatgaggtccgcttgctctcgcgaggtcgcttctctttgtatgcgccattgtagcacgtgtgtagccctggtcgtaagggccatgatgacttgacgtcatccccaccttcctccagtttatcactggcagtctcctttgagttcccggccggaccgctggcaacaaaggataagggttgcgctcgttgcgggacttaacccaacatttcacaacacgagctgacgacagccatgcagcacctgtctcacggttcccgaaggcacattctcatctctgaaaacttccgtggatgtcaagaccaggtaaggttcttcgcgttgcatcgaattaaaccacatgctccaccgcttgtgcgggcccccgtcaattcatttgagttttaaccttgcggccgtactccccaggcggtcgacttaacgcgttagctccggaagccacgcctcaagggcacaacctccaagtcgacatcgtttacggcgtggactaccagggtatctaatcctgtttgctccccacgctttcgcacctgagcgtcagtcttcgtccagggggccgccttcgccaccggtattcctccagatctctacgcatttcaccgctacacctggaattctacccccctctacgagactcaagcttgccagtatcagatgcagttcccaggttgagcccggggatttcacatctgacttaacaaaccgcctgcgtgcgctttacgcccagtaattccgattaacgcttgcaccctccgtattaccgcggctgctggcacggagttagccggtgcttcttctgcgggtaacgtcaatgagcaaaggtattaactttactcccttcctccccgctgaaagtactttacaacccgaaggccttcttcatacacgcggcatggctgcatcaggcttgcgcccattgtgcaatattccccactgctgcctcccgtaggagtctggaccgtgtctcagttccagtgtggctggtcatcctctcagaccagctagggatcgtcgccttggtgagccgttaccccaccaacaagctaatcccatctgggcacatccgatggcaagaggcccgaaggtccccctctttggtcttgcgacattatgcggtattagctaccgtttccagtagttatccccctccatcaggcagcttcccagacattactcacccgtccgccactcgtcagcgaagcagcaagctgcttcctgttaccgttcgacttgcatgtgttaggcctgccgccagcgttcaatctgagccatgatcaaactcttcaatttaaaagtttgatgctcaaagaattaaacttcgtaatgaattacgtgttcactcttgagacttggtattcatttttcgtcttgcgacgttaagaatccgtatcttcgagtgcccacacagattgtctgataaattgttaaagagcagtgccgcttcgctttttctcagcggcgcggggtgtgcataatacgccttcccgctacagagtcaagcatttctttgcttttctctgttgagattctcaggagaaccccgccgacccggcggcgtgtttgccgttgttccgtgtcagtggtggcgcattatagggagttattccggcctgacaagcgaaaaatataaaaactttatcgttcgctcacttttcaggcaaaacatcttaaatatagtcttttccgtctaacttatagacaaaaacgagccccgaagggctcgttttatcatttactggacggcgacaatccggtcttcattaacttccaggcgaatcactttacccggaaccaattcaccagacagtatttgctgtgccagcgggttttcgatctgctgctgaattgcacgtttcagaggacgtgcaccatagaccggatcgtaaccgttctcgctcagcagtttcagcgcctcgtcagaaatgtggatttcataaccacgttcttccagacgtttgtacagacgtttcaactgaatctgcgcaatcgaggcaatgtgctgttcacccagcggatggaagaccaccacttcatcgatacggttaatgaattccggacggaagttatggcttaccacaccgagcaccagctctttcatgtgcgcataatccagttcaccgaagcgttcctgaatcagatcggaaccgaggttagaggtcataatgacgaccgtattacggaagtcgaccgttctcccttgcccgtcagtcagacgcccatcatccagtacctgcaacagaatgttgaagacatccggatgcgctttttccacttcatccagcaggatgacggaatacggacgacgacgcaccgcttcggtcaggtagccaccttcttcataaccgacatatcccggaggcgcaccaaccaaacgagacaccgagtgtttctccataaactcggacatatcgatacggaccatcgcctcgtcgctatcaaacataaagttcgccagcgccttacaaagctctgttttccccacaccagttgggccgaggaacaggaatgaaccaatcgggcgatttggatccgccagccccgcacggctacgacgaatagcgttagataccgcatcaaccgcttcgttctgaccaattacgcgatggtgcagttcttgctccatacgcagcagtttttcgcgctcgctttccatcatgcgagaaaccggaatccccgtccaacgcgccagcacttcagcaatttcggcgtcggtcactttattacgcaacagacgcatagttttgccttcgagctgcgttgcggcttccagttgcttttccagttccgggattttgccgtattgcagttcagacatccgcgccaggtcccccacacggcgagcctgttcaatagcgattttcgcctgttccagttccgctttaatggtctgcgtaccagaaagcgatgccttctctgctttccactcttcttctaactcggagtactgacgttctttgtcgctcagttcttcgttgagcatatccagacgttttttactggcttcatcagactctttcattaacgcctgttgttccagtttgagctggatgatacgacgatcgagtcggtcgagttcttctggttttgagtcaatctgcatacgaatgctggatgctgcttcatcgatcaggtcgatggctttatccggcagctgacggtcagcaatgtagcgatgagacaacgtcgccgctgcaacaattgccgggtcagtaatttgcacatggtggtgcaattcgtaacgttctttcaggccacgcagaatcgcaatggtatcttcaacagaaggctcggcaacaaacactttctggaaacgacgttccagcgcagcatctttttcaatgtactggcgatattcgtcaagcgtcgtggcacctacgcagtgcaattcaccacgcgccagcgccggtttcagcatgtttccggcgtccattgcgccatcggctttacccgcgccgaccatggtatgtaattcgtcgataaataggatgacgttgccttcctgtttggcaagatcgttaagcacgccttttaaacgttcttcaaactcaccgcgatatttcgccccagccaccagcgcgcccatatccagcgccagtacccggcggcctttcaacccttccggcacttcgccgttgataatacgctgcgccagaccttcaacgatggcagttttaccgacgccgggttcaccaatcagtaccgggttatttttagtacgacgttgcagcacctgaatggtacggcgaatttcttcatcacgaccaatcaccggatcgagtttgccctgttcggctcgttcggtaaggtcgatggtatattttttcaaagcctgacgttggtcttcagcaccttgatcgttcacgctttcacctccacgcatttgttcaatcgcttgagtaatgttggcggtggtcgcccctgctgctttcaggatgtcggccagcgtgccgcgagactcaagtgccgccagaacgaacagttctgacgagataaagttatcaccacgtttttgcgccagcttgtcgcaaagattaagaacgcgcaccagatcctgtgatggctggacatcaccaccagtaccttcaacctgcggtaaacgatttaatgcctgattgatatctgtgcgcaactggccagcatttatgccagcggatgttaataaaggactaaccgaacccccttcctgattcagcagggcgctcattaaatgaagtggttcgataaattggttgtcgtgcccgagtgcaagtgattgggcatcggcaagagcaagctggaatttattagtaagacgatccagacgcataactcctcccataacggatcaaagttgctactggagattaaatgaggtcatccctcaattattcaaggttattgaccagattaatgtgaaaagaaaatcacgcgtaccggatcgtcttgattctttaggttatatcagccaaatgaaacttgccatacgaccggtggtcttgtcgcgacgataagagaagaaagtctcattttccgtatatgtacaacggtcgccgccgaaaatttgctcaacacccacgttcgccagacgctgccgggcaagctgataaatatccgccagatacttatcaccatgctgaatgaaagctgcacttgctttagcgtctactgccataaacgcctcgcgaacctccccccccacttcgaacgcgcgtggaccaattgccggccctaaccaggcgagaatattttccggattatcagcaaaacaggaaaccgtctcttccagcacgcctgcgcacagtccacgccagccagcatgagcggcggcgacttccgttcccgctcgattgcaaaacagcacagggaggcagtcggcagtcatcactgcgcaaaccgtgccgggcgtattgctataagaggcatccgcccgttttgaggcataaggttcgccagtgagcttaagcacatctttgccgtgtacctgctcaagccagaccggtttagaaggcaaattgcccgcagcaaaaagtcgcttgcgattctcctcaacgtgatccgggttatcgccacaatgggcaccgaggttgagtgagtcatacgggggcaagctcacgccgccgatacgagtggagctacaggccgcaacaccttttggctgcggccactgcgggacaatcagcttactcataaccagtccacttcatccttatgttcttcgaaatcggcgcgcatcacctcaatcagctccaccatatcttgtggaataggcgcatgccattccatttcgatgccggagatcgggtgataaagacgcagcatggttgcatgtagcgcctggcggtcaaacttacgcagcgtggagataaatgcttccgaagcaccttttggcggacgcggacggccaccataaaccggatcgcccaccagcggatgagtgatatgggccatatgcacgcggatctggtgcgtacgtccagtttccagacgcaaccgcagacgcgtgtgcacacggaagtgttccatgatgcgatagtgagtcaccgctggtttgcccatcggatgcaccgccatatgggtacgtttggtcgggtggcgactgattggctcgtccaccgtgccacctgcggtcatatgaccaatcgccaccgcttcatactcacgagtaatttcacgccgttgcaaagattcgactaaacgcgtctgagccggaacggtttttgccacaaccatcaggccagtggtgtctttatccagacgatggacgatgcccgcacgcggtacatcggcaatgggtggatagtaatgaagcaacgcattcagtaccgtgccatccgggttacccgcgccaggatgtaccaccaggtcgcgcggtttattaatgataataatgtcttcatcttcatagacgatatccagcgggatatcctgcggttcaaaacgcgcttcttcttcaatctcagcgttgatggcaacctgctcgccacccaatactttttctttcggcttatcacaaactttgccgttaaccagcactcgctggtcgaggatccattcttttattcgcgaacgtgaataatccgggaacatttcggccaaagcctgatctaagcgttgaccgagttggttttcggacaccgttgcagtgagctgtactcgttgtgccatatatactgcttcttcgtttatcgttggggttttacggctttgccgtttaatatagtgtgctattgtagctggtcttaaccgggagcaggaacagagaatctcccgtattacattttgaggaaagtcaaaacgtcatgacgcgcatgaaatatctggtggcagccgccacactaagcctgtttttggcgggttgctcggggtcaaaggaagaagtacctgataatccgccaaatgaaatttacgcgactgcacaacaaaagctgcaggacggtaactggagacaggcaataacgcaactggaagcgttagataatcgctatccgtttggtccgtattcgcagcaggtgcagctggatctcatctacgcctactataaaaacgccgatttgccgttagcacaggctgccatcgatcgttttattcgccttaacccgacccatccgaatatcgattatgtcatgtacatgcgtggcctgaccaatatggcgctggatgacagtgcgctgcaagggttctttggcgtcgatcgtagcgatcgcgatcctcaacatgcacgagctgcgtttagtgacttttccaaactggtgcgcggctatccgaacagtcagtacaccaccgatgccaccaaacgtctggtattcctgaaagatcgtctggcgaaatatgaatactccgtggccgagtactatacagaacgtggcgcatgggttgccgtcgttaaccgcgtagaaggcatgttgcgcgactacccggatacccaggctacgcgtgatgcgctgccgctgatggaaaatgcataccgtcagatgcagatgaatgcgcaagctgaaaaagtagcgaaaatcatcgccgcaaacagcagcaatacataacagaaacctgaaacacaaaacggcagcccttgagctgccgtttttttattctgtcagttgtgaaactgaagcgatttagtcgctatcgatctcatcaaatatggctcgctttgagatattcctcaagtaaaaaaacatctcttcctgcgatttctcacaaaaaagattcgttgacaaaaagtgacaaaattatgagattttcatcacacattttgacatcaggaacggtatgctgaattcaccaagacgggaagacaagaggtaaaatttatgacaatgaacattaccagcaaacaaatggaaattactccggccatccgccaacatgtcgcagaccgtctcgccaaactggaaaaatggcaaacacatctgattaatccacatatcattctgtccaaagagccacaagggtttgttgctgacgccacaatcaatacacctaacggcgttctggttgccagtggtaaacatgaagatatgtacaccgcaattaacgaattgatcaacaagctggaacggcagctcaataaactgcagcacaaaggcgaagcacgtcgtgccgcaacatcggtgaaagacgccaacttcgtcgaagaagttgaagaagagtagtcctttatattgagtgtatcgccaacgcgccttcgggcgcgttttttgttgacagcgtgaaaacagtacgggtactgtactaaagtcacttaaggaaacaaacatgaaacacataccgtttttcttcgcattcttttttaccttcccctgaatgggaggcgtttcgtcgtgtgaaacagaatgcgaagacgaacaataaggcctcccaaatcggggggccttttttattgataacaaaaaggcaacactatgacatcggaaaacccgttactggcgctgcgagagaaaatcagcgcgctggatgaaaaattattagcgttactggcagaacggcgcgaactggccgtcgaggtgggaaaagccaaactgctctcgcatcgcccggtacgtgatattgatcgtgaacgcgatttgctggaaagattaattacgctcggtaaagcgcaccatctggacgcccattacattactcgcctgttccagctcatcattgaagattccgtattaactcagcaggctttgctccaacaacatctcaataaaattaatccgcactcagcacgcatcgcttttctcggccccaaaggttcttattcccatcttgcggcgcgccagtatgctgcccgtcactttgagcaattcattgaaagtggctgcgccaaatttgccgatatttttaatcaggtggaaaccggccaggccgactatgccgtcgtaccgattgaaaataccagctccggtgccataaacgacgtttacgatctgctgcaacataccagcttgtcgattgttggcgagatgacgttaactatcgaccattgtttgttggtctccggcactactgatttatccaccatcaatacggtctacagccatccgcagccattccagcaatgcagcaaattccttaatcgttatccgcactggaagattgaatataccgaaagtacgtctgcggcaatggaaaaggttgcacaggcaaaatcaccgcatgttgctgcgttgggaagcgaagctggcggcactttgtacggtttgcaggtactggagcgtattgaagcaaatcagcgacaaaacttcacccgatttgtggtgttggcgcgtaaagccattaacgtgtctgatcaggttccggcgaaaaccacgttgttaatggcgaccgggcaacaagccggtgcgctggttgaagcgttgctggtactgcgcaaccacaatctgattatgacccgtctggaatcacgcccgattcacggtaatccatgggaagagatgttctatctggatattcaggccaatcttgaatcagcggaaatgcaaaaagcattgaaagagttaggggaaatcacccgttcaatgaaggtattgggctgttacccaagtgagaacgtagtgcctgttgatccaacctgatgaaaaggtgccggatgatgtgaatcatccggcactggattattactggcgattgtcattcgcctgacgcaataacacgcggctttcactctgaaaacgctgtgcgtaatcgccgaaccagtgctccaccttgcggaaactgtcaataaacgcctgcttatcgccctgctccagcaactcaatcgcctcgccgaaacgcttatagtaacgtttgattaacgccagattacgctctgacgacataatgatgtcggcataaagctgcggatcctgagcaaacagtcgcccgaccatcgccagctcaaggcggtaaatcggcgaagagagcgccagaagttgctcaagctgaacattttcttctgccaggtgcagcccgtaagcaaaagtagcaaagtggcgcagtgcctgaataaacgccatattctgatcgtgctcgacggcgctaatacgatgcagccgagcgccccagacctgaatttgctccagaaaccattggtatgcttccggtttacgtccatcacaccagaccacaacttgctttgccaggctaccgctgtccggaccgaacatcgggtgtagccccagcaccggaccatcatgcgccaccagcatggcctgtaatggcccatttttcactgatgccagatcgaccagaatacaatctttcggtaaaggcggtaatttgccaataacttgctcagtaacgtggattggcacactaacaatcaccattccggcatcggcaacaatatcagccgctcgatcccagtcatgttgctccagaatccgcacctgataacccgagagggtcagcatcttctcgaacaggcgtcccatctgaccgccaccgccgacgataaccaccggacgcagtgacggacaaagtgttttaaatcctttgtcgttttcactggagtaagattcacgcatcacccgacgcaaaacatcctcaatcagatctggcggtacacccagagcttccgcctctgcacgacgcgaggccaacatagatgcctcgcgctccggaacataaataggcagtccaaagcggcttttcacctcgcccacttcagcaaccagttccagacgcttcgctaataaattcagcagcgctttatcgacttcatcaatttgatcgcgtaatgcggtcaattcagcaaccataataaacctcttaagccacgcgagccgtcagctgcccgttcagatcctgatgaatttcacgcagcaaggcatcggtcatttcccagctaatgcaggcatcggttacggatacaccgtatttcatttcactgcgcggttgctcggaagactgattgccctcgtggatattactttcgatcatcagaccaataattgagcgattgccatctttgatttgagcaaccacggattctgccaccgcaggctgacggcgataatctttattggaattaccgtggctgcaatctaccatcagagacgggcgcagtcccgcctgttccatctctttttcacattgcgcaacatccgcagggctatagttcggcgctttaccaccgcgcaggatcacatggccgtccggattcccctgagtttgtagcaacgcaacctgccctgcctggttaatgccaacaaaacggtgcggctgggcggcggcgcgcatagcgttaattgctgttgccagactgccgtcggtgccgtttttaaaaccaaccggcatggaaagcccggaggccatttcacggtgagtttgcgattccgttgtacgagcaccaattgctgaccagctaaacagatcgcccaggtattgcgggctattcggatctaacgcttccgtcgccagtggcagtcccatattcaccagctcaagcagcaatttacgcgcgatctgcagcccggcttctacatcaaaagagccatccatatggggatcgttaattaaccctttccagccgacagtggtacggggtttttcaaaatagacgcgcattaccagatagaggctatcgctgacctctgcggcaagggctttaaatcgacgagcatattccagagcagtttccggatcatgaatggaacaaggaccacatactaccagcagacgaggatcgcgcccggcgataatatctgaaatgcttttacgcgagtcagcaatctgggcttcttgttgcaggctcaatggaaaagcggccttcagttgttccggagtcattaaaacctgttcgtcggtaatatgtacgttattcagcgcgtctttttgcatgatggcgatcctgtttatgctcgtttgcgatagttgatcctcagcgaggatgacgtaacgataacacataaagtaaagttttcaatccatatttcgtacatttttatttacacaggcaatttagtcgcgctttcaacccttacctctgtatagataaatttacactccctttgaaaacaatccgctatgctttgaaaaaggagaaagaaatgatgaaaaagtttatcgcccccttgttggctttactggttagcggatgtcagattgatccttatactcacgcgccaaccttgaccagcaccgactggtatgatgtcggtatggaagatgcgatatcgggcagcgccataaaagatgacgatgcatttagcgattcacaggcggatcgcggtctataccttaaaggatatgccgaaggacaaaagaaaacttgccagaccgattttacttatgcccgaggactttccggtaaaagctttcctgccagctgcaacaatgttgaaaatgccagccaactgcatgaagtatggcaaaaaggggctgatgaaaatgccagcacaatacgattaaattaattaaaaccccacaaataaattaaacataagattttactcattgtgttttatttctcacattgatgacggtcgcatgaaaaaatgatattttaatgagcattctgaaaaaatatcgatgcatttcgagcgaagatggtggggatccctgaatgcgtttttctcaccgactgttcttacttctgattctcctgctgacgggagcaccaatactcgctcaggagccttctgacgttgcgaaaaacgtgcgtatgatggtttccggtattgtcagttacacccgctggcctgcgctatcagggccaccaaagttatgtatcttttcatcttcacgttttagtaccgccctacaagagaatgccgcgacatctttgccttatctgcctgtcatcattcacactcaacaagaggcgatgatttcaggctgcaatggtttttattttggcaacgagtcaccgacattccagatggaattaaccgaacaatatccgtcaaaggcgttattattaattgccgaacaaaataccgagtgcattattggtagcgccttttgtctgatcatccacaataatgacgtcagatttgccgtaaacctggatgccttatcgcgtagcggtgtaaaggtcaacccggatgtcttaatgctcgcacggaagaaaaatgatggataacgataattctcttaataagcgccccacgtttaaaagagcattacgcaacatcagtatgaccagcatatttatcactatgatgctgatctggttgctgctttccgtgacctcggtgctgaccctgaaacagtacgcgcaaaaaaacctggcactgacagcagcaacaatgacttacagtctggaagcagctgtcgtttttgccgatggccctgcagcaactgaaacactggcagcgctgggccagcaagggcaattttcaactgcagaagtacgtgataagcagcaaaatattctggcatcctggcattacacccgtaaggatccaggcgatactttcagtaatttcataagccactggctcttccctgcccccatcattcagccgattcgtcacaatggtgaaaccattggcgaagtacgcttaaccgctcgcgacagttcaatcagccattttatctggttttcgctcgccgtactgaccggttgtattctgctggcatcaggcatcgcaattaccctcacccgccatttgcacaatggcctggtagaagcgctgaaaaatatcaccgatgtcgtacatgatgtgcgttccaaccgcaatttttcccgacgagtttcggaagaacgtatcgctgagtttcaccgcttcgctctcgacttcaacagtctgctggatgaaatggaagagtggcagcttcgtttacaggctaaaaatgcgcagcttctacgtaccgcgctacatgacccattaaccgggctggctaaccgcgcagcgtttcgtagcggcatcaacacgttgatgaacaattccgatgcccgaaaaacgtcggcgttactatttcttgatggcgataatttcaaatacatcaatgatacctggggtcatgcgacgggcgatagagtcttgattgaaatcgcaaaacggttagctgaatttggcgggctgcgacataaagcataccgcctgggcggcgatgaattcgctatggtgctctatgatgtacagtcggaatctgaagtgcagcagatatgttcagcactgacacaaatctttaatctcccgtttgatcttcataatggccatcagaccaccatgacattaagcattggttacgcgatgaccattgagcacgcctctgcggaaaaattacaagagcttgccgatcacaatatgtatcaggccaaacaccagcgtgccgaaaagctggtgagataacaaggatatatcgatatgataaagcacctggtagcacccctggttttcacctcactaatactgactggctgccagtcccctcagggaaagtttactcctgagcaagtcgccgctatgcaatcttatggatttactgaatccgccggcgactggtcgctgggcttatcagatgccattctgttcgcaaaaaatgactacaaattgctcccggaaagccagcaacagatccaaaccatggcagctaaattggcctcgacagggctaacacatgcccgtatggatggacacaccgataactatggtgaagacagttacaacgaaggcttatcattgaaacgggcgaatgtcgtggccgatgcatgggctatgggtggacaaattccacgcagcaatctcaccacacagggtttaggaaaaaaatatcccatagccagtaacaagaccgcccagggccgcgccgagaaccgccgcgtcgcagtggtgattactaccccttaaaacaccagcaaacagataaaaaagggccagccaattggccagcccttcttaacaggatgtcgcttaagcgaaatcttagttaagacgctctttgatacgagcagccttaccagtacgctcacgcaggtagtacagtttagctttacgaacagcaccacgacgtttgacagaaatgctgtcaactaccggagagtgagtctggaagacacgctcaacgccttcgccgttggaaattttacgaacagtgaatgcagagtgcagaccgcggttacgaatagcgataaccacgccctcgaatgcctgcagacgttttttggaaccttcaacaacccatactttcacttccacggtatcacccggacggaaggaaggtacgtcctgcttcatctgctcttgttcaagttgcttaataatgttgctcataatttaatctcttatcctgggtaaactgatatctcgggggcttacgccatcccatcatgtttatgttgctgttgtgcgtgttccgttttgaactccgccagcaaccttgcttgctcttcagtcagagccaggttttccagaagttcaggtcttctaagccaggtacggcccagcgactgtttcaaacgccagcgacgtatctcggcatggttgcccgacagtaacactggcggaacttccatcccttctaacacctcaggccgcgtatagtgcgggcaatccagcaatccttcagcaaaggaatcttccgttgccgaggcttcatgtcccagtactcccggaataaaccgggaaacggagtcaatcagcgtcattgctggtaactcaccaccactgagaacgtaatcgccgattgaccattcttcgtcaatttcggtttggatcacgcgctcatctataccttcgtagcgaccgcacaccagaatcaatttttgattcgttgccagttcgctgacgcccgcttgatcaagcttgcgtccctgtggtgacagataaatcacctttgcgccttcacccgccgcggcttttgctgcatgaatggcgtcccgcaagggttgcaccatcattaacatccccggtccgccgccgtaaggacgatcgtccacggtacggtgccggtcatgcgtgaagtcgcgaggactccagctctggatgctcagcaggccatttttaactgcccggccagttaccccgtaatcggtaattgcgcggaacatttcaggaaacaggctaattatgccaatccacatagcgccgtcttttaccgtttatccggtggtttaaaaaccaggatcccaatctacttcgattgaacgagtagtgagatcgactttcttgataacctgcccatcgaggaacggtacgagacgttccttgataccaaacgcatctttcaggtttgccttaatgacgagaacgtcattagatccggtttccatcatatcgacgactttaccgagatcgtagccttcagtggttactacctggcagcccatcaggtctttccagtagtagtccccctcttcaagctgaggcagctgcgatgaatccacgacaatttcacaattcgtcagcaggttcgccgcatcacgatcgtcaacgcctttcagcttgatgatcatgtcctgattgtggtgcttccagctttccagctggacttgctgccactgacccgccttctggataaaccagggctgatagtcaaaaatgctttcggcgtcttcggtggaagaaaacactctgagccacccacgaataccgtaagacgaacccatttttcccaaaacgatgggatcaacaggtgcttgcgcggtgagttgtttgctcatcatgaccaccgtgacagattaagctgctttgtttacttctttgatcagcgcagcaacgcgatcagaaatagttgcgccctggccaacccagtgagcgatgcgatccagatccaggcgagtgccttcttctttttcgctagcgattgggttgaagaaaccaacgcgctcgatgaagcgaccgttgcgtgcattacggctgtcagcgacaacaacctggtagaacggacgctttttagcgccgtgacgtgctaaacgaatagttaccataacatcctcttgtgtgaataaaacaaccggaccccatcgaggaacggagtccggtgtcatattaaaagcccgaaaattttactcatttttgcgggaattgcaatcaacagttgctaactctgctgtaaaaggccgtcggcggtgcagccagtttggtgccggagtgcgcgcagtcaccggagcgtacacgcagtacgtgaggatgacgagcacatcccggtgccaaaatggcaaacaagccaggccgattagcgaccagggaagcctgggggcatcatacccttcatgcttctcatcatcttcgccattccgcccttcttcattttcttcatcatgcgctgcatgtcgtcgaactgtttcagaagacggttaacgtcctgcacctgcataccgcaaccggcagcaatacggcgtttacgcgaacctttgatgatttctggcttagcgcgctctttcatcgtcatcgagttgatgatggcttccatacgcaccagcactttatcgtccatctgtgacttgacgttatccgggatctgccccatgcccggcagcttgcccatcagactagccatgccgcccatatttttcatctggcgcagctgctcaagaaagtcgttgagatcgaagccgtcaccttttttcagcttgctggctaatttctctgcctgcgcgcggtcaactttgctttcgatatcttcgatcagcgacagtacgtcgcccatgccgagaatacgcgacgcgatgcggtccggatggaacggctccagcgcctcagttttctcgccaacaccgaggaacttgatcggtttgccagtgatgtgacgaatagagagcgccgcaccgccgcgggcatcgccgtccactttggtcaacactacgccggtaagcggtaacgcttcattgaatgcttttgccgtattggccgcatcctgaccggtcatggcgtcaaccacaaacagggtttcaaccgggttaatcgacgcatggacttgtttgatctcgtccatcatcgcttcgtcaacgtgcagacgaccagcggtatccaccagcagcacgtcgtagaatttcagtttggcttctttcagcgccgcgttaacgatatctaccggcttctgaccaacatcagaagggaagaaatcaacgcccacctgctctgccagcgtctcaagctgtttgattgccgccgggcgataaacgtcggcagaaaccaccagcactttcttcttgtgcttctcgcgcaggaacttaccgagtttaccaacgctggttgttttaccggcaccttgcaggcccgccatcagtacgaccgcaggcggttgcgcagccaggttcagggtctggttctcttcgcccatcgccgcaaccagttcgttacggactattttgacgaactcctgccccggcgtcaggctcttattaacttcatgaccaaccgctttctcttttacgcgattgataaactcacgcactaccggcagagctacgtccgcctccagcagcgccatgcgcacttcgcgcagcgtatcttttacgttgtcttcagtgaggcgtccacggccactgatattgcgcagcgtgcgcgacaaacgatcggttaaattatcaaacattgtctctcgcctggggtggaaacggttggccgcaatcgcgacacatcatcagtattttgccgcagtataacatgaaggcgtctttgttgttatgcaacggttggagcagcgttcacctgacgctatactgcttctctttcttattgctcaaactgtcgacatcactatgcccgtttttgctctgctcgcgcttgtcgcctactccgtcagtcttgcgctgattgttcccggtctgctgcaaaaaaacggcggctggcggcgcatggctattatttctgcggtcattgcgctggtctgccacgcaatcgctctggaagcccgcatcctgcccgacggtgatagcggacaaaacctcagcctgctgaacgttggttcattggtcagtttgatgatctgtacggtaatgaccattgtggcttctcgcaatcgtggctggctgctgctacccattgtctatgcctttgcgcttatcaacctggcgctggcaaccttcatgcccaatgaatacatcacccatctggaagctacgcctgggatgctggtgcacattggcttatcgctcttttcctatgccacgctaattatcgccgccctgtacgcgctgcaactggcgtggattgattaccaactgaagaacaagaagctggcgtttaaccaggaaatgccgccattgatgagtatcgagcgtaaaatgttccacatcacgcagattggcgtggtgctgctaacgctcacgctttgcactggcctgttctacatgcacaacttatttagcatggaaaatatcgacaaggctgtgctctctatcgtggcgtggtttgtctatattgtgctgctgtggggacattatcatgaaggatggcgtggacgccgcgtcgtctggtttaacgttgcgggcgcggtaattctgacactggcctacttcggcagccgaattgtccagcagttaatcagctaaacccagaaaaggagtttcccctggaacacatttctactactacgttgatcattattctgatcatcatggtggtcatttcagcctatttttccgggtccgaaaccggaatgatgaccctcaaccgctatcgtctgcgacatatggcgaaacagggtaatcgctcggccaaacgcgtcgaaaaattgctgcgtaagccagaccgcctgataagcctggtgttaatcggcaataacctggtcaatattcttgcctccgcgctcggcactattgttgggatgcgtttgtacggcgatgcgggcgtggcaattgcgactggtgtgctgacttttgtcgtactggtatttgctgaggtattgccgaaaaccattgccgcgctgtacccggaaaaagtcgcttatccgagtagttttctgctggctccgctgcaaattttgatgatgccgctggtctggttgctgaatgctatcacccgtatgctgatgcgcatgatgggtatcaaaaccgatatcgtggttagcggctctttgagcaaagaagagttgcgcactatcgtgcacgaatcacgctcacaaatttcccgtcgcaatcaggatatgctgctgtcggtgctcgatctggaaaaaatgaccgttgatgacatcatggtgccgcgcagtgaaattatcggtattgatatcaacgatgactggaaatcgattctgcgccaactctcccactcacctcacgggcgcatcgtgctctaccgtgattcgctggacgacgccatcagtatgctgcgagtacgtgaagcctggcggttgatgtcggagaaaaaagagttcaccaaagaaaccatgctgcgcgccgcggacgagatctattttgtgccggaaggtacgccgctcagcacgcagttggtaaagtttcagcgcaacaaaaagaaagtcggcctggtcgtcaacgagtatggagacattcaggggctggtgacggttgaagatattctggaagagattgtcggcgatttcactacgtcgatgtcgccaacacttgccgaagaggtcacgccgcaaaacgacggttcggtgattatcgatggcaccgccaacgtgcgggaaatcaacaaagcctttaactggcatctaccggaagatgatgcccgcacggttaatggcgtcattcttgaggcactggaagagatccctgtcgcaggcacccgcgtgcgtattggcgagtacgatatcgatattctcgacgtacaggacaatatgattaagcaggtaaaagtttttcctgtgaaaccgctgcgcgagagtgtggcggagtaacgaaaacggcccggcattcgcatgcagggccgtgaattattacgaaagcagaaattaagcttttgctttcgctacagtaaccatcgccgcacgaatcgtacgaccattcagcgtataacccttctgcataatgcccagtacgttacctggcgcaacgtcatcagattccaccattgcgatggcctgatgcacattcgggtccagtgggacgttagtttcggcgatcacttcaacgccaaacttacgcacaacatccagcatcgacttcagcgtcagctcaatgccttcaaccatcgcagacatatccgggttagctttatcagccacttccagcgcacgatccaggctatcaatcaccggcagcaattcgttgatgaatttctccagcgcgaatttgtgggctttttcaatatccagttcagtacgacgacgcaggttttccatttcggcttttacacgcaaaatgccgtcacgttcacgggtctgggcttcagccagctgagcttcgagattcgcaactttttcatcgcgcggatccacctgctcagcagaagcttctggctcaactgcctcaatctcttcgtgctgatccatgataatttcttccggggcttgcccctcaggcgttttctgttctttactactcatgaatttctccgcgtttttttcgcattcatctcgctaacttcgcttattatggggatcagtttcagggtttcaagggaagcactcacattgtcatcaatcttcgcaacaaggacctcggaaaaatgaataatcatttcaagtgtattggcattgtgggacacccacggcaccccactgcactgacaacacatgaaatgctctaccgctggctgtgcacaaaaggttacgaggtcatcgttgagcaacaaatcgctcacgaactgcaactgaagaatgtgaaaactggcacgctcgcggagattgggcaactagctgatctcgcggtagtcgttggtggcgacggtaatatgctgggcgcggcacgcacactcgcccgttacgatattaaagttattggaatcaaccgtggcaacctgggtttcctgactgaccttgaccccgataacgcccagcaacagttagccgatgtgctggaaggccactacatcagcgagaaacgttttttgctggaagcgcaagtctgtcagcaagattgccagaaacgcatcagcaccgcgataaatgaagtggtgcttcatccaggcaaagtggcgcatatgattgagttcgaagtgtatatcgacgagatctttgcgttttctcagcgatctgatggactaattatttcgacgccaacaggctccaccgcctattccctctctgcaggcggtcctattctgaccccctctctggatgcgattaccctggtgcccatgttcccgcatacgttgtcagcacgaccactggtcataaacagcagcagcacgatccgtctgcgtttttcgcatcgccgtaacgacctggaaatcagttgcgacagccagatagcactgccgattcaggaaggtgaagatgtcctgattcgtcgctgtgattaccatctgaatctgattcatccgaaagattacagttatttcaacacattaagcaccaagctcggctggtcaaaaaaattattctaattttacgccagcctctttactgtatataaaaccagtttatactgtacacaataacagtaatggtttttcatacaggaaaacgactatgttggcacaactgaccatcagcaactttgctatcgttcgtgagcttgagattgattttcatagcggcatgaccgtaataactggcgagaccggcgcgggtaaatctattgcaatagatgccctcggtctttgtctcggtggtcgcgctgaagccgacatggtgcgtaccggcgctgctcgcgctgacctgtgcgcccgtttttctctgaaagatacgccagcggctctgcgctggctggaagaaaaccagcttgaagacgggcatgaatgtttgcttcgtcgcgtgatcagcagcgatggtcgctcccgtggtttcatcaacggtacagctgttcctctgtcacaactgcgcgaactgggtcagttgctgattcagatccatggtcagcacgctcatcaattactcaccaaacctgagcaccaaaaattcctgcttgatggctatgccaatgaaacctctctactgcaggaaatgaccgcacgttatcagttgtggcatcaaagctgccgtgacctcgcgcatcatcaacagttaagtcaggaacgcgccgcccgtgcggaactgctgcaataccaattaaaagaacttaacgaatttaatccgcagcccggagagtttgaacaaatcgacgaagagtacaaacgtctggcgaacagcggtcaattgctgaccaccagccagaatgcattggcattaatggccgacggtgaagacgcaaacctgcaaagtcagctttacacggctaaacaactggtgagcgaattgattggcatggacagcaaactgtccggcgtacttgatatgctggaagaagctaccatccagattgctgaagccagcgatgaactgcgccactactgcgatcgtctggatctcgatcccaaccgactatttgaacttgaacagcgcatctcaaaacagatttcgctggcacgtaaacatcacgtcagccctgaggcattgccacagtattaccagtcgctactggaagaacagcagcaactggacgatcaggccgactcacaagaaacgcttgcgctggcggtaacgaaacatcatcagcaggcactggaaatcgcgcgcgcattacaccaacaacgccagcaatatgcagaagaacttgcacagctgatcaccgacagtatgcatgcgctctcaatgccgcatgggcagtttacgatcgatgttaaatttgacgagcatcacctgggcgctgacggtgccgatcgtattgagtttcgggtaaccaccaacccaggtcagccaatgcagcctattgccaaagtcgcatccggtggtgaattgtcccgcatcgcactggcaatccaggtcatcacggcgcgtaaaatggaaaccccggcactgatttttgatgaagtggatgtagggattagcggtccaacagcggcagttgtcggcaaactgctgcgtcaactcggcgaatcaactcaggtgatgtgtgttacccacctgccacaagtcgcgggatgtggtcatcaacactattttgtcagcaaagaaaccgatggtgcgatgacagaaacgcatatgcaatccctgaataaaaaagcgcggttacaagagctggcgcgcctgcttggtggcagtgaagtcacacgtaatacactggcgaatgcgaaagaactgcttgcagcgtaaacttttttcctgcttcacggtcagagtaaacagcaaaacgccgtaagaccggaaagcaaaaggttttaaagtgatgaaaggtctattatcatcggcatattacagatgagccacgtactgctcgggcccgaaaaggaatcaaatcactatgcgctgtaaaacgctgactgctgcagcagcagtactattgatgttgaccgcaggctgttccactctggagcgagtggtttaccgtcctgacatcaaccaggggaactatctgaccgctaacgacgtatccaaaatacgtgttggcatgacgcaacaacaagttgcgtacgcattgggtacaccgctgatgtccgatccatttggtacgaatacctggttctatgtcttccgccagcaaccaggtcatgaaggtgtaactcagcaaacgctgacgctgacctttaacagtagcggtgtgttgaccaatattgataacaaacctgcgctgagtggtaactaataataaagttgctctcaaagacgttaaaaaaggtgctcaatgagcaccttttttctgtctgttatttattcgctgatttttctgctcgttgcctgcgaagctctttcggatcggcaatgagagggcgataaatctccacccgatcgccatcatgcacactatcgcttagttttgccggacggctgtaaatgccgactttgtttttagttaaatcgatatcggtacgcaattccagcaagccactggcgcgaatagcttcttcaaccgtcgcgccctcctgcagcgtcactcgctgcaggtactgcttctcaggtagcgcataagccacctcaacggcaattttacctggcactgtaaacctctttcgcacgaaccgtaaaagcctggaccatattagccgccagctctttaaacacgcgaccaaaggcgagttcaatcaacttattggtaaactcaaagtcgagatgaaactcgatacgacacgcctcctggctcagcggcgtaaacttccatccaccaatcaatttcttgaacggcccatccaccagattcataagaatactttggttactggtcaactggttgcgggtagtaaacgttttgctgatcccagccttagagacatctaccgccgcagtcatctgcccaggagtggactccagaatccgacttccggtacaacccggcaaaaactgaggataagactgaacgtcattcactaactgatacatttgctccgcgctgtagggtaccagtgcggtccggctaatctgaggcataacaatttccatcaacaaaaatccaacaaataatatcatttatcctgctgtaaaaaaaacgctatcccggcgctgggtaacatcgggttcatgctaagatagagccttgtcccccgcaggattgatatggggtgttttcgatttcagattaccgatgattcacgacgcttatgacgaagaaaaaagcacataaacctggttcagcgaccatcgcgcttaacaagcgcgcccgtcacgaatactttatcgaagaagagttcgaagcgggacttgccctgcaaggctgggaagttaaatccctgcgcgcaggaaaagccaatatcagcgacagctacgtccttctgcgtgacggagaggcatttctgtttggcgctaacatcacgccaatggccgtggcctccacgcatgtggtgtgcgatcctacccgtacccgcaagttacttctcaaccagcgcgaactggactcattgtacggtcgcgtcaatcgagaaggctataccgtagtggcgctctccctgtactggaaaaatgcctggtgcaaagtgaaaatcggcgtcgccaaaggtaagaaacagcacgataaacgttcagatatcaaagagcgcgaatggcaggtggataaagcacgtatcatgaaaaacgcccaccgttaaacctgcactccaattattgaccagttcctcaccgcgcctccctctccggcggcgcgaatgaacatcttattggctatcacatccgacacaaatgttgccatcccattgcttaatcgaataaaaatcaggctacatgggtgctaaatctttaacgataacgccattgaggctggtcatggcgctcataaatctggtatacttacctttacacattggggctgattctggattcgacgggatttgcgaaacccaaggtgcatgccgaggggcggttggcctcgtaaaaagccgcaaaaaatagtcgcaaacgacgaaaactacgctttagcagcttaataacctgcttagagccctctctccctagcctccgctcttaggacggggatcaagagaggtcaaacccaaaagagatcgcgtggaagccctgcctggggttgaagcgttaaaacttaatcaggctagtttgttagtggcgtgtccgtccgcagctggcaagcgaatgtaaagactgactaagcatgtagtaccgaggatgtaggaatttcggacgcgggttcaactcccgccagctccaccaaaattctccatcggtgattaccagagtcatccgatgaagtcctaagagcccgcacggcgcaagccctgcgggcttttttgtgccctcaatttgtcccgcgaagtccgaagagaactaattaaatccgaaccttttaggcccattgataggcccaacgaaaagctctattgtttacgttgggcctaaacgcagggagactccccatggcaagaaaaaccaagccgttaactgatacggaaatcaaagccgccaaacctaaagatgccgattaccagctttatgacggtgacgggcttactctgttaatcaagtccagtggcagtaagctttggcaattccgttactatcggcctttgaccaagcagcgaaccaaacagagcttcggtgcctatcctgccgtctcgctttctgatgcacgtaaactcagagccgaatctaaagttttattggcgaaagacattgatcctcaggaacatcagaaagaacaggtgaggaattctcaagaggccaaaaccaataccttcttgttagttgccgagcgttggtggaatgtgaagaaaaccagcgtaacagaggactatgccgacgatatctggcgctcgcttgagagagatattttcccggcaatcggtgatatcagtatcactgagattaaggctcatactctggttaaagcagttcagccggttcaggccagaggtgcattagagactgttcgccgcctttgtcagcgtattaacgaagtcatgatttatgcgcagaacacaggcctgattgatgctgttcctagtgtaaatatcggaaaagctttcgagaaaccgcaaaagaaaaacatgccaagcatccggccggatcaacttccgcagctaatgcacaccatgcgtacggcaagtatcagcatgtccacaagatgcctgttcatgtggcaacttctaaccatcacccgccctgccgaagctgctgaggctcgatgggatgagatcgatttcaatgctagcgaatggaaaattcctgcagctcgaatgaagatgaaccgggaccatacggttccactatctgatggggctcttgctattctggaaatgatgaagcctctcagtggtggccgagaatttatctttcctagccgtatcaagcccaaccaaccaatgaatagccaaacagtgaatgcagcactcaagcgtgctggcttaggaggtgtacttgtttcacacggcttgcgttctatcgccagtacggcactcaatgaggaaggatttccacctgatgtcattgaagcagcgcttgctcatgtagacaaaaatgaggtgcgtcgcgcttataaccgcagtgattatcttgagcaacgtcgtccgatgatgcaatggtgggctgatctcgtaaaagcagcagatagtggtagcatcgttttaactcatttgagcaaaattcgtcttgtcggataaaatatttatcagcccagctctctgggctgatatttctaaaagatcgcactaaatagctacgcggaatagtgctctactttcgtttagccctttcagaggtaagacattagggcaatttcactgtatgactgcgcagtcatcgagtctgtggggtgttgctccttttgcaacgtatcacttgtcaataaatagaaagtgtagatgtattaggcgcagctatttagtctatatggcaagtagtaattatttacttcttttttttctacgaacagcgctatcgaaagcttgttttacatcttcattttttaaagaccattgatttaaaatagtatcaaccaaagcatcttgactcattgttgctacacgatattttttattttgattatttatctcaaactctgacatttgaataaaatcccatagcggttcgataagttcattaactgctacaaccttatttttccacccatcattcggaacagagtcattaattagctcaaccaacttcagttgaatgatatggtacacttccgctttgcttttgccacccttctttcctgcactccgcctgacttctgataattttttttgattacaaacagagatgttaaaccaagtcatacctatgcacttatcaaataactccgcagcccgatgaaatgctttaaaggcaacgttttcattttcagacatgatagattttccccagaaaaaagagattgaggcgaacataaggtgtgccttgaaaatgtcattaatggaaaatggctcgataacaagaggtaaaaacgtttccttggtaaggtttgaacttagatttttccagcattcttgagctggatcatataattcagtgtattcttcctttatctccagttgcccattcactgtatggtgccttgtttcccatggtacatcgcaggaatataacctcacacgagtacctattttctcagagctccagaattgctctcgcattctgcctagctcaatccgtatttccggatgatcttcctctagaacatcagtatccaccgcccattcgcattcggacatgtgataggcgagatcacgtcgttttctacaaatttgttcataaaaatcattcagagaaatcataaaaccaccataaatcaatgtattagaggttgtaaaaattgtatttttggtacatgggttttttgccttaaagatacccattaatctctctgcaaccaaagtgaaccaatgagaggcaacaagaatgaacaatcgatcggccgttagaatactacggttaccagcggttatccaaaaaacaggtatggcacgggccaccatctatgactggttgaaccccaaatcaccacgatacgatgccacctttcccaaaaagcgaatgctcggcgtgaaatctgtcggatggattgaggccgagattgatgagtggttatcacaacgctgtaaacttatttgagggtgttacatgaattcatactcaattgctgtcatcggagtgtaaacatcctgctatttccgccattaatagcggaatagccatatttgctaaacaatttcttaatttaattaaataagaggcattgcatgttcaatggtcgtcctttccctgtagatgcatttcctaaaattatcaggaatgcaatttatgaagtggaacagcatacgcaggcccctcaaggtttgattgctgcttctgctcttggggtaatttctcttgcctgtcagaaccggattgatgtttgccgattgaataatctacgtggcccggtatcacttttcttaatgactctggctgaatcaggtgaacgtaagagtacggttgataaactgctgatgaagccattatatcaactggaagaggatttatttgaaaaatacacccacgatcttaccgcatggagaaatgatgaagcaatttttaatattgaaaaaaaagcactgatgtcaaaacttaaatcagatattcgacgtaacaaagatcacttggcaacaaatgaaagacttaaagaactacttacgacaaacccgaaagctccagtgagattcaaatttttatttaacgatgccacacctgcagctattaaagctcatctctgtgggcactggcgatcagtcggcatcatgtctgatgaagctgggatcatttttaatggttacacacttaacgagctgccgtttatcaataagatgtgggatggttcaatatttacggtggaaaggaaaaacgagcccgagaaattaattagagatgcaagaataacactgtcgctgatggtccagcctaatgtttttaagggttatatcgacaggaaaggagatatggcaaaggggattggattttttgcacggtgcctcatgtgccagcctgcttcaacacaaggtaacagaaaaatttccaacccaattttttcaaatgaacatttgccggtatttcaccaacgtcttatggaaattgttaatgagagcatcattaaaattaatgaaaataatcgcatctgcctccgattctctgcagaagcagaaagacattggatcgaattctacaaccaggtcgagtcagaaatgagaatgattggccttctttatgattttaaggattatgcttctaaaatggcggagaacatggcgaggcttgctgccttacttcattacttcagcggtgatggaggcgatatatctgttaccgcagtaaaagcagcagtggagatagtggcttggtatattgaagaatacatccgcttgttctctaaaaaagaagagttttctttagatgtttcagaagcagatgagctttattgttggataaaagattactgcacgcaaaaattttcttcctgcatcaagaaaaatattatcttacaatttgggccaaataaatttagaaatcgtgacaaggcaaatgaattaattagaatcttaatttcacaaaacaaaatatttatatcttcatggggtaaaacaaaaataataaacataactcattgtgttttttgattttaatgacaatctaaaaggacttaatttaagagtaaaaacaaactctaaacccagttcggataaaagcttgtcatcttgataggtaatatataggtacatagacacatcagaacgatcacttactccaatatcattggccaggatactatatgacatacgatagtgaattcggatcacatgtatccctatatcgggatagaatcaaacaggttattgatgactccctaaacgaacatcttaactcaatgattctacgtgttgatctgcatgacccaattgatacagaaaatatggataacccattctttcaacccagggttgactctggtgctatatctcgctttaccagtgcgttaaaagcaaagcttaaacatgataagcatattaaaactcaacggaaagactggcctgatagtcgacattccactttacgttacgcatgggtcagagaatataccaaaaatagaaagcggcattaccatttgatactgtgtttcaatcaggatgcttattatcatttaggtgattacgacttaaaccgtaacacgttacgtacaatgataacgacagcttggtacagtgcacttggcatccctatagatagctcggggaagttagttaattacccgccaaatggcaaataccttctcaatcgtaaaagggacaactttgagcagacttatagcgatttgatgaatagggtggattacatgaccaaagtaaggactaaaatagtcggtgacggagaccgtaatttcggctgcagtcgcgggtaatttattttttacaacaatggcctttcttatggctggaaaggcctgatttgtttgtattaagatatcggtaatcttttgatggttggaagcccgtcctggtagacgacctagcctaccgaagatgtgagttattcaaaaatgtcgctttcccgcgttccgtagacaaacgtacctaaatcaatgtcgtctaataccgagcgcgcgcctgataaacatctgatcaacgtacccaatcgatctactccaaatgtcctgagtatcccgaagatactggctcaactcatccacatcagcctcgtcggaaaattccagcaagtctaccagtcggtgtaacgtctgaatgggaatgccaatctcttctaaggcattgacacctggtggtagatggaaactttcgaacgccaatttgacatgtgtgtaatcgactttgctgcgtataccacgctttacagcgtggtgtttaactacatcctccatcaagctgagcaccttaggtagggtatagccgaaggtattggttatgagcttcaaatcattgttgagggcaatggaaagagtacgtttctccccttcagaaatccactgtcgtgcataatcgatctgatttttcagatattccgaataactttcagcacttaaatagccggcaagttttgcgatcatgacatccgtaggcttaacagggaccccattgcgactgaacgtatggggaaccagtctggcaatgatctttgcaaaggtcttgaggaagtttgtcgcgggagtccagtgaaacactaacgaggaaaattcgttatcgtccatcatctcgaacatgctttgcagcatttcgaactgctcgacacggaagtacgaatgcttcttcacaaggtcgatggaaacacggtcgtttatgaaaacctcatcaaagcgatcctgtgaaaactcggacaagtggtctggttgaacgctggctaacaggttgattggggtatcaatgccctgaataccgagcggaatatccacctcttgattgagattgtcttccgggatttcctccaggcaaaagattttgccgacgaagtgaacgcccatgcgcccggcgcgacctttgatgttcccatgggtgaatttgtcaatgctgcgagttccatcgcggttgtcgtagatcacaacgttcttagcgatagtgttgactccttcaatgatcgtggaggtgcagagcaaaaagcgcagttttccagcattgaattggtcggcagtgtattgctgcagtgccctcggtagcgcgccaaaatgcaagccaataccgtttctaagggcgactgtgtaatcccagtcggcatcgaactcttcgctgacccagtcgacatggggattctcagtcggagtgccatgcccaagcctgatcagctcgcgcgccaccaggcccgcaacagttggtgacttgcaataaatgatcgttgcgtcgacacatgcgtgcgcgatttcccccagcgctttgagcttggctttgtcgtcattcgctttgatgccgaacgtcttaacatctagcgcgactgtattgaagtcggtagaaacgaaagtatgcggatatccaagtttttcgagaccgcgaatgctgttaacgaacggtcccgtcaggtaaaactgcctggagaccttaagcagtttgcttaacgcaatgttgagctcgatgactcgttcgtcttgatgatcaatgtccccgcttttcagttgtcggaacgccaacttgtaaaactcgtcaatgacgaagaggtcaatgtcgacgatgtcgtcacgctcgttcactcgctcctgagttaacacataaacagcctgatcggaatggcacacttgggaactgtggtggatgatctgatatcggtcaccgaatcgctcttgcagtcggcgacgggtttcgtcggcaagagccacggttggaacaaccagaacaagccgtttcaaagttcccatgccgagcaatgaatcgacgattgcacttttgcccatgcttgtaggtgcactcagcaccacgttttgaccagacttgagcagatcgaatatgtggaactgcattgagtggaaaacataaccatccgagaatggcgtccggtatagctcaagcaccctcaggtcatccggtgtcaggctggtgaactcctttttgagatacgggaacaaacctgattttctcaccatatttttcaaaattgtggtgtgctcggaaaaccgctcgcgcgaatcgagagctcgcacgatcaagtcccgtcccaagtcatacgaaacagggttagacaacagcttgttaaccgcaaacagataattgaacgatgagaagtcctcaccctgcaggctatgtttcgcctgttcatagatctctgtcatacgacctctctcaccttctcatcaactaattgggttaaccgctcaagactcggggctggataaatgaatacgtggatgcaaagattcgcaaacggcgaatcctcgatgaggtcagccgcgaatttttcgaacagcaccgctgtttctttctccaggtcatcctcgaaccccggcgtttcaggctcggttagtagattagagtcgtagcccacgaacagaacaaacgtgaaacgatcgaggtgagcatcgaaaggttggctgccatcaagaatttcgtcaatgtcgtggcgaagcaggtagttatcgtctttaatgtcgaggatttttttgcgcgcggtatcgatgcaatccgaaatgtcctcgtacaactgatcccgtatctccggcaatctgacggcaatgttaatatcagtcaccaactcgctgaagccaatccaaagctgatcaccttctggatcgcggcgaacgatatgcacgttttcaagaattttttcggcccctgctttttccacgtatagcatgcaaggaataggctggctttcgtggtgctgccggatcgttgcgtgcaacagcactcgacccaaaaattcgctgacgtcatggagcgatttgaagacggaattctttagtcgttctcgcttttcaatgaatgtcagtttatgaatatcagacatttcttttggtcggagaaaaacctcatccaaccattgacagacgttatccgcgatgtgcttgtagcggtatttcttaagtgagtactgctgatgtagaacctggcctttacgcttagcgcagaccgaagccataggcgctctaaatggcgtaaggatgtggggtaagtcccgtttgacgtagattttgcggcctgaccgagattggtcatcttcgacacgctgcttgaaccactcaagtaggtctggtcgtaagtaggacttgtcatcagcactgtgaatgcgtcgagaatgctcgcccttgcgcgtcacagtatcaaggatgcggcaccaaatgtcttcggcgacggtttcggaactgagaatgaccccatgtagatcttgggaggccagccgtatgttcttgatccctagaagttccagttcgcgcagggatgaaaacacttcccatgtagccgcatcgatccaatctgaaacgcttatacctgagtctgttaaaaaattgtctgtgcgtttgttgaggtcatcgatgagttcctgtcgacctggcttatctagtcgggcgtttgggctgatcgtcaagtactcaagggttttgttgaccttttcctctgtgacgatggagtacctacgtccaagggacaggtcagactcacactgcattgatttgtgcaaaattgaactgcaggggatcgtctttttatcagcaccttttgaattctgaacgatgtccgaaatgttccaacgtgttttgccggtgctttttacctgaacgaagtcgatgtatccatcagatacaatgtcgatatcgtctgtgacctcgcagcgcacactgcggatagtcttgtcacgaagcattcgggtgacatggtaagcggctacgcagtcctgaaataagaaaccgtgcttggcggctactccgcctgaatcgttcgactccatttagacatccgtgacaattttgcgaaaattaaggagatgttatgacacagtccaatcggatcactgcatcatcaccagtgatctaaatacttcacagccattctcggtcgcaggtatcaagcttttcaggattccacaaatattgtaaccctgacgtctaatttggttatataacatactgccccaactaacgtaaggtaggcacagccttaatcaaggttttggttttcaaatagttcagagctgagaccgccaaccgcactatggcactatggcactatggcactatggcactatggcactatggcaccgccagcgattgtaatcacacttgatattataaaacacagttgcacgcattatttcctggttggtagggtcatatctcgatgctctttgagcaatgtcaacatcgcgtgttcatggctttctatattgttgatgccttgcccatccggaccccactccttatagctcatcatgatggcttgttttgggctctctgctcgttctgtttcgacgtagaattttttcttgtctgctggcgaataattactaagtatcgagttgctgcttggtgagatcaggaagaggttaccgaaacgatggacatcatcccccattttgtggactgcccccccggtagacgatcctgccctatagttggagtgccccctattcaggtggctaaatttagcaaatcaatacacttcaggggggtattattgtagagtttccccatatgtttctatgggatccaggaaatgacaatcaggagttacaaaaacttaaatctggtcagggcaaatatcgagactgaatccagacaattcattgaaaataaaaactattcaatccaatcaattggtcctatgccagggtcaagggctgggcttcgggtcgtatttaccagaccaggggttaacttggcaactgtggacattttttataacggggacggttcgactacaattcaatatctcactggagccaatcgttctctgggccaagagttagcggatcatctttttgaaaccatcaatcctgctgaatttgagcaggtaaatatggtactgcaaggatttgtagagacaagcgttctacctgtacttgagctatcagcagatgaatcgcatatagagttcagagaacactctcgtaacgctcataccgtagtgtggaaaattatttccaccagctatcaggacgaattgactgtgagcctgcatatcacaacaggtaagctccagattcagggccgaccgctgtcatgttacagagttttcacgtttaacttggcagccctgcttgatttacagggtttggagaaagtgctaatccgccaggaggatggtaaagctaatattgttcaacaggaggttgcccgcacttacttgcagactgtaatggccgatgcttacccgcatctccacgtgactgccgaaaaattgctcgtttcagggctatgtgttaaactcgccgcccctgatttgcctgactactgtatgttactttatcctgaactacgcaccattgaaggtgtcttaaaaagtaagatgagtgggttaggcatgccagtacagcagccggcaggttttggaacttactttgataaacctgctgctcattacattctgaaaccgcaatttgcagctactcttagaccggaacagattaacatcatcagcacagcctatactttttttaatgtggaacgtcattctctgttccacatggaaactgtggtcgatgccagccgtatgatttctgatatggcccggttgatgggtaaagccactagagcgtggggaataatcaaggacttatatattgtttgaaatcaccggaattaacgtctcaggggctctaaaagctgtcgttatggcgaccggcttcgagaaccctttgtcctcagttaatgaaattgagacgaaactttctgccctactgggtagtgagaccactggtgaaatcctttttgacctcttgtgcgctaacggtccagagtggaaccgcttcgttacgctggaaatgaaatatggccggatcatgctggatacggccaaaattattgatgagcaggacgttccgacacatatcctgagcaaactgacttttactttacgtaatcatcctgagtacctagaagcctctgttttgtctcccgatgatgtacgccaagtcctgtcaatggatttttgaaactcttctttctaaacgaaccagtatagaattcgcccttttggcatgatattaacttgtccaatatgatcaaatagcattaaccccccctcacaacgtcctgcatagggaacacgttttcccctgtgcacccacgactaaatttccccccctttaaacttctcaataatgtcaccaattttctggaaatcctatgatgcctttcccggtaaatggtgctgtgagttcagaaagattctgcaatctatgtgcattgaaaaaatcttcagatagatatcattctcctgaacaatccgatgaacggcagaacctcgcggttctgccgtttttgttttacttttcagaggagtggtgatgaaaaattttgaagttctgcagccactacagaactccctttccggtctaccgctatgggtatctgaacgtatattgcagcagataaatcagttaacccactacgagccagtgatcggcatcatgggtaaaactggggcgggaaagagtagcctttgcaatgccctgtttgccggtgaagtatcgccggtcagcgatgtagcggcctgtacacgtgatcctttacgctttcgcctgcagattggagaacactttatgaccatcgtggatctgcccggcgtgggcgaaagtggcgttcgcgataccgagtatgctgcgctgtaccgcgaacaacttccccggctcgacctgattctgtggctgattaaggctgatgatcgggcactggcgactgatgagcatttttaccgtcaggtgattggcgaagcataccggcataagatgctgtttgttatcagccagtcagacaaagctgaacccaccagcggtggaaatatcctttccacagagcagaaacaaaatatcagccgcaaaatctgcctgctgcatgagctattccagcccgtgcatccggtgtgtgccgtgtcggttcgcctgcagtggggactaagggtgatggcagagcggatgattaagtgtctgccgcgtgaggccagcagcccggtagtagcgctactgcaacatccctttcgaacaacggtagcccgggagcaggcacgtgacgatttcggtgaaaccgtaggtgccatactcgatacggtaagcacctttccccttattcccgccccggtgcggaccattattcaggccgtgcgttcctcggtggtgtcagtggcccgcgctgtctgggatttcttcttctgagtgtttaattctgccctattattctccgagccctgtcgcaagtgcggcagggctttctttatttgttttacccatactgaggagtctgcttatgacccgtctggcttcgcgctttggcgctgcaaatcttattcgccgtgaccgtccgttaacccgtgaagagttatttcgcgtggtgcccagcgtattcagtgaggataaacacgaatcccgcagtgaacgctacacgtatatacccacaatttccctgctggacagcctgcagcgggaaggcttccagccattctttgcctgtcagacacgggtacgtgacccccgtcgtcgtgagcatactaagcatatgctgcgcctacgtcgggaggggcaaattaccggtaaacaggttccggaaattatcctgcttaactctcacgatggcaccagttcgtaccagatgctgccgggcatgttcagggcggtgtgccagaacggtctggtctgcggcgagtcgtttggcgaggtgcgggtgccacacaagggggatgtggtgagtcaggttattgagggggcgtatgaagtgctggggatttttgagcgtgtggaagaaaagagggatgccatgcagtcgttgcttttaccgccacctgtgcagcaggcactggcaaaagcagcgcttacgtatcgctttggtgaggaccaccagccggttactgaatcgcagatactctccccacgccgctggcaggatgagagcaatgacctttggaccacctatcagcggattcaagaaaacctgattaagggcggactcagtgggcgtaatgctaaaggcggacgaactcatactcgtgccgtgcgtggcattgacggggatgtgaagcttaaccgtgcgctgtgggtgatggcagaaacactgctcacgcaactgcagtagacgtttcatgttgccacgttgttaatatcggacaccacctgtccgcatcgctatgtgctcgtgtgcctcaatcccccggttatagcttttaacccccgttacatctggcttttgcagaaataaaaaatagtttctgcgttgtccataccctgtccgcccccctctttaaagtaatcacatcattttcagtcagttaactttcctggagaatctctcatgacacaggcagaacgccgccatgaccggctggctgtcaggctgtcactgataatcagccgtctggttgcgggtgaaacgttgagcgtgcgcaaactggcggctgagtttggcgtgtcagtgcgcacgctgcggcgtgattttcgtgaacgactgatgtatctggacctggagtatcagtccggatactgccgcttacgcactgctggcagtgagatgcagatggtgcccgacgtgcttatctttgcccaccgcagcgggctggccgggctttttcccggccttgaccgccgtctggtgaatgcactgctgatgtgcgatgagtctccctgcgtgatagcaccagccaatccggttccttcgccttcaggagcattgtctttctggagactgattcaggccattaccgggcgcaggcgggtgacgctgattgcagaggggcgacgctgtgagcgcctagctccctgccggttactcatccaccagcagacctggtatctggtggctgaacacgaagggcatatcgccgtattcacacttgatgaaatccatctgattcagcctttgcaggagacttttcgccgcaatgacagtctgtgtcgcctggttgaagacccggtcttcattcaggccttaccccattttcgctttatccagcattcactgcttacgtttgttccggccgacagcccaccggaatagcgcaggcgttgttatcaacccggcaacatggaggagcccagtgcccgttattgccattatcgccattgttatcatcgtcatcattctgaacaaaaccggagtgtccgacagcctcacggccctgacacttgcaaccgttgccgcactactgacgggaggtggtgcagccggtgctgccagtgtcgcgctgacgccgttcgtcggcgtgccggtgggtatttttgtgggaatttatgtctttgccaaagtggttcgtctgatttcagggaaaaaataatgaaacgtaaaacactacctctgctggcgctggttgccacctctctgtttctgagcgcctgcgatgacaggagtgatgacctcaaagctatcagtaaatttaaggacctcacgcccccgcgcttcagcgatgtggtcagccgtcaggatgatgtcagcgaagaatggtcacaggttggcttctcatccggtctcaccctgcaggtcttacgtacccgtgagtcgcccgatggttgcgagggtggcagttactactatctggtagatatggaggagaaaaccgtccagccgctgatgaatgcgctttgtattgccgacaatatcaaactggaataccacgaagttacggacccgtatacgaaagaaaaatacttcgaatattcccatgacggcaaactgatgggacggctgctgataccgtcaaaccctgataaccgggaataaaaacaacgagaaaggagacataaatgaaaatacgttcactaagccggtttgtactggcaagtacaatgttcgccagctttacagcctctgcggtccccggactctggcaacaggggtacggtcagggcaatgcggaatacagtgtgacggatgccagcggaaagatgtttaccatcaactgcacgggaaatccggaccagaacggtatttaccagcactcggtttttctgatcctcgccggggataaaacggtcagctcgcatgatgacagtaccggcatcacagtggtgatggaccataagcaatatgccattccctcaacccttggctggcgtaacggagataatgcctggttcagcttcatcatggatatccgtaaggcccggcagttcgacgtctacgtcaatgaccagaaagttggatcgtttaaccctgatgttcggaatgcacaaaaggtcctgccaacattagcggactgcactaacgactgacggctgcgccttccctaccataacaaccctgattgcctccggcggtcgggggtttcttttttctccttaatctccagaggtaggccacgtactttcgaacgatgagcgcagtggtcagtttttttcagatatatttatctttttttggctgtaagctccgctgtgagcgcaggctgtgttaaaactcctgatcactttttggtctaagcgatggtttcatatgatcaaccattcttgataaacccatgagacggactaactttttcattaaaattaaaaagatatgaatgaatactgcggatatcaacatggccaatcacattcaaggacaaggcaggcatcaggtgacattgctccctgatgcactcgatgattttgtcactgaagatatctgaaataagtttaatcagttcatcacgggtcggtggcatatcgagataattaattattgtcggttcgttgccgttgttatgaagcatctccagcgtgttgcgtgaggtgccacaggccgggttgtgatagatggtaatgttgctcatatcagtatctaattacaaagtgacagagagccgccacgccagcgcggccagagtgacaaacagcaccggcacagtcatgacaatgccggtacggaagtaatatccccaagtgattgtcatatttttctgggcaagcacatgcagccacagcagagttgccagactgccaatcggggtgattttcgggcctaaatcacagccaatcacattggcataaatcattgcctctttgacgacgccagtcgccgtactcccgtcaatcgacagcgcaccaatcagcaccgtcggcatattgttcatcactgatgagagaaatgccgtcaagaagccggtgccgaacgtcgctgcccataaccccttgtctgccagcagattcagcacgccagacaggtactccgtgaaccctgcattgcgcaggccatagaccacgatgtacatgcccagtgagaaaataacgatctgccatggcgcaccgcgcaggacttttccggtgttgatcgaatgacctcttttcgccaccacaaacagcactgctgcgccagcggccgctatcgcactgaccaggattccctgcggctccagaaagaagaaaccgacaagcagcaataacaggacaatccagcccgccctgaaggttgccagatccttgatcgcactggcaggcgtcttcagcagcgaaacttaatacgttgccggaataactctgcgaaagaagagatacagcataatcagcgtggccgcaatcgctgccgcatccacggagatcataacggaggcgtactgcgcaaagctcagaccgaagaagtccgccgagacgatattcaccaggttagaaacaatgagcggcaggctggccgtatctgcaataaatcctgcagccatgacaaaggccagtgtcgtgccctggctgaacccagtgcgatcagcatcgcaatcacaatcggcgtcaggatcagcgcggcgccgtcattggcaaacaacgcatcaacagcggcaccgagcaagactttccaggtgaacagcgctctaggtaggaactttgtcgttgatagagtcttcagccatcaacactgtatcgagtaatgaaattggttgctagaaagtcgatgatttgttgcgtatgattaaaaatcaaccttaaaggctttatacatggatttgctatggcttttgtatcagaaagagaaattgtaagaaagatatttagcaaaaaaattgactttacgatcttggcatttttctatatttcctctattttttttcttctttgtagtggcgttctctttcaatattttaccgctgccttcacaaaaggtaattgttatgaatgctcaatgaaacttgattacataaaacaattttatttttcactggaaaccgcatggtacctcatatctgctgttgcagtatttattgcatctgtttttatacagcatagaattaaagcttatttaacattattagctattacatggattgtactaacaataacagatgtggcgttaatacacgccttagacaatatagccatgaataatattttgttaaatatactatataatctttttggggcgattttattgtcactgtttatgtgtttatcaaattccctccttttccaccttaataagataaaacatattccaatgattttatcggcaatgattccattagtttccgcaataataatagccatactcataaccgctgttatatatttattgtttgcccggcaggcggtagagattgagatggatatatctgaaggttcagacatcgcatatgtaggtgtaaaagataatgaggaatcatttgggtttttaaatgataaaaaaacagacacaccaacgtatctggatgtaatcaaaaatggtagtttgatatataatgatacacagggtttaagtggtgctgatatttatattgtctccggttgttatgcccttccagatttacttcgcaatgtaccgcttgatgctaaaaaatcttttctgaatgtaaaaaagctagaaatcacacagaaacttccaatgatggggttcatacaaggtgaatccgctgatgtgatgcctaaagcagcatccaggttaagtttgagcaagcaagatgataaatttatgctagcctcaagtgttactgactctcaaataaaatttaaatcaaacaatgcacaattgatggttgctttcgcatttatgccaataacaacgaatggtattttacatgattatacatacgatataataataaatgataaaaaatataaaattgaaaatcatgttgcacctctatctaggcttgataaaaataagaagatgaagtgtgaataccagcaaatatcggatttaacaaatacgtataacattaatgcaaattacttaacgggttttttacttgtcctaaaaccagatgatattattaattacaacaatagcccttccgtactactcaagactgattttgcgttctataaaaaaacataccagaagcttgataaaatatatgatgacataagcaatggaaaattatcttcactgagagcaacaggtatctcccagtttagtatcaacgggaaacatttgtcgttaaggccagaatcggagattattatttctgaagggagtttgtatggactagttaataaaagcaaaaaaatcaaaatatatggcacagcagatcttgtttttgttgataacaagataatgaaccttcgtaaaataacttatttgcaatctaagctagaaatttttggttcttctattatggatatattaaagtatatatttggtttaggtctgctagcaatttctataaaattcattcattcttactttaagaatgatgtgaatgaaaatttattcttgtaacgcatttggctccaattggagcctttttatgactatttattaaaatatcctaagttaagcctgtttttaaagcaggcttgagcgtgaagcggacactcatacctgctttaaagtggcgtttttgtcgttacccatacctatattttctgttgtttaactgccagaactgagcggttgaaaagccagaaatatgccgagccagcggcatggaagcgccagcagctgttgaatggagtactgtaggcaaatggtgccgtaaccggctttcgtactgaaaggttctgtctatcccatcccttctcttgtatctaacatttagttgtgaatagctactgtaaatgcccctacaaaatgaaccattatttttagagggcgtctggcactccaacttccgcttttggcacagaacggcctatcagcaatataaaagcattcagatatatatcatttctacaaacatacccgattaacggcagaatctcaggattctgccgcttttttattatttttcaggggagtagtaatgagcaactctgaaggttggtagtcattttagcaaacgctttctggtctgccgcagtgggcatcggctgattgcgtagcagggccactggtatctgccggtatcaccgacattaacattgaagacgaccagggcattcacgtccgcctgatagttcgtgatgccgaaggtcggatggttggcgggcatggaactttgaaccggacgccggtgaaggttttaaccgctatatccacaggtcaggcatccgcaccgacaccttcccccgctgactccgaatcatttaccagcaacatttcaccttcccaaacgcgctttattacctcatacgccagccatcgccgctggcgttttttattcacggagacatacccatgacaacacagacacagtacgacctcgtacccgctaacggatccgaatttgagttgagcgtaacgcaggtacccgatgaacagcatatccgcttctggccgcagcactttggcaccatcccgcagtggataacgctggaaccgcgcattttcgcctggatggaccgcttctgtgatgagtactgcgggggtatctggtccttttacacgctcagcaatggcggagcgtttatggctcctgatgctgacggtgacgataaatggcatttgctcaacggcatgaatggcaatggtgcggaaatgagcgcggaagccgcaggtatcgctgtctgcctgattgaatatagccatcacgcctgcctcaccgaatgcgatgccatgacggagcactattaccgcctgcgggattacgctctgcagcaccctgaatccagcgccattatgcgcattattgattaaggatactcatgatggaacagtcactcatcccacagacaccggtacttccactgaccgcacaacgcacggtaaaacgcgccttaacgctgcttgaccgacacctgcgcgaaacaggcgtggcattcacctccactcaggctgctcgtgactggctgaagctgaaaatggcggggctggagcgtgaagaatttatgatgctgtatctgaaccagcagaaccagttgattgcccacgaaaccctgtttgccggttctattagcagtaccgaggtacatccccgtgaggtggtcaaacgcgccctgtatttcaatgcagcagcagtgatactggcgcataaccacccctccggcgacactactcccagccaggcagataagactataacgcagcgtctggtgcaggcgcttcagctcgttgatatccgtgtccctgaccatctgattgttggtggcaggcaaatctattcgttcgcagaacacggtctgctttgaggtattacatgagaattatcagtaaacgccgggcaatgacgatataccgccagcatcctgagtcccgaatctttcgctactgcaccggaaaatatcagtggcacggtagcgtctgtcattacaccggcagggatgttccggatatcacaggagtcctggctgtgtacgccgaacgccgcaggaccgcagcggaccgtatgcttgactgatgagtatcaccctgaactgacaataaagaggttatgaatgagcaacaccacatggggcctgcagcgagatatcacgccgcgcctgggagcacgtctggtgcaggagggcaaccagctgcactatctggctgaccgggccagtatcaccggtaagtttagtgacgccgaatgtcctaagctggatgtggtatttccacattttatcagccagatagagtcgatgctgaccactggtgaactgaatccccgccatgcccaatgcgtcaccctgtaccacaacggttttacctgcgaagccgatactcttggtagttgcggctacgtatacatcgctgtttaccccactcaacgctaactaatttcacgagagcaagcatgaacactctacctgctacaatttcgcaggcggcgaagccctgcctgtcgccagtggctgtctggcaaatgctactgacacgcctgctggaacaacactatggcctgacactgaacgacacgccgttcagtgatgaaactgttattaaggaacatatcgatgctggtatcactctggccgatgcagtcaattttctggtggaaaagtacgaactggtacgtatcgatcacagaggattttcgtggcaacaacagtctccatatatttccgtagtagatattctgcgagcaaggcgctctaccggcttgctaaaaactaatgtgaaataaacgcttaaatacagagcagactgaaggaaagcaaaatgctaatctcatagacgaagagactcccgctgtaacctcccctcccccgaaaaaacctgacattttcttttaggaccaacaatgggaccaaaatgaaaattgaactgaagattacaatcaatttaacaacaagttacacaaccaattcagactccgccagcccaccaatcatgattggacggtgtaaggacaacaccaacaaaaacaggaagttagaagtctcagcaaaacaccgaccagacggtgaggagacataaaaggatacgcaaaggagccgcggctcctggtaacatgaaagcccacagatgtgggctttttcgttgatggtcagaacgaccagttcacaccagctaccgcgttccacggggattccacaccggcactatggctataccccaccccaagatgcccgcttaacgtactgctgaatgaggctttaatacctgcctggtatattccacgtctgcccgacaaataattgacgaaattaccgtcactattcactttcacccggttatcatcgacaaattctttgcgcacagccgccttcagccacggctcaacttccataccgttccccagacgcatgttgtaactcagcgttgcgcccagttcacgatatatactgcgggtatcgactgatttcgatttcatgccattggataaatgatattcggggttatcagcggtgaaccccgttaacgatgcatacggcgtcaggttccagttaccatcggtaaatcgcatcccggtttcaatgtgaccgcccagcccgttgctgtggtaactgccattggcggctccaccgctgctcattttacctgctacgttacttttaaaacggttcagcttcacgacaccgtccagatagaaaccactttcatgttcccaactggcatagccgcccagagaataactgcccacactgccatgtcctccgcgatcaaaaccgatatgtgaatgggaatagcccataaaagcgcctagcgtggtaattccttcaggaatatcattacggctgtcgatccccactgtcattccggtcagcgtctgctcaaacccggcacccgcatcggtggtgacattattacgggtgttatacgtcgccccccagacattattgttgtgtggactcgctttcattatgttcaaccgctcgcgaatactgtttagctcagcatcaaataccaacggtaatgttgctgccatattgagtacggctgccgtagaaggcgtaatgcgtttctccggaacgggtgtcggcgttggatcgggagtagggtctggttttggatttgggtctggctttggatcgggttttgggtctggctttggatttgggatggggtccgggttgggtttgacatcattggtcaggttccagttgctgttgccgtcacttttcaggacatactcataggtcccaagatcaacgaaaccgccggtattgcccagcgtaaacgaagcatcccctccccctgttttcaccagcgtcatcgcgtcgtcagactgtgggctgacgccggtatcctgaacaaagattttaaaattaccagtggcgttgttgttgacgaccagttgatcgccccgggagcctgcaacgttggtatgcaggtagaaattaccgctaccggaaagttcattggttgtcagcgtattgtagataccgttagttgtggcaggcgctgctgtttgtgctgacaaataaacatcaccgtcgttgagtagcaaactgtttactctatattcgcagttgctggtacctgcacaggaattattgctgttaagccagacactgccccggctggcagccgtcaggtcggcaagcgtggtatcgacgccatttcccagagtcaatgtcgcgctatcggtaatccggaccgccccttcgagtttaactggcgtaacattatcccgtggcgtcattaacgacaggcttcctgtcgcgccactgaccgatgcatccgccagcgtacctgcgtagacgattgccgtaccgccagcgacctggagatcttctgcccgggccagagcctgaaactcatcttttgaccgcccaagggtatattgcccgccagagttaacctttgtggcggagtcctgacccaggttttgcattgccccacccttgccaaccgtggagtcgcgagcttcggtacctgctaataccaataaattaccgccattttccagcaacatattggtcgctaaattgccggaaatggaaaaagtaccgtactggtgagtaccgctgatttcaataccgttagccgtgctcgtctggagagcggcaccgctgttctggacgatatctgtcgctttgccattatcgttgactgtcagcgtaccgccttcattgatctttgtttttattgcctctccgttagctgaaactgtttgtattccgccgtcgttaattgttgtctcattcgccacaccctcgacaatttgttcaccgccggtgagcgtcgtgcctgtcgcagtggcttttgttttgacgatctcccgtccgcccatattgacctgtgttttgtcagaagaggtgtctgactccacggttaacacgccgccatttgccagcaggatattgttcgccgcaccctgctcgatgctgaacgcgacgccatccgcgcgtgttcctgtgacccgcgtcgccctggtggttgcaaccaaagcgccctggctactctgctgtatccccgttgcgctgcctttctcccgcacatcgagtgtgccgccgtcattaagcaccgagttttcagccaggccgccctcattaactacctgtgaacccccattaataatggaaccttccgctgtcccgtttgccataatttgttgtaggccagagacgatatcggtattgattgccttaccataattctgaacggtttgcgtgccaccattgatgtgtgttttctctgttgacccaccatcaacaatttgttcaccactttcgatatttgcttcagtggctaaaccatataccgtttgcttgccacctttgatatttgctttatcagaagtggcactggcatatattgtttgggtgccagcactattgagtacagtgccaacatcttttccataaacatccattttgccgttggcattaataatcgtgtcaactgcgcgggaaccagtgacgactgttaatgagccagcgttttccagcactacatttttagcttctgaattcctgatgtagaaagcatcaccataactgttggttccttcgataagtgttccggaggtcgtggaagcaattaatgcgccgccggattgttgctcaacatgcttagcctcaccaccgtcctgaacctccagaacgccgccattattaagtctggtgctatctgttttagcctccttctggacaatcagcttaccgccagtatcaatggtagtatttttcgccgaggttttagccactaccgtcagttcgccggtattttccagcacaacataattagcctcccctccggtaatagtgaagtgagagagcttgttgtatccttcgatatcagtccctgcacccgtgttggcaactaaagcactgcccgtctcctggttaaccccatgtgcaataccgccggtatagacaatcagcgagcctccggcgctaatattgctgccaattgccgtaccatctttctcaacaacctgccggctcccggaggatataattgttgtgtcagctttcccgccgcttttgatattttgcgttccgctgttgatattggtgcctgtggctatgccataattattaatattctgtgtgccaccattaattatggtatttgtcgcgtttcctgcaacatccataaccccgccattatctattcgggtcgcatcagctttagcattggttaaaactgacattgttcctttatctttaataatcgtcttgtttgccgaaccatatgcgtttatgtctaaatgaccaccgttttccagcaacacattgtctgccacgtgattgtggatggagaatgcaccttcactattcgtaccgctcaccgtcgtaccgttagtgttagtttttaaaattgcaccatcgtgctgggtaacatttgttgccgtaccacccctaacatcaagcacgccaccagaataaacttcaataacatccgaggtgctggtgttatcaacaatttgcgtgccaccagaatagatatgcgtattttttgccgttgacttactattcagagactgagttccgccttcaatcgtcgtgtccagcgcacggctctcatatactctttgctcaccgccatttttaatggttgttgtttctactgtgctctgttcaacatactgtcgaccaccatttatggttgtgttcgttgccagacttccttgtactacgtcctgagagccagacttatttatcgttgtaccatcagcatgcccttgaacttttactatctggctaccaccatcaatgagtattccattcgcactccctccctctacgcgtgaagcaccgcccttaattgtcgttccattgctgataccccctttataaacgtcctgattgccactctcgattgtcgtacctgtggaaatacccccgtcatgaattgactgtctgccaccgttaatggttgtattattagcctgccccacaaaattgttatgacttcctatatcttgatatccaccagattcaataagacttccattagataccccgccatgaacattctgctggccatggttgataatatgagtgttatttgttgtacctcgttcatccactttttggttgccatctacagtctcatcgtttaccacaccaataacattagtagtgaaggcagccatcccgggcggggcatatatcaaggcagatatcaataaggaaagtactgagcggcgacaataatagggactggtcctgttcataaatttcatcctctgaaaagtgaatactgagtagcgtttaagcgaccttagctttgctgcaacatcagcccacaggcaccagaccaggggattcatcctgaagagacagcgcaagtgtattgtgttcaccgctcatcaaagacatcatgatgaaatgatgatattccgcataagaatgaggcattttttaaacgcagtgcgctgaagtgtggttggataaaaaagtcaatccattcaggaaatacgggcgtattcttttctttcgacaatgaggccgttggcaaaataaaatgatttacataatcgtttctgatgaatatcttctgctcacataaaaatcacacaataactttgagatcgcagattgttttacttttacagcattcgtccccccattgttgggcaaatatagattgggccagagcacgaaagttaataccacgttcgcacagctcctccaacagcacgacaagatgccacatactgcgccccagtcggttcagtttacagactagcagtgcgttccctgccgatgatgtcctgaccagttttttcagtccggacctcctgccacggttttacgttgaagtggtaaccctgagcacgcagttcttcagtcaggcgtggtgcaccgtaacgctgttattgctgggtaagatcaaaaaactttcaggcagctaaggaaagttgaaccagacattagatgaaatatttcaaccaattacagcaccaattcagtcactgccagcccaccaaataaatcaaggggttacatgaaaacgtagcccctttttctttggtagtgacactaaaatggatgtagtgtgaagaataatcccgtttactcaatcaataatacatattgtttcaatctacgttattatctctttgtaaaaattgccatttattaatcattgaaaactgcttttagaacttgatacaacgggactagtcacaacaggactattctcaacgggatcatcctcagaggaactatcatcaaagtcatcatccataaataaaatatcatcgaatggtgccacgcccgtgatgagttttattttattattacgatcagtcaatactccacttaaaccgttttcgctcacaggttttaatgatttttcattactcttgttgtaagcaggcgcattaaaaatacacggagtatcaacatcaaacaatgacgttccccagttcacatattgaatatcatagttactgaagttctgtccagaaaagaagcaccccttaaaatccaatccacgtaaattatataaaccaccctcttctttttggagagtaatgttaattttggctatctcccggacatcatcgccatttttgtatttgaataccgtttcaagatgttctccagacagcttgacttcaggaaataatttgaaatcaaagcctatattattatgtgtcaacgtagatgaacaaaaaatggaaaaagcttgcagtgctgaattatagctatcgattttatcttgaggctgagctcttggtaaaaacttatagcaacactcataaaaattaaacagaagctctgaagaccttgtatttttatcaaataatacccccttgaactcattcacaaacgcatcttttttttcttgaatatctatggggtgttcctttgactctgacaaagatgaaatctcatctattttgttttcatatgaattacgtgattccatacagacatttggcggcgtttctaaaataacactacgcgtactacttggcttaagtaaaccaacatgaaaatcactttttcttatattatcgaaaaggttctattcatttcttttagcgcattcaaaaaactgatcggcattatttttattcgataattttttagtttcagaaaacacattttcattgttttccagctttagtttaatgagaagattttcccagacctgcttgcttaaacatattacgtcaggctcaccagaactaactaactcgtgattattattaaagtgtacgttgaatacctttaagttattttcaccaacttcatatttaatacgttttaattgttctccagctcccataatgacaaaggcgttgccttcttgatatatacattcagacatcattttttgtaaagtttcaagagcaccgcgatacgtctctgatgcagcttccttacaaattaattttaaaatactatgagctagtagctccatgtgtttagaagatttattttcattataacttccactacccaaaactgcgctagcgttaaatccgttgcttttactaactaacattgtctattcctcaattaatgtctacatggctatttttaatgttattactgtttgtcactataaaaaaacgctcatttgagacaattactgacattaactgcttcacttgctacgcatggaacttttaattaaattagcacaggaatgttaaatttaataaacaaaaggttatttcgctgtatgataaaaaaaaccgttataatttattagtgaaaatcgtttttcaagtgttagaaatttatatctcaatagcgttggttaatgagcatagccacgctcctgtaacgctcacaaaactcatctgcctgcggcgggtgttctggtcagtagtagatgtttaaggcgtggcagagacatttcatccttactctacggcattgttctacatacattggttgtggtactcacttatcatcagtgagcgaacagagaatagttcagtgatttgagtaattaacctgattaaatgaaggggtataataaatgataatactctggctttatcgttaattacttaattccacatgtaagcaatttgcccgcttggcatagcaggcattttttccaggtacttttgaatgagtactgatggataaatacattgcagtggcgtgccacgtaccaaaacaccagccctcattcgaaaccacccaccgcacttcttccttgaaatggcgttagtcatgaaatatagaccgccatcgagtaccccttgtacccttaactcttcctgatacgtaaataatgatttggtggcccttgctggacttgaaccagcgaccaagcgattatgagtcgcctgctctaaccactgagctaaagggccttgagtgtgcaataacaatacttataaaccacgcaataaacatgatgatcatatgatgtaaataacagatttttatgcgttcccattcaccttgggtcgtgattacacgcgacataaaacccgacaccgcctccattcgcaaagtcgatactcgcagtcaacaagcaaatgttaataattagcactatctatagttatcatcgattcaatgatactttgtaatgattttgtatctaataatataactttattacattagctgaagagttttcgcatcattatgatatctgttacttttcactccataaaaataaacttcgtatagcaatatattctttcatagatcttattctgctaatcattagtttcgtatgagcgatttttgacagttgcctctccagaccacatcgataattaataaaacagatttaagcattatccttttccatataaatattggataaaagtaggacatctgtttgcaattactttcacaacaattaaacatttttatgtttccgtatacatcatattactctaccattagaggaactttattatgttttctataaaaccaggacccagaaatttacctatcgacaaccccacattgttatcatggaacattactgacggggatctaaattccaaattaaatacattagaatatctaaactgtataacaaatattattaattcttgtggagtttaccctcaaggattaaaagacagagaaattatatcaacttttcacgcagaaaaagttattaatgatctgttaaaaaacgattataaaatttccctttctccagatacaacttaccgagagttgaataaagcagcacagcgtagcattacagcgccagacaggataggagaaagaaaaacataggtttatcaacgagatacaatgattgaaagaggtgataacagcggtgtttatcagtatggtcgtgctgaacatttcacccacattatatctgacaaaccttccccaaaagataaatatgttgcatatgctattaacattcctgactatgagctggcagccgatgtatataatattaacgtgacgtcaccttccggacagcaagaaacatttaaaatattaatcaatctagaacatctacggcaaacacttgaacgtaaatctcttactgctgttcagaaatcacaatgtgaaatcatcacccccaaaaaacctggcgaagcgattcttcatgcttttaatgccacctaccagcagatcagagaaaatatgtctgaatttgcacgttgccattatgggtatatacaaatccctccagtgacaactttccgcgccgacggaccagaaactcccgaagaagaaaagggttactggtttcatgcttatcaacccgaagatctttgtaccatccataatccaatgggagatttgcaggattttattgcattggttaaagatgctaaaaaatttggtatcgatatcattcctgattatacctttaactttatgggaattgggggtagtggtaaaaatgacctggattatccctctgctgatatacgagcgaagatcagtaaagatatagaaggtggtatccctggctattagcaaggtcaggttttgattccattcattaaagatccagtaacaaaagaacgtaaacaaatccatccagaagatatacatctcactgcaaaagacttcgaagcaagtaaagataacatctctaaggatgaatgggaaaacctccatgcattaaaagaaaagcgtttaaatggaatgcctaaaacaacacccaaaagtgaccaggttattatgttgcaaaatcaatacgttcgtgaaatgcgaaaatatggcgtacgaggtttacgttatgatgcggcaaaacactcaaaacatgaacaaatagaaagatcaataaccccaccgcttaaaaattataatgagcggttacacaatactaacttatttaacccaaaatatcataaaaaagccgttatgaattacatggaatatctggtaacttgtcagttggatgaacaacaaatgtcatcactgctttatgaaagagatgatttaagcgccattgatttttcattgctcatgaaaacgataaaagccttttcatttggtggagatcttcaaacccttgcatcaaaaccgggttccacaatctcaagtatcccatcagaaagacggatattgattaacattaaccacgattttcctaacaatggtaatcttttcaatgactttctatttaaccatcaacaagatgaacaattagcaatggcatatatagccgctctgccgttcagcaggcctttagtttactgggatggccaagtattaaaatcaacgactgaaattaaaaattatgatgggtccacgcgtgtcggcggtgaggcgtagcttaataaaggttgctctacctatcagcagctctacaatgaattccacgcattatatatagataaagcaggaatatggagcgcatttgagggtgtatctgcaactaaaaacgttctggcctttagtcgtggggattctgtgaacattaatcactctcctcatgatggactagttataataaataaaggaaacgaagaagttgaaggtacctggcctaacaaattgcaacctggaatatacaaaaacatggggagtaatagcgttaacattattattaataatacccgaaaaattatcccccctggtaaagtatttacgcttagaggcggaactctaaatatcaatattcctgggcgtagcgctcttcttttagggaaaacaggagaaccgccgaactatctctatttataatttaatgttatatctgccccgataaaacggggcagataatatgtttagtttactaacggtcattttgcagtgaagccatttactgttttttatcgaccagataatctgttctctaatgttaactccccctaacctgttgctttagttattcatttcctgtctcactttgccttaataccctacgttaaatgttactaatttgttgcttttgatcacaataagaaaacaatatgtcgcttttgtgcgcatttttcagaaatgtagatatttttagattatggctacgaaatgagcatcgccatgtcaccctacatctcataagaggatcgcttctgatgaatgcactgaccgccgtacaaaataacgctgtcgattcaggccaggactatagcggattcaccctcaccccgtcggcgcaatccccgcgtctgctggaactcaccttcaccgaacagacgaccaaacagtttcttgagcaggttgccgagtggcccgtgcaggcgctggagtacaaatcgtttctgcgttttcgggtagccaaaattcttgacgatctatgtgcgaaccagctgcaaccattgctgttgaagacgttgctaaaccgcgctgaaggtgcgttgttgatcaatgcggtgggtgtcgatgatgtgaagcaagcggatgagatggtgaagctggcgacggcggtggcgcatctgattggccgttccaatttcgatgcgatgagcggtcagtattacgcgcgttttgtagtgaaaaatgtcgataactcagacagctatctgcgccagccgcaccgcgtgatggagctacacaacgacggcacgtatgtcgaagagataaccgattacgtgctgatgatgaaaatcgacgagcaaaacatgcagggcggaaattcgctgctgctgcatctcgatgactgggaacatctcgacaactatttccgccacccgctggcgcgtcgcccgatgcgctttgccgcgccgccgagtaaaaacgtcagcaaagatgtttttcatccggtgttcgacgtcgatcaacagggtcgcccggtgatgcgctatatcgaccagttcgtccagccgaaagacttcgaagaaggcgtgtggttgagcgagctttccgacgccattgaaaccagcaaaggcattctttctgtgcccgttcccgttggcaaattcctgttgattaacaacctgttctggctgcacggtcgcgaccgctttactccgcacccggatctgcgccgtgaactgatgcgccagcgtggctatttcgcttacgcctctaaccactaccagacgcatcagtaagcgcaaaggaattgagcggatgtatgattttgtgattattggcggcggcatcatcggcatgtcgaccgccatgcaactgattgatgtctatccggacgcccgcattgcgttgctggaaaaagagtccgccccggcctgtcaccagacgggccacaacagcggcgtgatccatgccggggtctattacacgcccggcagcctgaaggcgcagttttgcctggcgggaaaccgcgccaccaaagccttttgcgatcaaaacggcattcgctacgacaactgcggcaagatgctggttgccacgtccgatctcgaaatggaacggatgcgcgccttatgggaacgcacagcggcgaacggtatcgagcgcgaatggcttaacgccgacgaactgcgcgagcgcgaaccgaatatcaccgggctcggcggcatttttgtgccgtccagcggcattgtcagctaccgcgacgtgacggcggcgatggcaaaaatcttccagtccagaggcggtgaaattatctataacgccgaagtcagcgggcttaatgagcataaaaacggcgtggtgatacgtacccgtcagggcggcgaatatgaagcatcaacgctgattagctgttccgggctgatggctgaccggctggtgaaaatgctcggactcgaaccgggctttatcatctgcccgttccgtggcgagtatttccgccttgcgccggagcataaccagattgttaaccacctgatttaccccattcccgacccggcaatgccgtttttgggcgttcatctcacccgcatgatcgacggcagcgtgaccgtcgggccaaacgcggtgctggctttcaaacgcgaaggctatcgcaagcgcgacttctcatttagcgacacgctggagattttgggctcgtcggggattcgccgggtgctgcaaaaccatctacgctcaggactgggcgagatgaaaaactcgctgtgcaaaagcggctatctgcggctggtgcaaaagtattgtccccggctttcgttaagcgatctccagccctggcccgccggtgtgcgggcgcaggcggtatcgccggacggcaagctgattgacgattttctgtttgtcaccaccccgcgcacgatccacacctgcaatgcgccctccccggcagcgacatcagcaattcctattggtgcgcatattgtcagcaaggtacaaacgctgttggcaagccagagtaaccccggacgcacgctgcgagcggcacgtagtgtggatgccttacacgccgcatttaatcaataacctttgaaaacaggatgtagcgatgaaacttaacgacagtaacttattccgccagcaggcgttgattaacggggaatggctggacgccaacaatggtgaagccatcgacgtcaccaatccggcgaacggcgacaagctgggtagcgtgccgaaaatgggcgcggatgaaacccgcgccgctatcgacgccgccaaccgcgccctgcccgcctggcgcgcgctcaccgccaaagaacgcgccaccattctgcgcaactggttcaatttgatgatggagcatcaggacgatttagcgcgcctgatgaccctcgaacagggtaaaccactggccgaagcgaaaggcgaaatcagctacgccgcctcctttattgagtggtttgccgaagaaggcaaacgcatttatggcgacaccattcctggtcatcaggccgataaacgcctgattgttatcaagcagccgattggcgtcaccgcggctatcacgccgtggaacttcccggcggcgatgattacccgcaaagccggtccggcgctggcagcaggctgcaccatggtgctgaagcccgccagtcagacgccgttctctgcgctggcgctggcggagctggcgatccgcgcgggcgttccggctggggtatttaacgtggtcaccggttcggcgggcgcggtcggtaacgaactgaccagtaacccgctggtgcgcaaactgtcgtttaccggttcgaccgaaattggccgccagttaatggaacagtgcgcgaaagacatcaagaaagtgtcgctggagctgggcggtaacgcgccgtttatcgtctttgacgatgccgacctcgacaaagccgtggaaggcgcgctggcctcgaaattccgcaacgccgggcaaacctgcgtctgcgccaaccgcctgtatgtgcaggacggcgtgtatgaccgttttgccgaaaaattgcagcaggcagtgagcaaactgcacatcggcgacgggctggataacggcgtcaccatcgggccgctgatcgatgaaaaagcggtagcaaaagtggaagagcatattgccgatgcgctggagaaaggcgcgcgcgtggtttgcggcggtaaagcgcacgaacgcggcggcaacttcttccagccgaccattctggtggacgttccggccaacgccaaagtgtcgaaagaagagacgttcggccccctcgccccgctgttccgctttaaagatgaagctgatgtgattgcgcaagccaatgacaccgagtttggccttgccgcctatttctacgcccgtgatttaagccgcgtcttccgcgtgggcgaagcgctggagtacggcatcgtcggcatcaataccggcattatttccaatgaagtggccccgttcggcggcatcaaagcctcgggtctgggtcgtgaaggttcgaagtatggcatcgaagattacttagaaatcaaatatatgtgcatcggtctttaactggagaatgcgaatgaacagcaataaagagttaatgcagcgccgcagtcaggcgattccccgtggcgttgggcaaattcacccgattttcgctgaccgcgcggaaaactgccgggtgtgggacgttgaaggccgtgagtatcttgatttcgcgggcgggattgcggtgctcaataccgggcacctgcatccgaaggtggtggccgcggtggaagcgcagttgaaaaaactgtcgcacacctgcttccaggtgctggcttacgagccgtatctggagctgtgcgagattatgaatcagaaggtgccgggcgatttcgccaagaaaacgctgctggttacgaccggttccgaagcggtggaaaacgcggtaaaaatcgcccgcgccgccaccaaacgtagcggcaccatcgcttttagcggcgcgtatcacgggcgcacgcattacacgctggcgctgaccggcaaggtgaatccgtactctgcgggcatggggctgatgccgggtcatgtttatcgcgcgctttatccttgcccgctgcacggcataagcgaggatgacgctatcgccagcatccaccggatcttcaaaaatgatgccgcgccggaagatatcgccgccatcgtgattgagccggttcagggcgaaggcggtttctacgcctcgtcgccagcctttatgcagcgtttacgcgctctgtgtgacgagcacgggatcatgctgattgccgatgaagtgcagagcggcgcggggcgtaccggcacgctgtttgcgatggagcagatgggcgttgcgccggatcttaccacctttgcgaaatcgatcgcgggcggcttcccgctggcgggcgtcaccgggcgcgcggaagtaatggatgccgtcgctccaggcggtctgggcggcacctatgcgggtaacccgattgcctgcgtggctgcgctggaagtgttgaaggtgtttgagcaggaaaatctgctgcaaaaagccaacgatctggggcagaagttgaaagacggattgctggcgatagccgaaaaacacccggagatcggcgacgtacgcgggctgggggcgatgatcgccattgagctgtttgaagacggcgatcacaacaagccggacgccaaactcaccgccgagatcgtggctcgcgcccgcgataaaggcctgattcttctctcctgcggcccgtattacaacgtgctgcgcatccttgtaccgctcaccattgaagacgctcagatccgtcagggtctggagatcatcagccagtgttttgatgaggcgaagcagtagcgccgctcctatgccggaggcgacgctgcgcgtcttgtccggcctacggggatccaggtcggataaggcgtttacgccgcatccgacaatctgtacgtgaacaggaagaaatctatgttggccgggtaaggcggagccgctctccggcaaaaagaatcaataacaattatacgcgtgacccggcgcgggaaatgtcggggcgctctcccaagtgacacactttcgagaggattcaggatggggcaatcatcgcaaccacatgagttaggcggcgggctgaagtcacgccacgtcaccatgttgtctattgccggtgttatcggcgcaagtctgtttgtcggttccagcgtcgccatcgccgaagcgggcccggcggtattactggcctatctgttcgccgggctactggtggttatgattatgcggatgttggcggaaatggcggttgccacgcccgataccggttcgttttccacctatgccgataaagccattggtcgctgggcgggctataccatcggctggttgtactggtggttttgggtactggttatcccgctggaagccaacatcgccgccatgatcctgcactcatgggttccaggcattcccatctggttattttccctcgtcattaccctcgccttaactggcagtaacttattaagcgttaaaaactacggcgaatttgagttctggctggcgctgtgcaaagtcatcgctatcctggcctttattttccttggtgcagtcgcaattagcggtttttacccgtatgccgaagtgagcgggatctcaagattgtgggatagcggcggctttatgcccaacggtttcggtgcggtattaagcgcgatgttgatcaccatgttctcgtttatgggcgcagaaattgtcaccattgccgccgcggaatccgacacgccggaaaaacatattgtccgcgccaccaactcggttatctggcgtatttctatcttctatttatgttctatttttgtcgtcgtggcattaattccgtggaatatgcccggactaaaagccgtcggttcttatcgctcggtactggaattgctcaatattccccatgcgaaattaatcatggactgcgtgatattactttccgtaaccagttgcctgaactcggcgctgtataccgcgtcaaggatgctctactccttaagtcgtcgcggtgatgctcccgcggtaatgggtaaaatcaaccgcagtaaaaccccgtacgtggcggtgttactctccaccggcgcggcattcttaacggtggtggtgaactattacgcgcctgcgaaggtatttaaatttctgatcgacagctccggcgctatcgccctgctggtttatttagtcatcgccgtttcacagttgcggatgcgcaaaattctgcgagcagaaggaagcgaaattcgcttgcgaatgtggctttatccgtggctcacctggctagtcatcggctttattacctttgtgttggtagtgatgctattccgtccggcgcaacagttagaagtgatctccaccggcttattagcgatagggattatctgtaccgtgccaattatggctcgctggaaaaagctggtattgtggcaaaaaacacccgttcataatacgcgctgatcatgatcaggagtcacaccatgaccattacgtctctggatggctatcgctggctgaagaacgatattattcgcggtaattttcaaccggatgaaaaattacgaatgagtttgctgacatcgcgttatgcacttggcgttgggccgttacgggaagctctttcgcaactggtggcggaacggctggtcacggtggtgaatcaaaaagggtatcgggtggcgtctatgtcagagcaggagctgctcgatattttcgacgcccgcgccaatatggaagcgatgttagtgagtctggcgattgcccgcggtggcgatgagtgggaggcagacgttctcgcaaaagcgcatctgctgagtaagcttgaggcctgtgacgccagcgagaaaatgcttgatgagtgggatctgcgtcatcaggcgtttcatacggcaattgtggcgggctgtggttctcactatttgctgcaaatgcgtgaacggttgtttgatctggcggcgcgttatcgatttatctggctgcggcgaacggtgctttcggtggaaatgctggaggataaacacgatcagcaccagaccctgactgcggcggtactggcgcgagataccgcgcgcgccagtgagttaatgcgccagcatttactgacgccaattcccattatccagcaggcgatggctggcaattaactactcttccggaatacgcaacacttgccccggataaattttatccgggctttttagcatcggtttattcgcttcgaagattttattgtacagattagcgttaccgtagacctgtttggaaatggcactcagagtgtcgccagacttaacggtataaaactggctggcagtggctggtgtcgccgttttcacctgatcatcgacactggcaataccggaaatattccccaccgcaacaaggattttctccttcgcctcctgactcaggccgtcaccagtgaccgtcgctttgccgtcggcaatttgaatattcactttatcggcatccggtataccggttttgttcagatgctcctgcaccttcttcgcctgatcgtctttatcgtgctgacctgtaaccgcgtcccagagtttttctccggcatctttcacaaaattgaacagacccatagctacctcattcgttaacggaaacactcagaaagtgtagcagaggaacgcggcgcgttaacgccgcggggatgagcacaggtttaatcgcgggtttgcacccagaacgcgtgaatcaaaccggggatatacccaagcagtgtcaacagaatattaataatgaacgcccaaccgaaccctttaccgagcagcacgccgagcggcggcagaatgatggtgatgacgattctccagaaacccatatgtactccctataagaaaattactcattgtttaaaaagagattttatctcttaagcgtagtaattttagcggagcctgccagtttcagcttacgcttttactctcatttacgctgctgaggctggtatatgttgcatttttagtttagagtttacttaatttagaaaatacttaaataaatatgactgaactcgcgcaattacaggccagtgccgaacaggcagcggccttattgaaagcaatgagccaccctaaacgattgctgattctgtgcatgcttagcggttcccccggcaccagcgcgggagagctgacgcgcattaccggactgagtgcctctgcgacatcacagcatctcgctcgtatgcgggacgaagggcttatcgacagccaacgggatgcccaacgcattctatattccattaaaaatgaggcggtaaatgccattatcgccaccctgaaaaatgtctattgtccgtaaggagtcactatggctttgacaaccatttcgccgcatgatgcacaagaattaatcgcacgcggcgcaaagttaatcgatattcgtgatgctgatgaatatcttcgtgaacatattcctgaagcagatctggctccattatccgtgctggaacagtcaggtcttccggctaaattacgtcacgagcaaattatattccactgccaggcaggtaaacgcaccagtaataatgccgataaattagcagcgattgccgcccccgcagaaatctttttactcgaagatgggattgatggctggaaaaaagcaggattgccagtagcggtaaataaatctcaacccttgccgttaatgcgccaggtgcagatcgctgcgggtggtttaatattaatcggcgttgtactgggttataccgtaaatagcggtttcttcttattaagtggctttgttggtgccgggttactgtttgcaggaatcagcggtttttgtggaatggcaaggttgttagataagatgccgtggaaccaacgagcttgagaagcgacgccggacgcgccctagcagcgacatccggcctcagtaattagatcaggaaatcgtcgagagatttaccttctgccagcgcctgagcaattggcttcggtgtacggccctgaccggtccaggttttagtttcaccgttaacatcggtgaatttatatttcgccggacgcggctggcgttttttaccagcgcgtggtgcagcagcagagctattacccaataactcttccgggttaattccgtcagctttcatcagctccagccaggtgctaattttttcctggcgctctgccagttcacgctgctgctgttcttcttcttcacgtctttctttagtgacaaccctgaatttttcgagcatttcttcaagaacgtcaatggagaattcgcgagccatcgcacggagggtgcgaatgttatttaaactttgtaacattacggacataataaagaaaaccttttaacgccaaaacaaaaaaagtatttcgtcgcgtagtgtaagcgatcacttattatatttccacaaaatttaatctatttacagtcctgcgcgagattatttcagctgttattttctgaaactctcagaataatttcaagattatatattagccattttgatgagtaatttagattattggtgaacagagcggcgctctctgctcgctaattccgcaagcctgacaaaatcaaagtgaataaaaatgcaatataacagaataaaagaaaacatccatcactggtgctttctgctgttaatgtacattgtctggcataaaaaatgctgaaaatgacccagctactacatacaccgaattctctacgcttatagcgttacctcacccccaaactttcattagtgatattaaaggtaaggccatatctaattgatttaattaaaaataaatcatatcggcatgtaaaaatccacaatgtacaaaaaacgagccgttacggaatattttatctacaaaaactgactaaataaaaatttttcactaattgattagtcatagccagcgatatacgctatgcgaaaatgcagatggcaatgagatccactgctttcatctccattaacatcccattacgcttttattaaggagcattagcatgttctcaccgcagtcacgcttgcgtcatgcagttgcagatacgttcgcgatggttgtttactgttctgtcgtgaacatgtgtattgaagttttcctctccggaatgagcttcgaacagtctttttattccagattggtagcgattccggtgaacatcttaattgcatggccatacggtatgtaccgtgatctgtttatgcgcgcggcacgcaaagttagcccgtcgggctggataaaaaatctggcggatatcctggcttatgtgacgttccagtcaccggtgtatgtggcgatcttgttagtggtgggcgcagactggcatcagattatggcggcggtcagttcaaacatcgttgtttcgatgttgatgggggcggtttatggctacttcctcgattattgccgccgactgtttaaagtcagccgttaccagcaggtaaaagcctgactcttcttttcgcgactggcatcgccagtcgcgtctttaactggcttcgccaaataaaccattcaaataacgttcaagcgcaacacgcgaactaaagccatgcgggataccgtaatgctcgtgtcgctcgcctgctaaatagagcggaaattgctggtaatgatcgcaagttttaatatcggaagcgggttcagccagtgtcgaactgcgttcttttaatgttggatgaattaccagagcggtacgtcccattcgcgcttcgcgattaacatagacataattttccccacggcggtaaccatacgctttctgggttaccacatcgacagtaaaaccgactttttcaagtacgcgcgccacctcgtctggtcgtaaatacatatttgatcctcgttattatcaaccgcgggcctaccttacctgattgcgcattcacaacgctttcagaaaagtccataaagccgcgatgaacctcagttaagaaaattatggtctacactgaaaattacatcgaattctaatgggggatcatatgtttaaccgaccgaaccgcaacgacgttgatgatggcgtgcaggatatccagaatgatgtcaatcaattagctgacagcctcgaatctgtattgaagtcctggggcagcgacgccaaaggggaagctgaagccgcacgcagtaaagctcaggcattgctgaaagaaaccagggcgcgaatgcatggtcgtactcgcgtccagcaagccgcgcgcgatgccgttggctgcgcggattcttttgttcgtgaaagaccctggtgtagcgtgggtacagcagctgcggtaggtatttttatcggcgcactgttaagcatgcgcaaatcgtagtgcaaaaatgataataaatacgcgtctttgaccccgaagcctgtcttcggggtttctttttgcctggtgaatcacaaaaatccccctaccccgtcacgctcatatccagggtaatttcgaccactatttgctatatattgtgtggttgaatcttttttcaactacatctagtatctctgtatcaacagagagacaacccgacgcgtatcatcgcgccgtatcttcattttaaacggaaatacgaatcatgcgcattactatttacactcgtaacgattgcgttcagtgccacgccaccaaacgggcgatggaaaaccggggctttgattttgaaatgattaatgtcgatcgcgttcctgaagcggcagaagcgttgcgtgctcagggctttcgtcagttgccggtagtgattgctggcgatcttagctggtctggtttccgtccggacatgattaaccgtctgcatccagcgccacacgcggccagtgcatgagccagctcgtctacttctccagcagctccgaaaacacgcagcgttttatcgaacgtttaggtctgcccgcggtgcgcatcccgctcaatgagcgggaacggattcaggtagacgagccttacatcctgatcgtgccctcttacggcggcggcggtacggctggcgcggtgccacgacaggtaattcgctttttaaacgacgagcacaaccgggcgttgcttcgcggcgttattgcttctggtaatcgcaactttggtgaggcgtatggccgcgccggagatgtgattgcccggaaatgcggcgtgccgtggctgtaccgttttgaactcatgggtacgcaaagcgatatcgaaaacgttcgtaaaggagtaaccgaattttggcaacgacaaccgcagaatgcctgacgcaggaaacgatggattaccacgcgctgaatgcgatgcttaacctctacgatagcgcaggtcgcattcagttcgataaagaccgccaggccgttgacgcctttattgcgacgcatgtgcgtccgaacagtgtgaccttcagtagccagcagcagcgcctgaactggctggtcaacgaaggttactatgatgaaagcgttcttaatcgctactctcgcgactttgtcattacgctgtttacccacgcacacaccagcggttttcgtttccagacattcctcggggcatggaagttttacaccagctatacgttgaagacattcgacggtaaacgttatctggaagattttgccgatcgagtaacgatggtggcgctgacgctggcacaaggcgatgagacgctggcgttgcaactgaccgatgaaatgctgtcaggacgctttcagccagccacgccaacattcctcaactgcggtaagcagcagcgcggcgaactggtttcctgttttttgctgcgtattgaagacaatatggagtcgattggtcgggcggtaaattccgcactgcagctgtcgaaacgcggcggcggcgtagcatttttgctgtcgaatctgcgagaagcgggcgcgccaattaaacgtattgaaaatcaatcttctggcgtaattccggtgatgaaaatgctggaagacgcattttcctatgccaaccaactcggcgctcgtcagggggctggtgcagtctatttacatgctcatcatcccgatattctgcgttttctcgacacgaaacgggaaaatgccgacgaaaaaatccgcattaaaacactgtcgcttggcgtggtgatcccggatatcactttccatctggcaaaagagaatgcgcagatggcgctgttttcgccttatgacgtagagcgagtttatggcaagccgtttgccgatgtggccatcagccaacactatgacgaactggttgccgatgaacgcattcgcaaaaaatacctcaacgcccgtgatttcttccagcgactggcagaaatccagtttgagtccggctatccctacatcatgtatgaagacacggtaaaccgtgctaaccctatcgccgggcgcataaatatgagtaatctctgctcagaaattttgcaggttaacagcgcctcagagtatgacgagaatctcgactatacccgcacaggccatgatatttcctgcaatttaggttcgttgaatattgcgcacaccatggattcccccgattttgcccgcacggtagagactgccgtgcgcggtttaacggcagtatcagatatgagtcatatccgcagcgtgccgtccatcgaagccggaaatgccgcctcgcacgccatcggactggggcagatgaatttacacggctatctggcgcgagaaggcatcgcttatggttcgccggaagcactggatttcaccaatctctatttctatgccatcacctggcatgcactgcgtacctcgatgttgctggcacgcgaacgcggtgaaaccttcgccgggttcaaacagtcacgctatgccagtggtgaatattttagccaatatctgcaagggaactggcagccgaaaacggcgaaagttggcgaactgtttacccgtagcggtattacgttacctacccgtgagatgtgggcgcagctgcgcgacgacgtgatgcgctacggcatatacaaccagaatcttcaggcggtgccgccaaccggttctatctcttatatcaaccatgctacgtcgagtattcatccgattgtggcgaaagtagagatacgcaaagagggcaaaacaggacgcgtttactaccctgccccgtttatgactaacgagaatctggcgctgtatcaggacgcttacgaaattggcgcagaaaagatcatcgacacctacgcggaagcgactcgccatgtcgatcaggggctgtcgctgacgctttttttccccgataccgccaccactcgcgatatcaacaaagcgcagatttacgcctggcgcaagggtatcaaaacgctctattacatccgcctgcgtcagatggcgctggaaggcactgaaattgaaggctgcgtctcctgtgcactttaaggaatatctatgaaactctcacgtatcagcgccatcaactggaacaagatatctgacgataaagatctggaggtgtggaatcgcctgaccagcaatttctggctaccagaaaaggtgccgctgtcgaacgatattcctgcctggcagacattaactgtcgtagaacaacaactgacgatgcgcgtttttactggcctgacgctgctcgacacgctgcaaaatgttatcggcgcgccttctctgatgcccgatgcactcacgcctcatgaagaagcggtattatcgaatatcagctttatggaagcggttcatgcccgctcttacagttcgattttctcgacgctatgccagaccaaagatgtcgatgccgcctacgcctggagtgaagaaaacgcaccgttgcagcgaaaagctcagattattcagcaacattatcgcggtgatgatccgctgaaaaagaaaatcgccagtgtgtttcttgaatcttttttgttctattccggtttctggctgccgatgtatttttccagccgcggaaagctgaccaataccgcggacctgatccgtctgattatccgcgatgaagcagtccacggttactacataggctataaatatcagaaaaacatggaaaagatatctctgggacaacgtgaagagttgaagagtttcgccttcgatttgttgctggaactctacgacaacgagttgcaatacaccgatgagctgtacgccgaaaccccgtgggctgacgatgtgaaagcgtttctctgttacaacgccaataaggctttgatgaatctgggctacgaaccgttatttcccgcagaaatggcggaagtgaatccggcaatcctcgccgcgctttcgccgaatgccgatgaaaatcacgatttcttttccggttcaggctcctcttatgtgatggggaaagcggttgaaacagaagatgaagactggaatttctgagggtgttattttcaaaaatatcactacccgcagcagggaaataattcccgccaaatagctttttatcacgcaaataatttgtggtgatctacactgatactctgttgcattattcgcctgaaaccacaatattcaggcgttttttcgctatctttgacaaaaaatatcaactttctcgatttgctctcagcccttatatcacgggaaattccggcgatttgctcgcatcaatattcatgccacatttgccatcaggggttgcctcagattctcagtatgttagggtagaaaaaagtgactatttccattgggtaatatatcgacatagacaaataaaggaatctttctattgcatggcaattaaattagaaattaaaaatctttataaaatatttggcgagcatccacagcgagcgttcaaatatatcgaacaaggactttcaaaagaacaaattctggaaaaaactgggctatcgcttggcgtaaaagacgccagtctggccattgaagaaggcgagatatttgtcatcatgggattatccggctcgggtaaatccacaatggtacgccttctcaatcgcctgattgaacccacccgcgggcaagtgctgattgatggtgtggatattgccaaaatatccgacgccgaactccgtgaggtgcgcagaaaaaagattgcgatggtcttccagtcctttgccttaatgccgcatatgaccgtgctggacaatactgcgttcggtatggaattggccggaattaatgccgaagaacgccgggaaaaagcccttgatgcactgcgtcaggtcgggctggaaaattatgcccacagctacccggatgaactctctggcgggatgcgtcaacgtgtgggattagcccgcgcgttagcgattaatccggatatattattaatggacgaagccttctcggcgctcgatccattaattcgcaccgagatgcaggatgagctggtaaaattacaggcgaaacatcagcgcaccattgtctttatttcccacgatcttgatgaagccatgcgtattggcgaccgaattgccattatgcaaaatggtgaagtggtacaggtcggcacaccggatgaaattctcaataatccggcgaatgattatgtccgtaccttcttccgtggcgttgatattagtcaggtattcagtgcgaaagatattgcccgccggacaccgaatggcttaattcgtaaaacccctggcttcggcccacgttcggcactgaaattattgcaggatgaagatcgcgaatatggctacgttatcgaacgcggtaataagtttgtcggcgcagtctccatcgattcgcttaaaaccgcgttaacgcagcagcaaggtcttgatgcggcgctgattgatgcgccgttagcagtcgatgcacaaacgcctcttagcgagttgctctctcatgtcggacaggcaccctgtgcggtgcccgtggtcgacgaggaccaacagtatgtcggcatcatttcgaaaggaatgctgctgcgcgctttagatcgtgagggggtaaataatggctgatcaaaataatccgtgggataccacgccagcggcggacagtgccgcgcaatccgcagacgcctggggtacaccgacgactgcaccgactgacggcggtggtgctgactggctgaccagtacgcctgcgccaaacgtcgagcattttaatattctcgatccgttccataaaacgctgatcccgctcgacagttgggtcactgaagggatcgactgggtcgttacccatttccgtcccgtcttccagggcgtgcgcgttccggttgattatatcctcaacggtttccagcaattgctgctgggtatgcccgcaccggtggcgattatcgttttcgctctcatcgcctggcagatttccggggtcggaatgggtgtggcgacgctggtttcgctgattgccatcggcgcaatcggtgcctggtcgcaggcaatggtgactctggcgctggtgttaaccgccctgctgttctgtatcgtcatcggtttgccgttggggatatggctggcgagaagtccgcgagcggcgaaaattattcgtccactgcttgatgccatgcagaccacgccagcgtttgtttatctggtgccaatcgtcatgctatttggtatcggtaacgtgccgggcgtggtggtgacgatcatctttgctctgccgccgattatccgtctgaccattctggggattaaccaggttccggcggatctgattgaagcctcgcgctcattcggtgccagcccgcgccagatgctgttcaaagttcagttaccgctggcgatgccgaccattatggcgggcgttaaccagacgctgatgctggccctttctatggtggtcatcgcctcgatgattgccgtcggcgggttgggtcagatggtacttcgcggtatcggtcgtctggatatggggcttgccaccgttggcggcgtcgggattgtgatcctcgccattatcctcgatcgtctgacgcaggccgttgggcgcgactcacgcagtcgcggcaaccgtcgctggtacaccactggccctgttggtctgctgacccgcccattcattaagtaactctgcacttgcccggtgacgccgggcattatcaccctgccaaaaaaaggaataacaatgcgacatagcgtactttttgcgacagcgtttgccacgcttatctctacacaaacttttgctgccgatctgccgggcaaaggcattactgttaatccagttcagagcaccatcactgaagaaaccttccagacgctgctggtcagtcgtgcgctggagaaattaggttataccgtcaacaaacccagcgaagtagattacaacgttggctacacctcgcttgcttccggcgatgcaaccttcaccgccgtgaactggacgccactgcatgacaacatgtacgaagctgccggtggcgataagaaattttatcgtgaaggggtatttgttaacggcgcggcacagggttacctgatcgataagaaaaccgccgaccagtacaaaatcaccaacatcgcacaactgaaagatccgaagatcgccaaactgttcgataccaacggcgacggaaaagcggatttaaccggttgtaaccctggctggggctgcgaaggtgcgatcaaccaccagcttgccgcgtatgaactgaccaacaccgtgacgcataatcaggggaactacgcagcgatgatggccgacaccatcagtcgctacaaagagggcaaaccggtgttttattacacctggacgccgtactgggtgagtaacgaactgaagccgggcaaagatgtcgtctggttgcaggtgccgttctccgcactgccgggcgataaaaacgccgataccaaactgccgaatggtgcgaattatggcttcccggtcagcaccatgcatatcgttgccaacaaagcctgggccgagaaaaacccggcagcagcgaaactgtttgccattatgcagttgccagtggcagatattaacgcccagaacgccattatgcatgacggcaaagcctcagaaggcgatattcagggacacgttgatggttggatcaaagcccaccagcagcagttcgatggctgggtgaatgaggcgctggcagcgcagaagtaatttttattcgggcggataaggcgtttttgccgcatccgccgttctgtgcacaatgcctgatgcgacgctggcgcgtcttatcatgcctacaaaccacatcgcacatttcaacaatctatctttcatcccatattcatcaacatccgctattattgatttccagcttaatcatcacctgatgaacaaaaataatgactaaacctaatcatgagcttagcccggcgctgatcgtgctgatgtctatcgccaccggtctggcggtagccagtaactattacgcccagccattgctcgacaccatcgcgcgtaacttttccctttccgccagttcggcaggctttattgttaccgccgcgcagttgggctatgccgcaggtctactgtttcttgttcccctcggtgatatgtttgaacgccgccgcctgattgtctcgatgaccttactggcggcatgttgattaccgccagcagtcagtcgctggcgatgatgatcctcggtacggcattaaccggtttattctcagtcgtggcacaaattctggttccgctggcagcgacgctggcttcaccggataaacgcggcaaagtggttggcactattatgagcggtctgctgttggggatcttgctggcacggacagttgccggattgctggcgaatctcggcggctggcgcaccgtcttttgggttgcttcggtgttaatggcactgatggcgctggcattatggcgtggtctgccacaaatgaaatcagaaacccacctcaactacccacagttgttgggttccgttttcagtatgtttatcagcgataaaattctgcgtacccgcgcgttgctgggctgcctgacctttgccaatttcagcattctctggacctcaatggcctttttgcttgccgctccaccttttaactacagcgatggtgtcattggtctgtttggacttgcgggagctgccggagcgttgggcgctcgtccggcgggcggttttgccgataagggcaaatcgcaccacaccacaactttcggtctgctgctgctattactttcatggctggcgatctggtttggtcacacttccgtactggcgttgattatcggaatcctggtgctggatctcaccgtgcagggcgtgcatatcactaaccagacggtaatttatcggatacatcctgatgcgcgcaatcgcctgaccgcaggttacatgactagctactttattggcggtgccgccggttcgctaatttcagcctcagcctggcaacatggcggttgggctggcgtttgtctggctggcgcgacgattgccctggttaacttactggtctggtggcgaggttttcatcgtcaggaagccgcaaattaagcaatcagcaaccgttttcgtggctttacacttataagggtgttaagaagcccatcagtctgataaggttaagatattcattcagtctatttataatattaacaatcgttaagcgtacactctatggaaagccctactccacagcctgctcctggttcggcgaccttcatggaaggatgcaaagacagtttaccgattgttattagttatattccggtggcctttgcgttcggtctgaatgcgacccgtctgggattctctcctctcgaaagcgtttttttctcctgcatcatttatgcaggcgcgagccagttcgtcattaccgcgatgctggcagccgggagtagtttgtggattgctgcactgaccgtcatggcaatggatgttcgccatgtgttgtatggcccgtcactgcgtagccgtattattcagcgtctgcaaaaatcgaaaaccgccctgtgggcgtttggcctgacggatgaggtttttgccgccgcaaccgcaaaactggtacgcaataatcgccgctggagcgagaactggatgatcggcattgccttcagttcatggtcatcgtgggtatttggtacggtaataggggcattctccggcagcggcttgctgcaaggttatcccgccgttgaagctgcattaggttttatgcttccggcactctttatgagtttcctgctcgcctctttccagcgcaaacaatctctttgcgttaccgcagcgttagttggtgcccttgcaggcgtaacgctattttctattcccgtcgccattctggcaggcattgtctgtggctgcctcactgcgttaatccaggcattctggcaaggagcgcccgatgagctatgaggttctgctgcttgggttactagttggcgtggcgaattattgcttccgctatttgccgctgcgcctgcgtgtgggtaatgcccgcccaaccaaacgtggcgcggtaggtattttgctcgacaccattggcatcgcctcgatatgcgctctgctggttgtctctaccgcaccagaagtgatgcacgatacacgccgtttcgtgcccacgctggtcggcttcgcggtactgggtgccagtttctataaaacacgcagcattatcatcccaacactgcttagtgcgctggcctatgggctcgcctggaaagtgatggcgattatataacccacaagaatcatttttctaaaacaatacatttactttatttgtcactgtcgttactatatcggctgaaattaatgaggtcatacccaaatggatagttcgtttacgcccattgaacaaatgctaaaatttcgcgccagccgccacgaagattttccttatcaggagatccttctgactcgtctttgcatgcacatgcaaagcaagctgctggagaaccgcaataaaatgctgaaggctcaggggattaacgagacgttgtttatggcgttgattacgctggagtctcaggaaaaccacagtattcagccttctgaattaagttgtgctcttggatcatcccgtaccaacgcgacgcgtattgccgatgaactggaaaaacgcggttggatcgaacgtcgtgaaagcgataacgatcgccgctgcctgcatctgcaattaacggaaaaaggtcacgagtttttgcgcgaggttttaccaccgcagcataactgcctgcatcaactctggtccgcgctcagcacaacagaaaaagatcagctcgagcaaatcacccgcaaattgctctcccgtctcgaccagatggaacaagacggtgtggttctcgaagcgatgagctaacgcgtcatctcgctcaaaaatccagatttataaaagaaaaaatgactggccagcatcgcaacatgctggcctttttggcaagcaggtcggctcagccgatgagttaagaagatcgtggagaacaatatgagcgcaaatgcggagactcaaaccccgcagcaaccggtaaagaagagcggcaaacgtaagcgtctgctcctccttctcaccttgctctttataattattgccgtagcgatagggatttattggtttttggtactgcgtcacttcgaagaaaccgatgacgcatacgtggcagggaatcaaattcaaattatgtctcaggtgtctggcagcgtgacgaaagtctgggccgataacaccgattttgtaaaagaaggcgacgtgctggtcactctcgacccgacagatgctcgccaggcgtttgaaaaagccaaaactgcactggcttccagcgttcgccaaacccaccagctgatgattaacagcaagcagttgcaggcgaatattgaggtgcagaaaatcgccctcgcgaaagcacaaagcgactacaaccgccgtgtgccgctgggcaatgccaacctgattggtcgcgaagagctgcaacacgcccgcgacgccgtcaccagtgcccaggcgcaactggacgtcgcgattcaacaatacaatgccaatcaggcgatgattctggggactaaactggaagatcagccagccgtgcaacaggctgccaccgaagtacgtaacgcctggctggcgctggagcgtactcgtattatcagtccgatgaccggttatgtctcccgccgcgcggtacagcctggggcgcaaattagcccaacgacgccgctgatggcggtcgttccagccaccaatatgtgggtggatgccaactttaaagagacgcagattgccaatatgcgtatcggtcagccggtcactatcaccacggatatttacggcgatgatgtgaaatacaccggtaaagtggttggtctggatatgggcacaggtagcgcgttctcactgcttccagcgcaaaatgcgaccggtaactggatcaaagtcgttcagcgtctgcctgtgcgtatcgaactggaccagaaacagctggagcaatatccgctgcgtatcggtttgtccacgctggtgagcgtcaataccactaaccgtgacggtcaggtactggcaaataaagtacgttccactccggtagcggtaagcaccgcgcgtgaaatcagcctggcacctgtcaataaactgatcgacgatatcgtaaaagctaacgctggctaatccagaggtgcgtgtgatgcaacagcaaaaaccgctggaaggcgcgcaactggtcattatgacgattgcgctgtcactggcgacattcatgcaggtgctggactccaccattgctaacgtggcgatccccactatcgccgggaatctgggctcatcgctcagccagggaacgtgggtaatcacttctttcggggtggcgaatgccatctcgatcccgcttaccggctggctggcaaagcgcgtcggggaagtgaaactgttcctttggtccaccatcgcctttgctattgcgtcgtgggcgtgtggtgtctccagcagcctgaatatgctgatcttcttccgcgtgattcaggggattgtcgccgggccgttgatcccgctttcgcaaagtctattgctgaataactacccgccagccaaacgctcgatcgcgctggcgttgtggtcgatgacggtgattgtcgcgccaatttgcggcccgatcctcggcggttatatcagcgataattaccactggggctggatattcttcatcaacgtgccgattggcgtggcggtggtgttgatgacactgcaaactctgcgcggacgtgaaacccgcaccgaacggcggcggattgatgccgtggggctggcactgctggttattggtatcggcagcctgcagattatgctcgaccgcggtaaagagctggactggttttcatcacaggaaattatcatccttaccgtggtggcggtggtggctatctgcttcctgattgtctgggagctgaccgacgataacccgatagtcgatctgtcgttgtttaagtcgcgcaacttcaccatcggctgcttgtgtatcagcctcgcgtatatgctctacttcggcgctattgttctgctgccgcagttgttgcaggaggtctacggttacacggcgacctgggcaggtttggcctctgcgccggtagggattattccggtgatcctgtcgccgattatcggccgcttcgcgcataaactggatatgcggcggctggtaaccttcagctttattatgtatgccgtctgcttctactggcgtgcctatacctttgaaccaggtatggattttggcgcgtcggcctggccgcagtttatccaggggtttgcggtggcctgcttctttatgccgctgaccaccattacgctgtctggtttgccaccggaacgactggcggcggcatcgagcctctctaactttacgcgaacgctggcggggtctatcggcacgtcgataaccacgaccatgtggaccaaccgcgagtcgatgcaccatgcgcagttgactgagtcggtaaacccgttcaacccgaatgcccaggcgatgtacagtcaactggaagggcttgggatgacgcaacagcaggcatcaggctggattgcccagcagatcaccaatcaggggctgattatttccgccaatgagatcttctggatgtcagccgggatattcctcgtcctgctggggctggtgtggtttgctaaaccgccatttggcgcaggtggcggcggaggcggtgcgcactaagtacaactaagccagttcatttgaactggcttttttcaattaattgtgaagatagtttactgactagatgtgcagttcctgcaacttctctttcggcagtgccagttcttcgttgctgttgatgcgtacgtcacgttccagaatgctacgcgcaatatcctgcgcttcctgcaacgagtgcatctggtaagtgccacactggtagacgttcagttccgggatctgattctgatcctgcactttcagcacgtcttccattgccgctttccaggcatcagcaacacgctgctcatctggcgtaccaatcagactcatataaaaaccggtgcggcagcccattggcgagatatcgataatctctacaccattaccgttaagatggttacgcataaaaccagcaaacaggtgctccagggtatggatccctctttctggcatcacttctttgttcggcacgcagaagcgcagatcgaacacggtgattgcgtcgccatgcggggtgttcattgttttcgccacccgaactgcaggcgcttccatccgggtatgatcgactgtgaagctatctaacaacggcatttagccacctccggtaatttttttaaaaattttctgaactctttcttcccaggcgagtctgagtatatgaaagacgcgcatttgttatcatcatccctgaattcagagatgaaattttggccactcacgagtggcctttttcttttctgtcaggcgtgtttttccagccacaccgcaaacggttcggtatcagcggcttccatttcctgctgacggcgttcagacgcctcgcgctcggctacaaaatcctcttcgcgcagaatttccagcggctcttcacgcagcagattacggtaggcttctgcaaatgctttgcctgttccgccaataccagtatcaatcatagaccttaagatacgggcagagaaagtcagatcgggattatcgaagcaggcaaccagttcatcacacactttctgatacgcttcgccgccgttaatactatccagcgtttgcgcgacgcgtttcagatcgcggaacagatctttacccacctgcggtaacgggaactgtgcggtttcgcagccgatacccagcgtcagacccggtttgcgaccttcgaggatcacccggttccagttaacgcgtgtacaggcaagttcgctactgctcatttccggtgcatcagccagcgcacaccagaccataaacaggtcgaggaatcgcacctgctgttcatctacaccaatcggcgagaacgggttgatgtccagcgaacgcacttcaatatattcaatgccgccacgtaacagcgcatcagaaggcgactcgccgctgcgggtaacgcgttttggacgaatcggcgcgtacagttcgttttcaatctgcaacacgttgctgttgatttgcagcctcttaccgtctttctcaataccaatcttcgcgtactcttccgatggcgttttgattgcctgtttaaggcccgctacgtactcgtaaagatcgttgaaggtaataccaagattgctttgcgatttattggtatagccgagatcgctcaaacgaagagaggtcgcatacggcaggtaatacataccgcactcggttttctcaaacggcagcgacgttggttttccttgcaggaaagaagaacaaatcgccggagatgcaccaaacagataaggaatgacccaaccgaaacgatagtaattgcggataacgcggaaatagcccgcagaaattttctctttggcatcagcgcccgagatatcaccgcacttcgcttgccagaatgccattggcaaagagaaattgtagtgcacgccggaaatggtttgcatcagcgcgccgtagcgatttttcagcccttcacgatacagcgttttaaagcgtccggtgttagaagtgccgtactgtgccagttcgatgtcctgaccttctgcgatgtagcatggcatacttaacggccacatccgctcatcgcccatattgcgcgccgtataacgatgcagatcgcgcataaaggtcagcatatgttcaatatcaccatccactggtgtaatgaattccagcaatgcttccgcaaaatcggtagtaatccatttgtgcgtcagtgcggaacctaatgcttcaggatgacctgttgttgccagtgtgccatcagcattaacacgcaaagtttcgcgctccagcccacgctgtatcccctttaacgcctgaggatgtttttccagccaggccagcgcctgtgatacgtccgggatcaaattgacctcccgcctgtcaaaatcgttttaattagcataactgtaatggtgaccatatgtgcaggcctacaattagtgccaccacatcatgccctgaacggtcgctgctgcaactgcaacatagcgtaacgctttaccaaggcacaaaaaaaagattaccggtccccacgagatgcgcatccatcccgctaacagacacagtaaatcgccaaccacgggcatccagcttaataatagcgtgactgcaccatagcgtttcagccagccggtagctttctcttgccagcgcgatgttttacgcaatggaaagaaacgcccaaggataacgttagttaaccctccaaggctattacccattgttgctgttaaaactaaaacccagggatgactgatcccggaaagcaacattgccaccagcacgacttcggagttgccgggtaatagtgtagcgctgagaaaactactggcaaacaacgagaaaagcgataacgcttcactcacagcaagcgaacatccacggcgtccatgcctgctgcacgggccgcctgaataccgaaatcggcatcttcaaagaccacacactgcgtcggttgcacgcccatacgctgcgcgcacaacaaaaatgtgtctggcgcgggtttatggtgtttgacgtgatcggcagcgacgacggcgtcaaaataatggcgtaatcccaggtgcgccagcaatgcctcagcgatggcgctttcactccccgttcctacagccattgggcgacgaccatgccaacttttcaccacatcaacaagaggaagcggttcgacgctatccagcagcatacttcttactgcttctgttttttcacgcgctaacgcatgcgggtcgagatcggcctgattcagctcaataattgcctgagcaatacgccaggtgggcgatccattaagcgcaatcatcgcctgaatatcgtactgaagaccgtagtgccctaatacttcgcgccacgctttacggtgcgtaggctccgtatccaggattgtgccatccatatcaaaaattaaacctgcataacgctcgtacatggtcttctcgcaagtcgaaaaatatgacgctactttagcgtaattgcttgattttgtcgctgatggcgaaggagaagaaaattcaggaaatggataaaggagttatttagaaatgagatatttttgaaggaaattttttggagaagatggtgcatccgggaggatgactcactgacgttcgcccttcgggccgttgctggcgcaacgttatccttcctggtgcctgcggttaataccgctatctcttcgataccttcattgctgaaggttacggagaatatggtgcatccgggaggattcgaacctccgaccgctcggttcgtagccgagtactctatccagctgagctacggatgcatcgggaaaacttattctactgctgatattgataccgctactaaagccatatcaattaagagatggtgcatccgggaggattactcgccttgcggctcgcccttcgggccgttgctaaagcaacgttatcatccctagtgcctgcggttaattccgctacctcttcgataccttcattgctgaagatttcggagaatatggtgcatccgggaggattcgaacctccgaccgctcggttcgtagccgagtactctatccagctgagctacggatgcatcgggaaatttattttactgctgatattgataccgctactaaagccatatcaagtaagagatggtgcatccgggaggattcgaacctccgaccgctcggttcgtagccgagtactctatccagctgagctacggatgcatcgggaaacttactttactgcagattttttgataccgctactaaagccgtatcaagtaagagatggtgcatccgggaggattactcgccttgcggctcgcccttcgggccgttgctaaagcaacgttatcctccctggtgcctgcggttattaccgccacctcttccataccttcatcgctgaaagtacgtagaatatggtgcatccgggaggattcgaacctccgaccgctcggttcgtagccgagtactctatccagctgagctacggatgcaaatggcggtgaggcggggattcgaaccccggatgcagcttttgaccgcatactcccttagcaggggagcgccttcagcctctcggccacctcaccacacgcctcttacgagtgcttcgaagaacttgtttatcgctcatcgtcgctgcgtggcgcacatattactttctgagacttataagtcaaacaatttttcctacacttttatcgtttgcacacttcacgttcaattagtctgtaaaaacgtcaaaaagagtgttttatcaacagaagaatggaggtctgacagatagtagtaatgcaaaaaaatggagacttaagttgaatgaacgggagtaaagcgaaaagactatagagtgaaggagaaattttgagggtgcgtctcaccgataaagatgagacgcggaaagattagtaactggactgctgggatttttcagcctggatacgctggtagatctcttcacggtgaacagaaacttccttcggggcatttacgccaatacgtacctggttgccctttacccctaaaactgtcacggtgacctcatccccaatcatgagggtctcaccaactcgacgagtcagaatcagcattctttgctccttgaaagattaaaagagtcgggtctctctgtatcccggcattatccatcatataacgccaaaaagtaagcaatgacaaacacattacatctaagcagtcatggcattacattctgttaaacctaagtttagccgatatacacaacttcaacctgactttatcgttgtcgatagcgttaatgcgaatgccgtgaagcgagtccacggcattgcctgacgcttatattattgcaatttcgcgctgacccagcctttcacactggctaacgctgcaggtaaggccgcagcatccgtaccaccggcttgcgccatgtcaggacgtccaccacccttgccgcccacctgctgagcgaccataccaatcagttcccctgctttcacacgatctgtgacgtccttagatacgcctgcaatcagagaaaccttaccttcgactaccgttgccagcacgataattgtcgaccccagctgattttttaaatcgtcaaccatggtacgcaacattttcggctcaacaccgctaagctcgctaaccaacagcttaacaccattaacatcaattgccttactggaaagatttgcgctctcctgtgcggcagcttgttctttaagctgttgtaactctttttccagctgacgcgtacgttccagtactgagcgcactttatcagccagattattgctatcgcctttcagcagatgcgcgacttcgcttaagcgatcgctgtctgcatgaacggtggcgatagcaccttctccggttaccgcttcgatacgacgaacgcctgcagcagtacccgattcagagatgatgcggaacagaccaatatcaccagtgcggctggcgtgagtaccgccacacaactcggtagagaaatcgcccatgctcagcacgcgtacgcgctcatcatacttctcgccgaacagcgccatcgcacctttcgctttcgccgcttcgagatccatgatgttggtttcgatcggcaaattgcgacgaatctgtgtgttcaccaggtcttcgaccgcacgaatctcttctggtttcatcgcttcgttgtgtgagaagtcgaagcgcagcaccttgtcgttaaccagtgaacctttctgcgatacatgagtacccagaacctggcgcagcgcagcgtgcatcaggtgcgttgcggagtgattcagacgaatacgggcgcgacgagcctcatcaacatcagcctgcaccgcgtcgcccactttcagagaacccgcagcaagtttaccgatgtgaccaatcgcctggccgtatttctgcgtatcttccaccgcaaaggagaagttagcgcctttcagttcgcctttatcgccaacctgaccgccggattccgcatagaatggcgtttgatccagcacgaccacagcttcctggcctgcattgatggcatcaaccgctttaccatcaacaaacagcgcagtcactttgccgttcagttccagatggtcatagcctttaaattcagatgcactgtcaacacggatcattgcgttgtaatcggcaccaaagccgctggcttcgcgcgcgcgacgacgctgctcttccattgcagcttcaaaaccagcttcgtcaactttgatgttgcgctcacgacaaacatcagccgtcaggtcaaccgggaagccataggtgtcgtacagacggaaagcagtttcaccatccagcgtatcaccagaaagttttgccagctcttcatccagcaacgccagaccgcgctccagagtacgagcaaactgctcttcttcagtcttcagcacctgctcaacctgcgcctgctggcgtttcaggtcttcacccgcagagcccataacgtcgatcagcggaccaaccagtttgtagaagaaggtttctttcgcgccgagcatattaccgtgacgcactgcgcgacgaatgatacgacgcagtacataaccacggttttcattggacggcattacgccatccgcgatcaggaacgcacaagaacgaatgtggtcagcgattacgcgcagcgatttattgctcagatcggttgcgccagtgactttcgctaccgcctggatcagcgtgcggaacaggtcgatgtcatagttagagttaacgtgttgcagcaccgcagcaatacgctccagacccataccggtatctacagacggcttcggcagcggttccatcgtgccatcggcctggcggttgaactgcatgaagacgatgttccagatctcaatgtagcggtcgccgtcttcttccgggcttcccggagggcccccccaaatgtggtcgccgtgatcgtagaagatttcggtgcacgggccgcacggaccagtgtcacccatctgccagaagttgtcagatgcgtatggcgcacctttgttatcgccgatgcgaataatacgttcgcgcgggatccctacttctttttcccagatttcgtaggcttcgtcgtcgctttcatagacggtaacccacagacgctctttcggcagggcaaaccatttttcgctggtcagcagttcccatgcaaactgaatggcatcgtgtttgaaatagtcgccgaagctgaagttgcccagcatttcgaagaaggtatggtgacgcgcggtgtaaccgacgttttccaggtcgttgtgtttaccacccgcacgcacgcagcgttgggaagtggtagcgcgggaataattacgcttgtcgagcccaaggaacacatccttgaactggttcatcccggcgttggtaaacaacaaagttgggtcgttatggggtaccagggagctgctggcaactacctgatgtcccttactatggaaaaagtcgagaaacgcctgacggatctcagcggtgctcttgctcataattatcctgaaatcaagctaacgaaatatcgccaccagctccagcgtgtcttaaccgccgggctggtaactgaaaagtgggaataagataagttttcttgactgggaagtaaaataccgtatgcgttcagtcggcaaaatttcgccaaatctcctggatatcttccatcagatagccacgatagagcagaaaacgctggatcttaactttttctgaaaagacagttggcaaaggttcgccatattttcgcgtcgcctgatcgcgcgccagtgcgcaccagtcgatgtcacattcacgcatcgctttttctgtcgcttcgcgggaaatacctttctgattcagttcctggcgaatacgcgcaggtccataacctttgcggctacggctggcgataaagcgcgcaacaaatcggctgtcatcgagatagccatgttcatggcaccaggcaataacgcgctcgtaatcttctgccgtagcatcaatctcttctgggccatttttgcccataatcggtgccgcgagtttacgtcgcagttcttgctcactgtgatcgcgcaccgccagaatgcgtaccgcacgatccaacaggcgagcatatgccgggcgacgggatgttgattctgtcatggcatatccttacaacttaaaaaagcaaaagggccgcagatgcgacccttgtgtatcaaacaagacgattaaaaatcttcgttagtttctgctacgccttcgctatcatctacagagaaatccggcgttgagttcgggttgctcagcagcaactcacgtactttcttctcgatctctttcgcggtttccgggttatctttcagccaggcagtcgcattcgctttaccctgaccgatcttctcacctttgtagctgtaccacgcgcctgctttctcgatcagcttctcttttacgcccaggtcaaccagttcgccgtagaagttgataccttcgccgtagaggatctggaattcagcctgtttaaacggcgcagcgattttgttcttcaccactttcacgcgggtttcgctacccaccacgttttcgccctctttcaccgcgccgatacgacggatgtcgagacgaacagaggcgtagaatttcagcgcgttaccaccggtagtggtttccgggttaccgaacatcacaccaattttcatacggatctggttgatgaagatcagcagcgtgttggactgcttcaggttacccgccagcttacgcatcgcctggctcatcatacgtgccgcaaggcccatgtgagagtcgccgatttcgccttcgatttccgctttcggcgtcagtgccgccacggagtcaacgacgataacgtctactgcgccagaacgcgccagggcgtcacagatttccagtgcctgctcgccggtgtccggctgggagcacagcaggttgtcgatatcgacgcccagtttacgtgcgtagattgggtccagcgcgtgttcagcatcgataaacgcacaggttttaccttcacgctgcgctgcggcgatcacctgcagcgtcagcgtggttttaccggaagattccggtccgtagatttcgacgatacggcccatcggcagaccacctgccccaagcgcgatatccagtgaaagcgaaccggtagagatggtttccacatccatggaacggtcttcacccaggcgcatgatggagcctttaccaaattgtttctcaatctggcccagtgctgccgccaacgctttctgtttgttttcgtcgatagccatttttactcctgtcatgccgggtaataccggatagtcaatatgttctgttgaagcaattatactgtatgctcatacagtatcaagtgttttgtagaaattgttgccacaaggtctgcaatgcatacgcagtagcctgacgacgcaccgcatcacggtcgccgctgaagcattcccgccgggtaatgccttcaccgcgggcagtggcaaaagcaaaccagacggtgccgacaggcttctcttcactgccgccatccggcccggcgataccactaatagacacggcataatcagcacgagccgctttcagtgcgcctatcgccatttccaccacgacgggttcactcaccgcgccatgctgcgccagcgtctcttcgcgtacgccgatcatctgcgctttggcttcgttactgtaggtgacaaatccgcgttcaaaccaggcggagctaccggcaatatcggtaatcactttcgctacccaaccaccggtacaagactcggcagttgttacggttgcgccacgggctttcagcgcctgcccaacctgttcacttaactgcatcagttcactgtcagtcatcacaacctctgtcagtcaaaaatttatgccggacaagatagcactttcgtcaggaagatggtgttggcgttgcaattttacgaggaggattcagaaaaaagctgattagccagagggaagctcacgcccccctcttgtaaatagctactgtactcgcgccagcgccacggcttgtcctaactgccagaccgccattgcgtaatgggtgctgtggttgtaacgggtgatggtgtagaagttcggcagaccgtaccagtactggtagccggtgccaacatccagacgcagcaggctggcttgttgatggttgcccagcggctgctgtggcgttaaacctgcggcggcaagctgcgaaatgctgtacttagttttgaagccatttggcaagcctggagcctgaccgtttgccattaccgcgacctgatcgcctttcacccagccgtgcgctttgaaatagttcgccacgctaccgatcgcatcaaccggatcccacaggttgatatgcccgtcgccgctgaaatctaccgcatattgtttgtaagacgacggcataaactgtccgtagcccatcgccccggcaaaggaacctttcagattgagcggatcgtcctgctcgtcgcgcgccatcaacaggaaggtttccagctcgccagagaaatactccgcgcggcgtgggtagttaaatgacagcgttgccagcgcatcgaggatgcgagttttccccatcacgcgcccccagcgggtttcaacgccgataatcccgacgataatttccggcggtactccatacacctgccacgcgcgattcaacgcatcttcatactgattccagaaaaccacaccgttctgcacgttgtccggcgtaataaattttttgcgataacggagccatgcgccgttcggacctgatggcggtttcaccgatgtggttggtgcctggttatccatcagccgcagtaccgaatccagacgcttcgcctgggagagaatttcctgcaactgctgacgatcgaaaccgtgtttgttcaccattttgtcgatgaactgctgggcattcgggttattagcgaaatcgccgcccatctgcatcacattgtgctgcggctcaagcaggaagccgccagacggcgttccggtggtcgtatcagtctcagtaggttttggcttgctgctacaggcggcaagcaacacaaaaaggggaagcaatgttacataacgacgcttgaacatgaggggtccatttaacagattcaaccaggggcaagtatggtaaagcatcacgccccgcacaaggaagcggtagtcactgcccgatacggactttacataactcaactcattcccctcgctatccttttattcaaactttcaaattaaaatatttatctttcattttgcgatcaaaataacacttttaaatctttcaatctgattagattaggttgccgtttggtaataaaacaataaatcctgaaggagagaacaatgatagaaaccattactcatggtgcagagtggtttatcgggctgttccaaaagggcggagaggtgtttaccgggatggtgaccggcattcttccgctgttgattagcctgctggttatcatgaacgcactgattaattttatcggtcagcatcgtattgaacgttttgctcaacgttgcgccggtaaccctgtttcccgttacctactgttaccgtgcattggcacgtttgtcttttgcaatccgatgaccctaagcctgggtcgctttatgccggaaaagtacaaacccagctactacgcggcggcctcttatagctgccactcaatgaatggcctcttcccccatatcaaccctggcgaactgtttgtttatcttggcattgccagcggtctgacaacgctgaacctgccacttggcccactggcggtgagttatctgctggttggtctggtcaccaatttcttccgcggctgggtgaccgatctgaccaccgccatttttgagaaaaagatgggcattcaacttgaacaaaaagttcacctggcaggagcaacatcatgacgcatattcggatcgaaaaaggaacgggtggctggggcggcccgcttgagctgaaagccacgccgggaaaaaaaatcgtctatatcaccgccggtacccggcctgcgattgttgacaaactggcacagcttactggctggcaggctattgacggatttaaagaaggtgaacccgcggaggcggaaattggtgtcgcggtaatcgactgtggcggcacattacgctgcggcatctatccgaaacgacgtattcccaccattaatatccactcgacgggcaagtccggtccgctggcgcagtacattgtggaagatatttatgtctctggcgtaaaagaagaaaacatcactgtagtaggtgatgcgacaccacaaccctcttccgtgggccgtgactatgacaccagtaagaaaatcaccgaacaaagcgatggtttactggcgaaggtgggaatgggcatggggtccaccgttgcggtgctgtttcaatctggtcgtgacaccatcgacactgtattaaaaaccattctgccgtttatggcattcgtctcggcgctcattggcatcattatggcttctggccttggtgactggattgcccacggtcttgctccgctggcgagccatccactgggtctggtcatgctggcgctcatctgttccttcccactgctttcacctttcctcggcccaggcgcagttatcgcacaggttatcggcgtattgattggcgtgcagattggtctcggcaatattccgccgcatctggctttaccggcactgtttgccatcaacgcgcaggcggcctgcgacttcatcccggtcggtttgtcgctggcggaagcccgtcaggacacggttcgcgtcggtgtcccttctgtactggtgagccgctttttaaccggcgcgccgactgtactgatcgcctggtttgtctccggttttatctatcaatagaggctgaaacatgaccgttatttatcagaccaccatcacccgtatcggcgcgagtgccattgacgccctcagtgaccagatgctcatcacctttcgtgaaggcgcgcctgcggacctcgaagagtattgcttcattcattgccacggcgagttgaaaggtgcactccatcccggtttgcaattttcactcgggcagcatcgctatccggtgaccgctgttggcagcgtggcggaagacaaccttcgcgaactgggtcatgtcaccctgcgcttcgatggtttaaacgaagcggaatttccgggcactgtccatgtggcaggccctgtccccgacgatatcgcgccgggatcggttttgaagtttgaatctgttaaggagtaaaaaatgaatcaggttgccgttgtcatcggtggtgggcaaaccttaggcgcgttcctgtgccacggtctggctgccgaggggtatcgcgtcgcggttgtcgatattcagagcgacaaagccgcaaatgtggcacaagaaattaacgccgaatatggtgaaagtatggcgtacggttttggtgctgacgccactagcgagcaaagcgttctggcgctctctcgtggggtagatgaaatctttggtcgcgtggatttgctggtctacagcgccggaatagcaaaagcagcctttatcagcgacttccagctcggcgattttgaccgttcgctacaggtgaatctggtgggttatttcctgtgtgcgcgtgaattttcgcgtttgatgatccgcgacgggattcaggggcgcattattcagatcaactcgaaatccggcaaagtgggcagcaaacacaactctggctacagcgcagcgaaatttggtggcgtcgggctgactcaatcactggcgctggatctggcggagtacggcattacggtgcattcactgatgctcggtaacctgctgaaatcgccgatgttccagtcactgttgccacaatacgcgaccaagctgggtatcaaaccggatcaagtcgagcagtattacatcgacaaagtaccgctcaaacgcggctgcgattatcaagatgtgctgaatatgctgctgttctacgccagtcctaaggcgtcgtactgcaccggacagtcgatcaatgtcaccggcggtcaggtgatgttctgatcaacagcggagatccattaaggatctccgtgagactatagaatgcctgatgcgctacgctcatcaggcatacaggacttccgccactacattaaggaaaagttatggtatccgcactcatcaccgtcgccgttatcgcctggtgtgcgcaactggccttaggcggctggcaaatttctcgttttaaccgtgccttcgacacactatgccagcaagggcgggttggcgtgggccgttccagcgggcgctttaaaccgcgggtcgtggtcgccatcgcgctggacgatcagcagcgcatcgtcgacaccttgtttatgaaaggactgaccgtcttcgcccgaccgcaaaaaattcccgcaattaccggtatgcatgcgggtgatttacagcccgatgtgatctttccccatgatccactatcacagaatgctctatcattggcgcttaaactgaaacgtggataatttcgttgtgaatgttacttgcttgcgaagttatcattttgaaacctaaatcaggtaatcacgcccatgaaacctcgtcagcgtcaggccgccattctggagtatctgcaaaagcagggtaaatgctcggttgaagaattggcgcaatactttgacaccacaggcacaaccattcgcaaagatctggtcattctggaacatgccggaaccgtcattcgtacttatggcggagtggtgttgaataaagaggaatccgatccgcctatcgatcataaaacactcatcaacacccacaagaaagagctgattgcagaagctgccgttagttttatccatgatggcgattcgatcattcttgatgctggcagtaccgttttgcagatggttcccctgctctcgcgctttaataacatcacggtgatgaccaacagcctgcatatcgtcaatgcgctatccgaactggataacgaacaaactatcctgatgccaggcggaacgtttcgcaaaaaatcggcctcatttcacgggcaactggcagagaatgccttcgagcatttcaccttcgataaattgtttatgggcaccgacggcatcgatctcaatgcgggcgtaaccacctttaacgaggtttataccgtcagtaaggcaatgtgcaatgccgcgcgcgaagtgattttgatggcggactcatcaaagtttggccgtaaaagccccaacgtagtttgcagtcttgaaagcgtcgataagctgattaccgacgcaggtatcgatccggcgtttcgtcaggcgctggaagagaaagggatcgatgtgatcataaccggagagagcaatgagtgaagcactactgaacgcgggacgtcagacgttaatgctggagttgcaggaagcaagccgtttaccggaacgtctgggcgatgattttgttcgcgccgccaatatcatcctgcactgtgaaggcaaagtggtggtttcgggaattggcaaatcgggccacattggtaagaaaatcgccgcaacgcttgccagtaccggcactccggctttttttgtccatccggcagaagcgctgcacggcgatctggggatgatcgaaagccgcgatgtgatgctgtttatctcttactccggtggcgcgaaggaactggatctgattattccgcgtctggaagataaatctatcgcgctgctggcgatgaccggcaaaccgacgtcaccgctgggcctggcggcaaaagcggtgctggatatctccgtagaacgcgaagcctgcccgatgcaccttgcgccgacctccagcaccgtcaataccctgatgatgggtgacgcgctggcgatggcggtcatgcaggcgcgcggatttaatgaagaagattttgcccgctcccacccagccggggcactgggcgctcgcttgctgaataaagtgcatcatctgatgcgccgtgacgatgccatcccacaggtggcgttaaccgccagcgtgatggatgcgatgctggaactcagccgcaccggtctggggctggtggcggtatgtgacgctcaacaacaggtacaaggcgtctttaccgacggcgatttacgtcgctggctggttggcggcggcgcactcaccacgccagtcaatgaagcgatgacggtcggcggcaccacgttgcaatcgcaaagtcgcgccatcgacgccaaagagatcctgatgaagcgcaaaatcactgccgcaccggtggtggatgaaaacggcaaactcaccggcgcaataaacctgcaggatttctatcaggccgggattatttaatccttcaatcccagacgtttcgccagccgatgcaggttggcgacgtcggtttccagcatccgcgcgcaggcagcccagttgtgatgattttgtgccagtgcctgacgaatagtttcacgctggaacgcttctgtcgcttcacgcaggttttgcttaacaacgggcaccgccgccacttctggcgtcggcaacgtcacctcaggaaaagcaaaatgttgcgcctcaagaatcacttcatcgccgctgcgggtggctctcgccagaactaccgcccgatgaatagcatgttccagttcgcgcacgtttcccggaaaactgtagtgttgcagtaaatttcgcgctccggcacttaataccacgcgggagagcccctgccgcaaacgacactgctcgcagaaataccccgccagcagaatgacatcatcgccccgctcacgcagcggcggcaccgaaagtggaaacacgctcaggcgatgaaacaaatcggcgcggaatcgccctgccagcacctcttcgcgtaaatcgcggttagtcgccgccagcacgcgcacatcgacccgcaaacaacggtcatcgccaacgcgctgaatatcgccatactgcaacaccctcagcagcttggcctgcaatgccaacgacaactcgccgatctcatccagaaacagcgtgccgttatccgccatttcaaacttcccgctgcgattactgatagcgccagtaaacgctcctttcacatgcccgaacaactcactttccgccacactttccggcagtgcagcacagttgagatagaccagcggattcaccgcccgtggcgaggcttcatgaatcgctttcgccaccagctccttaccggttccagtctcaccgctgatcaggacgttgagatcggacgccgccacaatctcaatctcttttttcagttgcgtcatgccaggggacaagccaatcatctgcgtctgtttcaccgcttcaaacggcgtggcatcgcctggcagcatattctggctttccagttgttcaatcagcaacgcattgcttaacgctcccgccgccagcgcagcaatcagccgtagctcttcgtcgctgaaaacatcgaactgatcgggctgcatcccgtcgagcgtcagtgcgccgatcaggttttgcccggcaaacaatggcagaccaacgcaggcgtgaaccttcagactctcctgcccaggaatcaaaccgtcatagggatcgggcaattcgctgtctgcgggaaagcgcaccacatccccggcgcgggcaatcgcttccagccgtggatgcccttccagcgcaaagcgtctaccgagtacatcctttgccagaccgtcgatggcaagcggaataaactgccgcgaatcgtaacgtagcaacgcagacgcatcgcactccagcacctgacgtagcgtggtgatcaggcgctgaaaacgatcctggtgaccaatcccacgctgcaattcgatggcgatattcgccagcacatcaacggaaaaactcatctttgcctcactgtcaatttgactatagatattgtcatatcgaccatttgattgatagtcattttgactactcattaatgggcataattttatttatagagtaaaaacaatcagataaaaaactggcacgcaatctgcaattagcaagacatctttttagaacacgctgaataaattgaggttgctatgtctattgtggtgaaaaataacattcattgggttggtcaacgtgactgggaagtgcgtgattttcacggcacggaatataaaacgctgcgcggcagcagctacaatagctacctcatccgcgaagaaaaaaacgtgctgatcgacaccgtcgaccataaattcagccgcgaatttgtgcagaacctgcgtaatgaaatcgatctggcggatatcgattacatcgtgattaaccatgcagaagaggaccacgctggggcgctgaccgaactgatggcacaaattcccgatacgccgatctactgtacagccaacgctatcgactcgataaatggtcatcaccatcatccggagtggaattttaatgtggtgaaaactggcgacacgctggatatcggcaacggcaaacagctcatttttgtcgaaacaccaatgctgcactggccggacagcatgatgacttacctgacaggcgacgcggtgctgttcagtaacgatgctttcggtcaacactactgcgacgagcatctgttcaacgatgaagtggatcagacggagcttttcgagcagtgccagcgttactacgccaatatcctgacgccgttcagccgcctggtaacaccgaaaattaccgagatcctgggctttaacttaccagtcgatatgatagccacttcccacggcgtggtatggcgcgataacccgacgcaaattgtcgagctgtacctgaaatgggcggctgattatcaggaagacagaatcaccattttctacgacaccatgtcgaataacacccgcatgatggctgacgctatcgcccaggggattgcggaaaccgacccacgcgtggcggtgaaaattttcaacgtcgcccgaagcgataaaaacgaaatcctgactaatgtcttccgctcaaaaggcgtgctggtcggcacttcgacgatgaataacgtgatgatgccgaaaatcgccgggctggtggaggagatgactggtttacgcttccgtaacaaacgcgccagtgctttcggctctcacggctggagcggcggtgcggtggatcgtctttccacgcgcctgcaggatgcgggtttcgaaatgtcgcttagcctgaaagcgaaatggcgaccagaccaggacgctctgaagttatgccgtgaacacggtcgcgaaatcgcccgtcagtgggcgctcgcgccgctgccgcagagcacggtgaatacggtagttaaagaagaaacctctgccaccacgacggctgacctcggcccacggatgcagtgcagcgtctgccagtggatttacgatccggcaaaaggcgagccaatgcaggacgttgcgccaggaacgccgtggagtgaagtcccggataacttcctctgcccggaatgctccctcggcaaagacgtctttgaagaactggcatcggaggcaaaatgagtaacggcattgtgatcatcggttcgggcttcgccgcccgccaactggtgaaaaatattcgcaaacaggacgccactattccattaaccctgattgccgccgacagcatggatgagtacaacaaacctgacctcagccatgttatcagtcaggggcaacgtgccgatgaccttacccgccagacggcgggtgaatttgccgagcagtttaatctgcacctgtttccacaaacctgggtgacggatatcgatgccgaagcccgtgtggtgaaaagccagaataatcagtggcaatacgacaagctagtactggcaaccggtgccagtgcctttgtcccgcctgtgcctgggcgtgagttaatgctgacgttaaatagtcagcaagagtatcgcgcctgtgaaacgcaactgcgggatgcccgacgcgtgttgattgttggcggtggtttgattggtagcgaactggcgatggatttttgtcgtgcaggcaaagcggtcacgctaatcgacaacgctgccagtattctggcgtcgttaatgccaccggaagtaagcagccgcttgcagcatcggttgacggagatgggcgttcatctgctgttgaaatctcagttacaggggctggaaaaaacggattctggcattcaggcaacgctggaccgccagcgcaatatcgaagtggatgcggtaattgccgccaccggactgcgcccggaaaccgccctggcacgacgcgccgggctgacgattaatcgcggcgtttgcgtcgatagttatctgcaaaccagtaataccgatatttacgcgctgggcgattgcgcggaaattaacggtcaggtattgccgttcctccagccgattcaacttagcgcgatggtgctggcaaaaaatcttctcggcaataacacgccgctgaaactcccggcgatgctggtgaaaatcaaaacgccggaattaccgctgcatctggcaggcgaaacccagcgtcaggatttacgctggcaaattaataccgaacgccagggaatggtggcgcgcggcgttgacgatgctgaccagcttcgcgcctttgtggtcagtgaggatcggatgaaagaggcatttggattgttgaaaacattgccgatgtaggtgggctactgtgcctaaaatgtcggatgcgacgctggcgcgtcttatccgacctacggggacgcatgtgtaggccggataaggcgtttacgccgcatccggcaatggtgtccaaatgcaacacgttttatccgttctggacttcacccgctaaccaacgcgccgcagcaataaccccctgccccagagacaaaccgccatcacccgccggtaaactctgtggaaagagcaatgtgaaatcagcgagataatgcgccagacgtgcacgcagcaaacggttatgaataaccccgccgctaaataccagcgtagtgataccacgcatcgtggcctgctcacgcatcaacgcggcaaaaccctgcgccagcgcatcatgaaacgcccacgcgcgttgattaaccggtgcctgccagttcagccactgctgccagaaagtggcgagatccagttgattgtccacccgcggcattgtcaccggatgcgtcactccgtggcatgaggctgcgagcgcctccagagcacaagccgcttcaccttcataacttaacgtggctggcgcacagcccagtgccgccgccactgcatcgaaaaaacgcccacacgatgacgccagcggcgcgttaattccacgctcaatggcccgcgccagcacgctccagttttgctgttgcacacttgctgtttcagagtaattctgccactccggcacaaagcgcaggcactgcgccagcaggtttcgccacggctgcttcgctgccaaatcgccacccggaagcgccactgcaggcaagccgcccaggtgctcacattcgcgatagttcacccgcaggcactcgccgccccacaaagcgccgttctcccccataccgataccgtcgagcgtcaaagcaatgacatcaccgccatccagcggccactgatgctctgccagacacgccgctgcatgggcatgatgatgcagtaccgtttgcgtcggcagattcatttcacgcgcccactggctggagacatagcccggatgcgcgtcatgcacaacgtattgcggggtaaaatcgtagatgttttgcatcaggcgtaacgcttcgcgccactgcatctggatgccatcgtcacttaaatcgcccagatgctgactcaacaccgcttgttcaccgcgcaccaggcagaaggtatttttcagatccgcgccgagacacagcacaggcggaacatttttaaagcccggaggcaaagccagcgcatccggcacatacccccgcgaacggcgcagcatttcgccgctttcgcgcaccaccgaatcatccatccgctgcacgatgtcgcggttatgtatcaagaatccgtcggcaatgccctgcaaatccgccagcgcctgttcgttgctgatagctggtggtttaccgctcaggttgccggaggtcatcaccagcgggcattgcagttcctgtaacagcaaatgctggagcgggttcgcaggcaacattaccccgacttcgttaaggtcaggggcgatatcatcacaaagctcaggaacgtattttttatccaccagcacaatcggcgcggcgggcgtggtaagcaactggcgcgcagcgtctggtaaaccgtcagccactggcaacatgaccgccagcggtttcgccgggcgatgtttgcgcgcccgaagtgtcgccaccgcgttactgttacgtgcatcgcaggcaagatgaaatccgccaatccctttgatggcgacaattttgcccatttttaactgtgcgatagctgcctgtaatgccgcctcttgttccgcatgttcaccatgacttacccattcaagatgcgggccacactccgggcaggccaccggctgggcgtggaagcgacgatcgagcgggtcacggtactctttgtcacaggccggacatagcggaaacgccgccatcacggtaaacgggcggtcgtaaggcatggcgcgaataatggtgaaacgcgggccgcagtgggtacagttgataaacggataacgataacgccgttcgcctggggtattcatttcggcaaggcaagcagggcaagtagcggcatcgggaacaatttgcgtattcatggtgccgcctgtgctctggcgtatagtgaactcggtgggcagttgtgaccagataaacggctcacgctcgacgctatcaatacgcgccagcggcgggcagtgctgatacaattgaacaagaaacgtttccgggtcttcccgcagccggacttctacgccatcgccgtcattacagacatcgccgtgaagatttaattgctgtgccagctgccagacaaacggacgaaaaccgacgccctgcactttgccacgaatacgcagttggacaccgcaagatgtgttttttgccattgagttattcccgccatcatgaattgcgtaacccgccctgccggacacgacagcgtcgcatccggcagtcacaggtcggcgataccgcccgctccgtattctacgaatatttccgggaattcctttgatgccagaacagttctgtaagatttttagaacatcagcgccgtacggcggcgtttttctgcgctcagttgttcaagtttattacgatcgacacaaatcagcgcatgagtcgggcaagccgccatacacgccgggccgtcttcacgatggttgcacaggtcgcatttattggcttcggctttgtcagcccgtacattcagacccgcgccgctgttgcggatcaccggacgtaccaccacttccatcgcaccatacgggcaagccacaacgcaggttttgcaaccaatgcaacgttcctgcatcacatgaacaaaccctttatcacggctgatagcaccattcgggcagacgttagcgcacggtgcatcttcacactgacggcaaactgtcgccgtggaaatgttcacacctttaatgacatggatacgcggtaaaaaagtttccggggtcagcgatgcacagtcctgattttcctgatgagaaaccacgcacgctacttcacaggtacggcaaccaatacatttactcgcgtcagcaatgatgaaacggttcatcaaattctccagcaatgacagttaatgcgccgatacattcacaaatcatgccagtttttaatttactgttatttaaggaaattaatttctgtaatgcaggaaaaacgatgtcatcgacactagtgacgatgacatgtgatgacaatgtttatcgcgaaggagcaatgagtgagtcgcggcggatcagttttccgctgaaggttttcggcggtgagaaatccccgccatcgagcataaaaatcagccgtccaataatttcctgaatcatctcagtcaccggaatttttacgctggagagcgccggaacggtgtagggggcaatagcgatatcatcgaatccgataactgacacctgctctggcaccgctacgccgcgctcgtgtaacgctttcatcgcacctatcgccatatcgtcgttactggcaactaacgcgctaaatttagccccacgttcgagcaacatttctaccccttcggccccgctggcaggcgtccatttaccgttagcgataagtttttcattgagcgcaataccatgctgcgccagcgcgtctttatacccggcaagacgttcaatgctggtgggggaatccatcgagccggtaaggaaagcaatctcctgatgcccggcgtttatcaactctgccacggcgttaaaactggtctgtttatgatcgcaccagacgctatggctgctgtttttgcgcaggcggcgattaagcaccattatcggctgactgtgcgcgtcaatgatgtcatcgatctcatccacgcttaaaaaacgcgggtaaatcatgatcgcgtcgcagcgcagatccagcagatactgaatcgcctggcgctcttcttctgcgctgtgtttaccatctgccaatagcaactgccgccctttctcttccgccattcgcgcggcatgaaagagtaattcactaaaataaatgccgtggtaaagcgtgttggtcactaccagccccagcgtctgagtactcttcgccgacagattgcgcgccagcaagtttggacggtaaccgctctcttctaccgcctgaaacacgcgatctttagtctcctggctgacgtagccattacctgaaagcacgcgggaaacggtcgcttttgaaaccccggcgcgcttcgccacttccagcatcgtcgtcatcattttcatccctttacacgcaatcaacgcagtgtactgcaccgtttgccgattgtccttgcacaatcggcgggaaaaatattcaggtgaccggtttcacaaatataaaaaatgaacaattcactctcttgcttatttagtgacaactattcatgattttgtgaaaccggtttcttaattccgtttcagcatcggcatttttccgtcacgtcgactgataacaactacatctaccctactgataacaggataaaatccgatggccaaaaattatgcggcgctggcacgctcggtgatagcggcactgggcggcgttgataacatctcggcggtcacgcactgtatgacgcggttgcgctttgttatcaaagatgatgcacttatcgacagcccgacgttaaaaaccatccccggcgtgctcggcgtggtacgtagtgacaaccagtgtcaggtgattatcggcaataccgtttcacaagcctttcaggaagtcgtcagcctgctgccgggagatatgcagcccgcacagcccgtgggtaaacccaaactcacgctacgtcgcattggtgcggggatcctcgatgcgctgatcggcaccatgtcaccgctgatcccggcgattatcggcggatcgatggtcaaactgctggcaatgatcctcgagatgagcggcgtgctgacaaaaggatcgccgaccttaaccattctgaatgtgattggtgacggtgctttcttcttcctgccgctgatggtcgcggcatctgccgccatcaaatttaaaaccaatatgtcgctggcgattgccatcgcgggtgtgctggtacatccgagttttattgaactgatggcgaaagcggcccagggtgaacatgtcgaatttgccctgattccggtcaccgcggtgaaatacacctacacggtgatcccggcgctggtgatgacctggtgcctgtcatatatcgaacgctgggtggacagcattacaccggcggtgaccaaaaacttcctcaaaccaatgctgattgtgttgattgccgcaccgctggcaatcctgctgattggcccgattggtatctggatcggtagcgccatttcggcgctggtttacaccattcatggttatctgggctggctttcagtcgccattatgggcgcgctgtggcctctgctggtaatgaccgggatgcaccgcgtctttacgccaaccatcattcagaccattgccgaaaccggcaaagaagggatggtcatgccgtcagagatcggcgctaacctgtcgctgggcggttcatcactggcagtggcgtggaaaacgaaaaacccggaactgcgtcagacggcgctggctgcggcggcatcagccattatggcggggatttccgaaccggcgttatatggcgtggcgatccgcctgaaacgtccgcttatcgccagtcttatcagcggttttatttgcggcgcggttgccggtatggcggggcttgccagccactcaatggcagcgccggggctatttaccagcgtgcagttcttcgatccggcgaatccaatgagcatcgtctgggtgttcgcggtcatggcgctggcggtggtgctgtcgtttatcctcacactgttgctcggctttgaggatattcctgttgaggaagcggctgcccaggcgcgaaagtatcagagcgtacaaccgaccgtcgccaaagaagtaagtcttaattgaggatgaaaatgtcagtatttccagaaagttttttatggggcggcgcgcttgccgccaaccagtctgaaggtgcgttccgtgaaggtgacaaaggtctgaccactgtcgatatgatcccacacggcgagcatcgaatggcggtgaaactggggctggaaaaacgttttcagttgcgagatgacgagttttatcccagccatgaggcgacggatttttatcatcgttataaagaagatatcgccctgatggcagagatgggattcaaggttttccgtacctcaattgcctggagccgtctctttccgcagggcgatgaaatcacgcccaatcagcagggcattgctttttatcgttctgtctttgaagagtgtaaaaagtacggtatcgaaccgctggtcacgttgtgccacttcgatgtgccgatgcatctggtcaccgaatatggctcctggcgtaaccgcaagctggtggagtttttcagccgctacgccagaacctgctttgaagcatttgatggtctggtgaaatactggctaaccttcaatgaaatcaacattatgttgcatagcccgttctccggcgcgggtctggtgtttgaagaaggtgaaaatcaggatcaggtgaaatatcaggccgcgcatcaccagctggttgccagtgcgctagccaccaaaatcgcccatgaggttaacccgcaaaatcaggtgggctgtatgctggcgggcggtaacttctacccttacagttgcaagccggaagatgtctgggcggcgctggagaaagaccgggaaaacctgttttttatcgatgtgcaggcgcggggcacgtatccggcttactctgcccgcgtattccgcgaaaaaggggtaaccatcaacaaagcaccgggcgatgatgaaatcctgaaaaacaccgtcgattttgtctctttcagctattacgcctcgcgctgcgcctcggcggagatgaacgccaacaacagcagtgcggcgaacgtggtgaaatcgctgcgtaatccgtatctacaggtgagcgactggggctggggaattgatccactcggtctgcgtatcaccatgaatatgatgtacgatcgttatcagaagccgctgtttctggtggaaaacggcctgggcgcaaaagatgaatttgctgccaatggcgagattaacgacgactatcgcatcagctacttacgcgaacatatccgcgcaatgggcgaagcgattgcagacggcattccgctgatgggctacaccacatggggctgtattgatttagtttccgcctctacgggtgaaatgagcaaacgctacggctttgtctttgttgaccgtgacgacgcaggcaacggtacgctgacgcgcacgcgtaagaaatcattctggtggtataaaaaagtgattgccagtaatggggaagatttagagtaggtaacagtgccggatgcggcgtgaacgccttatccggcctacatgtcgcacgaaccatgaaggcccgataagcgcagcgcatcgggcaatttagcatttggcatcagagctggttcaccccatcaagaacatccctgtcctgattccttaatgaaaaactactcttcttccaccgctaactgcgcgaagccgccatttccttcccagccttccagtcgttgataaacggtttctaccgcatctttaatcggctgggtcatcgggtagtaaaagccgacgatatccggctgaatgccgaggaaaatcacttcgccaatatcttctttcaactggtcgataaggtaattcaacggcatgttatgggtagtcatcataaacatctcggcgatatcatccgggtcgatgatgcggatctcgccggggtttagccccatatccgtggcgtcgacaatcagcagtcgtgtcgggcgcagttcacggatagcgacgatgtcgttttccggtgcgctaccgccgtcaatcaccacccagttacctttcggcgcggcggcgcacttttccgccagcagcggacctgcgccatcatcgcccatcatgctattgccaacacagagtaaaacgtcagtcacgcagtctcctcaccatcaaatagatggcgttttcctgatgaatatcatgcagcatacttaacagcattgtactccattcctgctgctgcgaagtttgcgctgcccgggctttatcgaatgcgttggccagcatcggcacatggttaatgtcgatgacgatctcaccatatttcggcacgccttccattttgcggcgggcttcactgcctgcctccagagtggcaatccatgccagatattcatcccacgggcaggtgagcgccgcttccaggcaatcgataaccccaaggtggtgaccaatcgccaggctgtaatagaccacctgctgcgcctcggcgggcgtggcatcgttctcatcaataaatttacggctcagttgactgaacaccaccttttcactcatcggatacgcgcctcttcaacaacatgattcagatggctgacaatctcgttcagacgcggatcgttttccgcttccagccagcgtgcaacctgttcttcgccctgccctaactgtgtaaggtaatcatcggcaatctgacgaccgtaacgataacccgccaggcgacgtgcttcgcgatccactttcacgcgcagcggctgcaccatatcaccatgcaggatctccgccggttgttcatccagttcacccggcccacgggcgtgaattttctgctccagcaggccgagcgccattgcaaagccgtacagcgtggcggcaggcgttggcgggcagccagggatataaacatccacagggacaattttatccgtaccgccccacacgcagtagagatcgtggaagatcccgccactgttaccgcaggcaccgtaggagatacaaattttcgggtccggcgcggactgccacgcacgcagcgcaggggatcgcattgcacgggtgaccgcgccggtaaacagtaaaatatccgcatgacgcggtgaaggaacgactttaatgccgaagcgttctgcatcaaacagcggcgaaagcgtggcgaaaatttcgatttcgcaaccgttgcagccgccgcagtccacgcggtaaacataggcagaacgtttgatttttttcagtaacgacgccttcatgctggcgatggattcatccaccgtcatggggaccggaatgccgttggcgtcacgggggcctaataaattgctcatcagatggcctctttcatatggcgagtcagttcaatacggtcggacggcaccaggcatttctggcgcttacattccgggcaagtctcaaagctttcgcggtggttttccgcgcggctgtcgccgttgtgcttaagcagcgcaatggcgtagtcgatctctttctggacggcgaaaggacgattgcagacgcggcagttgcacagcgcgaagcgggactgttgcaggaagtcttctttcttccacaccgccagttcgtactcttgcgacagtttgatcgccgccgtcgggcagacttcttcgcagcgtccacagaagatgcagtgcccaagattaaactcccaggcaagctctcctgtggcgaggtcagtttcaaccgttaaggcgtttgacgggcaggcattgacgcaggccgcgcagccgatgcactgctgcgggttctgctctggcttaccacggaagtttttatcaaccgcaatcggctccagcggataagacgaggtcgccgtgccggttttgatgacttttttgataaaggtaaacatggcgattccttatttcagcggcgagtttttacgctcaatgctgtaacgctcgagttctttgtacggcaccactttgctcttcttcttacgcacatcgaccacggtcatgcggtcggtacaggagtagcaagggtcgaggctaccgataatcagcggcgcatcggaaacggtgttgccgcgcagcatgtagcgcagggtcggccagttcgcgtaggtcgcggcacggcagcgccagcggtacagcttctggttgtcgccggtcatgctccagtggatatcatcgccgcgcggcgcttcggcaaagcccagcgcaaagcggtgcggaatgtaggtaaagccttccaccatcagtgggccacccggcaggttatccagaccgtagtcgatcatgttcagcgcggtatagacttcgttgatacgcactttcagacgggaaataacgtcgcagccctgctcgctgtggacttccattggcagcaggccatagccgacaaacgggtgatcggcgcgggtatcacgggcgtgaccgctggcacggaccatcgggccgacgttactgaagtcgcgagcgatttccgggtccagacgaccaatgccgacagtgcgctgttccatgttcggagtgctcagcagcacatccaccagctcctgcacttcacgacgcatctgttgtgccagctggcgggtctggatcatgtcgtctttcagcagatcgcgacgaatcccgccgatcaagttcaggccgtaggttttacgcgcaccggtaaggatctctgccattttcatggaggtttcacgcacgcggaagaactgcataaagccggagtcgaagccggtaaagtgacaggccaggccaaggttgagcagatgcgagtgcaagcgttctacctccagcagaatggcgcggatcatctgcgcacgttctggcacctgaatacccatcgcgttttccaccgacgtggtgtaggcggtgctgtgggcaaagccgcagatcccgcacacacggtcagagaggaaggtcacttcgttataacccatacgggtttccgccagtttttccatgccgcgatggacgtagaacagacggtagtcggcgtcgataatgttttcgccatcgacgaacagacggaagtggcccggttcatcagaagtgacgtgcagcggaccaatcggcacgacgttgtttttcttgtcgcccagttcgttgatgaactcgtaggtttcagcatcggtggtcggtgccggacgctgacgataatccatgctgtctttacgcagcggataaagttcatccggccagtcatccggcagcaccagacgacgttcatccggcagaccaaccggaatcaaaccgtacatatcgcgcacttcacgctcgccccacaccgccgccggaacgcgcggcgtcacggacggatattccggtttgttggcgtcaacttcgacgcgaaccgtaatccaacacttagtgcccttctccatcgacagcacgtagtaaacggcgtaatgaccattcagtttgcgttcgtcgttaccaaacagcaccgacagccagccaccctgtttgtagtaaagaaactccaccacttccggcaggtagttcacctttacggtgacagtcagctgatctttggtctgccaggcgtggtccagcacgacgcccggaaatgcctcattcagcgcggcgagataatgttgacctaatttttcttcagacatgctcaaactctctttaatcacgccgccagcaaggagacgaacgctaaaaatgcaaagccaaacccagcccaggtaatgcgcggagtaatatcaagacgcagacgggccatgctgttttcgaacagcgcgataaccaggacgccgaccaccagttttacgatggcaatcaccagcgccagcagcagtccaccggcggtgaaggtttccatttgtccccacggaataaacaccccgacgaacatctgcaacaccaccagctgtttcaggctgataccccatttcatgacgccaaagccgctgccgctgtattcagagagcgggccttcctgcagctcctgctcggcttccgccaggtcgaacggcagtttgcccatttcgataaaggtggcgaacgcacaggcacaaagcgccagtaccagcgggatgctctggctcagcggccagtgataaacggtgtcggtgatgttgctgatgttggtggaaccggcaacctgtgcggcaacccacagaccaagcagcagcatcggttcgaccagcacgccaagcatcgcttcacggctcgcgccgatagcggtaaacgggctaccggtatccagaccagaaatggcaaagaagaaacgcgcgatggcaaagagatacagtaaggtgatcaaatcacccagttgcggcagcggagaaccgacggtcaccaccggcagcgcagtagcgatagtcagcatgacgcccaccatcacatacggcgtcaggcggaacacccagccggaggcatccgggccgacgctctgacgccccagcagtttgataatgtcgcgatactcctgcaacacgcccggcccgcgacggttatgcaagcgggcgcgcgccacgcgggttataccggagagcagcggcgcaacggcaaataacaccagcgcctgaattaacggatataaaacactcattctcaggctcctcgtgaaacaataatcaccaccagtaccgccagttcaaccagcgccatccggcggaacagcaacgcactcccctcgcactgccagcccggcaccagagacaccggattcagccatttgcgtagtttcagcaccggcgcaaacgcctgtttcaccggcatggcaaaaccgtgagcggtaatcaccattgatttttcgtggtcgtaaccgcacacccaggccgcaccgcgggaacgcgatggcaaacgatcgcctttgcaaatcgccataatgatgaatggcagcagcgggcaggcaatcagcagcaacgtgatcatcggttgagaaacggtggtgttagcaggctccagcggcagaggtacagcagcagagagcatcggcagtagccacggcgcagcaacaccgccaattacgcagcaaatcgccagtgccactacgcttacgctcatcaggagcggcgcacaggtggcgttttcggcttctttggtgcgcggcgcgccgaggaacgtgacgccatagactttcgccatacacatcaccgccagcgcaccggtaattgccagccccacagcgagcagcggccccagcagacgggcaacaaacgcgccactattgctcagtttgaaaaatgattgatagataacccattccccggcaaaaccattcagcggcggcagcgcagccattgccatcagcccgactaacatggcgatggagataaccggcattttcttgccaataccaccgagtttttcgatatcgcgatgaccggtacggaaccagacgctccccgccccgaggaacagtacgcttttgaacaggctatggttaagcagatggtacagaccaccgaccaggccaagagcaatcagcgccggttgttcgagcgcgatacccgttacgccagcgcccagccccagcaggatgatgccgatattttccagggtgtggtaagccagcaggcgctggatgttgtgctccaccagcgcatacagaccaccgacaaacgcggtgatcatgccgagcaccagcagcgcgatcccccaccacagcggtgcattaccgcccagcagtgacagggttaaaatgcccagcaggccaattttcatgactaccgtagaaaacaacgcggcagctggcgcagaggcgttcgcatgtgcctgcggcacccagccgtgcagcggaataatcccggccagcaggccaaagccaatcactccgagcagccagatatcggaaccgagcggcagctgttgcatacgcatatccagcaggcgcagatccagcgtgccgtaacgctgccacagcagccagcaagcaatcgccagcagcagagtgccaagacgccccagcgcaaaccacagtttgccctctttgctgttgctggtgaggaacaccgcgcacagggccatgatttcggccattaccacgaacatgccgaggttgctggcaatgacggcgcagacggcggcagccatcaacatattgatctgcaagccgttgcacttcacctgcgcgtggcgatgccagtcaatgttgtagaggctgacaaacagaccgcacagaccgagcgtaatcagccaaatcgcgttaagcggagagatttgcacatcgtagcttaccagcgacagcgcaccgctcacgccaaccgcgccagtcagtacagtgaagcccgcggctgccgtatacagactaccaaccgcgccgccaattccagctatccagccacttaacgctttttgaaaagaaaagagaaatgccagaacagcggcggcgacaaaccacgccacgccgctattgatcagggaaattgcgctcatttagcctctccactttgagcctgctgaaacaaggtgagatcgccaaagtccgtgttaaaggtcagctcacgcttacgtttgctgacgcgggcgatatcggtgttatccaccagatgcagggctttagtcgggcacatccgcacgcaggccggaccttgttcatcaaagctacaaaggtcacatttgacggcgatcgcgcgaatacctggcacccagtcaagcaatgtgctgacacgcgccggagcaggcggtgccggtggcgctttcggggtattggcgtttgccggaatatccagcggacggctgccggaaaattcaattgcgccaaacgggcaggcgatgccgcacagcttgcagcttacgcacaggctttcattcaactgcacggccccatcgacgcgggtgatggcgttaaccgggcagaccaccgcgcagggtgcatcttcacagtggtgacagagctgcggcgcagattctttttcattcagcatcactctcaggcgcggcattgattgcaggccgtgctggcgatgcgtctctgaacaggcggcctcacaagtgtggcagccgatacagagcgtggagtcagcaattacaaaacgattcaccaggcattcctcaggtgattgtcatttttgacgaaaacatgccgatgaaatgtcattttcgacactcatcgacacgcccatccccaaacaggcgtaacgcctgcaaaacgggcaaagcctcagctcatgctgccgggctttgtccctttaccagttggcttaaattcaccggcacattgttttcaatagcggtgtataagctgtcgtaaacgccagcgattttttcgagatagtgttccagaacctgttcgcgatcgcggatgttgaccttgccatcaatcatgccgtcaatgctcagttgcgcctgcgcaatccgctgtttgtcttcgccatcttttgtttcgacgtaatactcgatggtgtggctgttaaagccatccgccagggtgacgtaaatgcgaaaatgttcaaaaaggacgaaacagagttctttgtccggcgcgcagctcatggcgtgatgcaggcgcgctttcgataacgtgatcccctgaaccagcgaattgcagtagatgtgccactggtcctgtaggcgacgatgccgctgtgcgatgtaatcggctttctcgcttatttcccaaatagtcattgtcaggttacccgtttaacagagatgccagctttaagcattttttgtgccaacttttaatttattgttattaaagagatttttaagctaaagatgaatttcgtcgccgtgtcgacgtgtcatttcgacatcatcgacattattcaccgcagggataatcaacactggcacaattattgcttgtagctggcaatagttaatgggaggcgatatgcacgaaataaccctctgccaacgggcactggaattgatcgaacagcaggccgcaaaacacggcgcaaaacgcgtaactggggtctggctcaaaattggcgcattttcttgtgtcgaaaccagctctcttgccttttgttttgatctggtttgccgcggcagcgtggcggaaggttgtaaactgcacctcgaagaacaagaggccgaatgctggtgtgaaacatgccaacagtatgtgacgctactgacccagcgcgtccgccgctgtccacagtgtcatggtgacatgctgcagattgtggcagacgacggtttacagattcggcggatagaaatagaccaggagtgagcgatgtgtacaacatgcggttgcggtgaaggcaacctgtatatcgagggtgatgaacataaccctcattccgcgtttcgtagcgcgccatttgccccggcggcacgcccgaagatgaaaatcaccggcattaaagcgcctgaatttacccccagccagactgaagaaggcgacctgcattacggtcatggcgaagcgggcactcacgcaccgggcatgagccagcgtcggatgctggaagtcgaaattgacgtgctggacaaaaataaccgtctggctgaacgcaaccgcgcgcgctttgctgcccgcaagcaactggtgctcaacctggtttccagccctggttccggtaaaaccaccctgctgacggaaaccctaatgcgcctgaaagacagcgttccgtgcgcagttattgaaggcgaccagcaaaccgtgaacgatgccgcacgcattcgcgctaccggcacaccagcgattcaggtgaacaccggtaaaggctgccatcttgacgcacagatgattgccgacgccgcaccgcgtctgccactggacgataacggtattctgtttatcgaaaacgttggcaacctcgtatgcccggccagcttcgatctcggtgaaaaacacaaagtggcggtgctttccgttaccgaaggtgaagacaaaccactgaaatatccgcatatgtttgccgccgcctcgctgatgctgctcaacaaagttgacctgttgccgtatctcaactttgacgttgaaaagtgcatcgcctgcgcccgcgaagtcaatccagaaattgaaatcatccttatttccgccaccagcggcgaagggatggaccagtggctgaactggctggagacacagcgatgtgcataggcgttcccggccagatccgcaccattgacggcaaccaggcgaaagtcgacgtctgcggcattcagcgcgatgtcgatttaacgttagtcggcagctgcgatgaaaacggtcagccgcgcgtgggccagtgggtactggtacacgttggctttgccatgagcgtaattaatgaagccgaagcacgcgacactctcgacgccttacaaaacatgtttgacgttgagccggatgtcggcgcgctgttgtatggcgaggaaaaataatgcgttttgttgatgaatatcgcgcgccggaacaggtgatgcagttaattgagcatctgcgcgaacgtgcttcacatctctcttacaccgccgaacgccctctgcggattatggaagtgtgtggcggtcatacccacgctatctttaaattcggcctcgaccagttactgccggaaaacgttgagtttatccacggtccggggtgcccggtgtgcgtactgccgatgggtagaatcgacacctgcgtggagattgccagccatccggaagtcatcttctgtacctttggcgacgccatgcgcgtgccggggaaacagggatcgctgttgcaggcaaaagcacgcggtgccgatgtgcgcatcgtttactcgccgatggatgcgttgaaactggcgcaggagaatccaacccgcaaagtggtgttcttcggcttaggttttgaaaccactatgccgaccaccgctatcactctgcaacaggcgaaagcgcgtgatgtgcagaatttttacttcttctgccagcacattacgcttatcccgacgttgcgcagtttgctggaacagccggataacggtatcgatgcgttcctcgcgccgggtcacgtcagtatggttatcggcaccgacgcctataattttatcgccagcgattttcatcgtccgctggtggttgctggattcgaaccccttgatctactacaaggcgtggtcatgctggtgcagcagaaaatagcggcccacagcaaggtagagaatcagtatcgtcgagtggtaccggatgccggtaacctgctggcgcaacaggcgattgccgatgtgttctgtgtcaacggcgacagcgaatggcgcggcttaggcgtgattgaatcttctggcgtgcacctgacgccggattatcaacgattcgatgccgaagcacatttccgcccggcaccgcagcaggtctgcgatgacccgcgcgcgcgttgtggtgaggtattaacgggcaaatgtaagccgcatcaatgcccgctgtttggtaacacctgtaatcctcaaaccgcgtttggtgcgctgatggtttcctccgaaggagcgtgcgccgcgtggtatcagtatcgtcagcaggagagtgaagcgtgaataatatccaactcgcccacggtagcggcggccaggcgatgcagcaattaatcaacagcctgtttatggaagcctttgccaacccgtggctggcagagcaggaagatcaggcacgtcttgatctggcgcagctggtagcggaaggcgaccgtctggcgttctccaccgacagttacgttattgacccgctgttcttccctggcggtaatatcggcaagctggcgatttgcggcacagccaatgacgttgcggtcagtggcgctattccgcgctatctctcctgtggctttatcctcgaagaaggattgccgatggagacactgaaagccgtagtgaccagcatggcagaaaccgcccgcgcggcaggcattgccatcgttactggcgatactaaagtggtgcagcgcggcgcggtagataaactgtttatcaacaccgctggcatgggcgcaattccggcgaatattcactggggcgcacagacgctaaccgcaggcgatgtattgctggtgagcggtacactcggcgaccacggggcgactatccttaacctgcgtgagcagctggggctggatggcgaactggtcagcgactgcgcggtgctgacgccgcttattcagacgctgcgtgacattcccggcgtgaaagcgctgcgtgatgccacccgtggtggtgtaaacgcggtggttcatgagttcgcggcagcctgcggttgtggtattgaactttcagaagcggcactgcctgttaaacctgccgtgcgtggcgtttgcgaattgctgggactggacgccctgaactttgccaacgaaggcaaactagtaatagctgttgaacgcaacgcggcagagcaagtgctggcagcgttacattcccatccactggggaaagacgcggcgctgattggtgaagtggtggaacgtaaaggtgttcgtcttgccggtctgtatggcgtgaaacgaaccctcgatttaccacacgccgaaccgcttccgcgtatatgctaataaaattctaaatctcctatagttagtcaatgaccttttgcaccgctttgcggtgctttcctggaagaacaaaatgtcatatacaccgatgagtgatctcggacaacaagggttgttcgacatcactcggacactattgcagcagcccgatctggcctcgctgtgtgaggctctttcgcaactggtaaagcgttctgcgctcgccgacaacgcggctattgtgttgtggcaagcgcagactcaacgtgcgtcttattacgcgtcgcgtgaaaaagacacccccattaaatatgaagacgaaactgttctggcacacggtccggtacgcagcattttgtcgcgccctgatacgctgcattgcagttacgaagaattttgtgaaacctggccgcagctggacgcaggtgggctatacccaaaatttggtcactattgcctgatgccactggcggcggaagggcatatttttggtggctgtgaatttattcgttatgacgatcgcccctggagcgaaaaagagttcaatcgtctgcaaacatttacgcagatcgtttctgtcgtcaccgaacaaatccagagccgcgtcgttaacaatgtcgactatgagttgttatgccgggaacgcgataacttccgcatcctggtcgccatcaccaacgcggtgctttcccgcctggatatggacgaactggtcagcgaagtcgccaaagaaatccattactatttcgacattgacgatatcagtatcgtcttacgcagccaccgtaaaaacaaactcaacatctactccactcactatcttgataaacagcatcccgcccacgaacagagcgaagtcgatgaagccggaaccctcaccgaacgcgtgttcaaaagtaaagagatgctgctgatcaatctccacgagcgggacgatttagccccctatgaacgcatgttgttcgacacctggggcaaccagattcaaaccttgtgcctgttaccgctgatgtctggcgacaccatgctgggcgtgctgaaactggcgcaatgcgaagagaaagtgtttaccactaccaatctgaatttactgcgccagattgccgaacgtgtggcaatcgctgtcgataacgccctcgcctatcaggaaatccatcgtctgaaagaacggctggttgatgaaaacctcgccctgaccgagcagctcaacaatgttgatagtgaatttggcgagattattggccgcagcgaagccatgtacagcgtgcttaaacaagttgaaatggtggcgcaaagtgacagtaccgtgctgatcctcggtgaaactggcacgggtaaagagctgattgcccgtgcgatccataatctcagtgggcgtaataatcgccgcatggtcaaaatgaactgcgcggcgatgcctgccggattgctggaaagcgatctgtttggtcatgagcgtggggcttttaccggtgccagcgcccagcgtatcggtcgttttgaactggcggataaaagctccctgttcctcgacgaagtgggcgatatgccactggagttacagccgaagttgctgcgtgtattgcaggaacaggagtttgaacgtctcggcagcaacaaaatcattcagacggacgtgcgtctaatcgccgcgactaaccgcgatctgaaaaaaatggtcgccgaccgtgagttccgtagcgatctctattaccgcctgaacgtattcccgattcacctgccgccactacgcgagcgtccggaagatattccgctgctggcgaaagcctttaccttcaaaattgcccgtcgtctggggcgcaatatcgacagcattcctgccgagacgctgcgcaccttgagcaacatggagtggccgggtaacgtacgcgaactggaaaacgtcattgagcgcgcggtattgctaacacgcggtaacgtgctgcagctgtcattgccagatattgttttaccggaacctgaaacgccgcctgccgcaacggttgtcgccctggagggcgaagatgaatatcagttgattgtgcgcgtgctgaaagaaaccaacggcgtggttgccgggcctaaaggcgctgcgcaacgtctggggctgaaacgcacgaccctgctgtcacggatgaagcggctgggaattgataaatcggcattgatttaactgcaaattgccggacagatctgcctgtccggcatactattcatgaggttttttcggacgatatttttccggcagttctggcaccggacgcttgtcatcgatgagatgacgcacggttaagatcggatgacgccacagcattctcggcccggcccaacgcataatctgtttcatctcttcacgctttgcaggctggtaacagtgcaccggacactgcttacaggctggtttctcttcgccgaacacacatttatccagccgcttttgcgcgtaaacaaacaacgcctcgtaatgctccggctccgctgacgcctgcgggcatttcgcttgataaagatcgatcatttttttaatcgtcagtttttcacgagagatacgcttgccggacatgctgcctccacctcattaagatgtatttatattacatcttaatcttaaagggcactatgactccaaagaagaagggttagccaaccgatacaattttgcgtacttgcttcataagcatcacgcaaaagctgcaaaacagcatctttcccggaaccagcatcaagaactcgccgttcgcttcttcccctgaaatgattaactccggtatcatgtgcgccttatgtgattacaacgaaaataaaaaccatcacaccccatttaatatcagggaaccggacataaccccatgagtgcaatagaaaatttcgacgcccatacgcccatgatgcagcagtatctcaggctgaaagcccagcatcccgagatcctgctgttttaccggatgggtgatttttatgaactgttttatgacgacgcaaaacgcgcgtcgcaactgctggatatttcactgaccaaacgcggtgcttcggcgggagagccgatcccgatggcggggattccctaccatgcggtggaaaactatctcgccaaactggtgaatcagggagagtccgttgccatctgcgaacaaattggcgatccggcgaccagcaaaggtccggttgagcgcaaagttgtgcgtatcgttacgccaggcaccatcagcgatgaagccctgttgcaggagcgtcaggacaacctgctggcggctatctggcaggacagcaaaggtttcggctacgcgacgctggatatcagttccgggcgttttcgcctgagcgaaccggctgaccgcgaaacgatggcggcagaactgcaacgcactaatcctgcggaactgctgtatgcagaagattttgctgaaatgtcgttaattgaaggccgtcgcggcctgcgccgtcgcccgctgtgggagtttgaaatcgacaccgcgcgccagcagttgaatctgcaatttgggacccgcgatctggtcggttttggcgtcgagaacgcgccgcgcggactttgtgctgccggttgtctgttgcagtatgcgaaagatacccaacgtacgactctgccgcatattcgttccatcaccatggaacgtgagcaggacagcatcattatggatgccgcgacgcgtcgtaatctggaaatcacccagaacctggcgggtggtgcggaaaatacgctggcttctgtgctcgactgcaccgtcacgccgatgggcagccgtatgctgaaacgctggctgcatatgccagtgcgcgatacccgcgtgttgcttgagcgccagcaaactattggcgcattgcaggatttcaccgccgggctacagccggtactgcgtcaggtcggcgacctggaacgtattctggcacgtctggctttacgaactgctcgcccacgcgatctggcccgtatgcgccacgctttccagcaactgccggagctgcgtgcgcagttagaaactgtcgatagtgcaccggtacaggcgctacgtgagaagatgggcgagtttgccgagctgcgcgatctgctggagcgagcaatcatcgacacaccgccggtgctggtacgcgacggtggtgttatcgcatcgggctataacgaagagctggatgagtggcgcgcgctggctgacggcgcgaccgattatctggagcgtctggaagtccgcgagcgtgaacgtaccggcctggacacgctgaaagttggctttaatgcggtgcacggctactacattcaaatcagccgtgggcaaagccatctggcacccatcaactacatgcgtcgccagacgctgaaaaacgccgagcgctacatcattccagagctaaaagagtacgaagataaagttctcacctcaaaaggcaaagcactggcactggaaaaacagctttatgaagagctgttcgacctgctgttgccgcatctggaagcgttgcaacagagcgcgagcgcgctggcggaactcgacgtgctggttaacctggcggaacgggcctataccctgaactacacctgcccgaccttcattgataaaccgggcattcgcattaccgaaggtcgccatccggtagttgaacaagtactgaatgagccatttatcgccaacccgctgaatctgtcgccgcagcgccgcatgttgatcatcaccggtccgaacatgggcggtaaaagtacctatatgcgccagaccgcactgattgcgctgatggcctacatcggcagctatgtaccggcacaaaaagtcgagattggacctatcgatcgcatctttacccgcgtaggcgcggcagatgacctggcgtccgggcgctcaacctttatggtggagatgactgaaaccgccaatattttacataacgccaccgaatacagtctggtgttaatggatgagatcgggcgtggaacgtccacctacgatggtctgtcgctggcgtgggcgtgcgcggaaaatctggcgaataagattaaggcattgacgttatttgctacccactatttcgagctgacccagttaccggagaaaatggaaggcgtcgctaacgtgcatctcgatgcactggagcacggcgacaccattgcctttatgcacagcgtgcaggatggcgcggcgagcaaaagctacggcctggcggttgcagctctggcaggcgtgccaaaagaggttattaagcgcgcacggcaaaagctgcgtgagctggaaagcatttcgccgaacgccgccgctacgcaagtggatggtacgcaaatgtctttgctgtcagtaccagaagaaacttcgcctgcggtcgaagctctggaaaatcttgatccggattcactcaccccgcgtcaggcgctggagtggatttatcgcttgaagagcctggtgtaataacaattcccgatagtcttttgctatcgggaatattaacgacaactgacgaataaaataaaaacaccctgtataataggaaagcttattttacagggtaaaaccatgccatctacacgctatcaaaaaatcaatgcccatcactatcgccatatatgggtcgttggtgatattcatggtgaatatcagttattacaatcccgcttacatcaactctcttttttccccaaaatcgacttacttatttctgtcggcgataatattgatcgtggaccggagagtcttgacgtcctgcgcctgctaaaccaaccctggtttacgtcggttaaaggcaaccacgaagcgatggcgcttgaggcattcgaaactggcgatggcaatatgtggcttgccagcggtggtgactggtttttcgatttaaatgattcagagcaacaagaggcaatagatctgttgctgaaattccatcaccttccacatattattgaaatcactaacgacaacataaaatatgccatcgcacatgcagattatccggggagtgaatatctctttggtaaagaaatagcggagagcgaattactctggcctgttgatcgtgtgcagaaatcgcttaatggcgagttacaacaaataaacggcgctgattattttatatttggacatatgatgtttgataacattcagacgttcgctaaccagatttatattgataccggatcgccgaacagcgggcggctgtcattttataaaataaagtagtctcatgcttcttctgtgaagcatgagtaacccggtgttattgcaggccattattcatttttcgctaccagcaaagagagatcctgcttcaccagcgcgcgactggcactctccggcaaaccgtcgtctgtaataatctgatcaaactcgcttaatggtaacgccagccatgtcgccacctgaccatatttcgtcgcatcacagaccaaaactcgctggcggctggcactggcaatcgcccgtttcaccgtgactttatcttccgctggcgtagaaatcccccgcacactccatgacgatgcagaaataaaagcctgatcaatcatcaggctgcgcagcatggtcgcagcggcttccccgacacaggaacggttttcccgacacactgcaccgccagtgtgaataattgtgcaattactgttgtcgagcaagtagtccgcaataacgaaatcgtttgtgaccacagtcagtgactccatgtgaatcagatgctgtgctatcgctaacgtggtcgttcccgcatccagatagatacaacttcccggctgaacaagacttgccgccagcttgccaatagccgctttttgcgtcattgccagcgcagtttttacctgatgagaaggttcatgcgccacgcgtcccggagactggacgcctccggacaccagcacaacggctccctgctgctccagtttttgtaaatcccgacgaatggtcatatgtgacacattcattctgtccgttagttcagcaatactgacaatgcctttttcagctaccatctcaaggatgatttggcgacgctctacgggtatcaacttttgctccttcctttgtcctgctgacattctacgctatttgcctgcgaaacgtgcgcggcgcaactaacgcttagttcacataaaataacacacaatgttaatttatgtgaatcagatcaccataccgttatcttccagcgcttatattcacaatatcaaacaaaatatcacttaaattaacaaggagagcagatgaaaacgggatctgagtttcatgtcggtatcgttggcttagggtcaatgggaatgggagcagcactgtcatatgtccgcgcaggtctttctacctggggcgcagacctgaacagcaatgcctgcgctacgttgaaagaggcaggtgcttgcggggtttctgataacgccgcgacgtttgccgaaaaactggacgcactgctggtgctggtggtcaatgcggcccaggttaaacaggtgctgtttggtgaaacaggcgttgcacaacatctgaaacccggtacggcagtaatggtttcttccactatcgctagtgctgatgcgcaagaaattgctaccgctctggctggattcgatctggaaatgctggatgcgccagtttctggtggtgcagtaaaagccgctaacggtgaaatgactgtcatggcctccggtagcgatattgcctttgaacgactggcacccgtgctggaagccgttgccggaaaagtttatcgcataggtgcagaaccgggactaggttcgaccgtaaaaattattcaccagttgttagcgggcgtacatattgctgccggagccgaagcgatggcacttgcagcccgtgcggggatcccgctggatgtgatgtatgacgtcgtgaccaatgccgccggaaattcctggatgttcgaaaaccggatgcgtcatgtggtggatggcgattacaccccgcattcagccgtcgatatttttgttaaggatcttggtctggttgccgatacagccaaagccctgcacttcccgctgccattggcctcaacagcattgaatatgttcaccagcgccagtaacgcgggttacgggaaagaagacgatagcgcagttatcaagattttctctggcatcactctaccgggagcgaaatcatgatcaagattggcgttatcgccgatgattttaccggcgcgacggatatcgccagttttctggtggaaaacggtctaccaacggtacaaattaacggtgttccaacaggtaaaatgccggaagcaatcgacgcactggtgatcagcctgaaaacgcgctcctgtccagtggttgaagccacacagcaatcgctggcggctctgagctggttgcaacagcaaggttgcaaacagatctatttcaaatactgctctactttcgacagtacggcgaaaggtaatattggcccggttaccgatgccttaatggatgctctcgacacgccgtttacggtcttctctccggccctgccggtcaacggacgtacggtttatcaggggtatttgttcgtaatgaatcaactgctggccgaatccgggatgcgccatcacccggtaaatcccatgaccgacagctatcttccccgtctggttgaagcgcaatccacagggcgctgcggcgtcgtttcggcacatgttttcgaacaaggtgtggatgccgttcgtcaagagctggctcgcttacagcaagagggctaccgctacgcggtgcttgatgcgctgaccgaacaccatctggaaattcagggagaagccttgcgcgatgccccactggtaacgggcggttctggtctggcgattggcctggcccggcagtgggcgcaagaaaacggtaaccaggctcgcaaagcagggcgtccgctcgctgggcgcggcgtagtgctctccggttcatgctctcaaatgaccaaccgccaggtagcacattaccgtcaaattgcaccagcccgtgaagttgatgtggcacgctgcctctcaattgaaactctggccgcttatgcacacgaactggcagagtgggttctgggccaggaaagtgtacttgctccactggtttttgccaccgccagcactgacgcattggcagcaattcaacagcaatacggtgcacaaaaagccagtcaggcagtagaaacactgttttctcaactagcggcgcggttagcagcggaaggcgtgacacgctttattgtcgcaggcggtgagacctccggcgtagtcacacagagcctgggaataaaagggtttcatattggcccaaccatttccccggcgtgccgtgggtaaacgcactggataagcctgtctcactcgcccttaaatctggcaacttcggtgatgacgcctttttttcacgagcccaaagagagtttttatcatgagcgatttcgcaaaagtagagcagtctttgcgagaggagatgacgcggattgccagttcattctttcagcgcggctatgcaaccggttcggctggcaatctgtcgctgcttttacctgacgggaatttactggcgacaccgacaggttcatgcctgggcaatctcgatccgcagcggctttccaaagtcgccgcggatggcgaatggttaagtggtgacaaaccctcgaaagaggtgctctttcatctggcgctgtatcgcaacaatccgcgctgtaaagcggtggtgcatttgcacagcacatggtcgacggcgctttcctgcctgcaagggctggacagcagcaacgttattcgtccgttcacaccatacgtggtgatgcggatgggaaatgtcccgctggtgccttattaccgaccgggcgataaacgcatcgcacaggatctggcggaactggcagcagacaatcaggcttttttactggcaaatcatggcccagtggtttgcggtgaaagcctgcaagaagccgccaacaatatggaagagctggaggaaacggcaaagctgatttttattctcggtgaccgcccgatccgttatctgaccgcaggtgaaattgcggaattaaggagttaatgcaatgcctcgttttgcagctaatttatccatgatgttcaccgaagtgccttttattgaacgcttcgccgcagcgcgaaaagccgggttcgatgctgtggaatttctgtttccctataactactccaccctgcaaatccaaaagcaactggagcaaaaccatctgacactggcgctgttcaataccgctcccggagatattaatgcgggggaatggggattatccgcccttcccggacgtgagcacgaagcacacgcagacatcgacctggcactggaatatgcattggcgctcaattgtgaacaagtccatgtgatggcaggcgtcgtgcccgctggcgaagatgctgaacggtaccgggcagtatttatcgataatatccgctacgctgccgaccgctttgcgccacacggcaagcgaatattagttgaagcactcagccccggcgttaagcctcattatctcttctccagccagtatcaggcactggctattgttgaagaggttgcgcgagataacgtgtttattcaactagatacttttcatgcgcaaaaagtagatggcaacctgacgcatttaatccgcgactacgccgggaaatatgcgcacgtacaaattgccggactacctgatcgacatgaaccggacgatggagaaatcaactatccgtggctgttccgcctgttcgatgaggtgggatatcagggctggatcggttgtgaatataaacctcgtggcctcaccgaagaagggcttggctggtttgacgcctggcgctaattcgttaaatccctaattacaacgtacccatacatccccccatctacggatggggtaggttaactataactttcagacagggtttcccatgtccacaattacattgttatgcattgcgttagctggcgtaatcatgctgttgctgctggtcatcaaggcaaaggtacaaccattcgttgctttgctcctcgtcagcctgttagtcgcacttgcggcaggtataccggcgggcgaagtgggtaaagtgatgatcgccgggatgggcggtgtgcttggttccgtcactattattattggtctgggcgctatgctggggcgtatgatcgaacactctggtggtgcagagtcactggctaattatttcagtcgcaagttaggtgacaaacgaactatcgctgcgctgactctggcagcgttcttcctcggtattcccgtcttctttgatgtcggctttattattcttgcgccaatcatttacggttttgccaaggttgccaaaatatcgccactcaaatttggcctgcctgtcgctgggatcatgctcactgttcacgtggcggtaccgccgcatccaggccctgtcgccgcagcggggttactccacgcagacatcggctggctaaccatcatcggtattgcgatttctattcccgtaggggttgttggctactttgcagcgaaaataatcaataagcgccaatatgcgatgtcagtagaagtactggaacagatgcaactggctccggccagtgaggaaggcgcgacaaaattaagcgataaaataaatccaccgggcgtcgcgctggtcacctcgctaattgttattcctatcgcgattatcatggcgggtacggtttccgcaacactgatgccgccttcgcatcccctgcttggtacgctacagctgatcggctcaccaatggtagctctaatgattgcgctggtgctggcattctggttattggctttacgtcgcggctggagcttacaacacaccagcgacattatgggctcagcgcttcctactgcggcggtagtgattttggttactggtgctggaggggtatttggcaaagtgctggtggaatcgggcgtcggcaaagcccttgccaacatgctacaaatgattgacctgcctctgttaccagccgcatttattatttcactggcgctgcgtgcatcgcaggggtcagcaaccgtagcaatactgacaaccggcgggttactctcagaagcggtgatgggattgaatccgattcagtgcgtattggtgacgctggcagcctgctttggtgggcttggtgcgtcacatattaatgactcagggttctggattgtgaccaaatatctggggttgtcggtagcagacggtctgaaaacctggacagtgttaacgaccattctcggttttaccggattcttaattacctggtgcgtatgggcggtaatttgaccttaataaaaaggtccgatgggcatcggaccttttattgtgcacagaaaaggccagcctcgcttgagactggcctttctgacagatgcttacttactcgcggaacagcgcttcgatattcagcccctgcgtttgcaggatttcgcgcaaacggcgcaggccttcaacctgaatctggcgaacacgttcacgggtgaggccaatttcacgacctacatcttccagtgttgccgcttcgtaccccagcaaaccgaatcgacgtgccagcacttcacgctgtttggcgttcagctcgaacagccatttgacgatgctctgcttcatatcgtcatcttgcgtggtatcttccggaccgttctctttttcatcggccaggatgtccagcaacgctttttcggaatcaccacccagcggggtgtctaccgaggtaatgcgctcgttaagacgaagcatacggctgacgtcatcaactggcttatccagttgctctgcgatctcttccgcacttggttcatggtccagcttatgggacaactcacgtgcggttcgcaggtaaacgttcagctcctttacgatgtgaatcggcaaacgaatagtacgggtttggttcataatcgcccgttcaatcgtctggcgaatccaccaggttgcgtatgttgagaagcggaaaccacgttccgggtcaaacttctctaccgcgcggatcagccccaggttgccctcttcgataaggtccagcaacgccagaccacgattgccataacggcgggcaatttttaccaccagacgcaagttactctcgatcatccggcggcgagaggcgacatctccacgcagtgcgcgacgcgcaaaataaacttcttcttcggccgttaacagtggtgaataaccaatctcaccaaggtaaagctgagtcgcgtccaacacacgctgtgtggctccctgcgataacagttcctcttcggccaaatcgttatcactgggttcctgttctactaaggccttttcgtcaaaaacctcaactccgttctcatcaaattccgcatcttcatttaaatcatgaactttcagcgtattctgactcataaggtggctcctacccgtgatcccttgacggaacattcaagcaaaagcctggttccgccgatttatcgctgcggcaaataacgcagcgggtttacggatttccccttgtaacgaatttcaaaatgcaagcgtgttgaactggttccggtgctacccatggtcgctattttttgccccgccttaacttcttgttgttcccggaccagcattgtgtcgttatgggcgtaggcactcaggtaatcatcattatgtttgatgataatcagattaccgtagccgcgcagcgcgttaccagcataaacaacgcggccatctgcggtcgcgataattgcctgtcctttgctgcctgcgatatcaatccccttgttgcccccctcagaagcgccaaaggtttcgatcactttgccctcagtcggccagcgccaggtggagataggcgtactggttgatgtactgctgacagtcggctcggttgtgcttgctgttggtaccgttacaggcgctgtgaccgtggtcgcagttggcttgttgttcggcaacattttgttagcactctgttcacccgaagactcagaatacgtaattgtcggttgcgacgcaacagcaacggtggaattttgtgcaggcttgatcacaactccttgctctgctgcgtcggcctgggtaatggcatttccgccagtgattggcgtaccggaagcattacccacctgcaaggtctgaccaacgttcagcgcgtatggtgcctgaatattgttgcgctgagcaaggtcacggaaatcgttgccagtaatccaggcgatatagaaaagtgtgtcgccttttttcacggtataggtactgccgctataactgcctttcggaatgttcccatactgacggttatagacgatgcgtccgttttccatctgtaccggctgctgagctactggctgcactggctggatttgcggttgttgagtagcctgaatttgtggctgctgcaccggctgaatttgcggttgctgcgctgtagacgtcgtccccattttcggcggcggcgtaatcaacataccagaattagtatttgcaggcgcattgccattaacggagctgaccggtgccggtggatttgaagtgtcagaacagcctgccagccatagcgaaaccagtgacaaagccgcaatgcggcgaacggtgaattttgggcttcccgcgctcatttatcccccaggaaaaattggttaataaccagtgacataattaccgtgcaaggcaccctactgaacactggaaaagatgttcacgatacgctgacctgcggcaaaataaccaggaaaaatccaggtatttcctcacgttttaagccagctcacccttcactaaagggacaaagcgcacggcctccacggtatcgataataaattcgcctccccgacgacgcacccgtttcaaatactggtgctcctcccctacgggtaagacgagaatcccgccttcgtccagctgcgtcattagcgcagttggaatttccggcggtgccgccgtaacaatgatagcgtcaaacggcgcacgtgcctgccaaccttgccatccatcgccatgacgggttgaaacattatgtaaatcaagatttttcaggcggcgacgtgcctgccactgcaagcctttaatccgttcaaccgagcaaacatgctggacaagatgcgccaggattgccgtttgatatcccgaaccggtgccaatttccagcacccgcgactgcggcgtcagctcgagtaattcggtcattcgcgccaccatatatggctgcgaaattgtctgcccctgacctatcggcaaagcgatattgtcccaggctttttgttcaaacgcttcatcaacgaatttttcacgcggcacggcggcaagtgcattcagcacctgctcatcctgaataccttgcgcacgtaattgatccagaagtgcttgtacgcgtctgcttaccattgcgtgccaactcccacgctgtttaaccagtctgaaaccacatcttgcgcgctatgcgcagttaaatccacatgcagcggcgtgatggagacatagccctcatctaccgcagcaaaatcggtccccggaccagcatcacatttaccgcccggcgggccaatccagtacagcgtattgccgcgcggatcttgctgcgggatcacctgatctgccggatgtcgtgtaccgcagcgcgtcacgcgaatacctttgatttgatccaagggtaaatccggaacgttaatattaagaatacgcccggtgcgcagcggctctttacacagtgcgcgcaaaattgaacaggttaccgccgcggcagtgtcgtaatgtttatgcccgtcaagcgagacggcaagcgccggaaaacctaaatgacggccttccatcgcggcggctaccgtaccggaataaataacatcatcccccagattcggcccggcgttaattccggacacaacaatgtccgggcgcggacgcatcagagcattcacgccaagatagacgcaatcggtcggggttcccatttgcacagcaatatcaccattttcaaaggtaaacgtgcgcagggaggattccagtgtcagagaatttgaagcgccgctgcggttacgatcgggggcgaccacctgaacgtcagcaaactcacgcaaggctttcgccagcgtttgtataccgggtgcatgtaccccgtcatcattactcagcaatatgcgcataatcacctgttgtgttgataagttccctgacaacgctggttgcaaaactacccgccggaagccagaaacggatctctacggtgacgtcatcccaccaattccagcttaattgttgcggatacagcagcatcgctctgcgcgcggcttcaactttttcgcgcaccagtaaagcttgtaattcagtttctgcggcgacagctgcttgttcgaatgccagcgcttcacgctgagttccccattcgccactgcctggcaatgcggcggttatcatcaactctttatcgttgacgcgacgctgtaattccgccagttcttcggtggttgcgacaaaccagctaccacgtccggctaattgtagcgcatcgccgtcaacaacttgattaacgtctgcttttttgaggcgctcagcaacaatctgattaaacaacgcactgcgggctgccgacaaccaaaaactccgtttattgcgatcgcgcaccggagtattggtttgcgcccagcgctgcgccccctgcaagttgctaccgccaatcccaaaacgttgggcaccgaagtagttcggtacaccttttacgcaaatatcgatcagacgttgttcaacgtcatcgcgattgctcacttcgcgcagaaccagggtaaaggcgttacctttcagcgcgcctaaacgcagcttgcgcttgtgccgcgcatactccagcacctggcagccttccagttgaaaggcgctcagatcgggcatttccttgcccggcacgcgagcgcataaccactgttccgtaacagcatgtttgtctttttgcccagcgaagctgacttcacgggcatgaattttcaggaatttcgccagtgcatccgccacaaaacgggtattgcagccgtttttgaggattctaaccagaatatgctcaccttcaccatcaggctcaaagcccaaatcttccaccaccacaaagtcttccggattggctttcagcagcccggtgccttgcggtttaccgtggaggtaagtgagattatcaaactcaatcattttgttgccttaatgagtagcgccaccgcttcacaggcaatcccttccccacgtccggtaaatcccagtttttccgtagtagtggctttcacgttaacatcatccatatggcagccgagatcttcggcaataaacacgcgcatttgtggaatgtgcggcaacatcttcggtgcctgagcgatgatagtgacatcgacgttgccaagggtataacccttcgcctgaatacgacgccaggcttcgcgtagcagctcgcggctatcggcacctttaaatgccggatcggtatccgggaacagcttgccgatatcccccagcgccgccgcgccaagcaatgcatcggtcaacgcatggagcgccacgtcgccatcagaatgcgccagcaatcctttttcgtaaggaatgcgtacgccaccaatgataattgggccttcaccgccaaaggcatgtacgtcaaaaccgtgtccaattcgcattatgtattctcctgatggatggttcgggtgaggtaaaactcggccagtgccaaatcttccgggcgcgtgactttaatgttatccgcacggccttcgaccaactgaggatggaatccgcaatattccagcgccgaggcttcgtcggtaatagtcgcgccttcatttagagcgcgcgtcagacagtcatgtaacagctcacgagggaaaaattgcggcgtcagcgcgtgccataagccgttgcgatcaacggtatgagcaatggcatttttgcccggttcggcacgtttcatagtatcgcgcactggtgcggcgaggatcccccccgtgcggctggtttcgctcaacgccaacaatcgcgcgaggtcatcctgatgcaaacaaggacgagcggcgtcatgcaccaatacccactgcgcgtcgccagcggctttcagacctgccagcacggaatcggcacgctcatcaccgccatctacaacggtgatttgcggatgattcgccagaggaagttgtgcaaaacggctatcgccaggacttatggcaatgacgacacgtttcacccggggatgcgccagcagcgcatgcaccgagtgttcaagaatggtttgattaccgattgagagatattgcttaggacattccgtttgcattcgacggccaaatccggccgccggaaccacggcgcaaacatccaaatgagtggttgccatgttaattcccgggctgatttatcgattgttttgccccgcagactgtgcgcgcttcgacgcgtcaggcaccagacgataaaaagtttcgcccggcctggtcatgctgagttcattacgcgcacgctcttcgagcgcctcctggccgccattgagatcgtcaatttcggcaaaaagttgatcgtttcgcgctttaagtttcgcgtttgtagcttgctgtgccgccacatcatcattgacgcgggtatagtcatgtataccgttcttaccgaaccacagcgaatactgtagccagaccagaatagccagcaacagcagcgttagtttacccatcctgccccctgaaaaacggcatcatcatcccatgcatccgaagacgactctacatcctctgttggggataccgcgacaacgcgggcaaatgtaccacatttgtccattgttacgtatacccagggcgtgcagaacataatctcattattagttacggtttgaattatgaacagaggagacgggaaagtacaaattagcccagtagccacataaacagtgcgccaaacataatgcctactgtcaccagggtgaaaacaatactgtagcgtagctttccgtccatcaatgaatgcagcgcaatccccaccactaccgcgacgggcatcagcgccagaaagaaaggccaggtgtagataaagaagaacagcgtgttagagccataaatcaacatcggcatcgccagcgcaaataaccaggagataaaaccgaccacggcaccaggcagtgaccatgtggtttcttcatcctcagtaaggctgtcgttatttgttagtgtaatgttatggctattacgcatatttgatcctgttactttgacgaaccgggcatggaaacccggtggtgtctcaggatctgataatatcgttctgtctcaacagatctaataattgctgtaccaaatttgttactaattgttcaccattgagatgaatttctgccgattcaggcgcttcgtaaacggaatctattcccgtaaagttgcgcagttcaccggcacgcgctttcttatataagcctttgggatcgcgggcttcgcaaatcgccagcggcgtatcgacaaacacttcgataaagcgcccttctcctacgcgttcgcgaaccatctggcgttcggcgcggtgtggcgagataaatgcggtcagcaccaccagtccggcttcaaccatcaaattcgccacttcaccgacgcgacggatattctctttacgatcggcatcgctaaaaccgagatcgctgcataatccgtggcgaacattgtcgccatccagcagatacgtactgacgccgagtttatgtaacgcctcctccagcgccccggcgaccgttgatttaccggacccggagaggccggtaaaccacagcactacaccacgatgaccgtggtgtagctcgcgttgttgcacagtgaccggatggctatgccagacgacgttttcgtcatgcagcgccattatttatcccccagcaaatcgcgcgcgccccagtgcggaaagtggcgacgaaccagagcattcaattccagttcgaatgcactgaattcagatggcgcagcagttgcctggctaactggctcgtgcaccataccggcacccacggtcacattgctcaggcgatcgataaaaatcagcccacccgtcaccggattttgttgataacgatctaacaccagcggctcgtcaaaagtgagatccacgaggccgatcccattcagtggcaggttttcaacttcacgctgggtaaggttattaatatcaacctgatagcgaatgccatcaacacgcgcgcgcgtcttcttaccggcaattttgatgtcgtaactctgccctggagaaagcggctgttccgccatccataccacatccaccgacgcgctctgcaccgccggtaacgcttcgtctgccgccagcagcagatcgccacggctgatgtcgatctcatccgtcagcaccagggtgatcgcttctccggcaaaggcttcttcgcgatcaccatcaaaagtcacgatccgcgcgacgtttgattccacaccagagggcagcactttgacacgttgcccgacttccacgcgaccggatgccagcgttccggcgtaaccacgaaaatcgagattcgggcgattaacgtactgcaccgggaagcgcattggctgagcatccaccactcgctggatctccacggtttccagcacttcgagcagtgtcggaccgctgtaccacggcatactttcactttgcgatgccacgttgtcgccttccagtgcagagagcggcacaaagcggatatccagattacccggcagctgcccggcaaaggtcaaataatcttcacgaatacgggtgaacgtctcttcactgtaatccaccagatccattttgttgatcgccacgaccagatgtttgatccccaacagtgtggagataaaactgtgacgacgggtttgatcgagcacgcctttacgggcatcgatcagtaagatcgccagttcacatgtcgatgcgccagtcgccatattgcgggtgtactgctcgtgccctggggtgtcggcgataataaatttacgcttctcggtagagaaatagcggtaggccacgtcaatggtgatgccctgttcgcgctcagcttgcaggccgtccaccagcagagccagatccagcttttcgccctgggtgccgtgacgcttactgtcgttatgcagcgatgagagctgatcttcgtagatttggcgggtatcgtgcagcagacgaccaatcagagtacttttgccgtcatcgacgctaccacaggtcagaaaacgcagcaggcttttatgttgttgcgcaatcatccaggcttcgacgccgccttcattggcgatttgttgtgcaagtgcggtgttcatcttaaaaatacccctgacgttttttcagctccatagaccccgcctggtcgcggtcaatcacgcggccctgacgttcactggtggtggaaaccagcatctcttcgatgatttccggcagtgtttgtgcatttgactccaccgcaccggtcagcggccagcagcccagcgtacggaaacgcaccatccgttttttaatcacttcgcccggttgcaggtcgatacggttgtcatcaatcatcatcaacataccgtcgcgttccagaaccggacgttccgcagcgagatatagcggaacaatgtcgatattttccagccagatgtattgccagatatcctgctcggtccagttagagagcgggaagacgcggatgctttcgcctttgttaatttgcccgttgtagttgtgccacagctccgggcgctgatttttcggatcccagcgatggaagcggtcacggaaagagtaaattcgctctttagcgcgggatttctcttcgtcacggcgcgcaccaccgaaggcggcatcaaaaccgtatttgttcagcgcctgtttcaggccttcagttttcataatatcggtatgtttcgcgctgccgtgcacgaatggattaatccccatcgccacgccttccgggtttttatgcaccagcagttcgcagccgtaggctttagcagtacgatcgcggaactcatacatctcgcggaatttccagccggtatcgacatgcagcaacgggaaaggcagcgtacctggataaaacgccttgcgcgccagatgcagcatgacgctggaatctttaccgatagagtagagcatcaccggatttgagaattctgccgccacctcgcgaataatgtggatgctttccgcctccagttgccgcaggtgagtaagtcgtatttgatccataaccgttcctttgcaataccgctattttcttgccatcagatgtttcgactatagggagcgtaagagaacgaatgaaattaccaattagaatgagtagttccttaacggaataacgatttggcaaagctaatatcaaaaagtgcttaaggcaccggatttcgggcgtttaggaagatttgaaattgttttagcgcagcggcagtttcatactatggcggtaaaaaaatttgcatggtatttaaggactcactatgttttccgcattgcgccaccgtaccgctgccctggcgctcggcgtatgctttattctccccgtacacgcctcgtcacctaaacctggcgattttgctaatactcaggcacgacatattgctactttctttccgggacgcatgaccggaactcctgcagaaatgttatctgccgattatattcgccaacagtttcagcaaatgggttatcgcagtgatattcggacatttaatagtcggtatatttataccgcccgcgataatcgtaagagctggcataacgtgacgggaagtacggtgattgccgctcatgaaggcaaagcgccgcagcagatcatcattatggcgcatctggatacttacgccccgctgagcgatgctgacgccgatgccaatctcggcgggctgacgttacaaggaatggatgataacgccgcaggtttaggtgtcatgctggaattggcagaacgcctgaaaaatacgcctaccgagtatggtattcgatttgtggcgaccagcggcgaagaggaagggaaattaggcgctgagaatttactcaagcggatgagtgacaccgaaaagaaaaatacgctgctggtgattaatctcgataacttaattgttggcgataaattgtatttcaacagcggtgtaaaaacccctgaggcagtaaggaaattaacgcgcgacagggcgctggcaattgcgcgcagtcacggaatagccgcaacgaccaatccgggtttgaataaaaattatccgaaaggcactgggtgttgtaatgacgcagaaatattcgacaaagcgggcattgctgtactttcggtggaagcgactaactggaatcttgggaataaggatggttatcagcaacgcgcaaaaacacctgccttcccggcgggaaatagctggcatgacgtaagactggataatcaccaacatattgataaggctcttcctggaagaatagaacgtcgctgccgtgacgttatgcggataatgctacctctggtgaaggagttggcgaaggcgtcttgatgggtttgaaaatgggagctgggagttctaccgcagaggcgggggaactccaagtgatatccatcatcgcatccagtgcgcccggtttatccccgctgatgcggggaacaccagcgtcaggcgtgaaatctcaccgtcgttgccggtttatccctgctggcgcggggaactctcggttcaggcgttgcaaacctggctaccgggcggtttatccccgctaacgcggggaactcgtagtccatcattccacctatgtctgaactcccggtttatccccgctggcgcggggaactcccgggggataatgtttacggtcatgcgccccccggtttatccccgctggcgcggggaactctgggcggcttgccttgcagccagctccagcagcggtttatccccgctggcgcggggaactcaagctggctggcaatctctttcggggtgagtccggtttatccccgctggcgcggggaactctagtttccgtatctccggatttataaagctgacggtttatccccgctggcgcggggaactcgcaggcggcgacgcgcagggtatgcgcgattcgcggtttatccccgctggcgcggggaactcgcgaccgctcagaaattccagacccgatccaaacggtttatccccgctggcgcggggaactctcaacattatcaattacaaccgacagggagcccggtttatccccgctggcgcggggaactcagcgtgttcggcatcacctttggcttcggctgcggtttatccccgctggcgcggggaactctgcgtgagcgtatcgccgcgcgtctgcgaaagcggtttatccccgctggcgcggggaactctctaaaagtatacatttgttcttaaagcattttttcccataaaaacaacccaccaaccttaatgtaacatttccttattattaaagatcagctaattctttgttttcaaacaggtaaaaaagacaccaaccttaaaccatccaaatctaccggggtacgcctgtttaacccaaatgtctggaactcaaatcccgtttccgtattcgttgcccatgccatcactacattgccttcttccgccagtccagctatttgttcccagatcatttcacgaatttttgcggatacatcacctacatatacccctgcacgtacctccaacaaccagatggctaatctgcctcgtaagcgcggaggtacattttcagtgaccacgaccaacatactcatttcagctactccgatggcctgcatctcccagtgaaacaggaagcggaatggcaacaggctgtgcatcttcaggtggggccggcggttgtatttctccagcggcaagcacgtcctctataagcggaatcaatttggctaatgttttactactgcgaaaaatatccctgcacgccaaacggacttcccggtccggctcaccagggttacgacgcgctatctcaaaagctttcggtacaacagtgtcaaatttaatgatgtctgcaatatcgtaaacaaaggaaagaggctttcctgtatgcacaaacccaatagctggtgcataaccagctgcaagtatcgccgcttcagttacgccgtataaacaggaagttgcagcgctaatgcattggttgatcgtatcgcccttttcccagtctttcggatcgtagcgacgtccattccatgtcacgccgtattgcttcgccagaagtgcgtaggttgcccgcacgcgactgccttctatacctctgagttgctctacggagcgccgggcaggcgcaggttctccaaaccgaagttcaaacattttacgtacgaccttcagacgcaaatcttcatccagagcaagttttgcctgatagagcagcttatctgaacgcgcacctccaggctgaccagaagcataaacacgaacgcccgcttcccccacccataccaacaatgttccaacttgcgcagccaggcgtacagctgcatgcgaaacccgtgtaccaggttccagcatgatgcaggcaaccgagccaacaggaatatgagtgcggatccctgtcttgtcgataagtacaaacgcgccatctattacatcgatctgcccatattgcagaaagatcatggagacgcgatctttgagtggaatgggattaaggggaagccaggtcattttattacacctcaatcacagtggagccaaagatagcaagccacatcccatcgatttagctggcccaataccttgctgtacaagatctattaacgctggcgcgtcgttgatggtgagcacaccttcaaagcaaaccgtttggatctttccacttttaccatcaccagaaaaatactgtggccgttccgatatgggatgcacatcttcaacgcgcgccgcattgcccaatttacgttgcaaccacgcgatttgttctgcttcttttattaacggaacccgacagcgtttaatattccctttactgtccaggcgcttttgattgtcgagaatagttttgatcggatttgcccgaagccgaaaatagagtggaacaccaacctgaagttgaaattcaacctgtttagttttaatgactgtcgcaacggcagttgaaacaggcatttgcgctgactgcaataaaacatgacagccttctggtgtgtttcgcttctcaacatgaaaaagaaaatcacgagcagcatccggtctgtttggaaataaatgccataatccctggtgaagttggtaaagatccctgctccaggccctggcaatgatgactttactgagatacatccatacctcctttaatcacataccattctcgggaagcaaattgtcgaggcaaggtgatcatcggttcgtcgcgcgccgtaaattttaaatgatgccctgtaactgattcctcactatatatatcgccgccaacgggctcataatttaatagcgccttctgaggatccgatgcctgacatgtccccaaaaaaagcgggtgtgttagtgggcaacttctccgccccaggtaaggtgtataccgaggctttaatactgctttttcaagttctgagataaccatcgttgcatggggtgttaaccagagagcgacggtaaaggaggcatcacataaatattcgcgccatgtttgaatcgtttcatgacttttcaaaccacggtaatcttctcgcgctccaaggactgtatggtaatcacgcaaccccgttacagacacacgacgatcgtcaagaatgagttcatcgcagcgcactgcaaattgcacactctctgataacgcctgtaatgaagaagtatcatcacgttggatcccaagacaagccccgagtagccctaataacccgcttcgggtcggaaatcttccggtaggtcgcgttccttcaaaggtcggctgcccccaggcttgcattggcccagcaagccgcaagatcaaataagatctcatgttcacgcctcgccattattacgaacccaggattttaactgttctaaagtaggcatttgtttaacttgagcagtaattgggtctacatcagataagctgaattgcgcagcagctccgttcagaccatatccattggcaacgcgatcccaatattgattaaacgcctgtatagacggttgcaaaaagccatctttcgctttaaccgctttttcaaaagcatttgccatagaaagtggcatatcggagaaattaaccattaccatatccgcagggttaaaagcggcataagtacgctgttttgctccagggacctctgttgccagcatatgaacaacatgggttgcaatttccagagcctgctccctggaggcaccacctaaattttcctgaagttgagcgaggttaatgttggcataacgataaaaaacacccgatgaaaattcctgagttcccagatgtgcagaaccttgttcctgtaaatcatctacagcggtgaaccagtcaatatcagaatcaacctgatgagtagtgatcgcatgcgcaatggacattgcaccatcaacttttcccaactcagtcatcatgccgctggttgccattcttccactaagcgcaatatcaacaccctgctgtaaattcacacgtatggcggcaatatcttccttaagaactttgagcagctttttatcatccagattatcagcctctgcttttgcaacctgctcacagaaccaggctatttctcccacaacccagggagtaaccgcatcggcagaaatcttttcggcttcatcaactgatttaccggagagcagcgctaatgtcttatcgatgattttttggtcaaaacgttcaccaagtttttgccgaagaacatcacgtaattgtgcaagatgaatggttctgagactggattcaccaatattttgtgcgtaataaccacttttacgcatcgcacgtttaaggctttgacttgaaattcttactcgtcttttgccgccgaaaatagcgtctttctgcatgttcatatcgtcgcggttcagacatgaagggctgtgagagatcagaacatgaatattgataaagttagacatagaaaggtttccttacgcatttttgtttgtggtcaatacaaaatcttccagaagttgctggcgttcgcgctttccccaccaggtcaacatcctggccattaatggccagtcaagtacgggttcggcgtgagtaagtaatcgacgtaactggaccatatcggctgttctgtcagcccgaattaattgaaagatacggcgctcgttaattcttccactattggctaaagctcttcccaacgagatacctgttgtttgctccgattttttgtcctgatgtcggatgacattctttcctgcgctcaggcaaaacaccatgcgcaaaagagcctgctggtgacgtgggttttcccaaccaaaaggttgcaccagcctataaaacgcagggatatcgcgtaattcatcaggttctgaaacacgtctaatttgcgcacatgatccattatccagttgttgccaggctcgatataaagccattgcatcaatttcatcagccatttgatggccctccttgcggttttaactcccgtaaatgtttgtatagcgtggcgcgggcaagcgctaatgtgcttattaatttaggatgatgtgcatagggagctacagattgattaaatagcatttcacacaattgatgaagtttgtctcgtaaatcagctattacctcatcagcctgggaaaaattaacattcgccagtacatcgggaattaataattcactctgtcgatagaaatgcctttctgcagtctcatgaacagagactccggcccctttgaagtctttatttttaaacccttctgcaaaggtatataacgccttgcgtaaggctgttttatatcccaaaccaacagtcactatttcgtttatcacattgccgtattgttgccacccctgattaaacatcaacacatcatgacgccgttcaagaatagatgcttgattattacgatatccccccataatcaattcaagaggactttgcggcgcaatatttctgaattgattcacaaccgccgccacgcgatttccattttcattttgaataatcttatctaccacaactcggctgatttgtgtccatgatggtgcggaggtggtgaaagcaagaaatttttcctcaacctcccctttcttgactgttaccagacaaggggaatgcggatggggccatagcccattaactgtaaaggtaaatttttccttaagaaaaccggtataacgcaaattgctttcctgtccacagcaagaacatttaccaatcccaatgggatcgcataattcaatatgcgctggttgccagaatagaccacggacaaacccaattgacgaagcaggtatagactcattggacttgataggtttaatccaggtaggttggttttccgtatgtgattcattaggaaattgtttttgaagacgaggtaatgtgaggacattgagtaacaccgttgaacgaagatcgatcccacgtacgaacgttgttacaggtgttcctccacgtaaaccgcttttaaaaccaccaccaaaacctggtgcctgattcgcctggttgaataacgcaatcgcagtgcatccaccacataatgcttcaccctgccccggttgattgacaaatgcacaattcgtcgcgccgcttaccccagccaacagtttttccattggagtcacatcatttgctttgacacctttggtctgcataaagggatgttctgcgtgattaaggtagaacatatctatccacggcgcgatgagttgttgaaactcatcttcagtgagcggattcattatgcgatgtcgaaattcaacgtcatcttttgccggggcgataatttgcccaatgcaaaccagcagtgctaaagcggccagttccatatcgtcacggggcaaacttaatcgccactgatctctactgcagtatagcgattgcagatttatgatttggactttccccccgtttcgcgggcgtacagggatccagttatcaataagcaaattcatttgttctccttcatatgctccgacatttctcctgcatttctatacgtcggcacacttccgttatcggtaaaaacaaagaaaaaatacggcgtaattaattcaataatcacattcactgcaaaaatatattcattggtttaatacaattaacctatacatatattaagatgtgttgaattgtttaaagacaataatgcatgcatttcaaatctgcaagttattcgttttattattaaagaaacttttagttataataattaccatgaattttattacataaaatattcatactgtgaatataaaatctcataccgggaaattaaaagaagatgtacattgtgcaccttccctacttaagtagggataaaccgttattggtcttattatcgtcattgataacaatcattcccgaagttatttgggatttgcagggatgactctggtcatcccttcatcccctgtataggtaataacaatactgttaccctgccagacccatccatccagattctgtttcccttccagccaaagtaacccatcttcatctactacttcagaaaaactacgtttccaggtgaagggtacattgacgcgattaagtgcaagcgcctcatactgctgttcatgacttaggtcctcgtagacctggccatcgagcagttgtttacctgaagacgtttgtacataaggcaataatggcaggctcatttccccatccctcgttaccgcaagaatggtttcatcgttatcctgcaagctatattcttcagcccactgcaggaccttgcgagccttgaaccttttttcacactcggcgctttcaaatttatccatgccattgccgacccattctggctcatccatttccgcatcatcgtaaatgctatccagccattgccggtaagcatcagggaaaaataaggatgctccattaagctcctcaatatgttgctgcgtccgccacatgactctaacgttgctataaatatgctcatgtcgtccgtaaccctcgccatcaggcagcaaaatggtggcaacaggaatctcaaaaccagcgggacgatatttgcgatgatggcgatgtaaacggcccaatcgttggaaaagcaaatctgcaggacaatgctgagtaattaaccaatcaaaatcaacgtcgagtgattgttccacgacctgggttgcgacaagtatccgtccaacatttcgcttcccatttttgccgaaattgctaataactcgattctctttttcacgacgatcgttcagcgtaaagcgcgcatgaaacaaatctatatctacttgcgtgttatttagctcctttagccgttggtagcatacttgtgcaacgtcaaccaaattgcaaataagacagacctgtgcacccgcgtttgccgctgcgatcattcgctctaacatcgtaaggtcaggtaacatgtcagctaaacaaataggttctggctgaatcgaaaagcggggcgggagttgttctggatgagctagcagatcaaaacgttgcgcaccattcacacctcgccagttaatgagtggatatgcggagttattttccactggatctgtatgcagaccataagtatccagaagtttctgtttttgtttcattggtagggttgcggaaagaagaataacactccctcccacatcagcctgagccttgagcactgcctccagcaagccgttcatataggtgtcgtaagcatgaacttcatcaacaattaaaacacttcgaccaattcccaaaccacggataaagcggtgtttaactggcaataccgatatcaacacctgatcaatcgtgcaaacgccgatttgcccaagaaacactttcttattgctttgtgacaaccactgacaacactgaacccacgcttcttcttgcccctgttcagtaatcgcgcgtgattttattgattgaaagaggtggttaaaccgtgaattgccatgagcaagaataagatttggggatgaaaataagtggctcgcgctcgcttccattctcgtaagcatagcattcgcggtagcttgtgttgggagggcaaaaataacactatccgcaatttgttgatcaataagtttccaagcataggccagcgctgtttccgttttaccggagcctgtaggtgcctctattaccgtcagcccgggagctactggaagagcatcaactaacacctgtaattgtctgggttgatagccattgtccagtagtgcatgaacaccttcataacatcgcttatttgatacaagtccactcaactccaatacccggctcgcatcctgctgtcggtcctggaaatacgttctcagagcatttatgtcggaaggcgcatcctcattaaacagaaaggtattcgttgtagtccaggagcctaaccagtcagcaagcgagcaaaaacctgctaacagtgatgaacaatcaggtggtatatcgtttatagataaccccgctggcgttaaaaataatgcttccagtacagatatccactcctcacgagcctgtttatcttgcgcagcataagatgccagagaagctggcatttcccaacgcgacttatcttgatcctgggaatgtaatataaaaccatgatgtcctgtaacggcctctacccatggaaaccaggactcataaggatgaggagcggcatcaaaaaaactgaaaaaatccccgagagattgctctgaaagtgaatcctggttaaaccaatacagaccggctgcaccatgattaaatttacggcacatttgtgttgatggaccattaagtgatggcgttgcaggatttaatttcagccaactttctgctgatttatattggaatcgtatatcaaactttccaatatcatgaagagcaatgaaaaataacagccaggccttcaccctctgttttgatagcatttcatttcggcaaaaagtattttgcagtacgactgattgatcccaccagcaatctgcaacagcagcaacatcaaggcaatgataaattaacagatgaatatcatttcctttcgtcaagctttttgaggattttccccagtaatggcatatatatttaaaaggttccattaatagcctccctgtttttttagtattatcgatgatatcagcgggctatttttcgatgctgctcataaatatcgaattacagtgatatacacatgtcttgcctccctgcaaagaagagactaacattcgaattgtttgggttcgaacgctggcctcaggttgatagaaatatcgcctggggcttttgtccatctggaacctcgcgaatgcttaacgccagacagcctcaagcacccgacgccattctatacctgataattcttcccgcggcgttcacgtttaaaatcaggaatgctgctcgcaaaataaaaacgcccccatcatttctgacagaggcgtttaatttgtccggcaatatttacccttcgtgtaacccacattccctttttaagccaaagaaacgcgtttcttcttccgccatgccgggttcccatttacgggttgtatgggtatcgcccaccgataaatatccttcatcccataatgggtgatatttcaggccatgtttttgcaggtactgataaatagttcggttatcccagtcgataatcggcagcactttaaatacgccacgctgaattgccagcaccggtaaattggcacgactgccggattgttcacggcgcaggccagcaaaccaggtttgcgcattcagttctttcagagcccggttcatcggttcgactttgttgatgtcattgtacttttcaatgccttcaacgccctgctcccacagttttccgtagcgtgcttcctgccaggctgcgctttcggtagcacggtacactttcaggttgagcttgagtttgtccgttaactcgtcaataaagcggtaggtttccgggaacaagtaacccgtatcggtgaggatcaccggaatatccgggcgaatttgattcaccagatgcaggctcaccgccgcctgaatgccaaagctggaagaaagtacatattcaccgggcagattatccagcgcccaggctacgcggccttcagcgtccagtttttccagttcggcgttagtttccgccagcgccagaatgcgatctaccttcggcagttcgttcagggcgtttagatcgagtttggacatagattcctcactgtttgccttgcctgatgcgacgctcacgcgttcttatcaggcctacaagaccgggctgatggttaatcccacaaatcacgcgccggatcgagcaccgggcgaatgatgcccgcacgcaccgtaaagtcgccgaagccttcacccgcttcgcgctctttcgcccagcgccctatcagttcatcaagcgacgccaggatttccggctcggtgatgttttctttatacatccgtgggatacgtgtcccaatgcggttgccgccaagatgcaggttgtagcgacccggcgctttacccaccaggcccacttccgccagcatcgcgcgaccacaaccgttcgggcagcctgttacacgcatcacgatatgctcatcgctgacaccatgtttcgccattaaattatcgatgttgtcgataaaagacggcaggaaacgctctgcttccgccatcgccagcgggcaagtcgggaatgacacgcaagccatcgagttttcacgctgcggcgtgacggcattcattaacccgctctctttggcgatcttctcgatcttcgctttctcgctttccggtacaccggcgatgatcagattctggttcgccgtaatgcggaaatcgcctttgtggatcttcgcgatctccagcaggccggttttcagcggacgcgccggataatcaaggatgcgaccattttcgataaacagcgtcaggtgccagttatcatcaatgcccttaacccagccaatacgatcgcctcgtccggtgaactcatatggacggatcggttcaaatttgatccccgcgcgacgctccacttccgctttaaacgtctcaacccccacgcgctccagcgtgtatttggttttggcatttttacgatcggttcggttaccccagtcacgctgagttgtcacgacggcttcggccaccgccagcgtatgctccagcggcagatagccaaactcactcgcggtgcgggcgtaggttttcttgttgccgtgttcgatggaaagcccaccgcccaccaacaggttaaagcccaccagcttgccgttttcggcgatcgccacgaagttcatgtcgttggcgtgcagatcgatatcgttctgtggcgggatcactaccgtggttttgaatttacgcggcaggtaggtctggccgaggatcggttcttcatcagtagtggcgactttttcctggtcgagccagatctccgcatacgcgcgggtacgaggcaacagatgctcagaaatcttcttcgcccactcgtacgcttccgcgtgcagctgcgactcgtaagggttcgaggtgcagagtacgttacggttcatgtcgttagctgtcgccagcgcatcaagaccgaccgagtgcagcatctggtgcaccggtttgacgttctttttcagaatgccgtggaactgaaacgtctggcggttggtcaggcgaatgctgccatagatggtgttttcaccggcaaatttgtcgatcgcctgccactgtttagtggtaatcaccccacccggcagacgacagcgaagcagcatcgcgtggcgcggctccagcttctgttcagcacgttcggcgcggatgtcgcggtcatcctgctgatacatgccgtggaagcgaatcagcaggaagttgtcgcccttaaagccgccggtcagaccgtcgtttaaatcttccgcaatggtgccgcgcaggtagttgctttcatgcttcatgcgctcggcgtctgtcagttttccttcgaccactaaaggccctggatgtttttcgctcattagtagacatctcgctgataacggcgctctacgcgcagctcacttaaaaattcatccgccgcttcggtgtccatgccaccaaattcggcaatcacttccagaagtgcctgctcaacgtctttcgccatgcgattagcgtcgccgcagacataaatgtgggcaccatcattgatccagcgccacagctccgcgccctgttcgcgcagtttgtcttgtacgtaaactttttctttttgatcgcgcgaccaggcaagatcgatacgtgtcagcacgccatctttgacgtagcgctgccactccacctggtacaggaagtcttccgtaaagtgcggattaccaaagaacagccagtttttacctggcgcttcgtcggcggcgcgttgctgcataaaggcgcggaacggcgcaataccggtgcctgggccaatcataatcaccggggtttctggattggctggcaggcggaagttatcgttatgttcgataaatacgcggacttcgccctcttcttccacgcggtcagcgaggaagctggaggcaccaccggcacgggcgcggccttccacgtcgtaacgcaccacaccaacggtgacgtgtacttcgttctcgacttccgcctgcgaggaggcgatggaatacagacgcggcgtcagcgggcgcagcagattaattagcgcttcggcatcaagctgtgccggggagaaacgcaccatgtcaacaatcggcgtcgtcgcggcgtaatgctgtaacttcgctttatcgcccaccagcggcagcagtgtttcactgcgggtaagcgtggcgtaattctcaacaatgttggcggtgttgacggtcagttcgaagtgccactgtagcgcttcgttcagaggcaacgttttgccctcgacggtgacaggttcatcgcctttcagccacagcagttcgacaagttctttcaccagtgccggatcgttctgataccagacgcccagcgcgtcacccggctggtaacgcatgcccgagtcacctaagtcaatttcgatatggcgaacgtctttttcagagttacgcccggtaattttctggttaacagagaggctagccaccagcggcgcgtctttgctgtacgggctggtgtggatttcatttaccgcgccagtagcgacggattgcgaaggtgccgcgacaggcgcacgcgatttaagcgcatcaaccacgcgggcgcgccactcgctggcagcagcctggtattcaacatcggcatcgacacggtcgagcaggcgttcaccacccagttccgccagcttgctgtcgaaatctttcccggactggcagaaaaattcataagagctatcgccgaggctaaacacggcaaacgcggtgttttccagctttggcgcttttttggagaacaggaacttatgcagcgcgacggcttcttccggcggttccccttccccttgcgttgacgtcactacgatgagcagtttttcgctggcgatttgtttgaatttatagtcgcccgcgttcaccagcttaacgttcagttttgctgctaataaatcatcacgtaatgcttcagcaacccggcgcgcattgccggtttgcgaggcggagataatagttatacccggcatttctgcggctggcgctggcgtcgctgcaagcgcagcaggctgctgattgagtacgccccagaaatagccagaaacccaggcaagctgggtgggagttaaatcggtcgtggccgcctgaaggcgtgccagttgctccgggttcaacggaagcaacgcggaaggtgggacctgtgtcgtcatgcgtcgttatgttccagtaagcaaagctgtttctgcgccctgtcagcgcccataaaacagaagagaaggtaaggttaacggggcaaacggtgtggattaaagacgggatagcgataactaataaccaaatcgactaacctgttttagcaatagtctttaacaacaaaatagattaaccaacctaatgaaaaacaaatgaatttagccaatcattaagataaatcagcgattttgcgcaacaaagtcgttttagataatgcgaaaaaacagcctttccggtactctacggcggttttatcgtcctgtagagaaattatgatgtccaccacgttatttaaagatttcaccttcgaagccgctcaccgcttaccacacgtcccggaagggcataaatgtggtcgcctgcacgggcattcctttatggtgcgactggaaattaccggggaagtcgatccgcatacgggctggattatcgatttcgctgaactaaaagcggcgtttaaaccaacctacgagcgcctcgatcaccattatctcaatgatattccaggtctggaaaacccaaccagcgaggttttagcaaaatggatttgggatcaggttaaacccgttgtgccgctgttaagtgcggtgatggtaaaagaaacctgcaccgcaggttgtatctatcgcggcgaatgataagagtgtgtcggcggtcaatttcccttaagtaacgctatgttagggtgttgtgttctggatatctggggcatgacatggaagacgactgcgacattattattattggtgccggtattgcaggcaccgcttgcgcgttacgctgcgcgcgagcgggtttatccgttttgttactggaacgcgctgaaatccccggcagcaaaaatctttccggcgggcggttatatacccatgcactcgcggaactcctcccgcaatttcatctgaccgcgcctcttgaacgacgcatcactcacgaaagcctttccctgttaacgcccgatggcgtaacgacgttttccagcttacagcccggcggtgaatcctggagtgtattacgtgcacgattcgatccgtggctggttgccgaagccgaaaaagaaggtgtcgaatgcatccccggagcgacggtggatgcactgtatgaagaaaacggcagagtctgtggcgttatttgtggtgacgatattctccgcgcccgttatgtggtgctggcagaaggtgccaacagcgtcctggctgaacgtcacgggttagtgactcgtcctgctggcgaagcgatggcgttggggatcaaagaagtgctgtcgctggaaacatccgctattgaagaacgttttcatctggagaataacgaaggcgcagcgttgctgttcagcggcaggatctgtgatgacttacccggcggcgcatttctttatactaatcaacaaacgctctcgttagggattgtttgcccgctctcttcccttacgcaaagtcgtgttccggcaagcgagctgctgactcgctttaaagcgcatccggcagtgcgcccgcttatcaaaaacacggaatcactggagtatggtgcgcatctggtgccagaaggtggcttgcacagtatgccggtgcaatacgccggtaacggctggctgctggtgggcgatgcgttgcgcagttgcgtcaataccggaatttccgtgcgcggcatggatatggcgctgactggcgcgcaggcggcggcacaaacgctgataagcgcctgccagcaccgcgagccgcaaaatctgtttccgctttatcatcacaacgtagagcgcagcctgctgtgggatgttctacagcgttatcagcatgttccggcgcttttgcaacgcccgggatggtaccgtacgtggcctgcgttaatgcaggatatttcccgcgatttatgggatcagggtgataaacctgttccaccgctgcgccagttattctggcatcatttacgtcgtcacggcctgtggcatctggcgggcgatgttatcaggagtctgcgatgtctgtagcccgtaatctctggcgcgttgctgatgcgccgcacattgttccggctgactccgttgagcgccagacggcagaacggttgattaacgcctgtccggcaggtcttttttcgctcacaccggaaggtaacttacgtattgactatcgcagttgcctggagtgtggcacctgccgtttgctgtgcgacgaatcaacactacaacagtggcgctatccgccttccggattcggcatcacctaccgctttggataaataataaggataatttatgcccctcttacacctgctccgccagaatccggtgattgctgccgttaaagataatgccagcctgcaactggcaatcgattctgaatgccaatttatttccgtgttgtacggcaatatctgcaccatcagtaatatcgttaaaaagattaagaacgccgggaaatatgcttttattcatgttgatttgctggaaggcgcgtcaaataaagaagtcgttattcagtttttgaaactggtgaccgaggcggacggcattatcagtaccaaagcctcaatgttgaaagcggcaagagcggaaggttttttctgtattcatcgcctgtttattgttgattcaatttcgtttcacaacattgataagcaagttgcgcaatcgaatccggattgtattgagatcctgccaggctgtatgcccaaagtgctgggctgggtgacagagaaaatccgccaaccgctgattgccggtgggctggtgtgcgatgaagaagatgcgcgtaatgcgattaacgcgggtgtcgtggcgctttccaccacgaataccggggtctggacgttagcgaaaaaattactttgacgggataatcgtaaccaattgaatttggtttgatttgtaggccgcacgccacatccgacattcagcgcctgatgcgacgcttgacgcgtcttatcaggcctacaagtccccaggccagaaccgtaggcaggatcatccggcaacacgttattggcaatctgcgtgaatgtttgtcaccagtgcctccagcaccactttccagtcatcaaccacgccaacatctgcctgtgaaaataccgcagcgctggcgtcatgattaatcgccaccacaaacttgctattgcgtacgcccgccattaacgctgctgcgccagaagcgccaacaacaatacacacctcaggtgccagcagatgtccggaaataccaatcactttttcagcatcaacgccaccgttcatcactcgcgcccgactgtagcccacttcggctcccagcttttctgccagcatagcgatttcctggttatctgcctctccgccctgccccaccaccagcacccgtctggcctcagctaatgggtcgcgggtaacatttttcagatcctctgtgctaaccagccagtccggaagcgcacccgggacaatgttcagttgttgcattccagagggcaacgtggcgtttttcgctgctcccgcctgacgcgccagggaaaggcatagcgggcgtttttctgtttgcagcgtcgccgttagcgcatttccccagtgggatttgcgcacgcttacggttggaatatctaacgaagtcacctggcagatgcttgcaccatgtaaacgccaggccagccgggtcgacagttcatcgccaaacgttcccggcggaaagagaacaacgtccgcaggcgttcgctgccactgttccaccaacgcatccagcacctgttccgccactacaggctgaggttcaatctgccagtgcgccagggtacaaccgctgaaatcctgcgccgccagccagcttgctattgcggcattctcctgatttattgtcacaattgcgatattcatggctgcatcctttggcgtaaatagtcctgccatagcttttgagctttttctgctaccgtttgcccatcaatcagcgtcgctccgcgtcgttgctctgctcttgccagttgcagacactgcatcgctggcatttcggcagcaacagttttacggataatttctgctttccccgcagccattcgctggcgcattcccggtactggcaaggccacttcaccgcactgacgcacggcaatcaccgcaggcaagcgaacccggcaacaacgcaacccatgttcagtacgctgttcgagggtgataaacagcgcgtcgagagtgaaacgctccacctgggtgaagcagggccagcccagcatttccgccagcaaaaatggcgtttgcccattctgcccttcgctgctttggcagccggtaattatcagatccagcggattctgatgctgccattcggcaatatggcgagcgacaaattccggcgcaaagcgcagatctgccgccgtctccagcaatacagcttcctcaaacccaagagccatgagatagcgcagccagtgcaatgcccgttcatcccccatgctcaacgcggttaaagacatcggcgtaccgttttttctctgcgccaacagcagcgcggcagcggcctgttcatcagcaccgagtaaacttcgcagtagcgaaatatccggtccgcttttaccctgagccgccgcctgccactctttttccgccagcattccggcatccggttcggctttaaacgctaacagaatgttcattcgcacctcctacatttcccgccgccaccagcgggagggctttagtttctggtgcccatagccaggtcacaacaaaaccaaccaacaacactgtcgccaggagcaataaggtgacttgcattccccactgcgccagcacccacggcagcaggccagtacttaccgccgcgccaagtcgactcatggcagtggcaaaaccgacgcccagcgagcgaatgtcagtaggaaaactttccgcaggcaaaatgcccaccagattactgactgccgaaatggtggtgctgaagagaacaaaaagcagcagcgttaatgaactgccggaaggcaaacaggccatgactaccagcgttgccgccagcagcaaaaaacttcccagcaaaaatttgcgatgtgccagcaggtgcgtcagaactaatcccagcagcgcgcccacaattaacaacgcattaagcatcaggctggcagtcagcgcatcttccagaccaatagtctgggcgatagttggcagccaggtataaatcacaaaccatgggattacgaggcagacaaagaagacgctgttaaacgccgtgcgccgccagtaacgcgaagagaacaaggttttgatgtgtttatgggtcgccgttaccacttcatcgcccagtaaaacatggggaccaaaatagcgatgcacgatagcgtgagcttctgcaaaacgcccctggcgcagtagccagcgtggtgattctggcgttccccagcgtaataacgtaatcaacaacgcgggcagagctgccgatgccagtagccagcgccaggcctccgggttttcggaaataaagtgatgtccggcaatacttgccagcacatagcctacggtccacaccacgctgaatgcgcccagcaaaataccgcgatggcggcgcggggaaaattcagccagcaaggtgtgacctactgaataatcgcctcccagaccaatgccaatcaaaatgcgcagtccaataagatgctctggcgtggtggcaaaaaattgtaaaaacgaagcaagcgtaatcagcaaaaagctgaaggtgaagattttttgccgaccaatatggtcggagatccacccaagaaccaggctgccaaggaacaaaccaaggagcgccgagccgccgatcattcccgccataaacggcgtcagttgcatggcgggcgtaagctgaataatggcgtaaccaatgacgccgagaacataaccgtcggtcaggtgtgcgccgaaagtgagcgcagcaatgcggcagtgaaaacggttaagcggtaaatcatccattcgcaccggtgaagtgttcatctttaccccttcattgtccggtaataagaacggcttctcgcctgagaagccgaaaaggcaacgccccgtcatcgcggaacgctgcctgacacattatttttcaatcggatagatagtacccgtattcataatgccattaggatcgaactgctttttcagcccttccagcaacgcccacgcgctgccgtgttccagtttgctccagtgaacgcgatgtttaccgataccgtggtggtgcaccatcgaaccgccgaggcgaatggtttcttcacagatgatcttgttgagcggattgtggtacttgtcgatttcctcttccggcttacagtcaacgacgttgtaatcgtagacgaagtacatgttggtgccgttctgatagctatgagaggaatgaccgcccagcatggtgatgtcgtcggcgtgcgggaactcagtacgaatacggttaataacgctttcgtagatttcgtggatgcagctccagcagccggatacttcggtggtaaagcccatgttgccggttttgaggatctgcacacgttcggcagccactttatccggtccccagttcaggttgttaaaccaggtttcgatcagcttgctgtccacgcgctggcattgcgggtagcgggcaacgatttccgcaatcccttcgcccgtcaccttcgcaatgcgagggttaccttcagccataaagatcagcacgcattttccgtcggcaaaatgggtgaagtgttgggtgccatcttcagcgtcatacaaacgagcgattgacggacgatacccttccaccatgatttcacgcaggatgttgaagccggttttcatgtcttccaggatatagccgtagaagaggttgttttccggggtgaatttaaagattttcactgttacttcagtgatatagcacaatgcaccttcgttgccgatgatgatgtgacgaatgtccgggccagccgcgcggcgtggcacgtttttaatgcgtgtgacggtgccatcagccaatactgcttccagaccaacgaccatatcttcgattgcgccgtagagtgtggagaactgcccgatacttcgggttgctaccaggccgcccatctgcgccagcggctttgactgcggagaatgccccgtggtgtaacctttttcacgcaacgcgttttccagcacttccagcggaacaccacattgcgccgtcgcctgcatattctcaatatcaatattaatgatttgattcatggcggagccgtcgagcaccaccgagttttctacaacagtttccagcccaccttcggtggcggaagcaccggtacgcggcacaccgttaattttgtgcgcattcataaaattcagcacacgggatacttgctctgtggaaccgagttttacgaccgctgccggaatcggcaaagtataaatgccatgaatatccggaaatttacgaaaacggtcaatactgtttttctttaatactgtttcatcggtaattacgcgatctgcaccaacaatttcctttagctggtcgacaatcgctgcgcgagataaagacatagtaattccttcctgataataaaaatggaataatcattaataagagaaaacagaaaccaccgttatgggttagcgcactaaataaccgccatcaaccactaataaatgcccgttgacataattcgatgccggacttgcgaggaatacggctgcgcccattaaatcctgagtatcgccccaacggtttgccggaatatgatcaagaacgcgctgattggtttctggattactgcgtgtcgccagcgtaatatctgttgcataatagccaggggcgataccatttacctgaatattatattgacctagttcatcacaataagctttggtgaacccggcaagagcatgtttagtggcagaatatgcaggtgaccattgtccacctaagtaagagaacaatgaacagatattaataattttgccgcttttctgcgggatcataatttttgcagcttcatagcttaactcgaatgcggcggtcaggttcacatcaatcatcggatcccagtcggcacgaccgaagtccagcaccttattcagcttacaaataccggcattgttaaccagaatatcaactgtaccgaaacgctcacagcaagcagcgataatcttctgcggcgcgccttctgcggtgatacccacctgcatgaagtccacctcaacaccctgtttttcaatcatttcctttgtttcgccgttatctttgacgaaactaggaataaagatatttgcgccagctttggccaacgccatggcaaatgcctggcctaaaccgctattcccaccggtaacaattgcggttttacctttcagggagaaaaaatccattgagaacgcattgagagattcgattgacatagttagctccaatttccgtaaggcaaaaaaaaagaaaggtaacttcccccgcgagagggaagttacctttctcattatctctggtaactggagataatttttagcataagggcataactgctaatgtgatcgtaatcacagtgtgatattcgtattgtcaaataattttaaaaagcagaagcgtgattactctcacacaacacctctgctttccatgttatttattatttcaattactagagacctgagaaaagtaatccacctgaaagggcggcttacttttctcttttttttgtctattacaaatgggaatacgatatgcaacacaactcatatcgccgttggataaccctcgcgataattagttttagcggcggcgttagtttcgacctggcttatttacgttatatttatcaaattcccatggcgaaatttatgggattcagcaataccgagataggtttaataatgagtacctttggtattgcggccattattctttatgcccccagcggcgttattgccgataaattttcacaccgcaaaatgattacttccgcgatgatcattaccggattactgggtctgttaatggcaacgtatccaccgctgtgggtaatgctctgtattcagatcgcctttgcgataacgacgattttaatgctgtggtcggtgtcgattaaagctgcatcgttgcttggcgatcatagcgagcaagggaaaattatgggctggatggaagggctgcgcggcgtcggtgtaatgtcgctggcggtgtttaccatgtgggtcttttctcgctttgcaccggatgacagcaccagcctgaaaacggtcattatcatctatagtgtggtttacatcttgttggggattctgtgctggttttttgttagcgataacaacaacctgcgcagtgccaataacgaagaaaaacagtcattccagcttagcgacatcctggccgttttgcgtatcagcaccacctggtattgcagcatggtgatttttggcgtcttcaccatctacgccattctgagttactccaccaactatctgaccgaaatgtatggcatgtcgctggtggcggcgagctacatggggattgtgatcaacaaaatattccgcgcgctgtgcggcccacttggcggcataatcaccacctacagcaaagtgaaatcccctacccgcgtgatccaaatcctttccgtactcggcctgctgacgttaactgccctgctcgtcacgaactctaacccgcaatcggtcgcgatggggattggcctgattttactgctgggattcacctgttacgcctcacgcgggctgtactgggcctgccctggcgaagcgagaacaccgtcttacattatgggcaccacggtaggtatttgttcggtgattggattcctgccggatgtcttcgtttacccaattatcggccactggcaagacaccctgcccgctgcagaagcctaccgcaatatgtggctgatgggcatggcggcgcttggcatggtgattgtctttacctttttgctgttccaaaaaattcgtactgctgatagcgcccccgcaatggctagcagcaagtaagccaggaaaattacaggagaaaaatcatgtcgaaaaaatacatcatagggattgatggcggaagtcagagcacaaaagtggtgatgtacgatctggaaggtaacgtggtttgcgaaggcaaaggcttattacagccgatgcacacgccagatgccgatactgcagaacatcctgacgacgatttatgggcatcattatgttttgccggtcacgatttgatgagtcagtttgccgggaataaagaagatattgtcggtattggtctgggatccatccgttgctgccgtgcgttattgaaagccgatggcacgcctgctgcgccgttgattagctggcaggatgcacgcgttacacgcccttacgaacacactaaccctgacgtggcatatgtcacctctttttcgggttatctgacgcatcgcttaaccggcgagtttaaagacaatatcgccaactattttggtcagtggccggtggattataagagctgggcatggagcgaagatgctgcggtaatggataagtttaatatcccccgtcatatgctgtttgatgtgcaaatgcctggcaccgtcctcggacatatcacaccacaagccgcactggcgacacatttcccggcaggactgccggttgtttgtaccaccagtgataaaccggtagaagctctgggggccggattactggatgatgaaacggcggtaatttctcttggcacttacatcgcattgatgatgaacggcaaagcactgccgaaagatccagtagcgtactggccgattatgtcttctattccgcaaacattgctgtatgaaggttacggtattcgcaaaggcatgtggacggtgagctggctgcgcgacatgctaggcgagtcgttaattcaggatgccagggcgcaggatctttcaccggaagatttactcaacaaaaaagcttcttgtgtgccgccaggctgtaatggtctgatgacggtgctggactggctgaccaatccgtgggaaccgtacaaacgcgggattatgatcggctttgattccagcatggattacgcatggatatatcgttcgatactggaaagcgtggcgctgacgctgaagaacaattacgacaatatgtgtaatgaaatgaatcactttgcgaagcatgtgatcattactggcggcggttcgaacagcgatctgtttatgcagatttttgccgacgtgttcaaccttccggcacgacgtaacgccattaacggttgtgcaagcctgggggcagcgattaatacagcggtaggtctggggctatacccggattacgcaacggctgtcgataacatggttcgcgtgaaagatatctttataccgattgagagcaatgccaaacgctacgacgcgatgaataaaggcattttcaaagacctaaccaaacatactgatgtgatcctgaaaaaatcgtatgaagtgatgcatggggaattggggaatgtggattcgatccagagctggtcgaatgcgtaagtgaggaaggccgggcgggaaactgcccggcctgaacatacctgaatggttatccccgctgacgcggggaacataagttcgacaacttaaaaaatgataacaagtccggtttatccccgctgatgcagggaacataataaaaactttaactagttcggtttatccctgtttttacaaggaatattaactacactcgatgtctttagaataaaagacaatacgaatcgcactttatcaattttcacttaaagtatgaactggatatctttattcataagaactattcatcaacagcgtatagaggcggttatgtaaaaccactcattagcctcaaaacaaagacaaacttccagatttattacttaaccaatgaataacaagcttaaaaaatatactgttattctaaagaaaaaattaacaggcattaattcaatattaaaaaaataatagattaaaatttcttaacgatttaagaatcatacaaataacactttgattaaatttaattttttgtatcgataattgtgaacctctctggcatggagaactattttgaacatgaggtgttacgtggatatgttgcttattacaagtactgctaatataaaaacttgagaaagagataacgggttatatggtggtttatccccgctggcgcggggaactcgacagaacggcctcagtagtctcgtcaggctccggtttatccccgctggcgcggggaacacctgttttcgcaaatctatggactattgctattcggtttatccccgctggcgcggggaacacgggcgcacggaatacaaagccgtgtatctgctcggtttatccccgctggcgcggggaacactggctctgcaacagcagcacccatgaccacgtcggtttatccccgctggcgcggggaacacgaaatgctggtgagcgttaatgccgcaaacacaggtttatccccgctggcgcggggaacacattacgcctttttgcgattgcccggtttttgccggtttatccccgctggcgcggggaacactctaaacataacctattattaattaatgattttttaagccagtcacaatctaccaactttatagtatcacacaaacaacacatccattatgttaaagagcacttaatccattgattaaaaaggtaaatatttaaaataactctatacaaactaaaatctaccaaactttaccgcaataattttcactccagcgaaaaattaatgccacagaatttgtagagaatgctaatgattagccctggatgggtaaaatggaggagttttcagaggcgacaaacaatataaatgagtagaagtctttacaggttccacccatttataacgcttataaatgtttaatcaggcaatatttagatatttatgtgtttgcatcgacaaacgccaattacgcgcaatgcaggtttcaatgcacaaacgtgtggcatcatccttttggctaatcggctgcagtgcaatgactcgcggtttatcatcggtcagcgttgccagtagttcatccagtgcttcaatatcgcgtacgcgccccactggatgcttgatttcgttggctcgctccagtgcctgtgacaacacttcatagccgccgcgcatgttcagctttggcgatacggtaacccaggtattcggtgtgcagcgtacctcatgagtaccactggtttcgatctggcagctaaaaccgttcttttcgagcagatcagtcagtggcagcaaatcatgaatgcaaggctcaccacccgtaatcaccacatgccgcgcggtgtatccctggcgaccaatgacagccagcaaatcttcactgctcgcagccccccacttatcactctctttggtcttcgccagaatgctgaaaagggagacttcccgatcctcaagcttttcccaggtgtgtttggtgtcgcaccaggcacagccaaccgggcatccctgtaaacgaataaaaatggcgggaacgccggtaaagtaaccctcaccttgcagggtctggaacatctcgttaatcgggtactgcatagcattctctgtgaagtggataattgttaattattgcagatcctgccacaacaatcatgtcttattaacattctgttacaggcaggtttaaagaaaaatgcgaaacatatcgttaataattaaagggagtaacgtattatgtcagaagaaaataaagaaaatggatttaatcatgtcaaaacattcaccaaaattatatttattttttctgtattagtttttaatgataacgaatataaaattaccgatgccgccgtcaatttatttatccagatttaatgagaaatttataatgcgctatttcatactaatgttcactttcgtatgttcctttgttgcagcccaaccaactattgtcccacaattacagcaacaagttacggatcttacgagtagcttaaactcacaagaaaagaaagaactgacgcacaagttagaatctattttcaataatacccaagtgcaaattgccgtattaattgttcccacaaccaaagacgagacaattgaacaatatgctacaagagtttttgacaattggcgtttaggagatgccaaacgtaatgatgggatactgatcgttgttgcctggtcggatcgcactgtccgcatccaggtaggttatgggctggaagaaaaggtaaccgatgctctggctggagatatcatccgtagcaacatgatacccgcatttaaacaacaaaaattagctaagggattagagctagctataaacgctttgaataaccaactcacttcacaacaccaatatccgactaatccttcagaaagtgaatcagcgtcttccagtgatcattattactttgctattttttgggtatttgcagtgatgttcttccctttctggttttttcatcaaggcagtaatttttgtcgcgcatgtaaaagtggagtctgtatttcagcaatctatcttttagatttattcctgttctccgataaaattttttccattgctgtattttccttcttttttactttcaccatatttatggtctttacctgtttatgtgtacttcagaaaagagcatctggtagaagttatcattcagacaacagcggttccgctggaggctcagatagcggcggatttagcggcgggggcggttcttctggaggtggcggcgcatccggccgctggtaactcaaccataaaaaatgccagcccggaggctggcatttttaaatcagataaagtcagtcttatgcctggcctttgatctctttacgaccgttgtacggtgctttttcgcccagagcttcttcgatacgaatcagctggttgtatttagcaacacggtcagaacggctcatagaaccagttttgatctggcctgcagcagtaccaacagccaggtcagcgatggtagcgtcttcagtttcgccagaacggtgagagataactgcagtgtagccagcatctttcgccatcttgattgcagccagagtttcggtcagagaaccgatctggttgaatttgatcaggatggagttagcgatacctttttcgataccttctttcaggatcttggtgttggttacgaacaggtcgtcaccaaccagctggattttgtcgcccagaactttggtctggtatgcgaaaccgtcccagtcagattcgtccagaccgtcttcgatagaaacgatcgggtactgtttggtcagttcttccaggaagtgagtgaattcttcagaggtgaacgctttgttgccttcgccagccagaacgtatttaccatctttgtagaattcagaagctgcgcagtccatcgccaaagtgatgtctttgcccagttcataaccagcagctttaacagcttcagcgataacagccagagcttcagcgttggaacccaggttcggcgcatagccaccttcgtcaccaacagcagtgttcatgcctttcgctttcagaacttttgccaggtgatggaaaacttcagaacccatgcggatggcttctttcacagttttcgcgccaaccggctgaatcatgaattcctggatatcaacgttgttgtcagcgtgctcaccaccgttgatgatgttcatcatcggaaccggcatagagtatttgcccggagtaccgttcagttcagcgatgtgctcgtacagcggcatacctttagcagctgcagcagctttggcgttagccagagatacagccaggattgcgttcgcgccgaatttggatttgttttcggtgccgtccaggtcgatcatgatcttgtcaatgccagcctgatctttagcatctttgccaatcagcgcctgagcgatcgggccgtttaccgcagcaacagctttggttacgcctttacccaggaaacgggatttgtcgccatcgcgcagttccagagcttcacgggaaccagtagaagcacctgacggagcagctgccataccgacgaaaccaccctccagatgtacttcggcttcaacagtcgggttaccacgggagtcgatgatttcacgaccgatgatttttacgattttggacattaggttttcctcaagtcactagttaaactgaaactccagacaaacaacgcgtacccagggtacgcgttgccgctctaacttttttacttacttcgcctgacgtttctggaactcgctggcggctttcacaaagcctgcaaacagcgggtgaccatcacgtggagtagaagtaaactccggatggaactggcaagccacgaaccacgggtgattcggaacttcgatgatctcgaccaactgatcatccccggaacggcccgcaacgcgcagacctgcatcttcaatctgtttcaacagcatgttgttgacttcgtaacggtgacgatgacgctcaacaattgtcggcgcattgtacagctggcgaaccaggctatcgtcaaccaactggcactgctgtgcgccgagacgcatggtaccgccgagatcgctcttctcgctacgaacttcaacgttgccgttttcatcgcgccactcggtaatcagcgccacaaccgggtacttacagtctggcacaaattccgtagagttggcgttctccatgttggcaacatggcgagcgtaatcaattaacgccacctgcatacccaggcaaatgcccagataaggaatattgttctcacgcgcaaaacgcgcggtcgtaatcatgccttctacgccacgatagccgaaaccgccaggtacgaggattgcgtccagacctttaaggatttcaacgccgcgcgtttcaacatcttgtgaatcgatcagtttgatgttgacgctgacacgattcttcagcccaccgtgtttcagtgcttcgatcactgatttataagcatccggcagttcaatgtacttgccgaccataccgatggtgacttcacttaccgggttcgcttcttcgaagataacctgttcccattcggacagattcgcttccgggcagtttaagctgaatcgtttacaaatataatcgtccagcccctgagatttcaacaggcccggaattttatagatggaatcgacgtctttcagagaaataaccgctttttccggaacattacagaacaatgcaatcttcgcacgttcgttcgccggaacagcgcgatctgaacgacaaatcaggatgtcaggctggataccgatggagagcagctcttttacagagtgctgagtcggtttggttttgacttcaccagacgctgccatgtacggcaccagcgtcaggtgcataaacagagtgtgctcacggccaatttcaacagccatctggcgaatcgcttcgaggaacggcaaggattcgatatcacctactgtaccgccgatttctaccagtactacgtcatgaccttcgccaccttccagcacgcgctctttgattgcgttagtgatgtgcggaataacctgcacggttgcgccgaggtagtcaccgcggcgttctttacgcagaacgtcagagtagatacgacccgtggtgaagttgttgcggcggctcattttggtacgaatgaaacgctcgtagtgccccaggtccaggtcggtttcagcgccgtcttcagtaacgaacacttccccgtgttggattgggctcatagtacctggatcgacgttgatgtacggatccagtttcatgatggtcacattgaggccacgggcttcaagaatggctgcgagggaggctgcggcaatgcctttacccagagaggatacgaccccgccggtcacaaaaatatagttcgttgtcatgctgaacctgagaagttaggttgaaaagacgatggaataaccaagacgggaaagcagtatacccgaacatgacctgtgccacaaactttcattatccctcctcttcgccagcgcactattgaaatcaggagtgagaaaatagcccctttggggtaaatgtttttgacgcaaatcaagcgcttgtcatttaaaaaatgacacaaatggcgcttgaccgcgtaattcccttagagatcaatttcctgccgttttacctgttgccagacttcttccattgtttcgaggtcaacacctgtcatttccagtccacgcgcggcaacaatacgctccacttcgcgaaaacgacgctcgaatttttcgttcgctttttgcaatgcgatttctgctttcgtccctaaatggcgagccagattaaccgtggcaaacagcaggtcccccatttcctcctccagtttagcctggtcgacaacagcctgccgcgcttcgtacatcacctcgtcgatctcttcgtagactttatcgactaccggaccaagcgtcgtccaatcgaagccaacgttggcgcaacgtttctggattttttgcgcacgcattaaagccggtaaactacgaggaatatcgtccagcgccgaatgctgcgctttctgcgcgcgctcttcggttttgatttgctcccaacgggcaagcacttcactactgttttcggcagaactatcagcaaaaacatgcggatggcgacgctctaatttatcgctaatagcagcgcaaatatcattaaagtcaaagcgcccttcttcctgagccatttgcgcgtaaaacaccacctggaatagcagatcgcccagttcaccgcgaagatcgtcaaaatcttcacgggcgatggcgtccagcacttcgtaggtttcttcaagggtgtaaggcgcaatggtggcaaatgtctgctctttatcccacgggcagccgttttccggatcgcgcaggcgctgcataatagtgagcaaacggtcgatttgattcattgaattgtcctgaaaattgcgggtctgtcaggtggaaacctgtgaccagaatagaagtgagttagtaacactacccaatcagtacgttaattttggctttaatgagttgtaattcctctggggcaactgttcctttcttcgttgctcctcttgcccgccaggcgatactttttacctgatcagctaacgctacgccatcacgttcctgaccggataaaacaacttcgaacggatatccttttgattgcgttgtacaaggaacacacagacacatacctgttttgttgttgtacatgaaaggactcaggacaacagctggacgatgtccagcttgctcgctaccttttgtcgggtcaaaatcaacccaaatcagatcgcccatatcgggtacgtatcggcttaccattaccagacttccttatctttcggctctccccagtcgatattctcgtggaggttttccggcgtgatgtcgttgaccagttcagcaagcgtaaatacgggctctttacgcactggctcaataattaatttgccatccaccaggtcaatcttcacttcatcatcaatattcagattgagcgcctgcattaacgtagccgggatccgcaccgccggtgaatttccccaacgctttacgctactgtggatcataaccctttcctcaaaccgctatcatatgtagatacagtatatatcaatctacattgtagatacgagcaaatttcggcctaactcccgtgcaaccgacgcgcgtcgataacatccggcacctggttgagtttacccagcacgcgccccagcacttgcaggttgtaaatctcaatggtcatgtcgatggtcgccagttgctgtttggtgtcgctacggctggcaacgccaagcacgttcaccttctcgttggcgagaatggtcgtgatatcacgtaacaacccactacgatcattagctaccacgcggaccaccagcgaatatccggcggagtagctctcaccccataccgcgtcaacaatgcgttctggcgcatgggagcgcagttccgccagttgttcgcaatcggcgcggtgtactgaaataccgcgcccctgggtaatgaagccgacaatctcatctccaggaatcggctggcagcagcgcgcgatgtggtgcatcaggttgccaacaccttcgactaccacgcgaccgttatctttactgcggttttgcggcgtgtagcttttttgctgaagttgcttcagcgcggcggcgtcctgctcttcggcactcggcttattaaattgcgattgcaggaagttcaccatctgattgagacggatatccccgccaccaatcgccgccagcaactcgtcgacatcattgaagttgtaacgcggcagcagatgtttttctgcttctttcaggctgatccccagatgttccagctcgtcgtcaaggatttgccgcccagccagaatgtttttgtcacggtcctgtttacggaaccaggcgtgaattttcgaacgcccacggctggttgtgacgtaaccgaggtttgggtttaaccagtcacggctggggttcggctgtttctgggtgataatttcaatctggtcgcccatctgcagctggtaggtgaacggcacaatgcgcccgccaatttttgccccgatgcagcggtgtccgacatcactgtggatgtggtaagcgaagtccagcggcgttgatcccgcaggcaaatcaacgacatcacctttcggcgtaaagacgtacacccggtcgtcaaagacctgactacgtacttcgtcgagcatttcgccggaatcagccatctcttcctgccacgcaatcagtttacgcagccaggcaatccggtcttcatgtcccgaacgtgcgccgccagcagccgcgccctctttatatttccagtgcgcagcaacacccaactctgcatcttcatgcatctgtttggtgcggatttggatctcaacggtttttccacccggccccagaaccacggtatgaatagactgataaccgtttggtttcgggttagcgacgtaatcgtcaaactcatccggcaggtggcgatagtgagtgtgcactatccccagtgcggcatagcaatcctgtaaacgctcggcgacaatacgtaccgcacgcacatcaaacagctcatcaaaggcgaggttctttttctgcattttacgccagatgctgtagatgtgtttcggacgaccatacacttccgctttaacgccttcagctttcatctcagcgcgcagatgaccaacgaactcttcgatgtagtgttcgcggtcgagacgccgttcatgcagcagtttggcaattcgtttgtattcggttggatggaggtaacggaagcagtaatcttccagttcccatttcagttgtccgattccgagacggttagccagcggtgcgtagatgttggtacactcttttgccgccagtacacgttcatcttccggcgcatcttttacttcgcgcagatgagcaatacgctccgccagtttgatgactacgcagcgaaaatcatcgaccatcgccaataacatccggcgaacgttatcgacctgttcggaggaaacagaatcagtgtgcgtcgctttcagctggcggatcgccgccatatcacgcacgccgtgaataaggttaacgaccgacttaccgacgctctcacgcagcacatcttcgctgactacgttggcatccgccagagggaaaagcagcgccgcccgcagcgtgtcaatgtccatacttaatgtcgagaggatctccaccatctcaacaccacgccacaataacagactggcatccggatgcccctgcgtctgttgcagacaatacgcccaggtttcggctaagcactcacacgacttctggctggtaatacccagacttgcgatccatttttccggatcaaattcaccagccttattgatatgtgcacttcttaccgcaaccatcgtcctctcctttagggaccagacctgccgaaatcggcaaatcgcaactatttaacgcgcgagaaaagtaccatcgattccagatgtcccgtgtgtgggaacatatccagcatcgccagtcgcgcaatggtatatcctgcttttaataacgcttcgctatcccgagccagcgttgcagggttacaggatacataaactatacgaataggttccagttttataatttgctgcataacacctgcggcacctgctcgcgccgggtccagcaacactttatcgaagccgtttttcgcccacggctgctttgtgacatcttcttcaagattttcgtgataaaacgtcacattctgtaagccattaagacgcgcattctgctggcctttttccaccagcgccggaacaccttctacaccgaccacactggcagcttgtgtcgccaatggcagtgtaaagttgcccataccgcagaacagatccagtacgcgatcttcaggttgcacatccagccattccaacgcacgcgctaccattttttggttcacacccgcattgacctgaataaaatcgcgcgggctaaaagttaagcgcaacccgtttgagtcataccagggcatctcaccagagacggtttcgagtatctcactatcgggggcgagatacagatccaggccttcagaatgcgaaaagcgttccagtttttcgcgatctgccgaacttagcggtgcggtatggcgcaaaatcatcagcgtgccgctggttgcctgtaccagttcaacatgaccaagatggcgcatagcttgtaagctgcccagacatgccctgactttgggcagcaatgcttcaagttggggcgctaaaatggggcattgtttgacgtcgacaatgtcactggagcccgctttgcgaaaccccatctgaagttgctgtgttttcggtaagtagttcagacttaaacgcgcgcgacggcgatagccccagggaacatcggcgatcacttcagagacatcgtgtttcattaatcgggcgagtgccgcacttttgcttcgctgctgtaaatccacgctggcgtgttgttgctgacagccaccgcatacgccaaaatgaggacagcgtggcgtttcgcgttccgggctatcgcttaaccggcgtacgactttagcgcgggcatactgttttttatcttcagtaacagtaacttccgcgttttcctgcggcaataatccggggataaatagcgttttgccgttatgtcgcgccacgccctgaccaaaagagtcgaggtcgttgactgaaacggttatgatctgacgcgtcgtcgtgcgtcgttttgcagagtagaattgcgccattggcgagactttctcaatttaacagtgtgaccttaattgtcccataacggaactccatgaccaactacagcctgcgcgcacgcatgatgattctgatcctggcaccgaccgtccttattggtttattgctgagtatctttttcgtcgtgcatcgctataacgacttgcagcgtcaactggaagatgccggtgccagcattattgagccgcttgcagtttctactgaatatggcatgagcctgcaaaatcgcgaatctatcggtcagttaataagcgtactgcatcgtcgccattccgatattgttcgcgcgatttcggtttatgatgaaaataaccgactctttgtcacctccaattttcatcttgatccctcatcaatgcagctcggcagcaacgtgccgtttcctcgccagctcactgtcactcgtgacggcgatattatgatcctccgcacgccgattatttctgagagttactcccccgacgaatcgcccagtagcgatgccaaaaatagtcaaaatatgttgggatatattgcgctggagctggatcttaaatcggttcgcttgcagcaatataaagagatctttatttccagcgtgatgatgctgttttgtatcggtattgcgcttatttttggctggcgcttaatgcgcgatgtaaccggtccgattcgcaacatggtgaataccgtcgaccgcatccgtcgcgggcaactcgacagccgggtggaaggatttatgctcggcgagctggatatgctgaaaaacggtatcaactcgatggcaatgtcgctggctgcttatcacgaagagatgcagcacaatatcgaccaggcgacgtccgatctgcgtgaaacgctggagcagatggaaattcagaacgttgagttagatctggcgaaaaagcgcgcccaggaagcggcgcgtattaaatccgagtttctggcaaatatgtcacacgagctgcgtacaccactgaatggtgttattggctttacccgcctgacgctgaaaacagaattaacaccaacgcagcgcgatcacctgaatacgattgaacgttcggcaaataatttgctggcaattattaatgatgttctcgacttctcgaaactggaagcaggtaagctgattctggaaagtattccattcccactacgcagcacgctggatgaagtcgttactctgctggcacattcttctcacgataaagggttagaactgacgctcaatattaaaagcgacgtgcctgataacgtgatcggcgacccgctgcgattacagcaaatcatcactaacctggtggggaatgcaattaaattcaccgagaatggcaacattgatattctggtagaaaaacgtgcgctgagtaataccaaagtgcagattgaagtgcagattcgggataccggcattggtattcctgaacgcgatcaatcgcgcttattccaggccttccgacaggctgatgccagtatttcccgccgtcatggtggcaccgggctggggctggtgattacacaaaaactggttaatgaaatgggcggcgatatttcgttccatagccagccgaatcgcggttcaactttctggttccacattaatctcgatctgaacccgaacattattatcgaagggccatccacccagtgcctcgcaggtaagcgcctggcctatgtcgaaccaaactccgcagcagcgcaatgcacgctggatattttaagtgaaacgccgctggaagtggtttatagcccaacgttctccgcgctgcctcccgcgcattacgacatgatgttgttaggcatcgcggtgaccttccgcgagccgctaacaatgcaacatgagcgattagcgaaagcggtatcgatgaccgatttcctgatgctggcacttccttgccatgcacaagtcaatgctgaaaaactcaagcaagatggtatcggcgcgtgtctgctgaaaccattaacacctacacgcctgttgcctgccctgacggaattttgtcatcacaaacaaaacacgcttttgcctgtaaccgatgaaagtaagctggcaatgacagtcatggcggttgatgacaaccccgctaacctgaaacttatcggcgcattgctggaagatatggtgcaacatgtggaactttgcgatagcgggcatcaggcggttgaacgggcgaaacagatgccgttcgatttgatcttaatggatattcaaatgccggacatggatggcattcgggcctgcgaactcatccaccaactcccgcatcagcaacaaacgccggttatcgcggtaacggcgcatgcaatggccgggcaaaaagagaagctgcttggcgcagggatgagcgattatctggcgaaaccgattgaagaagagcgattgcataatttgttgttgcgctacaagcctggcagcggtatttcctctcgcgtcgtgacgcccgaagtcaacgaaattgtggtgaacccgaatgcgaccctcgactggcaactggcactacgccaggcagcaggaaaaaccgatttagcgcgcgatatgctgcaaatgttactcgatttcctgcctgaagttcgcaacaaagttgaggaacagctggttggagaaaacccggaaggcctggttgatttgattcataaactgcatggcagttgcggctatagcggtgtgccacgtatgaagaatctctgccaactgatcgaacaacagctacgtagcggtactaaagaagaagatttggaaccggagctgctggaactgttggacgagatggataatgtcgcgcgcgaagccagcaaaattctcgggtaatggatgtcttgtcgagtagcaatcggctttttatgacgctggtttcagattggtgacaaagtgcctgtgtttatgccggatgcggcgttaacgccttatccggcctacaaaaccaattaaattcaatgaattaaaaaatgatgtagacctgatacatagcacaacaggctattttgcgtttagcatcagtctcaaaccggctccagatagagccggttttggttttctgtcttaacgcaccatgcacgggcgcttgttatcgaacgtccagccaggaatcagatactgcattcccatcgcatcgtcacgcgcgccaagcccgtgtttctgatacagctcatgggctttcatcacttgatccatatcgatttctacacccagccccggtttttctggcacctgtaccagcccgcctttgatctcaaacggttctttggtcaggcgctgattgccttcctgccaaatccagtgcgtatcaatagcagtaattttacccggtgcagcggcggcaacatgggtaaacatcgccagggaaatatcgaagtggttgttagagtgtgaaccccaggtcaggccaaattcatggcacatttgcgccacacgtaccgaaccttgcattgtccagaaatgcggatccgccagcgggatatcaacggattgcagggagagcgtatggcccatttgccgccagtcggtggcgatcatattggttgcagtcggtagacctgtcgcgcgacggaactctgccatcacttcacgcccggagaaaccttgctccgcaccacacggatcttctgcataagccagcgaacctttcaggtatttaccgattttaatcgcttcgttcagcgaccaggcaccgttaggatcgagcgtaatacgcgcctgcgggaagcgttgcgccagtgccacaatagactcggcctcttcttccccggccagtacaccgcccttcagtttgaaatcgttgaagccatatttttcatatgccgcttccgccaggcgcaccaccgcatccggcgtcatcgcttcttcatgacgcaggcgataccagtcgcatgagtcatccggctggctttgatacggcagcggcgtggctttgcgattaccgacgaagaacagataaccgagcatttcgacttcgctacgctgttgaccatcgcccagcagcgatgccacgtttacccccagatgctgccccagcagatccagcattgccgcttctatcccggtaactacatgaatagtggtacgtaggtcaaatgtctgcaaaccgcgcccaccagcatcacgatcggcaaaagtattacgcaccagcgtcagaacgtttttgtattcacccagcgttttacctaccaccagcggaatcgcatcttccagcgttttacggattttctcgccgccgggaatttcccctacgccagtgtgaccagaattatctttgataatcacaatattacgcgtaaagaacggtgcgtgtgcaccactcagattcatcagcatactgtcatgacccgccaccgggataacctgcatttcagtaacaacaggcgtcgtaaattgagaactcatatttatgtcctttttcagaatcaatgacggccgaaaacgggacgtttacggtcaaaggtccagccggggatcaggtactgcatcggacctgcgtcgttacgcgcaccgccaggcagacgtttataggcctcatgtgccttttgtacctgttcccagtccagttccacgcccagaccgggcgcatcaggaacggcaatttttccgtttttaatctccagcggattttgggtcaggcgacaatcgccctcctgccaaatccagtgggtatcgatagcggtaggattacccggtgccgccgcgcccacatgggtaaacatcgccagagagatatcgaaatggttattagaatggcagccccaggtcagcccccagtcgtcgcaaagctgcgccacacggactgcaccggaaagcgtccagaagtgcggatcggcaagtggaatatctaccgcattgagcatcaccgcatgacccatttcgcgccagttggtggcgatcatgttagtcgcgacgggcaagccggtcgcccgtcgaaattccgccatcacttcacgtccggagaagccctgttctgcgccgcatggatcttcggcataggtaagaacatcattcagccctttgcataaagaaatggcttcatcaagcagccatgcaccgttgggatcaacggtaatccgcgcatccgggaagcgtttcttcaatgcacgaacagtgtcgatttcttgctcgccaggtaacacgccgcccttaagtttgaaatctttaaagccgtagcgatcctgtgaggcttccgccagacgcacaacggcttcgctgttcattgctttctgatgccgcaactgataccactcatggttgcccggcgtattttccacataaggaagatcggttttggtccgatcaccgatataaaacagataaccgaggacggtaatagcctcgcgttgcttgcctggccctaacagttcgcagaccggaacattcagcgccttacctagcaggtcaagcaaagcggcttccagcgccgccacggcgttaacgcgtaattcaaaggtccaggcacctttaccgaaggtatcaaaatcggcggcctgattacctttatgcacctgctggaccactttattcagtcgcgcaacttcctggcccagaaccatcggaatagcatcgacaagcgtctgataaatcacatctccgcccggcgcttcaccaatgccggtatgcccggcgttatcggtgagtaccacaatattgcgggtgaaatatgcgttatgtgccccaccaatattaagcaacatgctgtcatgcccggccaccggaatgactttcatatcagtaataacaggactggattgtgtcgccatcttattgccccgcaacaggtttcaactcgatacgcttgatatcgcccaccagcaccaggtagctcagtaccgcgattaaggcatgaacaccaacataaatcagcgccccattaaacgagccagtcgtgccaacgatataaccaattgcgattggcgtgacgatgccagaaatgttaccgaacatgttgaacaggccaccggaaagaccgctgatctcttttggcgcggtatctgccattactgcccaacccagcgccccgatgcccttaccgaagaaggccagcgccataaagccgatgatcatccactcaacgttgacgtagttgcagaacaccatcaccatcgacagcaacatgcccattacgatcggtgttttacgcgcaatgttcagcgatcccgtgcggcgcatcagccagtcggaaataatcccacccagcacaccgccgataaaaccgcaaaccgccggaacggaagccacaaagcccgctttcagaatcgacatcccgcgtgcctgcaccagataaaccgggaaccaggtaataaagaagtaagtcagggcgttgatacagtactgaccgatataaacgccgatcatcatccgtgaccctagcagctgtttgatctgcccccacttcacgctgaacggcactttaactttggtgttttgctgatccatattgatcagcgcaccacccgcggcgatgtactccagctctttcttatttacccccggatgttgatttggctcgtggatgactttcaaccagataaagctgatgacaatccccagaccgcccataaagaagaagacgtgtgaccagcccacttcatgcgtcagccagcccataatcggcgcgaagatcaccgttgcgaagtattgagcggagttaaaaatcgacaccgccgttcccctttcctgcgccggaaaccaggccgcaacaatgcgactgttgccggggaaagatggcgcttcagcaagcccgaccaggaagcgcagcgtaaacagggcaacgataatgccgaatccactaaagatatcgacgaagccttgcagcaaggtaaacatcgaccagataaagatcgaccagaagtagacgcgttttgaaccaaaacggtccagcaaccagccaccagggatctgcccgataacataagcccatgagaaagcagagaacacatagcccattcccacgggatcaaggccgatatctttggccatttccgaaccggcgatagagagcgtagcgcggtcgccgtagttgaaggatgtgacgataaacaacatcaccactatccagtaacgagcatttgtgcgtttttccacactgctcgcagcctgacttaaagaactcattgttgcactcctgaaaattcgcgttagccacgctcactctggactgcgacatcgccaggaaatcagaggtgacgtagggtgttttttgccgtttttataggtcgttcgccgaatacggcgcgtgtttatatctggcaatagcagtataaaaagcgcgccatagcggctcaccgtgcaacaacacaacattaatgcgttcaatgaggcccgattttggcattagccctggacggtggaatccacttcacggaaatgaaaacaagaacaagaaaggaagggttaaaacgaagaaataaagaagagtatgaaatggatcgcttgactccaggcaaacgccagtaaaaatccgcgctatgaagcagtttttactggcatttgcctgaaaagattcgattcagcaccgctaaaacgacatttaccgctcgctgaacatatcaggacaacagcgtgccccactgttcgacccacggatttgattccgtttccggttccgggttctcactggcgtcaatcaacagcatttcgccaacccgctgagcgctctgttcctgcaacaaggcatcgaactgtttgccgccattgcagaaattcacataactactgtcgccgagcgcaatcacgccataacgcagattcggctggaagcccagactatctttgattccctgaaagagtggcacaatgctatcaggaaggtcgccctgcccggtcgtggacgtaaccaccagaacatacttatcctgatagggcagccagtcgcttaattcaggatcttcaaataccgttgctttgtggccctgcgcggtcagaatcgcttccgcttcttcggccactaacagtgaattcccgtacatggtgccgacaaaaataccaatttccgccataccgttttctccctggattaggaacttatctctccatcctgacccgatggcgcactgaactcaaccctttcattttcaggaagcagaccgcgccagccaaattgtgataacgcctgcatccaggtgtcgtccaggcccgcgtgaatagtcagcggctcgccagtaaaaggatgcgtcaatgacaactgactggcatgtagcattaaccgctggaggccaaaatgctcagcaccgctgcgattctggcgtaaatcgccatgtttgctatcgccaataatcggatgacgcaaatgggcaagatgtcggcgaagctgatgtttgcgtccggttttcggctccagttccaccaggccgtagcgcgtggtcgggtaacgtccggtcgctaccggcatttctacggtcgccagaccgcgataatgcgtcactgctggctgcgggcctttatcttcgcgggcaaatttatcagcgattttgtccagttcttccaccagtggataatccagcaccgcttcttccatcaaccagccgcgcacaatcgcatggtaacgtttctggatttggtgctgttcaaactgttgtgccagcagccgtccggcctcgctggataatcccatcaacaacacaccagaagtgggtcggtccagacgatgagcagtaaaaacatgctggcctatctggtcacgcacggtttgcatgaccactactttctcgtcgcgatccagccagctgcggtgaaccagccagccggagggtttatttaccgcaaccagccattcatcctgatagagtatttccagcattagctcgcatcatccgcaaaaagagcatccagtttttccagctcagccagaataagcgcgcgttgcggatggtccgtcgccagcgccatttcataatagggtgcaacggcaaaagcgcccggtaacggctgtttgttatctaacaaatcgtgcattcgcgggatcagcacccactgcaaccactccagtggttccatggtgtccataaagaacggttgggtactattaaattgatgcggctggggttcatcgtttcgccagtgctgatgttcacgcagtaacgcttcaagcgcctgcaactggagacgaacgcggtcatgagtggtcataaagcaacctcaataagaaaaactgccgcgaaggatagcaggaataaaaaaagggagcactgtattcacagcgctcccggttcgtttcgcagcattccagctacttttgttgctccctgctcatccttgacaacttttcctctggccttgcggccaatcgttcatcctgaactattgcttcctgctcacaccaccccgatgtgatacttcatcctgaagtgtccctggccttcctgacccaccgaatcatcctgaccggttctcattctccatcctggaggtgtcctttaacgcgtcctgcgtcatcctcttcgcttcatccagaagcctttccctgaaacaccatcctggtgtgtcctgcagaagtgtcatcatcctgatgttcacttcgttgtctgactccctgtcgacgaagatagaatcgtctttttcgcgaagtcttacaaggcgcttacagacaatgccttaaggaaaatttcatatgaaagttaagaattaacaatcaacattttgattttaaatgaaaataacgattcttatctttttaagtattcgcttatttcctggcgatctcctacagagtctgtaagagatctctcacaaccagatggggtatttggattacagaagaggcttaagttgattaaggaattccgcaagatttgaggctaaatgcgtccgtttacgtgttcccagcgtctctttgcacacttcaccggagagattacacaccgagatgacctctaactcttcttccagcgtcgcgataaatagtgtgggcggcagttttagccttttctgagtcaccagatgaccaatcagattttcctgcacccgacggaagtcgtcttcactccaggtttgcagcaatgtcagtttgatatcgccaaactgcgcgtgcatatccccggcaaactgagtcgtataaaaggtatgaattgtgggttgtatcacaatatcaaaagcgcgttcaaccgcgtttacattttgttccccggtaaacggctggggttgccagtatacggcatcttcggtagttgaaataatgcacggtgaaggaacaccgtacagttcctcacttaacggccagcttttatgctcttcatgccacgcatcgcagtagcgtgcagtaaaatctttcagggcttgtgcggtcaaatcgtccactaatttctctcttcacttaaaccagatacacttgtcgtttagtttatctggtttatgacggtgaaacatgtcttcttatgcaaaccatcaggcacttgcgggcctgactcttggaaaatcaaccgattaccgggatacctatgacgccagcctactgcaaggcgttccacgcagcctgaatcgcgacccgctgggtctgaaagcggataacctgccttttcacggtacggatatctggacgctgtatgaactttcctggctgaatgcgaaaggtttgccgcaggtcgctgtcggtcatgttgaacttgattacaccagcgtaaatctgattgagtcgaagagttttaagctctatctcaacagttttaaccagacgcgttttaataactgggatgaggtgcgccagacgctggagcgcgacttaagcacttgcgctcagggtaagattagcgtggcgttatatcgtcttgatgaactggaaggccagccgataggtcattttaatggcacttgcattgatgaccaggatatcactatcgataactatgaattcactactgactatctggagaatgccacctgtggtgaaaaagtagtggaagagacgcttgtcagccacctgctgaaatcaaactgcctgatcacccatcaaccagattggggttcgctccaaattcagtatcgtggacgccaaattgacagagaaaaactgctgcgttacctggtctcattccgtcatcacaacgagttccacgaacagtgcgtggaacgcatctttaatgacctgttacgcttctgccagccagaaaaattgagcgtttacgcacgttatacccgtcgtggcggtctggacattaacccgtggcgcagtaatagcgattttgtcccatcgaccacaagactggttcggcaataaattttttctcaattttgcgtgctggattcacgcagaaggttgtgaaaggtcatcaggcagggctattgtaatcaaagggaatgacgatattcgtcccataaggagtttttcttgattacacatattagcccgcttggctccatggatatgttgtcgcagctggaagtggatatgcttaaacgcaccgccagcagcgacctctatcaactgtttcgcaactgttcacttgccgtactgaactccggtagtttgaccgataacagcaaagaattgctgtctcgttttgaaaatttcgatattaacgtcttgcgccgtgaacgcggcgtaaagctggaactgattaatcccccggaagaggcttttgtcgatgggcgaattattcgcgctttgcaggccaacttgttcgcggtcctgcgtgacattctcttcgtttacgggcaaatccataacaccgttcgttttcccaacctgaatctcgacaactccgtccacatcactaacctggtcttttccatcttgcgtaacgctcgcgcgctgcatgtgggtgaagcgccaaatatggtggtctgctggggcggtcactcaattaacgaaaacgagtatttgtatgcccgtcgcgtcggaaaccagctgggcctgcgtgagctgaatatctgcaccggctgtggtccgggagcgatggaagcgccgatgaaaggtgctgcggtcggacacgcgcagcagcgttacaaagacagtcgttttattggtatgacagagccgtcgattatcgccgctgaaccgcctaacccgctggtcaacgaattgatcatcatgccagatatcgaaaaacgtctggaagcgtttgtccgtatcgctcacggtatcattatcttccctggcggtgtgggtacggcagaagagttgctctatttgctgggaattttaatgaacccggccaacaaagatcaggttttaccattgatcctcaccggcccgaaagagagcgccgactacttccgcgtactggacgagtttgtcgtgcatacgctgggtgaaaacgcgcgccgccattaccgcatcatcattgatgacgccgctgaagtcgctcgtcagatgaaaaaatcgatgccgctggtgaaagaaaatcgccgtgatacaggcgatgcctacagctttaactggtcaatgcgcattgcgccagatttgcaaatgccgtttgagccgtctcacgagaatatggctaatctgaagctttacccggatcaacctgttgaagtgctggctgccgacctgcgccgtgcgttctccggtattgtggcgggtaacgtaaaagaagtcggtattcgcgccattgaagagtttggtccttacaaaatcaacggcgataaagagattatgcgtcgtatggacgacctgctacagggttttgttgcccagcatcgtatgaagttgccaggctcagcctacatcccttgctacgaaatctgcacgtaatctccgctcccccggtgacgtttgttgccgggttttctcgtttttggtcacttactcatcaactcatttcatttgttatatgaatgtttcttaccaccctcacgcgacaaatatcatcacagttaatatgtcatacaatttatgttgcaacgcaaacgtttccctattttcataaaccgtattttatcgctatgaaaaagaaattatcgccatgattaactaaaagtattgattttttcagttcaacctacatatattgcgcgccccggaagaagtcagatgtcgtttaatgggcaaatattgcccttaaattctcttttacttttgatttacagagtaaagcgttgggataatctatcttccaagtagattattgtatttgagatcaagatcactgatagatacataacttgtgtgtatctttccgccctcaaattattacggcggtaaatgattaagccatcgccgatagacagatttcatttttacggtcaggcaccttcccgggctgaactggctaaaagctgaattatttgcattcctccaggagaaatagatggaaacgactcaaaccagcacgattgcgtcgaaagactctcgtagtgcctggcgcaagacagacaccatgtggatgctgggcctttacggcacggcaatcggcgcgggcgtgctgttcctgccaatcaacgccggtgttggcggtatgatcccgctgatcatcatggctatccttgcgttcccgatgacgttttttgctcaccgcggcctgactcgcttcgtactgtctggtaaaaacccgggcgaagacatcaccgaggttgtagaagaacactttggtattggcgcaggtaaactgattaccctgctctacttcttcgctatctacccgatcctgctggtttatagcgtggcaatcaccaataccgttgaaagcttcatgtctcaccagctgggtatgacgccaccgccgcgtgcgattctgtcgctgatcctgatcgtgggtatgatgaccatcgttcgcttcggtgagcagatgatcgttaaagcgatgagtattctggtattcccgtttgttggcgtactgatgctgctggctctgtacctgatcccgcagtggaacggcgctgcactggaaacgctgtctctggacactgcatctgcaaccggaaacggtctgtggatgaccctgtggctggcaattccggtaatggtgttctcgttcaaccactctccgatcatctcttctttcgccgttgcgaagcgtgaagagtacggcgatatggcagaacagaaatgctcgaagatcctggcattcgcacacatcatgatggtgctgaccgtaatgttcttcgtcttcagctgtgtactgagcctgactccggcagacctggctgcggctaaagagcagaacatctcgattctgtcttacctggctaaccactttaacgcaccggttatcgcgtggatggctccgattatcgcgattatcgctatcaccaaatccttcctcggtcactacctgggcgcacgtgaaggcttcaacggtatggtgattaaatctctgcgtggtaaaggtaagtctatcgaaatcaacaagctgaaccgtatcactgcgctgttcatgctggtaacgacctggattgttgccaccctgaacccgagcatcctgggtatgattgaaaccctgggcggtccaatcatcgcgatgatcctgttcctgatgccgatgtacgcaattcagaaagtaccggcaatgcgtaagtacagcggtcacatcagcaacgtattcgttgtcgtgatgggtctgattgcaatctccgcaatcttctactctctgttcagctaagtcctttcgcgccgctttcgggcggcgcttcctccgttttaacgcgatgtatttcctatgattagcgtattcgatattttcaaaatcggcattggcccttccagttctcataccgttggaccaatgaaagcgggtaaacaatttaccgacgatctgattgcccgtaacctgcttaaagacgtgacccgcgtggtggttgacgtgtacggctcgctctctctgaccggtaaaggccaccacactgatatcgccattattatgggcctggcgggtaacctgccggataccgtggatatcgattccatccccagttttattcaggatgtgaatactcatggtcgcctgatgctggcaaacggtcagcatgaagtggagttcccggttgatcagtgcatgaacttccacgccgacaacctttctctgcatgaaaacggtatgcgcattaccgcgctggcgggcgataaagtcgtttacagccagacttactactctattggcggtggctttatcgttgatgaagagcattttggccagcaggatagcgcaccggttgaagttccttatccgtacagttcagcagccgatctgcaaaaacattgtcaggaaaccgggctgtcactctctggcctgatgatgaaaaacgagctggcgctgcacagcaaagaagagctggaacagcacctggcgaacgtctgggaagtcatgcgcggcggtattgagcgcggtatttccaccgaaggcgtgttgcctggcaaactgcgcgttccacgccgtgctgcggcactacgccggatgctggtcagccaggataaaaccaccactgacccgatggcggttgttgactggatcaacatgtttgcactggcagtgaacgaagagaacgctgctggcggtcgcgtggtgactgcgccgactaacggtgcgtgcgggattatcccggcagttctggcgtactacgacaagtttatccgcgaagtgaacgctaactcactggctcgttacctgctggtagccagcgccattggttctctttataagatgaacgcgtcgatttctggtgctgaagtgggttgccagggtgaagttggcgtggcgtgctcaatggcggcggctggtctggcagaactattaggcgcaagcccggcgcaggtgtgcatcgcggcggaaatcgccatggagcacaacctcggtctgacgtgtgacccggtcgccggacaggtacaggtgccatgcatcgagcgtaacgccattgcggcagtaaaagcggtgaacgccgcacgtatggcgctgcgccgtaccagcgagccgcgcgtctgcctcgataaagttatcgaaaccatgtacgaaacaggtaaagatatgaacgccaagtaccgcgaaacctctcgcggcggcctggcaatgaagatcgttgcctgcgattaatcgctctccaaaggcctcgttttgcgaggcctcttcccgatttctcatccagccgtagcctgttccggcatcgaatgttacccttatcgcctgatctttaagggggttatcgtggctgttcatttgcttattgtcgatgcactgaatcttattcgtcgcattcatgccgttcaggggtcgccctgtgtcgaaacctgccagcatgcgctcgatcagctcattatgcacagccagccaacccacgcggtcgccgtttttgatgatgaaaaccgcagtagcggctggcgtcatcagcgtttaccagattacaaagcgggtcgaccgccaatgccggaagagttgcacgacgagatgcctgcattacgcgccgcctttgagcaacgcggcgtcccgtgctggtcaaccagcggcaacgaagccgatgacttagccgccacgctggcggtcaaagtgacacaggccgggcatcaggcaacgattgtttcgacagataaaggctactgtcagttactttcaccgacattacgtattcgtgattacttccagaaacgttggctggatgcgccatttatcgataaagaatttggcgttcaaccgcagcagttgcccgattactggggacttgcggggatcagcagttcaaaggtaccgggtgttgcgggaatcggaccaaaaagcgccacgcagctgctggtcgagtttcagagtctggaagggatatatgagaatctggatgcggttgccgaaaagtggcgcaaaaaattagaaacccataaagagatggcgtttctgtgccgcgatattgcccgcttacaaaccgatttgcatatcgacggcaatttacagcaattgcggttggtacggtaacggcgagccggatacgccgcaaacgtcgtatccggcattatcacatcagcgcatttaccaggcggtatggtaaagctctacaatatcctcaagcgttgcttcacgcgggttgccaccggtacaaacatcatccagtgccgcctgcgccagtgccggaatgtcttccttgcgtacaccaacatcacgcaaatgtggcggaataccgacatcacggttgagagcaaacaccgcttcaacagcggcattacgcgcctcttccaggctcataccttccactttcacgcccataacgcgcgcgatatcgcggtacttctcaccggtaaagtcagcgttataacgcatgacatgcggtaacaggatggcgttcgcaacaccgtgtggagtgttataaaacgcgcccagtggatgcgccataccatgcaccaaccctaacccaacattcgagaagcccatacccgcaacatactgcccgagcgccatttcttctccggcatccttatcaccagcaaccgatcctcgcagcgccccagcaatgatttcaatcgctttaatgtgcagtgcatcggttagcgcccacgcgccacgggtaatatacccctcaatagcatgagtgagcgcatcgacacccgtcgcagctttcagcgctggaggcataccatccatcatgtcagcgtcaataaacgccacctgcgggatatcatgcggatcaacgcaaacaaacttgcgccgtttctcttcgtcagtgatcacgtagttaatggtcacttctgccgcagtacctgctgtggtaggaattgccagaatcggtacactgggtttattggtcggggaaagcccttccaggctacgcacatcggcaaactccgggttgttgctgataatgccaatcgctttacaagtatcctgtggagaaccaccaccaatagcgatcaggtaatccgcgccgctattctggaatacaccgagcccttctttgacgacagtaattgttgggttgggcactacgccgtcgtaaatcgcccatgccagccctgcagcatccatcttatcggtcactttcgccaccacgccgcattgcaccagcgttttatcggtgacgatcagcgccttctgataaccacggcgtttcacctcatcggttaaagccccaacagcaccccgaccaaaccatgccgtttcgttcagaatcattctgttagccatcatccttctccttgttgctttacgaaattactcttcaattcgtaacccataggttttgaatttctccagcactacggcaatctcttcatcgctcagcactggcaccgggtccgtaatcgccagggtcgtcaggtaaagttgcgccagcacttcaacttcatgcgccagccataacgctttttccagattcacctcacaagcgataagcccatgatgttgtaacaaagttgccttacgatttttgagagccagcgcaacatgttcagaaagttcgcgtgttccaaaggtcgcataaggcgcgcaaggaatagaattaccgccagccgccgcaatcatgtagtgaatagcggggatcgatcggttaagaatggaaactgccgtgcaatgaacggcatgattgtgaacaaccgcgttggcatccggtctgctttgataggctgccatatggaaacgccattcgcttgaggggagctttccttcctcatgtttaccgttgccatcaataaagacaatatgcgactccgtcagtttttcatatggaatgcctgtaggcgtaatcagcatcccatcctgataacgtacactgacgttccccgctgtcccctggttcagtcccaggcgggtcatttccaggcaagtgtcaataatctgacgagcaagtttatttcgttccattagctacctctctctgattcaaaacagggcaataatgttgttcctttcacactattgaattagccgtttaattacccaccatcttcttcctgattaacaagaaagaaattcacaagcttatattttgtgacctggttcaactaatcacagtaaataactgcaagttctctttttataaccccattaaaaatgaccgctcttaaaaatatttatcaaaacggtcatttttctattcctccaagcccggaatgaccgttttcggcacaaacaattaatacggtcatctgatttgtgttttttatgatttattttctgaaacgggcatgaaatttcgattattaaagtgatggtagtcacataaagtcaccttctagctaataagtgtgaccgccgtcatattacagagcgttttttatttgaaaatgaatccatgagttcatttcagacaggcaaatattcactgatatgaagcccgaactcgctggttttgcacttttgaaaacataaccgattacgtgcttaagcttctgaacctaagaggatgctatgggaaacacatcaatacaaacgcagagttaccgtgcggtagataaagatgcagggcaaagcagaagttacattattccattcgcgctgctgtgctcactgttttttctttgggcggtagccaataaccttaacgacattttattacctcaattccagcaggcttttacgctgacaaatttccaggctggcctgatccaatcggccttttactttggttatttcattatcccaatccctgctgggatattgatgaaaaaactcagttataaagcagggattattaccgggttatttttatatgccttgggtgctgcattattctggcccgccgcagaaataatgaactacaccttgtttttagttggcctatttattattgcagccggattaggttgtctggaaactgccgcaaacccttttgttacggtattagggccggaaagtagtggtcacttccgcttaaatcttgcgcaaacatttaactcgtttggcgcaattatcgcggttgtctttgggcaaagtcttattttgtctaacgtgccacatcaatcgcaagacgttctcgataaaatgtctccagagcaattgagtgcgtataaacacagcctggtattatcggtacagacaccttatatgatcatcgtggctatcgtgttactggtcgccctgctgatcatgctgacgaaattcccggcattgcagagtgataatcacagtgacgccaaacaaggatcgttctccgcatcgctttctcgcctggcgcgtattcgccactggcgctgggcggtattagcgcaattctgctatgtcggcgcacaaacggcctgctggagctatttgattcgctacgctgtagaagaaattccaggtatgactgcaggctttgccgctaactatttaaccggaaccatggtgtgcttctttattggtcgtttcaccggtacctggctcatcagtcgcttcgcaccacacaaagtcctggccgcctacgcattaatcgctatggcactgtgcctgatctcagccttcgctggcggtcatgtgggcttaatagccctgactttatgcagcgcctttatgtcgattcagtacccaacaatcttctcgctgggcattaagaatctcggccaggacaccaaatatggttcgtccttcatcgttatgaccattattggcggcggtattgtcactccggtcatgggttttgtcagtgacgcggcgggcaacatccccactgctgaactgatccccgcactctgcttcgcggtcatctttatctttgcccgtttccgttctcaaacggcaactaactgaacatattttccgaataaagtgaggaatctgtaatgaaaaaaatcagcttaccgaaaattggtatccgcccggttattgacggtcgtcgcatgggtgttcgtgagtcgcttgaagaacaaacaatgaatatggcgaaagctacggccgcactgctgaccgagaaactgcgccatgcctgcggagctgccgtcgagtgtgtcatttccgatacctgtatcgcgggtatggctgaagccgctgcttgcgaagaaaaattcagcagtcagaatgtaggcctcaccattacggtaacgccttgctggtgctatggcagtgaaaccatcgacatggatccaacccgcccgaaggccatttggggctttaacggcactgaacgccccggcgctgtttacctggcagcggctctggcagctcacagccagaaaggcatcccagcattctccatttacggtcatgacgttcaggatgccgatgacacatcgattcctgccgatgttgaagaaaaactgctgcgctttgcccgcgccggtttggccgtcgccagcatgaaaggtaaaagctatctgtcgctgggcggcgtttcgatgggtatcgccggttccattgttgatcacaacttctttgaatcctggctgggaatgaaagtccaggcggtggatatgaccgaactgcgtcgccgtatcgatcagaagatttacgacgaagccgaattggaaatggcactggcctgggctgataaaaacttccgctatggcgaagatgaaaataacaaacagtatcaacgtaatgccgagcaaagccgcgcagttctgcgcgaaagtttactgatggcgatgtgtatccgcgacatgatgcaaggcaacagcaaactggccgatattggtcgcgtggaagaatcacttggctacaacgccatcgctgcgggcttccaggggcaacgtcactggaccgatcaatatcccaatggtgacaccgccgaagcgatcctcaacagttcatttgactggaatggcgtgcgcgaaccctttgtcgtggcgaccgaaaacgacagtcttaacggcgtggcaatgctaatgggtcaccagctcaccggcaccgctcaggtatttgccgatgtgcgtacctactggtcaccagaagcaattgagcgtgtaacggggcataaactggatggactggcagaacacggcatcatccatttgatcaactccggttctgctgcgctggacggttcctgtaaacaacgcgacagcgaaggtaacccgacgatgaagccacactgggaaatctctcagcaagaggctgacgcttgcctcgccgctaccgaatggtgcccggcgatccacgaatacttccgtggcggcggttactcttcccgcttccttaccgaaggcggcgtcccgttcaccatgactcgtgtcaacatcatcaaaggcctgggaccggtactgcaaatcgcggaaggctggagcgtggaattgccgaaggatgtgcatgacatcctcaacaaacgcaccaactcaacctggccaaccacctggtttgcaccgcgcctcaccggtaaagggccgtttacggatgtgtactcggtaatggcgaactggggcgctaaccatggggttctgaccatcggccacgttggcgcagactttatcactctcgcctccatgctgcgtatcccggtatgtatgcacaacgttgaagagaccaaagtgtatcgtccttctgcctgggctgcgcacggcatggatattgaaggccaggattaccgcgcttgccagaactacggtccgttgtacaagcgttaatacattactccctgatgtgatgcccggtcgctccggctaccgggcctgaacaagcaagagtggttagccggataagcaatgttatccggctatattgcaggagcgattatgaaacaagaagttatcctggtactcgactgtggcgcgaccaatgtcagggccatcgcggttaatcggcagggcaaaattgttgcccgcgcctcaacgcctaatgccagcgatatcgcgatggaaaacaacacctggcaccagtggtctttagacgccattttgcaacgctttgctgattgctgtcggcaaatcaatagtgaactgactgaatgccacatccgcggtatcgccgtcaccacctttggtgtggatggcgctctggtagataagcaaggcaatctgctctatccgattattagctggaaatgtccgcgaacagcagcggttatggacaatattgaacggttaatctccgcacagcggttgcaggctatttctggcgtcggagcctttagtttcaatacgttatataagttggtgtggttgaaagaaaatcatccacaactgctggaacgcgcgcacgcctggctctttatttcgtcgctgattaaccaccgtttaaccggcgaattcactactgatatcacgatggccggaaccagccagatgctggatatccagcaacgcgatttcagtccgcaaattttacaagccaccggtattccacgccgactcttccctcgtctggtggaagcgggtgaacagattggtacgctacagaacagcgccgcagcaatgctcggcttacccgttggcataccggtgatttccgcaggtcacgatacccagttcgccctttttggcgctggtgctgaacaaaatgaacccgtgctctcttccggtacatgggaaattttaatggttcgcagcgcccaggttgatacttcgctgttaagtcagtacgccggttccacctgcgaactggatagccaggcagggttgtataacccaggtatgcaatggctggcatccggcgtgctggaatgggtgagaaaactgttctggacggctgaaacaccctggcaaatgttgattgaagaagctcgtctgatcgcgcctggcgcggatggcgtaaaaatgcagtgtgatttattgtcgtgtcagaacgctggctggcaaggagtgacgcttaataccacgcgggggcatttctatcgcgcggcgctggaagggttaactgcgcaattacagcgcaatctacagatgctggaaaaaatcgggcactttaaggcctctgaattattgttagtcggtggaggaagtcgcaacacattgtggaatcagattaaagccaatatgcttgatattccggtaaaagttctcgacgacgccgaaacgaccgtcgcaggagctgcgctgttcggttggtatggcgtaggggaatttaacagcccggaagaagcccgcgcacagattcattatcagtaccgttatttctacccgcaaactgaacctgaatttatagaggaagtgtgaaatgctgaaaacaatttcgccgttaatttctcccgaactattgaaagtgctggcagagatgggacatggagatgaaattattttttccgatgctcactttcccgcccattcgatgggaccgcaggtgatccgcgctgatggcctgttggtgagcgacttgctccaggcgattatcccgttatttgaactggacagttatgcaccgccgctggtgatgatggcggcggtagaaggtgacactctcgatcctgaagtagaacgacgttaccgtaatgcgctttcactacaagccccgtgtcctgacatcatccgcatcaatcgttttgcgttttatgaacgggcgcaaaaagcctttgcgatcgttatcacaggcgaacgagcgaagtacgggaatattcttttaaaaaaaggggtaacaccgtaatctcataccggtacgcccgcatgacgcgggcggttatcgaatgatggggtgaaaaatatgaaagcggcacgccagcaagcgatagtcgacctgctgctgaaccataccagcctgaccacggaagctctctctgaacagctaaaggtcagtaaagaaaccattcgtcgcgatctcaatgaattacagacgcagggtaaaattctgcgcaatcatggacgcgctaaatatatccaccgtcaaaatcaagacagtggcgatccctttcacatcaggctgaaaagccattatgcgcataaagcagatatcgcgcgcgaggcgctcgcgtggattgaagaagggatggtgatagccttagacgccagttcaacttgctggtatctggcacgccagttgcctgacatcaacattcaggtcttcaccaatagccatccgatttgccatgaactcggtaaacgcgaacgcattcaactgatcagttccggcggcacacttgagcgcaaatatggctgttacgtcaatccctcgctgatttcccaacttaaatcgctggaaatcgatctgtttattttttcttgtgaagggatcgatagcagcggcgcactgtgggactccaatgcgatcaacgctgattacaaatcgatgctattaaaacgtgccgcgcaatcgttgttattgattgataaaagtaaatttaatcgttcaggggaagcccgcatcgggcatctggatgaggtaacgcacattatttctgatgagcgccaggttgcaacttctttggtaacagcctgacggaaagggtagcaggccggagacgacgccccggccttgcctgttatcgctcgtcgcgacgaccacccaccgcagcccagatgcggcggacgtgcaccgtcacttcttcgcgatcgtgatacaactgccgcgcctgaatctgagcatttatgccatgttcatcaagctgtgcctgaatatacgccagattgtgtgacacttcttcgtagcgttttttcatcggcagtttgaggttgaaaatggtttcacggcaccagccattaaccagccactgcgccatcaatgccgcaactttcgccggtttttcaaccatatcgcataccatccaggagatattgctgcgcgtcggacggaatttgaaaccgtcttcccgcagccacgtcacctgtccggtatccatcagactttgcgccatcgggccgttgtcgacggaataaacccacatgttgcgcttcaccagttggtaggtccagccgccagggcaagcgcctaaatccaccgcccacatcccgttcgccaggcgttcatcccactcatccgcaggaataaacacatgaaatgcctcttccagtttgagcgtggaacgactcggcgcatctgccggaaatttcaggcgcggaatgcccatatagaacggcgaattattgttgctgtatgagtaaccggtatagcagcagcctggtgcaataaagaatacatgcacaaccggacgcttcggcgtttcatagttcgccagcaccccggcatcgcgcaaggcagcgcgtagcggaacagtaaatttacggcagaatttcagtaactctttgctttcgttggtatcggcaacttcaacacgcagttcaccgcccttctctactacgccctgtaacatgccgacaatgggggtaatacgatcttctggcggcaaatgctgcaggagttcccccaccacaaaccactggcgggcaaaaattaatgaactgaacggcagctcacggattaacttatcgccatcatcaggttgataacattcataaatgacataacccgcattctctttcacgcgggcaaaaccgaaaatttcccgctggccggctttatcggtaatttctgcggcgcactctttttcaaagcccggacggcacagcaatacaaccttattcatgacttacgcccttgcgctttaaacggatagcaccaactaacattaacgcccagcccgcgaggaagctcacgccgccaaccggagtgacaaacgcccacaaacgcagatgggacagcgccaggcaataaaggctgccgctgaacaacaccgtgcctaacgcgaggaaaacgctactccagtaaaaccagatactgatgcgacgctgcattgccaccgccagacctaagatcgccagcgtatgaaacgcctggtattcgaggccggtctggatccagcccatctcaacggcccccatggttttacttaacacatgcgcgccaaaagcgcccagagccacaaaaatgaagccgctaatggcggcgaaaatcagcataaaacggctggtcatggtcgtaccctacgtaaattattgttcataacgaaagcggaatttttcttgttcagcagcggctttcgccaggatccattggcgaaaggcggctattttacccagttctgcctgactgtcatgacaaaccagataaaaagcatttttactgaccagaacatcattaaacgggcaaacaagacgtccggcctcgatttcagattgcgccatcacgttatttgccagcgccactccctgcccgtggatagccgcttgcagcaccatggcgctatggctaaaaattggcccttgctgaacgttgatatgatttaaccccaactgtcgggtatatgtctgccagtcacggcgcgaagcatcatgtaataacgtatgtttagccagatcttccggtgtcttcaagggtttttcgccagtcagcagtagcggcgaacacaccggcaataaatattcggcgtacagtttttccacccgtagccccggccagttgccccgaccataaaatatcgccacatcaacatcatccgccagcttatcttcctgacgatcaaccgcctggattcgaacgtcaattcccggataagctgaattaaagctggaaagtcgcggaaccaaccaatgaatggcgaaactggggagtaaactgaccgtcaacgcccccttggcgctacgggcctggagtttacgcgtcgcttcggttaattgcgaaaatatctctttgatatcgaggaaatagctttgcccttcctcggtcagcaggagtgaacgattacggcggcggaacagttttagccccaaaaaatcctcaagagacttgatttgatgacttactgcggcttgggtcacaaaaagctcttctgctgcgcgagtgaaacttaaatggcgtgctgcggcatcaaaaactcgtaaggcatttagcggtggtaatcgtttagacatggctattaaactttgatgttaaatgaatttaacaattagatcacactatgtaacctattagtttttttaatctgagccattataaattgtccgttgagcttctaccagcaaatacctatagtggcggcacttcctgagccggaacgaaaagttttatcggaatgcgtgttctggtgaacttttggcttacggttgtgatgttgtgttgttgtgtttgcaattggtctgcgattcagaccatggtagcaaagctaccttttttcacttcctgtacatttaccctgtctgtccatagtgattaatgtagcaccgcctaattgcggtgcttttttttaccttgcgatcgcgaattactgatccagttcgaccatctctttcacgtcagtacggttgatctgctgtttgttgccattagcgtctttatacgaaatcataccggtatcgttatcagtctgtggtttgccgtcagagacgatggtacgtccgtcattggtgtgcatcacatagttcgaaccggaacaggcgctcagggcaaaagtcagcatacaggcagaaataattgcggcagtctttttcatcatcttctccttaaagcgattaataaatcttaatagtattgattaacaggctaaaattaacgcctaacactattcagcatatgttacttacgcggcttcgccaggatatccagataattctgatggttagcactctccttgtatcaaagtgaattttgcgtcacgatcggtgcatcaagccgaggagtaccatgaacgtttttaatcccgcgcagtttcgcgcccagtttcccgcactacaggatgcgggcgtctatctcgacagcgccgcgaccgcgcttaaacctgaagccgtggttgaagccacccaacagttttacagtctgagcgccggaaacgtccatcgcagccagtttgccgaagcccaacgcctgaccgcgcgttatgaagctgcacgagagaaagtggcgcaattactgaatgcaccggatgataaaactatcgtctggacgcgcggcaccactgaatccatcaacatggtggcacaatgctatgcgcgtccgcgtctgcaaccgggcgatgagattattgtcagcgtggcagaacaccacgccaacctcgtcccctggctgatggtcgcccaacaaactggagccaaagtggtgaaattgccgcttaatgcgcagcgactgccggatgtcgatttgttgccagaactgattactccccgtagtcggattctggcgttgggtcagatgtcgaacgttactggcggttgcccggatctggcgcgagcgattacctttgctcattcagccgggatggtggtgatggttgatggtgctcagggggcagtgcatttccccgcggatgttcagcaactggatattgatttctatgctttttcaggtcacaaactgtatggcccgacaggtatcggcgtgctgtatggtaaatcagaactgctggaggcgatgtcgccctggctgggcggcggcaaaatggttcacgaagtgagttttgacggcttcacgactcaatctgcgccgtggaaactggaagctggaacgccaaatgtcgctggtgtcataggattaagcgcggcgctggaatggctggcagattacgatatcaaccaggccgaaagctggagccgtagcttagcaacgctggcggaagatgcgctggcgaaacgtcccggctttcgttcattccgctgccaggattccagcctgctggcctttgattttgctggcgttcatcatagcgatatggtgacgctgctggcggagtacggtattgccctgcgggccgggcagcattgcgctcagccgctactggcagaattaggcgtaaccggcacactgcgcgcctcttttgcgccatataatacaaagagtgatgtggatgcgctggtgaatgccgttgaccgcgcgctggaattattggtggattaatgacaaacccgcaattcgccggacatccgttcggcacaaccgtaaccgcagaaacgttacgcaataccttcgcaccgttgacgcaatgggaagataaatatcgccagttgatcatgctggggaaacagcttccggcattgccagacgagttaaaagcgcaggctaaagagattgccggatgcgaaaaccgcgtctggctgggatatacagtggctgaaaacggcaaaatgcatttctttggcgacagcgaagggcgcattgtgcgcggcctgctggcggtgttgttgactgccgttgaggggaaaaccgccgccgagttgcaggcacagtcaccactggcattgtttgatgagctgggattacgtgcgcagcttagcgcctcacgcagccaggggttaaatgcgttaagcgaggcgattatcgctgcgacgaagcaggtttaagcacagaaccgggtcggataagacgttcgcgtctcatccgacctgattgtttaaccctgacgcgccgctttcgccatcatcttcttcagcgcatgagaaaccgcaacaaacccaaaggtggcggtcaccatcgttgccgcgccaaatccagatgcacaatccatccgcttcggcccttctgccgtggctttcatcgcacacaccgtaccgtctgactgcgggtacaccagcgcttcagtagaaaacacgcaatccacgccgagcttacctttactgtttttcactacgccaaaatcgcttttcaggcgctcgcgcaacttcgccgccagcgggtcctgaatcgttttcgccagatcggtaacctgaatctgcgtcggatcaatctgcccacccgcgccaccggttgtgaccagtgggattttattgcgccgacaataagcaatcagcgccgctttgggccgtacactatcaatggcatcaatcacgtacgaataacccacgctcatatactgcgctacgttatccggcgtcacgaaatcatccaccaccgttacacggcactccgggttaatctggcgaatacgctccgccataacttccgcttttgccagcccaacgttatcgcgcagggcatgaatttgccgattggtattggtgacgcacacatcatccatatcgataagcgtgattgcgccaatccccgtgcgcgccagcgcttccgccgcccaggaaccgacaccaccgataccaaccacacaaatatgcgcgtcagcaaacagttgcaacgctttttcaccatacagacgcgctgtgccaccaaaacgctgacgccatgcatcactaattaccacagacatagcacctcagaattaaaaagggcgaggttatccctcaccctaaacgcataaatgcctgatgcgctacgcttatcaggcctacataactcctgcaatattttggatttgcatgatttgtaggccggataaggcgttcacgccgcatccggcatgaacaacgcgcacttagtcaataatcaggatgtgaggttacccctcaccctgtcatatccgtaaaaacggcatacagaatatcacatcagccgctaaagacgttacctgcgcccggggcggttttcagcacccagacacgtccatagtggttgtaccaacctgcgcggtgtccggcttccggcccgatcccttgatagatatcgaagtgttggcctttgattgcaccaccgacatccagcgccaccatcagacgcagttcgtactgaccattaaatttgccgttattatccagcaacggcacttctgccagcaaggtagtacctggcggaataatggaacgatcagaggcaactgacgcgcgaccaaccagcggcaccgcacttgcccctttcaccggagcaaaagattgcggtttaaagaagacgaaagacgggttctgttccagcagctcgcgaacctcggcttcactgtgtgtttcgccccagtgacgaatcgcctgcatcgacatatcttcttttttcacttcgccacggtcgatcagcaccttaccaatgctgcgataggcatgaccgtttttccctgcatagctgaaaaagttaagcggactgccatcaccaaagtcgatatacccactaccctgcacatccataatgaagttatccatcagggagttactgtaagcgagaatatatttatcactcaatgcccccgcgtagatctccgcacgagacggcagacgaccacgttttggcggcatacggtaaataggatactggaactcgccctggcgggtatggcgcgcctgaattaccggcgtgtaataaccggtaaactgcacgttaccatagttgtcggcaccttccatctgccaggcatcaatgccgaactggcgcatattgcgggtatcaccgcctgcgcgcagccactcttgcaccgcgttataaacattactctggttgccatacagacgcggtgacgaattacggatatggttaatttgctcggcaaaatcaccggcgttaatcggcgcgccaacggcatctggctggttcaccagagagaaaggctgggtaaatttcccgtctttatattgctgtccgcgatcggttggtttggaagagcaggcggcaagcattgccacaaccgtgcccataagaaggtactttacccaacgtcctttcattgttctcttcttcaggttaaaaaataaggcgcaacgaagataacaaaccgccgcgtttaatgaaatgagcagcctctccctgacgcaaattttgcacaaaaaataggctttagtgatttgtttttgttcaaaatcatgccaaatccgtgatcggggtaaaaaaaaggttgcatgaaaacgcgagcggagtatagtgcgcatccacggacgcggggtggagcagcctggtagctcgtcgggctcataacccgaaggtcgtcggttcaaatccggcccccgcaaccaattaaaatttgatgaagtaaagcagtacggtgacgcggggtggagcagcctggtagctcgtcgggctcataacccgaaggtcgtcggttcaaatccggcccccgcaaccaatcaaatttgatgaagtaaaagcagtacggtgacgcggggtggagcagcctggtagctcgtcgggctcataacccgaaggtcgtcggttcaaatccggcccccgcaaccaattattgaacaccctaacgggtgtttttttgtttctggtctcccataaaaaagcgccattcagcgcctttttatcatccccttctcgccagcgtcgccccatcggcaaaatacgctttaatccccgcaagaatagactccgcaacttcctgctggaaagtcgccgttttcagtttacgctcttcctcaacgttactgataaacgccgtttcgaccagaatggagggaatatctggtgcctttagtacggcaaacccggcctgttcaacttgatttttatgcagcttgttgattttaccgagcttattcagtaccgctttaccaaacttcaggctgtcggcaatggtcagcgactgtaccatatcgaacatggtgtggtcgacatagcggtcaccgcttttgctcacgccaccaatcaagtccgaggcgttctgggtttgtgccagatattttgccgcagtactggttgcacctttggttgagagcgcaaacacagaggaaccgctcggctgacgactggtaaaggcgtcggcatggatagagacaaacaggtcagcacgctgtttctgggcttttgctacgcgcacttgcaatggaatgaagatgtcttcattgcgcgtcatgtacaccttcatattgccctctttctcgatcagagagcgcaaacggcgagctatttgcaataccacatctttttcgcgcgttttgtatttccccaccgcaccggagtcttcgccaccgtggccagggtcaagcataatgacaatcggacgatcgcgccctgctttacccggttgtggaccactttgcgctggcggcacctgcttttcgaggtcgcctttgttgtaatcctccagcagcgccagcagcgggtcctgcatatcctgtgcattggccggatagaggtccatcaccagacgctctttaaacccggcgaccggcgcaagggcaaacagctgcggttttacgttttgctttaattcaaaaaccatccgtacggtttgcgggtcaaattgcccgacgcgcgccgacttgatgaacgggtcgtctgcacgaatttgtgccgccatccccttgagtaccgagttcaggtttacatcttcgatatccaccaccacgcgttcagggttactcaacgcgaactgcttatatttcagctgacgatttgattccaccgtcacgcgggtgtagctggacgcaggccagacgcgcaccgccacgacctggctgaccgcagccagactgacctgacttacgctcaatagccacatggcacccgcgccttgcagtaaacgacgacggctgattgcagtgttggatcctgacatgcctctcccgagcaaaagaaatctaagctgtgtaacaagtaaacgactaatttgaccggaaactttagcgaaagacgcataatctgtcatctaataaacggtaaacattctttttatattcacggcattactgataaaaaagtcgctctcgcataaaatttacacttgcaccctgcgaaaaaacagaataaaaatacactaatttcgaataatcatgcaaagaggtgtgccgtggtaaaggaacgtaaaaccgagttggtcgagggattccgccattcggttccctatatcaatacccaccggggaaaaacgtttgtcatcatgctcggcggtgaagccattgagcatgagaatttctccagtatcgttaatgatatcgggttgttgcacagcctcggcatccgtctggtggtggtctatggcgcacgtccgcagatcgacgcaaatctggctgcgcatcaccacgaaccgctgtatcacaagaatatacgtgtgaccgacgccaaaacactggaactggtgaagcaggctgcgggaacattgcaactggatattactgctcgcctgtcgatgagtctcaataacacgccgctgcagggcgcgcatatcaacgtcgtcagtggcaattttattattgcccagccgctgggcgtcgatgacggcgtggattactgccatagcgggcgtatccggcggattgatgaagacgcgatccatcgtcaactggacagcggtgcaatagtgctaatggggccggtcgctgtttcagtcactggcgagagctttaacctgacctcggaagagattgccactcaactggccatcaaactgaaagctgaaaagatgattggtttttgctcttcccagggcgtcactaatgacgacggtgatattgtctccgaacttttccctaacgaagcgcaagcgcgggtagaagcccaggaagagaaaggcgattacaactccggtacggtgcgctttttgcgtggcgcagtgaaagcctgccgcagcggcgtgcgtcgctgtcatttaatcagttatcaggaagatggcgcgctgttgcaagagttgttctcacgcgacggtatcggtacgcagattgtgatggaaagcgccgagcagattcgtcgcgcaacaatcaacgatattggcggtattctggagttgattcgcccactggagcagcaaggtattctggtacgccgttctcgcgagcagctggagatggaaatcgacaaattcaccattattcagcgcgataacacgactattgcctgcgccgcgctctatccgttcccggaagagaagattggggaaatggcctgtgtggcagttcacccggattaccgcagttcatcaaggggtgaagttctgctggaacgcattgccgctcaggcgaagcagagcggcttaagcaaattgtttgtgctgaccacgcgcagtattcactggttccaggaacgtggatttaccccagtggatattgatttactgcccgagagcaaaaagcagttgtacaactaccagcgtaaatccaaagtgttgatggcggatttagggtaagcgatgaaaatcgtcggatgcgacatgcgtaacactcgtacgtcgcatccggcaattacgtttattcccgtgaactaaacaacgccgccagaccactgcgccgctcagtacgagtggcgattgccgcacttaatatgcgctcatcggcatacagcgacagacggcgacgcgcgcgggtcaccgcggtataaaccagctctcgcgttactaccggcgtgcgttggctcggcaaaatcaacgccgcatggtcgaactccgatccctgcgatttatgtaccgtcatcgcccacgtagtttcgtgctctggcaagcgactcggttgcacagacttaatattgccgtccggcatcgcaaaccagacgcgcgtcccctgcccgcgatccagcgcaataccgatatcgccattaaacaacccaagcgcgctgtcattacgggcaatcatcaccggtcgaccttcgtaccaacgagagtgcggatgacgatgaattttgcgcttctgttgcataaactgctcaattcgctcattcagtccagccacgccaaacggcccttcccgcagggcgcacaaaagctggtactcattgaacgcctgaatgattaaatccggctcggcacgcgcttgcagcagatccagataacgtccgtaacccgcaagagcttcctcaagcatcgcaatataatcttcgccgctctgtaaaagccgtttttcgatatcagtaaaatcctgctgaaaaacggttttcactgccgttttatcaccacggttgatcgccgcagctaactgaccaatgccagaatcgctgccgaaacgatagcttttttgcagcaggcagagactgtcgcgcaaagatgccgcttctgtgccggttcctgccggaacgtgagtccccgtcaggcggcttagctgcctggcacgctcggcggtaaagcccgcgttggcataagcgcagatatcgcccagcacagccccagcctcaaccgaggccagttgatcacgatcgccgagaaagatcactcgcgcatgatcgggcaaggcgtcgatcagtctcgacatcataggcagatcgatcattgacgcttcatctaccaccagcacatcaagatgcagcgggttaccggcatgatgacgtaaacgctggctacccggctgcgcgcccagcaatcggtgcaaagtgctggcatcttccggaatgcgtttcttttgttcatcggtcagcggtaactgtcgcaaagccttgccgagagattcggttaagcgcgcggcagctttacccgttggtgcagccagacggatacggcagcgttcgccgtcggccatttgaattaacgctgccagcaacttcgctacggtggtcgttttaccggtgccagggccgccggaaatcaccgagatccgccgcgtcagcgccactgccgccgcaactttttgccagttaatttcatcgcttactggaaaaagtttgtccagggtttgcgccagtagagcttcatcaacctcaatggcatgattcacttcgttgaaaaagcgtgccactgtgcgctcgttacaccacatgcgattcaaataaagacgatcgccacagaggatcatcggcgtgggttcatctcccctgctgaccgcttgagaagccagcaagcattcttcccaattttgtagctcaccgatttcactgacacaggtcgccaacagcggatgcgacgcctcgttattttccagtcgtgaaagcggcaaacaaacgtgtccctctccggcatcatgacttaacagtgccgccgcgagggtgacggcaggatgttcatctcccgccacggtcagggcaaattgcacatccagcgggcgtagctgtttgtgctccacagcttccagtaattgcttttgcaatttcattacgcctcctccagggtcataccggcaaacatctcatccatcagggcaatcaacccggcgttgggtcgggttgtgtaaatcccctgttgcggatgttctttatcaacgccacgcaggaacagataaataacgccgccaaagtggtgctcatagtcgtaatcagcaatgcgatggcgcagataacgatgcagcgccagggtataaagctgatattgcagatcatagcggtgtgcctgcattgccgctgccatagcctgttgggtgtaagccgaactgtcttcacccaaccagttggatttatagtcgagcaggtaataacgcccttcgtggcggaacaccaggtcgataaagccttttaacatgccacgtacctgcatgaactccagcggcgggcagcctgcggatagcgggtcaaactggcggattaacgtatcaagctgactggcgataagcggttcactaatcggcagataaaactccatctccacctgtttattgcgggcggaaagttgactcaggcttacgccggtttcattgagaggtgcctggaggacagccgtgatccactcggtcaataccggttcccactgcgattcaaagccgccgagttccagtttttcccgcacccagttcgggtcaaccggctgggtaaaatccaggtcttcaaacaaactgtgcaagaacgtccccggtgacgcaccgcgcggaaactgatgtggtgttaacgtcggttcttcaacgacgctggcaacgcctgcagcatcgacatccagccgaggcatcaaatcctgggcgataccgtgaccacgctgttgcaaaccagagtagctggtgacgcgccagttatcgccgggcaatcgttgtaacgtcttcgcattcagctctgctgtagaaacatcattaacctgccagggttggttatcaccagtttgtgccgtttgccaggcaatatcatcatcgcataacgcttcaatacaggtgcgaagccctgccgcatcttgcggttcccctttttgcagcaaacgcccgagcgcactttggtggacgtcggtgtcaccttttttatcgccacgacggcgcaccagcggtgcaacgccgagactgcaatgccaaaccgaacgtgtcagcgccacgtaaagcaaacgcagatcttccgccagacgttcggcctccgcgaggtcgacgctttctggcgcagcattaagatccagaactgcctcaaacgagtggcgatcgtgataaaacgcctgctcctggacgcggaaattggtgataaacggcagccagaccaatggatattccagccctttcgatttgtggatcgtgacaatctgcaccagatgtttatcactttcgagacgcatttgttggctggaggcattactgtctggctcgaggatatgttgcgataaccagcgtaccagcgcatgttcactttccagctgcgttccggcttcttgtagcagttcgctgatatgcaagatatcggtaagacgccgctcaccgcctgccgttgccagcaagttttcagcaatgttacgcgccgacatcagcgcccgcagcatcggcataacgccacgtttgcgccagatttgccgataaccatcgaactcttcgactaccacatcccacgcatgttcgtcattgttcagcgtttcgatatccagcgcgttcagccccatcattgacgttgccagcgcactacgcagggtgttctcacgttcgggcgtcatcaccgcctgcaacaaccaaagcatttcctgcgcttccagagtttcaaaaacactgtcgcggttcgaaaggtaaacggaagggatttccagcaacgttaaggcatcgcgcacctgggcggcctcctggcggctgcgcaccagcacactgatgtccgaagcacgcaccggacgcgcgtcgtcgccgttcatcagcaacgcttcgccccgctgtccggcttgtagccagtcgcggatttgcgcagcacatacctgcgccatggtactttgataatcgccaacgccgcagctttcgccttccatcagccacattttcatcgcaggctgtgtttcacctttaaatacaaaacgtaacgcctgatttttcccggctgatttcactggaataaacggtatttcgcgaaacatgaacgcgtcatcagtctggctgaaaagcttattcacgctgttcaccattcctggtgcggaacgccagttggtgtctaaagtgtagtgggcgtgaacttcgctacgcgccttcatataagtgaagatatccgcaccccggaatgcatatatggcctgcttcgggtcgccaattagcaacaatgcggtttccggctgatggtgccagatacggcgaaaaattcggtactgctgggggtcggtatcctgaaattcatcgatcattgccaccgggaatcgcgtacggatcgccgctgccaacacctcaccgctttcgctacgcagcgcggaatcgagccgacttaacatgtcatcaaaacccaattcgccacggcggcgtttttcacgcgctactgtttcgcggatctcagccaatgcgcgggtgatcaccagatcgcggatcgacaatggttctgcaagcagttgatcgatcgcctcaaacagtggatgtcgcggggtttcccccccggccttcgtgcgatcttctaagaaacgctgggagaatttttccagcgactccggcaactgataactgtttgtctcttcttctgcccaggcgctgatcttgtcgatccatttagcctgattgctacggttaaacttgcgtcgatcaataccagaagattcgatcagcgcatccagttcacccactgcgtcgcgccactgctgttttaccgtatcaatacgcgccacaatttgcgcgtgacgggaagccagcgtttcatcatcgggcggcggtgctttgataaccggcgcttcgccttgcagataacgattaatatcgcgcagcaacgcctgcggccctttccaggtttcaaagacgacctgggctatttcacgcggcagcgggtagcagtggcgacgccagaaatcggcgcaggcctggtagcgtagcagagactcatcttcaatcagctgctgctcaaacagcatgccggattcaaaggcattcaggttgagcatgcgctggcaaaagccgtgaatagtaaagactgccgcttcatccatctgccgttcggctaacaacaaccactgcgcggcttgcgctttatcgtcgatctcttccagcaggcgttcgtacagtggattgtcggtggtttcacgcagacaggcgatgcgcaactcgtggatattgctacggatacgaccgcgcaattctgccgtggcagcctcggtaaaggtgaccaccagcagttcttcaacggtcagcgggcggggaaaggcggcggaaccgcctagtccaagtaacaggcgcaaatagagcgccgcaatcgtaaaggttttgcctgtgccggcagaggcttcaatcaggcgctcaccctgtaagggcaagcgcaaaggatctagtgtctcggcgacatcactcattcttttcactcatcaggggcattgtttgctgcaacgcgctgacgttctcccacactttccagccttcagggtgtacatattcggctttcccgttctggctgccggaaatctgcgacagaatagccatgccttgcggctcgaccaccgcctgatggaagaaatcagcaagtttttgcggcgtcagcagttttatctgggccacgattttatcacgcgaatcgaagcgcatattgccgcgatcgaaatctttacttaacttcgatgcttcttcgccgagcgtttgcggtgcctgcagcatctgggtaattaccgcctgctggatttgcgcaaactcatctggcttcatcgctcgcaattttgcctctgcggttgggaaaaacgccttgtaacgctcccacaagaatgaaggctgtttatcattgctttgcaaaaggaagcccatgccccactgacgccccacgctcattggaaacgcaaacacggcatagcccaattgttcttcggtacgcaactgattgtagaaccacggctgtacgatctgccccaacagagagctataggctgagctggtgtattcatcgtagccagtcggtacaaataccgctgccagtgcggagtcggtgctgttaccggctttttcaaagatgacggattgttttttatcgaccactacatctttgtttcgacaccactctgaaccatcagcgcccaactgtttttgcacatcgcgtgccagcgttgttgcctgggcctcggtcatgttgccgataaccataaactctggtcgagcccctgattttaaggcgtcgcgataggccagcacctctttcaacgtaatggagggcaaaattttacgccgttcatctcgcgagaagtacggcacttgcgagagcatctgcgcgggcataatcgcctgctcaaacgctttacccttttctgcggaatccatcatctggttataccaggacttcgcctgctcaagctgatcttccgtagcggtatagctaaagtacccctcgagcaatgcctggaacagctgcggcagacgctgggtgtaaccattagcattaaccataaggccgttgttagcgttggtggaaaaacttatgccaccaaccgacgcctggttgcttaactgatcaagcgccagccctgcgagataatcattgagcgcaaacatcacctgattgcgggcgctgtccatggctttcggattacgcaaaatcaggctgacatcagctttgggctcgctggcaaaataacggcttggcgcatacaccacgcgcagattcgactcatcaacaatcagctctggatggtcgtatttcttctctgacttaatcagcgagaaatcatcaggaatataagggttaagctctggcaaagagagcgcaatgtcggcggcttttttctgccagtcggcgaaagtttgtgcgctgattttatcgacctgatacggcgcatcgacaaagtaagccgttttgttgtgcggctctttcgggctgatataccagatacgcgcattctgcggcgtcatcatcgccagacgttcctttactgctttagcatcgtaccgatcggcaatattgactgcatccagcgtatgctcaacaggaacgcgaatcatggtatctgccagccattcgacgtaatccatatcacgggtgatcgacggataacggaagtcgatatccagcacattcgccagttcatcgaagtattgtttatcaatgcctttttcacgtaacagattgagatagctaaaaattgccgccacaacctgatcgcgattagccaggcctttatcggttaaagacgcagagatcgctaatacgccgctgttgccgttgacgataggatcggagttggcgctaatgccctcaactaatccctgcttttgcagccagtcagaaagtgtacctgggctgcgattgccaatcagataggtaatcaattcatcggttttactacggaacttcgctgagttgttatcgatgcgaaactcaacgcgcaacactttacgcggcagcgcagggacgtaatgaatgataatgcccttttgcgcgtcggtgactaccggcacggtgatttccggttttttgctctctttgttcggcacgcgaccaaaggtgtccgccgccatttttgccaactccggcagcggtttattactgtaaataaccgccttcatcaaattggcggaatagtacttctcgtggaaatctttcagcgcctgctgcaccggattaccaggtttgtcgcttaaagtttcgaggttaccaccagaaaactttgaaccggggtgtgccgggttaatggtttctgcgctgacctgtgccatgcgcatcccgtcacgcgtacgcgccatggttaattcagcgttcaccgcattacgctcacgttcggcatatttcttgtcgagcaaaggttcagcaatagcatcggccaggcggtctaccgcaccaggcaaggcgtcgttctcaacttccagatagaaagccgtgcgatacggcgcagtgctggcattgtgactaccgccgtgcattttgagatattcggccagactgtcagcctgcgggtactttttcgaccccatcagactcatatgttcaaggtaatgtgccagcccctggtacgcctcgggatcttccagcgacccaacgggcaccaccagcgccgagagcgatttaactgcctgcggatcagaaaccagcaagaccaccataccgttatccagacgtatagcctgatactggcggttatctttatcacttttacggatggtttcctgaatcggctgccatcccgtttctgcctgacttaagggtgcccaaagggcaactaacaacaataatgctttgaaccaggtgctgcggggcattcacggacctcataatcaacttaattttctgtccagattcaacacgttaacgcaaatcatctgccagaatttaatcttgtgctgcacgagtcagcctatgtttatataaccatcagtccgtgactggtgcgcatcataaagtaagcggatagattgcgcaatttttatacagcactcatgactgattaaagcgaaacagcggtaacaggaaacgttgcgactgttcaacgatggcctccattgtctctggtgttaattgccgccagagcctttgataccagatatcatcaccttcgccacgcaccatcatgttgccttcgtaagcctgaaggaatttcgtacgggctttttgcaacgtggaatcgtcatccagcatggcatcgttttgcgcgtcataacaggtttttagccacgcgccgccactttcaggtaacaccagcaatggcgcggacattccttcacgatacccctcaatcagttgtgagaggtaatgcaaagcctgttcggctgcaagcggcggaaaacgccactcgccgtctttgcgtagaaaaaggcgactttcaccattaccaccgctggcacagtagacaaggtgttccagccaaagttgcattccctgggccacacttaataaagagggacgccagcgcaacaggccatccggctgcacctgcggcaaccagccagttatctgcacaccgttgcaggcgagatcaatttccatactctgccccggctggcgacaggcaatgactctgtcggcaagctgctgcatctcctggcactgtgtttcccagaaaatttcaccaaaagcgccatacggtaaatcccctgccgctcggaagcggcggaacaagcgttcggcatcatcctgctcaaccagtgcattcaataactgctgattgatttgataacggctaagtccttccagaataaatggctcggtgtcggggatttcgctgtcttcagtacggaagttcacctgcaaacgcatctggaaaaatgcccgcaccggatgtgcccagaatcgttgtagcgtttccagcggcacggtttccggtaaggtaaacggcagcggctgaacaaattcagaatgtgctttaccagcctggctggccgcaggtagccattcacgagcatagctttgtcgttcgcctggctggtagttttgtggatcaaacggcatccgggtatggaggcaagtaagatgcgcttttacccttgcctcgctttcatcacagttgagcgcttcatcgcccggtagataatgactttgcccgatgtagtcgatcagttcctgcaccagtaccgacgggaaacgctcactgttatcctgaatggaacgaccgatatagctgatatagagtttttgctgcgcggaaattaacgcttccaggaacagatagcggtcgtcatcgcgacggctacggtcgccacgcttcggtttctggctcatcaggtcaaagcccaatggcgcaagctgacgtggataaacgccgtcgttcattcccagcaggcaaaccactttgaacggaattgaacgcattggcatcagagtacaaatgttaaccggtccggcgagaaaacgctggctgatacgttcttgatccagacgctgtgccagttcatcacgcaatagtgacagcggcaccgcgtcgccatactgcgcacctaaaccttcggcgataatcgcctgccattgttgttcgatcagcgtcatcgccgcttcggtttccgcatccggcaggaagaaggcgttgagcatatcgcgacaaaccggcaaccactcttccagcggacgctcctgtgccagcccgcgacgccagatgtttagctgcattagcagtgaagccagatgccccaccagttctgcaattaagccgctcgattcatcataaggtagaaccgattgccactcgccctgcgcgctctccatcgcgtagcccaacaacatacgcgtcaggccaaatcgccaggtgtgttgtccggtggcggggagttccagctcgcgaacgttgtcgtcatctatgccccaacgaatgccggattcgttgacccactggcgtaaataacgcagcccttcttcggtgatgtcaaaccgcgccgccagcaccggcacatccagcaacgccagcacatcctctgacacaaaacgactgtcaggcagtgataacaggctgataaacgcttccagtaccggatgtgactgccgcgcacgacggtcggaaatggcgtaaggtaggtaacgatccgcaggtgcgctaccaaacacagcctgaataaacggactgtagctgtcgatatcagccaccatcacgatgatgtcgcgcggagtaagtgtcgggtcttcctccagcatcgccagcaggcgatcgtgtaaaacttcaacttcacgctgcgggctatggcaaacgtggaaggtgatactgctatccagtggatcaagcgggcgtttgttatcgctacgggaaaactcttcgatgttcacaccagcaacggcgcggttttccagttccagaatgtcagactgaatgttatgcagcaggttatctggcgtgacatcgacaaaggcgtccagctcctggctgctctccaggtcagaaaggagataaatgtagtcgcgcccaagcttaccccatgaagccagcagcgggttgccgacatcctgttcaccatcgctgttaaagagctgcccggcattttcgctatcacgaaatagcggcaattcgcgatcttcaaaactgtgtcgacgctgacgggtcagcagtttcgccagataagcaggatctttaatatcgccccagtaataacggcaggggttggtaaacaggagatggatttcaatatgtttacccagcgcctgtagcgcctggagataaacaggcggtaacgcggaaataccgcatataaagacgcgcgaaggtaaccccggcgggcaggtcgtcgcggactccagcgtttcgataaagcgctgatagagattggcgcggtgccagcgcggttgcccgagttgatgggtatattccaccagcgccttccacaacggggcttgccaggcctgtgcttctcccagcccttcaaccaaatgtcctgtttcccactgtgccagccagtccggacgatagaccagatactggtcaaacaggtccgccgcttttgaggaaagctggaacagttttcgcttgtcgctatcgtcagtcagataatgccgcaacagggtaaagtcttcgcgctccagcaattgcggcagcagagtcatcagtttccagctcatgctctgtttgttaaaggcgctctctttggggatttccggtaacacccggacgaacatatcccagataaagctcgctggcagcggaaaatcaatgtttgccgcaataccaaacttttgcgacagggtcatttgcagccactgtgccataccggtactttgcaccagaatcatctctggttcgaaaggatcgtccagccgttcgcgttcgacaataaactccatcaacgcttccagcacgtccagacgattggaatggtagacccttaacatagcggctcctgactactgacgattcgggcaatgcaggcgggtcatctcgccttctctgcccccgggtgaaactagcgtaacgctgatgctgacacatcccgcctgcgatgtctgcattcggttgacctgccagttggcaggtggcgaaatcgcgcgcagttgcgtttgctgccagccatgccgccagagctgttggtactggtttctgctggcaagactgttcattaatgttcgctggaaacccgataacgcagtgacaatcatcaccatcaacaccatcgccaacattacctccggcaggctaaagccttgttgattcttcagggaagctgacataacgccctctctttcagcggacaaaaatcgctccagccgcgtggcgaaaaaacaatgtttccatcaatgacttcgcctgttcgccacaacgaaacgccttcataaccggcaatcaataaggcttcattatctgccagtaaacgcaaacaaacctgggcatcggtttcagcgtactgcgagcactgaactgctggctgcgtctgccagcagtgcatttttccccacgccagcgccgactgaacgatggcctggcggcgcaatgactgactttccatgctcacgcgagaggcaaaactgcgatcctgttggctcattccttgtaatagcaaactacccaaaaccagcagcatcaggaccagagccagtgacgaaacacccttttcgcggttcacaggttgaatcctgtcacgctatagctggcattcaccacggtttgcggttcagacttactggcagcacgcatattaaccgtcaacaccggcgagaagccgctgacatcctgacgtacgacctgaaaagtgtcgataatgatggcatccggattagtgactttatcccagcccttaccttcacaggatgtcgcaccgcgtagcgtttccagcacatgctccttcagacgaaatccaatctggtcggactcttttaccggttcgcgatcccagataccgttactgttcgcatcccactgcacaatgacacagtcaccctgtccgacaatttccagcccttcgccggtacagatgccatgacaataacccgccctctggagatgcttcgcgacggtaaatacccgcagccagatttcatcttccagcgccagcttacgggtgctcgttaaactttcacgctgtaacgcaggcagaaagcgtgccgcccccagcaacaatacgctactgatcgccatagcaatcaacacttccagcagagaaaaaccttgctcttttacaggcatccttctgtttctccttgctgacaaagccggagtcttccccacggcgaaaccaccagccaccactcgcccgttgagtttttgaagcgaatatgcccggcccatgcggtattgcgcaggccaaagaaagcaagcgaaggtgtcaggtcgctcatttcgacttcgggccagcgtggcacaaagaccaatggtgaactgccatgacaggtattggccccagcagcggaactcacaaggcaccataacgtcccctccctgataacgctgatactgtggtcgcggttatgccagttggcatcttcacgtaaatagagcaaatagtcccgcgcctggctggcggtttgccatagccgttgcgactgctgccagtattgccagccatagagtccacttgcgcttagcatgaccaaaatcagcatcgcgaccagcgtttcaatcagcgtataaccacgttgtgttttcatgccggcagtatggagcgaggagaaaaaaagacgagggccagtttctatttcttcggcgcatcttccggactatttacgccgttgcaggacgttgcaaaatttcgggaaggcgtctcgaagaatttaacggagggtaaaaaaaccgacgcacactggcgtcggctctggcaggatgtttcgtaattagatagccaccggcgctttaatgcccggatgcggatcgtagccttcaatctcaaagtcttcgaaacggtagtcgaagatggattcgggtttacgtttgataatcaacttcggcagcggacgcggttcgcggcttaattgcagatgagtttgatccatatggttgctgtacagatgcgtgtcgccaccggtccagacaaaatcacccacttccagatcgcactgctgcgccatcatatgcaccaataacgcgtagctggcaatgttgaacggcaggccgaggaagacgtcacaggagcgctgataaagctggcaagagagtttgccgtctgccacatagaactggaagaatgcatggcacggtgccagcgccattttatccagttcgcctacgttccacgctgaaacaataatgcggcgcgaatccgggtcgtttttcagctggttcagtaccgtagtgatctggtcaatatgacgaccatctggcgttggccaggcgcgccactgtttaccatacactggcccgaggtcgccgttttcatcggcccattcgtcccagatggtgacattgttttcgtgtagataagcaatgttagtgtcgccctgcagaaaccacagcagttcatggatgatggaacgcaggtggcaacgtttagttgtcaccagcgggaatccatcttgcaggttaaaacgcatctgatgaccaaaaatggaaagcgttccggttccggtacggtcgtttttctgtgtgccttcgtcgagcactttttgcatcagttctaaatactgtttcatggttcctcaggaaacgtgttgctgtgggctgcgacgatatgcccagaccatcatgatcacacccgcgacaatcatcgggatggaaagaatttgccccatgctgatgtactgcacccaggcaccggtaaactgcgcgtcgggctggcggaaaaactcaacaatgatgcgaaacgcgccgtaaccaatcaggaacaaacctgagacagctcccattgggcgtggtttacgaatatacaggttgaggataataaacagcaccacaccttccagcagcagctcgtaaagctgtgatgggtggcgcggcagcacaccgtaagtgtcgaaaatggattgccactgcgggttggtttgcagcagcaaaatatcttctgtacgggagccagggaacagcatggcaaacgggaagttcgggtcaacgcggccccacaattcaccgttaataaagttgcccagacgcccggcaccaagaccaaacggaatgagtggtgcgataaaatcagagacctggaagaaggaacgtttagtacggcgggcgaagataatcatcaccacgataacgccaatcaggccgccgtggaaagacatgccgccgtcccagacacggaacagatacagcggatcggccataaactgcgggaaattgtagaacagaacataaccaatacgtcccccgaggaagacgccgaggaagcccgcatagagtaagttttcaacttcatttttggtccagccgctgcccggacgattcgcccgtcgtgttgccagccacattgcaaaaatgaaacccaccagatacatcaggccgtaccagtgaagcgccacgggtcctattgagaaaatgaccggatcaaactccggaaaatgcagatagctactggtcatctgtcaccacaagttcttgttatttcgctgaaagagaacagcgattgaaatgcgcgccgcaggtttcaggcgctccaaaggtgcgaataatagcacaaggggacctggctggttgccggataccgttaaaagatatgtatatgatccgcgctataaccctccgcgaatcagcccgcccatgccgcgacgctccataaaggctgcaacctgatggcgaacttcggtcgccagttgcgcttccagactacgctgcgcaagattttctgcttcggcataatcaatgcgccgcagcaggtattttgcccgcgctacagaacgtccgttcatagacagatggcgatacccaagcccaatgaggattgccacgcacatgggatcgcccgccatttcaccgcacaaacggagatcgattccatgtatttccgcttcccgggcgatcatcgccagagctcgtaacattgcaggatgaagactgtcataaatgttcgccacccgggtattgttgcgatcaacggccagaatgtattgagtcagatcgttggtgccaacagagatgaaatcgacccgctttgccagatgcggcagcataaataccattgacggcacttccagcatgatgccgatacgtggtttgggaatttcgtaaccgatcatctcctcgacttcacgtccggcacgttcaatcaggcggcgtgcttcatcaacttcatcgaggcttgtgaccatcggcaacagaatattcaggttgcccgtagcggcattagcacgcagcatcgcccgcacctggatcaagaagatctccggctgatcgagcgtaatgcgaatcccacgccaacccaggcatggattctcttcgctgatcggcatgtaaggcagctgcttatctgctccgacatccagcgtacgcaaggtgacgggtttatcattgaacatttgcagcatcccctgatactgcgccacctgttcttcttccgacgggaaaccactttgcagcatgaatgggatttcagtgcgataaagaccgatgccatcaatacggctgcccagtttttcttcatgttccgggcttaaaccagcattgagcatgacttttatacgctcaccgctttttaactgcgcgggtaaattgacgtcatcttccgccagacggctaagctcaatctcttcactaattagccgctgatattcttgcagcagtaccggctccggatcgaccagcaattcaccgcgatagccatcaacgatcagcgtcctacgatgcagcaccgaaggctgaatatccgcgcccatcacggtagggatccccagcgcacgtaccatgatcgcagcatgggagttggctgcgccatctcgcacgacaacaccgactaagcgatcctggggcagctcagcaagcgttgtcgctgacagttcatctgccaccagaatgaaacgttccggccaggcgttcggcccttgattagcgtcatcaagatgaaacagcaatcgctgacccagcgcacgtaaatcgccagcccgctctttgagatagttatcacttagcgcggcaaactgttcggcaaatttttcaatgaccgtttttaccgcccactctgccaccgagcctttatcaacctcggcaaacaattcgcgacgcagccgggtgtccgaaagcaggtgcgagtaaagatcgaaaatagccgccgtttctttttgtgcaccggcggcaaagcgtttgctgtagcggcgaaactcgtttgccgcttcttccagcgccccggtcagtcgttcgcgttccagagccggatccagcgttgatgcctgatacacctgttccattaaaggtaacgtggcatcctgccagccttcggcaatcgccacaccaggtgctgccggtaatgcgcggattcgcgtctggcgatattgcccaaacaaggcagtcaactgcgactgagaaagaatagctgccatctgggtggcaagcgtcaccaggaaggattcttcactttcgtcatactggcgcaactctcgttgctgtaccaccagtacaccaagcaactggcgacgttgaataattggtacgcctaaaaacgcgcggaaacgttcttcttttacggaggggatgtatttgaagctggggtgcttttgcgcatctgcaaggtttatcggttccgccagcctgccaaccaggccgacgatcccttcatcaaacgcgagcgttacagtgcgaccgcgtggttttttcagcccccgggtcgccatcaggtagtaacaacgtcgatcatgatcggccaggtagaccgaacagacctcggtatccatcgcaagacagatgtcggtaaccagaatatttaacgcctcattcaggcgtggtgcgctggctaccttttcgactatttcgcgcaggcgagtgagcataattggcgtgacttaacctcttttacgtcgataagcagatgcgttttgtggttttggcgtattttcctgcagtgacatcaccacactcgcgaactctttcattaccctacggtagacatcacgtttaaatgacaccacctgtctgaccggataccagtaacttacccatcgccagccgtcaaactctggtgtactgctggtttgcatattgatttctgcatcgccgctcaccagctgcaagagaaaccatttttgtttttggccgatacaaaccggcttcgtgtcccaacgcaccaaacgtttcggtaatttgtagcgcaaccagttacgcgttgaagcaaggattcgaacgtctttgcggcttaatcctacttcttcaaacaattcacggtacatcgcctgctctgcggattctccggggttgattccgccttgcggaaattgccaggagtgctgaccaaatcgccgggcccacattacctgcccctggcgattacaaatcacgatacctacgtttgggcggtagccatcgtcatcaatcaccggactacctcaaaataaagctttatatacgaatgattgtttcatactccaggaagacggtaaaccactctctgcagggcattacacactaataacaattgaataactcacagttatgtgcagagttataaacagaggaaggggtggatagccgtttttattcaccttttctgtggatagagttgtgaagaactacggaattactacgggaaaacccggagcattctgaataagcccgatatagacattttaaaatattcattatcagtcaatgcattacatgtaattttagtaatgaaaaagagtaattcgtgacccaggtcacacctctcatttacgggttggcgaaagatcaaccaatgccgtatttatccacagaatgtgccactaagttaagcactgaaccactaaaaactggagtttcgtcgcacgtcaaggctgtaaatggaaacagtagtggaggtttttcacagttatcccagctttctgtggataacatggtgtaagatcctgtttattttcagtgaccagatttggaaaacccgttgcagtgttgcgcaactcgattaccggcaacctaaaaagcaatataaatcagagaattgaacaacgcatgtggaaaaagttacactgcgaatattcggcacataattgctgtttgttttttaatcaaggtatcatgacatgtcccaacctcgcccactgctctctcctcccgaaactgaagaacagttgttagcgcaagcacagcaactttctggttatacattgggagaactggcggcacttgtcgggctggttacgccagagaatttaaaacgcgataaaggctggattggcgtgttactggagatctggctaggtgccagcgcagggagtaaacctgagcaagattttgctgctctgggcgtggaacttaaaactatccctgtggatagtcttggtcgtccgctggaaacaacattcgtttgtgttgccccgttaacgggcaatagcggggtgacctgggaaaccagccacgtgcgccacaaactcaaacgcgtactgtggataccggttgaaggcgagcgcagcatcccgctggcgcagcgtcgcgttggatcaccgttgctgtggagcccgaatgaagaggaagaccggcagctacgcgaagactgggaagaattaatggatatgattgttctcggtcaggttgagcggattaccgctcgtcacggggagtatttacagatacgaccgaaagcagcgaatgcgaaagcgcttaccgaagccattggtgcccggggcgaacggattctgacgctgccacgcggcttttatttgaagaagaatttcaccagtgcactactggcccgtcattttctgatccagtagccatcgctttgacctgccgctttccgggcatataattaccgcttcatttttttggcagggctttttagatgttatttgcatggataaccgatcctaacgcctggcttgcgctcggtacgctgacgctgctggagatcgttcttgggatcgacaatattattttcctttctctggtggtggcaaagcttcccacagcacaacgtgctcatgcgcgccgtctggggttggcgggagccatggttatgcgtctggcgctgctggcatcaatcgcctgggttacgcgcctgacaaatccgctttttacaatattcagtcaggaaatttctgcccgtgatttgattctgcttctgggtggcttgttccttatctggaaagccagcaaggaaatccacgaatccattgaaggtgaagaagaagggctgaaaacacgcgtttcatcattcctcggcgctatcgtgcagattatgctgctggatattatctttagcctcgactcggtgattacggctgtgggtctgtcagatcacctgtttattatgatggcagccgtggtgattgccgtaggcgtgatgatgttcgccgcgcgctcgattggtgattttgtcgaacgccatccttcggtaaaaatgctggcgctctctttcctgattctggtgggctttaccctgattctggaaagtttcgacatccacgtaccgaaaggttacatctacttcgcgatgttcttctctattgcggttgaaagcctcaacttgattcgcaacaaaaagaatccgctctgatactccgtacgctctcctgcgggagggcgtactcactccttttaccctcacagtttaagattttcctgctttcaagatatataacgtcggtttataaacagactattatcataggtaggccaaatgaggataaccggatgaaaaaatgggcagtaataatttctgcagtcggactggcgtttgctgtttccgggtgttccagtgattacgtcatggcgaccaaagatggccgtatgattttgaccgatggaaaacctgaaattgatgatgataccgggctggtgagttatcacgatcagcaaggtaacgcgatgcaaattaaccgtgatgatgtttcgcaaattattgaacgttaacaaataaggtcagcatccggctggccttaagatttttctctttcccttttcccttccctctgccatttttatattccttatgtcgtgattataaaaaggaaacggctatgcaatatcaccgtataccccacagttcgctggaagtcagcacgctggggcttggcacgatgacgtttggtgaacagaacagcgaagccgacgcccacgcacaactcgactatgccgtcgctcagggcattaaccttatcgacgttgccgaaatgtacccagtacctccgcgccccgaaacgcaagggttaaccgaaacctacgtcggcaactggctggcgaaacatggcagccgcgaaaagttaattatcgcctccaaagtgagcggaccgtcgcgcaataatgacaagggcatccgcccggatcaggcgctggatcggaagaatatccgcgaagcgctgcatgacagcctcaagcgcctacagactgattacctcgatctttatcaggtgcactggccgcagcgcccgaccaactgcttcggcaaactcggttatagctggacggattctgcgcctgcggtttcgctgctggatacgctggacgcactggcagagtaccaacgcgcgggaaaaattcgttatatcggcgtgtcgaacgaaactgcatttggcgtaatgcgctacctgcatctggcggacaaacacgatctgccgcgtattgtcaccattcagaacccttacagtctgttaaaccgcagttttgaagtaggtctggcagaagtcagccagtatgaaggggtcgaactgctggcctattcgtgcctgggtttcggcacgctgaccgggaaatatctcaatggtgcaaaacccgctggcgcacgtaatacgctctttagtcggttcacccgctatagcggtgagcaaacgcaaaaagccgtcgcggcgtatgttgatatcgccagacgtcatggcctggaccctgctcagatggcgctcgcgtttgtacgccgtcaaccgtttgttgccagcactctgctgggcgcaaccacgatggatcagctgaaaactaacatcgaaagtttgcatctggagttaagcgaagacgtattagctgaaattgaagcggtgcatcaggtttatacttatccggcaccataagattaacgccggttaaaaccggcgttaaatattaatgacggcgctgccagatccacagcgccgttattgccagcgcaaacagcgcaccgaagccaatgccaatgggcacgaccgggatgcctatcattaccgccagcgagtaaatgcccagcatcaacaacatggcgctgttttcgccaaggttttgtactgcaatcgcattccccgccccgacgctttttttaccccgctcctgtagcaacgcattgagcggaacgacaaaaaagccccccatcacgccaatcagcatcaacaaggcataggctggcagcagctcgtgttgcagggaaaaaatcagtaccaccacgccaatcaaaatcccggctggcatacagcgtgacacggtttccagcgtaactaacttcgctgccgcacctgcgccaaccacgataccaatcgctaccatcgcgttgagataggtgggcgtagcgttatcggtaatgcccagcgccaccggtacccacagcaccaacaggaaacgcagcgtgacacccgctccccagaataaactggtgcccaccagcgaaaaacgcgtttcaccattgcgccatagcgaggtgcaggcattcaggaaactgcgggtcatgttgatgagattccaggactgccccggacgcgccgccgccagtttgggaatgtagatattggcaacgaccgcaccaccgtaggccagtgcgcatgcggccagggcgacgaggacatgccagtcagccagcacaccaccggctacggaaccgagcaaaatcgccgctatggtagaagcttccattaaaccgttagctttcactaacttactacccgtggttaattcgccgagaataccgtatttcgccggtgaataggctgcagcaccaacacccaccagcgtatagccgagaaacggattgataccaaagcagatactggctgcgcccagcagcttcaggccgttggcaaacatcatcacccggcctttggcgaagctatccgccacctgcccgacaaacggcgcaaaaagaatgtaagcacctacaaacaccatttgcaggatgggctggctccactccggatagaactgcgctttcagtaacgccagagtggcaaacagtagggcattatcgccaaacgcagagagaaactgcgccacgataaccgctttcatccccttcgaccacaacgaagtgttagtgtgcactgactcactcatcgtgttgttccgcttcgtctacccagcttttcaacgtgacaaagtcaggtttgccgctgccaagtaatggcatctgtttcagatagcgaatatcgcgcggtacagcaagctccggcacgccgtgctcgcgggcatactgttgcaacttatcgcgcgtcagttcgttatctgtggtgaaaagcaccagtgcctcgcctttgctggcatcgctcttaatcgcagtggcatggactttatctggcgaaacaccaagtgccagttgttccaccatttccagcgacaccatttcgcctgcaattttggcaaagcgttttgcgcggccctgaatctgcacaaagccctgctcgtcaaaacgcacaatatcgccagtgtcataccagccgcgctccatttcgccgcgaacattctcggcggtgggcacttccagtacacctggcttctccacccgcagatagccgttcattatgttcggccctttcagttgcaggcgtccgccctcttcgataccagggaccgacaacaggcgcgcatccattcctggtagaatacgccctaccgtaccgggtttcgccgccatcggtacgttgatagaaacgacaggcgcgcattcggtcacgccgtagccttcaaggatgcgcaggccaaatttatcctgccaaagctgtttggtactttcttgtaatttttctgcgcctgccaccacatagcgtagacgatagaagtcatacgggttggcgaaacgcgcgtagtgaccgaggaaagtcgaggtgccgaacaacacggtgcaactgcggtcatacaccaactccggcacaatgcggtaatgcagcgggcttggataaaggaacacttctgcacctgtaagcagtggcgtaaacaggcctaccgtcagcccaaaggagtgaaacagcggtaacgccgacataaagcgatcgttggtggtgaagtcggcaatcgttttaatctgctcgacattcgccagaatgcttttatggctatggacgacgcctttcggatggccttcagaaccggaggtaaaaaggatcagcgcctcttcttccggctgctgtttaacctgtgccagacgcggcatcagcaaatgagcgaagatccatactttgtcggcagtggtgacatctgcttttaaatcttccagatagacccagcgcacctgagtaagttgctccggcagatgccagagtttgcctttatcgagaaactggcgggaagtgaagatggttttgatttcagccgccgtaatagcactggtcagcccttttaccccggcagtgtagttcatcattgcgggcatgcggcgacgggcgatggccccaaaaatcactgccgcactgatgcctgcattgggcagcattaagccgatgcgttcgccttcaacactgtatttttcaaggatgcgtccaacaaacagcgttttcgtaagcaatttgcgataggagtctggggtaaagttgacgtcttcgacacatttcttcccggctccgaagcggtacattgcactcagtaaagattcgtacagcgtttcacgcgggcgcaccgccattcgcgcttccatcattatttgatgcagcatttcgccagcgattttgcgacggtcacgggcacgcggcgcatccggcatcgccacctgcgttggtggcaaaatatgcagagtaatttgcgggaacaagcgacgtttaaccagacctttcaggcggctgaagtgcgtaagttccgccccttcaatacgcacaggaataaccgttgcaccagacttcgccgcgacaaaacccgcgccatcgtagattttcatcagcgagcctgtcgtggtgatgcgtccttcagggaaaatcaccactggtcggccctgttccaccagacgtaccagatgtttaatagccataggttgcgtcgggtcgagaggaacaaagtcgataaatgatttcagccaacgcatataccactgttggcttattgaggtgtaaacggcaaacactggacgcacaggtaaaaacagtccaagcaaaatgccatcaataaaagagacgtgattaggcgtaattagaacgcgctcgcccttcagtgcctgggtgtcacccgtaacgcgaacgcgatacaaaacacggcacaaatttcgaaaaaagctaaaaagcattccaactccctttgctctgattcagtaaaagcgaatggagggagattacacgagataaagaacgcgagcgacagtaaattaggtgcgaaaaaaaacctgcgcatccgcgcaggttggtgcaagagacagggtacgaagagcgtaccgaataatctcaccaatcaatacctctgggatcttgattgtggtctgcacgacgactcttcgccagcgagaaaacgcaaaggaatgaagggaaatgcaacgaggtgtgtaaattgtcggttactgttacagattgatgaccggcaaaaaaaacctgcgcatctgcgcaggctggtgtaattcatgtgctcaacccgaagttgacttcacctatcaatacctctgggatcaccactttagcaacctgaagccaaacgccaccagcggtcaatcgcaacagcgtttcgcaaagtgtaaccaaaggtttgcaatctctttttttgtcttacttatttgcgtttggctcacattcccacgatgaaaacacgccaccccttgaaccaacgggcgttttccgtaacactgaaagaatgtaagcgtttacccactaaggtattttcatggcgaccataaaggatgtagcccgactggcaggcgtttcagtcgccaccgtttcccgcgtcattaataattcacccaaagccagcgaagcttcccggctggctgtgcatagtgcaatggagtctcttagctatcacccgaacgccaacgcccgtgcgctggcgcagcagaccactgaaacggtcggtctggtcgttggtgatgtttccgatccgtttttcggtgcaatggtgaaagcggtcgaacaggtggcttatcacaccggtaattttttattgattggcaacggttaccacaacgaacaaaaagagcgtcaggccattgagcaactgatccgccatcgctgtgctgcgttggtcgtccatgccaaaatgatcccggatgctgatttagcctcattaatgaaacaaatgcccggtatggtgctgatcaaccgtatcctgcctggctttgaaaaccgttgtattgctctggacgatcgttacggtgcctggctggcaacgcgtcatttaattcagcaaggtcatacccgcattggttatctgtgctctaaccactctatttctgacgccgaagatcgtctgcaagggtattacgatgcccttgctgaaagtggtattgcggccaatgaccggctggtgacatttggcgaaccagacgaaagcggcggcgaacaggcaatgaccgagcttttgggacgaggaagaaatttcactgcggtagcctgttataacgattcaatggcggcgggtgcgatgggcgttctcaatgataatggtattgatgtaccgggtgagatttcgttaattggctttgatgatgtgctggtgtcacgctatgtgcgtccgcgcctgaccaccgtgcgttacccaatcgtgacgatggcgacccaggctgccgaactggctttggcgctggcggataatcgccctctcccggaaatcactaatgtctttagtccgacgctggtacgtcgtcattcagtgtcaactccgtcgctggaggcaagtcatcatgcaaccagcgactaaccgcagttaaagcaattccagcgccagtaattcttcgatggtctggcgacggcgaatcaaccgcgcctgaccattatcaaacagaacttctggtaacagcggacggctattgtagttggatgacattgatgcgccatatgcccctgtatcatgcagtaccagataatcacctgccttcacttccggcaaggcgcgggtttcaacatttcccccttcctgctgggtaaagacatcgcccgattcacataacggtccggcgacgacggtttccaccgttggcgcgtgttccagagaacgaccatcagctgccagggcactgatatggtggtaactaccgtacattgccgggcgcatcagatcgttgaacccggcatcaaccagcacaaagtggcggctccccatttgtttgacgctccgcacctgagtaattaatacgccagactgcgctaccaggaagcgacccggttcaatttccagtttcacagggtggcccaaatggcgggcgatttgctcacgcgcggcattccacagaccataataatgttcggtatcaaccgcctcttcaccctgttgataaggaacagaaagcccaccgcccgcagaaatagcctgtaaatcctgaccgaattcgatgacctgacgcaccatagcaccacacacctgttccagatgggcataatcaacgccagaaccaatgtgcatgtgaatgccgaccagctgcagatgatgacgttgtatcacgtccagtgcggcgggcagatcggtgtaccagataccgtgcttgctgttttcgccaccggtattggttttttggctatgtccgtgaccaaaccccggattaacgcgcagccatacccgatgccctggcgaaacctggcccagttggtcgagcatatcaacagaacccgcattcaccggaatttgcaattcactgacgcgttcaagcgtcgcctgatcgataacatctgccgtaaaaacaatatcatcggggtgcgtttgcggattgtaacccgccgccaacgcacgctctatttcgcctaacgagacggaatccactttcacgccctgctcacgcattaagcgcaaaatatgaatattggaacaggctttctgtgcaaagcgcaccacatcaaactgtttcagcgctgcaatctgccgacgaataatttgcgcatcgtagacccacaccgggcagccaaattcagcgggcaaacgcagcagattttcggcggtgagatcggtatcggtgctgaacagtgaatgtggcataacaaactccagataagtgcttttttatgattacgccacatcataaaaagaataaaaaatatcgatttatgtcgagtctatgcaaaaatgatatggattaccggattgcgagagagcgctaatggccgccgttaacttacgtcatattgaaatttttcatgcggtaatgaccgccggaagcctgactgaggcggcacacctgctacacacctcacagccaaccgtcagccgcgaacttgcgcgctttgagaaggtgatcgggctgaaattgtttgagcgcgtacgtgggcgattacatcctaccgtgcaaggactgcgtctgtttgaagaagtgcaacgatcctggtacggactggatcgcattgtcagcgccgcagaaagtctgcgcgagtttcgccagggagaactgtctattgcctgcctgccggtcttttcgcaatcttttttaccgcagctcctgcaaccctttctggcacgttatcccgatgtcagcttaaatatcgtgccccaggaatcaccgctacttgaagagtggctctcggcccagcgtcatgatttaggactcactgaaacgctccatacgcctgcgggaacagaacgtaccgaattactctctttagatgaagtgtgtgtgttacctccgggtcatccgctggcggtaaaaaaggtattaacgccggatgattttcagggtgagaactacatcagcctttcccgtactgacagctatcgccagttgctggatcagctatttactgaacatcaggttaaacgacgcatgatcgtagaaacccacagcgccgcgtcagtctgcgcaatggtacgggcgggggtaggtatttcggtggttaacccgctcaccgcactagattatgcggcaagcggtttagtggtgcggcggttcagtattgcggttccgttcaccgtcagcctgatccgccccctgcaccgcccgtcatcagcgctggttcaggcgtttagtgggcatttacaagcggggttaccgaaactggtcacttctcttgacgctattttgtcgtcagctacgacagcataaaagcgacagcatcctcggcatggatcgccgcggtatcaaacacaggcaaaacactgcgctcttctggcaccagtaaaccaatttctgtgcagccaaaaatgacgccctgtgcgccctgttctgcaaggcgagcaatcacttgcgcacaataagcgcgtgacgcttcggtaaattgccccagacacagttcttcaaaaataatctgattaattttcgcccgttcatccgcttcaggaataagacaattgatggaaaattgttccgtcagccgcccgcgataaaaatcctgttccatggtgtaacgcgtacccagcagcgccacacgagtcattccggccccggtaattgcacgtccggtggcatccgcaatgtgtaagaaaggcagagtgcaacgtgactcaatggcatccgccactttatgcatcgtattggtacatagcacaataccttctgcgcccgcccgctgtaagccaagcgccgcctcagccagaatgtccccggttttatcccattccccgcgacgctggcactcttctatttcatgaaaatcgacgctatgtagcagcacttgcgcagagtgaagcccaccaagccgctgtttaatgccttcatttatcaaacgatagtaaggaatggtggattcccagctcattcctcccagcaaaccaattgttttcattcctctctcctgatgtgtgttaccgcaacaaggctgaataaggaacgagacaaacgcctcaacggccaagtgcccaatctctattaacgaaaaaagggccggatgtacagcacatccggcccgtgaaatcagacgccgatatttctcaacttctcgcctgccatcagtttgcgttcgatatgttccagcgtgacatttttggtttccggaatgagccagaaagtaatgcccacaaacgcaatgttcagcgcagtgtagagccagaacgtaccggcagcgccaatgctatcaagcagtgtcaggaaggtcgcgccgataatcatattcgacacccagttcgtggtggtcgaacaggtaataccgaaatcgcggcatttcagcggctgaatttcagagcacaggatccacaccactggcgcggcgctcatcgcataaccggcaatacacatcatcgtcatgccaacagagagccaggacaagccactggaagccgtaccgttatcaaactgcatcaggcaatagcccagcaccagagtgcctaacgccatcacgctgaaaccaattttcagagccggtttacgccctgctttatctaccgtaaacaccgcaataaaggtggcgaacataaaggtcagccctacgaccagagtcgcaatcatctgttgttctgtggtcgtaaagcccgccattttgaagatacgcggcgcgtagtacatgatgatgttcataccggtaaactgctgcatcgcctgcaacaacataccgagaaacacagcacgacggacgttacggttgatcttaaacagtgcccaaccgccctgttttaacttcaggctttcacgaatttcgttgagttcttctcgcgctttttccgacgtatcgcgcagcatacgcaatacttcttccgcctcaatatgacgccccttttccgccagccagcgcgggctatttggcaggaagactaccagaataatcagcagaactgctggtaaagcaagaacccccaacattgcgcgccagttaccgctataactgaacgctgtatcggataaaaacgccagcacgatgccgagtgtgaccatcaactggtacatactgatcatcttaccgcgaacgttttcacttgccatttcagaaagatacagaggagcggtgtaagacgcgatcccgacagcaatgcccagcaccacacgagcggcgattaacatctctacgctggtcgcaaaagcggaccctatagaaccgagtacaaacaggatggcccccgccatcaggctgtatttacgccccaggcggaacgacagccaaccattaaacagcgcaccaattgctgcaccgagcatcatgctactaaccacccattcctgcaaacgactggtcagcacaaagtgatcggtaatgaacggcaacgctccggcgattacgccgatatcaagaccaaataacaatcctgcgaccgcagcagctaccgaaacaaacatattcatacgccgcgtatcccgcaaagaacgtggcgttaaagcagattccgtattgatagtaaccattttttcctgccagcagagagtaagacatagtgaaaaaatacgtgaacaactcacgcaggtgtcaggtcggaaacagcataaatatggattaaattgctgcgacatgtcgttatgtgatggatattccaattttcaaattaagttgaattattgagattattattaaccacctaattttacagcagataaaattcataaagttcattaattgataattaatatggattatttcataaccatgatatggattatgatgatctacaggtataaaaaaccctgccatgcggcagggtcataaaagtaagaagaatgaattaacgcgccagccaaccgccatccacggcaatggtataaccattcacataatctgaagcgctggaggcaaggaacactatcggccccatcaggtcactcggcagtccccaacgaccagctggaatgcggtcgagaatttccgcgctacgttgttcatctgcccgtagttgttgagtattgttggtcgccatgtaacccggggctatcgcattaacattaatgttgtgtttagcccattcgttcgccatcaatcgcgtcacacccatcacgccgctttttgatgcggtataagaaggcacacggatcccgccctggaaggagagcattgacgcgatattgataatcttgccgccattgccttgcgcgataaagtgtttcgccgctgcctgagacatgaagaatacgctcttgatattcaggttcatgacatcgtcccagtccttttcgctgaactcgagagcatcttcgcggcgaatcaatccggcgttattcaccaggatatcaatatgaccaaactccgctaccgcgcgatccagcagtgctggaataccatcaatctttcgcagatcggcggtcaggcttaaaaaacgacgccccagcgctgtgacctgctcgatggtttcagtcggttcaacgatgttaatgccaacaatgtcacagcccgcttgcgccagccccaacgccatcccctgacccagtccagtatcacaaccagtgacgaccgcaactttaccttcgagagaaaatgcacttaaaatcataacaataccttattcgtttatgcccacaactagcgcaaatctttaacggccacatggtccatatcatcaaagacctggttttcaccgaccatgccccagataaaggtataagctttggttccgacaccggaatggatcgaccagctcggggagatcaccgcctgctcgttatgcatcacaatatgacgcgtttcttgcggctgccccatcatgtggaaaacgcaggcgtcatcatccatattgaaatagaaataaacttccatccggcgctcgtgggtgtgacacggcatggtgttccacaagttacccggagccagctccgtcagccccatactcaattggcaggtttccagtacatccgggacaaaatatttgttaatcgtgcgacggttactggtgaggttatcgcctaacgtgactggagatacttcgtccggtgtgacttttttggtgggatacgtcgtatgcgcgggtgcgcaattgtaataaaacttcgccggagtgccggtatcaatactggcaaagacaacttcttttgcacctttaccaacatacagggcgtcgcggtgaccgatttcatagcattggccatcgacagtaatcgtaccggcaccgccaatattgataacacctaactcgcgacgttcaaggaaatagcttacgccgagttgtttaccaacttccccgccaacggaaaccgttttagttatcggcataatgccgccaacaataattcggtcaatgtggctgtaaaccatggtgtactcatcggcgacaaataccttttcaaccaaaaattcattgcgcagcccttgggtatccagcgtttttgcgtgcgcactgtggatgctctgtcttacgtccacatcaacctccgataatcagtgaagcgtgaaaatagaaaacgatagtgaaacactgtttcgttttctctataaagggatgatatgcccatgggctagggttttcaattaaaaataaaacaatgtttcatttttaagttaaggattaaaaaaagtgcagtgtcgatcacgaatatgtcatgagaatggaaaaatgagggagcccagaaaatgtatgtcgacttgccagccatcattattcaacagattaatgacggcagatatttatcggtaaggaggaaatgcagagctattcgtcacgttcaatggtcaatgccacaccctggcccccgccgatacaaagcgttgccagtcctttgcgggcattacgtttcaccatttcatgaaccagagaaaccaggattcggcaaccggaagcgcctatcgggtgaccgagtgcgatcgcgccaccattgacattgacccgacgctcatcccactcaagcatcttgccaaccgaaagcgcctgtgcagcaaacgcttcattagcctcgataagatcgacttcagccaactgccagcctacacgctccaggcaacggcgggtcgcatacaccggcgcaattcccatcaatgccggatctacaccaacgctggcaaatgcgcgaatgcgggccagcacgggtaaattcaacgctcgtgctttggcttcgctcatcatcattaccgcagctgcgccatcgtttatggatgatgcattacccgctgtcacagaaccgagactatcaaatgaaggatttaaacgggctaagccttctgcgctggcgtcagtgcgtggctgttcatcggtatcaacaaccaacgtctgcccgttactttgggtcattaccgggacgatctcatctttaaatcgtccggcgtcaatcgccgctcgcgctttttgttgcgagctaagtgcgtaagcatcctgcaactgacggctgatgccatattcgcgagccagattttcggcggtgacaccaatatgataatcattgaaggcatcccacaacccatcatgcacaagactgtcaaccaactggctattgccaagctgtgcaccggtgcggctatcagtcagaacatgtggtgcgcggctcatgttttcctggccaccggcgatgacaatatcagcctcgccacactgtatcgcctgagtagccagatgcagtgctttaagcccggaaccgcaaacgtcattaatagtgattgcagaaacgctattaggcagaccacctttaatagccgattgccttgccggattctgccctgcccctgcagtcaacacctgaccaagaattacttcatccaccgcatatgcaggaacgccggtacgttctattaacgctttcacgaccagactaccaagttccacggcggaatgacccgctaacgcaccacgaaagcagccgataggtgtccgtaacgccccgacaatcacaacgtctttcatcacaacctcgcaccaattaacagtgcaatagtaaatgattgttaattacagttatcttaattgtttaaaaaaagtgatttttatcacaaaggaaatatgcctgagcagcagtcagagacataactggcacgtaaggtttgcaaccactaacccaccaatagaggggtagatagggcgttaatctcccatacttaacctggtttatggtaaattgccctccattttgtttaatttgtagatgatacgttcagataatgtctaatatttggtctaaagaagaaactctgtggagtttcgcgctctacggcacagccgttggtgcaggcacgctcttccttcctattcagttaggttcggcaggggctgtggtcctgtttattactgctctggtcgcctggcctttaacatattggccacataaagccttgtgccagttcatcctctcatcaaaaacatcagcaggtgaagggataacgggcgcggtaacacactactatggcaagaagattggtaatctgattaccacgctgtacttcatcgccttttttgtcgtcgtgttgatatatgcagtggcaattaccaactcacttacggaacagctggcaaagcatatggttattgatcttcgcatccgtatgttggtgagtctgggtgttgtattaattctgaatctcatttttctgatgggacgtcatgccactattcgggtaatgggatttttggtattcccattgattgcctatttcttatttctttccatttaccttgtcggtagttggcaacctgatctattaacaacccaggtagagttcaatcagaatacccttcaccagatatggatatcgattcccgtgatggttttcgcctttagccatacgcccattatttctacgtttgccatagacagacgtgaaaaatatggcgaacacgctatggataaatgcaaaaaaattatgaaagtcgcttatctcatcatctgcataagtgtactgttctttgtctttagctgcctgctttctattccaccttcgtatattgaagctgctaaagaagaaggggtcaccattttatcggcgctttctatgctgccgaacgccccagcatggttgtcaatttccgggattattgtcgcagtagttgcgatgtcgaaatcattcctgggtacgtactttggcgttattgaaggtgccacagaggtcgtcaaaacaacactacagcaggttggtgtaaagaaaagtcgtgcatttaaccgcgcactatcaattatgttggtatcgctgattaccttcattgtttgttgcattaacccgaacgcgatttcgatgatttacgcgatcagcggcccgctcattgccatgatacttttcatcatgcctacgctgtcaacgtatctcatcccggcgcttaaaccctggcgttccatcggaaatctgattacgctgatcgtgggtatcctgtgcgtatcggtaatgttctttagctaatatcagttgtggatggttcaaaattgctacaattttgaaccattccatttttcataatattcatttgttattattccaccctatcacttctctcgtcatatcctagtattatcagttagttaaacacacaaagagatctgaacatcttaaataagactatttaagatgcataacttagattcgcaagatatcttctggtcattcaaaaacaatttgcgatatagatattcttataccatgagatagttatctggaccgctctcaaccatgcaagattaaatcagtgaaacataatcatatttgataacgagaaatgcatttttaaatgccttactcagaattatagcaaatacagattaatcgcaatttttcccggcaaaattacaaaatcatggtgtattgacatcatcaataaccaatgaaattatgcaattatatacggatagggaggttcttaacatggggctttgtagtcgttataaaagtcttacatgcaatagttgctcaatgcattgccaaataatgccagaagagtcaccgcgtttgcagtattgcgcaaactcgtgtttttgtatgtggcccgaagaaagttcatattttaatcgtggtgtggtagaaggtatcttaacaaaaaaccacaatgcgagattaagcggatatatttttgtcgatttttcagtaagttttttacgtctattccttgaaaaagactggattgactatcttgcaagtactgacatggggattgttttagtcagcgaccgcaatatgcaatcgttagctaattactggcgaaaacacaactcagcaatatctgctgtcatatataatgatgatggtcttgatgttgccaatgaaaagatcagacaactatttattggtcgttatttatcatttaccggaggtaacacattaactcagatggaattcaccataatggggtatatggtttctggttataatccatatcagattgctgaagttctggatatggatatccgtagcatctacgcgtacaagcaacgaatcgaaaagagaatgggtggtaaaataaacgaattatttattcgttcacattcggtccaacattgatactcaacgaccagccagaatcatactctgtttatacgggcatttattgaaatgtccgtattttataaataggccgtcccctcaagagtaaacaccatagtatttaaaaccatcacacgaaaaattcagaagcattacgaaatatgaatttacaaacaatagtggcataaatgttaaccatgttaatttacgtaaagttttacgttgcaacattaaagcctcatttcaatcatcatgataaatataaaattaatatatatttatgccgtaaataccaatatacttagcaaactatgtgatctccatttcgattgatttagtgtttattgacgtatgtactggattattaacgataatatcgagttctggcctgagcaccgaaaattaatatcggtacataacgccgatcttaacgtcgttctgacaacgccagccagtcgatgtttatcacttctacttgaagcttttcctgatgtggttgcacaacaagattttttcaccagagtctgggaagaagaaggtatgcgtgtgcctactaacacgttatatcagaacatatccattatcagacgcggatttcgcgctgttggtgatactacccactcgctaattgcaaccgtgccgagaagaggattcaagatccataatgacattaacatacaaaatcatgtaataaactcgtcaacagacgcacatacacacaatgccccacctgccataaaagttaatgcgggatacaaagagagcattggtggcgcaaagaatttcaataacaaaatcctcaaacatataaaaagtcatctaattatgttgagcgcatttgtcataggcgcatattctgcatattggctatggaataataatcaaccgaagccatttttcaaggattacaagactgttgcggaaattaatggctgccattttaatgtaacagaagatacaattgatgggttgaaagagttcgataaatataaaacacggatactggattcggggattaactgtaaaaaacatccgtggttatacttccctcttgcaaaatcctcaccggggatgattgttatggcatgcaataaaaactataaccaacatgaagtggcaaactgtttaaccctgtcttaccgtgaggttaatcgtgattgattataaaaaaaacttattatttattttagtttttatcagtgggtttattctcttcactgtctattcttacactgcagaaaaaatgatatataacgaaacatgcactgcaaattgggtaatttttaatgaccagggacgagcaaatcttaccatcgactttatgtataacaaaaaaaataaaacaggaactgttgcgttgagtggaacctggcaacaaggtaacagagaaagtaaatcaatacggcgaaatattgaatacacatggattgaaaactatgacacagcccatttaacatcaaagaaagttaataagtttgagattatggatcaagttgatgatgatagacttgcacaacttattcctgatttttatgtctttccagaaaaaagtgtaagctataatatactaaagcaaggtaagcatgcttttattttgagcattggtaacagagcaataatgcattgtgcaaggtaaactaaaatagataacaaaaagatggaacctcgttaatcataaaacaataaaattaaatattctcgcagtatatggcagtctaaagcatcaaagatttgatcaacatctttcattttagacatctccttgcaatgtaaaatatcatgtatcaacaacatctggtgcaaatccatgagtcgaactcgacattcatcttagctcgattattattccttcgtacagtcgatgtaaacaatacagaaagaggattattaagaaccagtttactcagtgaatcaatagaggaaaggactaacgtttctttaaaagaattgatttcatcatctgttaaactaaactcatcattgacagatcgtgagatataactgtttttaactttactctttacgttgactttattgacagaattaacattcacatatcttgaatttaatgtccatgatgttgtttgcgtgagaacattctcagcattaaggaatttttttaacggaatccttggtttctttttcgagtccgaatttacaatatcatgcatatagaccatttcatgaatctgcgaaaattcaatgtccattgtatacctcacatttttaccgtgactcgatgttactgttcaataatcaccttccatcaatactaaaattaatacccctaatgtgccgataacaaatatagtcattctacgtaacgtctccataaggtgatatttgacattatcagaagctgcgaattcggattttgctctaatcaaatgagagaaatgtaaaatgaagccacgaaatattaataatagcctaccactgcaaccattagttcctgatcaggagaacaaaaataagaaaaatgaagagaaatccgttaatccagttaaaatcacaatggggtctggtttaaattatattgaacaagaatctcttggaggaaaatatctaacacatgatttgtcaataaagatagcggatatttctgaagagataattcagcaagcaatattatctgctatgagcatatataaattttcgataacagatgatttaatgagtatggctgtaaatgaactcataaaactgaccaaaatagagaataatgtagacctgaataaattcactactatatgcacagacgttctatccccccgcgtcaccagacataataaagaaaaaaacaaacgacattctacccttctcaaaaatcccctttttaattttcattgaaaaaatggcaattgatactatgaatccaggtcatacacattaaggcatttatgtaatgtcgtaattaagataactaataaggtgaatattagtaaaacaactaatgatgttattagtttgtagtgaacagtacttttaccaataatgaaaaatataccataagcaatgcaagcttaaaactcataatttaaaaaagataaatataaaaatatcaatgagtcaatcaataataatttggcatcacgagacacatcacagaggaatattatgagcacagaaacaattgaaatattcaataatagtgatgaatgggcaaatcaactaaaacacgcattatcgaaaggagaaaatctggcattactacatggtttaactcctgatatccttgatagaatatatgcatatgcattcgactaccatgaaaagggtaatataacggacgcagaaatttattataaattcttgtgcatttatgcgttcgaaaatcatgagtatctaaaagattttgcatcagtatgtcagcccaaaaagaaatatcaacaagcatatgacctttacaaactaagttacaattacttcccgtatgatgactattcagttatttatcgtatgggtcaatgtcagattggggctaaaaatatcgataacgcaatgcaatgtttctatcacattattaacaattgtgaggatgatagtgttaagagtaaagcgcaggcatatattgaactcttaaacgataattcagaagataatggctaagcattacaatcatttggttaaatttgctggttatagtgcagttaaccactataaccagcacctcttatgttttcttaaatcagcatcttaaaacagttaagagcatactataaatcattatttttcaatgcgttagagaacaatctactttatcaaaattgaataaggctatttcagattacatcactgaattcctaagataaattagtgaacacaaccatagatatgtcaaatgtaatttcctgtagcgttaatgacacataaatatgaatagccataatttctattgcttaagcaggatgcaagaaaccaattttttcatagaggttaactaatggacttagaaaataaattctcatatcattttcttgagggattaacgctcacggaagatggaattcttactcaaggaaatgagcaagtttatattccacagaaagagttaggtgtattaatagtattacttgaatccgctggtcatgttgtactgaaagatatgatcatcgaatcagtatggaaaaatattattgttagtgacgagtccctgacaagatgtatctattctttgcgctgcatttttgaaaaaattggctatgatcgttgcatagaaacaatctaccggaaaggttatcgtttcagcgggcaggttttcaaaactaaaattaatgaagataatacttcagactattccatagctatattccctttcactacttcattgaatacactggatccattaatacttaatcaggaattagtgcaaatcatttcaaataaaaaaatcgatggtctctatacctatccgatggctgcgacaaatttttgtaatgatcacatatctcaaaattcattcttgagcagattcaagccagattatttcgttacaggaagaataaaccagaataatgcagtgaacactttatacattgagttgatcgacgctaaaaaccttttcctcatcgccagtaatcatctccctgttgatgaactacataatacatcacaatttattatagataatatccttcaaacggtacataaaccagaacgatctgtaagattagctaagcaggaccaaggatataagaatcattatttatcagatgaaatgttagccggaaagaaagaactttacgacttcacccctgaaagcatttacagggccatgactatatttgatagattacaaaataaaagtgatatacagacgctaaaaacagaatgttattgccttctagcggaatgccatatgtctttggcacttcatggaaaaagtgaacttgaacttgctgctcaaaaagcattagagcttttagattatgtatcagacataaccactgtcgatggaaaaattttagctattatgggactgataactggtctgtctggacaagcaaaagtatctcatatcttatttgaacaggctaagatacactcaactgatatagcctctctctactactatagggcactagtccactttcataatgaaaaaattgaagaggcaaggatttgtatagacaaatcactacaactcgaacccagaagacgaaaagcagttgtgataaaagaatgtgtagatatgtatgtgcctaacccgctcaaaaacaacattaaactctactataaagaaactgagagtgaaagccatcgagttataattgacaacattttgaaattaaagcagctgacgagaatttgtatgcgataaatttttattgacgcaattttattatttagatgtatgcaacttgttatttaaacaacagagataaaaatatctaagatattcaccttattgcaagatatttaaaatgctctagagttaaaagtatgatgtaaagaccattggcctggacaattaaaaaagggagctttatgactaatccaatcggtatcaataatttatctcaaagttcaaatatagcgaatgcaacgggtgatgaagtcgtatcattagataaacacatcaacaccagtgctactgatacagatcaaatacaagcatttatagtttcaacatggatggcgccttttcaaaatgatatgtattcagaagataatcctatctcaccttactataaaattgagtggtagacgattgaccaaataaatcataacgagatacttttataatagtatctcgttcctttcattcaatcctcacacatgaaaaaatatgcgctcaccaaaagttaaattcttaaccatcttcacgttttgtatatttattacaaaaatgtctttcgccagcaactcttgctctaatgaagcaggaacaatgttcagaatcgaaccaaatttaattaaagctatcgctcttgttgaaagcaatctaaaaaaggatagcataggcaagaacagagataagaataacaatataaagagtttagattattggttaatgcagataaaccagatgcatattcccctgttaaaaaaacgtggaataataaaagatgaacgagatttgttagataacccttgtctgaacattaaaataggaaccgagattttatataaccatttttcacgttgtggagtaacgtggcaatgcctggggacttataatgcgggttttgcaatggataaccaaaaaaagagacagcaatatgccccaaaatatatattgtatataccaggcttaatgaactagacaatcgtaaggcttcagcaaaatgagcctaaagcctcttttttttatatagtgcaaacacccatacgtaaagctgttttgatcaactcgataccactgtgaacatctaatttcttcatgatattgagtctatgagtttcgactgttttcctgcttaactgcaagaaattagcgatttctttgtttgttttaccatcagctatgagttgtaatatttctgactcacgatttgtaagttgattatcagaggaatacctggaagatattttttcacaatccatatgtacactatcaaaataagtgtaaccattactaatcgaatcaatagcacgatttagtttcgccgggtgactggttttccatacgcatcctttcgcacctgcttcaagcaattttattgaatcaatatacggcatctttgctacaaatgtaataatatgagcatctatcttatgcgatttaacccattttacgagttcggcccccatcattccacctgcaaattctcctaaaataaatatttaggctgtagatttgttacactccgctatagctttcttcagatctttatagcccccaacaacctcatataaatcaggataatgtccgagaaatccaattatcccatcaatcataaacggctgctgatctgaaactacaattttaatttttcccatatattcatcctgagtgtaaatgctttaacgcattcatttataatcatcccttccattattattataagcaaaatccaaagaatacattgatgaaataataatgaaatataattaaaaataaaatttttgcgtaaaaaaataccacaggcattaaaaaatcatgagatgattaaaatattacaattagattatattcaaatcattaaacttgagccagggagctataagtcctcagggcttgccaaaacagaattattcatatccaaagaatgtgtttcaaacattttttcaactaaataatgtctggcttgttcgcagatttcgttaaccttgtcaggggagaaacaatgattattaattaaatattgctcacaattatccacaaattcctgcggactaaattcagcaataaattgatcggtaaaaaacacaaaacgcttatcatcatgaaatgtaatatggacattccatattgatttgtcgacaaaatatgactctacttcaagagacttatctttgaaactggtaggtatatggagatttacaggacctgatattgatggtaattttgttacccaactttcaaaaattttgataaaaacatcaacttcttctgaaggttttaacaatatactcttcagatcgtttatcatgtttattcttttttttcaagttctgagcatagcaagcttatcaagggtataaaattatccatctcatcaataatgccttttgtatagccatcataataaccttgaataaatttttcttctctcttttcctcaatactctgaatttttgcggtggtttcaagaaggattttttctttaagagaaactatttctttcaatccatcagaaatttttcttttaatcacaacaccatttgcaggagattttatcaagctcatctctattttttttcgcataaaatgtaattctctctaaaagtgttgatgcaagtggtaacggcgattgtatgtggtcaacaaaatcaggaaataataaattaaatcgttgctgcattgccaatggttgttgccttatatagggtaacaacgttgaaaaaccacatgtgatgatattgtgatagttagcgatgccgggtttgtatcgtgccttttcatttatttccagcggtatagctgataaataatcccttagtacatcaggaaccttataaaaaaacccgcgttctgcaaacctttctcgataaaagtgacaaccactgagtaaacagatcaatggaagtaaattccaattgtttattggatttgcccctatatttccagacatctgttatcacttaacccattacaagcccgctgccgcagatattcccgtggcgagcgataacccagcgcactatgcggatgccattcgttataatgctcgaacgcctctgcaaggttctttgctgccgttaacccgtctggtttgggcatgatactgatgtagtcacgctttatcgttttcacgaagctctctgctattccgttactctccggactccgcaccgccgtgttcttcggttcaagtcccaacatccgggcgaactggcgtgtttcattagcccggtagcatgaaccattatccgtcagccactccactggagacgacggaagatcgttgccgaagcggcgttccaccgctcccagcatgacgtcctgtactgtttcactgttgaagccgccggtagtgaccgcccagtgcagtgcctcacgatcacagcagtccagcgcgaacgtgacacgcagtctctctccgttatcacagcagaactcgaacccgtcagagcaccatcgctgattgctttctttcacggccactctgcctgtatgtgcccgtttcgatggcggtacagcaggttttcgctcaagcaacagcgcattctggcgcatgatccggtaaacacgtttggcattgatcgcaggcataccatcaagttctgcctgtctgcgaagcagcgcccatacccgacgataaccatacgttggcagctctccgataacatggtgtatacggagaagcacatccgtatcatcagtgtgacgactgcggcggccatccatccagtcatcggttcgtctgagaatgacgtgcaactgcgcacgcgacacccggagacaacggctgactaagcttactccccatccccgggcaataagggcgcgtgcgctatccacttttttgcccgtccatattcaacggcttctttgaggagttcattttccatcgttttcttgccgagcaggcgctggagttctttaatctgcttcatggcggcagcaagttcagaggcaggaacaacctgttctccggcggcgacagcagtaagacttccttcctggtattgcttacgccagagaaataactggctggctgctacaccatgttgccgggcaacgagggagaccgtcatccccggttcaaagctctgctgaacaattgcgatcttttcctgtgtggtacgccgtctgcgtttctccggccctaagacatcaatcatctgttctccaatgactagtctaaaaactagtattaagactatcacttatttaagtgatattggttgtctggagattcagggggccagtctaaacttgctcttttcttctggtgtttatctttgaaagatttgtaggataaataacattaagtaaagccgcatcggcttctctgtaatgtttatctttttccagataacctggggattctccccctaaatcaagctgtaacgttattctttcataacctttatctatgaggtggttcaacctcgttgttgaaagagtttcatccagttcattgactttagcttcgcgtagtaaatcagagacaaaaacagagtctttcttcgagagtaggtttgacaaacgttccagtccagaggtcaccagtgcaacggaagatgtgtttaatcgggcatcttcttcccatgctcaggaatcttccataacatagaaattggctttatccagataagcaatcagcagcgcaaccgactttaatcggtcacctttttgccaatcttcagcgttaatagtaccagtgttgattgcttgtataaggagatcaaggtaaagacctaaagcatcattttgtttatggttccacagctgcggcttgccttcttcctgcacatctgccatcacgggggagttgctgtcaaatcggatatgcacagcattcatttgcacgggaattccatccagtcgttttgggttgctaatgacgtcctgcatccgcttaatctggtcgggcgtagacatataatcccacagggtgagcagaaccttttttgcggctacactatttccctgatctgatactaatgccatatagccccataaactatccctcaaccagacagcatcatagtgggtttctgccgctgttttgtcatcttcgaaagtagaagcaagaataaacgttccccagggtttctccgtcaacgttaactttcgtgtgttttctgttaatgttagcaatccttgaatttcgtctttggtatagtggctctttatttcattttgtaatttggctgagtgaatcagaagacgataattaggatacttatctggatttaacgataaataacttttatctgttgctgcccccgtggaattaagaatgttaaatacagattcactcgtcacttctgcccctgtcgcctggcatgtgccgcacgaaaatataccagcgagcagaagagttaatgcagatttccctttcataaaatattccatcaatcgtttgttaaaagcgtagataaccacttatttaacaacttgaaaataaggtgttttacctgggttgttacaaaaggattgcattgcgtaaacgctttttatttacaacaaaatggggaagtattacggcgaagataaattggagcgggcgaagggaatcgaaccctcgtatagagcttgggaagctctcgttctaccattgaactacgcccgcttcgagatgcgtaaggcattataaaccttacgctctccttagcaagtgccacgctgctgactgctgattaattcgccatcagcattttggcttgctgccctgaggcggcaagtaacgtagcggatcaattgccgttgcacggtaacgaatctggaaatgcaggcgaacagatgccgcatccgtgctccccatagtggcgattttttgcccagccttcacgctttgcccattatttaccagcatcgtgtcattatgggcgtaagccgtaatgtaatcttcactgtgtttaatcatgatgagattaccgtagccacgcagctggttgcccacatacaccacctttcctgcacccgcggcgtaaataggtgtaccccgtggagctgagatatcaatccctttattgccgccatctgctgtcgaatacggcatgataactttccctgtcgttggccataaccaacaacgttgccctactggcggccaggatgatttcggtaccgctgatgacggtgtaaccgatgcggttttggtcgttgatttggcggttgatttacgtgtaatactgctacttttcgccccacccagttttagtttctgaccaacttcaatggtgtaagggggggaaatgccgttcagtcgcgccagttcttttacgctggttcccgtggtgcgcgaaatacgatatagcgtatccccccgtttcacggtgtaaacggagccggaatacgttcctgtatcggatgatttgctacccgaacagcccgccaaaagcagtccaaccgataacaacatcacgatacccagagattttttattcaggcgtcccgcactcaaaatctttcctcgcttaaaaaacaagacgccttatcatagcagccagcctcttgatacccaatctcttgcttctggaaaaacgtggtaatagagaaagaggttaatttcatttggcaaagggaagtatcatcagcaaaatattcgctgtagaggtatcgaacttcctgactttttaccctatttcccatcctgatgcgtaataatcccaatttatcacattgattttatcgccactcatattgatacgtatcactgcccctattcagagtcctgtttcgtatcatatctgtgtttttttaacgtcatcacacttcctacctcccctaacgcttatcgtcgtttctggcgtaaatcttgcctgcttagactaaatctttgccataagaaccaaatgttcaaatcgaggggatttctatggaagcgcgggaagcaaccgctacgggtgaatcatgcatgcgcgtcgatgccattgctaaggtcaccgggcgggcacgatatactgacgattatgttatggcgggcatgtgttatgcgaaatatgtacgtagccctatcgcacatggttatgccgtaagtattaatgatgaacaagccagaagtttgccgggcgtactggcgatttttacctgggaagatgtgcctgatattccattcgctacagctgggcatgcctggacacttgacgaaaacaagcgcgataccgccgatcgcgcactgctaactcgccatgttcgtcatcatggtgacgccgttgccatcgtcgtggcccgcgatgaactcacggcagaaaaagcggcgcaattggtcagcattgagtggcaagaattacccgttatcaccacgccagaagcggcgctggcagaagacgctgcaccaatccataacggtggcaatttactgaaacaaagcacgatgtcgacgggtaatgtccaacaaacaatcgatgccgccgactaccaggtacaggggcactatcagacccccgttattcaacattgtcacatggaaagcgtaacatcgctggcgtggatggaggatgactcgcgaattaccatcgtttccagcacccagatcccgcacattgttcgccgcgtggttggtcaggcgctggatattccctggtcatgcgtacgagtcatcaaaccatttgtcggtggcggttttggtaataaacaggatgtactggaagagccaatggcggcattcctgaccagcaagcttggcggcattccggtgaaagtttcccttagccgtgaagagtgtttcctcgcaacccgtacccgccacgcttttaccattgacgggcaaatgggcgtgaaccgcgacggaacattgaaaggttatagtctggatgttctgtctaacaccggcgcttatgcatctcacgggcactccatcgcttctgcgggggggaataaagtcgcttacctttatcctcgttgtgcctacgcttacagttcaaagacctgctataccaacctcccctcggctggtgcgatgcgtggttatggcgcgccacaagtcgtatttgccgttgagtctatgcttgatgacgccgcgacagcgttaggtattgatcctgttgaaattcgtttacgcaacgccgcccgcgaaggagatgctaatccgctcacgggcaaacgtatttacagcgcagggttgccggagtgtcttgaaaaaggccggaaaatctttgaatgggaaaaacgccgtgcagaatgccagaaccagcaaggcaatttgcgccgcggcgttggcgtcgcctgttttagctacacctctaacacctggcctgtcggcgtagaaatagcaggcgcgcgccttctgatgaatcaggatggaaccatcaacgtgcaaagcggcgcgacggaaatcggtcagggtgccgacaccgtcttctcgcaaatggtggcagaaaccgtgggggttccggtcagcgacgttcgcgttatttcaactcaagataccgacgttacgccgttcgatcccggcgcatttgcctcacgccagagctatgttgccgcgcctgcgctgcgcagtgcggcactattattaaaagagaaaatcatcgctcacgccgcagtcatgctacatcagtcagcgatgaatctgaccctgataaaaggccatatcgtgctggttgaacgaccggaagagccgttaatgtcgttaaaagatttggcgatggacgctttctaccaccctgaacgcggcgggcagctctctgctgaaagctccatcaaaaccaccactaacccaccggcgtttggctgtacctttgttgatctgacggtcgatattgcgctgtgcaaagtcaccatcaaccgcatcctcaacgttcatgattcagggcatattcttaatccactgctggcagaaggtcaggtacacggcggaatgggaatgggcattggctgggcgctatttgaagagatgatcatcgatgctaaaagcggcgtggtccgtaaccccaatctgctggattacaaaatgccgaccatgccggatctgccacaactggaaagcgcgttcgtcgaaatcaatgagccgcaatccgcatacggacataagtcactgggtgagccaccaataattcctgttgccgctgctattcgtaacgcggtgaagatggctaccggtgttgcaatcaatacactgccgctgacgccaaaacggttatatgaagagttccatctggcaggattgatttgaggataacatcatgtttgattttgcttcttaccatcgcgcagcaacccttgccgatgccatcaacctgctggctgacaacccgcaggccaaactgctcgccggtggcactgacgtactgattcagctccaccatcacaatgaccgttatcgccatattgttgatattcataatctggcggagctgcggggaattacgctggcggaagatggctcgctacgtatcggctctgcaacgacatttacccagctaatagaagatcctataactcaacgtcatctcccggcgttatgtgctgcggccacgtccattgctggaccgcagatccgtaacgtcgctacctacggtggaaatatttgcaacggtgccaccagcgcagattctgccacgccaacgctaatttatgacgcgaaactggagatccactccccgcgcggtgttcgtttcgtcccgattaatggctttcacaccgggccgggcaaagtgtctcttgagcatgacgaaatcctcgtcgcctttcattttccgccacagccgaaagaacacgcgggcagcgcgcattttaaatatgccatgcgcgacgcaatggatatttcaacgattggctgcgccgcacattgccgactggataacggcaatttcagcgaattacgcctggcatttggtgttgccgcgccaacgccgattcgctgccaacatgccgaacagactgcacaaaatgcgccattaaacctgcaaacgctggaagctatcagcgaatctgtcctgcaagatgtcgccccgcgttcttcatggcgggccagtaaagagtttcgtctgcatctcatccagacgatgaccaaaaaagtgattagcgaagccgtcgccgcggcggggggaaaattgcaatgaatcacagcgaaacaattaccatcgaatgcaccattaacgggatgccttttcagcttcacgccgcaccaggcacgccgctctcggaattactccgcgaacaaggactgctaagtgtcaaacaagggtgctgcgtgggtgaatgtggtgcctgtacggtgttggtcgacggcacagcaatagacagttgcttataccttgccgcctgggctgaaggaaaagagatccgcacgctggaaggtgaagcgaaaggcggaaaactttctcatgttcagcaggcttatgcgaaatccggcgcagtgcagtgcgggttttgtacgcctggcctgattatggctaccacggcaatgctggcgaaaccacgcgagaagccattaaccattacggaaattcgtcgcggactggcgggaaatctttgtcgctgcacggggtatcagatgattgtaaatacagttctggattgcgagaaaacgaagtaaaaggatatccggcctgaattcaggccggattcactgaggttatgtgtttaacaactcatatttcttaatcttgcgatagagcgtagcaatgccgatgcccagttcatcagcaacttgcttcttgctgttatgacgtgaaagcgcctcgcggatcatttgcttttccatctcctccagcgccgtgccgcccgcatcatcgagtgacaggtgcgcctcactgacctctgttacatcactttgctccgttgtgccattattcagcagatttggcggcaatagcgtgctgtcgataacttcacctgaaggaaccacgttaaccagatattccatcaaattgcttaactcgcgcaggtttccgggccaacgatgcttacgcaatatttcgacgacatcgggagcaatgccaggataaaccgatcccagacgacgggtatgcagatgtaaaaagtaatgcaccaatagttcaatatcttcctgacgttcacgcagcggtggcagagttatcgggataacattaagtcggtagaagagatcttcgcggaatttaccttcggcaatgaactgggccaaattctgattagttgcagaaatgatgcgaatgtcgacttgtattgggctactggcaccaatcggcagaatttcacgtgcctcaatagcgcgcagtaatttagcctgcaacattaatggcatatcacctatttcatcgagaaacagcgtgcccgtattcgccgcctgaatcaaccctgttttaccgttggcagaagcgccagtaaatgcacctttaacataaccgaacagttcgctctccagaagctgctccggaatcgcggcacagttgatagcaataaagggtttattccgtcttccgctcaacttatggattgcacgggcgacgacttctttacccgtgccgctttcaccaaccaccataacgctggatgggctgggtgcaatacggctaatgagtcgttttaattgccgcataacacggcactcgccaaccaattgttcaatatgcggttcatcaggtgcatttgctacagaaaaactggtatgcgattggtgaaacgccattaaaaataattgtcggccctgaatgttatgcaattgaccaatgattaattcacttttatcgtcccatgaaacaatatgctgcatatgtccatgggtaaaattactctcaaatgttaatggtctgaaacggataggtttcccaataatattattttgcacaacaccaagtgtttttaaggcagtctgattaacaaactgaacccgattttcatcatctacaactaatacgccctgatccatattatcgatcatggtcgcaaatattttactgatgttatctcctggcccctgatcctccagaagtttcgaaacaaaaatggtggatatatggcgaacataatcagaaaattcgcgtaaattatcactgatatgctcttgttgctcgtgggtaacggcaatcaaacttatcaccccaacacaacgatcctgtaaaatgacaggcgtacccagaaatgctttttcgcggcaattttctttactatcgcaaccttcgcaaaggggatcgaagcgagactgtgtcacaactttttcagttttcgtttccaggacgtggcggagcaggcgtgagttgccgctcaactggcgaccaagaaacttcccatacgcgcccgttccggcaacgcgacacaagttttcatcaacgatctcaacctcaagctgcaaaacgctggcaagcattctggcaaaacgctgaattgtcggttgaatttgcatcaatactgactgcgtagtagcaagctccatagctttaccttccagacttacttaaaagtcgatcattgaagacgttgatggttcacagatcatgatgatattaactcaggcgaaattggctttgataaaaacataagatttttatcattttctaatgaaattatggaagagatatcacatttctatatcaatatgagaattacggcggtgagtttatcaaactgaagagagatagcctgcccctttatcttatttctgatacttagcagcaaataaataacgcgataaaaaaagccaaacgttttcgtattttacaaacaaccagaagctggcatcaatttgtgatcaaccccacacattatccgtcaaattagtcttttgcagccgcgcggataattctggcacacttattgttagtcccaggtatagctgtgaaaacaccaatcactttggcaagtcacagtgaaataaaccactttgcctgtcattccactaccgggactttatgatgaaaactgttaatgagctgattaaggatatcaattcgctgacctctcaccttcacgagaaagattttttgttaacgtgggaacagacgccagatgaactgaaacaagtactggacgttgccgcagcattaaaagcactgcgtgctgaaaacatctcaaccaaagtctttaatagtggattaggtatttccgtattccgcgacaactccacccgtacccgcttctcttatgcttccgcgcttaacctgctcggccttgcacaacaagatctcgacgaaggcaaatcacaaatcgctcacggcgaaaccgtgcgtgaaaccgccaatatgatctccttctgcgccgacgctattggtattcgcgacgatatgtatctgggcgcaggcaacgcctatatgcgtgaagttggcgctgcacttgatgacggttacaagcagggtgtactgccacagcgtccggctttagtgaacctgcaatgcgatattgaccacccgactcagtcaatggctgacctcgcgtggttacgtgaacactttggttcactggaaaacctgaaaggtaaaaaaatcgccatgacctgggcctactctccaagctatggcaaaccgctctctgtaccacaaggcatcatcggtctgatgactcgcttcggtatggatgtcaccctggcccatccggaaggctacgacctgatcccggatgtggttgaagtggcgaaaaacaatgctaaagcctccggtggtagcttccgtcaggtcaccagcatggaagaagccttcaaagacgcagacatcgtttatccgaagtcatgggcaccttacaaagtgatggaagagcgtactgaattgctgcgtgcgaacgatcacgaaggcttaaaagcactggaaaaacagtgtctggcacagaacgcgcaacacaaagactggcattgtactgaagagatgatggaactgacccgtgatggcgaagccctgtacatgcactgcctgccagctgatatcagcggcgtatcctgtaaagaaggtgaagtgactgaaggcgtattcgaaaaataccgtatcgctacctacaaagaagccagctggaagccttatatcatcgccgcgatgatcctgtcccgtaaatacgccaaaccaggtgcactgctcgagcaactgctgaaagaagcgcaagaacgcgtgaaataacccctcgggccgatcagctggtcggccctctatttccagaggccaaaaggataggatatgtccgttttctcattgaagattgatatcgccgataacaaatttttcaacggcgaaacatcaccgctcttttcgcaaagccaggccaaactggcgcgccagttccaccagaaaatagctggttatcgcccaacaccgctttgtgcgctggacgatctcgcaaacctttttggtgtgaagaaaattctcgtcaaagacgaatcaaaacgattcggtctgaacgccttcaaaatgcttggcggtgcgtacgccatcgctcaattattgtgtgaaaaatatcatcttgatatcgaaacgctgtcatttgagcacctgaaaaatgccatcggcgaaaaaatgactttcgcgaccaccaccgacggcaaccacgggcgcggtgtggcgtgggcagcacagcaactcggacagaatgcggtgatttacatgccgaaaggttctgctcaggaacgcgttgacgccattctgaacctcggtgccgagtgcatcgtcacggatatgaactatgacgataccgttcgcctgaccatgcaacacgcgcagcagcacggctgggaagtggtacaggacacggcatgggaaggttacaccaaaatcccaacctggatcatgcaaggctacgcaaccctggcagatgaagccgtcgagcaaatgcgtgaaatgggcgtaaccccgacgcacgttctgctgcaagccggtgtcggagcaatggccggtggtgtgctgggttatctggtcgacgtctatagcccgcaaaatctgcacagcattattgttgaacctgacaaagctgactgtatttatcgctccggcgtcaaaggcgacatcgtcaacgttggcggtgatatggccaccatcatggcaggcctggcctgtggcgaacctaacccgctgggctgggaaatcctacgtaactgcgccacccaattcatctcctgccaggacagcgttgccgcattaggtatgcgcgtgctgggtaatccgtacggcaacgacccgcgcatcatctccggtgaatccggcgctgtcggtttgggcgttctcgcagcggttcattatcacccgcaacgtcaaagcctgatggaaaaactggcgctgaacaaagatgccgtggtgctggttatcagcactgaaggcgacaccgacgtgaagcactaccgcgaagttgtctgggaaggcaaacacgctgtagcaccttaatcaccctattggaactgctccctgcaaaacggggagtaaaaaatctggagaaaaataatggctaagaatattccattcaaactgattcttgaaaaagcaaaagattaccaggcggatatgactcgcttcctgcgcgacatggttgctattcccagtgaaagctgcgacgagaaacgcgtagtacatcgtattaaagaagagatggaaaaagtcggcttcgataaagttgaaatcgacccgatgggcaacgttctcggttatatcggccacggcccgcgtctggtggcaatggacgctcatatcgataccgtcggcattggcaacatcaaaaactgggacttcgatccgtacgaaggcatggaaactgatgaactgattggtggtcgcggtacttccgaccaggaaggtggcatggcctctatggtttatgccggtaaaatcattaaagacctcggtctggaagatgaatataccctgctggttaccggtacggtgcaggaagaagactgcgacggtctgtgctggcagtacattattgaacaatccggcattcgcccggaatttgtggtcagtaccgaaccaaccgactgccaggtataccgtggtcagcgcggtcgtatggaaattcgtattgatgttcagggtgttagctgccacggttctgcaccagaacgcggtgataacgccattttcaaaatgggtccgattcttggcgaattacaagaactctcccaacgtctgggttatgacgaattcctcggcaaaggcaccctcaccgtttctgaaatcttcttcacatccccaagccgttgcgctgtagcagacagctgcgcagtttcaatcgaccgtcgtctgacctggggcgaaacctgggaaggcgcgctggacgaaatccgcgccctgcctgcagtacagaaagctaacgcggttgtttctatgtacaactacgaccgtccgtcctggactggcctggtttacccaaccgaatgctacttcccgacctggaaagtggaagaagatcacttcaccgttaaagcactggtgaatgcctacgaagggctgtttggcaaagcgccggttgttgataagtggaccttctcaactaacggcgtatctatcatgggccgtcacggcattccggtgatcggctttggcccgggtaaagaacctgaagcgcatgcacctaacgaaaaaacctggaaatctcacctggtgacctgtgccgcgatgtacgctgcaatcccgttaagctggctggcaacagagtaattactcttcacttattcccctccggttcgccggagggtttttggagtttgctatgcgcgtattgatcaaaaacggcactgtcgttaacgcagatggacaagccaaacaggatttgctgattgaaagcgggattgttcgccagttgggcaacaatatttcgccgcagctcccgtatgaagaaattgatgccactggctgttacgttttccctggcggcgtggatgtccatacgcatttcaatattgatgtcggcatcgcgcgcagttgtgatgatttttttaccggtacccgcgcagctgcgtgtggcggtacaacaaccattattgaccatatgggatttggcccaaacggctgtcggttacgccatcaactggaggtttatcgtggttatgccgcccataaagcggtcatcgattacagctttcacggtgtgatccagcacattaatcacgcaatcctcgacgaaatcccgatgatagtcgaggaaggactgagcagttttaaactctatttaacctatcaatacaaactcaacgatgacgaggttttgcaggcattacgccgcttgcatgaatccggcgcgctgaccaccgtgcacccggaaaatgatgcggctatcgccagcaagcgggcggaatttatcgccgcagggttaaccgcgccgcgctatcatgccttgagtcgccctctggaatgcgaagcggaagccatcgcccgcatgattaacctggcacaaattgccggtaacgccccgctctatatcgtgcacctgtctaacggcttaggtctggattatctgcgtcttgcccgtgcgaatcaccagccagtctgggttgaaacctgcccacaatatctcctgttggacgaacgcagttacgatacagaagatggcatgaagttcattcttagcccaccgctgcgtaacgtacgcgagcaggacaaactgtggtgtggcatcagcgatggtgcgattgacgtggtggcaaccgatcactgcaccttctcgatggctcaacgcctgcaaatttctaaaggcgatttcagtcgctgcccaaatggcttacccggtgtggaaaaccgcatgcagttactgttttccagtggcgtgatgacgggacgtataacaccggaacgctttgttgaattaaccagcgcaatgcccgccaggttgtttggcctgtggccgcaaaaaggattattagcgcccggttccgacggcgacgtggtgattatcgacccacgtcagagccaacaaattcagcatcgccatctccacgacaacgccgactactcgccatgggagggttttacctgtcagggcgcgattgtcagaaccttatcccgtggtgaaacgattttctgtgacggcacctttacaggcaaagccgggcgaggtcgtttcctgcgacgcaaaccgtttgtccctcccgtgctctaaccactgccagggatctatacacaatcaagaatgatgagtgaggaaaaatgagtaagaaaattgttctcgccctgggcgggaatgcgctgggcgatgacctggccgggcaaatgaaagcggtaaaaattacttctcaggcaattgttgatttaattgcccagggacatgaagttatcgtcactcatggtaacgggccgcaggtgggcatgattaaccaggcctttgaagctgccgcaaaaactgaagcgcactcgccaatgctgccgatgtctgtctgtgttgcattaagccagggttatattggttacgatctacaaaacgctttaagagaagaactgctttctcggggcattaataaacctgtagcaacgctggttactcaggtcgaagtcgacgctaacgatccggcattcctcaacccgaccaagccgatcggttcgttctttaccgagcaagaagcagagcaactgacaaaacagggttacactctgaaagaagatgctggtcgcggctatcgccgtgttgttgcctcgccaaaaccggttgatatcattgaaaaagaaacggttaaagctctggtagatgcaggtcaggtggtgatcaccgttggcggtggtggtatccctgttattcgtgaaggtaaccatctgcgtggtgccagcgcggttatcgataaagactgggccagcgcccgtttagcagaaatgattgatgccgatatgctgatcattctgactgcggtagaaaaagtggccattaacttcggtaaagagaatgaacagtggctcgatcgcctgtcattaagtgatgctgaacgctttatcgaagaaggtcattttgcgaaaggttctatgctgcctaaagtggaagctgccgcctcgtttgctcgctctcgcgcaggtcgtgaagcactgattaccgtattgagcaaagcgaaagaagggattgaaggcaaaacaggaacggtgatttgtcagtaatttaaaggccgggtgggtaataccatccggccaaagattgtcaagtaagtgcgctttgttgatgccggatgcggcgcgagcgccttatccgtcctacaaaacatcgcaaattcaatagattgcaatgcacttgtaggcctgataagcgtagcgcatcaggcaatttggcgtttgtcatcagtctcaggccgggtgggtaataccatccggccattttcatttaagccacttccagcacttcttttgtcgctttcacgccctgatgcatcaacatcattaacgcctcaagtacgccgccgccaatcgcccgggctttatcagaaacgctggtgaaatcagcggtttcaccacgaggatcgatatcaccaattttaaaaccaccaaccactgccaggccgtcgttcaacaagccacgcaccatccccgtcaacggtgctttaatttcatgctcaccaatccaggcaatcacatcgccctctttcaccagatcgcctaatttcacgttggatcgcataatgcctgcagcaggagcacggatcacccgtcgggtggtatgccccataatattgccaggaacaccggtattctcctgcgcacaaccagagtaaatcacctgaccgagccagtgcccgcgatttgtttcaattaccgcatgacaatccttcccagcagtaaagcccggcccaagcgcgattgttactggtgccatatctgcccgcgttcccaaattctgtttcgccagaatagcgtccaccacgcaaagcggtttcagttcatcaagcaatgaacaggcgggatctaccatcacaggaatgaatccgcgttcggtaagtttcatcgcttccgcagagctggttgccaggcgagcagtgacgccttcgaccgtcatttcgccatcgaacacggcctgggcaaacgccacggtacaacgaatcactgtcggtttttccacttccagcatgatcactttaaaacccgcatgatacagacgtagcgccacaccactggcgatatctcccgcaccgcgaatcaccaccagctggtgtccggaaggatgagaaggtttcatcatcagcccacccggcgcgttatttttcacctgtaatatttctgccagcacgctgatggcgatctcctgcggcgtttccgcacctatgttgtaaccaacgggcgcatgtaaacgggcaatatgttcttcagccacgcctttctcacgcaattgacgcaggaaaagctgaaccttgcgacgacttgccagcaaccccaaccatgcaatgggctgttcaatgagtttgtcgagggcttcacgatcctgattattcgtggcaatcaggacaaaattatcagggcgaatatccagtgcttccactgccgcaccaaacgactcagcatggagaagcgtggttgatggtgggaatagttcaggattgaggctttcgcgataaatatcagcaacggcaatatcaaatcctaatagcgccgcactctgggctatcgcccggttgacatgccccgcgccaatcaacaccagacgtggacgcataccatggacgctgataaatactgacattgcacctccacaatctgacccgacagcatccgcaccgttacgagccatacgtccatggaataatcgcggcttacgttcctgcaatgcctgaagcgactcttcaatcaccttccgctcaaccattccgccaccaattgtaccgacgatagaaccatcggcgcgcactaacatttgtgcagaatggcggggagtcgagcctcggctatcaacaatttgcgccatagcaaacggacaattttgctcttcgagttttgcagcctctgtgaaaatattcataccaacctcaatggatatcctttcagtaacccggaatacccgggccgctaattcacaaatctgcgcgcgattgcaggatgttcttgtatatcgcccagccagattgcctctacgtcgtgttgttgcagcggttgaaggagctcgctttgtgcaatcgcattctcacattgagaaaaacggttaatgaaccagactcgccgacaaccttgcggtacgtttttaaacgccccctgagggtggcgaaccagcgcaacgagatcgctcagttgcaaggttgcatcaggtgttaacccggtaatatcagcaaactgcgaccagcgatggacattttctgtgctcactttcgcgcccaaagtatgtcctcccatcacagcaatcacgcagcaactgcttttgggtatgcaaggttcgtgctcatcaggcgcttttaacggcattccacgcgagccatctgcttcaatgagaattacgtcacactctggtcgttgcaccagtgcatcaatcgcttctggcgtaaatccctgcacttttccctggttcgctttccagctgtgaaaacaaaatgaaatgggggatgtaagagacgcatgaggaagcatggcgggatcacgacagaaaaccacgggccagtgagacgttggcataaacatatgtgtcgtcgtcgtgattaacacacgcctgccgctagcctggagcagttctgccagccaaaaaagcaagctggttttccccccagcaccaacaacagaaatcacagtgggacgtttctgcgcacctaaatcaatgactaatgccgatgggtcaactatacttttcacgagtctttatgacctctctgggataaattatccccaacttaatccatcaggaagtaacgcaattatcaggcgttattagcccctataaataatggaaccactatgtcagccatcgactgtataattaccgctgccggattatcatcaagaatggggcaatggaaaatgatgttaccctgggaacagggaacaattcttgatacaagtatcaaaaatgcgttgcagttttgtagccgaattattttagtcaccggctatcgtggtaatgaactgcacgaacgttatgcgaaccagagcaatatcactattattcacaacccagattatgcgcagggtttactaacatccgtcaaggccgcagtacccgcagtgcaaacagaacattgttttctcacccacggtgacatgccaaccctcaccatcgatatttttagaaaaatctggtcgttacgaaatgatggcgcaatactgccactccataatggcatccccggccatccgattttagtgtcaaaaccatgcctgatgcaggcaatccaacgacccaatgtcaccaatatgcgtcaggcactccttatgggagatcattattccgtcgaaatagaaaatgcagaaataattttagatattgatactccggacgactttattacagcgaaggaaaggtatactgaaatttagaaaacgtagttaaacgattgcgttcaaatatttaatccttccggcactcattatcataatgataaggaatcactgattttgagaaaagagaaaaattgataaatgggctggcaataataattttcaggagtgattttaattctcatttagcacctgtgagttcattcacaaaaagcccttaagtttcgagccgcctcacatttttttatatttcccgccaaacctggcaagagtggtgcgattgttgctctatccccctaaaccaccggatttctcaacaccggtcactcaatgatatctgtataagctaaggagagggttatgggggatattatgcgtcccattccgtttgaggaacttttgacgcgcatatttgatgaataccaacaacaacgctcaatctttggtattcccgagcaacagttttactcacctgtaaaaggtaaaactgttagcgtcttcggtgaaacctgtgccactcccgtcggccctgccgctggcccgcacacgcagctcgcgcaaaatattgtcacttcctggctgactggcggacgcttcatcgaactaaaaaccgtccaaattcttgaccgcctggagctggaaaagccctgtatcgatgccgaagacgagtgctttaacaccgaatggtctaccgagtttaccctgcttaaagcctgggatgaatacctcaaagcctggtttgccctgcaccttctcgaagcgatgttccagccttctgattccggtaaatcgttcatctttaatatgagcgtcggttacaacctcgaaggtattaagcaaccgccgatgcaacagttcatcgacaatatgatggacgcatctgaccatccgaaattcgctcaatatcgcgatacgctgaataaattactccaggatgacgcatttttagctcgccacggattgcaggaaaaacgcgaaagcttgcaagccttacccgctcgcatccccaccagtatggtgcatggcgtcaccctctccaccatgcacggctgtcctccgcatgaaatcgaagccatttgccgctacatgctggaagaaaaagggctcaacacctttgtgaaacttaacccgaccttactggggtacgcgcgtgttcgtgagatcctcgatgtctgcggtttcggttacataggcttaaaagaagagtcatttgatcacgacctcaagctgacgcaagcactggaaatgctggaacgcctgatggcactggcaaaagaaaaatcactcggctttggcgtaaaactgactaacactctcggcaccatcaacaataaaggcgcactgcctggtgaagagatgtatatgtcaggccgtgcgctgttcccgctctccatcaatgttgcagcagttctctctcgcgcctttgacggcaaactgcccatttcttattccggtggtgccagtcagctgactatccgcgatatttttgatacaggtattcgccctattactatggcaaccgacctgctgaaacctggcggctatctgcgcttaagtgcctgcatgcgcgagctggaaggctccgacgcctggggacttgaccatgttgacgtcgaacgactgaacagactggcagcagatgcgttaaccatggaatacacccagaaacactggaagccagaagagcgtattgaagtggcagaagacctgccgctgaccgactgctacgttgccccctgtgttactgcctgcgctatcaagcaagatattccggaatacatccgtctgcttggcgaacaccgctatgccgacgcgctggaactcatctaccaacgcaacgctctgcccgccattaccggtcatatttgcgatcaccagtgccaatacaactgtacccgcctggattacgacagtgcgctgaatatccgcgaactgaaaaaagtcgcgctggaaaaaggttgggatgaatataagcaacgctggcacaaaccagccggttctggttcacgccatccggttgccgtgattggtgcaggtccggcgggtctggcagcaggttacttccttgccagagcgggccatccggttacgctgtttgaacgcgaagccaatgcgggcggcgtggtgaaaaatatcattcctcagttccgtattcctgcagagttaattcagcacgatatcgattttgttgccgctcacggcgtgaaatttgagtatggctgctcacccgatttaaccattgagcagttaaaaaatcagggcttccactatgttctgattgccaccggcactgataaaaatagcggtgtgaaactggcgggcgacaaccaaaatgtctggaaatcactccccttcctgcgtgaatacaacaagggtacagcgctcaagctgggcaaacatgtggtcgttgtcggggcgggtaacaccgcaatggactgcgctcgtgcggcgttacgcgttccaggcgtagaaaaagcaacgatcgtttaccgtcgttcactacaagagatgcccgcatggcgcgaagagtatgaagaagcgttgcacgacggcgtagagttccgtttcctgaataatccggaacgtttcgatgctgatggcaccttaaccttgcgcgttatgtcgcttggcgaaccggatgagaaaggtcgtcgtcgtccggttgaaaccaatgaaacagtaacactgcttgtagacagcctgatcaccgccattggtgaacagcaggatactgaagccctgaatgcgatgggcgtgccgctggacaaaaacggctggccagacgtcgaccataatggcgaaactcgtctgactgacgtctttatgatcggcgacgtacagcgcggaccatcctccattgtcgctgctgtcggaaccgcgcgtcgggcgaccgatgccatccttagtcgggaaaatatccgttcccaccagaacgataaatactggaacaacgtcaatccagcggaaatctatcaacgtaaaggcgatatctctatcacgctggtgaacagtgacgatcgtgacgcgtttgtcgcccaggaagccgctcgctgcctcgaatgtaactacgtttgcagcaagtgtgtggatgtctgcccgaaccgcgccaacgtctccattgcggtcccaggcttccagaaccgtttccagacgctgcacctcgacgcttactgtaacgaatgcggcaactgcgctcagttctgtccgtggaacggtaaaccgtacaaagacaaaatcaccgtcttcagcctggcgcaagactttgataacagcagcaacccaggcttccttgtggaagattgccgggtacgagtacgtctgaataaccaaagctgggtgttaaacatcgacagcaaaggtcagtttaacaacgtaccaccggagctgaacgatatgtgccgcatcatcagccatgtccaccagcatcatcattatctgctgggccgcgtggaggtgtaatcatgttgattctgaagaatgtcactgcggtacagctacacccggcaaaagtgcaggaaggcgttgatatcgccatcgaaaacgatgtgattgtcgctatcggcgatgccctgacgcaacgctaccccgacgccagcttcaaagagatgcatggccggattgtgatgccagggattgtctgctcgcacaaccatttttactcggggctttcccgcggaattatggcaaacatcgccccttgcccggatttcatctcaacgctgaaaaatctctggtggcggctcgatcgcgcccttgatgaagagtcgctctattacagcggactgatttgttccctggaagcgattaagagcggatgtacatcggttatcgatcaccatgcctctccggcgtatatcggcgggtcgctctccacattgcgcgacgcatttttaaaagttggcctgcgcgcgatgacctgttttgaaactactgaccgtaacaacggcatcaaagagttgcaggaaggtgtagaagaaaacatccgtttcgcccgtttgattgatgaggcgaagaaagcgacaagcgagccgtatctggtggaagcacatatcggtgctcacgcgccgtttaccgtgccggatgccggtctggagatgctgcgtgaagccgtgaaagccacaggccgtggtttgcatattcacgctgcggaagacctttacgacgtttcctacagtcaccactggtacggcaaagacctgctggcacgactggcgcaattcgatctcatcgacagcaaaacgctggtcgctcatgggctgtacttgtcgaaagatgacatcaccctactcaatcagcgcgatgcgttcctggtgcataacgcccgttcaaacatgaacaaccatgtcggctacaaccatcaccttagcgacatccgcaatctggcgttgggaacggacggcattggttcggacatgtttgaagagatgaaatttgccttctttaaacatcgcgatgcgggtggtccgctgtggcctgacagttttgccaaagccctgactaacggtaacgaactgatgagccgcaactttggcgcgaaatttgggcttctggaagccggttacaaagctgatttaaccatttgcgattacaactcgccgacgccgctgctggcagacaatatcgccgggcatatcgctttcggtatgggctcaggcagcgttcacagcgtgatggtcaatggtgtgatggtctatgaagaccgtcagtttaacttcgattgcgattccatttatgcacaagccagaaaagccgctgccagtatgtggcgtcggatggatgcgctggcataaatgacagatgccctcttcccgcagggaagagggttaaataaggaaagaagatgattgaacaatttttcaggcccgactctgtcgaacaggcgctggaactgaagcgccgctaccaggatgaagccgtctggttcgccgggggcagcaaactcaatgctacaccaacccgtaccgataaaaagattgccatttccttacaggatctggaactggactgggttgactgggataacggtgcactgcggattggcgcaatgtctcgcttgcagccactgcgtgatgcgcgatttattcctgcagcgctgcgtgaagccctcggttttgtttactcacgccatgttcgtaatcagtcgaccattggtggtgaaatcgccgcccgccaggaagagtcggtgctgcttcccgtcctgttggcactggatgctgaactggtttttggcaacggcgaaacgctgtcaatcgaggactacctggcctgcccatgcgatcgcctgctaaccgaaattatcattaaagatccgtatcgcacctgtgcgacccgcaaaattagccgttctcaggcaggtttaaccgtcgtgacggcagccgttgcaatgacagaccacgacggtatgcgaattgcgctggatggcgtcgccagtaaagcactgcgtctgcatgatgtcgaaaaacaaaatctggaaggcaatgcacttgaacaggctgtcgccaacgccattttcccgcaggaagatttgcggggcagcgtggcctataaacgctatatcacgggagttctggtagccgacctgtatgccgactgccaacaggctggggaggaagccgtatgatcatccactttactttaaatggcgcgcctcaggagctaaccgttaatccaggcgaaaacgtgcaaaagctgttgtttaacatgggaatgcactctgtacgcaacagtgatgatggtttcgggtttgccggttctgacgcaataatctttaacggtaatatcgttaacgcgtccttgcttattgccgcacagttagagaaggcagatattcgtaccgcagaatctctgggcaaatggaacgagttaagtctggttcaacaggcaatggttgatgttggcgtggtgcagtctggttataacgatccagctgcagctctgattatcaccgatcttctcgatcgcatcgccgcacctacccgcgaagagatcgacgacgcgctttctggtttgttcagccgcgatgctggctggcagcaatactatcaggtcattgaactggcggttgcacgtaaaaataatccgcaggccaccattgatatcgctccgactttccgtgacgacctagaagtcattggtaagcattatcctaaaactgatgccgcgaaaatggtgcaggcgaaaccctgctatgttgaagaccgcgtaacggctgacgcctgcgtcattaaaatgttacgtagcccacacgctcacgcactgattactcatctggatgtcagcaaagctgaagccttaccgggcgtcgttcacgttattactcacctgaattgcccggatatctactataccccgggtggtcagagcgcaccggaaccgtcaccgcttgaccgccgtatgttcggcaagaaaatgcgtcacgtcggcgatcgtgttgctgcggtcgtcgcagaaagtgaagaaattgcgctcgaagcactgaagctcatcgacgttgaatatgaagtgcttaagccggtaatgtcgatcgacgaagcaatggcggaagatgcgcctgtcgtgcacgatgaaccggtggtgtatgttgctggtgcgccagatactctggaagacgataacagccatgcagcccagcgcggcgagcatatgatcatcaacttcccgatcggttctcgccctcgcaaaaatatcgccgccagtattcatggtcatattggcgatatggacaaaggctttgccgatgccgatgtgatcattgagcgaacctataactcaacgcaagcgcagcagtgcccgactgaaacacatatctgctttactcgtatggacggcgatcgtctggttatccacgcctccacccaggtaccatggcacttacgccgccaggtcgcgcgcctcgtgggcatgaaacagcataaagttcatgtcattaaagagcgagttggcggcggttttggttccaaacaggacatcctgctggaagaagtgtgcgcctgggcaacctgcgtgaccgggcgtccggtactgttccgctacacccgtgaagaagagtttattgctaacacctctcgtcacgtcgcgaaagtcaccgtcaaactgggagcgaaaaaagatggtcgcctgacggcagtgaagatggatttccgcgccaacactggcccttacggcaaccactcactcaccgtaccgtgtaacggaccggcgctgtcgctgccgttatatccgtgcgataacgtcgatttccaggtcaccacctactacagcaacatttgcccaaatggtgcttatcagggttatggcgcaccgaaaggtaacttcgctatcaccatggcattagcggaactggctgaacagttacagatcgaccaactggaaattatcgaacgtaaccgggtacacgaagggcaagagctgaaaattctcggtgcaatcggtgaaggtaaagcgccgacctccgttccttccgccgccagctgtgcactggaagagatcctgcgtcagggtcgcgagatgatccaatggtcgtcaccgaaaccgcaaaatggtgactggcacatcggtcgcggcgtcgccattatcatgcagaaatcgggtatcccggatatcgatcaggctaactgcatgatcaaactggaatcggacggcacctttatcgttcattctggcggtgcggatattggtactggtctggatactgtagtgacgaaactggcagcagaagtgctgcactgcccaccgcaggacgtgcatgttatctccggtgataccgatcatgcgttgtttgataaaggcgcatatgcctcgtccggtacttgcttctcgggtaacgcggcgcgtttggcagcggaaaatctacgggagaaaattctgttccacggcgcgcaaatgttgggtgagccagtggcagatgttcaactggcaacgccgggcgtcgtgcgcggcaagaaaggcgaagttagtttcggggatattgcccataaaggcgaaaccggcaccggctttggttcactggtgggaactggcagttatatcacgcctgatttcgccttcccgtatggcgcaaacttcgctgaagttgccgtcaacacgcgtacgggtgaaatccgcctggataaattctacgccttgctggactgcggtacaccggtcaatccagagttagcgttgggacaaatctacggtgccaccctgcgtgctatcggccacagtatgagcgaagagatcatttatgacgccgaaggtcacccgttaacgcgtgatttacgcagttacggcgcaccgaaaattggtgacattccgcgtgatttccgcgctgtgctggtgccgagcgacgataaagtcggcccgttcggggcgaaatcgatctcggaaatcggtgtaaatggcgcagctccggcgattgctaccgcaattcacgatgcatgcggcatctggttacgcgaatggcatttcacaccggagaaaatactcactgcgctggaaaaaatataaataataaatggccgcttcggcggcctgtttctctgtttgaacgatgactaaatagtgactgcgaaaatgagataagccgttctcaaggcgtcctgcgccccaaattcgtgggaatttattttactaattcagatgatcaaatttactttaaaaggagtgaagggatgtctgatataaaccatgcaggttctgaccttatatttgaactggaggatcgccctccctttcatcaggctctcgttggtgccattacccatctgttggcaattttcgttccgatggtaacccccgcgttaatcgtgggtgcggccttacagctttccgctgaaacaactgcctatcttgtttctatggcgatgatcgcctctggtattggtacctggttacaagtaaaccgctacggcatcgtcggttctggcctactctcaattcagtcagtcaatttttcatttgttacggtcatgattgcgctgggcagcagcatgaaaagcgacggttttcacgaagagttaatcatgtcgtcgcttctcggcgtctccttcgttggcgcatttctggttgtcggatcttcatttatcttgccctatttacgtcgggttattacgcctaccgtcagcggtattgtggtactgatgatcggcttaagcctgattaaagtcggcattatcgattttggtggaggatttgcagccaaaagcagcggtacgttcggcaattacgaacatctcggcgttggtttattggttttaattgtggtgatcggctttaactgctgtcgcagtccgttgctacgcatgggagggatcgccattgggctatgtgtcggctatatcgcatcgttatgcctgggcatggtggatttcagcagtatgcgcaatttgccgttaatcaccatcccgcatccgttcaaatacggctttagttttagcttccatcagttcctggtggttggcacgatttatctgcttagcgtgctggaagcagtcggcgatatcaccgccacggcaatggtttcccgccgccccattcagggggaagagtatcagtcccggctgaaaggcggcgtgctggcagatggtctggtttctgttatcgcctccgctgtcggttcattaccattaaccacgtttgcgcaaaataatggggttattcagatgactggcgtcgcttcacgttatgtcgggcgaaccatcgcggtaatgctggttatcctcggcttatttccgatgattggcggcttcttcacgaccattccctcggcagttctgggaggcgcaatgacgttgatgttttccatgattgccatcgcagggattcgcatcatcatcaccaacggtttaaagcgccgtgaaacacttattgtcgccacttctttaggtttagggcttggcgtctcctacgatcccgaaatttttaaaatattgccagcctctatttatgtattagttgaaaaccctatttgtgctggcgggttaactgcgattttattaaatattatcctccctggtggctaccgacaggaaaacgttctgcctggtattacctcagcggaagagatggattaacagtaaaggagtcaatgatgtcaggagaacacacgttaaaagcggtacgaggcagttttattgatgtcacccgtacgatcgataacccggaagagattgcctctgcgctgcggtttattgaggatggtttattactcattaaacagggaaaagtggaatggtttggcgaatgggaaaacggaaagcatcaaattcctgacaccattcgcgtgcgcgactatcgcggcaaactgatagtaccgggctttgtcgatacacatatccattatccgcaaagtgaaatggtgggggcctatggtgagcaattgctggagtggttgaataaacacaccttccctactgaacgtcgttatgaggatttagagtacgcccgcgaaatgtcggcgttcttcatcaagcagcttttacgtaacggaaccaccacggcgctggtgtttggcactgttcatccgcaatctgttgatgcgctgtttgaagccgccagtcatatcaatatgcgtatgattgccggtaaggtgatgatggaccgcaacgcaccggattatctgctcgacactgccgaaagcagctatcaccaaagcaaagaactgatcgaacgctggcacaaaaatggtcgtctgctatatgcgattacgccacgcttcgccccgacctcatctcctgaacagatggcgatggcgcaacgcctgaaagaagaatatccggatacgtgggtacatacccatctctgtgaaaacaaagatgaaattgcctgggtgaaatcgctttatcctgaccatgatggttatctggatgtttaccatcagtacggcctgaccggtaaaaactgtgtctttgctcactgcgtccatctcgaagaaaaagagtgggatcgtctcagcgaaaccaaatccagcattgctttctgtccgacctccaacctttacctcggcagcggcttattcaacttgaaaaaagcatggcagaagaaagttaaagtgggcatgggaacggatatcggtgccggaaccactttcaacatgctgcaaacgctgaacgaagcctacaaagtattgcaattacaaggctatcgcctctcggcatatgaagcgttttacctggccacgctcggcggagcgaaatctctgggccttgacgatttgattggcaactttttacctggcaaagaggctgatttcgtggtgatggaacccaccgccactccgctacagcagctgcgctatgacaactctgtttctttagtcgacaaattgttcgtgatgatgacgttgggcgatgaccgttcgatctaccgcacctacgttgatggtcgtctggtgtacgaacgcaactaataataaaactttaacatcctcgtgaggacatcattatgtctggagacatcctacaaacaccggacgcaccaaagccacagggcgcgctggataattattttaaaattaccgctcgtggcagtaccgttcgtcaggaagtactggctggcttaacgacctttctggccatggtttattccgttatcgtcgttccgggaatgctgggcaaagcaggttttcctcccgcagctgtgtttgttgccacctgtctggtcgcgggcttcggctcgttgctgatgggattatgggctaatttgccaatggcgattggttgcgcgatttccttgacggcgtttaccgcattcagtctggtactcgggcaacaaattagcgttcctgtcgcactgggcgcggtatttctgatgggcgtcatcttcaccgccatttccgtaaccggtgtgcgtacctggatcttacgtaatttgccgatgggtatcgctcacggtacaggtatcggtatcgggctgtttctgctgctgattgctgctaacggtgtgggtatggttatcaaaaacccgattgaaggcttgccagtggcgctcggtgcgtttacctccttcccggtgatgatgagcttgctggggctggcggtcatcttcggcctggagaagtgtcgcgtacccggcgggatcttgttggtgattattgcaatttcgatcatcggcttaatctttgacccagcggtgaaataccacggtctggtggcgatgccaagcctgactggcgaagatggtaagtctctgattttcagcctcgatattatgggtgcactccagccaactgtacttccgagtgtactggcattggtgatgaccgcagtgttcgacgctactggcaccatccgtgccgtcgccggtcaggcgaatttgttggataaagacaaccagatcatcaacggcggcaaagccctgaccagtgactcagtaagttcaatattctccggcctggtgggcgcagcgcccgcagcggtttatatcgaatcagcggcaggaaccgccgccgggggtaaaacaggtttaaccgcaaccgtagtgggggcgttattcctgttaattctgtttttatcaccgctgtcatttttgatccctggttacgccactgcacccgctctgatgtacgtaggtttgctgatgttaagtaacgtctcgaagctggatttcaatgattttattgacgctatggctggcctggtgtgtgccgtgttcatcgttctgacttgtaatatcgttaccggtattatgctgggctttgtgacactggtcgtaggccgcgtctttgcacgcgaatggcaaaagctgaatattggtacggtgatcattactgccgcactggtcgcattttacgcgggtggttgggcaatctaatagattctccgcgcctttcagcgcggagatttctttcagagaggattctcaccgctggcaacaatacgctgctggcggactcgcctgagttctctttcagtaagcaactgcagcgcctgtgttgggcaagattcaacgcaggctggcccctcttcccgctgttcacagagatcgcatttcacaatttgttgtcgggtatcccccggcaacgactgaatggtgatcattccaaacgggcacgcactgacgcaactctgacagccaatacaacgggcagaattggtctgcaccacctgctcgcccatcgtcagcgcccccacggggcaagcgccaacacaaggggcgttttcacactgatggcacatcaccggcgcactgatgctgtccagtcgctgtaccttcagccggggtaaaaagacatcggcattcaactcctgttctgaagggtgagcgaccacacaggctacttcacaagtacggcagccaatacagtcagccggattaacgataattaacgatttcatcacgatgccttcgtatcaaacagagttaacatatcgcgcgccgcctgccttcctgcggccattgcagtgacaaccagatccgcgccatgaactgcatcaccaccagcaaagacttttttcagatgcgtctgggtaggtaaatacccgacgtcaccggtttgaatcaggccccatttatcgagtttaattccgctgccctgcaaccacggcatggcatgcgcctggaaaccaaaggccataatcagaacatcggcgggcaattcaaactctgaacccgctaccggacgaggacgacggcgaccatccggccccggctcacccatggcggtacgaatcaggcccaccgcagttaaacgcccatcttcgtcacaagcgatatattgcggttgaacattgaactgaaactcgacaccttcctcgcgcgcattaaccacctctttgcgcgagcccggcatactgacttcatcacgacgatacgcgcaggtcacgctggcggcattgaggcggatggaagtccgcaaacaatccattgtcgtatcgccaccgcccaataccacgactcgcttaccttccacgtccgtcagcggatactcttcagactccggcaatcccatgagctggcgggtatgggcagtcaggaacggtagagcctgaatgacaccgggcgcatcttcatgcggcagatctgctcgcatcatcccgtaagtccccacgccgatgaaaactgcatcatattcagaagttaaatcgctaaaggtaatatcgcggccaatttcacagttaagatgaaagtcgattcccattgcggtgaatatctctcgccgctggcttaataccgttttatcgagtttgaaaggaggaatgccaaaagtcagcataccgccaatttctggatggcgatcaaagacatcgacctgaactcctgcgcgcgccagaatatcagcacaccctaaccctgcaggcccagcgccaatcaccgccactttttcgctacggggaacaactttgctgacatcgggacgccagcccatcgccagcgcggtatcggtgatgtagcgttccagattaccgatagagactgcgcccgagtgatctttcaaagtacatgcgccttcacaaagacggtcctgtggacataccctgccgcaaatttctggtaaggaactggtctggtggcaaagttctgccgcttcaataatctttccttcctgtaccagacggatgtaatccggaatagcgttatgcagcgggcaatgccagttgcagttagctttttcggcacaataaacacagcggtcactctcataagtcgcttgttgtggatccagcccgcaatatatttcgccaaagtgggttttccgttcactcgctgaaattttatctgcgcctttacgcgagttaacggggagcaacgctgcactgcgagatggctgagcgtctgatgacgcttttcctgctgccgttttgcgctggcgggccacctttatctgctgcaaccctttatcgtccatcagtcgtaacgcctgtgttgggcaaacttcaatacaggcttgcgtgccggaactgcgctggttacaaaggtcgcatttctgcgcaatcgtatcgaccatctcaacgacgccaaaggggcaagcgattgcgcatcttttacaaccaatacatttttgctcgtccagttgtacgctatcggactggaaagtcagagcattaaccggacaagccgtaacgcaaggggcattgttgcagtgatggcaggccaccggattcgcagcctggcctttccctacaacgtggatacgcggtcgaaagtcactgtgactcagcggccagttttcttgattgtgtgccaccgcacaggcaatttcacaagcatgacagcctatacattccgcagcttcagcagcaataaacttattcatttgcatccctttcatttaatgagttatgtcttctcaaatttcgcgatgcaataaacgggcatatattaggtagcatgaccgttttaattataattttgcgactgagttcaaattattgcccctcaatctatgccgctttcattatttcaacattgccgatcaaaagagcgctatccagataaaaacgattaaatgcgagagtgcgacatgccagaatgattaatgaaatatcaatatgagaaaattacagataattccattgtcaggttctcttctcattttcgtggtttaaccacgattatgtgattgcctccgcaattcctgtctctaactccccttcctcgcaaaaactggcactccacgagcatgtgtttagacagtttcattaacgtaaacggttgctttttactctggcgggcgaaaggagaaacactgatgagcgccatagattcccaacttccctcatcttctgggcaagaccgcccaactgatgaggttgaccgcatattatcaccaggaaagctgatcatactcggtctgcaacacgtccttgtcatgtacgcaggtgcagtcgctgttcctcttatgattggtgaccgactgggcctctcaaaagaagctattgcgatgctcattagctcggatctcttttgctgcgggatcgtcacattattgcaatgtatcggtatcggccgctttatggggatccgcctgccggtgattatgtcggtgacctttgctgctgtaacaccaatgatagccattgggatgaacccggatatcggcctgctggggatatttggtgccactatcgccgcgggttttatcaccacattattagcgccacttatcggtcgcttgatgcctttattcccgccactggttaccggtgtggttattacttctatcgggcttagcatcattcaggtgggtattgactgggccgccggaggtaaagggaatccgcaatatggtaatcccgtttatttaggtatctcctttgccgtcttaatttttatcttgctcattactcgctatgcgaaaggatttatgtccaacgtcgccgtattactggggattgtatttggctttttactttcgtggatgatgaatgaagtcaatttatccgggctacatgatgcttcatggtttgcgattgttacgccgatgtcgtttggtatgccgattttcgatcccgtttccattctgaccatgactgccgtgttaatcatcgtgtttatcgagtcaatggggatgttcctggcactgggtgaaatagtcggtcgtaaactctcttcgcacgatattattcgcgggctgcgtgtcgatggcgtagggacaatgataggcggcacgtttaacagcttcccccacacgtcattttctcaaaacgttggcctggttagcgtgacgcgcgttcatagccgctgggtgtgtatttcttcgggaattatattaatcctgtttggcatggtgccaaaaatggcggtgctggtagcctccattccgcaatttgtgctgggcggcgctggtctagtgatgttcggcatggtactggcgacagggattcgaattctgtcgcgctgtaactacaccaccaaccgttacaacctctatattgtggcgatcagtctcggcgttggcatgactccgacgctctctcacgatttcttttctaagttaccggccgtactgcaaccgctgctacatagcggcattatgctcgcaacccttagcgccgttgtgctgaacgtcttctttaatggctatcagcatcatgctgacctggtgaaggaatccgtctctgataaagatttaaaagtcaggacagtacgtatgtggcttctgatgcgcaagctgaagaaaaatgagcatggagaataatatgaattttttaatgcgcgctatattcagtctgttgttgctttttactctctctattcctgtcatttctgactgtgttgcaatggccattgaaagtcgcttcaaatatatgatgctacttttttaaatggtttttacctgtcggcatccgctcaaaacgggcggttgtcgataaacgctcacttggttaatcatttcactcttcaattatctataatgatgagtgatcagaattacatgtgagaaattatgcaaacggaacacgtcattttattgaatgcacagggagttcccacgggtacgctggaaaagtatgccgcacacacggcagacacccgcttacatctcgcgttctccagttggctgtttaatgccaaaggacaattattagttacccgccgcgcactgagcaaaaaagcatggcctggcgtgtggactaactcggtttgtgggcacccacaactgggagaaagcaacgaagacgcagtgatccgccgttgccgttatgagcttggcgtggaaattacgcctcctgaatctatctatcctgactttcgctaccgcgccaccgatccgagtggcattgtggaaaatgaagtgtgtccggtatttgccgcacgcaccactagtgcgttacagatcaatgatgatgaagtgatggattatcaatggtgtgatttagcagatgtattacacggtattgatgccacgccgtgggcgttcagtccgtggatggtgatgcaggcgacaaatcgcgaagccagaaaacgattatctgcatttacccagcttaaataaaaaaaccccgacatttgccggggttgtgagcataacgtaatgcttattttaccggacgcatcgccgggaacagaataacgtcgcggatggtatggctgttggtgaacagcattaccatacggtcgataccaattcccagacctgctgtcggcggtaagccatgttccagtgcggtgacgtaatcttcatcgtagaacatcgcttcgtcgtcacctgcgtctttcgcggcaacctgatccaggaagcgttgcgcctgatcttccgcgtcattcagctcgctaaagccgttaccgatttcacgaccaccaatgaagaactcaaagcggtctgtgatttccgggttaacgtcgttacgacgcgccagcggagaaacttctgccggatattcagtaatgaaggtcggctgaatcagatgtgcttctgccacttcttcgaagatctcggtaacgatacggcccagaccccagctcttctcaacgtggatgccgatagattcagcaattgctttcgcagagtcgaagttgtccagatccgccatgtcggtttccgggcgatatttcttgatcgcttcacgcatggtcagtttttcgaacggtttaccgaagtccagcgtcacgtcgccgtaggtcacttccgtcttaccgagaatatcctgtgccagagtacggaacagcgattcggtcagctcgatcagatctttgtaatctgcgtaagccatgtagagttccatcatggtgaactctgggttatgacgtacggaaataccttcgttacggaagttacggttgatttcgaatacacgctcgaagccaccaaccaccagacgcttgaggtacagttccggcgcgatacgcaggtacatgtcgagatccagcgcgttatggtgggtgataaacggacgcgcagcggcaccgccagggatcacctgcatcatcggcgtttcaacttccataaagccgcggttcaccatgaactggcgaataccagagaggatctgcgagcgcactttaaaggtgttgcgggattcatcgttggagatgagatcgagataacgctgacgatagcgcgcttcctgatcctgcaagccgtggaatttatccggcagcggacgcagtgctttggtcagcagacgcaactcggtgcagtggatagacagttcgccggttttggttttgaacagcttacctttcgcgccgaggatgtcgccgaggtcccattttttgaactgctcgttataaacgccttccgggagatcgtcacgggcaacgtacagctgaatgcgaccgccaacgtcctgcagggtaacgaaagacgctttacccataatacgacgggtcatcatgcggccagcaacggcgacttcgatgttcagcgcttccagttcttcgttctctttgccgtcgaattctgcgtgcaattggtcagaggtatgatcgcgacggaaatcgttcgggaaggcaatcccctgctcgcgcaggttcgccagcttctcacgacgcgttttcagttcattgttaagatcgactaccgcgtcagcgccctgtgcgtgttgttcagacatgttggttcctcataaccctgctttcaaacttgcttcgataaattgatccaggctgccgtccagcacggcctgcgtgttgcgggtttctaccccggtgcgcagatctttaatgcgggagtcatcaaggacataagaacgaatctggctgccccagccgatgtcggatttgttatcttccatcgcctgtttctcggcatttttcttctgcatctccagttcataaagcttcgctttcatctgcttcatggcctgatctttgttcttgtgctgggaacggtcgttctggcactgggtcacgatcccggtcgggatgtgggtaatacgcaccgcagattcggtacggttaacgtgctgaccgcccgcgccggacgtgcgataaacgtcaatgcgcagatccgccgggttgatttcgatatcaatatcatcatcaacttccggataaacaaacgcggagctgaacgacgtgtggcgacgaccgccggagtcaaacgggcttttacgcaccaggcggtgaacgccggtttctgtacgcagccagccgtaagcgtaatcgccggagattttgatcgtcacggatttaatacccgccacttcaccttccgactcttcgatgatttcagttttgaaaccacgcgattctgcccagcgcagatacatacgctcaagcatgctcgcccagtcctgtgcttccgtaccgccagaccccgcctgaatatcgaggtagcagtcggcgctgtcatattcgccagagaacatacggcggaactcaagctgcgccagtttttcttccagggcgtcgagttcagcaacggcttcgttaaaggtttcttcgtcgtcagcttctacagccagttccagcagaccagaaacatcttccagcccctgtttcatttggtcgagggtgtcgacaacggcttcgagggaggaacgctctttacccagcgcctgtgcgcgttcgggttcgttccagacatccggctgttccagctcggcgtttacttcttccagacgctctttcttggcgtcgtagtcaaagataccccctaagaacgtcggagcgttccgtgaggtcctgaatgcgattatttaccggattaatttcaaacatggtctgatttcttttattgagctagtcaaaatgcggtgataagagcgggattgtacccaatccacgctcttttttatagagaagatgacgctaaattggccagatattgtcgatgataatttgcaggctgcggttgccgcgaaactcgttgatatcgagcttataagccagttgcacttcgcgcacgccgttatccggccagagggcggtatcgacattaaaagcaataccatccagcagtggaccgccgccgaccggttcgaccatcaccttcaaatgacgttcgcccaccagccgctgttgcagcagacggaaatgaccgtcaaacagcggctccgggaacatctgcccccacgggccagcatcgcgcagcagctgcgccacttccatggtcatttcggccgggcttaacggaccgtctgataccacttcgccttgcaatagcgaagggtccagccactcagtaaccagttcgccaaaccgttgttgaaagagtttgaatttatcctcttccagcgacaaacccgccgccatcgcatgaccgccaaacttcagcatcatgccagggtagagtgtgtctaatcgctccagcgcatcacgcatatgcagcccctgaatggagcgaccggaacctttcagcgtaccgtcacctgctggcgcaaacgcgataaccggacggtgaaaacgctctttgatgcgcgaagccagaataccgacaacgccctgatgccattcggggtgatacattgccagcccgccgggtagcgtgtcacggctgcgctccagtttctcgcacagggtcagggcttcaatttgcattccttgttcgatctcttttcgcgtctggtttagcgcatcgagttcatttgccagcacgcgcgcttcgccgatgttgtcgcacaacaacagcgccacaccgacggacatatcgtccagtcgtccggcagcattgagacgtggccccagcgcaaaacctaaatcgctggcggcgagtttttgtgcatcacggtttgccacttcaagcagcgctttaatccccggacggcactttccggctcggatgcgactcatcccctgccaggtcagaatgcgattattagcgtccagcggcacgacgtccgccactgtccccagcgcgaccagatccagcagttctgccaggttaggaattgcgatgttacgctcatcaaaccagccctgatcgcgcaaaaaggtgcgcagcgccagcatcagataaaacgccacacccacgcctgccagtgatttcgacgggaaattacagtcgcgcaagttagggttaatgatcgcttccgctgcgggtaatgtgtcgcctggcaaatggtgatcggtaacaataaccgggatgcccaacgagcgagcgtgctcaacccccgcatgggaggaaataccgttatccaccgtgacaattaactgcgcgccacgggcatgggcctgatcgaccacttccgggcttaagccgtaaccgtcttcgaaacggtttggtaccaggtagtcgatattgctgcaaccaagcgagcgcatcgccagcacgcttagagccgtgctggtcgcgccgtcggcgtcgaaatcaccgaccacaataatccgcgttccttcgcgaaaagcgttgtaaaggatctcaacggccttttcgacgccgctcagttgctgccagggcagcatacctttaacactgcgttccagttcttgcgcactgcgtactccccggctggcgtataaacggcgcagcaagggaggcaattcagcgggcaagtctgccgtttcatcgacttcacggcgacgaagttgtatctgttgtttcacgcgaattatttaccgctggtcattttttggtgttcgtcgaggaattctttcatctctttcggcggctggtaacccggaacaagtgtgccattgctcagcacaactgccggagtaccgctaacgccaagctggacgccaagtgcgtaatggtcggcaatatccacgtcgcaactggctggtgcgacgcttttacctgccatcacatcatcaaacgctttgtttttatctttcgcacaccagatagctttcatttctttctctgcatcgctgtccagcccctggcgcgggaaagcaagataacgcacggtgatccccagcgcgttgtagtctgccatttgctcatgcagtttgtggcagtaaccacaggtaatatcagtaaacacggtgatgacgtgtttttcctgcggcgctttataaacgatcatctctttttcaagcgcattcaactgctttaacagcatcttattggtgacattgaccggagccgtgccactaacgtcatacattggcccctgaatgatatgtttaccatcatcggtgatgtacaacacgccgctgttagtcagaactgtcttcatgccagctacaggcgcgggctgaatatcgctgcttttgatgcccattttggctaacgtttgttgaattgccgcgtcatcagcctgagcaaagcctgaaaacgccgctaacaaagtaaacaacataaaacctttcttcataaatcttcccgttcttttcagacatcacgcccgcgggtgatgctgttgatgaagttgccgcagacgctcggtagcgacatgcgtataaatttgcgtggtggagagatcgctgtggcccagtagcatctgcaccacgcgtaaatccgcaccatgatttaataaatgagtggcaaaagcgtgacgcaacacatgcggtgacagcttttcgctgtcgatacccgccagcacagcataatgtttaatacggtgccagaaggtctgtcgcgtcatctgctgcgcacgctggctgggaaacaacacgtcaattgacacaccattcagcagccacggacgcccatgttccagataggtttccagccagtaaaccgcctcttcacctaacggcaccagacgctctttgttgcctttaccaatgacccgtaccacgccctgacgcaggctgatatcactcattgtcagtccgaccagttcagagacacgcagcccggtagcatacaacacttcaagcatggctttatcgcgtagctccagtggctgatcgattaatggtgcctgtaataaacgttcgacctgcgcttcgcttaaatcttttggcaaacgctggggcaatttcggtgaagcgagatgcgcactgggatcgtcttcacgaaacttttcgcgataaagatactggaacaatcggcgcactgcactcagcaaacgcgctgagctggtggctttatacccgccctccagccgttctgccagtaatgcctgcaaatcgtcactttgcgccgtcgccagcgtcaacccgcggtgatgcaaccactccaccatcattgacagatcgcgacggtaagcgttcaacgtattttcagccagatttttttccagccacagagcatcaagaaactgctcgatgcgtgccagatcctgtttcacttgcgccccttatggtcactcatttgatccattatgccttattgtgccgtgactaaagcgattctgatacactagccgcaaaagccacagcagaatcgagaagcttacgttatgaatatgggtcttttttacggttccagcacctgttacaccgaaatggcggcagaaaaaatccgcgatattatcggcccagaactggtgaccttacataacctcaaggacgactccccgaaattaatggagcagtacgatgtgctcattctgggtatcccgacctgggattttggtgaaatccaggaagactgggaagccgtctgggatcagctcgacgacctgaaccttgaaggtaaaattgttgcgctgtatgggcttggcgatcaactgggatacggcgagtggttcctcgatgcgctcggtatgctgcatgacaaactctcgaccaaaggcgtgaagttcgtcggctactggccaacggaaggatatgaatttaccagcccgaaaccggtgattgctgacgggcaactgttcgtgggtctggcgctggatgaaactaaccagtatgaccttagcgacgagcgtattcagagctggtgcgagcaaatcctcaacgaaatggcagagcattacgcctgatctcactgacggcttagcgcatatgctttgccgtcatctttatctttgcgtctcttgttgcaacaaaatccgccgtaaatcccgccattcagcttcgtccatgctgtcggctgccagccataaatgttgccgtttaccgccatcagaacgtaaacgcagcatcatgccgctcttaatcatccacggtgctttgacgatgctccactcctgcccttgccaacgcaaacgcccgtccatcaacaagcgaatttccccctggcgagcattaatacgccgctggctgcgaacgcaatcaaacaccaccagcgaaagtaacaccatccataacggggtgtaactgagtggccagggcatgagtaaaataacagcggcaaccagcccatgaatcagcaaggaaagccactgtgcgcgccaggagacgcgcaaatcagattgccacaggaccacgttcccggttccgtgtctggatgagtcggaccatcatttccagttctgcatcggccggtttaccgtgattcatcagccagttaaacaggtccggatcgtcacattccagcagacgaataaagatgcgtttttcgtcatcgcttaagctgtcgtactcatgttcgaaaaacggcatgattgaaatatcgagttcgcgcataccacggcggcatgcccaatgaatgcgggctttgttgttaatgtccatcttcttcctgtctcacgaaaatccagtacccggctattgtaacgtgtttttcgccttcttttacgggaatatcagtaaacaccatcgcgatcgcgaaattaattcacaacaattcaatggcttcatttttttggaagtcgcctcgcagaaggcacagatcgcgtagtgaaagcacttgcattgcctcatagctcttttaccattagtcattaatacgccgttaagcaactcaggactctattatggcttttacaccttttcctccccgtcagcctacggcttctgcccgtttaccgctgacgctgatgacgcttgatgactgggcgcttgccaccattactggcgcggacagcgaaaaatatatgcagggtcaggtgacagcagatgtcagccagatggcagaagatcagcacctgctcgccgcccattgcgacgccaaaggtaaaatgtggagcaatttacgtctgttccgcgacggcgatggctttgcatggattgaacggcgcagcgtgcgtgaaccgcagctgactgaactgaaaaaatatgcggtattctctaaagtgaccatcgcgccagacgacgagcgtgtgctgcttggtgttgccggttttcaggcgcgcgccgcgctggcaaatctctttagcgaactgccttcgaaagaaaaacaggtagtcaaagaaggcgcgaccactttgctatggtttgaacacccggcagaacgtttcctgatcgtaaccgatgaagctactgctaatatgctgaccgataaactgcgcggtgaagcggaactgaacaatagccaacagtggctggcattaaacattgaagcgggtttcccggtgattgatgccgccaacagcgggcagtttatcccacaggcgaccaatctccaggcgctgggcggtatcagctttaagaaaggctgttataccggacaagagatggtggcgcgagcaaaattccgtggtgccaataaacgtgcgctctggttgctggcaggtagcgccagccgactgccggaagctggtgaagacttagagctgaaaatgggcgagaactggcgtcgtaccggtacggtactggctgcggtaaaactggaagatggtcaggtcgtggtacaggtcgtcatgaataacgatatggaaccggatagcatcttccgcgtacgcgacgatgcgaatacattgcatatcgagccgctgccgtattcgctcgaagagtaaatctctttatcgcatcaggcatttatcgcctgatgcgacgctggcgcgtcttatcatgtctgggatttgatgcctttatcacaacagggacgaggcccgtagatcggataaggcgttcacgccgaatccggcagttgtgctccgatgcctgatgcgacgctggcgcgtcttatcaggcctacaaaggcatacccattacgcctgcccaatatacaaatagatcgccagaaagtggcacacactaccgccgagcacgaagccgtgccagatggcatggttgtatggaatgcgtttgcagacgtagaaaatcaccccgagcgaataaaccacgccgcctaccgccagtaaggtaacgctgcccgccgcgagcttaactgccatttcataaattaccaccagcgacagccagcccatcgccagataggtcaccagagataaaattttgaatcggtgcgcgatggtcagtttaaacagaatacccagcaatgccaggctccagataacaatcatcaacccgcgcgctaacggagaatccagccccaccagcaaaaacggcgtgtaggttccggcaatcaacaggtaaatagcgcaatggtcaaatttcttcagccacatttttgcccgttgatgaggaatggcgtgatagagcgtcgaagcgaggaacagcaggatcatactgccgccatagaggctgtagctggttatcgctgtggcgctggcattaagatccaccgcctgaaccagtagcaacaccagcccaacgataccaaacaccaacccaatgccgtgactgacgctgttggctatttcctctgccagtgaatatccctgcttaatgaggggcttctgaaccataacttactccggagaaacgtacacgcacatgtatacctctccagcgtaactgagaatagttccagtgaacacctgttagctaaaataaattctgatttgagactaatctcctaaaaatcatgaaattaaatgcgaaatttcaactaacaggcgtgagttcaatttaaagacatttaaattcaatcacataaaattgtgtctgaccgggatagatgtcagcaatgacttttttcagttcagtcagggtcatattttcctgctctgcatgtttttcagtcagcgtatccagcgttacggttgaggttgcggtgacttcaatcgtgcaaaaataaccgtcatcttcaaaacgtccgacacgaagcacatcacccgttttgaagtgcgattcagactcgtcgcggatggtgatggttttacgcccagccagaatgtcatcctggaaacgttgaaaaaaagtgatgtcgtttggctgcatggtactatttcctgtaagaattgactcatctggagcctatgatagtgaaaaaactcaccttaccgaaagatttcttatggggcggcgcagttgccgctcatcaggtcgaaggcggctggaacaaaggcggaaaagggccgagcatttgtgacgttctgaccggtggcgcacacggcgtgccgcgcgaaatcaccaaagaagtcttgccaggaaaatactatccaaaccatgaagccgttgatttttatggtcactataaggaagacatcaagctatttgccgaaatgggcttcaaatgttttcgtacatccattgcctggacgcgcatttttccaaaaggcgatgaagctcagccaaacgaagaagggctgaagttctacgatgatatgttcgatgaactgctgaaatacaacatcgaaccggtgatcaccctctcccactttgaaatgccgctgcatctggtgcagcaatacggtagctggaccaaccgtaaagtggttgatttctttgtacgtttcgcggaagtggtatttgaacgctataagcacaaagtcaaatactggatgaccttcaacgaaattaacaaccagcgtaactggcgtgcaccgctgttcggttactgctgctccggcgtggtgtataccgagcatgaaaacccggaagagacgatgtatcaggtgctgcatcaccagtttgtcgccagcgccctggcggtgaaagctgcgcgtcgcattaacccggagatgaaagtcggctgtatgctggcgatggtgccgctctatccttactcctgtaacccggacgatgtgatgttcgctcaggagtcgatgcgcgaacgctacgtctttaccgatgtgcagctacgcggctattacccgtcctatgtgttgaacgagtgggagcgtcgcggatttaacatcaaaatggaagacggcgatctggatgtgctgcgtgaaggcacctgcgattatcttggtttcagctattacatgaccaatgcagtgaaggccgaaggcggcaccggcgatgcgatctctggttttgaaggcagcgtaccaaacccgtatgttaaagcatctgactggggctggcagattgatccagtaggtctgcgctatgcactttgcgaactgtatgagcgttatcagaggccgctgtttattgtcgaaaacggttttggcgcttacgacaaagtggaagaagatggcagcatcaacgacgactaccgcattgactacctgcgcgcccatatcgaagagatgaaaaaagcggtgacttacgatggcgtggatctgatgggctacacaccgtggggctgcatcgactgcgtgtcgttcaccaccgggcagtacagcaaacgctacggctttatctatgtgaataaacatgacgacggtactggcgatatgtcgcgttcacgtaagaagagctttaactggtacaaagaggtgattgccagcaacggcgagaagctttaagtcgatgaagtaccggatgcaatacttgttgcatccggtcagacaacttccctgttttatttcccgcccgccaaatcgataaaacttcccgtgacgtaagaggctttatcacttagtagccagacaatggcctgcgcgacctcttctgcctgtccaccacgctgcatggggatgttcgacttaacgcgatcgacgcgtccaggctcgccgccgctggcgtgcatttcggtataaataaaccctggccgcacgcagttaacgcggatcccctgcgcggcgacttccagcgatagtccggtggttaacgtatcaatcgcccctttcgatgccgcgtaatcaacatattcccctggcgaacccaaccgtgaggccaccgaagagacattgacgatagcgccgccactgccaccatttttaagcgccatgcgttttaccgcctcgcggcagcagagaaaatatcccgtcacgttggtggaaagtactcggttgattcgctctgcggtaaggttttcaacggtgcactgggtaaacaagatcccggcgttattgaccagcgctgctagcggttcatcgtgctgatcgattgctgtaaacatcgcaacgacctggttttcgtcgctgatatccgcctggagcacgaatgctttgccaccggcttgcgttattaagttcatcacttcctgcgccgcgtggaggttttgctgataattaaccgccaccgtatacccttcttgcgccaacagtaatgcagttgcccgcccgatgccgcgactgccaccagtcacaagtgctatagccatttgtttttccgagaaaaattaattcgttgacgtatctttgagattgctaacaaactggctcaatcttcaatgttggcacgcttttccccctcgccctttcagggagagggccggggtgagggtaaatattcgcgccagtgccggcctgttcccctcaccctaaccctctccccaaaggggcgaggggactgtctgagcacttttgtactttgtcatctgactaaaaaggcgccgaagcgcctttagaaaatagtcgaatcagtgaattactggtattcgctaatcggtacgcaggagcagaacaggttacggtcgccgtaaacatcatccagacgtttcactgtcggccagtatttgtctgccacacctgccgggaataccgcaacttcacggctgtacggatgcgcccactcggcgaccagttcgctctgaatgtgcggcgcgttcaccagcgggttatcttccagcggccagacaccggctttcacctggtcaatttctgcgcggatagccagcatcgcgtcgataaagcgatccagttccactttgctttcagattcagtcggttcaaccatcagcgtacccgccaccgggaacgacatcgtcggcgcgtggaaaccgtagtcgatcaggcgcttggcaatatccagctcgctgatgccggtttcttctttcagcgggcgaatatcgagaatacattcgtgcgccacgcgaccgtcgcgaccggtatacagcaccgggaaggcatcctgcaggcggctggcaatatagttggcgttgaggattgccacctggcttgcttttttcagcccttctgcgcccatcatgcggatgtacatccagctgattggcaggatagaggcgctaccgaacggtgccgcagaaaccgcgccctgacgggttaacatgccttcgatttgcaccacgctatgacccggtacaaacggtgccaaatgcgctttcacgccgatcggtcccatacccggaccaccaccgccgtgcggaatgcagaaagttttatgtaggttaaggtgtgaaacgtccgcaccaataaagcccggcgaggtgatgccaacctgggcgttcatgttcgcgccatcaaggtaaacctgaccgccgaactgatgcacgacttcacacacttcacggatcgtttcttcatacacgccgtgggtagaaggataagtcaccatgatacaggagaggttatcgcccgcctgttccgctttcgcgcgcagatcagtcagatcgatgttgccgtttttatcacacgccacaaccaccacctgcattcctgccatatgtgcagaagcggggttagttccgtgcgcagaagccgggatcaggcagatatcgcgatgcccttcgttgcggctttcatgataatgacgaatcgccagcaggcccgcgtattcgccctgtgcgccagagttcggctgcatacaaacggcgtcgtaaccggtcagtttcaccagccagtcagccagctgcgcaatcatctgctgataaccttcggcctgctccggcgggcagaacgggtgcagttcggcaaattccggccaggtgattgggatcatctcggcggcggcgttcagtttcatggtgcaggaacccagcgggatcatcgcctgattcagcgccagatctttacgctccagcgagtgcatatagcgcatcatttcggtttcgctgtggtagcgattaaacaccggatgggtgaggatttcgtcgtcgcgcagcatcgcaggctggatagagcggctgtcgtgagccacgtctttgtccagcgtgtcgatgtccaggccgtggttatcgcccagcagcacgttgaaaagctgcattacgttttcacgcgtggttgtttcatcaagggtgatcccaaccgcgttcagaatatcgctacgcaggttgatttcagccgcttcggcacgcgtcagtacgcccgctttgtcggccacttccacacacaaggtgtcgaaatagtgcgcatggcgcagtttcagacctttttgttgcaggcccgccgccaggatatcggtcagacggtgaatgcggttagcgatacgtttcaggccaaccgggccgtgataaacggcatacaggctggcgatgtttgccagcagtacctgggaagtacaaatgttggagttcgctttctcacggcggatatgttgctcgcgagtctgcatcgccatgcgcagcgcggtattgccagctgcatctttcgatacaccgataatacggcccggcattgagcgtttgtattcatctttcgccgcaaagaatgccgcgtgtgggccaccgtagcccatcggcacgccgaagcgttgcgccgaaccaaaaacaatatccgcgccctgtttacccggcgcagttaacagcaccagcgccataatatcggcggcaacgctgaccacaattttgcgtgatttcagttcgctaataagcgcagtgtagtcgtgaatttcaccggtagtgcctacctgctgtaacagcacgccgaagacgtcctgatggtcgagcactttttgcgcgtcatcgacaatcacttcaaaaccaaaggtttcggcacgagtacggaccacatccagcgtttgcggatgcacatcggaagccacgaagaagcggttggcatttttcagtttgctgacgcgtttcgccatcgccattgcttcggcggcagcggtggcctcgtccagaagagaagcagaggccatatccagtccagtcaaatccagcgttacctgctggaagttgagcagtgcttcaaggcggccctgggagacttcaggttgatacggagtgtacgcggtataccagcccggattttccagcatgttacgcaggataaccggcggtagctgcacggcggtgtaacccatgccgatgtaagacgtgaagcgtttattgcgactggcaatagccttgagttctgccagtgcggcgtattcggtcgccggtgcgccaacctgcggtggtgtcgcaagttgaatatctttcggcacaatctggccggtcagcgcgtttaacgattgtgcaccaacggcattcagcatttcttgctgttgcgcggcgtccggtccgatatggcgttcaataaaagcgccgctgttttcaagctggcttaacgtctgtgtcatgagcgatggttcctgaaacgtgcagtgaattgtgaacctctctccttacgaagagagtgagggtgaggcataaattttcctcaccctgatcctctcccgcagaagaggaataaagccgttactcgtcttctaacaatgcttcgtatgcggtcgcatccagcagtgattccagttcgctttcatcgctggctttgattttaaagatccagccgcctgcatacggttcgctgttcaccagttccggggaatcgctcagtgcgtcgtttaccgccacgatttcaccgcttactggcgcataaatgtctgacgccgcttttaccgattcggcaaccgcgcagtcatcgcccgcgctaaccgttgcgcccacttccggcaggtcaacaaacaccatatcgcctaacagctcctgagcatgttcggtaataccaacggtgtaagtgccgtcggcttctttacgcagccattcgtgttctttgctgtatttcagttctgctggtacgttgctcatcaatcaatctccaaaaaagtaaatcacgcgacggctttgccgttacgcacaaaaacaggttttgtcactttaaccggcatttcacggttgcgaatttgcacaatcgccgtttcgccaataccttccggcacgcgcgccagcgcaatgctgtaacccagcgtcggggagaaagtaccgctggtgataatgccttcatgctggttgccctgcgcatcggtaaagcgtaccggcagttcattacgcagcacgcctttttcggtcatcaccagaccaaccagtttttctgtaccatgctcacgctgcacttccagggcttcacgaccgataaagtcacgatctgccggttcccaggcgatggtccagcccatgttggcggctaaaggagagatggtttcgtccatctcctgaccataaagattcatgcccgcttccagacgcagcgtgtcacgcgcgcccaagccacatggcttaacacccgcttccaccagcgcacgccagaaatcggccgctttttcattgggcagcgcaatttcatagcccgcttcaccggtataaccagtggtggcaataaacagatcgcccgcctgcacgccaaagaacggtttcatcccttccaccgcctgacgctgggcgtcattaaacagtgtggcagcttttgcctgcgcattcggcccttgcacggcaatcatggaaaggtcatcacgaacggtaatttcgatgccgaaaggttcagcgtgttgggtaatccaggagaggtctttttcgcgggtggcggagttaacaacgaggcggaagaaatcttcagtaaagtagtagacgatgaggtcatctatcacaccgccagaggcattcaacatccccgagtaaagggctttgccgcttttggtgagcttcgccacatcgttcgccagcagataacgcagaaactcccgggtgcggctgccgcgaagatcgacgatggtcatatgtgacacatcaaacattccggcatcggtacgtaccgcatgatgttcgtcgatttgcgaaccgtaatgcagcggcatcatccagccgtggaaatccaccatgcgagcgccgcaaagcgtgtgttgttcgtacaaaggagtctgttgtgccatcttgtcctcattgaataagcggggctgacaactttttcatggtgaaattatcaccacgaaacccagcatcggagccactcccggtccccaacgcaatcgttctcttttgcctgaacttaccaccgaaacagactgttaaccataaggtaaaattgatcatcacattagcttatggttaaaaaatgcaaaaatcgcgacagaataaaaaaccaaaaaatacaccagtttctatacaaagatgatgtgatgagaaagtcaatttgaataagacaatattaagagctaaaaaaatgtcaaaaaacactaaatcaaaaaataatggcattagaaaatataatgcgaaaacggaggtgaaattagtttatttcaaatgaggaaaatctcccggcgaaaaaaccgggagatgaaagtgtgatgggtatcaaataaacaacagaggagaaatttttaacgcagccattcaggcaaatcgtttaatcccattgcctggcggataagttgcggcttaacgccaggaagcgtgtcggccagtttcaaaccaatatcacgcagcagttttttcgccggattggtaccggaaaacagatcgcggaatccctgcataccagccagcatcaacgccgcactgtgcttgcggctacgctcatagcgacgcagataaatgtactgcccgatgtctttcccctgacgatgcaaccgtttcagttcggcaatcagctctgcagcatccataaagccgagatttaccccctgccccgccagcgggtgaatggtatgtgcggcgtcgcccaccagcgccagacggtgcgaggcaaactggcgcgcataacgccccgtcagtgggaacacctgacgcgcgctctcaaccttgcataagcccaggcgattatcaaaagcgatatttaacgcgcgattaaattcgtcttcacttgcctgctgcatccgctgcgcttcctctggcgacagtgaccagacaatcgagcaaagatgcggatcgctaagcggtaaaaaggccagaatgccttcgccatggaaaacctgccgcgccaccgcatcatgcggttcttccgtgcgaatggtcgctaccagcgcgtgatgctgataatcccagaaagtcagcggaatatcggctttgttgcgcaaccaggaattagcgccgtccgcgccaatcaccagacgcgccgttaacatgctgccatctttcagcgtcaggaaggtttcattttctccccaggcgacctgctgtaattctgcgggggctaacagagtgatatctgacgactgatgcgctttgttccacagcgcgtagtgaatcactgaattttcaacgatatgcccaagatggctatagcccatgctttgatcgtcaaacgaaatgtgaccaaagctgtctttgtcccacacttccataccgtgataacagctggccctacgagagagaatgtcctgccagacgccaagacgggtgagtaatttttcgctggcggcattgatagccgaaacgcgcagttgtggtggtgcattcgccgccagaggttcctgtacgcgctgctccagtacggcaacgcgtaagccgctcccctgtaagccacaggcaaccgccagccccaccatgccgccgccaacaatggctacatcaacactttgcattgtttattccttaaaaccgccttcaacgcgccacccaaccgagggtgcgctgcgccagcacatcgcgtgccggggtgaataattccatcgtcatcagcccgatgttgcgcccgacaaccagcggtgcccaacggttggcaaaaagatgtacaaggctgtccgtgacgccaatggttgcttcgcgatcgctctgtcgacgctgctgataacggcacaatacgccgtaatcccccatgtcttctccgcgctcctgcgcctgagtcagggtttccgcaagactcatcacatctcgcataccgaggttaaacccttgcccggcaatcgggtgcagagtttgcgccgcattgcccaccagcacggtacgatgggtaatagatctggcggcgtgggttaacgccagcggataagcactgcgtttaccagcgtgggtaattttcccaagtcgccagccaaaggccgactggagttcacggcaaaacttctcgtcactccacgacaacacctcttcgcgccgttccagtggatgacaccagaccagcgaacagcgtccgtcagacatcggcaacatcgccagcgggccatgttgcgtaaagcgttcaaaagcgcgcccttcatgcgcaacggaagtagcaacgttggcaatcacggccagttgttcgtaaggctcctgctgccagtcaacgccgcacgcggtggctaacgctgaatgggtgccatcagctgctaccagcacgcggcccgtcagcgtctcgccactctccagcgtcacttcaacgtgactctgagtacgggcaacgttagccacgcgatcagggcaatgcagcgttacgccaggtgctttacgcagcaatgcaaacagccgttgcccgacattgtgcaattcgacaacctgtcccagcgccgccagttggtaatcttctgcggcgagggtgacaaatccagcgtgaccacgatcgctgacatgcacggtggtgatggcagttgcgcaatccgccagagattgccagacgccgatgcgcgccagttgctgacaggtacccgccgccagcgctatcgctcgtccatcaaagcccggatgagcatgtgactctggcgcagtcgcttcaatcaaatgtaccggcagcgccccgtgacttaaccgggaaatagccagcgccagcgtcgcgcccgccatgccgccaccgacgatgattacgctcattgctttctcgcagcaaccatcaacgcttcgatttcttccggctttttcaccacgctggcggtgaggttttcgttaccggtttcggtaatcacaatgtcgtcttcaatacgaatgccgataccgcgatattgttctggcacttctgcatccggcgcaatatacagccctggctctacggtcagtaccatgcccggttccagaatgcgcgagcgatcctgaccataaacacccacgtcatggacatccagtcctaaccagtggctaaggccatgcataaagaaaggacgatgggcgttctgagcgatcagttcatcaacatcacctttcaggatgccgagttttaccaggccgctaaccatgatgcgcaccacttcaccagtgacttccagaatggaagttcccggacgatacaggcgcaggctggtttcgagagactccagcacaatgtcgtagatttcacgctgggcctgggtgaatttgccgttgaccgggaaggtgcgggtaatatcgccagcgtaacctttgtattcacaacccgcgtcaatcaacaccaggtcgccgtcgcgcatttcacactcgttttcggtgtagtgcagaatgcagccgttttcaccgctgccgacaatggtgttataggacggatagcgcgcaccgtggcggttaaattcgtggtgaatttcgccttccagatggtactcgaacattcccggacggcatttttccatcgcccgtgtatgtgccatggcggtgatttctcccgcgcggcggagtacggcaatctcttctggcgatttgaacaggcgcatttcatgaacaacaggacgccagtcgatcatcgttgccggtgcggtgagattttgccgcgaacctttacgcagtttttccagcgcactgttcacgattacatcagcatatgcatattcgccctgggcatggtaaaccacatccaggccgttaagtagttgataaagttgctgattgatttcgctgaatgccagtgcgcggtcaacgcccagtttctctggcgcggcatcctggcctaagcgacggccaaaccagatctccgccgtcaggtcgcgaacgcggttaaacagaacgctgtggttatgagtgtcatcgcttttaatcagcaccagcaccgcttccggttcgttaaagccggtgaagtaccagaagtcactgttctgacgataggggtattcgctgtcggcgctacgtgttacttctggtgcagcaaaaatcagcgcggcgctgccgggttgcatttgctccaccagggcctgacggcgacgctgaaactcttgccgggatatctcactcataacactctccttacgttttttgtttttagtgtagagtcggtttttgtacttctggcgcggtcggttgcggatgagtaaaggtgtcgtggcataacagcgcggcaacacgaacgtattcgatgatctcttcaagcgacatttcaagctcttcctgatcttcgtcttcgtcgtaacccagttgcgcaatgttacgcagatcgtcgatagcttcaccggtttcgccggtcactttatccagcttcggttgcgtaacgccaagaccaagcaggaagtgattgacccaacctgccaatgcatcagcccgatcgaaaacgctgacatcatcgccatcaggcagataaagctgaaaaaggaagccgtcatcctgcagggcatcgctggtggcagagtgcattttacgcagtgcctgtgccagctcatgaccgaaagccatgccttcgttcgtcaggtcgtgaagtagcggtagccatgagctgtcatcgttaccgccacatatcatcccgctgattaaaccatgcatctcagctggggtcagacccgtcccttgttggttcagatactggttcatttcgttgtaaccaggcatttcgttctgtatagacataagcattcgtcgtcaaagggaggaatattcatgatatgctaccactttgggccctggtggaccagaaaagggcttgtctcttctcatcagggtagctatagtgtcgccccttcgcagaccatgggtctaaagacgaaggcagcgcagtcaatcagcaggaaggtggcatgtctgcacaacccgtcgatatccaaatttttggccgttcactgcgtgtgaactgcccgcctgaccaaagggatgcgttgaatcaggcagcggacgatctgaaccaacggttgcaagatctgaaagaacgcactagagtcacaaatactgaacagttggtcttcattgccgcattgaatatcagctatgagttagcgcaagaaaaagcaaagactcgtgactacgcggcaagtatggaacagcgtattcggatgctgcagcagaccatagaacaagcgttacttgaacaaggtcgcatcaccgaaaaaactaaccaaaactttgaatgacacttttcggtttactgtggtagagtaaccgtgaagacaaaatttctctgagatgttcgcaagcgggccagtcccctgagccgatatttcataccacaagaatgtggcgctccgcggttggtgagcatgctcggtccgtccgagaagccttaaaactgcgacgacacattcaccttgaaccaagggttcaagggttacagcctgcggcggcatctcggagattcccttcttatctggcaccagccatgacgcaactaccagaactcccactgacattatcccgacaagaaatccgcaaaatgattcggcaacgtcgtcgtgcgttaacgccggaacaacagcaggaaatgggtcaacaagccgctacccggatgatgacttatcccccggtggtgatggcacatacggtcgctgtattcctctcttttgatggcgaactcgacacccagccactcatagaacaactctggcgcgccggtaagcgcgtatatcttccagttttgcatccctttagtgccggtaatttgctgttcctgaattaccatccgcaaagcgaactggtgatgaacaggttgaagatccatgagccaaaattggatgtgcgtgacgtgctacccctttcccgattagacgtgctgatcacaccgctggtcgcctttgatgagtacggtcagcgcctgggaatgggcggtggtttttatgatcggaccttacaaaactggcagcactataaaacgcaaccggtgggttatgcgcatgattgtcagttggtggaaaaactccccgttgaagagtgggatatccctcttcctgcggtggttacaccgtcgaaagtctgggagtggtaagggcgatacacccgcatcgccctgattgacatcgttgattctttgacctaatttagtgagtaagggtaagggaggattgctcctcccctgagactgactgttaataagcgctgaaacttatgagtaacagtacaatcagtatgatgacaagtcgcatcataacccttctccttcaagccctcgcttcggtgagggctttaccgttacagccccatgctgccctgccatcgtaaatccccattaaataaacacaacgcattgatctgactttgatttattttctggagcagactcgcaaagtagaatgcgcaacgcggcaacggtgtggagaagggataaaaaaacgggcaagtcagtgacctgcccgttgattttcagagaaggggaattagtacagcagacgggcgcgaatggtacccggaatagctttcattgcctgcagcgctttttcggcaacgtcttcgtcggcttcaatatcaataaccacataacccatctgggcggaagtttgcagatattgcgcggcgatgttgacgccctgctcggcgaagattttgttcagcgcagttagcacgcccggacggttttcgtggatgtgcatcagacgacgcccaccgtgcagtggcagcgagacttccgggaagttcaccgcagagagcgttgagccattgtcagaatacttgatcaatttacccgcaacttccaggccgatattctcctgcgcttcctgagtcgaaccgccaatgtgtggcgtcagaaggacgttgtcgaattcacacagcggagaggtaaatggatcgctattggtcgccggttccgtcgggaatacgtcgattgccgcccccgccagatgtttgctcgccagcgcatcacacagcgccggaatatccaccacagtaccgcgcgaagcattaatcagcagcgagccgggcttcattagtgaaatttctttcgcgcccatcatatttttggtggacggattctctggtacatgcagactcaccacatcgctcatattcagcaggtcagaaagatgctgtacctgagtggcgttgcccagcggcagtttattttcaatatcataaaagtaaacatacattcccagcgattcagccagaatgcccaattgcgtaccaatatgaccgtagccgatgatacccagctttttgccgcgcgcttcaaaagaacccgccgccagtttgttccacacgccacggtgcgctttagcattggcttccggcacgccgcgcaatagcagcagcagttcgccaatcaccagctccgcaacagagcgcgtatttgagaacggtgcgttaaataccgggatcccgcgctttgccgccgcatccagatcaacctggtttgttccgatacagaaacagccaatagcgaccagtttttctgcggcgttgatcacgtcttcagtcagatgggtacgggatcgcaggccgatgaagtgggcatcgcggatggattcttttaattgttcatcatccagcgcgcctttgtgaaattcgatgttggtgtaaccagctgcacgaaggctttccagcgccttttggtgcacgccttctaccagcagaaacttaatcttgtctttctccagcgatacctttgccatttacccaatcctgtcttttgaaatgttgtgtgcggatttgcatccgcctttcaacatatcaaaaaataatattgcggcaatatgaacgtttgcgtcgcgatgttgaggaaatatcacgcaaaggtaattcttggatgaatatgctggtttagaggatttatttagagcaatcgacaattgcctggtaaaagcgtgacacatgtcaccaaatttaatgaagagaatttttttaacgggggaggttcccccgtcagatcatttcacaatggttttgacaccgtcaggtgtgccaatcagcgcaacgtccgcgccacggttagcaaacaagccaacagtcaccacgccaggaatcgcatttatggcgttttccatcgctatcgggtcaaggatttccatgccgtggacgtcgaggatcacgttgccattatcggtcaccacgccctgacggtattccggacgaccgcccagtttcaccagctgacgcgccactgcactacgtgccatcgggataacttctactggcagcgggaatttacccagaatatcaacctgcttggaagcgtctgcaatacagataaatttttctgcaaccgaagcaatgattttttcacgggtcagcgccgcgccgccgcctttgatcatttgcatgtggccgttgatttcatctgcgccatcaacgtagatgccaaggctgtcgacttcgttgagatcaaaaacgtgaatgccgaggcttttcagtttttcagtggaagcatctgaactggaaacggccccttcaatctggcctttcattgtaccgagcgcgtcaataaagtgtgcggcggtggaacctgtacctacaccaacaatggtgccgggctgaacatactgaagtgccgcccatcctactgcttttttcaattcatcctgcgtcatgatcgtttcgcctgtggtatgaaatttcacacgcattatatacaaaaaaagcgattcagaccccgttggcaagccgcgtggttaactcatccataaaatatcgcgcaatggcaggcatcccctttcgccccgcaaataaagcatacaacggtctgggtatgccgctccacggtgcaaacaggcgcaccagttcaccgttcgcaagcccctgtttacaggcaaattgaggcaataacgccacgccattcaacacaaccagggcgcgaactcgctgagcgaaatgcattagcgcaaatccctgatcttttaagctgcgcttttaaccacggatacaaatgttacccgccgacggcttcggtatatgcaacctgacacaaaattgtgtcatagtgcaggaaaaagcatttaccaggagcagacaacagcaatgaaacgcccggactacagaacattacaggcactggatgcggtgatacgtgaacgaggatttgagcgcgcggcacaaaagctgtgcattacacaatcagccgtctcacagcgcattaagcaactggaaaatatgttcgggcagccgctgttggtgcgtaccgtaccgccgcgcccgacggaacaagggcaaaaactgctggcactgctgcgccaggtggagttgctggaagaagagtggctgggcgatgaacaaaccggttcgactccgctgctgctttcactggcggtcaacgccgacagtctggcgacgtggttgcttcctgcactggctcctgtgttggctgattcgcctatccgcctcaacttgcaggtagaagatgaaacccgcactcaggaacgtctgcgccgcggcgaagtggtcggcgcggtgagtattcaacatcaggcgctgccgagttgtcttgtcgataaacttggtgcgctcgactatctgttcgtcagctcaaaaccctttgccgaaaaatatttccctaacggcgtaacgcgttcggcattactgaaagcgccagtggtcgcgtttgaccatcttgacgatatgcaccaggcctttttgcagcaaaacttcgatctgcctccaggcagcgtgccctgccatatcgttaattcttcagaagcgttcgtacaacttgctcgccagggcaccacctgctgtatgatcccgcacctgcaaatcgagaaagagctggccagcggtgaactgattgacttaacgcctgggctatttcaacgacggatgctctactggcaccgctttgctcctgaaagccgcatgatgcgtaaagtcactgatgcgttactcgattatggtcacaaagtccttcgtcaggattaatccatcaaataatgcctgatagcacatatcaggcgttgtcctcacttctttttgtattccttgaatcacatcacaaaatagacaaatctcaggcggcaaaaaacgacgtctgaatgcattttttttgctggcgacaaacccacgtaaaaagctcaccgtaggcgcaaataccctcattttgattgcgttttacggagcaaataatgtctaacgtgcaggagtggcaacagcttgccaacaaggaattgagccgtcgggagaaaactgtcgactcgctggttcatcaaaccgcggaagggatcgccatcaagccgctgtataccgaagccgatctcgataatctggaggtgacaggtacccttcctggtttgccgccctacgttcgtggcccgcgtgccactatgtataccgcccaaccgtggaccatccgtcagtatgctggtttttcaacagcaaaagagtccaacgctttttatcgccgtaacctggccgccgggcaaaaaggtctttccgttgcgtttgaccttgccacccaccgtggctacgactccgataacccgcgcgtggcgggcgacgtcggcaaagcgggcgtcgctatcgacaccgtggaagatatgaaagtcctgttcgaccagatcccgctggataaaatgtcggtttcgatgaccatgaatggcgcagtgctaccagtactggcgttttatatcgtcgccgcagaagagcaaggtgttacacctgataaactgaccggcaccattcaaaacgatattctcaaagagtacctctgccgcaacacctatatttacccaccaaaaccgtcaatgcgcattatcgccgacatcatcgcctggtgttccggcaacatgccgcgatttaataccatcagtatcagcggttaccacatgggtgaagcgggtgccaactgcgtgcagcaggtagcatttacgctcgctgatgggattgagtacatcaaagcagcaatctctgccggactgaaaattgatgacttcgctcctcgcctgtcgttcttcttcggcatcggcatggatctgtttatgaacgtcgccatgttgcgtgcggcacgttatttatggagcgaagcggtcagtggatttggcgcacaggacccgaaatcactggcgctgcgtacccactgccagacctcaggctggagcctgactgaacaggatccgtataacaacgttatccgcaccaccattgaagcgctggctgcgacgctgggcggtactcagtcactgcataccaacgcctttgacgaagcgcttggtttgcctaccgatttctcagcacgcattgcccgcaacacccagatcatcatccaggaagaatcagaactctgccgcaccgtcgatccactggccggatcctattacattgagtcgctgaccgatcaaatcgtcaaacaagccagagctattatccaacagatcgacgaagccggtggcatggcgaaagcgatcgaagcaggtctgccaaaacgaatgatcgaagaggcctcagcgcgcgaacagtcgctgatcgaccagggcaagcgtgtcatcgttggtgtcaacaagtacaaactggatcacgaagacgaaaccgatgtacttgagatcgacaacgtgatggtgcgtaacgagcaaattgcttcgctggaacgcattcgcgccacccgtgatgatgccgccgtaaccgccgcgttgaacgccctgactcacgccgcacagcataacgaaaacctgctggctgccgctgttaatgccgctcgcgttcgcgccaccctgggtgaaatttccgatgcgctggaagtcgctttcgaccgttatctggtgccaagccagtgtgttaccggcgtgattgcgcaaagctatcatcagtctgagaaatcggcctccgagttcgatgccattgttgcgcaaacggagcagttccttgccgacaatggtcgtcgcccgcgcattctgatcgctaagatgggccaggatggacacgatcgcggcgcgaaagtgatcgccagcgcctattccgatctcggtttcgacgtagatttaagcccgatgttctctacacctgaagagatcgcccgcctggccgtagaaaacgacgttcacgtagtgggcgcatcctcactggctgccggtcataaaacgctgatcccggaactggtcgaagcgctgaaaaaatggggacgcgaagatatctgcgtggtcgcgggtggcgtcattccgccgcaggattacgccttcctgcaagagcgcggcgtggcggcgatttatggtccaggtacacctatgctcgacagtgtgcgcgacgtactgaatctgataagccagcatcatgattaatgaagccacgctggcagaaagtattcgccgcttacgtcagggtgagcgtgccacactcgcccaggccatgacgctggtggaaagccgtcacccgcgtcatcaggcactaagtacgcagctgcttgatgccattatgccgtactgcggtaacaccctgcgactgggcgttaccggcacccccggcgcggggaaaagtacctttcttgaggcctttggcatgttgttgattcgagagggattaaaggtcgcggttattgcggtcgatcccagcagcccggtcactggcggtagcattctcggggataaaacccgcatgaatgacctggcgcgtgccgaagcggcgtttattcgcccggtaccatcctccggtcatctgggcggtgccagtcagcgagcgcgggaattaatgctgttatgcgaagcagcgggttatgacgtagtgattgtcgaaacggttggcgtcgggcagtcggaaacagaagtcgcccgcatggtggactgttttatctcgttgcaaattgccggtggcggcgatgatctgcagggcattaaaaaagggctgatggaagtggctgatctgatcgttatcaacaaagacgatggcgataaccataccaatgtcgccattgcccggcatatgtacgagagtgccctgcatattctgcgacgtaaatacgacgaatggcagccacgggttctgacttgtagcgcactggaaaaacgtggaatcgatgagatctggcacgccatcatcgacttcaaaaccgcgctaactgccagtggtcgtttacaacaagtgcggcaacaacaatcggtggaatggctgcgtaagcagaccgaagaagaagtactgaatcacctgttcgcgaatgaagatttcgatcgctattaccgccagacgcttttagcggtcaaaaacaatacgctctcaccgcgcaccggcctgcggcagctcagtgaatttatccagacgcaatattttgattaaaggaatttttatgtcttatcagtatgttaacgttgtcactatcaacaaagtggcggtcattgagtttaactatggccgaaaacttaatgccttaagtaaagtctttattgatgatcttatgcaggcgttaagcgatctcaaccggccggaaattcgctgtatcattttgcgcgcaccgagtggatccaaagtcttctccgcaggtcacgatattcacgaactgccgtctggcggtcgcgatccgctctcctatgatgatccattgcgtcaaatcacccgcatgatccaaaaattcccgaaaccgatcatttcgatggtggaaggtagtgtttggggtggcgcatttgaaatgatcatgagttccgatctgatcatcgccgccagtacctcaaccttctcaatgacgcctgtaaacctcggcgtcccgtataacctggtcggcattcacaacctgacccgcgacgcgggcttccacattgtcaaagagctgatttttaccgcttcgccaatcaccgcccagcgcgcgctggctgtcggcatcctcaaccatgttgtggaagtggaagaactggaagatttcaccttacaaatggcgcaccacatctctgagaaagcgccgttagccattgccgttatcaaagaagagctgcgtgtactgggcgaagcacacaccatgaactccgatgaatttgaacgtattcaggggatgcgccgcgcggtgtatgacagcgaagattaccaggaagggatgaacgctttcctcgaaaaacgtaaacctaatttcgttggtcattaatccctgcgaacgaaggagtaaaaatggaaactcagtggacaaggatgaccgccaatgaagcggcagaaattatccagcataacgacatggtggcatttagcggctttaccccggcgggttcgccgaaagccctacccaccgcgattgcccgcagagctaacgaacagcatgaggccaaaaagccgtatcaaattcgccttctgacgggtgcgtcaatcagcgccgccgctgacgatgtactttctgacgccgatgctgtttcctggcgtgcgccatatcaaacatcgtccggtttacgtaaaaagatcaatcagggcgcggtgagtttcgttgacctgcatttgagcgaagtggcgcaaatggtcaattacggtttcttcggcgacattgatgttgccgtcattgaagcatcggcactggcaccggatggtcgagtctggttaaccagcgggatcggtaatgcgccgacctggctgctgcgggcgaagaaagtgatcattgaactcaatcactatcacgatccgcgcgttgcagaactggcggatattgtgattcctggcgcgccaccgcggcgcaatagcgtgtcgatcttccatgcaatggatcgcgtcggtacccgctatgtgcaaatcgatccgaaaaagattgtcgccgtcgtggaaaccaacttgcccgacgccggtaatatgctggataagcaaaatcccatgtgccagcagattgccgataacgtggtcacgttcttattgcaggaaatggcgcatgggcgtattccgccggaatttctgccgctgcaaagtggcgtgggcaatatcaataatgcggtaatggcgcgtctgggggaaaacccggtaattcctccgtttatgatgtattcggaagtgctacaggaatcggtggtgcatttactggaaaccggcaaaatcagcggggccagcgcctccagcctgacaatctcggccgattccctgcgcaagatttacgacaatatggattactttgccagccgcattgtgttgcgtccgcaggagatttccaataacccggaaatcatccgtcgtctgggcgtcatcgctctgaacgtcggcctggagtttgatatttacgggcatgccaactcaacacacgtagccggggtcgatctgatgaacggcatcggcggcagcggtgattttgaacgcaacgcgtatctgtcgatctttatggccccgtcgattgctaaagaaggcaagatctcaaccgtcgtgccaatgtgcagccatgttgatcacagcgaacacagcgtcaaagtgatcatcaccgaacaagggatcgccgatctgcgcggtctttccccgcttcaacgcgcccgcactatcattgataattgtgcacatcctatgtatcgggattatctgcatcgctatctggaaaatgcgcctggcggacatattcaccacgatcttagccacgtcttcgacttacaccgtaatttaattgcaaccggctcgatgctgggttaatgactcgtcccgtcacgatcttcagcaatatgctgaagcatcgtggcggtataacgatgatttctgattgaataaagatattcctgcatatacatcggcctgtgcggtgcatcaaaatatttcagcgttgccggattcaccagtcgccaggcaaaatgcgggatcaccgtcagaaaatgtccgcgctccacggcgctgattttggccataaaactgtagggacgataaataatggttggattgatcccacaaggtcgcatattcgcatcaatcattgcttcgaagttggcccggttctgaaagcgcatttgtagccagggcagctcctgaagcagctcttgctcttgtcgctcttcataacggcgagaaacgagaaagcctaatcgcagcggtggtagttcactgatagtcaggttttccagttcctgaactcgtgcagatacatgctgtggggagataataaaatctaactggcggtcaaaaagattatcgataacgccattttcgctgaactcaactggctgggcggtcacgccttcatacttatctccgagactaatcaactgatcgaaaataattgtcggataagtattatctatgccaatcacaatttctcgtgaacgacgccctgagttatggatttcattatcaatcgcagaaagccgttgataaaccgggaacagtttttgatacagttcctgtccggctttattgaggctgatattattatctttgcgggtaaatagcgtatagccaatttgttcttccagcgcggcaatgcttttaccaaatggcgaagccgtcatatggattttttctgccgcccgggcaatattattggtttgcgctaataaaatgaaattgcgcatctttttcgaaataaaaatgtccatccccctcccccgcatccttgtccgcttaaccgtttcagtcagcctatccttgatgaaaccgcgagcaaagataggtgattacgtcatggttttacagaaaattacagaaaaaggaggcaatatcgggtaaaggcattagcccgacgaatacgtcgggctacaaatattattgtgctgcaggtgttttagcgggttgttgatccacaggttctaactggaagaccacatcgacctgatcatcaaactgaatagcggcctgctcgtaagtttcctgggcggacaccggcgcggcatcggctttcatcatccgcaccattgggctgggctgatagttggaaacatggtagcgcacgctatataccggccccagtttacgatgaaagccgttcgccagttcctgcgcctgatgaatcgcgttatcaatcgctgccttacgcgctttgtctttataggcatccggctgcgccacgcccagcgacacagaacgaatttcgttaagacccgccttcagcgcgccatccagcaaggaattcagtttgtctaactgacggagcgtgacttccaccgttctcacagcgcggtagcctttaaggatacttttaccatcctgataatcataatctggctgggtgcgtaagttcgctgagctgatatcttttttcgcgatctgattgagttcaaggaaggaaatgtattgtgcgacgcgctcatctgcctgtttcttggcagtagcggcatccttcgcggccacgttaacttcaatcgcaagagtggcaatgtctggcaccgcatccacgcttgccgtaccggaggtgacaatatgcggtccatccggcaattcgttagcctgcgctgccatcccgctaatacccattaatgccgccagggcgataactttgaacttcacgttagtctctccgtgttaattgacttgcccaaaattcaggacctctggaggcaagcttagcgcctctgttttatttttccatcagatagcgcctaactgaacaaggcttgtgcatgagcaataccgtctctcgccagctgcaaggcaataaaccacataacacatcccacaaccagattgataatgcgctgtgcttttgccgtgcgcagacgcggtgccagccaggctgcgagaagagccagaccaaagaaccacaggaaagaggcgctaattgtcccgagtgcaaaccagcgttttggttccacatcaagttgcccgccaaggctgcccagtacaacaaaagtatccaggtaaacatgcggattcagccaggtcactgccaacatggtggcgataattttccatctgccttgcttcatgacttcggcgctggctaactcaatattactgctcattgctgttttaaaagcgccaaaaccataccacagcaagaaggctacgccgccccaggtgaccagcgccagcaaccacggcgactgcatcaataacgcgctgccaccaaaaatcccggcgcaaatcaggaccaaatcgctgatagcacaaagtaaggcaatcataatgtggtactgacgacgtatgccctgattcatcacaaaagcattttgtggaccgagcggtaggatcatagccgccccaagtgcaagaccttgaaagtaataagaaaacacgttggatattccgaattaagtatctgatgcagagactatatcgcgggattgttattagcggaaattgataatattaattggcaatcagaaaaactaataagagagaggccagagagtattatctggcctcagcgttgattacgcagctttgtcttctttcacccgcttaaagttcacatccatttgcgggtacgggaagctgataccggcggcatcaaattcacgtttaatacgctccagcacatcccagtacacgttttgcagatcgccgctgttgctccagacgcggaccacgaaattaatcgacgatgcaccaagttcgttcaggcgcacagtcatttcgcgatctttcaaaatgcgatcttcagactggataatattggtcaggatctgcttaacctgatcgatatcggaatcatacgccacgccaataataaattcgttacggcgaactggctcgcgggagaagttaataatatttccggcaataattttaccgttcggaataacgataattttaccgtctgcagtacgcatggtggtggagaaaatctgcacactcagcacagtaccggctacgccgcccaggtcaacatattctccggcacggaacgggcggaacatgacaagtaacacgccagcggccaggttagacagtgacccctgcaaagccagaccaacagctaagcctgcggcaccgagtacagcaatgactgacgcggtttgtacacccacgcgtcccagtgcagcgattagcgtaaaggcgataataccgtaacggactaatgcagaaagaaaatcagcaacagtggcatcgattttacgggagatcatcaggcgattcaccgcgttggaaatcatccgcgcgataatcaaaccaacgatgatgatcgcgagtgccgccacgatgtttactgcataacttagcagcagcgcctggttagctaccagccagcttcccgcgccgtttatgctatcgacaacattcaaatcttccattcaatattccttttcaactgactcaaaatggagaaatacactccgccgccttatgacgggcagtctgacaagggtaaacaataaagcataattttgccaaatagatcacagatttctcatctgaatcaccttgcttttggcgaaaaaatccccgcagagcggggctcagacagatatcaatgtgcgctttgtcatgccggatgcggcgtgaacgccttatccggcctacaaaaacctgcaaattcaatatattgcaggatacgtgtaggcctgataagcgtagcgcatcaggcaattttgcttttggcgaaaaaaagacccgcagagcgggccttgagataagcagaaaggaatatcttacagaacgtcgatcgcgttcagttcctggaatgctttctccagacgagcgatcatcgaagtctgaccggcacgcagccatacgcgcggatcgtagtatttcttgttcggctgatcttcgcctttcgggttacccagctgaccctgcagataagcttcgttcgctttgtagtagttcagaacgccttcccaggttgcccattgggtatcggtatcgatgttcatttttactacgccgtagcttacggagtctttgatttcctgagcagtagaaccggaaccaccgtggaatacgaagttcaggctgttgtgcggcaggttgtgtttcttggaaacatattcctgagaatcacgcaggatggtcggagtcagaaccacgttacccggcttgtaaacaccgtgtacgttaccgaaggacgctgcgatggtgaaacgcgggctgattttgctcagttcggtgtatgcgtaatcaacgtcttccggctgggtgtacagtgcagaagcgtccatgtggctgttgtccacgccgtcttcttcaccaccggtgcaacccagttcgatttccagagtcatgccgattttggacatgcgctccaggtatttagagcagatttcgatgttctcttgcagagattcttcagacaggtcgatcatgtgagaagagaacagcggcttaccggtagctgcgaagtgtttttcacccgcgtccaacagaccgtcgatccacggcagcagtttcttcgcgcagtggtcagtgtgcaggataaccggaacaccataatgttcagccatctggtgaacgtgatgcgcaccagagatcgcgcccaggatagcagcaccctgcggaacgtcagatttcacgcctttaccagcgataaaggaagcaccaccgttggagaactgaacgataaccggcgctttaactttagcagcggtttccagtacggcgttgatggagtcagtaccgacgcagtttactgctggcagtgcgaagttgttttcttttgctacctggaaaactttctgtacgtcatcaccagtgattacgccaggttttacgaaatcaaaaatcttagacatgtctcttgtcctgtatcgtcgggccttatactcgtcatacttcaagttgcatgtgctgcgtctgcgttcgctcaccccagtcacttacttatgtaagctcctggggattcactctcttgtcgccttcctgcaactcgaattatttagagtatgaaaaattgcgtgctctaaaagcgcgctgaaacaagggcaggtttccctgccctgtgattttttacttcttagcgcgctcttcgagcatcgctactgcaggcagtactttaccttccacgaattcgaggaatgcgccgccgccagtggagatgtaggagattttgtcagcaatgccgaacaggtcgattgctgccagagtgtcgccgccgccagcgatggagaacgcttcgctgtctgcgatagcgttagccacgatttcagtacctttgcggaagttcgggaattcgaacacgccaaccggaccgttccacagaatggttttcgcattcttcaggatttcagccagttcctgagcggaagcatcaccgatatccaggatctgctcgtcagctttcacatcgttaacagatttcagggtagccggtgcagtttcagagaactcggttgctacgcgaacatcagacggaaccgggatgttgcaggtggtcagcagacgtttagcttcgtcaaccaggtcagcttcgtacagggatttacccacatcgtggccttgtgccgcgataaaggtgttagcgataccaccaccaacaatcagctggtcagcgattttagacagggagtccagaacggtcagtttggtagatactttagaaccaccaacgatagccaccatcgggcgagcaggttctttcagtgctttacccagcgcgtccagttcagctgccagcagcgggcctgcgcacgcaacgtcagcgaatttaccgataccgtgagtagaagcctgcgcgcggtgagcagtaccgaatgcgtccattacgaacacgtcacacagtgcagcgtattttttggacagggtttcgtcgtctttcttctcgcctttgttgaagcgaacgttttccagaacaaccagttcaccttcagcaacgtcaacgccgtcgaggtaatctttaaccagacgaaccgggttagacagtttgtctttcaggtagttaacaaccggcagcagagagaattcttcgttgtactcgccttcggtaggacgacccaggtgggaagttaccatcacttttgcgccttgtttcagggccagttcgatggtcggcagagaagcacggatacgcgcgtcgctggttactttcccgtcttttactggtacgttcagatccgcacggataaatacacgtttcccagcaagatccagatcggtcatcttaattacagacatggtgaatcctctcgttgattctaaaagttttgcagacgctgcttgcgtcttacctgaaagcaacagtagccatagctaacgtcgtgtcgagcattcggttagcaaagccccattcgttatcgcaccagaccaacgttttgatcaggtgtgcgccactgacccgggtttgggtgccatcgacaatggcactgtgcggatcgtggttaaaatctacagagaccaacggcaattccgtatagtcaactataccatgaaatgcaccttgtgctgctttttgcagcaacaggttgacttcattggcttttacaggtttcttcaccgtcacgcttaaatcgattgccgtcacatttatggttggcacacgtaccgcaatcgcttcaaagcgatcgttaaattgcggaaaaaatcgtgtgataccggcggccagtttagtatcgaccggaatgatcgactggctggctgcccgggtgcgacgcaggtcaggatggtatgcatcaataacctgttgatcgtgcatggcggagtgaattgtggtcacagtgccggactcaataccgtacgcatcatctaacaatttgatgacgggaattatgcaattcgtggtacaggaagcgttagaaacgatgcggtgttccgcacgaagttgatcctgattgacgccgtaaacaacggtcgcgtcgagatcgttactgccaggatgtgaaaagagcacttttttggccccggcggcaatatgcgcttcgccatgctcgcgggagccatatacgccggtgcagtcgaggactacatcaacgccaagttcacgccaggggagcgattgcagtgaacgttcatgcaatacgcggatggcgtcatcaccaacaaaaagttgatcgcgttcctgtcgtacttcccatgcaaaacggccatggctggtgtcatatttcaacaaatgcgccatgcccgcagcatccgccagttcgttgattgccaccacggtaatttccgcccggcgtccggattcatacaaagcacgaaccacattacgcccgatgcgaccgaagccatttatcgctacgcgtacggtcatagatctcctgcaaggttttccctgagcaaatttgccagacagagtaatccagcaaatcgtccggggaaaccttacctgtcgcaaactgcgactgattggttaattgtcgaacatttaatcgactgaaacgcttcagctaggataagcgaaacgtggaataaaaggaatgtttgtccagccgaagaagacatttatctgactcacatcacacttttatccccttttgtgggaagctttattccaggctggcgtaataataaccctacaataactggaataaattgtcagcttgtgaagtgataccggccttcttcagtcatctctactatcagattggcctgacggctattcatcagcacacgctcgacattggggccatcggtgcgggcataaaatgcttcggctacttgccgcgttaatcctcccgcaattttacgactaatcaagcgctcccgcagaatttgagcaggtgcatgaataaaaatagaaaaatcgcagaaagatgccaactccagccacttttcatcatccagtaacaaccagtttccttcgacgatgacgagtggtgcggtaacgtgcaacgcatcttcaacaggatcatgcttttgtcgatcgtactgcggccacgtacaatccccttccacgacctggcgcagattttccgtcagtttcgcaacgtcaaatgtctctggtgcgcctttgaaggggcgcaattgatgcgcatccagccagctattgtaatggtgaaaaccatccatcgggagcgtctgaatagcgggcagttccgggtcttgttgcgcgagatattcccagaaggtggttagggttgatttacccgtccccggcggagcgcaaagaaaaaccaccgtacgccgctgcggatttaccgtctgtaaggccgccaacatgtgcagcaacggtttatgtacattttcaatctcttcgttctggtactgtgcctgtatcttcagcccattcaccgttaattcaattttcacggcgttaattcctttaaggtggtcgttactgccagcgtcagcgccgttttgaccattccgctaaaacgcgcctctgaccagacggagaaatcagcgaacttcatcgcttttaacgcgtcatagagcatcgcattgcgggttatgctattgacgttgctgataaaatcccaggtcatgtcatcggcaaatccgggcgtttcatcctgttcgttcaggtaatgccagaactgggaaaaatgcgtgatatcggcgtacaaccatttatccattttccccaacgcataaatcaaacgcagtgcaacatcaatatcgtcaagcgggccgctttgggcgagtaacggcttcactgcatattccacgatctcttcatcgttatcgacaaacagcgacggcagaaactggcgtatcccctggagcaaaatggtatgcgcagttttcataaatgaaaataaattgtcctgtgcatccagttgctcaagcacatcatcttctgtcagcgtcgccattggtcttccgatagatcaccatcaatgcagggagtctattatattacacgtttggtccgcgccgccgatcagtaatgtctgcgtccgcaccccattcgccgtctgttggataccgttcaccagctcaccgcccgtcacgcccgtagcgctaaagaggatatcgttccccctcaccagttcatcgagcgagtacacacggttaacgtcaacgcccattgccttgcaacgcttgcgctcctgctctgcaatctgccgattttccgtgtaatcccctttagcctggcaaaagtcaatcagctcggcctgcatatccccgcctaatgctttaacggcacaggcagaaatcacgccttctggcgcaccgccgatggtgtacatcacatcgtaaggattatcctgccagcaggtcagcacgctggcggcgacatcgccatccggcagggcaaaaaccttcacgcccagctgtgttgcttcctcaatcgcggcactcaggcgcggtttatccagcgtaaccatgcgcagcttatccagcggtttgcctaacgctttcgccacgttgcgcaggttgtccgtcagaggcaaagacagatcaatcgcgcccgccgccagccgattaacaaccagctttttcatatacatatcgggcgcatgtaacaggctatctcgaggggcgaaagccatgaccgccagcgcattgctctgccccatcgccaccatccgcgtgccttcaatgggatcaaccgcgatatcgacttctggcccatcgcctttgcccacctcttcgccaatccacagcatcggcgcatggtcaatttctccttcgccgataaccactcgtccacgaaaagcgacgtcgtttaatgcctggcgcatcgcggtgaccgccaggccatcaattttatttttgtcgccacatccggtttgcggccaggcagccaacgctgcctgttccgtaacgcgaaataatggccacgccagggacatcattgcgcggcctccccgatatcaacgccaaattgtgccagcagatatttctcggcctgttcattccagatgccgtgcgtttcctcaaccagccgcgccaactctttaaacagcggatcggttttgcctttttcggcaaaatcggcaatggcagtgagcggcatggtcacgccgttataaatgagttttttaccgccagggatatccggcagattgagcacggtttctggcaccgcatccaggccaccgatatgggtcaccataaacgacggctgtaactgcccagtggcgctaagggcaatcgcctctttcatgtcgtccgttgaaccgccagatgtaccgacgacgtgcgtgctgttgtaatggacgttgtagaaattaaacggcactttgaagtttttatccgtcggcccggcaaagaagttcagacagccatcttccgccagtaattcatcagccatctcaacgacagcaggcaccgccgcataaacaaaaatgtcatcgaacccggcatctcctgtcagcgcccgcagcatctggacaggatcgctcatccctttggtattcacatacaccagctcaatgcctttactggccgccagttccaccggcagcagcttctgtacctgcgccagacgtttgtcgtcgatatcgaccaccaccacccgcgacggttgtatgccgccgttaatggcgtaatcgatagcgccaatgcccatcggacctgcacacgccagcagtgcaatattgccgccaggtttgacgcccatgcgatgctcataaacatattgcgtggtgtgataattggcatgataagcaccaataatgcagcacataggctctgccagcgacgccgcagcaaaataagagccgtgatacggtaatacgcagcccaaattaatggcgatttcgggaataatcatataagtggcattgccgccaaaatattcgtagctgtagcccgctgaatatccgcttggtaaccccatcgccggttgcaatacaaaacgctggccttttttatatttgccagtgagatttttacccacttcgacaataaccccggcacattcatgcccggtaatgaccggatgattttctaaatcgtcgggtacgcgtttatgttcactaccgagtaacgccgctttccaggtcgataaacagacgctgtcagaaattacactcaccagtaattcattatcggtaatttctggcagttcaaatacgcgcagacggacatcccgcttgccataaatagcagcaactttggttttcatttttacctctgtaatcagtgtttatgttcggcggttaattgattaaataaagtgtcgagttttggatcgccaatatagttattaatcaatatcagtggtttatccgtcacacgtttcacgcgcccttccagactggcatgagtaacgacgatatccgcatccgcaggcacgttttctatggcgtaatgttttacttcaattgccagccccgctttttccaggcgtttacggaaggtggtcgcgcccatcgcactggagcccatccccgcatcgcaaacaaaggcgatacgcttaaccctgcttaacgagaatgcaccctcttgtttcatcgccttaaccgcattggctgactgagcaaactcatcttcgctctccgtttccaccgttttttccatcttcagtatcagcgaagtaatagcaaaggacaccagggtacctaccgtaacaccggcaattgtcgccaggaacgagcctttcggcgtcagtgccaggtaagcaaagatagaccccggacttgggccagccaccagaccaccgtccagtaagttaaacatccaggtgccagacataccgcccgcaatcatggcaataatggtcagcggcttcatcagcacatacgggaaatacagttcgtggatcccaccgaggaagtgaataatcatcgccccgggcgcagaacgtttactcatccctttaccaaacaaggtaaacgccagcagcagccccaggcccggacctgggttagaggccaccataaagaagatggatttaccgttaaccgaagcctgttgcattcccagcggataatagacgccctgatcgatcgcattattgaggaaaagcactttcgccggttcattgatgactgacaacaatggcagataacccgcatgtaccagcgcctcaatacactctttgacgaaagtattggcaattaacaccgccgggccgataacttcaaaacccagcagacaaaggagcatccccgcgatacctaatgagaagttattgataaccatctcaaaaccggcaggtatgcgtttttccagtgccttatcgacatattttatgaccaacccaccgagcggccccatgatcattgagccaaggaacatcgggatctctgcgccaacgatcacaccaatagtacctattccgcccatgaccgccccgcgtttaccgccgaccagatgaccacctgtagaaccaatcatcacgggcaataaataggtaatcatcgggccgacaattttggcgaaatgttcgttaggcagccaaccggtgggaataaataacgcagtaataaaaccccaggcaataaaagcaccaatattggggatgaccattgcagtcaaaaagcccccaaaagcctggacctttgcacgagcagacttgttttccataatattatcctgtagaggagagagtaattatccgcggctgataatgtccgctaattgtttttctgatgatgctgttaagagttgttcgagtatttcttcttcgcacagtaattcacttaacgcctgaatagcgccaatgtgcgaatcggcatcggcagcagagagtccgatgagtaatttaattggttcgtcattccccggaaaataaacaccttgttcaagtaatgtcaaagacatcccggttttaagcgccccacattccggtcgcgcatgaggcattgccacgcctggtgcgagaatataataagggccattgttaatggtggaatctttaattgcctgaatgtaattctcgctgatatagtttttatccagcaatgataccatcgagaaatcgatagcttcctgccaatcttttgctgaatgtataactgagattgatgattctggaaaataatcactaagccgcataaattatccttattttatttttagggtaccgtccggcggtaaaaataaaatactcgtgcggtttaatgaaagcaattgagcagggaaaccggtgttttgaaaacagtgaattattaatttcttatataacattgagttatagatataacaacaaatgtcaatacgcatatcgtgatgcatattacataattgatatttattgcatataaatatttgtgatctacaacacgccttatctattgcttgtccgcaaacggacatatcaaggtaataaaaaaggtcgccgaagcgacctttttacccgaaatgctaattacagcagttcttttgctttcgcaacaacgttatcaacagtgaagccgaactcttcaaacagcagctctgccggagcagattcaccgaaggtggtcataccgacgatagcaccgttcaggccaacatacttgtaccagtagtcagcaatacccgcttctacagcaacgcgtgcagtaaccgctttcggcagtacggattcacggtaagcagcatcctgcttgtcaaatgcgtcggtagacggcatggacaccacgcgcgctttcacgccttcggcagtcagtttttcgtaggcagcaacagccagttcaacttctgaaccggtagcgatgaaaatcagttccggctgaccggcgcagtctttcagcacataaccaccgcgcgcgatgtttgccagttgctcttcagttcgttcctgctgcgccaggttctgacgggagaggatcagtgcggtcgggccgtcctgacgctcaacaccgtatttccacgcgaccgcggattcaacctggtcacacggacgccatgtagacatgttcggggttacgcgcagagaagcgacctgctcaaccggctggtgagtcgggccgtcttcgcccagaccgatggagtcgtgggtgtaaaccatcacctgacgctgtttcatcagcgcagccatacgtacggcgttacgtgcgtattccacgaacatcaggaaggtggaggtgtacggcaggaagccaccgtgcagggagataccgttagcaatcgcggtcataccgaactcgcgaacaccgtagtggatgtagttacccgcagcatcttcgttgattgctttagaaccagaccacagggtcaggttagacggcgccaggtcagcagaaccgccgaggaattccggcaacagcggaccgaacgcttcgatagcattctgagacgctttacggctggcgattttcgccggattagcctgcagtttagcgatgaactctttcgctttagcgtcgaagtcagacggcatttcgcctttcatacggcgggtaaattcagcggcttcctgcggataagctttcgcgtaagcagcgaatttctcgttccatgcggattctttcgcctggcctgcttctttcgcatcccactgagcatagatttcagacgggatttcgaacggcgcatatttccagcccagttgttcgcgggtcagggcaatttcagcgtcgcccagcggcgcaccgtgggagtcgtgggtaccggctttgttcggggaaccgaaaccgatgatggttttgcacatcagcagggaaggtttgtcagtcactgcgcgcgcttcttctactgcgcgtttgatagatgccgcgtcatgaccgtcgatgtcgcgaataacgtgccagccgtaagcttcgaaacgcattgcggtgtcgtcggtgaaccagccttcaacgtgaccatcgatagaaataccgttgtcatcgtagaatgcaatcagtttacccagcttcagcgtacccgccagagagcaaacttcgtgggagatgccttccatcatgcagccgtcgcccatgaaggcgtaggtgtagtggtcgacaatgtcgtggcccggacggttaaactgcgccgccagcgttttttctgcaatcgccataccgactgcgttggcaataccctgacccagcggaccggtggtggtttccacaccagcggtgtaacccacttccgggtgacccggagttttagagtgcagctgacggaagtttttcagttcttccatcggcagatcgtaaccggtgaggtgcagcaggctgtagatcagcatggagccgtggccgttggacagcacgaagcggtcacggtcagcccaggacggattctgcgggttgtgtttcaggaaatcacgccacaggacttcggcaatgtcagccatacccataggggcacccgggtgaccggatttggctttctgtactgcgtccatgctcagcgcacgaatagcattggcaagctctttacgtgaggacattttgactccagatcggatgatgaagggcacgcccttaacgacttgacgacagcgcgttttgggctacgccggaaaatttgccaacaatttaccgcaagccgcgcgtcatgtacatggaacatccttttgccgcttcagaaatctctggatcatgctcgcatgttgcgcaatctactcgcccgtccgctgcgcttttccttatactgagactgagcgtcgattcacctgcaaacggcgcatttttagaataatcctgaccttgtgcggaagagaaaacatgaaaattcgcgccttattggtagcaatgagcgtggcaacggtactgactggttgccagaatatggactccaacggactgctctcatcaggagcggaagcttttcaggcttacagtttgagtgatgcgcaggtgaaaaccctgagcgatcaggcatgtcaggagatggacagcaaggcgacgattgcgccagccaatagcgaatacgctaaacgtctgacaactattgccaatgcgctaggcaacaatatcaacggtcagccggtaaattacaaagtgtatatggcgaaggatgtgaacgcctttgcaatggctaacggctgtatccgcgtctatagcgggctgatggatatgatgacggataacgaagtcgaagcggtgatcggtcacgaaatggggcacgtggcgttaggccatgtgaaaaaaggaatgcaggtggcacttggtacaaatgccgtgcgagtagctgcggcctctgcgggcgggattgtcggaagtttatctcaatcacaacttggtaatctgggcgagaaattagtcaattcgcaattctcccagcgccaggaagcagaagccgatgattattcttacgatcttctgcgccaacgcggcatcagcccggcaggtcttgccaccagctttgaaaaactggcaaaactggaagaaggtcgccaaagctcaatgtttgacgaccatcctgcatccgccgaacgcgcccagcatattcgcgatcgcatgagcgcggatgggattaagtaaagcctggtggtgtcgaacgtaggtcagataaggcgttcacgccgcatctgacatgaatggcacatttgttaccttgtgcgcattgccggatgcgatgctggcgcatcttatccggcctacgggtgccgaacgtaggtcggataaggcgttcacgccgcatccgacattaatggcacgttttacccgtgcgcatcgcatctggtgcttactcgccctttttcgccgcctgaatatacagcatttccagcgccagcgttgccgctgccagagcagtgatttccgactgatcgtatgccggagccacttccactacgtccatcccaacaatgttgagatctttcaggccgcgtaccagtttaatagcgcgatcggaggtcaggccgccaatcactggcgtaccggtgcctggtgcaaaagcaggatccaggcagtcgatatcaaaagtcaggtaaaccggcatatcacccacaatctgtttcacttgggcgataacgtcatccacgctgcgatcgttcacctggcaggcgtccagcacggtaaagccgttgtctttatcaaactcggtacgaataccaatctgcacggaatgattcgggtcgatcagaccttctttcggcgcggtatagaacatagtgccgtggtcaaattcacaaccgttcgcataggtatcggtgtgggcgtcaaagtgtaccagcgccattttgccgaaatgcttcgcatgagcacgcagcagcggcagcgtaacaaagtggtcaccaccgaaagagagcatacgcttaccggcagccagcagcttctcggcgtgcgcctgcagcttttcgctcatctcacgggcatcgccaaaggcatataccagatcgccgcagtccacgacgttcagacgctcacgcatgtcgaaattccacgggaagcggttgtgttcccaggccagattcgtcgaaacctgacggatcgctgccggaccgtggcgaccacccgcacgaccagaagtggccatatcgaacggcacgccagtaatcacccagtctgcatcgctgtcatacggctggaagttcatcggcaggcgtaaaaaaccaaaggcattggaaaccagtgagttatcgtattgatgacctaaggtgctcatggatggactcctattacaaagtcgatataaaaaaacccttccgcgtcgttaggcccgacgaggaagggttggatttgtcacaataaattgtggcggattatcaccgctaaattaagcggattcaagtaacacaggacttactcatcttcaagataagtataaccgtacaaacctgcctcgaactcttcaaggaactgttgttgcagttcagcatcaagatcggttttcttcacttgatcgcggaactgggttaacagcgttttcggatcgagctgtacatattgcagcatgtccgccacggtatcgccttcgtcagacagttctacttctacgctaccgtcagggaagacgaacacgtcaaccgcttcggtatcaccgaacaggttgtgcatgttgccgaggatctcctgatatgcgccgaccataaagaaaccgagcatcggcggattctctggatcgtactccggcattggcattgtcgtggcaataccgtcaccatcaatatagtggtcgatagcaccgtcagagtcacaggtaatatccagcagcacagcgcgacgttccggcacttgatccagcccttccagcggcagaaccgggaacaactggtcgatcccccatgcgtccggcatcgactggaacagcgagaagttgacgtacattttgtccgccatacgttcctgcagctcgtcgataatcggacgatgagcacggttttgcggatccagctgcttttgcacttcatggcacatgctcaaataaagctgctcagcccatgcacgttcttgcaggctaaagatgccggaagagtagccgatatgaatgtcgtgcagatccatctgactgtcgtgtaaccattcacgcagagaacggcgagttcccggttcgtgcatctcctgccaggtttcccacatgctttgcagcgcgcgcggcgcatcttctgcaggcgcggtcggcaccgtgtattcgttacgttccacgccgatgatattagacaccagcacggtgtgatgcgcagtcaccgcacgacccgattcggtgattaccgtcggatgcggcagaccgttttcttcacacgcatcgccaatcgcccagataatgttgttggcgtattcattgaggccgtagttcaccgaacagtcggactgcgaacgagtaccttcataatccacgcccagaccgccgccgacgtcgaagcactgaatattgacgcccagcttgtgcagttccacatagaaacgcgcggattcacgaacgcctgtcgcgatatcgcgaatattcgccatctgcgaaccgaggtggaagtgcagtagttgcaggctgtcgagacgcccggcttcacgcagggtttcaaccagttgcagtacctgagtcgcagccaggccgaacttcgatttttccccgccggaggactgccatttacccgaaccctgcgaagccagacgtgcacgcacgcccagacgaggaacgacattcagacgttctgcttcatccagcacaatggcgatttctgacatcttctcaatgaccagatagaccttgtgccccatcttctcgccaattaatgccaggcggatatattcgcggtctttataaccgttgcagacgatgacgctacgggtcatgccagcatgtgccagtactgccatcaactcggctttggaaccggcttccagacccagcggttcgcccgaatgaatcagggactcaatcacgcggcggtgctggttaactttgatcggataaacaaggaagtaatcgccgttatagccgtaggattccctcgcacgtttgaacgcggcgttaatggaacgcaaacggtgctgcaggatctgtgggaaacagaacagtgcaggcagacgctggccctgtgcttcacgagttttcactaactgcgcgagatcgacgcgagcttccgggacgtccgggtccgggcacacgctaatgtggcccagctcgttaacgtcatagtagttattgccccaccaggcaatattgtaagtacgcagcatcttgctggcttcctgggagctcattgcaacctcctgcatggagcgtagtacaccgtgttcgcccgctgacgaaggcaaacccatagacatgtcgtcagacatagcgaacctcaaattattttattaagtgtaaaacagttaacgactatcgcagcctggaactgcgataacaacccataagcacatggattttccagcagtgaatgctgacgctccaactgcgcaaccggtttctttttcataacattattaagcacataaccgaacgtaagtgtgaaagttcggcgaaaccacgagaaaactcttgtttttacaagagcgcccttgttcagtcctcagtaactgtaaccagctcttgaatcctgagaagcgccgagatgggtataacatcggcaggtatgcaaagcagagatgcagagtgcggggaacgaatcttcaccagaacggtgagacaggttaagcagcagacaacggttcattatttcgtatcacctccacggccgcctgttaagacgaacccacaagccaaaactctgatttcaacccggctggaagtggcaacacgaaagaaacgtcgtgtgctttttatttaagccgcgcgccgcgttttataccccacaatggcagaaaattgcaaaagataaatacgcagaatgccggcattgtcaggaaaaatttccagccacgtttttaacagaatgagacacgattcaaaaaaaagtggaaatagggtgaagaattgacctaaaatagccatccagatgttaatccatccataccgattaacactcagactgccagtgtttttaacctgcagagtcgtggtaggatccgctaccacagaaaatccacacaacagtttgagctaaccaaattctctttaggtgatattaaatatggcaaaacacctttttacgtccgagtccgtctctgaagggcatcctgacaaaattgctgaccaaatttctgatgccgttttagacgcgatcctcgaacaggatccgaaagcacgcgttgcttgcgaaacctacgtaaaaaccggcatggttttagttggcggcgaaatcaccaccagcgcctgggtagacatcgaagagatcacccgtaacaccgttcgcgaaattggctatgtgcattccgacatgggctttgacgctaactcctgtgcggttctgagcgctatcggcaaacagtctcctgacatcaaccagggcgttgaccgtgccgatccgctggaacagggcgcgggtgaccagggtctgatgtttggctacgcaactaatgaaaccgacgtgctgatgccagcacctatcacctatgcacaccgtctggtacagcgtcaggctgaagtgcgtaaaaacggcactctgccgtggctgcgcccggacgcgaaaagccaggtgacttttcagtatgacgacggcaaaatcgttggtatcgatgctgtcgtgctttccactcagcactctgaagagatcgaccagaaatcgctgcaagaagcggtaatggaagagatcatcaagccaattctgcccgctgaatggctgacttctgccaccaaattcttcatcaacccgaccggtcgtttcgttatcggtggcccaatgggtgactgcggtctgactggtcgtaaaattatcgttgatacctacggcggcatggcgcgtcacggtggcggtgcattctctggtaaagatccatcaaaagtggaccgttccgcagcctacgcagcacgttatgtcgcgaaaaacatcgttgctgctggcctggccgatcgttgtgaaattcaggtttcctacgcaatcggcgtggctgaaccgacctccatcatggtagaaactttcggtactgagaaagtgccttctgaacaactgaccctgctggtacgtgagttcttcgacctgcgcccatacggtctgattcagatgctggatctgctgcacccgatctacaaagaaaccgcagcatacggtcactttggtcgtgaacatttcccgtgggaaaaaaccgacaaagcgcagctgctgcgcgatgctgccggtctgaagtaatctttcttcacctgcgttcaaaggccagcctcgcgctggcctttttcttttggataggcgttcacgccgcatccggcaaaaaaaccgcccgcacaataacatcattcttcctgatcacgtttcaccgcagattatcatcacaactgaaaccgattacaccaaccacaacagacaaagatttgtaatattttcatattattattcggttttcacagttgttacatttcttttcagtaaagtcttaattgcagataacagcgtttaatctatgatgatataactcaattattttcatgcacttaaatcataactaagataaatgttagtgtaagcgattacactgatgtgatttgcttcacatctttttacgtcgtactcacctatcttaattcacaataaaaaataaccatattggagggcatcatgcctgacgctaaaaaacaggggcggtcaaacaaggcaatgacgtttttcgtctgcttccttgccgctctggcgggattactctttggcctggatatcggtgtaattgctggcgcactgccgtttattgcagatgaattccagattacttcgcacacgcaagaatgggtcgtaagctccatgatgttcggtgcggcagtcggtgcggtgggcagcggctggctctcctttaaactcgggcgcaaaaagagcctgatgatcggcgcaattttgtttgttgccggttcgctgttctctgcggctgcgccaaacgttgaagtactgattctttcccgcgttctactggggctggcggtgggtgtggcctcttataccgcaccgctgtacctctctgaaattgcgccggaaaaaattcgtggcagtatgatctcgatgtatcagttgatgatcactatcgggatcctcggtgcttatctttctgataccgccttcagctacaccggtgcatggcgctggatgctgggtgtgattatcatcccggcaattttgctgctgattggtgtcttcttcctgccagacagcccacgttggtttgccgccaaacgccgttttgttgatgccgaacgcgtgctgctacgcctgcgtgacaccagcgcggaagcgaaacgcgaactggatgaaatccgtgaaagtttgcaggttaaacagagtggctgggcgctgtttaaagagaacagcaacttccgccgcgcggtgttccttggcgtactgttgcaggtaatgcagcaattcaccgggatgaacgtcatcatgtattacgcgccgaaaatcttcgaactggcgggttataccaacactaccgagcaaatgtgggggaccgtgattgtcggcctgaccaacgtacttgccacctttatcgcaatcggccttgttgaccgctggggacgtaaaccaacgctaacgctgggcttcctggtgatggctgctggcatgggcgtactcggtacaatgatgcatatcggtattcactctccgtcggcgcagtatttcgccatcgccatgctgctgatgtttattgtcggttttgccatgagtgccggtccgctgatttgggtactgtgctccgaaattcagccgctgaaaggccgcgattttggcatcacctgctccactgccaccaactggattgccaacatgatcgttggcgcaacgttcctgaccatgctcaacacgctgggtaacgccaacaccttctgggtgtatgcggctctgaacgtactgtttatcctgctgacattgtggctggtaccggaaaccaaacacgtttcgctggaacatattgaacgtaatctgatgaaaggtcgtaaactgcgcgaaataggcgctcacgattaatctccccaagcttcctcccatcgcggaggaagccacctcttgcagtcatcttttcttcgctctatcctctgccgctatgaaaacatcccgtctccctatcgccatccaacaggccgttatgcgtcgcctgcgggaaaaactcgcccaggccaacctgaagctagggcgtaactacccggagccaaaactctcttacacccagcgcggaacctccgccggaacggcctggctggaaagctatgaaattcgcctcaatcccgttttgctgttggaaaacagtgaagcttttattgaagaagtggtaccgcacgaactggcacatttgctggtatggaaacatttcggccgcgtagcgccacatggcaaagagtggaagtggatgatggaaaacgtgctgggtgttcccgcccgtcgtacgcatcagttcgaactgcaatccgtgcgtcgcaacaccttcccctaccgctgcaagtgccaggagcatcagcttaccgtacgccgccataatcgcgtagttcgtggcgaggccgtctatcgctgtgttcactgcggtgaacagctggttgcgaaataaccatctgaactatcaggaactttcctgatctggctgattgcataccaaaacagctttcgctacgttgctggctcgttttaacacggagtaagtgatgtaccgttatttgtctattgctgcggtggtactgagcgcagcattttccggcccggcgttggccgaaggtatcaatagtttttctcaggcgaaagccgcggcggtaaaagtccacgctgacgcgcccggtacgttttattgcggatgtaaaattaactggcagggcaaaaaaggcgttgttgatctgcaatcgtgcggctatcaggtgcgcaaaaatgaaaaccgcgccagccgcgtagagtgggaacatgtcgttcccgcctggcagttcggtcaccagcgccagtgctggcaggacggtggacgtaaaaactgcgctaaagatccggtctatcgcaagatggaaagcgatatgcataacctgcagccgtcagtcggtgaggtgaatggcgatcgcggcaactttatgtacagccagtggaatggcggtgaaggccagtacggtcaatgcgccatgaaggtcgatttcaaagaaaaagctgccgaaccaccagcgcgtgcacgcggtgccattgcgcgcacctacttctatatgcgcgaccaatacaacctgacactctctcgccagcaaacgcagctgttcaacgcatggaacaagatgtatccggttaccgactgggagtgcgagcgcgatgaacgcatcgcgaaggtgcagggcaatcataacccgtatgtgcaacgcgcttgccaggcgcgaaagagctaacctacactagcgggattctttttgttaacccctaccccacgcgtacaaccgcgtggggagacgacgcggatttttaactatgcgtatcccccgcatttatcatcctgaaccactgaccagccattctcacatcgcgctttgcgaagatgccgccaaccatatcgggcgcgtactgcgcatggggccggggcaggcgttgcaattgtttgacggtagcaaccaggtctttgacgccgaaattaccagcgccagcaaaaaaagcgtggaagtgaaggtgctggaaggccagatcgacgatcgcgaatctccgctgcatattcacctcggtcaggtgatgtcgcgtggtgaaaaaatggaatttactatccagaaatcgatcgaactcggtgtaagcctcattacgccacttttttctgagcgctgcggcgttaaactggatagtgaacgtctgaacaagaagcttcagcagtggcagaagattgcaattgctgcctgtgagcagtgtggtcgtaaccgggtgccggaaatccgtccagcgatggatctggaagcctggtgtgcagagcaggatgaaggactgaaactgaatcttcacccgcgcgccagtaacagcatcaatacgttgccgttaccggttgaacgcgtccgcctgctgattggcccggaaggcggtttatcggcagatgaaattgccatgactgcccgctatcaatttactgatatcctgttgggacctcgcgttttgcgtacagagacaactgcgctcaccgccattaccgcgctacaagtacgatttggcgatttgggctaacggagaagaataatgatcaagctcggcatcgtgatggaccccatcgcaaacatcaacatcaagaaagattccagttttgctatgttgctggaagcacagcgtcgtggttacgaacttcactatatggagatgggcgatctgtatctgatcaatggtgaagcccgcgcccatacccgcacgctgaacgtgaagcagaactacgaagagtggttttcgttcgtcggtgaacaggatctgccgctggccgatctcgatgtgatcctgatgcgtaaagacccgccgtttgataccgagtttatctacgcgacctatattctggaacgtgccgaagagaaagggacgctgatcgttaacaagccgcagagcctgcgcgactgtaacgagaaactgtttaccgcctggttctctgacttaacgccagaaacgctggttacgcgcaataaagcgcagctaaaagcgttctgggagaaacacagcgacatcattcttaagccgctggacggtatgggcggcgcgtcgattttccgcgtgaaagaaggcgatccaaacctcggcgtgattgccgaaaccctgactgagcatggcactcgctactgcatggcgcaaaattacctgccagccattaaagatggcgacaaacgcgtgctggtggtggatggcgagccggtaccgtactgcctggcgcgtattccgcaggggggcgaaacccgtggcaatctggctgccggtggtcgcggtgaacctcgtccgctgacggaaagtgactggaaaatcgcccgtcagatcgggccgacgctgaaagaaaaagggctgatttttgttggtctggatatcatcggcgaccgtctgactgaaattaacgtcaccagcccaacctgtattcgtgagattgaagcagagtttccggtgtcgatcaccggaatgttaatggatgccatcgaagcacgtttacagcagcagtaacccaccttagcgagaaggatctcgttgagactctgagtgacagcgcccttctttccacgcatactgggcgctgttgcttttttgaaccaggaaacagaacctctgacaatgaatttacagcatcactttcttattgccatgcctgctctccaggatccgattttccgtcgttccgtggtctacatttgcgaacataataccaatggtgcaatggggatcatcgtcaacaagccgctggaaaatctcaaaattgaagggattctggaaaagctgaagatcacgccggagccgcgtgatgaatcaatccgtctggataaaccggttatgctcggcggtccgctggctgaagatcgcgggtttattttgcatactccgccctccaattttgcttccagcattcgcatttcagacaacacggtaatgaccacttcccgcgatgtgctggaaacgctcggcaccgataaacaaccgtctgacgtattggtggctctgggttatgcctcctgggagaaaggtcaactggaacaagaaattctcgataacgcgtggctaacggccccggcagatctgaatattctgttcaaaacgccgattgccgaccgctggcgcgaggcggcaaaactgattggtgtggatattctcaccatgcctggtgtggcaggacacgcctgatgagtggaaccttactcgccttcgacttcggcaccaaaagcattggcgtagcggtcggccaacgcattaccggcaccgctcgccctttgcctgcaattaaagcacaggacggtacgccggactggaacattatcgagcgtttactgaaagagtggcagccggacgaaatcatcgtcggtttgccgctgaatatggacggcaccgagcaaccattgactgccagagcgcgtaaatttgccaaccgtattcatggccgtttcggtgttgaagtaaagctccatgacgagcgtcttagcactgtggaagcccgttccggtctgtttgaacagggcggctatcgggcgctcaacaaaggcaaagttgactctgcctctgcggttattattctcgaaagctatttcgagcagggatattaaggcgatttaaacgcctggcggagtgtaaataatatcatcgcgtcttattgccggatgcggcgtgaacaccttatccagcacacatctggcagcggctataggtctgataagacgcgttagcgtcgcatcagacatttattgcctttgtaggcccgataagcttgcgcatcgggcatggcaacgtcacaaacgcccttcccccacccggtgctgataactctgctgaaacgttatcatccccacctgctgcccggtttgaataacatgcggtaactggtgggttttcccttcgcgaatcaaattccccaccgcgggtgtgttaatcagcaattcaaatagcgccacgcgtccttcctgtttatccacttccagcttttgtgacagcactgcccgtaaactacctgccagttgattacgcacggggtctttttcctgcgccggaaatgaatccaccagtcgctcaactgcctgcgcggcaccacgcgtatgtaatgttgccagcaccaaatgcccggtttctgccgccgtcagtgccagacggattgtctcgctgtcacgcagctctccgagcaaaatcacatcaggatcttcccgcaatgcggcccgcaatcccgatgcgaacgtcatacagtgcaaaccaatttcccgctgctggatcaaacatcgctggctggcatagagatattcaacaggatcttccagcgtcagaatatgcgcatcggcatgttgattgagatagccaaccatcgccgccagcgtggtagatttgccactccccgtcgcccccgtcaccagaatcaggccattctcgctcttgagtaattccggcaataccgttggtgcgccaagctgttcgagctgcgggcagtgcgaaggtaacagccgtaacgccagcgaaatgccatgccgttgcgcgaatgcgctgccacgcaatcgctggttttccgccagcgacacggcaaaatccagctgaccattctccagcaatattgcccgctgatcgtcatccagccactcccgcagtagctcttcgacgtccggcgtatcaaacggcgcagcttccattctgccgcgaatgcgccatcgtgcgggccaggcgctgcacaggtgtagatccgagacgttatgctttacactaagggccacaatttcttccatattcatactaagatcctcggaaaatgaacgatattgcgcataacctggcacaggtccgggacaaaatctcagcggctgcaacgcgttgcggccgttctccagaagaaattacgctgcttgcagtcagtaaaacaaaacctgcgagcgccatcgcagaagccattgatgccgggcagcgtcaatttggtgaaaactacgttcaggaaggggtagataaaattcgccactttcaggaactgggcgtaacaggattagaatggcattttattggcccgttgcagtctaataaaagccgcctggtggcagagcatttcgactggtgtcataccatcgaccgtttgcgcatcgctacccgtctcaacgaccagcgcccggcagaacttccccctcttaacgttctgattcaaattaacattagtgatgaaaacagtaagtccgggattcaactggctgaactggacgagctggcagctgcggtcgctgaactaccgcgtttacgtctgcgcgggttgatggcaatccctgcgcctgagtcagaatatgtaaggcagtttgaagttgcacgccaaatggctgtagcatttgccggactgaaaacgcgctacccgcatatcgacacgctctctctgggaatgtcggacgatatggaagccgccattgcggcaggtagcacgatggttcgtatcggcactgcaatttttggtgcgcgtgattactctaaaaaataaggaattaaaggaacgccatgaatacgttgactttcctgctttcaacggtcattgagctgtataccatggtgctgttattacgcatctggatgcagtgggctcattgtgatttttacaaccccttctcacagtttgtagtgaaggtaacgcagccaattatcgggccactgcgccgcgttattccggcaatggggccaattgacagcgcctcgctgctggttgcctatattctcagttttatcaaagccatcgtgctgtttaaagtggtgaccttcctgccaatcatctggattgccggtttactgattctgctgaaaaccatcggcctgctgattttctgggtcctgctggtgatggcgattatgagctgggtaagccaggggcgtagcccgattgaatacgtgctgattcagctggccgatccgctgctgcgcccgattcgccgcctgctaccggcaatgggtgggattgatttctcgccgatgatcctcgttctgctgctgtatgtcatcaatatgggtgtcgcagaagtattacaggcaaccggaaatatgctgctgccagggctgtggatggcgttatgaatgccgtaacagttaatgatgacggtctggttttacggctctatattcagccgaaagccagccgtgattctattgtcggtttacatggcgacgaagttaaagtcgccattaccgcgccgccggttgacggccaggccaacagtcatctggtgaagtttctcggtaagcaattccgggttgccaaaagccaggtggtgattgaaaaaggcgaacttggccgccacaaacaaattaaaatcattaatccgcaacaaatcccgccagaaatcgcggcgttaattaattaggtatcctatgcaaaaagttgtcctcgcaaccggcaatgtcggtaaagtgcgtgagctggcgtcgctgcttagcgacttcggtcttgatatcgtggcccaaacagacctcggcgttgattccgctgaagaaaccggcctgacctttatcgaaaacgcgattctgaaagcgcgccatgcggcaaaagtgaccgctttaccggcaattgccgacgactctggtctggcggtagatgtgcttggcggcgcgccgggcatttactccgcgcgttattccggtgaagacgcgaccgatcaaaagaatctgcaaaaactgctggaaacaatgaaagacgtaccggacgaccaacgtcaggcgcgtttccactgcgtgctggtatatctgcgtcacgcggaagatcccactccgctggtatgccacggtagctggccgggcgtgattactcgtgaaccagcgggcactggtggctttggttatgatccaatcttcttcgtaccttccgaagggaaaaccgccgccgaactgacccgcgaagaaaagagcgccatttcccaccgtggtcaggcgttgaaactgctgctggacgctttacgtaatggttaaattacctccgctgagtctctacattcacatcccgtggtgcgtgcagaaatgcccgtactgcgatttcaactctcacgcgttgaaaggagaagtgccgcacgacgattatgttcagcatctgcttaacgatctggacaacgatgtggcttacgctcagggccgtgaagtaaagacaatctttattggcggtggtacgccgagcctgctttccggcccggcgatgcaaacgctgctggacggcgtgcgtgcgcgtttgccgctggcagcggatgcagaaattactatggaagcgaaccctggcacggtagaagccgatcgctttgtcgattatcagcgtgctggtgtgaaccgcatctctattggtgtgcagagttttagcgaagaaaagctgaaacgacttgggcgtattcatggcccgcaagaagcgaaacgcgcggcgaagctggcgagcggtttagggttacgtagctttaaccttgatttgatgcatgggctgccggatcaatcactggaagaggcgcttggcgatctacgccaggccattgaactgaatccgccgcatctttcctggtatcaactgaccatcgaacccaatacgctgtttggttcgcgaccaccggtgctgccggacgatgacgcgttgtgggatatattcgaacaggggcatcagttattaaccgcagcgggttatcagcaatatgaaacttccgcttacgccaaacccggttatcagtgccagcacaatctcaactactggcgctttggtgactacatcggtattggctgcggcgcacacggcaaagtgaccttcccggatgggcgcattctgcgtaccaccaaaacgcgtcatccgcgtggttttatgcaaggaaggtatctggaaagccagcgtgatgtcgaagccacagataagccgtttgagttctttatgaatcgcttccgtctgctggaggccgcgccgcgcgtggagtttattgcgtataccgggctttgcgaagatgtgattcgcccacagttagacgaggcgattgcccagggttatctcaccgaatgtgcggattactggcagataacggaacatgggaagctgtttttaaattcgctgctggagctttttctggctgagtaaacttgtattgccggatgcggcgtgaacgccttatccagccgacatgtggcagcggttgtaggtctgataagacgcgcaagcgtcgcatcagacgttgattgccggatgcggggtcaacgccgcatcctgctacaaatcgtgcactatatcaaacttacttaatcaccccattgcgccgcagttgttcggtatcttttttccagcgttcattagcttggttgatatcgtcaattttcatcaaaatcgcgacttttttactgtttatttctgaaactttcatcgttaacggatattgccctttttcgagcgttacccagtcatcctgcaatttacggctaagtttttgtgattgcagaaaagtctgtcgccgttgttcgttgatatcgaaatctcgtttctgctgaatcggcacttcataacactcttcactctgtttatgacatgccgcaatcgccggttgataaacctctttgtcatatttaaccgcgaacgcctcgctatcgttctgtttattaaactcatcacgctgttggtgaatttttttaaaggcgtcttcgcgggtcatttgcttaccgtttgcatcttttccccaatatgcatccgctgctttctgcgccgccaccatttgcttatcaagcgctttcacttccttttccagcgcaggaatcgagttcttctgggtattcaacgcagattcaagctgactaaagcgataattgaaatcttcgctattcacgatcagatatttattattcgttttgatatcgtcgaccacccgcccacgatcgctggctgccgcctgaaaagagtaaaagttcaccgaccagccagacgcgggcgttcctttactggttaacatcgccgagaattttaccggtttatctttcgtccaggtctgttcgagcagttcgtaatctgccaactgaccgacccaggtatagagatcgtcactggaagagacatcgccttccgctgaccaggtggcctgattacccttagcatcaagattttttaaggtgatagcatcaagcttgagaatgccgtgatactgctttttgaattgatcttttaagatattttcagttggcggttcgccatctgcccaggcattaccagtcatcaacataagcagtgccgtgccaacaatccattgctttttcacccgaaaaacctcacgcggaataatttattccggtgattatcattagggtaattaaaattggcaatggacgtgagtctgaagtgaaaaagccccggcacgataccggggcgaggcgattagtactgattgaagatctgctggatctgctgcggatctttggtttgcgtcagagccagttgcagcagaacgcgcgctttttgcgggttcagcgtgccagaggcgacgaagccgtatttcgcatcatccacttcggcatcctgagtggtagcgcccgtcggtacgcgggaagaacgcacgactgcagtaccggttttcgcggcggtcgccagcgtgtcgaacacagatttatacaggttgccgttacccacaccagcgctaacgatgccatcatagcccgcatctaccagtgctttagccggaagatcggatgcgttagcgtagttataaacaatgccgactttcggcagttcattcagcttagagacatcgaatggcgtgtcgctggtatgcttacgtgccggggtacgctggtagtcaatcttaccgttgtgaatgtaacccagaggaccgtagttaacagacttgaaggtcgctacgtcggtggtgttggttttggtgacgtcacggccatcaagcacggtgtcattcatcactaccagcacgccacggttggcggaggctttatcagctgcggtcactaccgcgttatacaggttgaatggaccgtctgcgctcatagacgtggacggacgcattgcgccgaccatcaccaccggtttgtcgcatttcaccgtcaggtcgaggaagtaagcagtttcttccatcgtgtcggtaccgtgggtaatgacgaagccgtcggtcttatcgcagtcggtgttaatttttttcgccagtgtcagccagacattatcgttcatgtcctgggagccgatattcactacctgctcgcctttaacgttcgcaatgtcttttagttgcggcaccgcattaaccagattttctacgccaactttacccactgtgtagttagatttggttgcggagtcaccaccaccggcaatggtcccgccggttgctaaaatggtgatattgggtaatgccaatgctgcaccactaaaacccataaccagtgcggcaagtgccgtctttttgaaaaactccatttcattcctccagttacgtgaacgctacgcattatcccttagctctgtatgggaaatttgacgttaaacaatttacaacgtgaatatattttggagatctacaaagttagaggcaggtaacaaaacgaagaattaaacggcataaaaaagtattatgccgtcttaaaatagaggattattttaaattcccgaccagggctttgcggctatcttccagagtcacaacgcggctacaaacatctttgccaaactgctggaaatctttttcctgctttttccactcggtttggattgaggattgcagcccccccaggcttcccagcacattctgtaatgggttaccgccgcttttcagcaccgctttcgcgcccatttcattaatgctgtcctgtaaaattccacccattgcctgattcactaattgctggccttcggcgcgaacctgatcaatggctttatagtgaaacgtcaggccatcgctgcgcgtttcaataatgcggttcatctgctctttcagctgcgcatcaagtttggtcagacggctgcgcattttgctgctttcgcccatctcctgaacgataattttatccagagcaatacgggctttctcgacgcggcttttcgcgccttcatcaatccacggcagcgtgctgcgtagttcagcctgataatccttcgcctgctcgcgctgggcggcattcagggaatattgcttaccgttatacatcacgttgccgtctggcgtgatcaccagattgccgttttcgcccttcacctgcacggtttgcgggctgacaatcacatcgtcacgcggcgtgacgctgcactggtagtcggcgtgagcggtcattgccgtcactgaaagtgctgccgccagcagcattttgcgcatcatagtcttccctcaagaaaaaatcaggccagcatttgctggccccagattgataacaaagtacgcgttttccatgccggatgcggcgtaaacaccttatcccgcctactcgatcgtgcatctttccaggcctgataagcgtagcgcatcaggcagttttgcatttgtcatcgcccgtatgctttcttagtcccaccaaacgtcgaaaagttcgctggtgcgtacctcatccagtttgcgctcttccagccacttacgcacaatcgcctgatgttcttcggtgcatttgccgatttcctgcatgcagatcagaccttcccaggccagataaccgctgccgtcaaaggccagtttgttcggttcgataacctcgttaataaaatcatcaacggttttatcaatctgttcttccgatgtaccttccgggaatcgccatgccaccgaaaatcctaattcctggaattcgtcgatgtgcatttttttacgcagacgacggctacggttctttgccattatttcaccctctcgaacattaagtcccatactccgtgaccaagacgatgaccacgttgttcaaatttcgtcaccggacgtgatgccggacgcggtacgtaatcattgctctctgacaggtttttataaccgtcaatagaagacatcacttcaagcatatgttccgcataaggttcccagtcggtcgccatatggaatacgccccccagctgcagtttgctttttaccagttcggcaaacggcacctgaacgatacggcgtttattatggcgcgctttgtgccacgggtcagggaaaaagagctgcaccatgcgcaatgaattgtcaggaatcattttatgcagcacttcaaccgcatcgtgacacatcacgcgcaggttgcttaaaccttcttcatgcgcagaagccaggcacgcaccaacgcccggtgaatgcacttcaatgccgaggaagtcctgctcagggcgatctttagccattgccaccagcgacgcccccatgccaaaaccaatctcaagcgtcaccggcgcttcacggccaaaaagcgcggggaaatccagcatatcttcgctgaactcaacgcccatcaccggccagtagttttccagcgcatgttcctggcctttggtcagtcgcccctggcggcgcacaaaactacggatacggcgcagtgggcggccgttttcatcaaattccggtgaaatgacgtcgtttttcataaaggtttagtcgcttgtgaaagtgttctgaaaacgggcattatccaaagttagttgccggatgcaagcatgataaggccgtggctgcggaaagttccggtttacaccctgccgtcgctgtgctgcaatcttgcccccaacaacagtgaattcggtgaccatgcaagcgtcgcaattttcagcccaggttctggactggtacgataaatacgggcgaaaaactctgccctggcaaattgacaagacgccctacaaagtatggctctcagaagtgatgttgcaacaaactcaggttgcgaccgttatcccctattttgaacgctttatggcgcgcttcccgacggtgaccgatctcgccaatgcgccgctcgacgaagttctccacttgtggaccgggcttggctattacgcccgcgcgcgcaatctgcataaagcggcacaacaagtggcgaccttacacggcggtaaattcccggaaacctttgaggaagttgcagcactgccgggcgtcgggcgttccaccgcaggcgcgattctctcgctttctctgggtaagcactttccgattctcgacggtaacgtcaaacgcgtgctggcgcgctgctatgctgtaagcggctggcctgggaaaaaagaggtcgagaataaattatggagtttgagcgagcaggtgacgcccgcggttggcgtggaacggtttaatcaggcgatgatggatttgggtgcgatgatttgtacgcgctcgaaaccgaaatgttcgctctgtccgctacaaaacggatgtattgccgccgccaacaatagctgggcgctttatccgggcaaaaaaccgaaacagacgctgccggagcgcaccggctactttttgctattacagcacgaagatgaagtattgctggcgcagcgtccgccgagcggattgtggggcggtttatactgtttcccgcagtttgccgacgaagaaagtttgcggcagtggctggcgcaacggcagattgctgccgataacctgacgcaactgaccgcgtttcggcataccttcagccatttccacttagatattgtgcctatgtggcttcccgtgtcgtcattcaccggctgcatggatgaaggcaatgcgctctggtataacttagcgcaaccgccgtcagttggcctagcggctcccgtggagcgtttgttacagcagttacgcactggcgcgccggtttagcgcgtgagtcgataaagaggatgatttatgagcagaacgattttttgtactttcctgcaacgtgaagcagaaggtcaggattttcagctgtaccccggcgagctgggaaaacgcatctataacgagatctccaaagaagcctgggcgcagtggcagcacaagcaaaccatgctgattaatgaaaagaaactcaacatgatgaatgccgagcaccgcaagctgcttgagcaggagatggtcaacttcctgttcgagggtaaagaggtgcatatcgagggctatacgccggaagataaaaaataaaaacagtgccggagcacgcctccggcaacttgcataaaaacaaacacaacacgcacccggaatgatgaaaaaatatctcgcgctggctttgattgcgccgttgctcatctcctgttcgacgaccaaaaaaggcgatacctataacgaagcctgggtcaaagataccaacggttttgatattctgatggggcaatttgcccacaatattgagaacatctggggcttcaaagaggtggtgatcgctggtcctaaggactacgtgaaatacaccgatcaatatcagacccgcagccacatcaacttcgatgacggtacgattactatcgaaaccatcgccgggacagaacctgccgcgcatttgcgccgggcaattatcaaaacgttattgatgggtgacgatccgagttcggtcgatctctattccgacgttgatgatattacgatttcgaaagaacctttcctttacggtcaggtggtggacaacaccgggcagccgattcgctgggaaggtcgcgcaagcaacttcgcggattatctgctgaaaaaccgtctgaagagccgcagcaacgggctgcgtatcatctacagcgtcaccattaacatggtgccgaaccaccttgataaacgtgcgcacaaatatctcggcatggtccgccaggcgtcacggaaatatggcgttgatgagtcgctgattctggcaattatgcagaccgaatcttcctttaacccgtatgcggtcagccgttccgatgcgctgggattaatgcaggtggtacaacatactgccgggaaagatgtgttccgctcgcaggggaaatccggcacgccgagccgcagtttcttgtttgatcctgccagcaatattgataccggcaccgcgtatctggcgatgctgaacaatgtttatctcggcggaattgataacccaacatcgcggcgttatgccgtcatcaccgcctataacggcggcgcaggcagcgtgctgcgagtcttttcgaatgataagattcaggctgccaatattattaacaccatgacgccgggcgatgtttatcagacgctgacgacccgccatccctctgcggaatctcgccgttatctttataaagtgaataccgcgcaaaaatcctaccgccgccgataattccattaaccgcccctgacgatgctcaggggcaaaaatgttatccacatcacaatttcgttttgcaaattgggaatgtttgcaattatttgccacaggtaacaaaaaaccagtccgcgaagttgatagaatcccatcatctcgcacggtcaaatgtgctttttcaaacactcatccgcatcacgatgtgaggaaattaacatgaatcttaagctgcagctgaaaatcctctcttttctgcagttctgtctgtggggaagttggctgacgaccctcggctcctatatgtttgttaccctgaagtttgacggtgcttctattggcgcagtttatagctcactgggtatcgcagcggtctttatgcctgcgctgctggggattgtggccgacaaatggttaagtgcgaaatgggtatatgccatttgccacaccattggcgctatcacgctgttcatggcggcacaggtcacgacaccggaagcgatgttccttgtgatattgattaactcgtttgcttatatgccaacgcttgggttaatcaacaccatctcttactatcgcctgcaaaatgccgggatggatatcgttactgacttcccgccaatccgtatctggggcaccatcggctttatcatggcaatgtgggtggtgagcctgtctggcttcgaattaagccacatgcagctgtatattggcgcagcactttccgccattctggttctgtttaccctgactctgccgcatattccggttgctaaacagcaagcgaatcagagctggacaaccctgctgggcctcgatgcattcgcgctgtttaaaaacaagcgtatggcaatcttctttatcttctcaatgctgctgggcgcggaactgcagattaccaacatgttcggtaataccttcctgcacagcttcgacaaagatccgatgtttgccagcagctttattgtgcagcatgcgtcaatcatcatgtcgatttcgcagatctctgaaaccctgttcattctgaccatcccgttcttcttaagccgctacggtattaagaacgtaatgatgatcagtattgtggcgtggatcctgcgttttgcgctgtttgcttacggcgacccgactccgttcggtactgtactgctggtactgtcgatgatcgtttacggttgcgcattcgacttcttcaacatctctggttcggtgtttgtcgaaaaagaagttagcccggcaattcgcgccagtgcacaagggatgttcctgatgatgactaacggcttcggctgtatcctcggcggcatcgtgagcggtaaagttgttgagatgtacacccaaaacggcattaccgactggcagaccgtatggttgattttcgctggttactccgtggttctggccttcgcgttcatggcgatgttcaaatataaacacgttcgtgtcccgacaggcacacagacggttagccactaattacgcaaagaaaaacgggtcgccagaaggtgacccgttttttttattcttacttcaacacataaccgtacaaccgtttcacgccatccgcatcggtttcgctataaacaccttgcagctccggcgaaaatcccggcaacaaattcaccccttcttccagtgcaaggaaataacgttgaaccgccccaccccagacttccccgggtaccacgcaaagcacgccaggtggataaggcaacgccccttctgccgcaattcgcccttcggcatcacgaatccgcaccaactccacgtcaccgcgaatataagcgctatgcgcatcctgggggttcatcaccactgacgggaaactctgctggcggaacatcgctttttgtaggtctttgacgtcgaaactgacatacagatcgtgcatctcctgacacaactggcgcagggtgtagtcgcgatagcgcaccggatacttgttataaacgctcggcaacacctcaaccagcggcgagtcatcctcaatatgctgttcaaattgcgccagcatcgccaccagttgtgccagcttctcgtggctttccgccggagttaataaaaacagaatggagttgagatcgcacttctccggcacaatgccgttctcacgcagatagtgcgccagaatcgtcgccggaacgccaaagtcgctatattcgccggtttcggcatcgatacctggtgtagtgagtaacagcttgcacggatcaacaaaatactgatccgcggcatatccttcaaagccgtgccacttcgcccccggctcaaaactgaaaaaacggcggtcgctggctaacactgatgtcggataatcctgccacaatttgccatcaacaacgggcgggataaacgggcggaacagcttacagcgcgcaagaatagccttgcgcgcttcaatccctatctcaacacactcagcccacagccgacgcccactctccccttcatgaattttggcgttaacatccagtgcagcaaacagcggatagaaagggctggtagaagcatggagcataaaggcgttattcaaccgcttatgcgggcaaaaacgcgcctgtccgcggatatggttatcttttttatggatctgcgacgtctgtgagaatcccgcctgctgtttgtgcaccgactgagtcacaaagatccccggatcgttttcgttaagttctaacagcagcggcgagctatccgccatcatcgggataaattgttcataaccgacccacgcggaatcaaacagaatgtaatcacacagatgcccaacggtatcgatcacctgacgggcgttatagacagtgccgtcataggttcccagctgaataatcgccaggcgatacgggcgcggcaggtcggctttttctggcgcaacgtcgcgaatttgctggcgcagatactcttcattaaaacagtgcgcatcaataccgccaatgaaaccaaacgggttgcgtgaagcttccagatagaccggcgtcgcccccgcctgaatcagcgcgccgtgatgattcgacttatggttgttacggtcgaagagcaccagatcgccacgcgttaacagcgcattcgtcaccactttattcgctgccgatgtgccgttcagcacaaaataggttttatcggcatgaaagactttggctgcgaatttctgcgcatctttcgccgatccttcatgaataagcagatcgcccaattttacgtcagcgttacacatatcggcgcgaaagacgttctcaccaaagaaatcgtaaaaatggcgtccggcaggatgctttttaaaaaacgcaccatgttgatgtccagggcaagcaaaggtgctgttgcccatctcaacgtactgcgtcagcgtgtcataaaacggtggcagcaaattctcttcatactgacaggctgcggattccagctccagccactgctgctcgttgccgttgattaccgccgtaacgcccgcaggtaattcaacagcatgttcggaatacaaaaacaccggtagatgaaaaccggtgcgcttaagcaacgcaagaatgccactgcgactatccgcagcggtaatgacgactgccgcgacgtccgtaaaatcagtatctcccaacgccaccacgcgacgatgagaagaaagtcgggataccagttcactactggcggcaatattcattgatttcataagcgcaaacccgtttcggggaagtaagaataccggacaaggtggaaaaccctgccccatgagatatgggtcaaactggtcaccagctccgaccgccagacatcagtaaaagcagaaacgctctgattttactgttgtcctgcagtgagcgtgcgttaacttcaccgcatgagcagtaacatagaaagggaaacgtttcgcgcgaaacggcgataagcgagagaatgtaaggagatggcgtgcatcgggcaaactccgtacagagaggagaaaattcgcgcaatcatggcacctttcgctaaagcgtgcaagccaggactttgcgaacaaacaagccatcgacggcaccaaacggtcataataagaaaatcaaacaatacagctaacaggaactcttgtggtcatcggcccttttatcaacgctagtgcagtcttactgggtggcgttctcggcgcactgctcagccaacgcttaccggaacgtatccgcgtctccatgacatcaatttttggtctggcatcgctggggattggtattttactggtggtgaaatgtgccaaccttccagcgatggttttagctacgctacttggcgctctaattggcgaaatttgtttgctggagaaaggtgtcaatacagcagtcgccaaagcacaaaatctgtttcgtcactcacgtaagaagccagcgcatgaatcttttattcagaattatgtcgcgattattgtcctgttttgcgccagcggcaccgggatcttcggggcgatgaacgaagggatgaccggcgatccgagtattttaatcgccaagtcatttcttgatttctttacggcgatgatcttcgcctgctcgctgggtattgcggtatcggtgattagtatcccattactgatcatccagttaacgctggcgtgggctgccgcgctgattttaccgctgaccacaccgtcgatgatggcagacttcagcgccgtaggcggtttattgctgctggcaaccggattacgcatctgtggcattaaaatgttcccggtggtcaacatgcttccagcactccttctggcaatgccgctttccgccgcctggaccgcctggtttgcctgacaatgcgtgcaatatcggcaaagtgatgatagattgtgcagtctgcagtaaattgaagaaatttgattgacgagacgaggcgaatcaggtttaatgcgccccgttgcccggatagctcagtcggtagagcaggggattgaaaatccccgtgtccttggttcgattccgagtccgggcaccactaattcttaagaacccgcccacaaggcgggtttttgcttttggatctgacaataaccttcacgaaaaaaattagcttataaagtctgggggaattactctcgccacgttaacgagagtaattttattgatattaatctcctgatactttacccccgtccaaactccagccgctgcacattcaccatcccaggcttctcagcagcactgacatcaatttgtgtcacccgcagcgcatatttttcatccagtgcgtttaaccatttcagcaggtcattaaacaccacaggttctatccagacctgaatattctccccacgatcggctatccgcctgatgaccaccgagtgcgcggaagcactgtcactgatgacccgcgatacctgcgcaggcgttgttgtggcagattttcgcgctgcaataatatccggcgcggcgttcttcagtcgggtgttcatcgccaccagctgctgcaatattgtctcctgttgctcaatccgttcgctcaacggctgccagatgaggacgtaatatccgacgctaaacaggaacaccaccgctgccagtaacatgcccttttcacgcggagaacgccccgccaggtgttgtgccagccagtgttcgccacggcttaactggcgttcacgccattgctgaaaatagtgaataaatttatcgcgtaacatgttatttcctccgcaacgttacgccgccggaaaccgcatcaccctctttctgtaacgcgtcctgttgcacaacataatcggttgccagtacactacgcagtttgtcgaaactggcaaagttcgcggcccgtagctggaggtgaagtatctggcgtttttgatcaaaggtaaaaccacgcatttcgatgtcggaaagtgacgctgatttcagggtgctggctatcgctgacaactcggcgagcagccgggtatcgtcggcctgtgggcgatattttttcagcgccatcgtcacctgagagcgtaaattcacaatccgcttctgctccgggaacaacgttaagaactgttcctccgcctgggtgcggctttgcgccacctgttcgctgacgctccataacgtcacgccccgctccactgccagcgcaaccagaatcagcaatatcggcagaatcatcacccgccagcgcgcccactgttttcggtagctgacgcgaggctgccacggccctgtcagcaggttcccttccggttcgccataagtggtaatggcgggcagagctgtaacggtcaggcgttcagcgtctgcgccagcccatgctgatagcttttccggtgcaatgccgactacggttagcgaaagcggtaaatcctgctcattgagctgggcgcggaacatgaccggagccagcgccagcccggcgctccatccccggcattcatcgatgcggcagataacccgttgcgcatcgcaagccataaacccacaaggaatggacatccagtccggcgcgacggtagcgcgggtgatgccgttttcctgcaaccactgcgcaatgttgcgcatatgctgttggtgaatcactgctacggttgccagttgctggtcgatattcaacggggcgaaatgcagttcatcgatatcctggttcagctcttcttccagtaaggcgggcagaatagtcggtagcgcagcgcgatggaaatgtcgtggcgcgcacccttgcgtaaaaccgtaagttgaatggaatccattgaaggtaactgccgcatcagagcaatcattgctcgtggatcagtgaaatcctgctgatttagcgcaatggcgatatcgccttccttgaaaccgctggcatcgaacagagaacgatctgcccccggcttcgctgcataaccgacaatcccctccttacgcacaggcgtaagctggatatagttaaaaattttctgcggatctttcgccagtgcctgacgcacggcagccgggatctcaactggcacactgacagcaggctcagcaacagcttgctttgcttcgtcactgacggcttttttgttggtcacagcaacagtggaacgttcctcttctgccagactcagacgctctatttttccctgataacgcagcatcacatggtcgcggttgatttcctcaatcaccgcgttgtgagagccaagcgtttcaccctgcaaatagacctgctgtttaccgccttcttcaataaccgcgccgggtctggcaccaaaggcgatcccacgcagcaccacattaagacgcgtttctgccacaggcacaggttcgggttgttttacctgcgcggcgacaggctgatatttgccaaaccagttttgctggctgattaattgcacgtcatttttatcgaacgtttttgcatccacacggctcggtttattcaccggttgagaaaccgccgtatattccgcagaaaaggagatatagcgccagagtgaatgcgccatttttgcagaaataataagcagcatcagccagaacatcccgcgtgcaatttttcgcagatgctctttgtctgtattaagagattgtctctggttaagagtgtgacgaatttttgtcagccattgaatgagataaattcgtgcgtcacgaaaaacaacccgcgccaatttatatctacccgacgttatgctttgactattccacaggtggtacgatccagtttccgctgatactggttacctgtacgtgtatcattaatcgttatgctgtaattaattccctcagtgatcattaatttcaccgtcgggtcagcgcacatttgtcgttgatagctggttaaaaaggcgtcaggcgtctgcgtggtttgtgtacccgcttcgctgataatggtcatttttaccgttgtgccgctactttgcgccagcactaaggtatatcccgcagatttaatcggcaggttttggctgatattttgcgcctgttttttcgccagtaaactggcattttcattatggctggcacagccacttaataatcctgtaacgctcaacaatagcgatattaataccctccctggcatttgttttatcgacatggtaaataatctctaaggttattaataagagttaaaatgtcactttgataatgacgtggttatcattaaaacaatgcctgtagataaagtgttgctataccgcccagacttaaacacggtccaaaaggcagtgtggttgatcctctttttgtaataacggcatatatcaggccgcagcatgaggcgattaaagcaacattgggcagcgacaatgcccccacccagccacctaacgcggcgaaaagtaatacatcgcccatgcctaatgcttctttacgcagaactattccggctatccaacgcagagagtaaaaagtgataaatcccaccaggacgccggtgactgcatcttgtagcgtgagcggactctgctgcgcccatgccgcaatcagtcctgtccacaatacgccctgagtaaaaacatcgggcagccattggtgatcgaggtcgatgacactcgcggcaatcagccaggcggataatatcatcaccgccagcccccatccactttctggccagaccagactcgccagcaaaaaagcaagtgctgtcaataactccaccagcggataacgcttgctgattttcgcctgacagtcgcggcagcgccctttgagcatcagccaggagaacagcggaatattgtcacgtatccggatggtctgctgacaatgtgggcagtgcgaacgcggtagcgcaaggcttatttttgactgcgcactcgacatttcaccgtgaaactccgccatttgttggcgcagcatgattgggtaacgccaaatcaccacattcaaaaaactgccgatgatcaatcctccgacggttgccaggacgggcatcgccgtggggtattgctgaaaaacatcaaaaagcatggttaaaggttgtttgttgtaacttgctggatgcggcgtaaaacgccttatccgtcctacgggtgtctgccagcgcaaataatcgcggctttccccgtctgtaggcccgataagcaggcgcatcgggcaaatgtgttaacccggtgcgccttatttcatgccggatgcggcgcgagcgccttatccggcctacgggcttactcggcagacatcttatgctcggtaacctgattaatggtttccggtccctgttccggtttcggcagatcgagtgacgcgagcgtgttgtaagccgactggctcacaccgccctcgaagctcatctcgctcgcccccggcagctggtaagcattcgcgcccggattccatttcttaaagaactccgaaagatccgtctgggcgacccaggaggcacacagcatcagcgtgtccgctgcgttaccgttggattcagcacagtaattcttgccgccaaacttgtcattgctgacctcatcgccgcgtgctttacgatgcatcaactggaacaggttccagcctttcatcccttcacgctcgctgtaaaactctggcagaggagtgccatctggataccatttcttgatatcaaagtttttctctgcccattccttcagctgtgcgtacatcagcagacggtcacccgcaccgccgcgtgcccatgcctggttgttgctctcctccagatattccggtgcgacggtaatatcgtcagcgacacggttcatcttgccgagataacgatcctgcatgtacagcgccagcacgttgttagcgacttcagttgcacccggtacagtcaacggcgtttctgcggcgttatgaccgacttcatgccagatcagccagtcgttcagcggcgtcgtcggcagcgtggtgctgttcggcgagaagctgctgttcattaccggataacccgaatgcgcatcaccgatggagatctgcacatcgttggtgaaacgatgtttgtggcccggcaagtttttataggtaaacatccggtgcttaccgtcttcgctatcacggccgtagaagtcattcatcgagctggcaaaggtatccagatcgttagcgaattgctccagtccgccagtgtaattgctggcattcaggttcttcttcggtgtggtatagacgaaagcgtctgattccagctcacccagcggagccggtgagttcagatcgtttttccatgcgccgtctttatagaacggtgcttttaccacgccagtaaaggtgaagctggcagattcattggtagagctattgcccttgatataaatcaggccaccgtaaggcaccttgaacttcaccgtaccgctagcgtccagagagtacgttttagtcactcttggcggacggttcagcgcaacttcatgcttctcacgtccggtcaggtcgtcagccagcgccacggtgacggtcacaggaacgttcgcattggacttaatggtgacctctttctgagccggtgcccacaggccagttgactgcatgttacctgcaaaccatttggtcggattcgagtacaggctgatggtttcagtaacgttctgtccctcttccgatactgctcccggatacttctcgacatcaactttgatgttcagatcccaccaggaacggcccagcatcaggcgtgtcagcggtttttccatatagttgagcgggtagctcgggttcatcatgcccgctttgctgctaccgtcaccgtagatcatgttgttatcgaccagcgattttttcagatctgcagaacacttggtgccgcctgcataggcatcattggcgtagcagttcaggaactcggtgaacgttttaaagcccagctcgtcatttttgccttcttcataacgatagctcgtatcgttccacagccagaccgacatgttctggtacagacgttccagatcgacgctgctcagacgctcacctttgcgaccattggtccggaagtagagctcatgctgatacagacgctgaatgttggtgcctaaatccgcagcctgcaccatcgcttttgcagtgtcggcgttaaggcttagttgcgtatactgtggaacatacatgccaccagtaaccggaacccccgtgccaggacgatattccaggcagttgacctcatagtgatatgccggattagtacactctttcagccccgggaacgcggcgaaaattttctccttcgcagccttcagagaatcctctgttttatgatcggcctcatcaataaaggcataacgcgtttcctgtttgccatctacatcttccagccagctggcaacttccagcttcggtttgtcatcaggtttgttttctacctgatatttccacttaacttcccctgtcttactatcgatggtgtacggcagcgcaccatctacggcaggataacgttcatagacccaaatgcccgttgcgcgctgctgacgaacgcggttcggatacccttgcggatcgttatttactaccgacttgttcagtgccatcgacagacctgcggcatccaacagacgcacaaaaccagacgcgctctcttccttaagattgctcatcacgttttccatgatcagcaccgatccacctttgttcagataggcgatcagatcggtcacatcctgctgagtcagcttcggtttgctggtatctgcacgcagcgggattgcataaggatcgttacccacctgagtcacatattcaaagccgttaaggatcagcagcggcatttcctgcggatcgagatcgccatagctacttaaatgctcaacagagatgcccgcaaaatccggatggaagtcgaacgcagcgctgtttcctgtaacctgaccatgacgtttaaaatagacagtatccaggttggtgcctacggtcatgctggctttcgcgtccggcttccatttatcgtcggacagatagcgcagcacgttctccatgaagttcttcatgtcatccgggtcgctgttgagcgtacactgcccatctttattaacgcccccgttccagctgtaaccgttcgggcaacgcaaaatgctgttgtagtgtgggttaccgataaccatcagtttgccctcaccgacttgccccagcgaaataaacggcaggttaaaggtggcggtatcgcgcgtaacgttttccggctcaacaagagaaggcgcttccgtaatgtacgccagctcgtttttatcccaggcgcgtttttcgccgaaggccagccagtagtttttatcattacgcgccatcagaatcgggaaggccgcgttggagatattcaccaccgcctgaccgcgcgcattacccgtgctgccatagaagttggtggagtcatggaatacatggaacttgctgacagatttgtagttcgtatccacgccccacagcttgttgataacgccctgaatctggccgtcattaacattgcgcgtcgtcagcgagaaccagcgagcctcgttacaaccatcggttttcgcacaaatcgcggtatcgatctctttggcctgacccgtattaaactgctcaataaattcgttaggcagattaacgacttgctcaccttcccccagcgtcgcaccgttggataacgagagattgataatctcgttgatcacgttgggatattcggcaaagaccttgcgtacatcgtccggaacaacacgggtattattttgcccggtcgtcgaatagcgatgaataagctgatcaatattcgccccgcgaacttcatcacccagttcagtcagcgcaatggtcgacttattgccgcgcactgaacccagttcaaaggtatcgataccaaaggagatggtttcgccccagctaaaggaaaattcaccattttcccctgtcacgccacggcctgaattggtgtagtagttgacgccagcaacaccatatccctggctatcgaccagtcgaccttcagagagaatgatttcagtgggttgatactgataaaactgttccgcgttagccgacacgaaggaagcgttcagatccggttttgttcccggcgtggtgacgggcacgaccggtgaagtatgagtggatggcgctttatcggtcgcagcattgttttccacctcttcattgaccagctttttgaactcttccggtgccagatcgatttgcttatacagcgagtcgaagcgtttactctcgatcaccgaggagaacgtcagacaaacctgttctgtattcgccggacagctgttactggacgttaccagcgaaaccgcattgcttttcttgtcatcggagcccgccagttcttgcgcgtcctcaaggctaaacgacactttttcaaccgcacgcaagctacgcgcagcttctgactgagtgttgaaggtggcaattgtcgtgttacccgccacgcaagtaacgtcctcgccaggtttaaatgtaaagccatcgctggattcaccattacaggtagcaccagttacccgctggcttccgcccagggtcagataacccgttttcgtaggaacaggttctggctccggttctggtgttggttcaggatcaggtatcggttctggcgtaggctctgggtccggcgttggctcaggcgtcggctccgggtttggtgttggatcaggtttcacttccggcaaagaccctgttccagaatctacaggcggcgtatcggaggaagatccggaaccaccgccatcacaaccggctaacagggttgcgctcaaaatagccgctaaaagcgatttcttatatttaaatttcttattcattaataacgcaagtgacaaaacaatgttaaaaaattcgtaactgggagaaatagttttatgctttatcttctctaataacttcctccattcttaagaaaacgacatcattgatagaaaacaggtgaaatttataagaataacccctatacgatgtctatctggctatttttacgaaatttcaacaaacaaaaaattaacaacatttcacaacgtaactatataaatttgttggtagttttaacgattaagattgcaaaagcaacagatagaacggtgtttgctcatcaagcgaacataattaatacagacttgttttgcgtgataaaaaaatagatgttctcacgctcttaattatttagcaggttatctgaacgcaaaacattattgctgcatggataataaagcgagaaatgattttcaattaataagacagaataatgtaaatgaagccggatgatattaacgatcatccggctttattgatttacgagactaacatcccggtaaacacatacgcctgcagcagggtgataatgccgataacgctggcaaaaatcagactgtgcttcacggtgtagcggaacagttcagattctcggcccaccatgcccgtcgcggcgcaggccacggcgatagattgcggggagatcatcttgccagttacgccgccgctggtgtttgctgccaccagcagggtgtcagagacgttgatttgctgcgccgtggtcgattgcagtgaaccaaacagggcgttagaggaggtgtccgagccggtaaggaatacgcccagccagccgagaaacggtgagaagaacgggaacatcacgcctgtacctgccagtaccagcgccagcgtggtggacatgccagaatagttggtgacgaaggcgaacgccagcaccatgccaatcgacagtatcggccacttcaagctaattagcgtttcggcaaagacgccaatacctttcttgatccccacaccgaggatgaagatagagataatcgccgcaataaaaatagcggtgccgccagccgagagggggtcgaatttaaacaccgcatccattggcgttggttgggcgacaatgggtgccgctttcaacacttgttgatgcaaatgagggatctggaaattaatcaccagtgaataaaacgcgccgcccggagcaaataacgctttaaacggcttcatggtccagatggtgaccagcaccgttaagattaaaaacggtgaccacgctcgaatgatttgccccagactatattctgaaggcacgggaccgccagaagatggcttatttaccaccatcgcacctgcggattgtcccatgctgattgccgtttcggtatttttcggccgccagactttaaggaataaagcgagtgagacgatactcaccagcgccgaagtaatatccggcagttccggaccaatatagttagaggtaaagaactgagtgacagcgaagcttcccccagcaaccagcgccgctggccacgtctctttcacccctttccagccgtccatcattgctaccagccagaacggcacaagaaccgacaggaacggtaactgacgtcccgccattgcgccaatgtggaacggatcgattcccgttacctgaccggcgaccagaatcggcacgcccaacgcaccaaacgccaccggcgcagtattggcaatcagacacagccccgccgcgtataacggtttgaagcccaggcccaccagcagcgcaccggtaatcgccaccggcgcaccaaagccagccgctccttccagcaacgcaccaaaggagaaaccaatcagtaacacctgcaaacgctgatcgtcggtgatggagataaccgagctgcggataatatcgaactgcccgctggcaacggttaatttatacaggaacaccgccgcgacaataatccacgctattggccataatccataaataaagccatagcccgcagcagcaaatgccatatcaatcggcattttaaaggcgaatattgcaatcaggatagataatataagggttattgctccagcgacatgtcctttcagacgtaataccgcgagtgcaacgaagaagaatattatcgggatcagggcgaccagagcggatagccccagtcctcccatcggcatatacatttgggtccaggtaaccatattgttcagtctcttattatctttatatgcttgatatacttaaggttgtaataagcaaaagaggactgaactgtaaaatataggcgttatactttacagcaacagtacgccgctaacgcaattgctacctctggcataacaagtatatcgggtaagggtttctgttccgcacacgcagacgcagagtatcgttaagatgtccatattgttgttttaggcccgctagtaatgcgctacgggtatttaatattgttaaaccctgataatcgctccggttatttccgggataaatgtactaccgcagttactatcatagccccgacaataaaacttgccggggcttttttgacgctattaatgactttctttttcgcgtaaacgccaggcgtgtaataacggttcggtatagccgtttggctgtttcacgccgaggaagattaaatcgctggcagctttaaaagcacacgagttagcgaaattccccgccatcggacgataagccggatcgccagcgttttgctgatcaaccactttcgccatattctccagcgacgcctgcacctgttctttggtcagaataccgtgacgtaaccagttggcgatatgctggctggagatacgcagcgttgcgcggtcttccatcaacgccacattgtgaatatccggcacttttgaacaaccaatcccctgctccacccagcgcaccacgtaccccagaatcccctgcacgttgttatccagctcttgttggatctcttgcgccgaccagttagcgttttcagcaaccggaatagtcagcagatcgtccagcagcggttcaaattcagcattgaactcggtctgggcaatgttggcttgtacgctctgtacgttggtttggtggtagtgcagcgcatggagcgtagcagcggttggtgacggaacccaggctgtgtttgccccggcacgcagttggtcgcccttctggctgtacatgtctgccatcaggtccggcattgcccacatgcctttaccaatttgcgctttaccgcgcagcccacagaacagaccggaaagcacgttattacgctcgtaggctttgatccaaggcgtcgatttcatctgatttttacgcagcatcgggccagcttccatcaccgaatgcatttcatcgccggtacggtcgaggaaaccggtattgatgaacgccacgcggttgcgcgcctgagcgatacagctacgcaagttcagcgaggtccgacgttcttcatccataatgcccattttcagggtattcggtgccataccgagcattgtctcaatgcgggtaaacagtttgttggcgaacgccacttcctgcggaccgtgcattttcggtttcacaatatagacgctgccagtgcgcgagtttttctgcacttttaaatcatagagggcaatcgcgccagtcatgacgccatcaagaatgccttccgggatttcattgccttcgctgtcccaaatcacaggaatggtcatcaaatgacccacgttgcggataaacagcagcgagcgtccgtgcagagaaatttcagagccatcggcggcggtgtaatgacgatcgtcattcagtttacgcacgatttgccgaccgtttttctccattttctcttgcagagtcccctgcatcaggcccagcaggttgcggtacagcaggattttatcttccgcatcaaccgccgcgaccgaatcttcgcagtcgagaatggtactgatagcagcttcgacgataacatcgttgatgtgcgccggatcgtctttgccaatccgcccattggcatcgatttgcagctcaatatgcaggccgttatttttcagcaaaatgcaggtcggcgcagcggcatcgccacggtaaccgacaaactgtgctggagtacgtaacgtggtttctttaccatttttcaactggatgcgtaattgtttatcaaccaccttaaacgccaccacatcctgatagctgccgttttccagcggtagagattcatcgaggaaacgccgaacccaggcgataacctgctcaccgcgttgcggatcgtagccgctgaccatcgccccttcctgcgggatgatgtcgctgccgtataacgcatcgtacagtgagccccagcgagcgttcgccgcgttcagcgcgtagcgggcgttcattgccggaaccaccagctgcggccccgcctggctggtgatttcgctgtcaatgcccgtggtttccaccgtcacgcgctccggttgcggcaccaggtagcccagttcacgcaggaaagatttataggccgctttatcttttaccggccccggattgctgcgatgccactcatcaagcgctgcctgaatgcgatcgcgttctgccagcaactgacgattttctggtgccagatcatgaacgatctcatcaaaattgcgccagaacgccgcagcgtccagccctgttcccggtaaaacttcttcatccacaaaacgtttaaaattggcgtcaatgcgtaaacggctctgggttatggtttgactcattgtttatctcctcgttttcgcttatttcgccaacaccgctgctgccgctttcgcgacctgcgcatcctgtgctccggttaaaccagaaacgcccacggcaccaataatttgcccatccacaacaaccggtacgccgccttccagcgacgttaataacggcgcagtcacgaacgcggtacgtccgttgttcaccatctcttcatagcccttagtttcacgacgccccagcgcggcggtacgcgctttctcctgggagatataagccgcaatcggcgcgcaatcgtccatgcgacttaacgccagcagatgaccgccgtcatcggcaacagcaatggaaacagaccagttatttttctgcgcctcttcctgacctgcggcaataattgcactcgccatttgctggctaagaatgactttagttttcattttgttattccttttcaagggcttgttctacaatttcaatccagtgacgcacagaggtacgaccggcgctcgccagatgcgtctggcaaccaatgttggcggtgacgatcatttccggtttgccgctttccagcgcattcattttgttatcccgcagctggcgtgccagatcgggatgcgttaacgcatatgttcccgctgaaccgcagcacagatggctgtcgggaacgtccgttaaggtaaatccaagacgaagcaacactttttccacttcgccgttcagcttttgcgcatgttgtagggtacacggacagtggaaggccagctttttatcgccgcgaattgccagtttttccagcggttcctcgcgcagaagttcgactaaatcgaccgccagttcactgacctgacgtgctttatcggcatataacgcatcgtttttcagcatctgcccatactctttgacaaacgcgccgcagccgctggcggtttgcaaaattgcctcggcacctgcttcaatcgcgggccaccaggcatcaatattattgcgcgcccgtgccagccctttctcctgcgcattaagatgatagtccaccgcgccacaacagcctgcttcgttagctggcatgacgctgatccccagacgatccagcactcgcgcagttgccgcgttggtgttgggcgaaagcgtaggctgggcgcagccttccaacattaaaacccgacgcttatggcgcagcggcggacgcggtttagctttcaccgtttcagcaggcagttttgctctgacctgttccggtaaaaacggtcgcagcaccagccctacctgcgtcagcgcacggaagaccgccggacgcggcactacctggcgcaatccttcgcgcagtattcgctccggcagtgggcgtttcactttctgctcgacaatatcacgcccgatatccagcaaattgtgatagcgcacaccagaaggacaggtggtttcacaattacggcaagtgaggcagcgatcgagatgctcctgtgttttaagcgtgacttcgttgccttccagcacctgtttaatcagatagatgcgcccgcgcggcccgtccagttcatcgcccagaagctgataggttgggcaggttgcggtacaaaatccgcagtgaacacaggcgcgcaggatgctgtcggcttccagcgcgcgcgcgttctgccgcatctcttcagttaattgggtttgcatagcctgctcctcaaagttccgcgtacatgcgaccggggttaaacacgccgcaagggtcgagctgctgtttaagctgctggtgatagcggaataaaggagccgatagcggggcaaagccaccatctccggcactaaagcgggtcgcatgaccgccagcgttgcgggcgatgcgatggatttgattgtcctcggctgtcgatttcagccagcgtaacgccccgccccagtcgatcagttgctcgccgggtaaatccatcatcggcgcatcactgggtaatgaaatgcgccataaggtacctggtaacgagaagaacggcagttgttgttcacgcaattgctgccagaactgaccggcaacctcttcgccacccagcagttcacgcgctgcttttaccgatccttcgccgccctcaaggcggatccacaacgcattgtcgaagtaacataagccactaatgggtaatggctggagttgccactcggcgatttcactcatggcttcttgcaggctgatttcccgacgcaggctcagggaggcgcgcggtcgcggtaacactttcattgagatttcagtgagcacgccaagacaaccgtagcttccgaccattaaccgtgagagatcgtatccggcaacgtttttcatcacttcgccaccaaaacgcagatgttttccagcgccggtaatgatgcgcgtgccgaggacaaaatcgcggaccgaaccgctccacgggcgacgcggccccgccagcccgcaggcgaccatcccgccccaggtggcttcttcaccataatgcggcggctcacaggggagcatttgccccgcgctttccagcgccgcttcaattgtcaccagcggcgttccgacacgcgcggttatcaccagctcggtcgggtcgtaattaacaatgccgcgatgacaacgaacatccagcgtttgcccggtgacagggcgacctaaaaaggctttgctattgctgccctgaatcaccagcggcgttttatcgctaatcgcctgattcacctgctccagcagcgcctggctgtaatcacactcgcgtagcatcagaaacgctccagttcagggaaaggtaaatgaccgtgatgcacatgcatggcaccaaattcagcacagcggtgtagcgtgggaatgtttttcccagggttcagcaaaccatcggggtcaaacgccgccttgaccgcatggaaggtcgtgatttcatcgctgttgaactgggcgcacatttgattgattttttctcgcccgatgccatgttcgccactgatgctgccgccaacttcaacgcagagttcgaggatcttcccgcccagctcttccgcgcgggcaaattcaccgggttcgttggcatcgaaaaggattaacgggtgcatgttgccatctccggcatgaaagacgttggcaacacgtaaatcatattgctgcgataaacgggcaatgccttccagtacgccaggcagggcgcgacgcgggatggtgccatccatgcagtagtaatccggggagatacgtcctaccgccgggaacgcatttttgcgaccggcccagaaacgtacgcgctctgcttcgtcctgtgccagacggacgtcagtcgcgcccgctttcaacaagatgtcgttaacccgctcgcagtcttcctgtacgtcagactccacgccgtccagctcgcataacaaaatcgcttcggcgtcgacgggataaccggcatgaataaaatcttccgccgcgcggatcgacaggttatccatcatctccagcccgccggggataatgccattggcgatgatgtcaccaaccgcaagtccggctttttctaccgagtcaaagctggctaacagaacccgcgccacgggcggcttcggcagcagttttaccgtcacttcggtggtcacgccgagcataccttccgatccggtgaacagcgccagcaggtcaaaaccaggtgaatccagcgcgtccgatccaagcgtcagtgcctcgccgtccagcgtttgcacttcaattttcagcaggttatgtacggtcagaccatatttcaggcagtggacgccgccggcattttcagccacattgccgccaatggaacaggcgatttgtgaggaagggtccggtgcgtagtagagattatgcggtgcaacggcctgggagatcgccaggttacgcacgcctggctgcacgcgcgcgcggcgaccaacggggttaatgtcgaggatctctttaaagcgcgccatcaccaacaacacacctttttccagcggcagcgcgccaccagaaagcccggtgcctgcaccacgggtcaccaccggtacacgcaggcgatggcagacagccagaatcgctgtcacctgttccatttgcttaggcagaacaaccagtaatggacgcgtgcgatacgcgctcaacccgtcacactcgtaaggaatgatctcctcatcggtatgcaggatctcaagtccagggacatgctcacgcagtgccatcagtaccgatgtgcggtcgacatcgggtaaagcgccatcaagacgctcttcgtacaagatgctcatgagtaggcttcgctttgttgtgttgtgtggcagctgatttttgcgcgctgcttctgtgaacagttattaagcgggcttttcgttttcgtctatctctttagctaccggtcagaccattttttttccagctctgtgaccttgtcttggttaactcaatgttaaattgatgtaacataatcacttacgtgatgtgcgtgttttgcgagttaagaacagaaaaattggtcctacctgtgcacgaggtccgggaatgaaagatgaacgtcgccctatttgcgaagtggttgcagagagtatcgaacggttaattatcgacggcgtactgaaggtcggtcagccgcttccctcggaacgtcgactgtgtgaaaagctcggcttctcacgctccgcactgcgtgaagggctgaccgtgctgcgcgggcgcgggattattgaaacggcgcagggtcgcgattctcgtgtcgcacggcttaatcgggtgcaggacaccagcccgctgatccatctgttcagtacgcagccgcgaacgctgtacgatctgctcgacgttcgcgcattactggagggcgaatcggcaaggctggcggcaacgctgggaacgcaggctgattttgttgtgataacccgctgttatgaaaaaatgctcgccgccagtgagaacaacaaagagatttcgctgatcgaacatgcgcagttggatcacgctttccatctcgccatttgtcaggcttctcacaatcaggtgctggtgtttacgctgcaatcattgaccgatctgatgtttaattcagtgtttgccagcgtaaataatctctaccatcgaccacagcaaaaaaagcagatcgatcgccagcatgcgcggatctacaacgcggtgttgcagcggctgccgcacgtcgcccagcgcgcagcacgcgatcatgtgcggaccgtgaaaaagaatctccacgatatcgagctggaaggccaccatttgattcgctcggcggtgccgctggagatgaacctgagttagctggtattaaatctgcttttcatacaatcggtaacgcttgtacggctccgccccaatgcgttccagcatgttattcatgcctgtattggtttcgaggatccatgacatctccagcgcatcgatcttccggcgggcaaacggatcgcgtaaggcttcaatcaataacagcgcaatcaccgggccgatgcggctgaactgatactcgtcgcgcacgcccatcagcggtactcgcgcagttcgcacaccgctgactttcaaacgccacagcaattttgcccagccgaagggaaagagcgatccgttcagatcggcaatcgcctcgttgatgttcggcaagccgacaataaacgcgcagggtgcagaatcaatctcagcgatatagatcatatcgtccggcaccagatatttaagttgatcgcccatggtcgcgaattcatgttcggtaaacggcacaaatccccagttgtgctgccagccagagttgaaaatctcacgcaggatctgcatctcttcggcaaaccgctgacgattgatgcagcgaatggtcacctttttgcgcacctgatccatcagtttttttagcgccggagagaaagtgagatcggttcgctgcatccaccacgccagtaaatcaatgcctttgtgataacccagttgttcaatatgcgcggcataccacggtttgccgtgtggcatcatcgcacagggtggtgtgtcaaaaccttcaatcagtaatccgctttcctgattgatattcaggctgaaaggaccgctgatcttacttgcaccttgtgacttcaaccacgcttccgctgcgccaaacaacgcggcaaaaacctgcggatcatcaatggcgtcaatcatgccgaaatgaccggtatctttgccgtaacgctcgcggtgcaaggtatctatttgcgcggtaatacgcccaactatctgccccgctttttttgccacccacgcctgccagatgatatggtccgtccccggatttttcgcagacaaatgctcgttgcgttcaatgaataaagggggtatccagtttggatcgtcgggataaagtgatgacggaaaagcgataaatgccttaaggtcatttttattaaggaaggtgcgaacaagtccctgatatgagatcatgtttgtcatctggagccatagaacagggttcatcatgagtcatcaacttaccttcgccgacagtgaattcagcagtaagcgccgtcagaccagaaaagagattttcttgtcccgcatggagcagattctgccatggcaaaacatggtggaagtcatcgagccgttttaccccaaggctggtaatggccggcgaccttatccgctggaaaccatgctacgcattcactgcatgcagcattggtacaacctgagcgatggcgcgatggaagatgctctgtacgaaatcgcctccatgcgtctgtttgcccggttatccctggatagcgccttgccggaccgcaccaccatcatgaatttccgccacctgctggagcagcatcaactggcccgccaattgttcaagaccatcaatcgctggctggccgaagcaggcgtcatgatgactcaaggcaccttggtcgatgccaccatcattgaggcacccagctcgaccaagaacaaagagcagcaacgcgatccggagatgcatcagaccaagaaaggcaatcagtggcactttggcatgaaggcccacattggtgtcgatgccaagagtggcctgacccacagcctggtcaccaccgcggccaacgagcatgacctcaatcagctgggtaatctgctgcatggagaggagcaatttgtctcagccgatgccggctaccaaggggcgccacagcgcgaggagctggccgaggtggatgtggactggctgatcgccgagcgccccggcaaggtaagaaccttgaaacagcatccacgcaagaacaaaacggccatcaacatcgaatacatgaaagccagcatccgggccagggtggagcacccatttcgcatcatcaagcgacagttcggcttcgtgaaagccagatacaaggggttgctgaaaaacgataaccaactggcgatgttattcacgctggccaacctgtttcgggcggaccaaatgatacgtcagtgggagagatctcactaaaaactggggataacgccttaaatggcgaagaaacggtctaaataggctgattcaaggcatttacgggagaaaaaatcggctcaaacatgaagaaatgaaatgactgagtcagccgagaagaatttccccgcttattcgcaccttccctaaatcaggtcatacgcttcgagatacttaacgccaaacaccagcgaaatgagcggcttgccgacgatcaacaccgcgagcgccaccagaataccgattccgcccgccagtaaaccggacttcacacctaacaaccacggtctggtggtgcgcggatctaaacgcatcacctctgggtaaaaacttttacccagcaaacccgctggcgttccggcggcgtcgaagaatgtcatggcgattttaaataacccggcggcagcgggtcctaacacgatccccaccaacactgtgctgcacgagttacgcgccgaccagatggagtgggcaatgttggttgaccagacaaaactccacgcgcctttaatgtatcgggcagactcaaacagattcaatttgaaggcgttatggatatttcggcggcgtaattcgcgcgcggcaaaccaccagtacatggtgccgccaaccagattcgacacgtaccaggcaataacaaaacccgcaaaaccaaagtcaaaataccaggctacgacgctccccgctgcgcgcagaaaaggtttcgtcgcctgctgtacagcaattaaatcgaagcgatctaccgcacgcagaatgccggtcggcgtggaggaagccattgaaggaatgagcgtgcaatagagcgctgccagccaaaaactttggtcatccagacctaatgaatgggaaaggaatggcagtaaggcaatgccaccgacaatcgccaccgcgccgctgacgatatccagcgagaaggaaaatgagacgacattgcggaattgctgcggattattgttggttaatgctggtgttccgtactgaaccaccagttgccatgtctgaaacttaataaaatcgctgatcgacttggcgtacgattgcacaatcaccagtacgccaaacatggcgggcgtcatccctttaccggcacacgagagcgccaacagacccagcaaggcgctcacgacattactggagcctaaccaggcgctattgcgaataatggtgcgaaacgcgccatctgcaaaccaatgtttgatgttaaaacccgccaattcagcctgaccttatcgttgatagtaaaaagtatcccgccagccttaagttaaacttcggcggtcagaaacgatggcaaccagagaaaccgccttctgtgcctgttccagcacttcgctgtagggcgctctggaatcaatctcaagaatttttgtgccgttatagccaatcttcgacatgacaccgattttgtcctgcagctcggcatagtcatggtcaggcttgcgggagatggcagtctcaatatcaatgcccaggcgaataattaattccgggcgatattgcgccatttgttggtataaacgccgttcgcgctgcgccagaaacatgctgattttcccggtcgcacgttcgacgccaatccccggtccatcataataaaagcccgaaatttcagcctgcgggaagcgatcgctgaccaccagaacgccactttgcgccagtcgctgaaccttgcgtagattcgccattcttcgcagcgagaagcagtacataatcaccgccgcccatagcgccggagatttggttttcatgctttgggttttcgaggatttggccgccagtcgccgttccagccagacgccaaccaacggcaatcgtttgattttgtcgccgtcttcgccggagagcagccccagatagcgccgctcggtttgccagtgttgttgcagcgatttcaccaggtcggtggtcagtgtggatttaccggtgccatcacacccgaccaccgcaatcagccccggaatgtagttgggctgcggcgcggttgtactattaacagtttgagtttgtagtgcatccattcgttaaatcatcccctatccattttggtgatcaggaaagcgcggcgtgaattgcgcgtagtgacgcttgcagaatttcatcggcggggtgtcgcccatccagttcaaggatctttgcgccattgaatgtcagttgcggcgtaacggcgattttttcctgtaacgctgccagttggtggtcaggtttacgcgcaaacgcggtttgttcatcaatgccaagacgaatcaacaatacgggcaaataagatgccatccattggtacagcttcagctcgcgctgccttaacatttttatccaaccgttaccgcccgtggtttttgccaattgcgggccatcaaagcgaaaccccggcacttcaacctgcgggtagcggtcggtgatgagcagaaagccttgctggcttttacacaacattttgcgaaacttgtacgcccgccagcaggaaagcagatagataaccagtgcagtaatattgccaggcggtgttgagggcttttcgtgcacatgtgccgctttacttcgcagataacgcccaaaaggtgcgccaataacagggagctgtgaaatccattcgccaattcgcccggacgattgcccgagataaatgtgttctgttggcattcttgctgccagttcatttaccaggcttgccgtgagggtcgatttacctgaaccatcacatcctacaatggcaataacacgcactggcgtggaattaattattgacatattacgttgattcacgaaaaacccggcagtaaataatgtattgaatattacgtggtccgtgctcagaatatccgttcaaccttattgtgacaatggttaattgtgacattgacctgaattacgctttcataaaaacatattaaccaaataaatatttttaatggatatttaaattaaaggatatattcatgcagtcaataacacctccattaattgccgttattggtagcgatggttcaggcaagtcaacggtgtgtgaacatcttattaccgttgtcgaaaaatatggtgctgccgaaagagttcatttaggaaaacaggccggaaatgtcggtcgtgcagtgacaaaattaccgttgatgggaaaatccttacataaaacaattgaacgaaatcaggtgaaaacagcaaaaaaattgcctggaccagttccggcgctggtaattacagcgtttgtcgcccgtcgcttactgcgctttcgtcatatgcttgcctgtcgtcgtcgcgggttaattgttctaaccgaccgttatcctcaggaccaaattcctggcgcttacgatggtacggtgttcccacctaacgttgaaggtggtcgttttgtctcatggctggcaagccaggaacgtaaagcgtttcactggatggcgagccataagcctgatctggtcatcaaactcaatgttgaccttgaagttgcctgtgcacgtaaacccgaccataaacgggaatcgctggcgaggaagattgccataacgccacagttaacctttggtggtgcacaactggttgatatcgatgccaatcagccactggaacaggtgttggttgatgcagaaaaagcgattacggattttatgaccgcgcgtggttatcactagtcaaaaatggaaatgcccgatcgccaggaccgggcattttcaggaaggttaaatcaactgcaatgctatccagtacagcccaccagaaagaaaaattgccgccggtaaagtaaatacccacgccatcaggatgctggttaccgttttacgctgtaacccaccgccgtccaccaccatcgtccctgcaactgcagacgagaggacgtgtgttgtggagacgggcatcccaatataactggcaagaccgatagacactgccgccgtcatttgtgccgccatgccttgcgcatacgtcatgccgcgcttaccaatcttctcaccgatggtcatcgctacacgacgccagccaatcatggtgccaatgccgagcgccagtgctaccgccatgatgatccacaccggagcgtactcaatggtgcttaacatatcgctgcgaagttttttcagcaggttctggtcttctttactgacgcctggcagtttcgctagcttcgcggaggtatcagagatgcacagcataatgcggcgcagctggctgcgctgactcacgcttaacggctcgtaactttccatattgcctggcagcatcgttttaacgcgcgcaatagcatcaaaggtatttgccggatgacagtgaaactctgttacttgcgtgccatcagtcgatgctgcaggcaatggaggttccatcgcaatcaacttctgcggcagttcaggatgctgttgcaggtagtgttcgaagttggtaacggcatcgcgggtacgggtaatttcatagccggacgcattcatattgacgacgaagccagcaggggcaatccccaccagtaccagcattaccaggccgatccctttttgtccgtcgttcgcgccgtgcgaaaacgccacgcccgcagcggaaacaatcagcgcaatacgcgtccagaatggcggtttacgtttgccttttttctttttgcgatcttccggaatgcggtgaatacggtcacgctttttcgtcccgctccagtagcgtcgcagcaggaatatcaggcctcccgcaatgaccaggccgacgataggggaaacaatcagcgaggagaaaattttggtcacttcacgcaggtttaacgcatccatcaccgatgagccggttaacagcgcgttggttaaaccgatgccgataatcgcaccaatcaaggtgtgcgaactggaggccggtaaaccgaagaaccacgttcccaggttccagataatcgccgccagcagcatggaaaagaccatcgccaggccgtgggttgaccccatattcagcaacaaatcggttggcaacatatggacaatggcataggcaacgctaagtccgcccaataacacgccaaaaaagttaaaaaatgccgccatcaccacagcaagttgtggttgcatggcacgagtataaataacggctgccaccgcattcgccgtgtcatgaaaaccattgattgcttcgtagaacaacacaaatgccagagcaagcaataacaaaagccctgtgtatatatcaaggccaacaaataaatttagcatatattagattacgccattttgaatttacgaacggacgcattatcagtgactttaacggcatgggcaaagtgaaatatcattttttaacgataaaaagagtgttatttcttgtgtatcagacaataagcattcattcaaaacctttagaaataatcaaaacacaggtattccactggttaatatattcacatatgaaatgaataaatattggaatatataaatattgaatattttgattaatccccgtactgattattcttcataatcagtacggggttgctacaacatgtattactttttcaccacaattaacggttcaatatcactctcttttttgatgaccagtgattcatcaccgcgcaaacacgtcccaccgtagttgccgccaacggtgaaggtacatacctgaatgtatttaccgtccactttcggcaaacaccacagttgctgatagatgtttttctgctcggcaaatttaccgctggttttgtccagcacctcttcatgatggctgacgaggtcgatattgctgccacagcgaccggcgatcggtttcactgcgtaacctgttttcaccagttcatcattaacagtgaaatcggtatccagcaggtaacgatggtgcgggaacagcgaccagaggatcggcagaatcgctttgttgccggggatcaccgtccacagcggctcaaagaccagcacttccgggcgcagcaatacgtcgataagacgcacttcgttttgcggatgaccggtacggattggcaccgcagcaaactcacggtcgctaacttcacgaatctgatcaaacgcggtttcccacgcccaggttttccacacgcagttaaccagtcgcccttccccatcaatcagttgcccggcagcatcccagcccagttcatccaatccacgcaagatacgcgtttcaaagcccgcctggtgcagcgcctgctccataaactgcgcgtgatagttttcctcgatatctttgtcctgcatgatatggacaaacggacgtgcacgactgtgtttccaggcaccagccaattcgttaatcagcccttccgccggattgaagccgttgcctttatagccctgctccgcccaacgttcgaggatcaagcccgcttcggtatgacaggaggcggagtcggcgttgtactcgtaaaccttcaggccacgctcatccatgcagaaatccatacgaccagtgatcatatggtgacggcgacgctgccaggagagacgcaaacgtggccagaggattttcgggatgtcgaacagcgccagcaggttgtcatctttcagcaccttgtcggttgcgtgaagatacatcaggtgcagctcgttggtggctttaattagctcctgctcggcactctcggtaatggtgtagtaatgataaggatcctgattgatcacctgaccgttggcctgcacataggcgttttgcagcggatctttttcatccagccatttaccgtcaaactggcctttgttttccaggcgcgctccgctgattttcagcagctcgcctgcaatttccggctgcggtaagctgtattcagtatcttccgtctggatcatccagcccagaatggtggtgtcatcaaaagtgtctttcagggtatagcagccgttttcgaccaccatctccagctcgcgcgtccactgttgcccttgcggcaacggggaatgaatcacgttctgttccgcaatacggactttgttgccatgcaattgggtaatgatggcgacatggccagtgtctttaaattcaccgcctttatcccagataagaagcgcacccgcgaccggcgcacgcggcgagccgttaggaaatgcctgcaatggcaggatgttgtcattaaccacttctcgcaggaagcgcagcgagaaaatctcccacgccatacccacgtcagtaaagaccacaccgtaattcagaaagagaaaacggcgagcaaattcaacgcattgccacttgtggcccatatattcgtcgtcgatatagctacggaatacggcgtcatcttcgtattcctgcggatcgagagaactgtaatctgaagagtagattgctaccccacctggggcgtagcccaataatgtcccgaacggggcatcctggctggtcgttcctttgctcatcactttacctttaacaatacaacctaagcagttggcgtaattgttgtgctctgattacctgctcagcgacattaaccggacagaggtcagactaatcatacacctcatcgcagcggctggcgcaaagggttaaaaaattcacattctgtacagcaagtgacctgctacactgcttcaacactaccactcagaaggcaactcactatgacagacaatacttatcagcccgcgaaagtctggacgtgggataaatccgctggcggcgcgttcgccaatatcaatcgcccggtttctggtccgacgcatgaaaaaacgctgcccgttggcaaacacccattgcaactttattcgctgggaacgccgaacggtcagaaagtaacgattatgcttgaggagctgctggcgctgggcgttactggtgcagagtacgacgcctggctgattcgtattggcgatggcgatcaattctccagcggctttgtcgaagtgaacccaaactcgaagatcccggcgctgcgcgatcatacgcataatccgccgatccgcgtgtttgaatctggttcgatcctgctttatctggcggagaaatttggctacttcctgccgcaggatttggcaaagcgtactgaaacgatgaactggctgttctggttacagggcgcggcaccgttcctcggcggtggttttggtcacttttaccattacgcaccggtaaagattgagtacgccatcaaccgctttaccatggaagccaaacgtctgctcgacgtgctggataagcaactggcgcagcataagtttgttgcgggcgatgagtacaccattgcggatatggcgatttggccgtggtttggcaacgtggtgttaggtggtgtgtatgatgccgctgagtttcttgatgcgggcagttataagcatgtacaacgctgggcgaaagaagtaggcgaacgtccggcggtgaaacgtgggcgtattgttaaccgcaccaacggaccgctgaatgagcagttgcatgagcgccatgacgccagtgatttcgagacgaatacggaagataagcgtcaggggtaagggttggtgttcgtcgcagcaagccatccaggccggataaggcgttcacgccgcatccggcaatcgtgcacaatgcctgatgcgacgctgccgcgtcttatcaggcctacgaaagctaatcatcacgcgctggtaatgtcgtaatccatttggcgcagtgcgtctaatgtggctttggcttcatcttcgtcgatgatgctcatggcaaatccgacgtgtaccagcacccactggcccagtagatcggcagggttaccttcacaaatcagggcgatattcacatcgcgcttgataccacatacttcaacctgcgcaagctggtgaatatcttcaccgacagccagcacctggcctggaacgccaatacacattattaactccggttattcaacttcaatacttttgacgatcagcgaatcgccggtatcgacacgcaaccgctcgccgtgacagagcggacactgcgcatcgtgctgatgaatctccaccacctggctgcaatcccagcaccaagcctgggcgggtttatagacgatatgtaaatcgcacccttgcgccaccgttccgtggcagacaatttcaaaactaaaacggacggcgctctcctcaacgcaggagagcgcgccaatttccagccacacggcggtgacgcgcttaacatcgtgctgctccgcctgccgttggataatttcaacggcgctctggcaaagagacaactcatgcattttcgccactcctgcgaccaaacagcagggcgcgacgccctgcgtgtggtacatccggattcgtgactggcagcgaaaggatcattcgtgcgcagtcatccgtcaggcgttggccctcttcaatcgacatgctgtgcgaaagcggcgacatcagcgaacaggagagatattgcgaaacaccgtccagttcgccaacggtaaaggtcatagtgccatacggcagttgcagaccaattttttcactcactttgcgcagcggccagagttgatccgggccggggaagataactgcactcagcatccacggggtgatcacacaccccgtccactgaccttcgaacagcgtaaaatcagaaacatacaccggcattgaaggatgcagaaaagagagatcgtgcatcgaacgccgggcaatttcttcaaacgctgcctgtacttgcgccttcggggaggtctggaaacctgctatctcttcagtcatgaatcgcctcccgtgggatggcttccacgccagattcacgcagcgcagccagaacctgctcaagcgcaggttcaatcattgcttcaaccgtcggcgttaagccgatgtgtggctccagcgattccgggatcacgccgaccagggtcagctttttcggaaactcgccggtgaagcgcagggccgacaagacgtcggccaggccaagctgatgcggagagattttgttggtaaacaacgccggaacttcttcatcccgcaggatcatcatcgttcccggcgcgttctttttcgagacaatggcatccgcaataatcaaatgatcgcgatttgccatgtcgccaagcagctccattcccgccgtgccgccatcgaggatctcaacataatccggcagaatgtatcgttgctctaacgcttcgacaatccgcacaccgatggcttcatcggtcagcaaaatattgccgacccctaagactaaaatacgcattacagaaccttcactgaaaccacttcgttgccgtcagcatccactacgtgtaccgcacaggccatgcacgggtcaaaggagtgaatggtacgcaccacttccagcggtttattcggatcggcaaccggtgtacccaccagcgactgctcgtaaggaccgacgtcatcattgaagttacgcggaccagagttccaggttgatggaacaaccgcctggtagttgctgatgataccgtctttaataaccatccagtgagagagcataccgcgcggcgcttcgaggaagccaacacctttgaattcacccgttgccggaatgttcggcttcacaaaggtggtgtgatcgcctttgccgatattggtgatcagtgcactgtattggttttgcaggatatcctgcaattcacagcagtgaacggtacgaccaataatacggcccagcgtggagtgcagctgtgccacttccagcgtgttgccagtcagtttctgataaatcgcaacgatttcattcagtttgttctgggtagattcgcgacctgccgccagtttcaccagcatattagccagtggccccacttctaccgttttgccgtagaaagtcggtgatttcacccaggaatatttcccgtcgtcagaccaaccatcataagccggaatggtggtgccttcccacggtgcctgcggcgcttcgtctttataccaggagtgcttcgcgctttcctgaatgcctttgatcaggtattcatcggaatgagaagtgatcggacgatacgaggacagatccgcattctcaatgtagccgcccgggaacaggaagctgccgtttttactgtcggtcgggaattccggcacgctcaggtagttcaccgcacctttaccgcgtgtcagccattccgggtagaacgcggcaataactgcggtatcaaccttataaacctgctcaacaaagtcgctcagtttgtcgatgaaagacttgatgtacatcaggcgctcaaggttcagcacgcccaaaccgtcgaggttgatcgggttcgcgacaccacctaccgccaggttctgaatgtgcggcgttttaccgcccagcagcgccacgacgcggttagcgtcacgctggcactccaacgcttgcaggtagtgcgctaccgcaatcaggttcacttccggcggcagtttcatcgccggatgaccccagtagccattagcgaaaatacccaactgaccgctggcaaccagatctttgatcttgttctgaactttggtgaactcttccggactgttcaggtgccaggtcgaaacgcctttcagcatttcggaggctttggttgggtcagcttgcagtgcagaagtgatgtccacccagtccagcgccgaaagctgatagaaatgaacaatatggtcatgcgtggtgtgcgcagccagaatgatgttacggatgtattgcgcgttaaccggaacgtcgatattcagcgcactttctgccgcacgaacggaagacagcgcgtgagtggtagtacatacgccacagatacgttgcacaatcatccatgcatcgcgcggatcgcggtttttcacgatctcttccatgccgcgccacatggtaccggaagcccatgctttcgaaacgacgccattttcgatttcgcaatcgatgcgtaaatgcccctcaatacgggttaccggatcaatagtaattctctggctcatgctttgctcgcctcatgacgattatgatcgttttgttttaaaggaggaagtatcggcagtagacgaatgagtacgatgtaagcgcaaatctcaatagccacaaaaccaatagaaatcaacagttcttcccaggtcgggaagtaggcgtaaccgccgcccgggttgaatgccaccagcgaataggtcagacgccaggttgcacaacctaacagtgcgctcagtgctgacaggaacagcatgcgggaatcattacgcagcttcgccacacgcagaacgaccagcgggaagagcatcagcaggacttcaatccagaacatcacggagtagaagtcaccggcaaacgctaacgacagcttgtcgcgatagataagctcgccaaagcgcagcacgatgaaaatcgccagcaacacactgatggtgttggtcagcttaacaaacagactcttttcatccggaccgttgccacgcagacccgcctgcaccagcgaaccttcaaagatgacaatcgagaagcccatgatgaacgccgtcagcagcgagaacagcggcaacatttcatagctctgccacaacggatgcaccttgtagcccgccgagatcatcagcgaccccattgaagactggtgcatggtcggcagcagcgcaccgagcgcgatgatgaagaacatcaccttgtttagtcgctgtagcgacaccttccaccccagacgttcaaacagtgccggagcaaactccagtgccatcacgccgatatagatggtcatacagaccgccgtctcgaacagtaccgagttcacgttgaagtgacccggaatgtagaagtacggcaggttccagtagcgacccacgtcgatagtgatcgacaagccacccagtgagtaaccaaacagactcgccaacagcgccggacgcaccagcggatggtattgcccacggttaaagacgtataccgcccacgccagcgcccagccgccacaggcaaagccggtgccaatcagcaggtcaaacgcgatccacacgccccacgggaagccgccgttcaggtcagagacagagcccagaccgaacaccagacgcttcacaatcaggagcatacagatgacgattaacggtccaaaaatcatgaccggtttactgatgattttgccgcccagcggttgtggatcatgactcatgatcgtctcctccgtcgtgatggtcgtttttggtgttgcgacgaaccagcacggttaagcccgccagcacagccagtggtagcatcatgcctttatacagggtgtgttgaatattttcggaacgcgcaccggtagaaagatcgtccagtttcggcaggtcgagattttcataaggcacacccgtcagtaccagaacctgagtaccgccgccctctttctcgccgtacagatgcggataatatttcggcaccgtatgcaggtaagtgtcgccagatttcagcgtctgacgcggatagtggtattcgctgccaggcttcagcgccagacgttttttcgcctccgccatcagctcttcacgcgtaccgaaaatcaccgcgcccgccgggcacacttctacgcagccaggtagaccgcctttatcgagacgttccacacctttctggttgcacagctcgcacttatgcagcgcaccaaacgggttgttgtagtcgtacttcggcacgttgtacggacaggcgaccatgcagtaacggcagccggtgcacacatctttgtcgtaatggacaatgccggttttcggatcttttttcagtgcagagaccgggcacacagagacacagttcggatcgacgcagtgcatacactgtttcttaatgtacgcgtagccgttctcctcctggtctttgttgacccctgtgccgctggtccacacctgaatgatgttattggtatacggcgacagtttgtcgttgttcgaccaggtctgttccccttgcgggttacgttcagggaaattgatatcctgacacttggtgacgcaagcctggcagcctacgcacaaggtcgagtcgtacaacatccccagcgatcccggaattggcgggcggttttcagcagccgcatgactgacagacggcagcgcgcccgtcagcaatgccccgcaggaggctgctttaataaaattacgtctgttcacggttattctccccgtgagtcagcgttatctttcttttgctgacgacccagttcacgcaccgccatcacgctgacaccggcaaccaacccaaccacaccgccgagcaaaccaatagcgcctgcagagacgttgccgccctctttagcgttaacatccggtttctgtgaacgcggagtttgattttcgacgttggcaagctgatggatgcctttatggaagccgataccttcttcgttacagccatagcaagggtgaccaatcgccaccggccacacaccgccaacatcgcagaattgcagcgttgagcagttgccgtaagtttctggccctttacagccgaggtggtacaggcaccagccttcgcggtggccttcatcaccgaactctttggcaaaacgaccagcatcgaagtgcgggcgacgttcgcagtgttcgtgaatcagacggccataggcgaaggtcggacggtttttgtcatccagtttcggcggtttgccgtaagtgatgatgtgcgcaacggtcgcgaggaagttgtgcgggttcggcgggcagcccggaatattgataacggttttgcctggcagaacttcttgcaggctgactgcgccagttgggttaactccagctgcggcaacaccgccccacgcagagcaggaaccgatagcgataatggctgctgcgccttccgccgctttgcggatgtgatccacaatcggctcaccggcaaccatgcaataaataccgttatcttttaatgggatggaaccatccaccactaacacatactgccctttgtacttctcgagagcgttatgtttgttctcttcgacctgatgaccgaaggcggcggaaagcacttcgtgatactccagagagatagtctccagtacgaggttttctaccgttggatgcgttgcacgaagcagagattccgtacaaccggtgcactcctgcgcgccaatccagataactggcggacgctgcgggttagtaaccgattcggccatctctgcagcggctttgctacttaaccccatggtggcggctaatgctgcacaaagcttcatgaaatcacgacggttaatgccgtgagaatggatgagggtgttatctccagtcatttatagttattccgttgcgaagacctggcatatattttgcctcaatcgcaaaatcaataatgcgatcgatgcgccatttaccacacatttattatggttatcgatatcatgatactgcggcggggcgctaaaacgaagggaagaagcattagtgtaattaattaaagcaagataatacgtatgtttgatcaattttcgaggcgataaccggccataaaaaagcgcaacgtagaacaggaattattctcacgaaagaaatccattaccatctctttatccagtccatagcggcgcgtcagaatacccgcttcccaggcgctaagctggcgatctccggtcttttcgtacatccggtgtgagtagcctaatacaaaaccgcgtttataatcggcacagaattttgtcacattaaccgcactgtcggcatgcgttgcttttaatcccgccattaagcctttaccaaaatggttattcatcgttcacctcattcgctatatattgtcatatatagcgatattttaggcaaagaacgacttttgcgcacgctattttttcatgcttgtttaagacgtaatcccgtaagagataaacctatcaggagagatatttatcgaaccatttcagtgtcctttgccaggcaagatcggcggcagatttgtcataacggggcgtggaatcattatggaatccgtgattaacccccggatagatatacgcctcataaaccttattattggctttcaacgccgcctcgtaagcaggccagccctcgttgattcgggtgtccagttccgcgaagtggagtagtaaaggcgcttcaatcttcgccacatcggcagtgggtgcctgacgaccataaaacggcaccgcgcaggccagttccggatacgcgacagccgccgcgttcgatacgccaccgccatagcaaaatccggtaatacccactttgcctgtcgcttgcggatagcgttgcataaactcaattgcggcaaagaaatcattcatcagtttgttggatcaacctgctgttgcagctcacgacctttatcatcatttcccggataacctccaacggaacttaagccgtcaggtgccagggcgatataccccgccttcgccactcgccgtgccacatcttcgatatacggattcagtccacgattctcatgcaccaccactacggctggcgttttgccgctcatctttgcgggcttcaccagataaccccgcacctcgccgtgaccatttggcgaaggatacgtgatgtactcagcaacaatttccgggtcggtaaactctacctgagtcgccagcgcataatttggcttgagcaaatcaaacaacgctaatgccgtcatcccgcctaccgcacttcgccgcaaggttgaggaactcacgtttcgagattttcccgtgagcgtaatagtcatagtaatccagcaactcttgtgggaaatctttggcggttaaacgcggcatcgttgcactcctcagttggtgtttttttaagcaaagcataagcacgtatttttgcccagtttttcgtcactctgtgagccagactacgggatacgcgctggcgaatcgctaaactagaaacattgtttcgaaattgaacggtggaaaggagaggtcatggtctggttagcgaatcccgaacgttacgggcagatgcaataccgctattgcggaaaaagtggtttacgcctgcccgcgttatcgctcggtttatggcacaatttcggtcacgttaacgcgctggaatcacagcgtgcgatcctgcgtaaagcgtttgatttgggcattacgcactttgatttagccaacaattacgggccgcctccaggaagcgcagaagagaactttggtcgcctgctgcgggaggattttgccgcttatcgcgatgaactgattatctctaccaaggctggctacgatatgtggcccggcccttacggctctggcggttcacgtaaatacctgctcgccagcctcgaccaaagcctgaagcgtatggggcttgagtatgtcgatatcttttactctcatcgcgtcgatgaaaatacgccgatggaagaaaccgcctctgcgctggctcatgcggtacaaagcggtaaggcgctgtatgtcgggatctcctcttactcgccagagcggacgcaaaaaatggtcgagttgctgcgcgagtggaaaattccgctgttaattcatcaaccttcgtacaatttactgaaccgctgggtggataaaagcggcctgctggataccctgcaaaataacggcgtgggctgtattgcctttactcctctggctcagggattgctgaccggaaaatatctcaacggcattccgcaagattcacggatgcatcgtgaagggaataaagttcgtggtctgacaccgaaaatgcttaccgaagccaacctcaacagcctgcgcttattgaatgaaatggcacagcagcgtggacaatcaatggcgcaaatggcgttaagctggttgctgaaagatgatcgcgtgacgtcggtattgattggtgccagccgcgcggagcaactagaggagaacgtgcaggcgctgaataatctgacatttagcaccaaggagctggcgcagattgatcagcatatcgccgatggcgagctgaatctgtggcaggcgtcttccgataaatgacctgttaataacgggcgcgcgaaccgcgcccgaatcagatcagtgattatgacgagtcagtcggtcaagatagcccatcacaaatgcagaaagcacaaacgtcagatggataatgacgtaccacatcagtttgttatccgggacatttttcgcatccataaagacgcgcagtaagtgaatggaagaaattgccacaatcgacgctgctactttgtttttcagcgacgttgcgtccattttccccagccagttcagcttctctttgttctcggagatatccagctgtgagacgaaattctcataaccggaaaacatcaccatcaccagcaaaccgccaaccagcgtcatatccaccagcgacagcaacacgaggatcaaatctgattccgccatcgagaagatattcggcagtacgtgaataatctcctggaagaacttcagcgccagggcaactaacgccagcgaaaggccaaagtacacgggggcaagcagccagcgagaagcatacattgcattttcaagaaaacgttccatacattcctgtcgtgtagttaaaacgggcaacagtatatcgcaattgagtaaacagcacgcaacagcaaatcaacatatacgttaaacctttgtcgcataattctgaggtttagggatcttcctggttcccttatcaacgcatcgagaacgtctacccttaaaggacgttgaacctgaagggagaaaaacgatgtctcatttaaaagacccgaccacgcagtattacactggtgaatatcccaaacagaaacaaccgacgccaggcatccaggcgaagatgacaccggtaccggattgcggcgagaaaacctatgttggtagcggtcgcctgaaagatcgtaaagcactggtgacagggggcgattccggaataggtcgcgctgccgccatcgcttacgcgcgtgaaggggctgacgtggcgatcagttatcttcccgtggaagaagaagacgctcaggatgtgaaaaagatcattgaagaatgcggacgcaaagccgttctgctgccaggcgatttaagcgatgagaaatttgcccgttcgctggttcacgaagcgcacaaggcgttaggcgggctggatattatggcgctggtcgccgggaaacaggttgccattccggatattgcagacctcaccagcgaacagtttcaaaagacctttgccattaacgttttcgcgctgttctggctaacccaggaagcgatccccctgctaccgaaaggtgcaagtatcatcaccacttcgtcaatccaggcataccagccaagtccgcatttactggactatgcggctacgaaggcggcgattctgaactacagccgtggcttggcaaaacaggtcgcggagaaaggtattcgggtgaatattgtcgcgccaggcccgatctggacagcactgcaaatttccggcggacaaacgcaggataagatcccgcagtttggtcagcaaacgccgatgaaacgtgcggggcaaccggcggaactggcccctgtatatgtttatctggcaagtcaggagtcgagctacgtcaccgcagaagtgcacggcgtgtgcggcggcgagcatttaggttaaaaaaatgcccggttgtgaaaagcaaccgggcatcattgtgaattcactcttacctgatgtggcgaaaacgccttatccgcctacaaacgcatgaagattcaacatgttgcaatagattttgtaggcctgataagcgtagcgcatcaggcattgagcacctaatgccggatgcgtcgtgaacgccttatccggcctacaaacgcacgaagattcaacatgttgcaatagattttgtaggcctgatgagcgtagcgcatcaggcaattctactttacttcgctttggcggtttcttcgccgaccagacctatcttcaggtaacccgcctgatgcagcgtatccattaccttcatcaacgtctcgtaatcgacggttttgtccgctcggaagaagatggtggtgtctttcttgccttcggttaacgcattcaacgccgtaatcattgtttcatcggtgaccggatcgttaccgataaacatcgagttgtctgccttcaccgacagataaaccggtttttccgggcgcggctgcggcgtgctggtagaagcaggcaagttcaccttcacatctaccgtcgctaacggtgccgccaccataaagataatcagcagaaccaacatcacgtcgataaacggcgtcacgttgatatcatgcatttcgccgttatcgtcgaggttttcgttaagatgcattgccatcggatattatcctgcgcgtaatttttgtgcgacacgaaccggatgcgcagcggcgctggcttccagatccaggtcacggctttgcagcaacaatacctgcgctgcaacatcacccagcatcgctttaaagccgccaatctggcgtgcaaatacgttatagataacgaccgcaggaatcgctgccacgaggccgattgccgttgctaacagagcttctgcgatacccggcgcaacgactgccaggttagtggtctgcgtttgcgcgataccaataaagctgttcatgatgccccagaccgtaccaaacagaccaacgaacggagaaatcgcgccgatggttgccagatagccgttaccgcggcccatttgacgacccactgcggcgacccgacgctccagacggaagctggtacgttctttaataccttcgttatcgtcgctgccttctgacagttccagctcattctgcgcttcattgagcaaatgcaggcttaagcttttgctaccaaaatcagcggcgatatcgttggcctggtttaaggaacgcgcttcagccagcagttgctgctcgcgcttaaggcgacgcttctgattgaagaactctacgctcttactgaagaagattgcccaggtgactacggaggccaaaataagcccaatcatcacgcacttaacgacaatatcggcgtgctgatacataccccagacggaaaggtccgtctgcattaaattattacccactgtgtatctccaggacgcaagtcacaaaatctgcgcataataatatcaaaacgacgtcgaattgatagtcgttctcattactatttgcatactgccgtacctttgctttcttttccttgcgtttacgcagtaaaaaagtcaccagcacgccatttgcgaaaattttctgctttatgccaattcttcaggatgcgcccgcgaatattcatgctagtttagacatccagacgtataaaaacaggaatcccgacatggcggacaaaaagcttgatactcaactggtgaatgcaggacgcagcaaaaaatacactctcggcgcggtaaatagcgtgattcagcgcgcttcttcgctggtctttgacagtgtagaagccaaaaaacacgcgacacgtaatcgcgccaatggagagttgttctatggacggcgcggaacgttaacccatttctccttacaacaagcgatgtgtgaactggaaggtggcgcaggctgcgtgctatttccctgcggggcggcagcggttgctaattccattcttgcttttatcgaacagggcgatcatgtgttgatgaccaacaccgcctatgaaccgagtcaggatttctgtagcaaaatcctcagcaaactgggcgtaacgacatcatggtttgatccgctgattggtgccgatatcgttaagcatctgcagccaaacactaaaatcgtgtttctggaatcgccaggctccatcaccatggaagtccacgacgttccggcgattgttgccgccgtacgcagtgtggtgccggatgccatcattatgatcgacaacacctgggcagccggtgtgctgtttaaggcgctggattttggcatcgatgtttctattcaagccgccaccaaatatctggttgggcattcagatgcgatgattggcactgccgtgtgcaatgcccgttgctgggagcagctacgggaaaatgcctatctgatgggccagatggtcgatgccgataccgcctatataaccagccgtggcctgcgcacattaggtgtgcgtttgcgtcaacatcatgaaagcagtctgaaagtggctgaatggctggcagaacatccgcaagttgcgcgagttaaccaccctgctctgcctggcagtaaaggtcacgaattctggaaacgagactttacaggcagcagcgggctattttcctttgtgcttaagaaaaaactcaataatgaagagctggcgaactatctggataacttcagtttattcagcatggcctactcgtggggcgggtatgaatcgttgatcctggcaaatcaaccagaacatatcgccgccattcgcccacaaggcgagatcgattttagcgggaccttgattcgcctgcatattggtctggaagatgtcgacgatctgattgccgatctggacgccggttttgcgcgaattgtataacattgccacttttggacaattttgcagacattttattgtgaaaagtcttaaattgttgcgtccgggatcaaggcgtcccggacgattcaggagtacaataggcagataaaggcttaaacgctgttccacaggaaagtccatggctgttattcaagatatcatcgctgcgctctggcaacacgactttgccgcgctggcggatcctcatattgttagcgttgtttactttgtcatgtttgccacgctgtttttagaaaacggcctgctgcccgcctcatttttgccaggcgacagcttgttgatactggcaggcgcattgattgcccagggggttatggattttctgcctacgattgcgattctgaccgccgcagcaagtctgggctgctggctaagttatattcaggggcgctggttagggaataccaaaacggtgaaaggctggctggcacagcttcctgctaaatatcaccagcgcgccacctgcatgtttgaccgccacggtctgctggcgctgctggctggacgttttcttgcatttgtccgtacgctgctgccaaccatggcgggaatttccggtctgccaaaccgccgcttccagtttttcaactggttaagtggattgctgtgggtcagcgtggtaaccagttttggctatgccttaagtatgattccgttcgttaaacgccatgaagatcaggtaatgacgttcctgatgatcctgccaattgccttgttaaccgctggcttgttaggcacgctgtttgtggtgattaaaaaaaaatactgtaacgcctgacgattttccccgttcccggttgctgtaccgggaacgtatttaattcccctgcatcgcccgcattcttgccgcatcttcccccggcgtcacaccgaagtaacgtttaaactcacggctaaattgcgatgcgctttcatagccgacgcgcatcgctgctgcgctggccttcatgccgtcatggatgatcatcatccgcgccttatgcagacggtaattcttcaaatactgcaacggcgaggtactggtgacagacttaaaattatggtggaacgccgatacgctcatgttggcttctgccgccagttgctcgacgctcaggttttcggtgtatttattctcaatccgtttcagcacgcggctaatcagactgaagtgagtctggcgactgaccagcgccagtaacgcgccgccgcaaggtccggtcagcacgtagtacagaatttcgcggatgatctgtttgccgagaatacgcgcatccagtggtcgctccatcacgtcgagtaaccgctccgccgcgcataaaatctcttctgataacgtggcggagttaatcccgctggctgccatcgacggctggaaatgctcatcttcgccaatgtccatcaacagttcctgtaactgcaaaatatcgacattgagacgcaaccctgccagcggcacctctgacgtggcataggtttcgcactcaaacggcaacggcaccgtcagcagcaggtattcattggcatcataacgaaacacgcgttcattgatataaccgattttatgcccggaaaagagaattatgatgccaggctcgtacatcaccggtgtacgtgcgaaaggcgtctcgccatacaacaaacgcacatcgggcaacagtcctgacaaactattttctttatttttcagtttattaactttatccgccagcaagcggcaaatctcttcacgtttcatatcgcgtaatttcttaggaataatgcggcaatttgattgtgcgcaattttgtagcatttctccagcactctggagaaataggcaagacattggcagaaatgagcattgagagccagggcgctggcgatcacaatgaaaaacatcaggcagatcgttctctgccctcatattggcccagcaaagggagcaagtaatgaacaactttaatctgcacaccccaacccgcattctgtttggtaaaggcgcaatcgctggtttacgcgaacaaattcctcacgatgctcgcgtattgattacctacggcggcggcagcgtgaaaaaaaccggcgttctcgatcaagttctggatgccctgaaaggcatggacgtgctggaatttggcggtattgagccaaacccggcttatgaaacgctgatgaacgccgtgaaactggttcgcgaacagaaagtgactttcctgctggcggttggcggcggttctgtactggacggcaccaaatttatcgccgcagcggctaactatccggaaaatatcgatccgtggcacattctgcaaacgggcggtaaagagattaaaagcgccatcccgatgggctgtgtgctgacgctgccagcaaccggttcagaatccaacgcaggcgcggtgatctcccgtaaaaccacaggcgacaagcaggcgttccattctgcccatgttcagccggtatttgccgtgctcgatccggtttatacctacaccctgccgccgcgtcaggtggctaacggcgtagtggacgcctttgtacacaccgtggaacagtatgttaccaaaccggttgatgccaaaattcaggaccgtttcgcagaaggcattttgctgacgctaatcgaagatggtccgaaagccctgaaagagccagaaaactacgatgtgcgcgccaacgtcatgtgggcggcgactcaggcgctgaacggtttgattggcgctggcgtaccgcaggactgggcaacgcatatgctgggccacgaactgactgcgatgcacggtctggatcacgcgcaaacactggctatcgtcctgcctgcactgtggaatgaaaaacgcgataccaagcgcgctaagctgctgcaatatgctgaacgcgtctggaacatcactgaaggttccgatgatgagcgtattgacgccgcgattgccgcaacccgcaatttctttgagcaattaggcgtgccgacccacctctccgactacggtctggacggcagctccatcccggctttgctgaaaaaactggaagagcacggcatgacccaactgggcgaaaatcatgacattacgttggatgtcagccgccgtatatacgaagccgcccgctaagctttttacgcctcaaactttcgttttcgggcatttcgtccagacttaagttcacaacacctcaccggagcctgctccggtgagttcatataaaggaggaacgtatggctaatccaaccgttattaagctacaggatggcaatgtcatgccccagctgggactgggcgtctggcaagcaagtaatgaggaagtaatcaccgccattcaaaaagcgttagaagtgggttatcgctcgattgataccgccgcggcctacaagaacgaagaaggtgtcggcaaagccctgaaaaatgcctcagtcaacagagaagaactgttcatcaccactaagctgtggaacgacgaccacaagcgcccccgcgaagccctgctcgacagcctgaaaaaactccagcttgattatatcgacctctacttaatgcactggcccgttcccgctatcgaccattatgtcgaagcatggaaaggcatgatcgaattgcaaaaagagggattaatcaaaagcatcggcgtgtgcaacttccagatccatcacctgcaacgcctgattgatgaaactggcgtgacgcctgtgataaaccagatcgaacttcatccgctgatgcaacaacgccagctacacgcctggaacgcgacacacaaaatccagaccgaatcctggagcccattagcgcaaggagggaaaggcgttttcgatcagaaagtcattcgcgatctggcagataaatacggcaaaaccccggcgcagattgttatccgctggcatctggatagcggcctggtggtgatcccgaaatcggtcacaccttcacgtattgccgaaaactttgatgtctgggatttccgtctcgacaaagacgaactcggcgaaattgcaaaactcgatcagggcaagcgtctcggtcccgatcctgaccagttcggcggctaacatgcaaattctcccggtggcggtaatgttccgctaccggacttttcagaaatcatttattcccctcgcgtcccgcccgttgttactcttccttgttcaggaatgccaaatataaggacatcatcatgcagagccggaagctcttaaaagaacaactcatctatatccgggataaacgcaacggagaggtgaaaaacagatgaaaataatacttctgtttttagcagccctggcaagttttaccgtacacgcacagcccccctcacagaccgtagaacaaacagtccggcatatttatcagaactataaatcagatgccactgccccttattttggtgaaaccggagagcgggcgataacttctgcgcgtattcaacaggcgcttaccctgaacgacaatcttacgctgccgggcaatattggctggctggattatgatccggtttgtgattgtcaggattttggcgatctggtgctagaaagcgttgcgataacccaaactgacgccgatcatgccgatgccgttgtgcgctttcgtatctttaaagatgataaagaaaagaccacgcagacactgaaaatggtggcggaaaatggtcgttgggtcattgacgatattgtcagcaatcatggcagcgtcttacaagcagttaatagcgagaatgaaaaaacgctggccgctttagcttcgttgcaaaaagaacagccggaagcctttgttgccgaactctttgaacatattgctgattatagctggccgtggacgtgggtggtttccgactcttaccgccaggcggttaatgccttctataaaaccaccttcaagacggccaataatcccgatgaagatatgcaaatagaacggcaatttatttacgacaatccgatctgttttggcgaagagtcgctattttcacgcgttgatgaaattcgagtcctggagaaaaccgccgattccgcccgcattcatgttcgttttacgctgaccaatggcaacaacgaagagcaagaactggttttacagcggcgcgaaggcaagtgggaaatcgctgattttatccgcccgaacagcggcagcctacttaagcagattgaggcaaaaactgccgccagattaaagcaatgagctgaattaaataacaattagccggaacaataaataaaagggaacactatatgaaaacgattttcaccgtgggagctgttgttctggcaacctgcttgctcagtggctgcgtcaatgagcaaaaggtcaatcagctggcgagcaatgtgcaaacattaaatgccaaaatcgcccggcttgagcaggatatgaaagcactacgcccacaaatctatgctgccaaatccgaagctaacagagccaatacgcgtcttgatgctcaggactattttgattgcctgcgctgcttgcgtatgtacgcagaatgataaaaaaatccccggtagcgtgtcagttgccggggatattttttaacgtccaaccgccgctttaggccgtttcttcgcaccagcattcaccggacgagattgcgtagacgacgctttttttgccgtagcaggcgtctgacgctgggtcgccatcggcgtatgtttcgtcaacgccggacgggtattgcggttctggcgacgagcttcacgcatctcttcaatggttggcgcaggcactaagcaatcgcgacggctgccaatcagatgctttttgcccatcgcttccagcgcctggcggattaacggccagtttgccggatcgtggtaacgcaacaacgctttatgcaaacgacgctgtttgtcgcccttcggtacgaagacgtcttcgctcttataaccaatcttcgccagcgggtttttcccggtgtaatacatggtggttgagttcgccagcggcgacggatagaagttctgcacctggtcgaggcggaagcggtgctttttcagccacagcgccagattcaccatatcttcatcacgcgtaccggggtgcgcggagatgaaataggggatcagatactgctctttacctgcctgttttgagtaagtatcgaacagctctttaaagcggtcatagctgcccatgcccggcttcatcatcttcgataacggcccttcttcggtatgttccggggcaatcttcagataaccgccgacgtgatgggtcgccagttctttgatatagcgcggatcttctacggctatgtcataacgcacaccagaggcaatcaggatctttttaatgcctttcagatcacgcgcacggcgatagaggttgatcgttggttcgtggttcgtgtccatgtgcggacaaatatccggataaacgcacgacaaacggcgacaagtttgttcagcgcgtggcgatttgcagcgcaacatatacatgttggcagttggcccaccaagatcggaaatcacgcccgtaaaacctggaacggtgtcgcggatcgcttcgatctcattaatgatcgaatcttcggaacggctctgaataatgcgcccttcgtgctcggtgatagaacagaaagagcagccgccaaagcagccacgcataatgttgaccgaaaaacggatcatttcgtaagccggaatacgggcattgccataggccggatgtggcacgcgcttgtatggcagcgcaaaaacgctgtccatctcttcggtagaaagcggaatagcaggcgggttgatccacacatagcggtcgccgtgtttttgcatcaatgcgcgggcacagcctgggttggtttcgtggtgcagaatacgcgaagcatgggcgtacagcactttatcgcccttcactttctcgaaagaaggcagcaacacgtaggttttttcccacggtttcgggcgcggtggctgcacggttacggctttggcttcctgctttttcggtgccaccggtttgttatccgcgcacggcaaatcttcaccatacggatgcgggattgggtcgatttttccaggggtatcaagacgggtggaatccacgccgctccagccaggcagcgcctctttcacgataatcgcggtattacgcacatcgcggatttcactaattggctcgcccatcgccagacgatgcgccacttccaccagcggacgctcaccgttaccaaacatcagcatgtcggctttcgaatccaccagcacggaacggcgcacggtatcggaccagtaatcataatgcgcggtacggcgcagactagcctcaataccgccgaggatcaccggtacatctttccacgcctctttacaacgctgggtataaaccagtgtggcgcgatccgggcgcttacccgcgacgttatccggcgtgtaggcatcgtcatgacgtaaacggcgatcggcggtataacggttgatcatcgaatccatgttgccagcagtaacaccgaaaaacagattcggtttacccagacgcataaagtcgtctttgctgctccagtccggctgggcgatgatcccgacgcgaaagccctgcgcttccagcatacgaccgcaaatcgccatcccgaagcttgggtgatcgacatacgcgtcgccagtaaccaaaatgatgtcgcagctatcccagccaagttgatccatctcttcacgagacatcggcaaaaacggtgccggtccaaaacaggcggcccagtactgcggccaggagaacaggtcgcgatccggttggatcagggagatagagctcattttgcttccagaaatgataaaaaaataatcaaaggccggggattataagccggaacgaaagagaaatcgaaaggtattccatactcgccctcctcgggcgagtatgaagattacggtaccggattgaccaacagttgcccaatcgagccacggtccgccatttccagcgtctgactgttgaagtagaacgggaagtgcgcccaggaaggctgaccgaaataaacaagcagctccacttgtccgtcaacccaaacggtatctttccagcctctgtcttccgggaacggcatcgcgccattcacgttacggatctggaacattacgccttcaatatggaacgcttgcggctcgtccgcgcgtaccgtccagcgttcccacgttccttgctgcgcggtgacatcaatacggttgacgtcccacagctgtccattaatacccgggtcatcacccagactgatatcgcgactgcgaattggcgaaccagccatgatttcagttggcagcaagcgcatcggaagactgtctgtgaccagcggcagaaggccggttgggcgcagcgttagcaccagggtagaaaccagaatactggatggctcaaagaagccacgaatacgatcaacaatgctcgccgcttcgccacaggtgatcgacacttcatcgccgttgctcatatccaccagaatctcgcggcgctcgcccggtgccagcgaaagttgcttcaccgatacaggagcaggcaggaatccctgatcgccagaaatcacatgtaacgggcgaccatcgttcatctgtagttgatagcgacgagagttcgacgcgttcagcagtcgcaagcgcacccagccacgcgagacttcaacgtacgggctttgtacaccgttaaccagcagcgtatcaccaacaaagccgccgcttcccggttcgttgtattctggcgtaccaaagttatccagccgtttatcctggataatgaccggaaaatcatccacaccataatggttggggataggcagcgacttgctgacttcatcttccaccagccacattccggcaaggccgttatagacctgctgagccgtgcggttgggagtattggcgtgataccacagagtagctgcgttctggcgaatgggcagtacgggtgcccagtcagcgtttggcgacatcatccgtgccggaccgcccatcagcgggcctggtacctgtagcccggccaccgtcattgagacattttctgtcaggcggttgctgtaaataagcttaacatcgtcgcccttccagacgcggatagtcggccccaggtaacgaccattgattccccagaccgacgcgcgtgtccctggcgtaaatgaccagtgcgcacgttgtacagtcataaacagcggttgcccacggcgagattcaagtagcggcggaacgggtagcggttgctgttgcccggctgcgctggccttcaggggaacagcgcctgcacaaagtgcaatccccgatgcctgaatgaactgacgccgactgagtgacatatttgctccatgtaaaactggctaaagtaataccgtgcaggaaagtgttccccgcaaaaatacagattgccgacttaaacttttccggcggcttcgcgttctgcgacttctttatcgagctcggcgattttttgttccattatcgaacgacaatgggcagccagctcacgaacctgatctttgccatactgactgacgtcaattggcggcagcatttcgacaatcaccagaccgttgtgcagtcgattaagattaatcttattcgaagttgtagagacgcacacgggaataatcgggacgcccgccgcaattgccgcgtgaaatgctccagtcttgaacggtagcaggccgcgaccacggctgcgggttccttccgggaacatccagatggaaatacggcgttttttgaagtgattcactacttccgcaatggtgccgtgagctttagtgcgattgtttctgtcgatcaataagttgccggttaaccagtacaactgcccgaagaaggggatccacagcaagctctttttacctaccgtcaccgtcggcggttgcacgatgttcgatgctgtcaccatgtcatagttgttctggtggttagcgatatagatagcattgccgtagctttcagcgtctgtaggtttacggcactcaactttcaggccaaacagcggcgcaagacggccaaacatatgcccaaaggtggccacatgtttcgggttacgcgggctgaaaaggcagtaaatggagccgaatacacagactaagatgctgtaaatcacggtaataataagacgaaagatatatagcataacaccctctgaaggtctgagagactggcattgtacgtcacctgaaatcaggttagggcattgttaaaagccgctctctggaaaagcgtattgttaatcgcaacgcatgaataaacaacggtttcaagggaatttttatcgtttccgggggttgaatacgctgccggatgacgacttaacgtttcatccggcgttccttgcaagcgggaggaaacagcgccctccccggcatattactcttcgctatcaccgctgctggcacggcgaggagagtcgatctcaacacgatcgatacgctgcaaaccgcgcatcaacgtaccgcggcgtccacgttcgccagtgactttctgtaactcttccgggcgcagtttaattttgcgtttcccaacatgaatggtcagcgtgctttgcggcggcagaacgtacaattgcgccagaccatcttctccacgcgcggcttctgccgatggaatgttgataatcttgttgcctttgcccttcgacagctgcggcagatcacttaccgggaacatcaacatacggcctgcctgagtgattgccagcagcatatcggaagcatcttcaatcaccaccggcggcataacatgggcattttccggtaaggtgatcaaagccttacctgcacggttacgcgccaccagatcgttaaaggtgcagacgaaaccgtaacccgcatcggaagccatcagcagtttctgatcgtcgctttccatcagcatatggtcaacggtcgccccaggcggcaacgttaatttgccggtgagcggctcgccctgaccacgcgccgacggcagcgtaatcgggtcaatggcatagctacgaccggtggaatcaacaaacactaccggttggttgctcttacctttcaccgccgctttgaagctatcacccgctttataattcaggcccggcgcgtcgatatcatggcctttagcgctgcgtacccagcccatctgcgacagcacaatggtgacaggttcagacggcagcatgtcgtgctcgctcatcgctttcgcttcttcgcgttcctgcaacggcgaacgacgatcgtcaccgtaggcttgcgcgtctgcctgcagttctttcttcagcaggttattcattttacgctcggaagccaaaatgccctgcaactggtcgcgctctttttccagttcactctgctcaccgcgaatcttcatctcttccagtttggcaagatgacgcagtttcagttcgaggatcgcttccgcctgggtttccgtaaggccaaaccgcgacatcagcgccggtttcggttcatcttcattacgaatgatctcaatcacttcgtcgatattgagaaacgccaccagcaaaccttcgaggatatgcaggcgcttgaggactttctccagacgatagttcagtcggcggcgcacggtatcgcggcggaacaccagccattcggagaggatttccagcaggtttttcaccgccggacgaccatccagaccgatcatattaaggttaatacgatagctcttttccagatcggtggtagcgaagaggtggttcatcacctgatccatatccacgcggttggaacgcggcacaatcaccaggcgggtcgggttctcgtggtcagattcatcgcgcagatcgtcaaccatcggcagctttttgttgcgcatttgcgcagcaatttgctccagtacgcgcgcacctgaaacctgatgcggcaatgcgctgataaccaccgcgccatcttctttcttccacaccgcgcgcatacgcactgaaccacgtccgttctcgtagattttacggatctcggcgcgcgaagtgataatttccgcttcagtcggataatccggcccctgcacgatatccagcagctgatcgagcgtggttttcggctggtcgattaatgcgattgccgcctgagccacttcacgcaggttatgcggtggaatatcggtcgccatgccgacggcaataccggtggtgccgttaagcaaaatgtttggcagacgggcaggtagcattttcggctcctgcaaagtgccgtcgaagtttggcacccagtcagccgtcccctgccccagctcgctcaatagcagctcggaatatttcgacaaccgggattcggtgtaacgcattgccgcgaacgatttcggatcgtccggcgcgccccagttcccctgaccatcaaccagcggataacggtaagagaacggttgcgccatcaggaccatcgcttcataacaggcgctatcgccgtgcggatggtatttacccagtacgtcaccgacggtacgggccgattttttaaatttggcgctggcattcaggcccagttcagacatcgcatacacaatgcggcgctgaacaggtttcagaccatcaccaataaacggcaacgcacggtccatgatcacgtacatggagtagtttaagtaggcgttttccgtaaattcatgtagcgcaaggcgctctgccatatcgctcattaattctgattcctcaacttattcgccagccttcaaaggggcaatattgccggagatactacattatctgccgcgtcgagtcacaggagatcaacgtgaatagcgccgccggacgtgctccgacggcgataaaggcatcaatgtgccttgatatacaactctttgctgtagacataatcctggggattatgcagcggaaaaccgccaacgtagggtttaagcagtttgattaacggctgatagtagataggaatcagcggtgcctgttggttgatgatcacttctgcctgctgatacaacgcattacgctttgtcgcatcagtgatctgcgtggcctggtttagtaaggcgtcatactgcgcatttttccagtgaccgacgttttcttcactatcgcttttgagcgtgttcaggaagctggaagcatcattgtacgtcgcatcccacgactgccgagacagcatgaaatcaccggctcgtcgggcatcaagataggttttccactccattgtgcgcagcgtcacctgtgcacccagccattttttccattcggaagacaacgctatcgcggtcttttcatgcagatcgtacttgttgtagaacagctcaaagcgtagcggatgagaggcgtcgtatcccgcctgtttcagcaaggcttttgccatcgcgacgcgctcactcattggcttttgcagttcatcgaacgtcgtcgcgctaaagccttttacctctggcggcgtcagcgtggttgcgggcgttctcaaccccagtaccttttgcgcaataagctgtcgatcaaccgtaagatatagcgcccgacgcactcgcacatcgttaaatggcggtttctcaaggttgaagttgtaatattcgctgttcagacgcggaataattcgtagctcgccaggcagtgatttttcaatggcgggaatttgctgcgccggaacccaggtgagatcgacctctcccgcgcgatagcggttatagccggtgaccgaattatctagcgccagatactcaacctgttgcaatactgtatgttgcgcatcgcggtactttggatttttgcgtgcagtaatcttttcgttaactacccactgatcaagcacaaaggcaccgttgtaaaccatgttctctggcttactccagctatcgccatgtttagcgatgacatgatgaggaaccgggaacagcgtcggccaggcgagcatcgtcgtgaaccaaggaaccggctgctcaagcgtaacttcaagagtacgatcatccgtcgctttgacacccagcgatgtaacatctgctttacccgcaacaatagctgcggcattgttaatgtgcgcctgtgccagatagccagcaaaagggcttgccgttttcgggtcaaccgcgcgctgccagccgaggacaaaatcctctgccgtcagaggctgaccgtcggaccactgcaaaccgctacgcagatggaaaatatagcgcttgccgccgtccagtatctcccagcgttcagcctgagcgggctgcacctggccttcaccgtccatccataccagaccttcaaacagatccagcacaatctgcgcggcagtattctcctccaccttttgcgggtcgagcgtacctgggtcgctatgattgttgtaacgaaagacttgttgcggggcgagcggtgtgttggcgggaacgtcagcagcgtagagaggagccgcacttaccaggctgaccagccataataaatttcgcgtatacatggtattccttaccggagaaattataagcccaacaacaatacgcctgtggcattgttcgctcaaacttatcgcgagtgatttggctcacactccggtaaagaaaaaagcgagttgcccccgcttttccattaattaacggatttcattcaatagttctggatgcttatccagaacacgtaaaagtttgattgtggaaggatgaggttgggcattgcctttttcgtaacgcgaaaacgcatttacacctcccccaaaaatttcgcttgcctctttttgggtaagagagagcttttttcgaaccttcactataaattcaggtgccactgtttcggcattcaccgaagcccgaaatgcctttacttgcgccatgaaagcatctgactcttctttattcatgatgctctcttcgcaatggacacaatataaaccgtggatacctttcaatactgtttttcgtccacggaaggtgtatggaatatctttaatgccagaaaccatttctccctggtggcaaaccggacatttcatattacttctccttaaacgagacgatcagtacgtcatgaattaccgtaattttaagataaacctggcctgtaacaagcctgggtctgtaaacatcctgccagatagtatgatcagagtaggtggtcatgcttttataaaagtcgctctctgataatccaatgataacattacacataccatcaaaatccaaacctaactcatctgcatttaacagggcactacgtgttgtacgaacttgcccggcattgacaagttttttaacctgactcaaacgtgtatgtggtgtgcgtttttccataacccccgcctccctgttactttagttataacctaaaaggttaattacagcaatgaaaaagcacctaaaaggttagttagatgtacggagatagtgaccacacaaaacgtattctttaaggaaagtgattgaccatataagaaagtggcgcattagtagcgccagtttgaagcaggaatttataagggaagctggagtcaggcatcacgccaacggcacataaacatccgtttccagtcgctgctctgtcaccccttcggcaagattggtgtagtgaaacagaatcggtgctttacgcattttctcgccgcttgcaggcagccagtggcgaatgatgccccataccgtgtgtgaaatatcgtccagctcgccaacgtggcgggccacggcataacgtccaccggtaagttcaccattgctcacaccataacgattatcgggaatcggttcgctaacgctgccgcagatatcaaagcgaaacgcttccggtgcggtggtggcagggtcgtcccaggcgacgccaaaagtctggctttggttaacaggagaaagccccgtctctttacgccacatgataaatttcgccacgctgtagttgagcaattcagggctacagcggtgcggcaacatcgccacaggtattgatgggaaatcgataatgtttacatccagtgtcaggtttgtcattttgcctccctgcgaaattattcccgggaacgcgtcccgggagcggtaacaattacggatttactttgcggatctgtttgacgtcaatttcaacagaattccagtctttatcgacttcaccctgaatctcaaccgtatctttcggcgtcaccgtcacgccgttccagcgtttgtggtcgatatcaacattgatagtaccgctggcatctttgaacacgtagagatcgtcagagatgcgttcaacgatattgccgcgcagggttacccaggtgtcgtcacgcagggattttgcgctttctacagtcgttacgctgccgttcggcccctggaatcctccggcctgactttgcgttgccgatgggccagaaaaaccgccctgctctgctgccatcaccggtgcgctgcacagggccattactgcgattactgctgcgaattttttcatgtttattactccctttaatgtctgtttccgagcatttaacaagatagtccttaacaacttcttaagggaaaaaaataaaatttagtgctgtacagagcgcgttacaacacggtttactggcagcaaatacggttatcgcagggatgaaaaaatgcgaattttactgatagaagatgacatgctgattggcgacggcatcaaaacgggccttagtaaaatgggttttagcgtcgactggtttacacaaggtcgtcagggaaaagaggcgctttatagcgcaccttatgatgcggtgatcctggatttaaccttaccaggcatggatggtcgcgatattttgcgcgaatggcgagaaaaaggtcagcgtgagccggtactgatcctgaccgcgcgcgatgcgctggcggaacgtgtagaagggctgcgtctgggagctgacgattatctgtgtaaaccttttgcgttgatagaagtcgccgccaggctggaagctctgatgcgccgaaccaacggccaggccagcaacgagctgcgccacggtaacgtcatgctcgaccccggcaaacgtatcgccacgctggctggcgaacccttaacactgaaaccaaaagaatttgccctgctggaattactgatgcgtaacgctggtcgggtactgtcgcgcaaactgattgaagagaaactgtatacctgggacgaagaggtcaccagtaatgccgttgaagtgcatgtgcatcatctgcgacgcaaactcggtagtgattttattcgtaccgtgcatggtattggttacacattaggtgagaaatgaaatttacccaacgtcttagtctgcgcgtcaggctgacgctaatctttttaattctggcctcggtgacctggctgctttccagctttgtcgcctggaaacaaacaacggataacgtcgatgaattgttcgacacccaactgatgctgtttgccaagcggttaagtacgctcgatctcaacgaaatcaacgcggcggatcgcatggcacagacgccaaatagattaaaacacggtcatgttgatgacgatgcgctgacctttgccatctttacccacgacggcagaatggtccttaatgatggcgataacggagaagatattccctatagctatcaacgggaaggttttgctgacgggcaactggtcggtgaagacgatccttggcgttttgtctggatgacctcacctgatggcaaatatcgcatcgttgttggccaggaatgggaataccgtgaagacatggcgctggcgattgttgccgggcaattgatcccgtggctggtcgcactgccgattatgttaatcatcatgatggtactactgggtcgtgaactcgcgccgctgaacaaactggcgctggcactacgtatgcgtgaccctgactcggaaaaaccactaaacgcgactggcgtacccagcgaagtgcggccactggttgagtcgctaaatcaactgttcgcccgcacacatgcgatgatggttcgtgaacgacgctttacctccgacgcagctcacgaacttcgtagcccgttaacggcgctgaaagtgcaaaccgaagttgcgcagctctctgacgatgatccgcaggcgcggaaaaaagcactgctccaattacattccgggatcgatcgcgctactcgtctggttgatcaactgctcacgctatcgcggctggactcactggataaccttcaggacgtcgcggagatcccgcttgaagatctcctgcaatcgtcggtgatggatatttaccacacggcgcagcaggcgaaaattgacgtgcgactgacactcaatgcccacagcatcaaacgcaccgggcaaccgctattgctaagtttgttggtgcgaaatttgctggataacgccgtgcgctacagtccacagggcagcgtggtagacgtcacgctgaatgctgataatttcatcgtgagggataacggccccggtgtgacaccagaggcactggcgcgaattggcgaacgcttctatcgcccacccggacaaaccgctaccggcagcgggcttgggctatcgattgtccagcgaatcgccaaattgcatggcatgaatgttgaatttgggaatgcggaacaaggtggatttgaggcgaaggtaagctggtaacttctctgtctatgagagccgttaaaacgactctcatagattttactaatagcaaaatataaaccgtccccaaaaaagccaccaaccacaaaccagacaaataccgagcgagaatacatatacccaaaactcgaacatttcccgcataaagagttttcttaagataagaataataagtggcgtaagaagaaaaaatgctgcaatcattgcttgcaatatacgatcttcgcctgaaacggaaggtatactgcaaatatttcctcccgactcaagcatccagtcatacttattgaaagcaaaaaaagaatctattaaccaataagtaagcattatatatagcaatgcttcaaatattgttttaattttctgctttaacatatatcagtacgctcataaaaatccatttataattatcaacatgacacgttgatactttcatcttttacttattcaaagccatattttcaatccccaaaaaaaccgaaccaaacgtgtaaattattccggtgcgagtaagaattatgaggaatggctatcagtattgtcattttcagaaaatatttatcctgcatcggtgagtcagagtaagatcagacttttgctaaattcgcaaaagactttgcacattttgctaatttcaccgtaccgctctgtgacgtactatagtcggcaaacgtctcaccttgaggttaaaaaatgagcaacatcctgattatcaacggcgcgaaaaaattcgcccactccaatggtcaactgaacgacaccctgaccgaagtcgcggatggcacactgcgcgaccttgggcatgatgtccgcatcgttcgcgccgacagcgactacgatgtcaaagcggaagtacaaaactttctctgggctgatgtggtgatctggcagatgccaggctggtggatgggcgcgccgtggacagtgaaaaaatacattgatgatgtattcaccgaaggtcacgggacgctgtatgccagcgatggtcgtacccgcaaagatccgtcgaaaaaatacggttccggcggcctggtacagggcaaaaaatatatgctttctctgacctggaacgcaccaatggaagccttcaccgaaaaagatcagttcttccacggcgttggcgttgacggtgtgtatctgccgttccataaagcaaaccaattcctcggtatggaaccgctgccgacatttatcgctaatgacgtgataaaaatgcctgatgttccccgctatactgaagaatatcgcaagcatcttgtggaaatttttggttaactagagctcaggctttagaaggagttaaccatgcttaccgtaatcgcagaaatccgtactcgtcctggtcaacatcaccgtcaggcggtattggatcagtttgctaaaatcgttccaaccgtactgaaagaagaaggttgccacggctatgcgccaatggtggattgcgcagctggcgtgagtttccagtctatggcaccggattctatcgtgatgattgagcagtgggaaagcatcgcgcatcttgaagcgcatctgcaaaccccgcacatgaaggcgtatagcgaagccgtaaaaggtgacgtgctggagatgaatatccgtattctgcagccagggatttaatcctgccttgtttgcccggccatcctgaccgggcaatgttctttcctttaaacctcaatctccgccatgtcgcctttctcttgcaaccagttgcggcgatcttccgagcgtttcttcgccagcagcatatccatcatcgcgtcagtacgctgatcgtcttcatcatcgatagtcaactgcaccagacggcgagtgttcggatcaagcgtggtttcgcgcaattgcatcgggttcatttcccccagacctttaaaacgctggacgttcggcttgcctttcttgcgttttaattgctcaagtacgccctctttctcttcttccgtcagcgcgtaataaacctctttcccgagatcaatacggtagagcggtggcagtgcgacgtaaacgtgaccgtgtttcaccaacgcgcggaaatgttttacgaacaaagcgcagagcagcgtggcaatgtgcagaccatcagagtccgcatccgcgaggatacagattttgccataacgaagctggctcagatcgtcgctgtcaggatcgataccgatcgctaccgaaatatcgtgcacttcctgcgaagccagcacttcgtcggaagagacttcccaggtgttaaggatcttacctttcagtggcatgatcgcctgatattcgcgatcgcgcgcctgcttggcagatccgcctgcggagtcaccttccacaaggaacagctcggtacggttaaggtcctgcgcggtacaatcagccagtttgccaggcaacgccgggccgctggtcagctttttacgcaccacttttttggccgcacgcatacggcgctgggcgctggaaatcgccatctccgccagcagttcagccgcctgaacgttctggttcagccacaggataaaggcatctttcaccacgccagaaacgaatgccgcgcattgacgcgaagagagacgctctttcgtctgcccggcaaactgcggatcctgcatttttactgacagcacataggcgcagcgatcccagatatcttccgccgacagctttacaccgcgcggcagaatattgcggtattcacagaactcacgcatcgcgtccaacaggccctgacgcagaccattaacatgggtaccgccctgcatcgttgggataaggttgacgtagctttcggtcagcagttcaccgccttccggcagccacagtagcgcccagtccacagcttcagtatcaccagcgaaattaccgataaacggtttttccggcagcgtcggcagaccatttaccgcttccgccaggtaatcattcagaccgtcctgatagcaccagcgttgttcggtattgttgatctcatctttaaaagtgatctcaacgccagggcacaataccgctttggctttcagcacatgcgtcaggcgtgaaacagaaaatcgcgggctgtcaaagaaggtttcatccggccagaagtgcacactggtaccagtattgcgtttaccgcaagtgccgacaacctgtaaatcctgcaccttttcgccattttcaaaggcgatgttataaacctgaccatcgcggcgcacgttaacttctacgcgcttcgacagggcgttaaccaccgaaatccccacgccatgcaggccgccagagaactggtaatttttgttagagaatttaccgcctgcatgcagacggcaaagaatcagttcaaccgccggtacaccctcttccgggtgaatatccaccggcatcccgcgcccatcgtcaataacttctaacgactggtcagcatgtaaaataacgtccacgcgttttgcgtgacccgccagtgcttcatccacactgttatcaatgacttcttgccccaaatggttagggcgagtggtatcggtatacatccccggacggcggcgaaccggctcaagcccggtgagtacctcaatggcatcagcgttataagtttgcgtcatggtttaagttagtaattcgagttgatcgtcagagatggtgcagaccaagaaaatcgacgatcgggttgaaataatcttcgaagcccgtgaatgcgtggttgccgccttctatgacagtctggcggcaggaagcgtagtacgccaccgcctggcggtaatccagcacttcatctcccgtctgttgcagcagccagatcaaatccggcgcttccagcgggtcaatctgcatgactttaagatcgtaaatatggcgtgactctagcacatattgctgcccggtgtaggggttctcgttctgaccgagatagtccgtcagcagttcaaacgggcgcaccgccgggtttaccaccactgcgggcagcataaaacattgtgacaaccaggtggcgtaatatccccccagtgacgaaccgacaatacccagcgaatcaccgccatgttccaggacaatggattccagcagctctgccgcgtcggaaggatacggcggcaactgcggaatgatcatctcaacgtcagggtgatgttccgccagccagttttttaacaagctcgcttttgcagagcgcggcgagctgttgaaaccgtgtaaataaagaagcgtagacatcagtagccttctgaagcggtatcaggttggaaacgtgtgtccgccaggcgatgcacctcggtggtcagcgtgccatcagcatgtaactcgagagtacgccagccgggcgcgatggtatccagcgtaaagttggaacagtgcggcttaaactgcacacaggtcgacggcgttgccagcaggcggcgaccattccagtcgagatccagctcctgatgaatatgaccgcacagcaagtatttgacgtgcggaaacttcgccagcacggtatccagttcgcccgcgttacgcagactgtgttgatcgagccaactacaacccgcaggtagcggatgatgatgcagcagcagcaacgtatggcgttctggcgcatcggccagtttacgttccagccactcaagctgaaactcgctcagctcaccgtgcggcacgccaaacacctggctatccagcaacaggatttgccattgctcaccaataaacacgcgcttcgccggggagatacccgcatcctgtaacgcgctgtacatcgcgggctggaaatcgtggttgcccggcagccagacgcagggcgcacgaaaacttgcgatgccttcagcgaaatgctgataggccgcagaggattgatcctgcgctaaatcacctgtcgcgacaatcaggtcgaattcgtgctggtgtggccgaatcgcctccagcaccgcctggtaactctcccaggtgtttacccctaacagggcttcgtgcttttgtgcaaacaggtgagtgtcggtaatttgtaaaatcctgactctggcctcaccagccagaggaagggttaacaggctttccaaatggtgtccttaggtttcacgacgctaataaaccggaatcgccatcgctccatgtgctaaacagtatcgcaaccagtccgctaaaaactgattaatttgatgcttttcgtcgcgttgatgcaactttttattaggataatcataccgcgctttgaagcgaaaaatctgctggcttgaacacacttcagccaccatcgcgtcatgatacagacgcaccgtcattgacggaaggctccagtaactgatcgcgggcgcagtctgttctattgtcaccagggtagtgtatcgggtcgattccacaatcgtcagccgatattgtgcgtttgccacctgatagcttacagtttcgccgggtgcgtcattgcgcggtaacaaacggcgcaattgtgaaaagttcatctcgcacaggcgcatcatttcaggaaagtcaggtgtgtaacgcttcatttatgcccactcattttttaacgcttgatgatgcagctgcagccattgcaaagcgatgaccgacgctgcgttgtcgattttcccctcttctacccactggtatgcctgttcccggcttaccacatgaacgcgaatatcttcgttttcatcagccagaccgtgaataccgcttgcggtcgtggcgtccacttcgcccaccataattgacgaacgctcactggtgccccccgggcttgccaggaaacttaacaccggtttggtccgtttgactatcagtcccgcctcttcaatcgcttcgcgacgggcaacatcttccacactttcaccctcttcaatcatcccggcaaccatctccagtagccaaggggtttcgctggtgtcgtacgcggcaatccgaatctgctcaatcagcacaacttcatcacgcactgggtcaaagggtagcaagactgcggcgtgaccgcgctcaaaaatttcccgccgcacctcatgactcatttgcccgttgaatagacgatgacgaaatctataaagatctaatgaaaaaaagccgcgataaagtgtttctcgtgcaataatttctacatcgtttttgccaaatgtaacgggcaggttgtctggcttaagcattgttaatgtcctggcactaatagtgaattaaatgtgaatttcagcgacgtttgactgccgtttgagcagtcatgtgttaaattgaggcacattaacgccctatggcacgtaacgccaaccttttgcggtagcggcttctgctagaatccgcaataattttacagtttgatcgcgctaaatactgcttcaccacaaggaatgcaaatgaagaaattgctccccattcttatcggcctgagcctttctgggttcagttcgttgagccaggccgagaacctgatgcaagtttatcagcaagcacgccttagtaacccggaattgcgtaagtctgccgccgatcgtgatgctgcctttgaaaaaattaatgaagcgcgcagtccattactgccacagctaggtttaggtgcagattacacctatagcaacggctaccgcgacgcgaacggcatcaactctaacgcgaccagtgcgtccttgcagttaactcaatccatttttgatatgtcgaaatggcgtgcgttaacgctgcaggaaaaagcagcagggattcaggacgtcacgtatcagaccgatcagcaaaccttgatcctcaacaccgcgaccgcttatttcaacgtgttgaatgctattgacgttctttcctatacacaggcacaaaaagaagcgatctaccgtcaattagatcaaaccacccaacgttttaacgtgggcctggtagcgatcaccgacgtgcagaacgcccgcgcacagtacgataccgtgctggcgaacgaagtgaccgcacgtaataaccttgataacgcggtagagcagctgcgccagatcaccggtaactactatccggaactggctgcgctgaatgtcgaaaactttaaaaccgacaaaccacagccggttaacgcgctgctgaaagaagccgaaaaacgcaacctgtcgctgttacaggcacgcttgagccaggacctggcgcgcgagcaaattcgccaggcgcaggatggtcacttaccgactctggatttaacggcttctaccgggatttctgacacctcttatagcggttcgaaaacccgtggtgccgctggtacccagtatgacgatagcaatatgggccagaacaaagttggcctgagcttctcgctgccgatttatcagggcggaatggttaactcgcaggtgaaacaggcacagtacaactttgtcggtgccagcgagcaactggaaagtgcccatcgtagcgtcgtgcagaccgtgcgttcctccttcaacaacattaatgcatctatcagtagcattaacgcctacaaacaagccgtagtttccgctcaaagctcattagacgcgatggaagcgggctactcggtcggtacgcgtaccattgttgatgtgttggatgcgaccaccacgttgtacaacgccaagcaagagctggcgaatgcgcgttataactacctgattaatcagctgaatattaagtcagctctgggtacgttgaacgagcaggatctgctggcactgaacaatgcgctgagcaaaccggtttccactaatccggaaaacgttgcaccgcaaacgccggaacagaatgctattgctgatggttatgcgcctgatagcccggcaccagtcgttcagcaaacatccgcacgcactaccaccagtaacggtcataaccctttccgtaactgatgacgacgacggggcttcggccccgtctgaacgtaaggcaacgtaaagatacgggttatctgccgcattcttcccccttctcgcttcaatttcgaccagccatcctctattctgatgggtatttaccactggtcccggaagacaaaaatgaaacggacaaaatccatacgccacgcatcgttccgcaaaaactggagcgcacgccatctgacaccagtcgctctcgcggttgccactgtttttatgctggctggctgtgaaaagagtgatgaaacagtgtctctctatcaaaatgctgacgactgttcagctgcaaacccaggcaaaagcgccgaatgtaccaccgcgtacaacaatgcgctgaaagaagccgaacgtactgcgccgaaatacgccacccgtgaagactgtgttgctgaatttggtgaaggtcagtgccagcaggcaccagcccaggctggcatggcaccagaaaaccaggcgcaggcccagcaatccagcgggagtttctggatgccgctgatggccggttacatgatggggcgtctgatgggcggcggcgcgggatttgcacagcagccgctgttctcctcgaaaaacccagccagtccggcttacggtaaatataccgacgcgacgggtaaaaactatggcgcagcccagccaggccgcaccatgaccgtaccgaagacggcaatggcaccaaaaccggcgaccaccactaccgttacccgtggcggttttggtgaatctgttgccaaacaaagcactatgcagcgtagtgcaaccggtacctcttctcgttcaatgggtggctgataccgatggaaagagtcagtattaccgagcgcccggactggcgtgagaaagcccacgaatacggtttcaattttcacaccatgtacggcgagccgtactggtgtgaagatgcttactacaagttgaccctcgcccaggttgaaaagctggaagaagtcaccgccgaactgcaccagatgtgcctgaaagtggtggaaaaagtgatcgccagcgatgagctgatgaccaaattccgcattccaaaacacacctggagttttgtgcgccagtcatggctgacgcaccagccatcgctttattcgcgtcttgatctggcgtgggatggcactggtgaacctaaacttctggaaaataacgccgatacgccaacgtcactatacgaggcggcgttctttcagtggatctggctggaagatcagcttaacgccggtaacttgccggagggcagcgaccagtttaacagtctgcaagaaaaactgatcgatcgcttcgttgagctgcgtgaacagtatggcttccagttgctgcatctcacctgctgtcgcgacacggtggaagatcgcggaaccattcagtatttgcaggactgcgcaacggaagctgaaattgctactgagttcctctacatcgatgatatcgggttaggtgaaaaaggtcagttcacggatttacaggatcaggtaatttccaacctgttcaaactgtatccgtgggaatttatgttgcgtgagatgttctcaaccaagctggaggatgcaggcgtacgctggctggaaccggcgtggaagagcattatctccaacaaggcacttctaccgctactgtgggagatgttcccgaatcacccgaacctgctgcccgcttattttgcggaagatgatcatccgcaaatggaaaaatatgtggttaaaccgatcttctcccgtgaaggcgcaaacgtgtcgatcattgagaacggcaaaaccattgaagcagcggaaggtccgtatggcgaagaagggatgattgttcagcaattccacccgttaccgaaattcggcgacagctatatgctgattggtagctggctggtgaacgatcaacccgccggaattggcattcgtgaagaccgtgcattgatcacccaggatatgtctcggttttatccacatatttttgttgaataagccacgataccggatggcactcgccatccggtaattgttagcctatctgcaccgacagcatactcaggctgcccatttctataccctcaaccggaatggtaattggctcctgcccatcccacgcacctaacacatacaacaacggcaaataatgctctggcgttgggttcgataacgtgccaccttcatggtcgaggtaattcaccagaggatgttgttccactggcccttgccacgtcagattcgctttcacatactcattaaacgacgtcgcccacggatacggtgaactatcaccgtgccacttcactgtgcgcaggttatgcaccacgttaccgctggcgaccaacattattccttcatctcgcagcgctgccagtttgcgccccatttcgaaatgccaggcggcaggtttgctactgtcgatactcaactgcaccatcgggatatcagcgtcaggatacatcttaatcagcacgccccacgagccgtggtcaaagccccaggcttctttatccagcgtcaccgggatcggcgctaacagctcaaccagacgctgtgccagcgcaggcgaacccggagcaggataatgcgtatcgtacagcgcctgcgggaagccaccaaagtcatgaatcgtgggcggcgtctccatcgcggtcactcctgttccacgggtaaaccagtgagccgaaaccaccacaatcgcttgcgggcgtggcaatgtcatccccaacttctgccagctgcgggtatacaaattatcttccagcacgttcatcggactaccgtgacctaaaaacaatgctggcatacgtgttgaagacatgatgatatccttaactaaaggtgtcattttgatatcctcacaatacgcttgttcggcggagtaagaacccggataacaatgatgatgatcatcagttattttgacgatctgcctgaaggtgaagatttataaggagttgtcgatgtcagtacctctcattctgaccatactggcgggggcagccacgtttattggcgcgtttctcggcgttctcgggcaaaaaccctcgaaccgcttactggcgttttcgctaggttttgcggcggggatcatgttgctcatctcattaatggaaatgcttcctgccgcactagcagctgaaggaatgtcgcctgtgttgggttatggaatgtttatcttcggtctgcttggctattttggcctggaccgcatgttgccacatgctcatccgcaggatttaatgcaaaaatcggtgcagccgttgccaaaatcgatcaagcgcacagccattctgctcactctcggcatcagtctgcataacttcccggaagggattgccacctttgtcacggcgagcagcaacctggagctgggatttggcatcgcactggccgtcgcgttgcacaatatccctgaaggtctggcagtggcaggcccggtttatgcggcaacggggtctaaacgcaccgcgattctgtgggcggggatttctggactagcagaaattcttggtggtgtgctggcgtggttaatcctcggtagcatgatttccccggtggtcatggcggcaatcatggcggcggttgcaggaattatggtggcgctctcggttgatgaattaatgccgctcgccaaagagattgaccctaataataaccccagctatggcgtactatgtggaatgtcagtgatgggattcagtttagtgctgctacaaacggcgggaattggttaaaaacaacatcagaagttgtccagcgcatggacaacttctgccagcttcacgaaagccttattctaccttttcggctgtctcttctctcgtactgtttaagtatttgttccgcgcttcaagcagtgcgtctctgtcctggcgaaacgcccgacaataacgtttcaaatgcaggaaataacccaccacaaccagagcaatcaatacaatccagtaccaggcgataaacatccttttacccttaatatttaacaatactaaacatttagcgtataaatttcacatatcctttttcggatatattcatatggtcgcataataacggaacaattatatgattttgatcataatgaaaaagaatgcctgatattaatgaaattttctcatagaaagagaagcggaattaacatcttgcatagcagggaaaaataaaaaccgaagcctgctacaacttcggtttcttgattaaggcagtaaattaagcagcggttttcagctggctttacgctcatgtgcctgacggtatgccaccaggtcttcaatagtcacgagcgccatattgtgtttattggcaaactcaatacactctggtgcacgcgccatcgtgccatcgtcattagtcagctcacacagtacaccagccggtttaaagcctgccagcgtcatcagatcaatagttgcttcagtatgaccgccacgcgtcagtacaccacctgcctgagcgcgaagtgggaaaacgtggccaggacgattcagatctgacggttttgcgccatcggcaatcgctgcgcgaacggtcgtaatacggtcagcggcagaaacaccggtagtcacaccttcagctgcttcaatggtcacggtaaaaccggtgccataggcgctggtgttattttctaccatcattggcagatcgagttgtttacggcgatcttcagtaatgcacaggcaaacaataccgctaccgtggcgaatggtcagcgccatctgctcaacagtcatggtttctgccgggaagatcatatcaccttcgttttcacggtcttcatcatcaagcaccattacaccgcgtccttcacgcagcgcagccagtgcattttcaacacgttcgaaaggcgtaccaaaagaggaaagtagcgtctgattcatggtaaaaaaacctcactaaaattatggttaccagaatcagggcagtcttaggagtggcggcatatagccaaaataacgtgagcgggtccatgcccgacagaatcgttactctctcccatccggactctaaccgtcggccccggaattacaccggatctgctgtcctttgagttcgcacccaaagcgctcgcgggctttcaactgagttgatttaccgccggtggggaatttcgccccgccctgagaataagcggattcactataacgctaatgattagcggcagcaacgcatagcttcacataattctggtttatgacttacccttatcgcactacaatggcactcaacacctatcagtacagggaaactacaatgattgacccgaaaaaaattgagcaaatcgctcgccaggttcacgaatcaatgcctaaaggaatcagggagttcggggaagatgtggagaaaaaaatccgccaaaccctacaagcgcagctgacgcgcctcgaccttgtaagccgtgaagagttcgacgtccaaacgcaagtcctgttacggactcgtgaaaaactggcgctgcttgaacaaagaatcagcgaactggaaaatcgcagtactgagatcaaaaagcagccagatccagagactctccccccaacgctgtaaacattcgtctttaatgcactgtaaattatgaattaatcctctaatttatagtgctttctattaccttatcgcgtaatcccattcagaaaaccatcacaaaaatgaatgagtacaattgaaagtataattgcaatgtattttttaagttttacttaatcgatatttagataaactaattttataaaaaacacaaaataaaatatcatatttcaatgattagtagtccttaaataacagttactaatcattctcttttctacttatctttatataaaggaatattatgtccgcttttaaaaagtcacttcttgttgctggcgtagcaatgattctttccaataacgtgtttgctgatgaaggtcacggtattgttaaatttaaaggtgaagttatctctgctccatgttctattaaaccaggtgacgaagatttaactgtaaatctgggtgaagtagcagataccgtactgaaaagcgatcagaaatctttggctgaacctttcactattcacctgcaggactgcatgctgagtcagggtggaactacttattcaaaagcgaaggttactttcactacagcaaataccatgacgggtcagtctgatcttctgaaaaataccaaagaaactgaaatcggcggcgccactggcgttggcgtacgtattctggacagccagagcggcgaagtaactttaggtactccggtagtaattacgttcaacaataccaacagctatcaggaactgaatttcaaagctcgtatggaatccccaagcaaagatgccaccccgggcaacgtttacgctcaggctgactacaagattgcttacgagtaatcgcatttggccgggttcgcccggccacatcattaacggattaatgataagtggatcagatgtataaaaaattaaaattaaccacaataagcgaattgattaaaaatatttattgttcattatccgttattagactggccccctgaatctccagacaaccaatatcacttaaataagtgatagtcttaatactagtttttagactagtcattggagaacagatgattgatgtcttagggccggagaaacgcagacggcgtaccacacaggaaaagatcgcaattgttcagcagagctttgaaccggggatgacggtctccctcgttgcccggcaacatggtgtagcagccagccagttatttctctggcgtaagcaataccaggaaggaagtcttactgctgtcgccgccggagaacaggttgttcctgcctctgaacttgctgccgccatgaagcagattaaagaactccagcgcctgctcggcaagaaaacgatggaaaatgaactcctcaaagaagccgttgaatatggacgggcaaaaaagtggatagcgcacgcgcccttattgcccggggatggggagtaagcttagtcagccgttgtctccgggtgtcgcgtgcgcagttgcacgtcattctcagacgaaccgatgactggatggatggccgccgcagtcgtcacactgatgatacggatgtgcttctccgtatacaccatgttatcggagagctgccaacgtatggttatcgtcgggtatgggcgctgcttcgcagacaggcagaacttgatggtatgcctgcgatcaatgccaaacgtgtttaccggatcatgcgccagaatgcgctgttgcttgagcgaaaacctgctgtaccgccatcgaaacgggcacatacaggcagagtggccgtgaaagaaagcaatcagcgatggtgctctgacgggttcgagttctgctgtgataacggagagagactgcgtgtcacgttcgcgctggactgctgtgatcgtgaggcactgcactgggcggtcactaccggcggcttcaacagtgaaacagtacaggacgtcatgctgggagcggtggaacgccgcttcggcaacgatcttccgtcgtctccagtggagtggctgacggataatggttcatgctaccgggctaatgaaacacgccagttcgcccggatgttgggacttgaaccgaagaacacggcggtgcggagtccggagagtaacggaatagcagagagcttcgtgaaaacgataaagcgtgactacatcagtatcatgcccaaaccagacgggttaacggcagcaaagaaccttgcagaggcgttcgagcattataacgaatggcatccgcatagtgcgctgggttatcgctcgccacgggaatatctgcggcagcgggcttgtaatgggttaagtgataacagatgtctggaaatataggggcaaatccagttatcatcattggttgtgcgtcagcttatgccgttgaattcaacaaagatttaatcgaagccgaagatcgtgaaaacgttaacctttcccaatttgaaactgatggccaattacccgtcggcaaatattcactaagcactctgattaataataagaggacgccaatccaccttgacctccaatgggtattaattgataaccaaactgcagtttgcgtgacaccagagcaattaacattattaggatttactgatgaatttattgaaaaaactcagcaaaacctgatcgatggttgttaccctatcgaaaaagaaaaacaaattacaacttatctcgataaagggaaaatgcaattatccatatctgcacctcaggcatggttaaaatacaaagatgcaaactggacgcctcctgaactttggaatcatggtattgctggggcatttcttgactacaatttatatgcctctcattatgcaccacatcagggcgataattcgcaaaatataagttcctatgggcaggctggggttaatcttggggcctggcgcctgcgtactgattaccagtacgatcagtcatttaacaatggcaaaagccaggcgaccaacctggattttccgcgtatttatttgtttcgcccaatcccagcaatgaatgcaaaactaactataggtcaatacgatactgaatcctctattttcgactctttccatttttctggcatttcgttgaaaagcgatgagaatatgttaccgccagacctacgtggttacgcaccgcaaatcacgggtgtcgcacaaacgaatgcaaaggtcactgtctcacagaacaaccgtattatttatcaagaaaatgttcctccaggcccatttgctattaccaatttattcaatacattacaggggcaacttgacgtcaaggttgaagaagaggacggacgcgttacgcaatggcaagttgcatctaatagtattccttatctgacgcgtaaagggcagattcgctacaccactgctatgggtaaaccgaccagcgttggtggtgattccttacaacaacccttcttctggactggtgaattctcatggggttggctgaacaatgtatccctgtatggtggttcagttttaacaaaccgtgattatcaatctctggctgccggcgttggttttaatcttaactcattaggttcattatcttttgatgtcacacgatctgatgctcagttgcataatcaggataaagaaacgggttatagctaccgcgctaactattcaaaacgttttgaatctaccggtagccagctcactttcgctggttaccgtttctctgataaaaactttgtgacaatgaatgaatatatcaatgacactaaccattacacgaattatcagaatgaaaaagagagttatattgtcacgtttaaccagtatcttgaatcattaaggttaaatacatacgtaagtttggctcgtaatacttactgggacgccagcagtaatgtgaattattcattatcacttagccgcgattttgatatcgggccattaaaaaacgtctccacttctctaacatttagccgaataaactgggaagaagacaaccaggatcaactgtacctaaatatttcgattccctggggaactagtagaacattgagctatggtatgcaacgaaatcaggataatgagatttcgcatactgcttcgtggtatgactcttccgatcgaaataattcctggagcgtttctgcttcaggcgacaatgatgaattcaaagatatgaaagcgtcactacgcgccagttatcagcataataccgagaacggtcgactctacctctccggtacatcacagcgagacagttattattctctgaatgccagttggaatggttcattcactgcgactcgccacggtgccgctttccacgactatagcggtagtgctgactcgcgttttatgatcgacgcagacggcactgaagatattccgttgaacaataaacgcgcggtaactaatcggtatggcatcggagttattccatcagtcagcagttacataacaacatcattaagtgttgatacccgaaatctgccagaaaatgtggatatcgaaaactcggttatcaccaccaccttaaccgagggtgctattggctacgccaaacttgatacccgcaagggctaccaaatcataggggttattcgcctggcagatggtagtcatccaccactggggattagcgtaaaagatgaaaccagccacaaagaattaggactggttgctgatggcggctttgtatacctcaacggcattcaggatgataacaaacttgctttacgctggggtgacaaatcttgttttattcaaccacccaatagcagcaacttaaccaccggaacggctattttaccgtgtattagccaaaattaattcaggatgaaactaatgcgctacttaaatacaaagaatatcattgcagcaggagtattactctcctgtatgagcagcattgcctggggtgccatcatcccggatcgtacccgtatcataatgaatgagtcagataaaggcgaagcattaaaacttactaatcaaagtaaaaacctgccctatctggcccaaacatggatagaagatacgaaaggcaataaatcgcgtgactttattgtcactgttcctccaatggtgcgtttaaatcccagtgagcaaattcaaataagaatgataactcaggaaaaaattgctcaacttcctaaagacagagaaacgctcttctattttaacgtgcgagaaataccgcccaaaacagataaaaaaaatgtgatgcaagtcactatgcagcacgcattgaaactattctggcggccaaaagccattgaattagaagacgatggggtaatgacttacgaaaaagttgaaatcattcgtagaaatgacggttcgatccgctttaacaataagatgccttatcacgttacgctgggttatatcggaacaaatggggtaacgatgttaccacaaacgcaaagcttaatggtaaccccttttagctatgcaaatacgcagtttaaaaatgttccgtcaacttttcaggtgggttatatcaatgactttggtggattaagtttttatgaaataaactgccctgtagtaaataacatttgtaatatttctgtagccaaccgagatcaataatatgcgctacttgttaattgttattactttttttatgggttttagttcattacctgcatgggcaatggactgctatgctgaacatgaaggtggaaataccgttgtcattggttacgtaccaagaatctctatccccagcgatggtaaaaaaggtgataaaatctggcaaagcagtgaatattttatgaatgttttctgtaataatgcactaccaggcccatctccaggagaagaatacccatctgcatgggcaaatataatgatgttgttagcatcaggtcaagacttttataatcaaaactcttatactttcggtgtaacttataatggggttgattatgattctacatctccactacctattgcagcacctgtatgtattgatataaagggagccggaaccttcgggaatggctacaaaaagcccgcagtctgtagtggcggtcctgaaccgcaattatcagtaacttttccagtacgagtgcagctatatattaagctagctaaaaatgccaataaagtaaataaaaaacttgtattacctgacgaatatatagcacttgaatttaaaggtatgagcggagcaggtgctatagaagtagataaaaatctgaccttcaggattcgcggattaaataacattcatgtccttgactgctttgttaatgttgatctggaaccagctgatggcgttgtcgactttggtaaaataaattcccgaacaattaaaaataccagcgtgagtgagacgtttagcgtagtcatgaccaaagatccgggtgcggcctgtactgagcagtttaatattttagggagttttttcactacggatattttgagtgattatagccatctggatataggtaatggtctgctattgaagatatttcataacgatggaacagcaacggaatttaaccgcttctcacaatttgcttctttttcatcgtctagtgcgccttcggtcaccgcaccattcagggcagaactgagtgcgaacccggcagaaacggttgttgagggaccgtttagtaaagacgtaatcctgaaaatcacctataactagtatctaatacaaacactaaaacgggccatcaggcccgttatatcagtgctctaactccagctctcttgcctgcatcatctgttgacaataccaggcataacgtgcgcaaaaccaggttctatgttcttcatccatgttaccagtaacggccagaatatcgaccgggcgaccttctgcgtgcattctggcaaaactacgcgccaggaaatcgaaattatttaaagaattaagactatgatccataagcacatcctccggttatcgcataccttttaaggccatatgctttttctgatttcagtattccccaatcagtgtagtgcctttaaacataacgtgcgtaaatatattgtccccgatcacactttttagtgaaaaataaaaaaccatattaaaagactttctcttccagaacttctctaacctgtgttattattaacacagataaatgtaagcaaggaaactattacaaagtaaatattgcgtcactaaatggacattggagtgatatatgattttattcgccgactataacaccccttatcttttcgctatttcctttgtactgttgatcggcctgttagaaatttttgcgcttatctgcggtcacatgctctccggtgctcttgatgcacatcttgaccattatgattctataaccacaggtcatattagccaggcacttcattatctcaatattggaagattgccagctctcgtcgttctctgcttactggctggtttttttggtcttattggcatcctgttgcagcatgcctgcatcatggtctggcaatcaccactgtcgaacctgttcgtggttcctgtcagtttactgtttacgattattgcggtgcattataccggtaaaatagttgcgccctggattccacgcgaccatagttcagctattacagaagaagaatatattggtagcatggcgttaattaccggtcatcaagccacttcaggtaatccctgcgaaggaaaactcaccgatcaatttggccaaatacattatttactactggagcctgaagaaggaaaaattttcactaaaggagacaaagtgttaattatttgccgactttctgcaacgcgatatttggcggaaaataatccctggccccaaatattgtaatttattaatcaaaaggaaatttaataatggatgatattgttaattctgtgccctcctggatgtttaccgcaattattgccgtatgcattctgtttattattggaattattttcgccaggctctatcgtcgcgcttcggcagagcaagcttttgttcgtactggtttaggtgggcaaaaagtggtaatgagcggtggcgcaatcgtgatgccgatctttcatgaaataatccccatcaatatgaatactctgaagctggaagtcagccgctcaaccattgatagcctgattacgaaagatcgtatgcgcgtcgatgtagtagtcgctttctttgtgcgggtaaaaccttcagtagaagggattgccaccgctgcccagacgctggggcaacgcaccctgtcgcctgaagacttacgtatgttggttgaagataaatttgtcgatgccctccgtgcaacagctgcgcaaatgaccatgcatgagttacaggatacccgcgagaactttgtgcagggggtgcaaaatacagtggcagaagacctgtcgaaaaacggtctggaactggagagcgtttcacttaccaactttaaccagacctcgaaagaacatttcaatccgaacaatgcctttgacgccgaaggtttaaccaaactgactcaggaaacagagcgccgtcgccgcgaacgtaacgaagttgaacaggatgtagaagttgcggtgcgtgaaaaaaatcgcgatgcgctatcgcgcaagctggagattgaacagcaagaagcgtttatgacgcttgagcaggagcagcaggttaaaacccgtactgccgaacagaatgcacgtattgcggcttttgaagctgaacgtcgtcgtgaagcagagcagacacgaattctggctgaacgacagattcaggaaacagaaatcgaccgcgaacaggccgtccgctcaagaaaggttgaagctgaacgtgaagttcgcattaaagagatcgaacagcagcaggtcaccgaaatcgctaaccagacgaaatcgatcgctattgccgccaaatcggaacaacagtcccaggcagaagcgcgtgctaatctcgcacttgcagaagcggtaagcgcccaacaaaacgtagaaaccactcgccagactgccgaagccgatcgtgctaaacaagttgccctaatcgctgccgcgcaggatgcagaaaccaaagcggttgaactgaccgtgcgggcgaaagcagaaaaagaagccgcagagatgcaggcggcggctatcgttgagttagccgaagctacacgtaaaaagggtctggcggaagcagaagcacaacgtgcgctgaacgatgctatcaacgtactttctgatgaacaaaccagccttaaattcaaactggccttgttgcaggcgctgcctgcggtaatagagaaatccgttgagccgatgaagtcaatcgacggtatcaagattattcaggtcgatggtctgaatcgtggcggcgctgcgggtgatgcaaacacgggtaatgtggggggcggaaacctggcggaacaagcattatcagccgctctctcttaccgcacacaggcaccgctgattgactccttgctcaatgaaattggcgtttcaggcggctcactggcggcattgacttcacccttaacctcaacaactcccgtcgaagaaaaagcagagtaaaccctcttccaggaataatccctggcccaaaaagccggggattttttatatctgcgttccgctaaaaagtgcaaatgatcaggttgttgcagcattttgcgtgacggctcggggaaggcaaaactgcatcagagaaagcattgcgtggggtctggcgctcatcaacaatcggggagtcagcagggggctgaaacgggaaagcccctcccgaagaagggggccttacagaaggaaagggttatgatgaagctcgtcatcatactgattgtgttgttactcgtaagtttcgcagcttattaacagccaatcagaggggggagaaatcctccctcacccttgttcctttactttaggttgaaaaaaaatcagcgtcaagaaggtttcattaacacatatccctggcccaaaaagccggggattttttatatctgcgttccgctaaaaggtgcaaatgctcaggacgttgcagcgttttgcgtgaccgctcggggaaggcaaaattgcctctgggaaagcattgcgcggggtccggcgctcatcaacaatcggggggcagcaaggggctgaaacgggaaagcccctcccgaagaaggggccttgtataaggaaagggttatgatgaagctcgtcatcatactggttgtgttgttactgttaagtttcccgacttactaacaactcatcagaggggggagaaatcctcccttacccttgttcctttactctaggttgaaaaaacaacagcgtcaataggcctgccatgtacgaagcgagatctgtgaaccgctttccggttagccttttttatcctgttggatcttcttgatgatgttggtcgtcgagcaaccgtcttcaaagttgagcaccaacacttcgccaccgttggcccagacttctttactcccggcaatctcttctggtttatagtcgccgcctttcaccagcagatctggcaagatcccggcgatcaagcgctgcggcgtgtcctcttcaaacgacactacccagtcgaccgcttccagtgcgcccagcacaatcatacgctgttcgagtgggtttaccgggcgggaatcccctttcagccgtttggtggaggcatcgctgttgacggcaacaatcaagcggtcacccagcttgcgggcatttgccagataagagacgtgcccggcgtgcaggatgtcaaagacaccgttggtcatcaccactttttcaccacgtttacgcgctgccgctacggccagcttcagttcctcttcggtcatcacgccaaagcctgtatctgcacgtccacgtacagcattttccagctcgatcggcgaaaccgtggaggttcccagtttgccgaccaccacgccagccgccgcattggcaaagaagcaggcttcttccagcgaattacccgctgccagcgttgccgccaggacgccaatcaccgtgtcgcccgcaccggtaacgtcatacacttcctgcgcttgggttggcatatgcagcggcgctttacccggttgcagcagcgacataccctgttcggaacgggtcactaacagagccgagagttcgtaatcggcaatcagtttcatgccgcgctcaacaatctcttcttcggtcttacatttaccgacaacagcttcaaattccgagagattcggcgttaacagcgtagcgccgcggtagcgctcaaaatcggtaccttttggatcaatcagcaccggaacacccgctttacgcgccagttggatcatctgctgtacgcttgccagcgcacctttggcgtagtcagaaagcaccagcgcgccaatcgaactcagcgcctgattaatccgctcgtgcagcggctgcggatcaacaccttcgaaaccttcttcaaaatccagacggatcagctgttggttgcgggaaagtacccgtaatttggtaatggtcggatgcgtcggtacagaaacgaagtcgcatttgacgttgacgtcggccagagatttactcagcgcgcgcgctgcatcgtcaatgcccgtcaacccgaccaggcgtgcattagcaccgagagaagcgatattcatcgccacgttagccgcgccgcccggacgttcttcgatggtattcactttaaccacgggcaccggcgcttccggcgagatacgactggtggggccgtaccagtaacgatccagcatcacatcaccaaccaccatcactcctgcacgttcaaactctggcagcgttactttcattcctgtctcctgagagattcaaaatttgcgcgcgataataccatacttcattcttccaccagccacttctgccagcttgcccgcaccagttcacgctctgcggtgaagcaatcctccgacacatggcccggcaattcctgtaatgccagatgatgaagttcatcgcgaagcgtagtgtaagcacgggtcagcgccatcgcttcctgctcttccataatgtcgttttgcgccagtagttccagaatacgcacgttgtctgaccagcgcgttaacttcggtttttcatgagcgtagcgcaacaccagatattgggtaataaattcgatatcggtaattcccccttcatcagctttgatatcaaagcgatcgcgatgtttattgccgagatgagcgcgcattttctcgcgcatttcccgcacttccgtttgcagagttttaccttcacgcggcagcgtcataatctcgcgacgcactgcgtcaaagtgcgcggtgagctgcggatcgccgtacactacacgcgcacgcaccagcgcctgatgttcccacgtccaggcctcgtttttctgataatcggcaaatgcttctgcggatgtcaccagcattcccgccgccccggacggacgcagtcgagcatccacttcatacaaaatgccggaagaggtacgcgtactgaacagatgcataatgcgttgcgccagacgcagataaaactgccgcccgtcgatttcccgctcaccgtcagtcatcgcatccattgggcaatcatggaggaagataaggtcaagatcggaactgtagcctaactcccagccgcccagcttgccgtagccgaccaccgcaaaaccacgcccttcgcgttcgttcaggtgattcggcttaccgtagcgggcaaccatttgaacccacgcctgctgaacgacggcatctatcatggcttccgccagccaggttaagtgatcgctcactttcatcaccggtagcgtaccggcgatatccgctgcggcgatgcgtaacagctgcgcctgtttgaactgacgcagcgcctcaagctgttgctcttcgtcatcttccggcacgcgcagcaaatactggcgcaactcatcgcggtaggcatcggtcgccgtcggctggtaaagggtgtttggatcgagcaattcatccagcaataatggataacgcgccagctggctggcaatcatcggcgacgcggcacacagagaaatcaaatgtttaagcgccgcggggaattcactgagcaattctaaataggtggtgcgggtaacaatccccaccagcaaggcggtaatgcgcgacagcgtaacggcagcgtcttcacgcgcacagacatcacttagcagatgcggcatcagatggtcgagcacctgacgtcctcgcggcccgatggtgcgcttatccagctctttgcggaaatcggcaatcagcgttagcacctgtttgcgatcatcctcgctaagatgcgccagcactggcgtagtgtcatcttcctgcaacgcatcctgccacagctcacgccactgttccgacagcgactcttcctgagtttcactttcatcgtcgccaatcaattcattaaacacccggcgcacattggtcatatgtgcggtcagcgccccggtcagttgcggccagtcagcaaagtccatcgcccacgccagccgcgcacgattaagctcatcagaaggaagcgtctgggtttgttcgtcgttaatgctttgcagcaggttttccagacgccgcaggaacagatacgccactcgcaattgttcagcatcgttttcagaaagcagatgcagctcggcaatggcgctgagcgttggcagtaaagagcgcgattgcagcgacggttcgcgtccgccgcgaatgagctggaacacctgaacgataaattcaatttcgcgaatgccgcctgcgccgagtttgatattgtcggtcaaaccacgtcgacgcacttcacgggcaatcatccctttcatgttgcgcagcgactgaatcacgctgaaatcgatgtaacgacggaaaacaaacgggcgcagcatcgcacgcaactcgttagcatagacgccttcgctatcgcccataatccgcgccttgaccatcgcgtaacgctcccagtcgcgcccctgctcctggtaataatcttccaacgcggcaaagctcagcaccagcgggccactttcgccaaacggacgcagccgcatatccacgcgatagacgaagccatcctgcgttggttgatccagcactttaatcagccgctgccccatgcgggtaaaaaactgcgcgttatccagttcccggcgtccaccctgcgtacaaccatgttccggccaggcaaaaatcagatcgatatcagaggagaaattcagctccccaccgcccagcttacccatgcctaaaatcagcagcggttgcgcttcgccctgcgcattgcacggcgttccccactcgcggcagcaggcgtcatacagccagtcacgcgccgcaacaatcagcgtctccgccagatagctgagctgctgcaatatgctctcttcagtaaccagtgccagcgtttgcgcccaggcgatgcgcaccataatgcgccgccggaatagccgcagctcgcgcattaacccggcttcgtcactcacattacagagcgcctcctgcaaccatgccgcgtaatgctgccattcgtcggcctgcggcggttggctttccagttccgtcagccactctggatgcgcaatcacgctgtcctgcacaaaatcactaaaagtaagtactgacttcgcctgtgcgctaagtgattcctcggctaaaggctctggcagccgctcaacaacggtctgccagtactgctgtaacggtgaagagagcggcttcataagcgattttatccttgcctgattaacgttttccgctgtgcaaccagaacggttcctgattgtttgcctcattacggaaatgttcaatttcgatgcgttgcccggtcgcaatagcgtgatgcagcccctgccagttctccagccaggcttgcgcgacgacaggatcatagtaacccgccagcaacagtattgagtcaatatcacgcgtcaggcgtggcaactggtcacggtagcgatcgcctaacggctggcagaaaacgcttttcagttcagcggcatggcgggaaagatggatatcggcaaagcgtttgaaggagtcgctgattttgccctgcgctttggcatctaaaaatggctgccatgctttgcttaccaaccattcggtcaacgccagcttcgccattgccgtttcggtagagtagaccgccgtcacggcagacaccgcagaagcaatggtcgcctcgcattgagtcagcagatcacgtaagtgagtgctcgctttacgcggcacaataccaccgaacagcatcagcgtatgacggaccaggctaatggctgccagcacctgttctttcgccgcatcgttgccgcgtacccacagttcttcatgatactgccattgcgctaacgccagctcgagcgccgcttccagcccctgttccacatcggcttttgccgcaacatgcaaaatggtggtcggtttgatttcacgcgccggattgccctgcgccagatgatagccacgcgccgctttgctcaggctgccctggcgtaatccggtttgcgataccagttggttcgccagtttcagcaccgcgcgcgtgtcgccgctaagcagttccagttccagctcacagataggttcagcaaattcacccgctttcacttccccctggtcgagggcgatttcaatttggctaccatcgaccgccaccagccatttttcgcgataaaaatcggtgctgaacagcggctgcacgcgggaggcgagatcggcgggcaattcgccgttcggccagacttccgtcggtaactgcgccaggtcgagcgtcggttcgctcaacgccacgttatattccgggcgctgatgtaagccgcctgtcactcttcctgcaactttcatggtcatctcatagcgaccgttttcgccacgaatacgtaagcccatatcgtgcccacgcagccagttatccggcgtttcgtagtaaatattcagcaactgcacggggtcatggtgctcgccgcccagcgtattgagatggtcacgcaacgcctcaacggcactgtgattaacaataaactttaattcgatttcctgagccatggcctttacttatcggttatgtcacataagtgacgatgaacggcgaacttaatgcgatcttttttgtcagtagatagtattttgcgccaaattgccatgcaacgggcaatttgacgggcgtaaaagtttgaagcagtggcaagacctgacacagaggattccgattgatgtcgaatgctttgcgtagcgacactgatgccactactatcgttccactttccatgacaataacgacagcctgatgccaaaattacgcctgatcggattaactttactcgcacttagcgcgactgccgtctcacacgctgaagaaacgcgctatgtttccgacgaactgaatacctgggtccgcagcggtccgggagatcattatcgcctcgtgggcacggttaacgccggcgaggaagtgaccttattacaaactgacgccaacaccaattatgcccaggtgaaagacagctctggccgtaccgcctggatcccgttgaaacaacttagcactgagccaagcctgcgctcccgtgtgccagatctggaaaatcaggtcaaaaccctgaccgataaactcaccaatatcgataacacctggaatcagcgcaccgcagaaatgcagcaaaaagtggcgcagagcgacagcgtgatcaacgggttaaaagaagaaaatcagaaactgaaaaacgagctgattgtcgcgcagaaaaaggtcgatgccgccagcgtacagctggatgacaaacagcgcaccatcatcatgcaatggtttatgtatggcggtggcgtgctggggcttggcttgctgctcggtctggtactgccgcacctgatcccaagccgcaaacgcaaagatcgctggatgaactaaatcgccttcttcgttgcactgtcttattattaggaattgtgtatttgacgaagggatgatggcgtgaagatttatctggtcggtggtgctgttcgggatgcattgttagggctaccggtcaaagacagagattgggtggtggtcggcagtacgccacaggagatgctcgacgcgggctaccagcaggtaggccgcgattttcctgtgtttctgcatccgcaaacgcatgaagagtatgcgctggcacgtaccgaacggaaatccggttccggttacaccggttttacttgctatgccgcaccggatgtcacgctggaagatgatcttaagcgtcgcgatctgaccattaatgcgctggcccaggacgataacggcgagattatcgacccgtacaacggtctgggcgatctgcaaaatcgtctgttgcgccatgtttcccccgcttttggcgaagatccgttacgcgtattgcgcgtggcgcgttttgctgcgcgttatgcccacctcggttttcgtattgccgatgaaactctggcgttgatgcgcgagatgacccatgcgggtgaactggaacacctgacgcctgaacgggtatggaaagagacggaaagcgccctcaccacccgcaatccacaggtgttcttccaggtactgcgcgattgcggcgcactgcgcgttttattcccggaaattgacgcactgtttggcgttccggcccctgccaagtggcatccggaaatcgatacgggtattcataccttaatgacgctctcaatggcggcgatgctgagtccgcaggtcgatgtccgtttcgcaactttatgccacgatctcggtaaagggctgacgccgccagaactctggccgcgtcatcatggtcatggcccggcgggtgttaagttagtggaacaactatgccagcgtctgcgcgtgccaaatgaaattcgcgatttagccagactggtggctgagtttcacgatctcatccacaccttcccaatgctgaacccaaaaaccatcgtcaaattatttgattccatcgatgcctggcgtaaaccgcagcgtgtcgagcaactggcgctgaccagcgaggctgacgtgcgcggcagaaccggttttgaatcagcggactacccgcaaggccgctggttgcgcgaagcctgggaagtggcgcagtcagtgccgacaaaagccgtcgttgaagcgggatttaaaggtgtggagattcgcgaggagctgacccgacggcggattgcggcggtagccagctggaaggaacaacgttgcccaaagcctgaatgagtattgggcattttgccggatgcggcgtaaacgccttatccggctacatgtcaacgacagttgtaggcctgataagacgcgcaagcgtcgcatcaggcgttgattgccggatgcggcgtgaacgccttattcggcctacgcaatcgttgacaacgccaagcatccgacactattcctcaattaaaagaacacgacatacaccgcagccgccacaataaagcgataaatggcgaacgggataaacgaaatgcgcttaatcaattgcaggaaggttttaatcgctatcagcgccaccacaaaagcggtgataaacccaacggcaaacatcgggatatcgccgcttgtcaggaagccccagcttttgtagagatcgagcgccgttgcgcccatcatcatcggcaccgccagcaggaacgaaaactcggaagcagcgtaacggctcacccccatcagcatcccacctgaaatggtcgccccggaacgggagaaacccggccacagcgccagacactggaaacagccaatcataaatgcctgacgataggtcatatcatcaagacccggcgcacgcggctctttcggcttcaggcattcggcggcaatcagcaacaaaccgccaacgaccagcgcatacatcacatttatcgggttaaacaatgacttaatcgtgtcgtggaacaacagccccaataccaccgccggaatcatccccagcaaaatgtggatcagcgttaaacgacctttgctttcaccttcgtgctgcaacgggcggccaaagtggatgccaatcaggccaaacagacgccgccagaacatcactactaccgccagaattgatcctaactggatcacaacttcaaaggttttcgccgtgtcgccctcaaaccccaacaagtgaccgacaataatcatatggcccgtgctggataccggcagaaattctgtcaatccttcgaccacacccaatattgccgctatcagcagcgagtgcatatcgctcatcaataaacccctaaattattaaaatgtaccgcttgtccgaactactgcgtatgaccaggttataaccgtttggtttaacagctgtaaaattaattattttctttcagattattgccacgctcaatgattacgccaacattcgccgcccgcgccactgcgcctggcttgctgagtttgatacgcacccacggcgagttgaagcgtgctaacagcagctccgccacctcttcagccacgcgttccaccagcgcaaaacgcgccccctcgacgtggctgaccaccgtttctgcaatgtcagcgtaactgaggcaatccgccacatcatcacttttcgccgctttacggttatcccacgccatttcgatatcgaacactaacttctgttcgatggtctgttcccagtcgtaaacaccaatagtggtgattaccgaaagttgctctataaatacaatatccatcacgtcctgcctgctttttggctaaccggataccacttccggcgaaatgtgcgtattatccacagattcatcgttgaacacgaattttcaaaacggaacagcttatgagtgcaatcgcgcctggaatgatcctcatcgcgtacctctgcggctccatttccagtgccattctggtttgccgcttgtgtgggctgcccgatccgcgaaccagcggctccggcaatccaggcgcaaccaatgtgttacgtatcggtggcaagggagcagccgtagcagtactgattttcgacgttctgaaaggaatgttgcccgtctggggcgcgtatgaattaggtgtcagccccttctggctaggcttaattgccatcgccgcctgtcttggacacatctggcccgttttcttcggatttaaaggaggaaaaggcgttgctaccgcttttggtgccatcgcacccattggctgggatctcaccggagtaatggcgggaacctggttactgaccgtgctattgagcggatactcgtcgctgggagcgattgtcagtgcactgattgctccgttttatgtctggtggtttaagccacaattcaccttcccggtttcgatgctctcttgcctgatcctgctgcgtcatcatgacaacatccaacgtctgtggcgtcgtcaggagacaaaaatctggacgaaattcaaaagaaagcgcgaaaaggatcccgagtgatttctggtggatctacatgacctgatagccttcatcgggcttgcccagccgttgctggcaccatgccgccagaaattccacgcagacacgtaatttcatgctgcgatagagcggctcccggtaaacagcccagatattggcgctttgtgcatactctggcaatacttgcaccagtttgccactctccagaaacggcaacacatcccactcggaacgcagcataatccctttgccctccagcgcccattgcagcacaatctcgccgctattggaggaaagatgcccgcttaccttcaccgattttttctcctgaccgttccccaactcccatattccatgggtcatatcgcgctctttggtcaccagacagtcatgacgacttaattcctgtagggattgtggctgcggatatttttgcagatactcaggtgctgcgcataatattcttttattttttgtcaaaagatgcgcaatataataatcaggaatttcgtcattaatacgaatatccagatcaatattatcctgcactaaatcaatttgccgatcgaacaattcaaaatgcacctgtaactcaggataattgcgcatcagttcggtaatagctggcgcaatatggctgcgcccaaaaccaaaactgcaaccaatacgaatcatcccctccgggcgcgttttgatttgcgtgacgtcatcgaccagtcgctgatattgggtgaggatttccaacgcatgttcgtaacaacgttggccactttcagtcagcgccacgccgcgagcggagcggttcagcagcgttgttgccagcgtattttcaaggatttggatccgcttggtgacaaatgcaggcgtctgcccaagcgtcgccgctgcggcgctaaaactcccgctgtgaacgatttctaccagtacctgcaagtctttggctaaaggccagctattcagcatcgttaattatccgcagttgtgataagcgcagtgtatttcgcaaaacattgccattccctgctctggcgcaatattcattcttattttcgcgttgattcacgaactgttaattacatattcacggtggcaaaaaatataaaaccacatttttagtggtagtttgtggcggtgaatttttccagacaaatacaaaaactggagttgccatgatgagcgaaagtaataagcaacaggcagtgaataagttgacagagattgtcgctaactttaccgccatgatttctacccgaatgcctgatgacgtggtggataaactaaaacagctaaaggatgccgaaacgtcgtcgatggggaaaattatctaccatacgatgttcgacaacatgcaaaaagcgattgacctgaatcgtcctgcctgtcaggacaccggggagattatgttcttcgttaaagtcggttcccgcttcccactgcttggcgagctgcaaagcatactcaaacaagccgtggaagaggcaaccgtcaaagcgccactacgtcacaatgcggtagaaatttttgacgaagtaaacaccggcaaaaataccggtagcggcgtaccgtgggtcacctgggacatcatccccgacaatgacgatgcggaaatcgaagtttacatggcaggcggcggctgcacgctacctggccgctcgaaagtgttaatgccgtcagaaggctacgaaggcgtggtgaaattcgtcttcgaaaatatctccaccctcgccgtaaacgcctgtccaccggtactggtgggcgtgggcatcgccacctcggtggaaaccgccgccgtactctcgcgtaaagccattttgcgcccgattggcagccgccatcccaatccaaaagcggcagaactggagctacgcctggaagaaggactcaaccgtctggggattggtccacaagggctgaccggcaacagttcagtgatgggcgtacatatcgaatctgccgcccgccatccgtcaaccatcggcgttgctgtctctaccggctgctgggcgcatcgtcgcggcacgctgctggttcatgccgatctcacctttgaaaatctgtctcacacccggagcgcgttatgaaaaagatcctgacaaccccgatcaaagctgaagatctgcaagatattcgcgtcggcgatgtgatctacctgaccggtacgctggtgacctgccgcgacgtttgtcaccgccgtttgatcgaactgaaacgtccgatcccttacgatctcaacggcaaagcgattttccacgctggccccatcgtgcgcaaaaacggcgacaaatgggagatggtctccgtcggcccgacaaccagtatgcgtatggaaagttttgaacgtgaatttattgagcagaccggcgtgaaactggtggttggcaaaggtggtatggggccgctgaccgaagaaggctgccagaaattcaaggcgctacatgtgattttcccggcaggctgcgcggtgctggcggcaacccaggtggaagagattgaagaagtgcactggacagagctcggaatgccggagtcactgtgggtctgccgggtcaaagagttcggcccgctgattgtctctattgatacccacggcaacaacctgatagccgaaaacaaaaagctgttcgccgaacgccgcgatcccatcgtggaagagatctgcgagcacgtccattacatcaaataaccctcccggagaggctcacccctctcctttttcgcaggcataacacgatgaaaccttccactgaatggtggcgatatcttgcgccgctggcggtcatcgccattattgctctacttccggttcccgcagggctggagaaccatacctggctctactttgccgtttttactggcgtgatcgttggactgatcctcgaacccgtgccgggtgccgtggtggcgatggtgggtatatccatcatcgccatactctctccctggctgctgttcagcccggagcagctcgctcagccaggctttaaattcactgcaaaatccctctcgtgggccgtttccggtttttctaattcggttatctggctgattttcgccgcctttatgtttggcacaggctatgaaaaaaccgggcttggacgccgcattgcgctgattctggtgaaaaagatgggacatcgcacgctgtttctcggctatgcggtgatgttctccgagctgatcctcgcacctgtaacaccgtccaactcggcgcgtggtgcggggattatctatcccatcatccgtaacctgccaccgctctatcaatcacaaccaaacgacagcagttcgcgcagcattggctcgtacatcatgtggatggggattgttgccgactgcgtgaccagcgccattttcttgacggcgatggcaccaaacttgctgttaattggactgatgaaaagcgcatctcacgccacgctgagttggggcgactggttcctcgggatgttgccgctcagcattttactggttctgctggttccctggctggcttacgtgctgtacccgccggtactgaagtctggcgatcaggtgccgcgctgggcagagacggaactgcaggcaatgggcccgctctgttcgcgtgaaaaacggatgctggggctgatggtaggcgcgctggtgctgtggattttcggcggtgattatatcgatgccgcgatggtcggttacagcgtggtggcactgatgctgcttctgcgcattatcagttgggacgacattgtcagtaataaagcggcgtggaacgttttcttctggctggcctcgcttatcaccctcgccaccggactcaacaacaccggttttattagctggtttggcaaactgttagcaggcagcttaagcggttattcgccaacgatggtgatggtggcgttgattgtggtgttttatctactgcgctactttttcgccagcgccacggcgtatacctccgctctcgcaccgatgatgattgctgctgcgctggcgatgccggaaatcccgctgccggtgttctgcctgatggttggtgcggcaattggtctggggagcattcttacaccatacgccaccggccccagtccgatttactacggcagtggttatctgccaacggcggattactggcgactgggggcgatttttgggctgatattcctcgtattgctggtgattaccggcttactgtggatgcccgtggtgttgctttaagtgaggacggtgccggaaattgctctccggcacccaatagttttacgcagccggtaactccgccagcggccagcgcggacgcacgctaacgccgagatccgccgtcgcgcctgctttaaaccgcaccattccggcataggcgatcatcgcgccgttatcagtacaaaattccggacgcgcgtagaacacttcgccgcggcgttttttcatcatttcagccagcttcgcccgtaacgtacggttagcactcacgccgcccgccatgaccagtcgcttaaagcccgtctgatccagcgcccgcttgcacttaatcatcagcgtatcgaccaccgcatcttcaaaggcgcgggcgatatcagcacgcgtctggtcgtcggtgccgttgtcacgaatggtatttgccgcgaaggttttcaggccggagaagctgaaatccagccccggacggtcggtcatcggacgcgggaagacaaagcgcccggcagtaccctgagccgccattttcgacagtaacggcccgccaggataatccagccccagcagcttcgcggttttatcaaacgcttccccggcggcatcatcgatagactcgccgagcagctcgtactgaccaatgccagtcacgctgattaactgcgtatgaccgccggaaacaagcagcgcaacaaacggaaattccggcgggttatcttccagcatcggcgctaacagatgcccttccatatggtgtacagggatcgccggaacgtcccaggcaaacgccagagaacgccccacggtcgcgccaaccagtagcgcgccgactaatccagggcctgcggtataggccacagcatcaatgtcttttgccgttaaaccagactcctttagcgccgcctggatcaacggtacggttttacgcacatgatcgcgggaggccagttcaggcacgacgccgccgtagtcagcgtgcaatttcacctgactatacaattggttggctaacaaacctttttcatcgtcgtaaatggcgatgccggtttcatcgcaggaagtttcaatacccagtacacgcatgacttgttttacctcgctttattaccgcgcagtgtaggaccaatgcgggttgatgtaaaactttgttcgcccctggagaaagcctcgtgtatactcctcacccttataaaagtccctttcaaaaaaggccgcggtgctttacaaagcagcagcaattgcagtaaaattccgcaccattttgaaataagctggcgttgatgccagcggcaaaccgaattaatcaaaggtgagaggcacatgccggtaattaaagtacgtgaaaacgagccgttcgacgtagctctgcgtcgcttcaagcgttcctgcgaaaaagcaggtgttctggcggaagttcgtcgtcgtgagttctatgaaaaaccgactaccgaacgtaagcgcgctaaagcttctgcagtgaaacgtcacgcgaagaaactggctcgcgaaaacgcacgccgcactcgtctgtactaattccccgagagcgttgctctccgatcagaccgagttgtagttgtaaggccgtgcttccgaaaggaatgcgcggcttattttcgtttatgaattgctaaaaatcggggcctatggctggacgaatcccacgcgtattcattaatgatctgctggcacgcactgacatcgtcgatctgatcgatgcccgtgtgaagctgaaaaagcagggcaagaatttccacgcgtgttgtccattccacaacgagaaaaccccgtccttcaccgttaacggtgagaaacagttttaccactgctttggatgtggcgcgcacggcaacgcgatcgacttcctgatgaactacgacaagctcgagttcgtcgaaacggtcgaagagctggcagcaatgcacaatcttgaagtgccatttgaagcaggcagcggccccagccagatcgagcgccatcagaggcaaacgctttatcagttgatggacggtctgaatacgttttaccaacaatctttacaacaacctgttgccacgtctgcgcgccagtatctggaaaaacgcggattaagccacgaggttatcgctcgctttgcgattggttttgcgccccccggctgggacaacgtcctgaagcggtttggcggcaatccagaaaatcgccagtcattgattgatgcggggatgttggtcactaacgatcagggacgcagttacgatcgtttccgcgagcgggtgatgttccccattcgcgataaacgcggtcgggtgattggttttggcgggcgcgtgctgggcaacgatacccccaaatacctgaactcgccggaaacagacattttccataaaggccgccagctttacggtctttatgaagcgcagcaggataacgctgaacccaatcgtctgcttgtggtcgaaggctatatggacgtggtggcgctggcgcaatacggcattaattacgccgttgcgtcgttaggtacgtcaaccaccgccgatcacatacaactgttgttccgcgcgaccaacaatgtcatttgctgttatgacggcgaccgtgcaggccgcgatgccgcctggcgagcgctggaaacggcgctgccttacatgacagacggccgtcagctacgctttatgtttttgcctgatggcgaagaccctgacacgctagtacgaaaagaaggtaaagaagcgtttgaagcgcggatggagcaggcgatgccactctccgcatttctgtttaacagtctgatgccgcaagttgatctgagtacccctgacgggcgcgcacgtttgagtacgctggcactaccattgatatcgcaagtgccgggcgaaacgctgcgaatatatcttcgtcaggaattaggcaacaaattaggcatacttgatgacagccagcttgaacgattaatgccaaaagcggcagagagcggcgtttctcgccctgttccgcagctaaaacgcacgaccatgcgtatacttatagggttgctggtgcaaaatccagaattagcgacgttggtcccgccgcttgagaatctggatgaaaataagctccctggacttggcttattcagagaactggtcaacacttgtctctcccagccaggtctgaccaccgggcaacttttagagcactatcgtggtacaaataatgctgccacccttgaaaaactgtcgatgtgggacgatatagcagataagaatattgctgagcaaaccttcaccgactcactcaaccatatgtttgattcgctgcttgaactgcgccaggaagagttaatcgctcgtgagcgcacgcatggtttaagcaacgaagaacgcctggagctctggacattaaaccaggagctggcgaaaaagtgatttaacggcttaagtgccgaagagcgatcgggaagcccccgacagccgcactgagaggcagcggcaaatatataagtacgccctcgtaattatcgttggcggtaaacaaccgttggatttcagcgttaacggctgaaggacatcgggtcaatcgcccaacaccaacctcatgaaataagtgtggataccgtcttatggagcaaaacccgcagtcacagctgaaacttcttgtcacccgtggtaaggagcaaggctatctgacctatgccgaggtcaatgaccatctgccggaagatatcgtcgattcagatcagatcgaagacatcatccaaatgatcaacgacatgggcattcaggtgatggaagaagcaccggatgccgatgatctgatgctggctgaaaacaccgcggacgaagatgctgccgaagccgccgcgcaggtgctttccagcgtggaatctgaaatcgggcgcacgactgacccggtacgcatgtacatgcgtgaaatgggcaccgttgaactgttgacccgcgaaggcgaaattgacatcgctaagcgtattgaagacgggatcaaccaggttcaatgctccgttgctgaatatccggaagcgatcacctatctgctggaacagtacgatcgtgttgaagcagaagaagcgcgtctgtccgatctgatcaccggctttgttgacccgaacgcagaagaagatctggcacctaccgccactcacgtcggttctgagctttcccaggaagatctggacgatgacgaagatgaagacgaagaagatggcgatgacgacagcgccgatgatgacaacagcatcgacccggaactggctcgcgaaaaatttgcggaactacgcgctcagtacgttgtaacgcgtgacaccatcaaagcgaaaggtcgcagtcacgctaccgctcaggaagagatcctgaaactgtctgaagtattcaaacagttccgcctggtgccgaagcagtttgactacctggtcaacagcatgcgcgtcatgatggaccgcgttcgtacgcaagaacgtctgatcatgaagctctgcgttgagcagtgcaaaatgccgaagaaaaacttcattaccctgtttaccggcaacgaaaccagcgatacctggttcaacgcggcaattgcgatgaacaagccgtggtcggaaaaactgcacgatgtctctgaagaagtgcatcgcgccctgcaaaaactgcagcagattgaagaagaaaccggcctgaccatcgagcaggttaaagatatcaaccgtcgtatgtccatcggtgaagcgaaagcccgccgtgcgaagaaagagatggttgaagcgaacttacgtctggttatttctatcgctaagaaatacaccaaccgtggcttgcagttccttgacctgattcaggaaggcaacatcggtctgatgaaagcggttgataaattcgaataccgccgtggttacaagttctccacctacgcaacctggtggatccgtcaggcgatcacccgctctatcgcggatcaggcgcgcaccatccgtattccggtgcatatgattgagaccatcaacaagctcaaccgtatttctcgccagatgctgcaagagatgggccgtgaaccgacgccggaagaactggctgaacgtatgctgatgccggaagacaagatccgcaaagtgctgaagatcgccaaagagccaatctccatggaaacgccgatcggtgatgatgaagattcgcatctgggggatttcatcgaggataccaccctcgagctgccgctggattctgcgaccaccgaaagcctgcgtgcggcaacgcacgacgtgctggctggcctgaccgcgcgtgaagcaaaagttctgcgtatgcgtttcggtatcgatatgaacaccgactacacgctggaagaagtgggtaaacagttcgacgttacccgcgaacgtatccgtcagatcgaagcgaaggcgctgcgcaaactgcgtcacccgagccgttctgaagtgctgcgtagcttcctggacgattaatcggtaggccggatcaggcgttacgccgcacccggcactaggccctctgcacaaacgccaccttttcggtggcgttttttatcgcccacgcactaccagcgcctggtccagctcgcgatacgcttcaaccagtttctccagtgaaacgcgacttaaaccgctgggatttggcagcacccaaatctgcgtcgaaccaatggtgagcgtttgtttcccccactgtgcaccgcgctggctgaatccctgttcatatgcttgtttgcccagaatcgccaacgcctgcggctgataatcttcaattttttcaatcagcttacgcccgcctgcgtgtagctcctgctttgaaacttcattggcttgcaccgttggacggtctaccagtttggtgacgccacaacgataatccagcagatgctgtgcctcctgcggcttcaactgacggtcggtaaacccggcctgatatatcaccttccagaagcgatttgccggatgagcaaagggaaaaccagtcccggcggatgaaagcccagggttgataccgcaaaacacgacccgtaaccctggagccaaaatatcctcaaccatatttactcctttctaacatcaccaggaaaagtataacggattgaaaatacattgtttataaaaacagcaggcgcgcggtaatggctggattgcgacacggagttactttataatccgctaccatggccccttagctcagtggttagagcaggcgactcataatcgcttggtcgctggttcaagtccagcaggggccaccagatatagcaaaggctgacgagaaatcgtcagcctttttctttttatatatcagttactttgcgtgccagtaagccgctgcacgtacccgctgtgggtcatactgttccgcttcaaagcggcggcttaaattcttaacgactttaccttcgccggttatccagatgaagtaatcatcggcagggatttgcatctgcgccagacgcgcatctaccgcctgctcatcatgtgccagccattcgatattaaaaccatcaaggtgcgcgagataatcctgacaggcgttatcccgcacgctaaccagcgcactaacttgcggtttaacggcaagtttgctcaacgtttccaggcggcggcgcaatgcaggcattccggattcatcgcagacatacagctgatacgcgtaatcttccggcaccaccagcgaaccgcgcggacctgccaccgtaagtttatcgcccggttgcgcctgcatcgcccagccgctggcgaccccaccgtcgtgaataaagaaatcaatcgccagttcatggcgtagttcgtcatacagcggcgtatagtcacgcgacggtgggcgtggtccttccggccagacgatgccctcttccgttaccgttggcggcacaaagtgagcgtcaggttgaggaaagaagagtttgctgtgatcgtcaaagccacgcgatgtaaaaccgtccagcgcctcgccgccgaggacaatgcgctgaaaaccggcgctgatgcgctcaacgcgtaacacagtcagttcacggaagcgcagatcattgcgaacgcgctgcgggtagcggggggtgttattcattgttatcgccttcgtgatggtaatcagatatatctaaataaaactcgcaaatgataatgattgttaatcatgataaatgcaagcgatttgtagaactgatatgtctatagtctgataagacgaaccgcctcttctcaggcatcattactcaacgccggatgcggcgtgaacgccttatccggcctacgtgtgagatgagtccacgtttaaaaatcatttttacacttgcaagaacgctcatatcagatataaattagatatatctaattaagcaaaaggaggctgatatgagccatcatcacgaagggtgttgtaaacatgaaggccagccacgccatgagggctgctgcaaaggtgagaagtcagaacacgagcactgcggacacggtcaccagcatgaacacggtcaatgctgcggtggtcgccacggtcgcggcggcggtcgtcggcaacgtttctttggtcacggtgaattacgtctggtgattctggatattctctcgcgcgatgacagccacggttacgaattgattaaagcgattgagaatctaacccaggggaattacaccccaagcccgggcgtcatctacccaacgctggattttctgcaggagcagtcgctgattaccatccgcgaagaggaaggaggtaagaagcagattgcgctgaccgaacaaggcgcgcagtggctggaagaaaaccgcgaacaggtggagatgattgaagaacgcatcaaagcgcgttgcgttggcgcggcgctgcgccagaacccgcaaatgaagcgggcgctggataattttaaagcggtgctggatttacgcgtcaaccagagcgatatcagtgatgcacaaataaaaaagatcattgcggtgatcgaccgcgccgcttttgatattacgcaactggattaatcgccgcatccgccagtggcgcggtgcaattgccggatgcgacgcttgacgcgccttatccggcctacacccgctacacaccccgcaggcctgataagatgcgccagcatcgcatcaggcattgtgctccaaccgccggatccggcataccgattaatgcagtaccgtcaccgcgtcttccagtcggctggcgcggtgtttcaccatcgccgacacctgcgcactctcttccaccagctcggcatttttctgggtgatcaggttaagctcatccactgcacgggtcaggctggaaagcccatcggcctgttccagcgttgaatggctaatctgggcgatcaactgggtgacgtttttcacctgtgccacaatatcttccatcgtccgtccggcggcgtgtacctgctgcgaaccggattgcaccttatcagcactggcatcaatcagcttgcgaatatcgttggcagcattagcgctgcggctggctaaatgacgcacttcccctgccaccactgcaaaacctttgccctgttcgccggcacgcgccgcttccaccgccgcattcagggccagaatattggtctgaaacgcaatatcgttaatcagcgaagtaatggtgccaatgcgctgggtactgtcggcgatatcgtccattgtcttgatcaccgtggtcatcgcctccccaccctgcactgccgcattactggcagtgattgacagtttatcggcagccgacgccgtggcagagttctgtttcaccgacgccgccatttggttcatggtcgccaccgtttgctgaacgttatcaactgtctgctgggtatgttcgttcagttcatcggtgcctttcgccagcgtctcactgccatttctgacactggacacctggcttgagacatcgttaattagccaacggcacatcaggccaagttgccctaccgcacgtaatgtcagccccagctcatcgctgcgattcagatgctcaacactattacgttctccggtcgccaccttcagtgcctgatgggcaacattttctatcgggcgcacaatctgccattcaaaacaggcgcttgccaacaataccactaacgcacagaggatatacgtcaccaccggggcagcaacaaaccaaagcatggccgccagcaagataaacatcagggtcatcactccacgcgcccgccagcgaagcggtaatgaaggcagtttacccagccagcctttacgcaccaccaggcctttatgaatacgcttactggtacgtccggcgttcaacgctttgtacagcggctccaccgccgcgatctcttcatccgtcgcccgggtacgaatcgacatatagccactgatttttccctcgcgcaccatcggtaccgcattggcccgcacccaataatggtcaccatttttgcggcgatttttcacgatgccgctccagggctccccttttttcagggtgaaccacatatccgcaaacgccgcttttggcatatccgggtgacgcaccatgttgtgcggctgcccttgtaactcttgcaaggtatagccgctcacctgcacaaaagtgtcattagcatgagtgatatagctttgcagatcggtagtggacatcagagtggtatcgtccgccagcggggtattttgctgggtgacatacggatgagaagacatgttcgcgtcctgtgcaggttatatggttgttaacttcttgtcagagtttatgtcggccccgctgcggttatctttaaccgattaatttgatttagatcgcaatttgcgatttaaacacaaatctaattccttgatttaaaatactttcactctgttactatacgaaaacgttaattatcttgcccaaaaatcaggcaattattgccctgaaaacgtgcatttgcgcagcaatcatcaaatccatacccgacaaaaaccgtgcaaaataacaacaaatgttaacagatagcattaaatattgcacaaatgataaccgaatttgtgtttatcccgattttcgcgatcgcagccggagtggcgcaatccctgcaatacttaaatcggtatcatgtgatacgcgagcctccggagcatattttgaacaggttaccttcgagcgcatcggctttagcgtgcagcgcccacgccctgaatctcattgagaagcgaacgctggatcatgaggagatgaaagcacttaaccgagaggtgattgaatacttcaaagagcatgtcaatccggggtttttagagtatcgcaaatctgttaccgccggcggggattacggagccgtagagtggcaagcgggaagtttaaatacgcttgtcgacacccagggccaggagtttatcgactgcctgggaggttttggaattttcaacgtggggcaccgtaatccagttgtggtttccgccgtacagaatcaacttgcgaaacaaccgctgcacagccaggagctgctcgatccgttacgggcgatgttggcgaaaacccttgctgcgctaacgcccggtaaactgaaatacagcttcttctgtaatagcggcaccgagtccgttgaagcagcgctgaagctggcgaaagcttaccagtcaccgcgcggcaagtttacttttattgccaccagcggcgcgttccacggtaaatcacttggcgcgctgtcggccacggcgaaatcgaccttccgcaaaccgtttatgccgttactgccgggcttccgtcatgtgccgtttggcaatatcgaagccatgcgcacggctcttaacgagtgcaaaaaaaccggtgatgatgtggctgcggtgatcctcgaaccgattcagggtgaaggtggcgtaattctgccgccgccgggctatctcaccgccgtacgtaagctatgcgatgagttcggcgcactgatgatcctcgatgaagtacaaacgggcatggggcgcacgggcaagatgttcgcctgcgagcatgagaacgtacagccggatatcctctgccttgccaaagcgctcggcggcggcgtgatgccgattggcgcgaccatcgccactgaagaggtgttttcagttctgttcgacaacccattcctgcataccaccacctttggcggcaacccgctggcctgtgcggcggcgctggcgaccatcaatgtgttgctggagcagaacttaccggctcaggctgagcaaaaaggcgatatgttgctggacggtttccgtcaactggcgcgggaatatcccgatctggtacaggaagcgcgtggtaaagggatgttgatggcgattgagtttgttgataacgaaatcggctataactttgccagcgagatgttccgccagcgcgtactggtggccggaacgctcaataacgccaaaacgatccgcattgaaccgccactgacactgaccattgaacagtgtgaactggtgatcaaagcggcgcgtaaggcgctggcggccatgcgagtaagtgtcgaagaagcgtaatatcaaatcggatggcgatacgacgtcgccatccgatctttttatacgacgcgtacgcccgcaggcatcatccgctccggcgttaacagcacgctttcactgccgtcatcggtttccgcacacaacagcatgcattccgacgtttcaccacgcattttcgctttttgcagattgcataagaccaccaccgttttccccatcagctcttcttcgctgtagtacggcaccaggctggtcacggtttgcagcgttttttgccccacatcaacctgtacgatgtacagcttgtcggcgttttcatggcgtttcacttccacaatctttccgacgcgcatttccagacgtgcaaaatcagcgtaagccacggtttccattgcttcctcccttagggtaaaattttactaaactatagcaaaagtttttctcaatcctgtaggctaaaaatggagaatgcaggcgtgatcacattcgtgagccgctgtgttaccgttacagcgtcaaagaaacgcgctttatttactgaaaacaggtgacccgataagcacttcctctacaatgggggcgcacatcagggaaagtaaaaaaggtaaacatggcaacactaaaagacatcgcaatcgaagctggcgtatccctggcgacagtatccagggtcttaaatgacgatccgacattgaatgtgaaagaagagacgaaacatcgcattctcgagatcgccgaaaagctggagtacaagaccagtagtgcccgtaaactccagacaggtgcagtcaaccaacaccatattctggctatctacagctaccagcaggagctggagatcaacgatccttactatctggcgatccgccacggcattgaaacccagtgcgaaaagctgggcatcgagctcaccaactgttatgaacacagcggcttaccagacattaaaaacgtcaccggtattttaattgtcggcaaacccacgcccgccctgcgcgccgctgccagcgcgttgaccgacaatatctgttttatcgactttcacgaacccggcagcggttacgatgcggtggatatcgatctggcacgcatcagtaaagaaatcatcgacttctatatcaaccagggcgttaatcgtattggttttattggcggtgaagatgagcctggcaaggcggatattcgtgaggtcgcctttgcggaatatggccgactgaaacaagtggtacgcgaagaggatatctggcgcggcggtttttccagttcgtcgggttatgaactggcaaaacaaatgctggcgcgggaagactatccgaaggcactgtttgttgcttccgattccattgctatcggcgtactgcgggcaattcatgaacgaggcctgaacatcccacaggatatttcgcttatcagcgttaacgatatccccaccgcgcgatttacctttccgccgctctccaccgtgcgcatccattccgagatgatgggaagtcagggcgttaacctggtgtatgaaaaagcccgcgatggtcgcgcgctgccgctgttagtcttcgttcccagcaaattaaaactgcgcggcacgacccgttaaatccccttacacactgtccggcaatcgtttttgccggacagtgctgccgtttattttcgtgatccagttaaagtaaatgcatttacctgctactttttagtaaaaattttactaaactccccagcaattacacaaactaccatcaccatgaatggttccgatttctctctaccgggaggccctatgaatcgctgggaaaacattcagctcacccacgaaaaccgacttgcgccgcgtgcgtactttttttcatatgattctgttgcgcaagcgcgtacctttgcccgcgaaaccagcagcctgtttctgcccttaagcggtcagtggaatttccacttttttgaccatccgctgcaagtaccagaagccttcacctctgagttaatggctgactgggggcatattaccgtccccgccatgtggcaaatggaaggtcacggcaaactgcaatataccgacgaaggttttccgttccccatcgatgtgccgtttgtccccagcgataacccaaccggtgcctatcaacgtattttcaccctcagcgacggctggcagggtaaacagacgctgattaaatttgacggcgtcgaaacctattttgaagtctatgttaacggtcagtatgtgggtttcagcaagggcagtcgcctgaccgcagagtttgacatcagcgcgatggttaaaaccggcgacaacctgttgtgtgtgcgcgtgatgcagtgggcggactctacctacgtggaagaccaggatatgtggtggtcagcggggatcttccgcgatgtttatctggtcggaaaacacctaacgcatattaacgatttcactgtgcgtaccgactttgacgaagcctattgcgatgccacgctttcctgcgaagtggtgctggaaaatctcgccgcctcccctgtcgtcacgacgctggaatataccctgtttgatggcgaacgcgtggtgcacagcagcgccattgatcatttggcaattgaaaaactgaccagcgccagctttgcttttactgtcgaacagccgcagcaatggtcagcagaatccccttatctttaccatctggtcatgacgctgaaagacgccaacggcaacgttctggaagtggtgccacaacgcgttggcttccgtgatatcaaagtgcgcgacggtctgttctggatcaataaccgttatgtgatgctgcacggcgtcaaccgtcacgacaacgatcatcgcaaaggccgcgccgttggaatggatcgcgtcgagaaagatctccagttgatgaagcagcacaatatcaactccgtgcgtaccgctcactacccgaacgatccgcgtttttacgaactgtgtgatatctacggcctgtttgtgatggcggaaaccgacgtcgaatcgcacggctttgctaatgtcggcgatattagccgtattaccgacgatccgcagtgggaaaaagtctacgtcgagcgcattgttcgccatatccacgcgcagaaaaaccatccgtcgatcatcatctggtcgctgggcaatgaatccggctatggctgtaacatccgcgcgatgtaccatgcggcgaaagcgctggatgacacgcgactggtgcattacgaagaagatcgcgatgctgaagtggtcgatattatttccaccatgtacacccgcgtgccgctgatgaatgagtttggtgaatacccgcatccgaagccgcgcatcatctgtgaatatgctcatgcgatggggaacggaccgggcgggctgacggagtaccagaacgtcttctataagcacgattgcattcagggtcattatgtctgggagtggtgcgaccacgggatccaggcacaggacgaccacggcaatgtctggtataaattcggcggcgactacggcgactatcccaacaactataacttctgtcttgatggtttgatctattccgatcagacgccgggaccgggcctgaaagagtacaaacaggttatcgcgccggtaaaaatccacgcgcgggatctgactcgcggcgagttgaaagtcgaaaataaactgtggtttaccacgcttgatgactacaccctgcacgcagaggtgcgcgccgaaggtgaaacgctcgcgacgcagcagattaaactgcgcgacgttgcgccgaacagcgaagcccccttgcagatcacgctgccgcagctggacgcccgcgaagcgttcctcaacattacggtgaccaaagattcccgcacccgctacagcgaagccggacaccctatcgccacttatcagttcccgctgaaggaaaacaccgcgcagccagtgcctttcgcaccaaataatgcgcgtccgctgacgctggaagacgatcgtttgagctgcaccgttcgcggctacaacttcgcgatcaccttctcaaaaatgagtggcaaaccgacatcctggcaggtgaatggcgaatcgctgctgactcgcgagccaaagatcaacttcttcaagccgatgatcgacaaccacaagcaggagtacgaagggctgtggcaaccgaatcatttgcagatcatgcaggaacatctgcgcgactttgccgtagaacagagcgatggtgaagtgctgatcatcagccgcacagttattgccccgccggtgtttgacttcgggatgcgctgcacctacatctggcgcatcgctgccgatggccaggttaacgtggcgctttccggcgagcgttacggcgactatccgcacatcattccgtgcatcggtttcaccatgggaattaacggcgaatacgatcaggtggcgtattacggtcgtggaccgggcgaaaactacgccgacagccagcaggctaacatcatcgatatctggcgcagcaccgtcgatgccatgttcgagaactatcccttcccgcagaacaacggtaaccgtcagcatgtccgctggacggcactgactaaccgccacggtaacggtctgctggtggttccgcagcgcccaattaacttcagcgcctggcactatacccaggaaaacatccacgctgcccagcactgtaacgagctgcagcgcagtgatgacatcaccctgaacctcgatcaccagctgcttggcctcggctccaactcctggggcagcgaggtgctggactcctggcgcgtctggttccgtgacttcagctacggctttacgttgctgccggtttctggcggagaagctaccgcgcaaagcctggcgtcgtatgagttcggcgcagggttcttttccacgaatttgcacagcgagaataagcaatgaggatcatcgataacttagaacagttccgccagatttacgcctctggcaagaagtggcaacgctgcgttgaagcgattgaaaatatcgacaacattcagcctggcgtcgcccactccatcggtgactcattgacttaccgcgtggagacagactccgcgaccgatgcgctatttaccgggcatcgacgctattttgaagtgcattactacctgcaagggcagcaaaaaattgaatatgcgccgaaagagacattacaggtagtggaatattatcgtgatgaaactgaccgtgaatatttaaaaggctgcggagaaaccgttgaggtccacgaagggcaaatcgttatttgcgatatccatgaagcgtatcggtttatctgcaataacgcggtcaaaaaagtggttctcaaagtcaccatcgaagatggttatttccataacaaataacaactacggcggcaaaaggagtttgccgccaccgctaccctactcattttcggagatgtgttatgtctgataccaaacgtaatacaatcggcaaattcggcttgctctcgctgacttttgccgccgtttacagctttaacaacgttatcaataataatattgagcttggactggcctcggcaccgatgtttttcctcgcgacgattttttattttattcccttctgtctgatcatcgcagaatttgtttcgttaaataaaaactcagaagccggtgtctacgcgtgggtaaaaagttcgctgggcggacgttgggcatttattactgcctatacctactggttcgtaaacctgttctttttcacctcactgttgccgcgcgttattgcttatgcttcgtatgccttcctcggatacgaatatattatgacgccggttgccaccaccattatcagtatggtgctgttcgccttctccacctgggtttccaccaacggggcgaaaatgttggggccaattacctccgtcacttcaacgctgatgctgctgttaacgctctcctacattttactggcaggtacggcgctggttggcggcgtacagcctgctgacgccatcaccgttgacgcgatgatcccgaacttcaactgggcgttcctcggcgttaccacctggatctttatggccgcaggtggcgcggagtccgtcgctgtgtacgttaacgacgtcaaaggcggttcgaaatcgttcgttaaagtgatcatcctcgccgggatttttatcggcgtactgtattccgtctcctcggtgctgattaacgtcttcgtcagcagcaaagagttgaaatttaccggcggatcggtgcaggtattccacggcatggcggcgtattttggtctaccggaagcgttgatgaatcgctttgtcggtctggtgtcctttaccgcgatgttcggttccctgctgatgtggaccgcaacgccggtgaaaattttcttctccgaaatcccggaaggcatctttggtaagaaaaccgtcgaactgaacgaaaacggcgttccggcgcgcgcagcgtggatccagttcctgatcgtcatcccgctgatgattatcccgatgctcggttccaataccgtgcaggatctgatgaatactattattaatatgaccgccgcagcgtccatgcttccgccgttattcatcatgctggcttacctgaatttacgcgccaaattagatcacctgccacgcgatttccgtatgggctcccgccgcaccggtattatcgttgtttcaatgctgattgcgatatttgccgtagggtttgtcgcttcgacattcccgactggcgcgaatattctgaccatcattttttataacgtcggcggtattgttatcttccttggctttgcgtggtggaaatacagtaaatatataaagggattaacggctgaagagcgccatattgaagcgacgccagccagcaatgttgattaagcagaataataaaaaatgagcaggcattttccctcttcctggatgaggagagggaaaatagtttctgcctttatatttttataattacaacgataaaaggctgtactttttctttagctcatggattaacacaatgaaattaatcactgcaccatgcagagcattacttgctctgccgttttgctacgccttttctgcggcaggagaagaagcacgtccggcagaacatgacgacacaaaaacacccgcaattacctcgacatcttctccttcatttcgtttttacggcgaattaggggttggtggatatatggatttagagggtgagaataaacataaatacagcgacggtacctatattgaaggtggcctggagatgaagtacggctcctggttcggcctgatttacggcgaaggctggaccgtgcaggccgaccacgacggcaatgcctgggtgccagaccatagctggggtggtttcgagggcggaattaaccgtttctatggcggttatcgtaccaatgatggcaccgaaatcatgctcagtctgcgtcaggattcctcgctggatgacctgcaatggtggggcgatttcacccccgatctgggctacgtcattcccaatacccgcgacattatgactgcgctgaaggtacagaacttaagcggcaactttcgttatagcgtcaccgcgactcctgccggacatcatgatgaaagcaaagcctggctacattttggcaaatacgatcgctatgacgacaaatacacctatccggcaatgatgaacggttacatccagtatgaccttgccgaaggcatcacctggatgaacggtctggaaatcaccgacggcacaggacagctctatctcacgggcctgctaactcctaactttgccgctcgcgcctggcaccataccggacgcgccgacgggctggacgtaccgggaagtgaaagtgggatgatggtgagcgccatgtatgaagcgttaaagggcgtttatctctccaccgcttacacctacgccaaacatcgccctgaccacgctgacgatgaaaccacctctttcatgcagtttggtatctggtacgaatacggcggcggacgtttcgccacggcttttgatagccgcttctacatgaaaaatgcctctcacgatcccagcgaccaaatcttcctgatgcaatatttctactggtaataaggactgtaatttcatgaaaataaaaactattttaacgccagtaacctgcgctctgctgataagtttttccgcccatgccgctaacgccgacaattataaaaacgtgattaaccgtactggcgcgccgcagtacatgaaggattacgattacgacgatcaccagcgttttaatccgtttttcgatctcggagcctggcatggtcatctgttgccagacggccctaacaccatgggcggctttccgggcgttgcgctgctgacggaagagtacatcaactttatggccagcaatttcgaccgcctgaccgtctggcaggacggcaagaaagtcgactttacgctggaggcatacagtattcccggtgcgctggtgcaaaaactgacagcaaaagatgtgcaagtcgaaatgactctgcgcttcgccacgccgcgcacgtcactactggaaaccaaaatcaccagcaataaaccgctggatctggtgtgggacggcgaactgctggaaaaactggaagcgaaagaagggaaaccgctttccgataaaaccattgctggcgaataccctgactatcagcgcaaaatcagcgccacccgtgatggcctgaaagtcacctttggcaaagtgcgcgccacctgggatctgctgacctccggcgaatcggaatatcaggtgcataaatccctgccggtgcagactgaaatcaacggtaatcgctttaccagtaaggcgcatatcaacggttcgaccacgctctacaccacctattcccatctgctgaccgctcaggaagttagcaaagagcaaatgcagatccgcgatattctggcgcgtccggcgttttatctcaccgcctcgcagcaacgctgggaagaatacctgaagaaagggttaaccaatccggatgcgacgccggaacagacgcgcgtcgcggtgaaagcgatcgaaacgctcaacggtaactggcgctcaccgggcggtgcggtgaaatttaacaccgttacaccgtcggtgaccgggcgctggttctccggcaatcagacctggccgtgggatacctggaagcaggcgtttgcgatggcgcatttcaatccggacatcgccaaagagaatatccgcgcggtcttctcctggcagatccagcctggcgatagcgtgcgtccgcaggatgtgggctttgtccccgacctgatagcgtggaaccttagccccgagcgtggtggcgatggcggcaactggaacgaacgtaataccaaacccagccttgccgcctggtcggtgatggaagtgtataacgtcacccaagataaaacctgggtggcagagatgtacccgaaactggtggcctatcacgactggtggttacgtaaccgcgatcacaacggcaacggcgtgccggaatatggcgcgacccgcgacaaagcccacaacactgagagcggcgagatgctgtttacggtgaaaaaaggcgataaagaagagacgcagtctgggctgaacaactacgcccgcgtggtggagaaaggccagtacgacagtctggaaattccggcacaggttgctgcatcgtgggaatcggggcgtgatgatgccgccgtctttgggtttatcgacaaagaacagttggataaatatgtcgctaatggcggcaaacgtagcgactggacggtgaaattcgccgaaaaccgcagtcaggacggaacgttgctgggctactcgctattgcaggagtcggtggatcaggccagctatatgtacagcgataaccattatctggcggagatggcaaccatcctcggtaagccagaagaggccaaacgctatcgccagttggcacagcagctcgcggactacatcaacacctgtatgttcgacccgactacccagttctactatgacgtacgtattgaagataaaccactggcgaacggctgcgcgggcaaaccgattgttgagcgcggtaaagggccggaaggctggtcgccgctgtttaacggtgcggcaacgcaggccaatgccgacgcggtggtgaaggtgatgctcgatcctaaagagttcaacacctttgtcccgctgggaacggcggcgttaaccaatccggcttttggcgctgatatctactggcgtgggcgcgtatgggtggatcagttctggtttggtctgaaagggatggagcgttacggttatcgtgatgatgccctgaagctggcggatacgttcttccggcacgccaaagggttaaccgccgatggaccaattcaggaaaattacaacccgctgacaggcgcacagcaaggcgcaccaaatttctcctggagtgccgcgcatttgtatatgttgtataacgattttttccgtaagcaataatttgcaactgctggcggatgcggcgtaaacgccttatccgccctacatgtgcaatcctcctggccggataaaacgcggcaagcgttgcatccggcaactgcaccgcgccactggcggatgcggcgtgaacgccttatccgccctacatgtgtgttcccgtaggtcggataagacgcgacaagcgtcgcatccggcatctgcaccgcgccactggcggatgcggcgtggacgccttatccgccctacatgtgcaattccgtaacctggataaaacgcgacaagcgtcgcatccggcgttatcaccgggcgtattctttttgaatcccatcacaaaccccgcactccccttttcccttttctccggcgacggctaaattagaactcatccgaccacataacaattattttacatactggacaattttatgagctacccgtcgctgttcgccccgctggatttaggttttaccacgttaaaaaaccgcgtgttgatgggctcaatgcacaccgggctggaggaatacccggacggtgccgagcggctggcagcgttttatgccgaacgcgcccgtcacggcgtggcgctgattgtcagcggcggcattgcaccagatttaacaggcgttggcatggaaggtggcgcaatgctcaacgacgccagccagatcccacaccatcgcaccattaccgaagcggtacatcaggaaggcggcaaaatagccctgcaaattttgcataccgggcgctacagctaccaaccgcatctggtcgccccgtccgcattgcaggcccccatcaaccgtttcgtgccccatgagttaagccatgaagagatcctgcaactgatcgacaatttcgcccgctgcgcgcaactggcgcgggaggcaggatacgacggtgtagaggtgatgggttccgaagggtatttgatcaacgaatttctgacgctgcgcaccaatcagcgtagtgaccagtggggcggcgattaccgcaaccggatgcgatttgccgtagaagtagtgcgtgcggtgcgcgaacgcgtcggcaacgacttcattattatctaccgactgtcgatgctcgacctggtcgaagacggcgggacttttgccgaaacggtagagctggcgcaggccattgaagcggcgggcgcgaccattatcaacaccggcattggctggcatgaagcacgtattccgaccattgccacgcccgtgccgcgcggcgcatttagctgggtcacgcgcaaactgaaaggccacgtctcgctgccgctggtaaccaccaaccggattaacgatccgcaggttgccgacgatattctctcgcgcggcgatgccgatatggtatcgatggcgcgaccgtttcttgctgatgcggagctgctgtcaaaagcgcaatcgggacgagccgatgagatcaacacttgtattggctgcaatcaggcctgtctcgatcaaatcttcgttggcaaagtcacctcgtgcctggtgaatcctcgcgcctgccacgaaaccaaaatgccaatccttcccgccgtgcagaaaaaaaatctggcggtggtcggtgcgggacctgctgggctggcgtttgccattaacgcggcggcgcgtgggcatcaggtaacattgtttgacgctcatagcgagattggcgggcagtttaatatcgccaaacagatccccggcaaagaggagttttacgaaacgctgcgctattaccgccggatgatcgaagtgacgggcgtgacgctaaaactcaatcacaccgtgacggcggatcagttacaggctttcgatgaaacgatcctcgccagtgggatcgtgccgcgcactccgcccatcgacgggatcgatcatccgaaggtattgagttatctcgatgtactgcgcgacaaagcgccggttggcaacaaagttgccatcatcggttgtggcgggattggttttgatacggcgatgtatttaagtcagccgggcgaatccaccagccagaatatcgccgggttctgtaatgaatgggggatcgacagtagcctacaacaggctggtggcttaagcccgcagggaatgcagatcccccgtagcccacggcagattgtgatgctccagcgcaaagccagcaaaccaggacaggggttaggcaaaaccaccggctggatccatcgcaccaccctgctctcgcggggtgtgaaaatgatcccaggcgtaagttatcagaagattgacgatgacgggctgcatgtggtgatcaacggcgaaacgcaggtattagcagtggacaatgtggtgatctgcgcagggcaagagccaaaccgcgcgctggcgcaaccgctgattgatagcgggaaaacggtgcatttaattggcggctgcgatgtggctatggagctggacgcacgacgggcaattgcccagggaacacggctggcgctggagatttaaatcgttatttgaagcgccggatgcaacgcatccggcacgtcgcgttaatcaataaacaaggcgggagaaatgccgaatcgcgttgccaattttttagcgtgttccagcgttaatttcctcttcccgctcaaaacgcgtgacaccatagatttactgccaatttccggcagatcggaaagggttaaaccatattgatccataagggtacgaatcacggctataccgccaggcatggcttgagccatggcattaaattccgcaaattcgggcgctgattcttcccacgcggttattttggcacacaccagatccagcaaggggttttcaggatcgttgagcagcagatgatctaccagttccagcgcctgggtgtattgttcctcgttctgaatacccgccagaaaaggtgccacagcagttagcttttctcctgcttgcaagatgtcggcaatcgcaatcattttttccccttagtacgatgaacagcggtaaagaaatcgtattctttatgcgtcataacttcacgtatgtagcacttttgcgattcaaaaaagaccattgctacaacacgtaattcattgcccccaacattgaaaacataatgcttatccagatatttgaagttatccagagatgggaatactgcttttaatgactcaggttttttgaaatatcccttagcaatcgtgttccccagagccaccaactccgttttatgttgcgggtatttttccgcagcatctttcaatgctttttgagttatcaggtgcattcttcatcacgtccgttgacaaattggcaatatgataacatccgttgccagattggcaacggatgaatttatctgtgtgacggaagaataaacgtagaaaaacgctaaacaagagaatgtagacgatggtgacagggattttttgttttatggaagcgcgattccagaactgggcagacattgccggatgcgacgcttgccgcgtcttatccggcctggagtaacgtgctgaacgtaggccggataaggcgtttacgccgcatccggcaggtaactcccaatcttaccgacgacgtcccagcttcaccgctttcagtaccacaaatttattattcgtcgcaatagtggtgcagttgccgaaaatcttcttcagtttatggaagtaatccaggtgacggttggcaacgatatacagctcgccgttgattttcaggcagcggcgggcgtggtggaacatctcccaggcgacgttatcggtcagcgcatgttgttggtgaaacggcgggttgcagagcacagcattaaagcggaaaggctccacgccggagagcgcgttgttgatcataaactcgcagcgatccaacgcctctggcatgttggtttcaacgttcaaacggctggaagcaaccgccatcggcgattcatcgacaaacaccactttcgcctgcgggtttttatcaagcagcgtcagaccaataacgccattaccgcaaccgagatcgacaatctccccttcgagattctctggcagatgttgcataaagaagcgcgcgccgatatcaagcccggtgcgggagaagacattcgcatggttgtggatagtccagtcagtaccttccagcttccagctaacggtctgcggcgcatcggccagctgcggttcattgaaagtgcaattaatcaggcgcgcttttttccatgccagcgtggtggtggttgggccgagcactttttcgaacagttccagcgtggaagtgtgaatgtcacgggccttggcaccggcaataatacgtgtatccgacgtgaccactttgcgcagcgcacgcagttgctgttccagcaatgccagtgttttcggcactttgatcagcaccacacccggctgttgcgggtagtcggcggtgctgtcgagaaacttcacgctcgactcatcaatcccgttgaggcgtaaattctcgcgcgtcgccagttcactgatgtatgagtcgccaatgctgtacggcttatgttccgccagtgcgcagcttaacgcaccaaaggcatcattcaggatcaacaccgggccgcggatttctgtgtcgtccaactgttgcagcaaatattcatccgccgcttcccacgcctgtagcgggttaacgtcatccgtcgccggaaaacgttgtagtgtcagtgaacggaaaccgttgtctaagtggctcatcggccctcctgaatgataaaatttcgacattgcccctgaaaagggtgcgtgagtataccctttttctctttttcgtgggcggttatgagcaatcttacttatcttcagggttatcccgagcagctactttcccaggtgcgaacactgattaacgaacagcgtctgggcgatgtgctggcaaaacgctatccgggaacacacgactacgccaccgataaagccctctggcaatatactcaggatctgaaaaatcagtttctgcgtaatgccccgccgatcaataaagtgatgtatgacaataagatccatgtgctaaaaaacgcgctcgggttacataccgctgtttctcgtgtgcagggcggcaagctgaaagcaaaggtggagatccgcgtcgctaccgtgtttcgcaacgcgccggaaccgtttttgcgcatgatcgtggtgcacgagctggcgcacctgaaggagaaagagcataacaaagcgttttaccagttgtgttgtcatatggaaccccagtaccaccagcttgagttcgacacccgactgtggctaacgcagttgtcgcttgggcagaacaaaatctgaaaatgatgtcaggcgttatcttttctttctttagcgcctaaaatcgacctcccccctttcgttaaggataacgaccatgctgcgcgcatttgcccgccttcttctccgtatttgtttttctcgccggactctaaagattgcctgcttactgttacttgtggcaggagcgaccatccttatcgccgatcgcgtaatggtcaacgccagcaaacagctgacctggagcgatgtcaacgccgttccggcgcgtaacgtgggtttattgctgggggcgaggccgggtaatcgctactttacccgacgtattgataccgcagcagcgttgtaccacgccggaaaagtgaaatggctgctggtaagtggcgataacggacgtaaaaattacgatgaagcatcaggtatgcagcaggctttgatcgctaaaggcgtaccagcaaaagtgatcttctgcgactatgccggattctcaacgctggattcggtagtgcgtgccaaaaaggtttttggtgaaaaccatatcaccattatctcgcaagaatttcataatcaacgcgccatctggctggcaaaacagtacggcatcgacgctatcggttttaacgcgccagacctcaatatgaagcacggtttttatactcaactgcgggagaaactcgctcgtgtcagcgccgtgattgacgccaaaatcctccatcgccagccgaaatatctcgggccttcggtcatgattgggccgtttagtgagcatggctgtccggcgcagaaataatgcgtatctgcgcacgtcgaagatgaaaaaggcgtgctacattgacgacagaatccctttatggagtatccacgcgttatgatacgtttcgctgtgattggtacgaactggatcactcgccagttcgtcgaggccgcccatgagagcggtaaatacaagttaaccgccgtatattcccgcagccttgaacaggcccagcacttcgccaatgatttttctgtcgagcatctgtttacctcgctggaagcgatggcggaaagcgatgccattgacgcggtgtatattgccagcccgaattccctgcatttttcccagacacaacttttccttagccataaaattaatgtgatttgcgagaaaccgctggcgtcgaatctggcggaagtggatgccgccattgcctgtgcgcgggaaaatcaggtggtgctgtttgaggcatttaaaaccgcctgcctgccgaactttcatttgttgcgccaggcgctgccgaaagtcggcaaactgcggaaagtctttttcaactattgccagtattcctcgcggtatcaacgttacctggatggtgagaatcccaacacctttaatccggcattctctaacggttcaattatggatatcggtttttactgtctggcgtcggcggtggcgttatttggtgagccgaaaagcgtgcaggcaaccgccagtttgctggcaagcggcgttgacgcccagggcgtggtggtgatggattacggtgatttcagcgtcaccttgcagcactcaaaagtcagtgattctgtcctggcgagcgagattcagggcgaagcaggatcgctggtgattgaaaaactgtctgaatgccagaaagtgtgcttcgtgccgcgtggcagccaaatgcaggatctcacccagccgcagcatattaataccatgctctacgaagcagagctgttcgctaccctggtggatgagcatctggtggatcatccagggctggcggtcagtcgcatcaccgccaaactgctgaccgagatccgccgccagactggggtgatttttccggcagatagcgtaaaactataattgccaaagtaaaacagtgtaaaaggtatgtaacagaccattgactggctgaatggtctgtcatactttgttacctgcaaaggggagtaacttcattgccggtcgatcgtcattacgatgtgtgaaaaaacacatccggtcaccgggcaacccgaaaggaatacgcagacgtattccttttttgttgtaagtgagaccttgccggaaggcgaggtctatgcataaaaagcagcggctgacgtcttccgacgttggccgtttttttatgtgtaaggaacttctatgaatactgtcggcacgccgttgctatggggcggattcgctgttgttgtcgccattatgctggctatcgacctgttgttgcaggggcgtcgtggggcacatgccatgaccatgaaacaggctgcggcctggtcgctggtctgggtgacgctgtcgttactgtttaacgccgctttctggtggtatctggtgcaaaccgaaggtcgcgccgttgccgatccacaggcactggcctttctcacaggttatctgattgagaaatcgctggcggtcgataacgtctttgtctggctgatgttgttcagctatttctctgttccggcggcattacaacgccgcgtgctggtgtatggcgtgctcggggcgattgttctgcgtaccatcatgatcttcactggcagctggctaatttcgcagttcgactggatcctgtatatcttcggtgccttcctgctgtttaccggcgtgaagatggcgctcgcccatgaagatgaatcaggcattggcgacaagccgctggtgcgctggctacgcggtcatttgcgcatgaccgacaccatcgacaacgagcatttctttgtgcgtaagaatggattgctgtacgccacaccgctgatgctggtactgattctggtggaattgagcgacgtgattttcgccgtggatagcattccggctatcttcgccgtgaccactgacccgttcattgtgctgacctcaaacctgtttgcgatcctcggcctgcgtgcgatgtatttcctgctggcgggcgtagcagagcgtttctcgatgctcaaatatggcctggcggtgattctggtgtttatcggtatcaagatgctgattgtcgacttctaccatattccaatcgccgtctcgctgggcgtggtgtttggcattctggtgatgacgtttattatcaacgcctgggtgaattatcggcatgataagcagcggggtggataatttttaatctgcctaagccgtgtaccctgtcattaacatgagcaccgttttctccctctcccttccagggagagggtcggggtgagggtaatttttcgcaccgatgctggcctgttcccctcaccctaaccctctccccaaacggggcgaggggactgaccgagtccttttttgatgttgtcatcagtctggaagccgcacgttggctttatttttatgtcaaagaaatgtaaccattaagtttcaaaatatgacctctctttaaaatccagcatttttcgcttcccgaagctgtaactttccttatactcgaccttgcaaacactttgttacatcctgaaagatgcgtcgacagaacgcaccagggatgtgcgacaacacaatgaaaggatcgaaaaatgactacgcaacgttcaccggggctattccggcgtctggctcatggcagcctggtaaaacaaatcctggtcggccttgttctggggattcttctggcatggatctcaaaacccgcggcggaagctgttggtctgttaggtactttgttcgtcggcgcactgaaagccgttgcccccatcctggtgttgatgctggtgatggcatctattgctaaccaccagcacgggcagaaaaccaatatccgccctattttgttcctctatctactgggcaccttctctgctgctctggccgcagtagtcttcagctttgccttcccttctaccctgcatttatccagtagcgcgggtgatatttcgccgccgtcaggcattgtcgaagtgatgcgcgggctggtaatgagcatggtttccaaccccatcgacgcgctgctgaaaggtaactacatcgggattctggtgtgggcgatcggcctcggcttcgcactgcgtcacggtaacgagaccaccaaaaacctggttaacgatatgtcgaatgccgttacctttatggtgaaactggtcattcgcttcgcaccgattggtatttttgggctggtttcttctaccctggcaaccaccggtttctccacactgtggggctacgcgcaactgctggtcgtgctggttggctgtatgttactggtggcgctggtggttaacccattgctggtgtggtggaaaattcgtcgtaacccgttcccgctggtgctgctgtgcctgcgcgaaagcggtgtgtatgccttcttcacccgcagctctgcagcgaacattccggtgaatatggcgctgtgtgaaaagctgaatctggatcgcgatacctattccgtttctattccgctgggagccaccatcaatatggcgggcgcagcaatcactattaccgtgttgacgctggctgcggttaatacgctgggtattccggtcgatctgcccacggcgctgctgttgagcgtggtggcttctctgtgtgcctgtggcgcatccggcgtggcgggggggtctctgctgctgatcccactggcctgtaatatgttcggtatttcgaacgatatcgccatgcaggtggttgccgtcggctttatcatcggcgtattgcaggactcttgcgaaaccgcgctgaactcttcaactgacgtgctgttcactgcggcagcttgccaggcagaagacgatcgtctggcaaatagcgccctgcgtaattaattgtttaacccctttcgtctacggcggaaggggttttctcaactttaaacggatcaattccccttttctgcatccgccagaaacgaatgatattcaggccattcataagcagaaaactaccctcaatcatcgtgccgcctatcgaccccgcccagaagttgtgaatcacccagcaacacgttgaaaaccacattacgcagcgcatggtcagccctttacagcagaatagcgcccaggtactgacaatcgtgccgataaccggcaatagttcgacaggatgatggaacttcgcgaggccaattccgccagtcagcacaataaaaatcgccattacccataagctgcgcgtgcgtaaggtaatcaatgtacgaatggcattaaggatggcactggcaccagcgggataggtgcccagaagaaaaaaatgtacgccaataacggcgctatagaccgaaagctgctttttgaagcgacgttcgtcacgattgaaaaatgttgtgataccaatcagaaaggcgatgacacccacgccctgggccagccaatacgcggtcatgataaatccttagcaggtatggaaaagcaaacggcgcttcacattatgaaacgccgttttttattaacaactcatttcgactttatagcgttacgccgcttttgaagatcgccagttcgcggaagtcgttacgctcgttacaggtttgcttaccgttggcaaactcaacgatggtgtcgataaattcttccagcaactgcggcatcgctttaccgtggatcaactgacccgcgtcaaagtcgatccagtgttttttcttcgccgccagttcactgttggtggcgattttcaccgtcggcacaaatccaccatacggcgtgccacgaccagtactgaacagcaccatatggcagcccgcacccgccagggcgctggtcgctacggcatcgttacccggcgcacttaacaagttcagccctggcgttttcagacgctcgccgtaacgcagcacgtcaaccacgacgctggaacccgctttctgggtacagccaagtgatttgtcttccagcgtggtgataccgcccgctttgttccccggcgatgggttttcatagatcggctgatcatgggcaataaagtactgtttgaagtcgttgaccatggtgaccagtttttcaaacgttgcttcgtcgcggcaatggtccatcagcaactgctctgcgccaaacatctccggcacttcggtcagtacggtagtaccgccgttagcaatcacgtagtcagagaaacgccccagcatcgggttagcagtaataccagaaagaccgtcagaaccaccgcactccagaccaaacttcagttcgctgagtttgcctggctcgcgtttatcgttgcgcatcacgttatacagctgatgcaaatgctcgattccggcttcgatctcatcatcctgctgttggcagatcatgaaatgaacgcgttcaggatcgatatcgcccagcgtttcacggaatgcggcaacctggttgttttcacagcccagaccaatcaccagcactgcgcctgcgttcgggtggcgcaccatgttttgcagcatggtgcgggtattaatgtgatcgtcgcccagctgtgagcagccgtaggtgtggctgaagaggaacacgccgtcagtaccttcggcgttgttggtctctttcagaaaacggttctggatctgccgcgcgatgccgttgacacagcccacggttggcaggatccacagctcattacgcaccccgacatcgccgttagcgcgacgatagatctgcacttcacgatctgccgcttgcgcaggcagatcctgaaaatcaggttgatagcgatactgatccagatcgctcagattcgtgcgcgtattgtgggcgtgaacgtgaacacctgccgcaatatccgccaatgcataaccaatcggcaggccatatttgatgacattggccccttttgcgatatccgttaacgcaaatttatgtccacgagcaacatcctggcgcagcgtaacagtctggttatcgacactgacttctgtgccttcagccaaatctgctaaagcgaccgcgacgttatccagcgcatggatcttgatgtattgcatatcaaccccagaccttagttcagttcaatggcgaagtagtcacgcgcattgttaaagcaaatatttttcaccatctcgcccagcaggttgatgtccgccggtgcttcgcccgcttccacccagcgaccgatcatctggcacagaatgcggcggaagtattcgtgacgggtgtatgacaggaagctacggctgtcagtcagcataccgacaaagcggctcagcagaccgagctgcgccagttgggtcatctgacgttccataccgtctttctgatcgttaaaccaccagccggaaccgaactgcattttgcccggcataccttcgccctggaagttaccgatcatggtgcccagcacttcgttatcgcgcgggttcaggcagtacagaatggttttcggcagcaggttttcttcattctgcttgctcagcaacttagacagctcttccgccatcggacggtcgttgatggagtcaaagcctacatccggccccagcagtttgaactgacgcaggttgttattacgcagcgcgccaatgtggtactgctgtacccagccgcgacgtgcatattcggcaccaaggaacaccagtaccgcagttttgaactgcgccacttcgtgctcgctcagggtttcgccagccagacggcgcgccagaatgctgtccagttccgcttcgttcgcttcagcaaacatcaccacatccagcgcgtggtcagacactttacagccgtgagcggcgaagtgatccagacgtttggtcagggcagtttgcaggtcagcaaagcggcgaatgtcggtatcggaaacttcgcccagcttcgccatgtagtcgttaaaggtcgcctgttcgatgttgaaggctttgtccggacgccagctcggcagcactttgatggtgaaagagccgtctttggcgatctctgcgtgatgctccagagaatcgatcgggtcatcggtggtgccgaccattttcacgttcatctgctgcatgatgccgcgcgcggagaagttatcctgcgccagcagttcgttacattcgttccagatttcatcggcagttgacggagaaagcaatttgccagtgataccaaacggacggcgcagttcgaggtgcgtccagtggtataacgggttgccgatagtgtgcggaacagtcgccgcccaggcgtcaaatttttcacggtcagacgcatcaccggtacacagacgctcggccacaccgttggtacgcatagcgcgccatttgtagtgatcgcctttcagccagatgtcatacaggtttttaaaacgatagtcttccgcaatctgctgcggcggcaaatggcaatggtaatcgaaaatcggctggtcttttgcgtagtcgtgatacagacggcgggcaaattcggtatctaacaggaaatcttcagtcataaacggagtcattttcgtcttcctctcaacgagtgagctagcttgcttatggtgcgatgctgacaaagttatcacaccaatttccagagtccgaagatattttcgtgagttagatcaataaacgtagttaaaaaaattactctcaaagtggtaaatctcgctgcaggccgcgccagtactggccttgctgtcgtcaggtaatgtccctacaaatattcccacatttgtgatggctctcaccttttaaagttgtatgacaagttatctttctgccgtcgcaaatcataagtcgacggaatgcaaattgccgattcattcatttgttagatgaatcgggttaaccggtacggaagccgaattagcacgaaactttcatggcaacgttcggggcgtgccggttttttttcggttacccggtcgtaactaacatcttcagcctctggcgggatgatggccgcgcttcctgcggatataacaaaacgatgaggttttacatgcgtaaaattaaagggttacgttggtatatgatcgcactggtgacgctcggcaccgtgcttggttacctgacgcgtaacactgtggcggcagctgcgccaactctgatggaagagttaaacatctccacccaacagtattcctatatcatcgcagcctattctgctgcttatacggtcatgcaaccggtagcaggttatgtactggatgtgctgggtacgaaaatcggttatgcaatgtttgctgtgctgtgggccgtgttctgtggtgcaaccgcgctggcaggtagctggggtggcctggctgttgctcgtggtgcggtcggtgccgcggaagcagcgatgatcccggcgggtctgaaagccagctccgaatggttcccggcgaaagagcgttccatcgcagtaggctactttaacgtaggttcttcgattggtgcgatgattgcgccgccgctggtggtatgggcaatcgtaatgcacagctggcagatggcatttatcatctccggtgcattgagctttatctgggcgatggcatggctgattttctataaacatccgcgcgaccagaagcatctgaccgatgaagaacgcgactatattattaatggtcaggaagcccagcaccaggtgagcacggcgaagaaaatgtccgttggtcagatcctgcgtaaccgtcagttctggggtatcgcgctgccgcgtttcctggcagaaccggcctggggtacttttaacgcgtggatcccgctgttcatgtttaaagtttacggctttaacctgaaagagatcgcgatgttcgcctggatgccgatgctgtttgctgacctcggttgtatcctcggtggttacctgccgccgctgttccagcgttggtttggtgtgaacctgatcgtttcccgtaagatggtcgtaacgctgggtgcagtgctgatgattggcccgggtatgatcggcctgttcaccaacccgtatgtcgcaattatgctgctgtgtatcggtggttttgcccaccaggcactgtctggcgcgctgattacgctctcttccgatgtgtttggtcgtaacgaagtggcaacggcaaacggtttaaccgggatgtccgcatggctggcaagtacgctgtttgcgctggttgtcggtgcactggctgacaccatcggcttcagcccgctgttcgcagttctggcagtgttcgacctgttaggtgcgctggttatctggaccgtgttgcagaacaaaccggcgattgaggtggcgcaggaaacacataacgatcccgcaccgcaacattaacgtttcgtgtaagttttagtttcccttcaaagccgccttctcaggcggctttttcatcactgcgagtagagctaaactcgcaaaagtggtataacaaatatagtctgccgtatcatgcctggagcgcatatggaaatcactgaaccacgccgtttgtatcaacaacttgccgctgacctgaaagagcgcatcgaacagggcgtctatctggtgggtgataaactgcctgcagaacgctttattgccgatgaaaagaacgtcagccgtacggtagttcgtgaagccatcatcatgctggaagttgaaggctatgtcgaagtgcgtaaaggttcaggtattcatgtggtttccaaccagccgcgccatcagcaggcggctgacaataatatggaattcgccaattacggtccgtttgagttgcttcaggctcgccagctcatcgaaagtaatattgccgaattcgcggcaactcaggtaacgaaacaggacatcatgaaactgatggccattcaggaacaggcgcgcggcgaacaatgcttccgtgattccgagtgggatttgcagttccacattcaggtcgctctggcgacgcagaactccgccctggcggctatcgtggaaaaaatgtggacccagcgtagtcataacccgtactggaaaaaactgcacgaacacattgattcccgtaccgtcgataactggtgtgatgaccacgatcaaatcctcaaggcgctgattcgcaaagatcctcatgctgctaagctggcaatgtggcagcatctggaaaacaccaagatcatgttatttaacgaaaccagcgacgacttcgagttcaatgccgaccgctatctattcgccgaaaacccggtggtgcatctcgatacagccaccagcggcagtaaatgaaattcctgtccgacaggcgctgcaatgcgcctgtttgtctcgtcggtaagcgaaaagtataaagtgtcagcctgtgtaaatcctctcgccaccctcccctgcattcagcaaaatcagactccacggacatgtaattttgataacgaacaacgttgacctttgttacaattagattcaatttgaatttatgtttttgaatgctttcttatctcacgatttaacagggaatagttcaggctgtgttgatgtatcaaacccgcagaacataccaaaacagcaataacattgcggtagtgcatcttttaaaaccagcgtggcgttaaccgattcaccaggaataatgaatggaacttttgacccaattgctgcaagccctgtgggcgcaggattttgaaaccctggccaatccatcgatgattggcatgttgtattttgtcttgtttgtaattttgttccttgaaaacggcttgcttccggcggcctttttaccgggcgacagtttactggtattggtcggcgtgttgattgcgaaaggcgcgatgggctatccgcaaacgattctgctgctgaccgttgccgccagcctcggctgctgggtcagctatattcaggggcgatggctgggcaatacccgcaccgtacaaaactggctatctcatttacccgcgcattatcatcaacgcgcacaccatctttttcataaacacggtttatcggcgctgttaattggtcgctttattgcgtttgtcagaacactgctgccgacgattgccgggttatcagggctgaataacgcgcgctttcagtttttcaactggatgagcggtctgctgtgggtattgatcctgacaactctgggttacatgctcggcaaaacgccggtatttttaaagtacgaggaccagctgatgtcatgcctgatgctgctcccggtggtgctgctggtgtttggcctggcaggttctctggtcgtgttatggaaaaagaaatatggaaatcgggggtaagggatgcaaatacctcgcatgtcgcttcgccagctagcctggtccggcgctgttttacttctggtcggcacgctgttgctggcctggtccgcggttcgccagcaagagtctacgctggcgattcgtgccgttcatcaaggcacaacgatgccagacggtttttcaatctggcatcaccttgacgctcatggcattcctttcaaaagtatcacccccaaaaacgacactctgttaattacatttgactccagcgaccagagcgccgccgcaaaagcggtcctcgacagaacattgccccatggctacatcattgcgcagcaggacaataacagtcaggctatgcagtggctgacccggttacgggataactctcatcgcttcggataacttcctgttatccgaaacatatcactcactttggtgatttcaccgtaactgtctatgattaatgaggcggtggttaacactaccgcttcgttgtctggacaatcgttcctttgtaataggtccgaatcacaatggaaggttcaagaatgaaataccgcatcgctttagctgtttctctctttgctcttagtgccggtagttatgccactaccctgtgtcaggaaaaggagcaaaatatccttaaggagatcagctatgccgaaaaacaccaaaaccagaatcgtattgacggtctgaataaagccctgagtgaagtccgggccaactgttcagatagccagctgcgtgccgatcatcagaagaaaatcgcaaagcagaaagatgaggtggcggaacgccagcaagatttagccgaggcgaagcaaaaaggcgatgccgataagattgccaaacgcgaacggaaactggcagaagcgcaggaagagctgaaaaagctggaagcgcgcgactactaactcacaatagtcactacttactcacctggagaaaactatgtcgaaagaacacactacggaacatctgcgtgctgagttgaaatccctttccgatacgctggaagaggtgcttagctcatctggcgagaagtcgaaagaagagttgagtaagattcgtagcaaagcggagcaggcactgaaacagagccgttatcgcctgggtgaaaccggtgatgccattgccaaacaaacccgtgtcgcggcggcgcgtgccgatgagtatgtgcgcgaaaatccgtggacgggcgtgggcattggcgctgcaatcggtgtagtgctcggcgttctgctgtcgcgtcgttaattatggcggacactcatcacgcacaagggcccggtaaaagcgttctgggcatcgggcagcgaattgtttctatcatggttgaaatggtagagacacgtctgcggctggcggtggtggagctggaagaggaaaaagcgaatctctttcaacttttactgatgctgggcctgacgatgcttttcgctgcatttggtcttatgagcctgatggtgctaattatttgggcggttgacccgcaatatcgcctgaatgcgatgattgccaccaccgtggtgttgctgctactggcactgattggcggtatctggacgctacgtaaatcgcgtaagtctacgttgctgcgccatacacgccatgagttagcaaacgatcggcagctgctcgaggaggagtcccgtgagcagtaaagtcgaacgtgaacgacgtaaggcgcaactgcttagccagatccagcaacaacggctggatctttccgccagtcgtcgtgaatggctggagacaacaggcgcttacgatcgtcgctggaatatgctgctaagtctgcgctcctgggcgctggttggcagtagcgtgatggcgatctggacgattcgccatcctaatatgctggtccgctgggccagacgcggttttggcgtatggagcgcctggcgtctggttaaaacgaccctcaagcagcaacagcttcgcggttaacttccctctggccggagccattccggccttatccctcaaattttttgaagatttttgacagttttccttgctaacaatcatcattcaccacgtttatgattctctccatcgacagcaacgacgctaataccgcgccattgcacaaaaaaacaatcagcagcctgagtggcgcagtggagagtatgatgaaaaaattagaagatgttggtgtactggtagcgcgcattttaatgccgattctgtttattaccgctggctggggaaaaattactggctacgcgggtacccaacaatatatggaagcaatgggcgtcccgggttttatgctgccactggtgattctgcttgagtttggtggtggtctggcaatcctgttcggtttcctgactcgcaccacagccctgtttactgcgggctttacgctgctgacggcatttttatttcacagcaactttgctgaaggcgtcaactcgctgatgttcatgaaaaacctgacaatttctggcggattcctgctgctggcaattaccggtccgggcgcgtatagcatcgaccgcctgctgaataaaaagtggtaagcacgcgctatacttaacgataaaaaacgaggaggaagctcctcgtttttgctattggaggagagaaaaatgggtcaactgattgacggcgtctggcatgacacctggtacgataccaaatctaccggcggtaaatttcaacgttcagcttccgcatttcgtaactggctcactgccgatggcgctcctggccccactggcacaggcggttttatcgcagagaaagatcgttatcatctctatgtttcactcgcctgcccgtgggcgcaccgcacgctgatcatgcgcaaactcaaaggactggaaccgtttatttccgtttccgtagtgaacccgctgatgctggaaaacggttggacctttgatgacagttttccgggagcaaccggagacacgctctatcaaaatgaatttctgtatcagctttatctccacgccgatccacactacagcggacgagttactgttcccgtgctgtgggacaaaaagaaccacaccatcgtcagcaacgaatcagcagaaatcatccgcatgttcaataccgcgtttgatgcgctgggcgcgaaagcgggtgattactaccctccagccctgcaaacaaaaattgacgaacttaacggctggatttatgacaccgttaacaacggcgtgtataaagctggttttgccaccagccaggaagcttacgacgaggcggtggcgaaagtgtttgaatcgctggcacgactggagcagattttaggccagcatcgttacctgaccggcaaccagctaaccgaagccgatattcgcctgtggactacgctggtgcgttttgatccggtgtatgtgacccacttcaagtgtgataagcaccgcatcagcgattacctgaatctgtacggttttctgcgcgatatctaccagatgccggggatcgccgaaacagtcaatttcgatcatatccgtaatcattacttccgcagccataagaccatcaaccctacggggattatttcaattggtccgtggcaggatctcgatgaaccgcatggacgagatgttcgcttcggttaaaaaaaggcaccttacgaggtgcctctgataattagctaagtgcatgttgttcatgtcggatgtggcatgaacgccttatctgacatacaaaacattgtacattcaatagattgcataacccgcgcagaccagataagcgtagcgcatctggcgattttgcgcttgtcatcagtcttagcgcgccttcacggcactttattaattccttgaacgaatatttactgccatttcattcacgtctattcttaatttgctgctttaaaaacaagtgattgagcaaaattgaggcaaaaatggactggtatctgaaagtactaaaaaattatgtcggtttccggggtcgtgcgcggcgcaaagagtactggatgtttattctggtcaacatcatctttacgttcgtgctggggctgctggataaaatgttaggctggcaacgcgctggtggcgaaggcatcctgacgacaatctacggtattctggtgtttttaccgtggtgggcggttcagttccgccgcctgcacgacaccgaccgctcggcgtggtgggcactgctattcttaatcccgtttatcggctggcttattatcatcgtctttaactgccaggcgggtacgccaggcgaaaaccgctttggaccagatccaaaactggaaccttaaaacaaatctgctcgccggatgtctgactcatccggcttttatcattatgttgatgaatgaataatttactaatgtttatttaaaatatttcaatgtcgttatataaattacctataaaaaataaccatgtatttatcttaaatatcaaaacctttataacatccgaaaaagaaagatacgaatagcatttacacaatacccggaatagactttcgtcacttttaattaaagggatgtttttatgcagtggtatttgtccgtattaaaaaattatgttggtttctctggtcgcgcacgtcgtaaagagtactggatgtttactctgattaacgccatcgtcggcgctattatcaatgtcattcaattgattttaggtctggagcttccatatctgtctatgctttatttgctggcaaccttccttcccgtccttgcgcttgctatccgtcgcttacacgataccgaccgttcaggtgcctgggccttgctcttttttgttccgtttattggctggctcgtgcttctggtttttttctgcacagaaggtacttctggcagcaatcgttacggaaacgatccgaagtttggttcaaattaatcttagaattggggcgatatttcgcccctttttattaacaataataaatattattttccgttaaaaagtttgggaatttcccgcagacaccaggatttcgcttcccccatactgtcacgacgccaggccataataatatcgatctcgctggtcgattccgggctgacgacacgcaaccgcccttccgcaatatctttttcgaccataggatacggcatcgtcgccacgccaagccccgccagtaatgcctgacgtttatcttcaatcgtgctcaccgttaagcgcggctgtttgtccagcagctgtacggtcaacaccgggcgctcacgagcggtatccgccaccgcaattccacgatatttcacacgcgtcacttcagataacggttccggctcctgatgaatcgggtgatcaggcgcggcaacgtagacgttcattaacgtatagagcttgcgcgagttgatctccgacgaggaacgaaaatgcatatccggcgcgataacaatatccgcccgcccctgctccagccgttcccacgcccccgccagcacttctgtgatgattgccagttgggtattggcttttgccgccagtttgtcgattaacgggaaaaaggcaggtgtcggtaccagcgcttcggtcacaatggtgagatgcgtttcccaaccgcgcgcgagagcttccgcatcagtagtcagtttatctgcggcttccagcaaaacgcgccctcgctccaacaacatcctcccgacattggtgaatttggtacgatggcccgagcggtcaaacagcaccacatccagctcttcttccagtttttgcatggtgtagctaagtgcggaaggcacgcgtcccagctcatccgccgccgccgcaaaactgccccggcgatcgatcgcatccataacccgtagtgcttccagcgttaatgccctttctttggccatttcgttctcattcaggaaatttgaacataccgggcagaatatctggctaacaatgtagcgtccagccccttaccataaaaggaagtaaagagaggtcaagaattatgattactacccgaactgccaggcagtgtggacaagcagactacggatggttgcaggcccggtatactttttcctttggacactacttcgacccgaaattgttaggctatgcctccctgcgtgtgcttaaccaggaagtgctggccccaggtgccgcctttcagccgcgaacctatcccaaagtcgatattttaaatgtgattctggatggagaagcagagtatcgcgatagcgaaggcaatcatgttcaggccagcgccggagaggcgttgctgctctctacccagccgggtgtcagctatagcgaacacaatctcagcaaagacaaaccgttaacgcgaatgcagctttggctggacgcctgcccgcagcgagagaatccgctgattcaaaagctggcgcttaatatgggcaagcagcaattaatcgcctcgccagagggtgcgatgggaagcctgcaattacgccagcaagtgtggctgcaccatatcgtgctcgacaaaggcgaaagtgcgaatttccagttgcatgggccacgcgcgtatttgcaatcgattcacgggaaatttcatgcgcttacgcatcatgaagagaaagcggcgctgacctgcggtgatggggcgtttattcgtgacgaggctaacattacgctggttgccgattccccactgcgcgctttgctgatagatttgcctgtctagttgtttttacagggagatgatgatgagtaaaaaattggccaaaaagcgccagccggtgaagcccgtggtggcgaaagaacctgctcgcaccgccaaaaattttggctatgaagagatgttgagcgagctggaagctatcgtcgcggatgctgaaacgcgtttagccgaggatgaagctaccgcgtaaagacaggttgccggatgcggcgaaaacgccttatccggcctacaaaatccaacaacattaacgaattaaacaacccgtaggccggacaagatgcgccagcatcgcatccggcacgatccccaaaacctggcgtttatctggccttgctcgccataatctcgataatctgccgatccgtttgctgcatcgaatggcttgctaacgcacacaggttggcaatcgactgctcaacatcatgcgccacaatcccttcattgccggtcacggcggtatcatccagcgccattaacaccgctttccacgcagccgaagcactggtcgaaaccttcatcgcgcagctgttcgacgcaccatcgcaaatcatgccgctgacatcgccgatcatactgctgatcgccatcgagatggtttcataacgcccatccaccagccatgccatcccggcggcggcccccattgctgcggtcgttgcggcacacagcgcagacaaacgcggtaactggttatggatgtaaattgcgctcaaatgcgaaagcatcagcgcacgcgccagccgttcatcatccgctccgaagtgttctgctaccaccaccacaggcattgttgcggtaatcccctggttacccgagccggagttactcatagccggaagcgtagcgccgcccatacgcgcatcggatgccgcgctggtacgaatcacaatggatgaagagagatctttcgccagcaaaccgcgctcgcactgtttttccagcgtcgcgccaatatgcagcccccacttaccgctcaaaccttcctgcgataacgcacaatttagcttcgcggaatcgagaataaagcggatcgccgcaaacgggacttcattgacgaacttcaggatctcagccagcgtcgttctggaaagcaccgtcagcggagactcttgctcgccctctgccacacacgcctgctgggtaaacaccacaccatcgtgcgtctcgatatgcacaatgttggtatgcccgccgacgatggtgacacacgcccacttctcaccgttccagactttggcgcgtgagaagaggatttcatcgcaaggttcctggatcttaacggagactttccccgccgccagcagtgctttggcatcggcaattgcctgcgctgttgcgtctttcagcacttccagcccggcgttggcatttccacctaacgcccccagcgccgccgcaatcggcagccccaccattcccgtgccgggaacggtgacgcccagaccgttcttcatcagatttggcgaaacccaggcttctacacgttcaaccggaccttccagttctgccgcagcaaccgccgccgccagcgccagtgaaatcggttcagtacatcccagcgccggttttacttcctcctgaacggcgaggatgtaacgctgccataacggatttaaagtcgaatcaaacatattaaaaaccttaaaatttcaggtaaatcaagaaaatgccaggaacggagaaacacacagcaacaaaccagtgacgataatcaggtacagagacatccctttgtatttgtgcaatgctggtactttgtaaaccagccacgccgggatcaggcaccctaccatgccgaaaatcgggctacagatagaggtgaagctcaacaccggtgcgttcagtacgatggcgctccaggccagcaaaatggcgaaaatcatgatgccgcgctgaacgagattttcgttaatcttctcggcaggcatcttgcgacgcaggatgttcattacgatcccttgcgttgcttcgcgaaagcctaaatagacgccaaagaatgcagtcatgacagcaaagatattgagaatgacgctgaccactttcacccacgctgcgccgtcaccgctaataaactgtgcggcaatcgccagcgcggaaatattctgctcataggcttttaccgcttcgtcatgtcccatcgccagcgtgaacgacacggcgtagaaaaagacggtgacaaacaaaatgccaaacgcgatattcattgcccgcaatgctttatgccgcgccacttcaattgatttttcccgcgagcgataagagatcaccatcggacttaacgtctggataaacagaatcgacgtcagggtaaacggcagcgtaataatggcgtttttcaccagcagccccagcggcggtagcgaaccgacgttatacagatgccacattcccaccatcgacacgcccagcgccgcgaccaccagcagcttggtcagcaccatgccggtcgaaattttgaataacaatttctcgccgcgtgaggagatcgccaccagaatgcaaatcagtaccagaccataaaagggactgtctgacagcaacccttccgtcacgccgaaggtatgcaggtaggaagcactatcgttggtgatggcggtggaatagacgaacatccaaatcaccagcattacgaaatagagcgcacctaacaggatgccccagtttttacctaaataaccgctaatgacgctcgggtaatctttacattctggtgattctgccagcgtattaataaacaatcgctgaaacagatacattgccgggtaaccaatcaccgatgagagcaaaaatacccacaatcccatcaaaccgacctgcaccgggagaaaaacaatccccgcgccaatcgccatcccgatactcataatcacccagccggtgtcagtactgtcgaatttgatcgcttctcgccactcgctctcactcattccagcacgacccgccggggtcgaagcgtctgcaatgacgcctttattcgatgcaatttccataatttctcgctcaatattttgtagggcttattatttttttccgagccgcatcaaggcgatatgcggtctacgtttttgcaggcgagttattagaataaagaaatgatacgcgcgaggtcagagaaaatcttcacaatcaagactttgaaataacggagatggataagaattttctactaaattaatcgcaggagaatattcattctctatttgcggcagatcacaaaaaaaaggtgcacatttgtgcacccaaggatgaaagctgacagcaatgtcagccgcagaccactttaatggccagtcctccgcgtgatgtttcgcggtatttatcgttcatatctttgccggtttcatacatcgtctcgatcactttatcgagtgaaacacgcggtgccgaggtgcggcgcatcgccatccgcgcggcgtttactgctttcacggcattaatggcattacgttcaatgcacgggatttgtacctgtccggcaaccggatcgcaggtcagcccaaggttatgctccatcgcgatttccgccgcattgcatacctgcgccggactgccgcccagtagttcagttaaccctgccgccgccattgaacaggccacgccaatctccccctgacagccgacttccgcgccagagatggaggcgttcattttatacagcgcgccaatagcccccgcggccagaaaatagcgggcaattgaccgctcgtttaccggacgacggaacttatcgtaataagccagtactgccggaataatgccgcacgcaccgttagtcggtgccgttaccacgcgcccgccagctgcgttttcttcactaaccgccagcgcgtacatgttgatccagtcgatgacattcatcggatcgttagagatgttatcgctggaaaccagctgacgacgcagcgctacggcacggcgcggcacattgagcggaccaggcagcacgccttcagtgttcatcccacgttcaataccgtcatgcatcacttgccagatacgggcaaaaccggcgtcaatttccgctttgctgcgcagcgctagctcgttgtgcatcatcagaccagatatagacaggccgttgtaatcacacattttcagcagttcacctgctgagtggaaatcgtaaggtacggacgtttcgacatcgtgcgacaggccgaagtgttcttcttcgacaataaacccgccgccgacagagtaataggttttacttaatagctcttcctgtcccttccaggcagtgatccgcattccgttctcatggcgaggcaacatttcgggatggaagataatgttctttgctacaggaaaatcaacaatatgcgcaccagatgccactggcagccgcccgctgcgcgttactaactctataaatgcagggatctcatcaatgacaacatcctgcggactgtttcctgccagtcccatgatgatggcgacatccgtggcatggcctttgcccgtcagtgacaacgacccgtacagatcgaccacaatatggctcgtcgcggttaataagccgctactttccagccgatcaataaaactttttccggcattcattggccccacggtatgcgaactggagggaccaatcccaattttgaaaatatcgaatgcactaatcatatccacaccctcggattgccgttcagtgaagtggagcggaacgaccttacgaccgtcccgctcacgaggctttacgcactacgtactgcgatggcttcaatttccagcttcacatctttcggcaaacgcgcgacctgcacacagctccgggtcggataggtcgcctgatgctcatcgaagaactgcttatagacttcgttgatggtggcaaaatcattcagatcggtgataaacacggtcatcttgatgatatcgcccacgctcagcccggcagcaaccacgatcgctttgacgttttcgaggcttaaacgcgcctgatcttgcacatcagccgggatctcaccggtctgtgggcaaaccggtatttgcccggaggtgaagaccatgctgcctaaatcaacgccctgaacataagggccgattgcgcctggggcacgttgcgtttcgataatctttttcatacatcctccggcgtcagagcgcctgggtaaaggtacgtgaaataacatcctgttgctgttcacgggtcagtgcgttgaagcgcacggcgtagccagagacacggattgtcaggttaggatatttttccgggtgctcgatggcatccagcagcatttcccgattcattacgttgacgttgaggtgttgaccgccttcgacatccgcttcgtggtggaaatacccatccagcaggccgacaaggttggttttacgtactggatcttctttgcccagcgccgcaggaacgattgagaaggtgtacgagatcccatctttggcgtaggtgaacggcagtttcgccaccgacgtcaatgaggccacggcacctttgcggtcacgaccatgcatcgggttagcgcccggcgcgaacggtgttccggcgcgacgaccgtccggcgtattaccggttttctggccgtacaccacgttagaagtgatagtcagaatcgactgggtagggacggcgttgcgataggttggcagcgctttaattttcttcataaagcgttcaaccaggtcgcaggcaatgctgtctacgcgctcgtcgttgttgccgtactgcggatattcaccgtcgatttcaaagtccaccgccaggccgttttcgtcacggattggtttcacgcgggcatatttgatggcagacagggagtccgtcgccaccgacaggcccgcgatgccgcatgccatagtgcgatagacatcacgatcgtgcagcgccatcagcgaagcttcgtagctgtacttgtcgtgcatgtagtgaatgatattcagcgcgctgatgtactgcaccgccagccagtccatgaagtgatcgaggctgtccatcactttgtcgtaatccagcacgtcgtccatcagcggtgctgttttcggcccgacctgaatcttcagcttctcgtccaccccgccgttaattgcgtagagcagcgttttcgccaggttagcgcgtgcaccaaagaactgcatttgcttaccaatcaccattgggctgacgcagcaggcaatcgcgtaatcgtcgctgttgaagtcagtacgcatcagatcgtcattttcatactgcaaggaagaggtgacgatcgacacctgcgcggcatattttttgaaggcaatcggtaattcttccgaccaaagaatggtcaggttaggttccggtgccggccccatagtgtgcagggtgtgcaaatagcggaaggagtttttggtcaccagcgtacgaccgtccagccccatcccgccgatcacttccgtcgcccagattgggtcgccggagaacagcgaatcaaattccggtgtacgcaggaagcgtaccatacggatcttcatgatgaagtgatcgatcagttcctgtgcctgctgctcattgagtacgccagctttaaagtcgcgctcaatgtagatatcgaggaacgatgccgtgcggcccagcgacatcgcgccgccattttgcgatttcactgccgccagataagcgaagtagagccactgcaccgcttcctgcgcattctgcgccgggcgagagatatcaaagccatatttcgccgccatttcctgaatctgcaacagcgcatgacgatgctctgccagctcctcacgcagacggatggtggcttccagatcctcgcctttttccagacgagactggagatcggcaaattgcagttcgcgttcacgtaccagataactgatgccatacagcgctacgcggcgatagtcaccgataatgcgcccacggccatagccatctggtaaaccggtcagcacgccagatttacggcagcgcagcatatccggtgagtaaacatcaaatacgccctggttatgggttttacgcagatcggtaaacagatattcaaattcactgtccatttctcggccataggcgtggaatgaacttttaatcatattaatgccaccgaacgggtgtagcgcacgtttcaacggcgcatccgtttgcaggccaacaattttttccagcggctggttaatatatcccgcatcatgagcggtaattgtggtggcaatattggtatcgaaatcaaccggcgcgtgggttgcattttcgatacggatgccttccattactttttcccacaattccgtggtggcaggcgtcgcttcggcgaggaaagattcatcgccttcatacggtgtatagttatgttgaataaaatcgcggacattaatttcgtttttccagtccgtacctttaaagccaagccatgcgtcggcgtacagcttatcgctggtatcaatatctaccttcatgaaaaataatctctctacaatacttcaactaaattatgcaaattctgcgggcgcgttaactttgcctaaatgaatggcatccaaagcaatcattttttcttcgttagtcggaataacggcacaaatgacacgcgcattttcactggaaacaattcgctcaccacaggagttagagcgattattcatttctgtatcaatctctaagcctaatacagccaaatgttccatgaccagacgacgaattaagcttgaattctctcctattccgccggtgaatataattccatccaggcgacgtaatgaagctgcgtgtccggcaatatgacgggcaattcggtgaacaaaggttttaattgccagttgcgcgcgttcgtgaccttcatgccaggctttttccagaacacgtaaatccgaagaaagaccggaaatacctaataatcccgactctttattcactacgcgttccaggtcacccaggctctggttggtttggctggcgacccaggacatcgcaccaaagtcgacatcgccactgcgggtacccatcatcaagccttccagcggcgtcattcccattgaggtatcaacactctgaccgttgcgaaccgcgcagattgacgcgccattgccaagatgcgccacaaccaggccggagtcatcttccgccagattcagcagcgaatgtgcgcgctgggaaacatagcggtgcgacgtgccgtggaaaccataacggcgtacacctaactcttcataatatttccacggcaggccgtataaataagcttccggagccatcgtctggtggaaactggtatcaaataccgccacctgagttacgcccggaaataattgctgcgccgattcaataccacttaaattggcgtaattatgcaggggtgccagtggagaaacgcgacggatattatcaatgacttcatcggtaataatggcggactcggtaaaaatactgccgccgtgagcgatgcggtggccaattaaggccacactgtcatttaaattccgtttttccagttcaaatgcaattgccttcaatgcaccttcgtagctgtggtgagccagcggtgctggctctcccccatttacggataagaatgcattttccgagttaataccgtcggcaatacctgacattaatacttcacagtcgctggcatcgagcacggaaaacttaatcgaagacgaaccacagttaataaccaaaacaaccggaaattcattcatctcttttctcatcctgagttacggattaaaacagtttgtatacgatgttcaggatggtcagcagaccaatcacggtaacaaacacgttatccagacgaccacggtatttcgccagagacggcgctttacggatggcatacatcggcaacaggcacagcagggatgcgataatcggtgcgcccatggcttcaatcaggtcaaggatgttcgggttggcgtaggcaacaacccaggtggagcccatgatgaagatcatgctgatagtgttcagtttacccagcgacactttagttttgtcgcctttataaccaaacttcaggaccaggccattcagaccttccagcgttcccagatagtgaccgaagaaagatttgaagatagccacgagtgcgatgatggaagccgcatattccagtgtaatcgcgaacgttgttttggtaccggtcatggacgcaaagtggttagccagataagaaagcactggaatattctgcgctttggcttccgccatgttggccggagacagagtaaacaggcagctaaaggcaaagaacatcaccactgcaaccatcagcatgctggcacgagaaatgatttgggaacatttacgttcggtgaagtcgcgaccgaagtctttctcatactcttcacgcttagaaaccacgaaggaagagacgattggcgagaagttaaaggagaaaaccatgatggaaatccccagccagacagtgatcaggataccgtcatgaccggttaacgacagcgaaccgaggtcaacctggtcgataactgcagagttccagtaagggatcagcgacaaagaaatcagcaccaggctggcgataaacggccataccaggtagctcatcactttaaccatcagatccttaccaaaccagatgacgaaagccatcagcagcaacaggaacagcgccacaaagccgcgattcagcggtgcaaagccgagctggttttcccagaacgtcataaaggtattggtaatagtaacgccataaatccacagcagtgggcaaatcgcgaagaagtacaggaacgtgataaccacgccgccagttttaccaaaatgctcttccaccgtttccgtaatgttgccggaagggttagagccagaaagacacagacgcgccagcgcccggtggcaataaaacgcgatggggtatgccaataccaacatcagaagaatcgggatcagtccgccaaaacctgcgcggatagggaagaacagcaccccggcgccgattgccgtaccaaacaagcctaacgtccatgtggtatctgatttacgccaggacgattgttttgtctggctggatacaatgctatctgaagtactcatatcctatcctcaacgaattaattaagcgtcaacgaaaccggtgatttgagagacgcgagaaagatcgatattgccgccggaaataatactgacggtttttctgttttgaatatattggtctaatttaccgcttaataatgcagcacatgccagagcgcctgcgccttcggtgacgactttattgcgctgaattaaggcaatcatactgtttctgatttcgtcttcgctgaccagcacgatgtcatcgactaattcacgaacgatttcgtaagttaaattacccgggcgggagacatcacaaccatccgccagggtgccggtagttcggtgcgtggttatttctccggagtggaaagaagccgccatgccgtgaacgttttcagactgtacgccaataacacgaatggtcgggttaatagatttaattgccaccgcaataccagcaattaaaccgccaccaccaattggcacaatcacgttatcgacatcatagagatcttccataatttccagaccaatcgttccctggccagcaatcactttcggatcatcgtaaggtgggataaaaatacggccttccatttcgacaatttcgctcactttagcgatagtgtcgttgaagttatcaccatgcagaacgacttctgcggagtagtcgcacgttgccgctactttggattttggcgcaccttttggcatcaccactttaccgtcgatacccagcatcgcgcaggagagggaaaccccttgcgcatggttgcccgcagaacaggccaccacgcctttgcgtttttccgcatcggtcagtgaacttaatttattaaatgcgccacgaattttaaatgaacccgtacgctgcatattttcaaacttcaggaatatttcacctttgcaacgttcactaaaatagttggagcgaggcatgcctgttttataaattcgcccagccagtcgttgtttcgcttcaataatgtcatcaatagcaaccggcagatcgtatgtaatatgcattataaaacctcttcgcctgaattaaatatgtaggtaaccgtaaccgacacctgcaagacagacaggtggattatttatgtttaaataaaaacaaataactaaccaacttctattaattgccttcgtctacacccattataagatgaatactctttggctaattccaccaaaaccgatgctgcttttttaatacgataatttttcgaccataccgcggcatattgtgccacaggtaatgtttcttcaaccggaatagtaataaattgattagaaccaaaaggtgacgtcatatcacaaggaattacagttaagaaatcagcattgagaacaagattataaattgtcacgactgagtcggttttaacgatgttttcaatactgatgccatttctttgtaacgtagtaagcagttcgctgtagtaccccatattagtttgtggcaacacccactgttcgttcttcaacgactccagcgtggtggtgccggtgcatgttcgggacttactggctaccagcacaaactcggactcgaacagcggctcaacatgtaaatcctgaagcttcatttctgcacttaacgtaccaatcgcaaaatccagtcgaccgtcgcggattgccggtaagaacgaagacagttgcgcttcatacatagaaacctgcgctttcgggaacacctctttgaacttgttgatcatccctgacataaaagtaaaaccaatcaatgaaggaaaaccaaatgagacttccaccaccgcctcagaagacataccgcttatctcattaaccatatttttcatttcacgggtaatggattcggaacgggagagtaacaattgaccggcaggtgttaatgttacaccggtatttttccgcaccactaattccacaccaaaataatcttcaatatcgttaatgattttactgacggccggttgagttaaccctaattcttttgcagccgagccgatagaaccacttctaatgacttcctgaaagactaccaggtgctgcgttttcggaagaagaatagtgctcataacgacctacgttaattacctcattgacggcatgaagtgtatcaaaatgaaatgaacaggatatgtgcgaccactcacaaattaactttcaatactttccagagtatcgttattacaattaaatacctttaaatatcaacaagttaaagtataaaaatcagcataaaccctgatttttgtcaaaaaaaatgacggggataaccatattttatggcgataacatcattcgttatgtggttaatacaaaaaaggggctgagaccatatttcaagcaattaccggataattaccaggcaaaatttgagttaaatttaatgagcaagttctcaaattttattataaataaaccattttcagtgataaataatgcggcatgtcacattttttcacgctatttgttggagaacaaacatttattttatcaatattttaaaatttcgaatacatgtattgatcatctcgaacaattgattaacgtcaactttttctcttctgacaggacgtcattttgtgaatgcaatcgttttccataaattcttctcccctcataggcgacgaatagcattttgtgttgaggatcacaaaacgaataattgctgatcgccgcgataaggtcagacaaagacaacaagggaaattttcacagagcttttgatcggcgtaggccacagaatgttgcttcgtttactgtaacgccgggtaaatgagcgttttttgatagtgcgaaagaaccctgcgaggaaaataagcatctattattgtttgtcatgatgacaaggcaggcatcaatgaaaggcttcccaattgcgcatatttttcacccttcaatcccgccaatgcacgcagtggttaacaatcacaatagaaatattgattattggacggtaaaaagaaagtttgcagaaattgtctccaccaatgacgttaataaaatttacagtataagtaatgaactgcggagagtattatctgcaataactgcattgaatttctatcatggcgatgttccttctgtcatgatccgaatccaaccggaaaatatgagtccattcattatagatatttctacaggagaacatgatgattatatcatacaaacattagatgtaggcacttttgcaccttttggtgaacaatgtacttgctcagccgtcaataaaaaagagctggaatgtattaaggagacgatttctaagtattgtgcaaaattcacccgaaaagaagccatcttaaccccccttgtgcactttaataaaaccagcattacttcagattgttggcaaattctctttttttcacccgatcattttaataatgatttttattgattatttataaaggataaaataatgttccctgtttcatcaattggtaatgatattagtagtgatttagtccgtcgaaaaatgaatgaccttcctgaaagcccaacaggaaataacctcgaagcactagcaccaggtatagaaaaactaaaacagacctctattgaaatggtcactttacttaacacgttacaacctggtggaaaatgcattatcactggtgattttcaaaaagaattagcgtacttacaaaatgtaattctttataatgtctcgtctcttcgtctggattttttaggttataacgcccaaattattcaacgatcggacaatacttgtgaacttaccattaatgaaccgttaaaaaaccaggaaatatccacaggtaatatcaatattaattgcccattaaaagatatttacaatgaaatcaggaggttaaacgtaatttttagttgtgggactggagatatcgttgatctatcctctctggacttacgtaatgtcgatttagattattatgatttcacagataaacatatggctaatactattttaaatccttttaaattgaattcaacaaattttactaatgccaacatgtttcaggttaattttgttagttcaacacaaaacgccacaatctcctgggattatttactaaaaataacgcctgttttaataagcattagcgatatgtattctgaagaaaaaatcaagtttgtcgaaagttgtttaaatgagcctggagacattaccgaagaacaattaaaaattatgagatttgcaattataaaatctataccaagggcaactcttacagataaattagaaaatgaattaacaaaagaaatatataaaagctcatcgaaaatcatcaattgcttgaacagaattaaattaacagagatgaaagaattctcatcagaaaaaatatatgattacatcgatataatcattgaagattatgaaaataccaaagaaaatgcttatctggtcgtcccccaaattaattatactatggatttaaacatagaagactctagctcagaagagttactttcagataataccctcgagaaagacgaaaattctccggacaatggctttgaggtcggggaatataacacatatgaagcatataactcagagaagcaatattttaccagagaggactatacgtatgattacgaccttttaaatgcaatatagacttaataacttcttacaaagtctattattaataccgtagatatttattcatcttaccctgtgcaccaaaagcaaaaactcactgacgcgggtttgaaactgatggcaaccgcaaaaatgcctgatgcgctacgcttatcaggcctacgccatctctgcaatatattgaatttgcgtgcttttgtaggcaggataaggcgttcacgccgcatccggcatgaataaagcgcactcaacaatctgaaacccgccggaacggtttattacgtacatcaggtaaaactgaccgataagccgctttcttttgggtatagtgtcgtggacagtcattcatctttctgcccctccaaaagtaaaaacccgccgaagcgggtttttacgtaaaacaggtgaaactgaccgataagccgctttcttttgggtatagtgtcgtggacagtcattcatctttctgcccctccaaaagcaaaaacccgccgaagcgggtttttacgtaaaccaggtgaaactgaccgataagccgctttcttttgggtatagcgtcgtggacagtcattcatctttctgcccctccaaaagcaaaaacccgccgaagcgggtttttacgtaaatcaggtgaaactgaccgataagccgggttctgtcgtggacagtcattcatctaggccagcaatcgctcactggctcaagcagcctacccgggttcagtacgggccgtaccttatgaacccctatttggccttgctccgggtggagtttaccgtgccacggactgttaccagccgcgcggtgcgctcttaccgcaccctttcacccttacctgatcccgcttgcgcgggccatcggcggtttgctctctgttgcactggtcgtgggtttcccccccaggcgttacctggcaccctgccctatggagcccggactttcctcccctccgcccgtctcccccgaagaggacgacgacgaagcggcgactgtctggtcagcttcggcgcgcagtatagagggtttgcgcgcccttgtcaccccgcgttgcgcattccaatcgccagtgtcgcggcgatattacgtgaagcacggcagatattgtcataagccccgcggaatgcttcgtccaacgtacctatgctggtcaatacgctgaagaccgcatcaatgccatgctgatgtacaacgccaacatcatcggtcaggctacccgcaatgccaatcaccggtttatggtacttcttcgccacgtttgcgacaccaatcggtaccttcccgtgaatactctggctgtcaatacgcccttcaccggtgatcaccagcgtacaatcgtgaatatgttcctccagattcagcgccgtagtgacgatttcaataccacttttcagttccgcaccaagaaacgccattagcgccgcgcccataccacccgcagctcctgcaccggggacatctttcacatcaacatgcagcgcttttttaatgacctcggcatagtgagagaggttattgtccagctcaacaatcatcgcttcactggctcccttttgtgggccaaagatgcgcgatgcgccgttatcgcccaccagcggattggtgacatcacaagcgacgcgaatgacgcaatcttttaagcgcggatcgaggccggaaatatcaatatcattcagagtattaagactaccgccgccaaaaccaatttcattgccgttggcgtcgcataatttcgcccccagcgcctgtaccatgcctgcgccgccatcatttgtagcgctgccgccaatgccgataataatgtttgtcgcaccgctctccagcgcctgcaggattaactcgcctgtgccgcgtgaagtggtcacgagtggatcgcgtttttccgcaggtaccagctccagcccactggccgccgccatttcaataaacgcggttttgccatcgccggagatcccccaactggcattcactttctcgcccagcggccctgtaacccaggcgtgacgttcagccccctgggtggctgcaatcatcgcttccaccgttccttcgccaccgtcggcaaccggaacagaaacgtactgtgcatcaggaaaaatttcccgaaatcctttttctatcgcctgcgcaacctcgctggcagataaactttctttataagagtctggggcgattacgattttcatacctatgcctgttaccacatgacgccggagggcgtttctcttattcggcctggattccaggcccggattgcaatacgccatccgggcacgacgtcattaacgagtaacttcgactttcgccagtttttcgtagtagcacgccagggcgctatgatccgccgttcctaaaccatctgctcgcagtgcctgcatcatctccataaccgcagctgtgagcggcagttgtgcgccgacgccgtgagaagtatccagcgcattcgccagatccttaatatgcagatcaatacggaagcccggcttgaagttgcggtccatcaccatcggcgctttggcatccagcacggtactgcccgccagtccaccgcgaattgcctgataaaccaggtccgggttaacgcccgctttagttgccagcgttaacgcttctgacatcgcggcaatattcagcgccacaatgacctgatttgccagtttggtgacgttacctgcaccgatttccccggtatgcaccacggaacccgccatcgctttcatcaaatcatagtatttgtcgaaaatagccttgtcgccgcccaccatcactgacagcgtaccgtcgatggctttcggttcaccgccgctcaccggagcatccagcatatcaatgcctttcgctttcagcgcttcgctgatttcacggcttgccagcggtgcgatagaactcatatcgatcaataccgtacctggcttcgcgccttcaataatgccattctcacccagcgccacctctttcacatgaggggagtttggcagcatggttatgatgacgtcgcactgttcagcgatcgctttagccgtagacgctgtttctgcacctgcagcaatcacgtcagcaatagcttctgggttacggtcagcaaccaccagcgagtaacctgctttcagaaggtttttactcattggtttacccataatccccaggccaataaaaccaactttcatagtcatatcaatcatctctcttgttgcggtggtggttattttttaaaggtatcagccagtttctgagtggcagagcggaagacgccgagatcgctgccgacagccacaaacgtcgcgccccattccagataacgacgcgcatcggcttcgaccggcgcgaggataccgctgggtttgccgtgcgcgctggcacggttaaaaatgtgctgaattgctttttgtacatccgggtgtgatgcattgccgagatggcctaatgccgcggccagatcgctggggccgacgaagatgccgtctacgccttcggtagcggcaatggcatcgacgttatctacgccctgctgactttctatctggaccagaatagtgatgttcttgttcgactgagcgaaataatccgccacggtgccaaacatattggcgcggtgagaaacggagacgccgcgaatgccttccggtgggtaacgggttgatgccaccgccagctctgcttcctcttttgtttctacaaaaggaatcaggaagttatagaaaccgatatccagaagacgcttaataattaccggctcgttggtcggcactcgcactactggcgcgctggcgctgcctttcaaggccattaactgcggaataaacgtggagatatcgtttggcgcatgttcgccatccagcaccagccagtcaaacccagccaaaccaagaacttcagtgctaatcgggttagagagtgctgaccagcaaccaatttgtacctgtttcgcagccagtgcggctttgaatttattcgggaaaacatcgttattcatcgcttatacctttgcttatttctgcaattccatacgtttaatgtcgccaactacgaagaggtagcagaccatcgccatcagcgctgaacatcccacgaaaaccagtgctgcattgaaggagtgcagttcacttaccaggtagccaatcaccagtggagtgacaatggaggcaacattgccaaagacgttaaagacgccgccgcagaggccaacaatctctttcggcgcggtgtcagaaatcaccggccagcccagcgcaccaaatcctttgccaaagaaagccagcgccatcagcatgaccaccagcgtggtgttgttggtgtagttacataagatgatggtggaagccagcaacattcccagcacaatcggtagcttacgtgccagggtcagggataaaccgcgtttgatcagataatccgagaagacacctcccagcacgccgcccgcaaaaccacacagtgctggaatcgaggcgaccagacccactttcagaatcgacatgcctttttcctgcaccagataaatcgggaaccaggtgaggaagaaccaggtgatggtgttgataaaatattgtccgaaaaatacgcccagcatcatgcggttagagagcaattgcttgatgtaatgcagtttgggtccgcttgctgccgcactgcccggctttttgtggtccatatcgaccaccgcgccattttcagagataaacttcagctcttccgcagacatacgtgggtgatctgtcgggttatgaatcaacttgatccacagcgccgtcagcacaaaaccaatcacccccataacggtaaagacgtgctcccagccccaggcgaaagtcagccagccaagcagcggcgaaaagagcgccagcgagaaatattgcgccgagttaaagatggcggaggcagtaccacgttctttcgtcgggaaccaggcggcgacaattcgggcgttcgccgggaatgatggcgcttccgagaagccgagcataaagcgcataaagaacatggagatccctgcccaggccagcgggaacatatcaacaaagccttgcaggaaggtgaatagcgaccagaaaaagaggctgtaggtgtaaacttttttcgagccaaacttatcaagcagccagccgccggggatttgcatcagcaagtaggcccagccaaaagcggagaagatgtaacccatcgaaaccgcacttaactgcaactcttttgccacttcggtaccagcaatagacagcgttgcacgatcggcgtagttaacggcggtaacaataaaaataatcagtaatattaaatagcgggtatgcacgcctttctttttttcgtcaacggtgtccagaatcattttatttacctcgggtacttatgctgatttttattattatggggaaggtgttatttatgagtttcatttatgccgtaacgacaatgaactcgggaattagtataagcagcgcgagaataataatcattgtgcaaatgctaatttaattaatactatttaaatattattttgagcatatgcacataaggttgcgcgctaaagcacagatttgcgctttaccttaccgggcggcactgcaatccctgaaatgattgacattgatcacatttctgcgtttaaactcctgacattcttatttcacccaatgaagtcatttatttttaaatgagaccaggtcctcattttaataacccctggctggagaatattgcacaatggccaacatcgaaatcagacaagaaacgccaactgcgttttatataaaagttcacgacacagataatgtggcaattattgttaatgataatggcctgaaagcaggaacgcgttttccggatgggctggaattaattgaacatattccccaggggcataaagtcgcattgctggacattccggctaatggtgaaattattcgttatggcgaagtgattggttacgccgtgcgtgcaatcccacgcggaagctggatcgacgaatcaatggttgtactaccggaagcgccgccgttacacacgctgccactggcaaccaaagtcccggaacccttaccgccgctggaaggatacacctttgagggctatcgcaatgccgatggcagcgtgggcaccaaaaacctgctcggtatcaccaccagcgtccactgtgtggcaggcgtggtggactatgtagtaaaaatcattgaacgcgatctgctaccgaaatacccgaacgtcgatggcgtggtggggctgaatcatttgtacggttgtggcgtggcgattaacgcaccggcggcagttgtacctatccgtaccattcacaatatttcgctgaatcctaactttggcggcgaagtaatggtgattggcctgggttgtgaaaagttgcagcctgagcgcctgctgactggaacggatgatgtgcaagctattccagtagaaagcgccagcattgtcagtttgcaggatgaaaagcatgtcggttttcagtccatggtcgaggatattttgcagatcgccgaacgccatctacaaaaactgaatcaacggcagcgagaaacctgcccggcttcagaactggtcgttggtatgcagtgcggtggcagcgatgcgttttctggtgtaacggcaaacccggcggttggctatgcgtctgatctactggtgcgctgcggcgcaacggtgatgttttcagaagtaacggaagtgcgtgacgcgatccatctgctgacaccacgcgcagtgaacgaagaggtcggcaaacggctgctggaggagatggagtggtacgataactatctcaatatgggaaaaaccgaccgcagcgccaacccttcgccgggcaacaagaaaggcggtctggcaaacgtggtagagaaggcactcggctccattgctaaatcgggtaaaagcgcaattgttgaagtgctgtcgcccggtcaacgcccgactaaacgcggattaatttacgccgcgacgccagccagcgattttgtctgtggcacgcaacaggtggcttcgggtatcacagtgcaagtgtttacgaccggtcgtggtacgccgtacggcctgatggcggtacccgtcattaaaatggcaacccgcaccgagctggcgaaccgctggtttgatttaatggatattaatgcgggcaccatcgctaccggcgaagaaactattgaagaggtgggctggaagttgttccactttattctcgacgtcgccagcgggaagaagaaaaccttctcggatcaatgggggctgcataaccagctggcggtgtttaacccggcaccggtgacctgatttcttttggaacgtccctcgcaaaacatggccttagtgccatgtttttattgtttaaagcccccacgtccattaataatgcatttgcattaccttagttcaagcttataatttgagcagaaaacaggctgtaaaaggacagtgaatcatgcccgctaatgctcgctctcacgctgtactgaccactgaatcaaaggtcacgatacgcggacaaacaactatccccgcgccagtgcgtgaggccttaaaactgaagccaggccaggacagcattcattacgaaattctgcctggtgggcaagtatttatgtgccgactgggagatgaacaggaggatcatactatgaatgcatttttgcgttttctggatgcagatatccagaacaacccgcaaaaaactcgtccattcaacattcaacaaggaaagaaacttgtcgctggcatggacgtcaacattgatgatgagattggcgacgacgaataatggattttccacaaagggttaatggttgggcgctatatgctcatccctgttttcaggaaacctacgacgctttagttgccgaagtcgagacattaaagggaaaagatcctgaaaattatcagagaaaagccgccacaaagttattggcggtagtccataaagtgattgaggagcatatcacggtcaatccatcatcaccggcattccgtcatggcaagtcgttaggctctgggaaaaataaagactggtcacgggtaaaatttggtgctggtcgttatcgtctcttctttcgttatagtgaaaaagagaaagtcatcattctgggatggatgaacgatgaaaacactctgcgcacctacggtaaaaaaacagatgcctataccgtattcagcaaaatgttaaaaagaggacatcctcctgccgactgggaaaccctcacccgagaaacagaagaaacccattgatggtgttcacaatgcccgccgaacgcattcgtgttgaccagcgggcatcctttctcactccccgaccagaatcacttcaaccccagcctttcgcagtccttccaggctatccgcaggaatgccttcatcaacaatgatcatgtcgatacgttgagtatcaatgatcttatgtaaactggaacgattgaacttactggaatcggtgaccacgatgatccgttccgcaacttcgcacatccgacggtttaaacgagcttcatcttcattatgtgtgctgacgccgcgctccagatcgatcgcatctacaccaagaaacagcatatcgaagtggtaattttgcagcgattgctcagcctgatcgccgtaaaaagattgcgactgacggcgcaaatgcccgccggtcatcagcagctcaacgccttccgcttccagcaacgcattagccacgttcataccgttggtcatcgcaattacgtcagtgtgcttgcgcatcagacgagcaatctcaaaagtggtggtcccggaatcgaggataacccgatgacctggctgaatcaactcaacggcagctttcgcaacgctgcgtttcatcgcggtgttcagtgcgcttttatcttccactgatggctcgactgacggcgtcgtgctatcgcagatcaacgcgccaccataggcacgcacagcgatcccctgcttttccagaaacgccagatcgttgcggatcgtcacagtagatacgccatacaatgccgacagatcgttaacctgcacactcccttgctgtcgcagacgctgaatgatctgttctcgtcgctcgctggtgccagtcactcgcttctcacctgaagcgtcggtattactcatagtaagtcctttcgtaaaactttcgtttcatttcgttttgcctattaacgcctttctattaagcaaatgcaagcccaccttgcccattgacgcaagctactctcgtttcagtgactttcattatgtttcttttgtgaatcagatcagaaaaccattatctttcgttttatttttatctcaccatgacgcagtatcaactgaaacaaaacgaaagattaatatcgcagtaatctgaactggagaggaaagtgaaacatctgacagaaatggtgagacagcacaaagcgggcaaaacaaatggaatttatgccgtttgttccgcacatccgctggtgctggaagctgcaatccgctacgccagtgcaaaccaaacgccgttactgattgaagcaacctccaatcaggtagaccagttcggcggttataccggaatgacgcccgccgattttcgcggctttgtttgtcagctcgccgactcgttgaatttcccgcaggatgcgttgattctgggtggtgaccatctggggccaaaccgctggcaaaacctgccggccgctcaggcaatggccaatgccgatgatttgattaaaagctacgttgcggcaggattcaaaaaaatccaccttgattgcagcatgtcctgtcaggacgatccgattcccttaactgatgacatcgtggctgaacgcgccgcccgtctggcgaaagtggcggaagaaacctgtcttgaacactttggcgaagccgatctggagtatgtcattggtaccgaagtgccggtacctggcggcgcgcatgaaaccttaagcgagctggcggtcaccacgccggatgccgcccgcgccacgctggaagcccatcgtcacgcctttgaaaagcaaggtttgaatgccatctggccacgcatcattgccctggtggttcaacccggcgtcgaattcgatcacaccaacgttattgattatcagcccgccaaagcgagcgccttaagccagatggtcgaaaactacgaaacgctgattttcgaagcgcactctaccgattatcaaacgccgcaatcgctgcgccagctggtgattgaccactttgccattctgaaagttggcccagcgctgaccttcgccctgcgtgaagctctgttctctctggcggcgattgaagaagaactggtgccagcgaaagcctgttctggtctgcgtcaggtgctggaagacgtgatgctcgaccgcccggaatactggcaaagccactaccacggtgacggcaacgcgcgtcgtctggcgcgtggttatagctactcggatcgcgtgcgctattactggccggacagccagattgatgacgctttcgctcatctggtacgtaatctggcggattcaccaattccgctgccgctgatcagccagtatctgccgctgcagtacgtgaaagttcgctccggcgagctgcagccaacgccacgggaactcattatcaaccatattcaggacatcctggcgcagtaccacacagcctgtgaaggccaataagcaaaacaaagaggaacacgctatgccaaatattgttttaagccggattgatgaacgcttgattcacggtcaggtcggcgttcaatgggtcggatttgcgggggcaaatctggtgctggtagccaacgatgaggttgccgaagatccggtacaacaaaacctgatggaaatggtactggcagaagggatcgccgtacgtttctggacgctgcaaaaagttatcgacaacattcatcgcgccgccgatcgacagaaaatcctgctggtttgtaaaacacccgccgatttcctgacgctggtgaaaggtggcgttccggtgaatcgcattaacgttggcaatatgcactacgccaatggcaaacaacaaatcgccaaaacggtttctgtggatgcgggcgatatcgcagcatttaacgacctgaaaaccgctggggtggaatgcttcgttcagggcgtcccgacagagcctgctgtggacctctttaaattactttgagggattcatcatggaaatcagcctgttgcaggcatttgcgttgggcattatcgcctttatcgctggcctggatatgtttaacggcctaacccatatgcaccgcccggtggtcctcggcccgttggtcgggctggtacttggcgatctgcataccggaattttaaccggcggtacgctggaactggtgtggatggggctggccccgctggcgggcgcacagccgcctaacgtgattatcggtactatcgtcggcacggcgtttgccattactactggcgtgaaacccgatgtcgcagtaggtgtcgccgtacctttcgctgtcgcagtacagatggggattaccttcctgttctcggtgatgtccggcgtgatgtctcgctgcgacctggcaacaaacccgcgccgcatttgatgctggtgccgacggcctggtgcattgctataacgggatgacaggtttacatcaccgcgaaccgggaatggttggcgcgggattaacggacaagcgcgcctggctggaactgatagccgatggtcatcatgtgcatccggcggcaatgtcgctgtgttgttgctgtgcgaaagagagaatcgtactgatcaccgacgcgatgcaggcagctgggatgccggatggtcgctatacgttatgtggtgaagaagtgcagatgcacggtggcgttgtccgtaccgcgtctggtgggctggcgggcagtacgctgtctgttgatgcggcagtgcgcaatatggtcgagttgacgggcgtaacgcctgcggaagccatccatatggcgtcgctgcatccggcgcgaatgctgggtgttgatggtgttctgggatcgcttaaaccgggcaaacgcgccagcgtcgttgcgctggatagcgggctacatgtgcaacaaatctggattcagggtcaattagcttcgttttgatagtttgctcctttattgggccttcacttcccccgtaaggcctttctttttctttcgttttgatctgtgcagcggtgtcggatgcgacgctaacgcgtcttatccgacctacagttggtgaccgcaaggccggataaagcgtttgcgccgcatccagcaatcccttttgcttcctttatcttttctttcaacgatcacaaatttcgttttatttcttttttctccattgaactttcagtttcttttctatagattttaatcaacgaaagacatcaccaagtgaaatgaaacgaaaggcaagtgaaagcgacaacgcccgacgtcaagttcatcagactaaggattgagttatgccagaaaattacacccctgctgccgccgcaaccggtacatggactgaagaagagatccgccatcagcctcgcgcatggatccgttcactcaccaacatcgacgcgctacgttccgcgctcaataacttccttgaaccgttactgcgcaaagagaatctgcggatcatcctgaccggagccggaacgtcggcatttatcggtgacatcatcgcgccgtggctcgccagccataccggtaaaaacttcagcgccgtaccgaccaccgatctggtcaccaatccgatggactacctgaacccagctcatccgctgctgttgatctccttcggtcgatccggcaacagcccggaaagcgtcgcagccgtggaactggcaaatcaatttgtaccggaatgctatcacctgccgatcacctgcaacgaagcgggcgctctttaccaaaacgcgatcaacagcgataacgcgtttgccctgctgatgcccgcagaaacgcacgatcgcggctttgcgatgaccagcagcattaccaccatgatggccagctgcctcgcggttttcgcacctgagacgatcaacagccaaaccttccgcgacgtggcggatcgttgccaggcgatcctgacctcactgggcgatttcagcgaaggtgtgtttggttacgcaccgtggaaacggatcgtttatctcggtagcggtggcttacagggcgcagcacgcgagtcggcgctgaaagtgctggaactgacggcgggtaaactggcggccttttatgattctccaaccggattccgtcatggaccaaaatcgctggtcgatgacgaaacgctggtggtggtatttgtctccagccacccttacacccgtcagtatgatcttgatctgctggctgaacttcgccgtgacaaccaggcaatgcgtgtaatcgccatcgccgcggaaagcagcgacatcgtcgctgccggtccacatatcatcctgccaccgtcacgtcactttatcgacgttgagcaggcattttgcttcctgatgtacgcccagacgtttgcactgatgcagtcgctgcacatgggcaatacgccggataccccatcagccagtggcaccgttaaccgcgtggtgcaaggcgtaatcattcatccgtggcaggcataagaggatcgcattatgagcattatctccactaaatatctgttacaggacgcccaggccaatggctacgcggtgcctgcttttaacattcataacgccgagacgatccaagcgatcctcgaagtgtgcagtgaaatgcgatcgccggtgatcctcgccggaacgccggggacctttaaacacatcgcgctggaagagatctacgccctgtgtagcgcctattccacaacctacaacatgccactggcgctgcatctcgaccaccacgaatcgctggatgatattcgccgtaaagtccacgcaggtgtgcgcagtgcgatgatcgacggcagccacttcccgtttgccgagaacgtgaagctggtgaaatcggttgttgacttctgccactcacaagattgcagcgtggaagcagaactgggccgcctgggcggtgttgaagatgacatgagcgttgacgccgaaagtgcattcctgaccgatccacaagaagctaaacgctttgtcgaactgactggcgtcgacagcctggcggtagcgattggtacggcgcacggcttatacagcaaaacgccgaagattgatttccagcggctggcggaaattcgtgaagtggtggatgttcctctggtgctgcatggtgccagcgatgttccggatgaatttgtccgtcgcactattgaacttggcgtcacaaaagtgaacgttgccacagaattaaaaatagccttcgctggcgcggttaaagcctggtttgcggaaaatccgcagggtaatgatcctcgttattatatgcgcgtcggaatggatgcgatgaaagaagttgtcagaaataaaattaatgtctgtggttcagcgaatcgaatttcagcataatcattagttttttatgatttatcccaatgtacttcccgattaatatcggggagtgccttaatggaaaaggagataactaaaccttaataaatacatcactacaatatcgcaacaataatatatttaaaaaaattatattattcaactttatggtgaggattacacaatgaccagtccaaatattctcttaacccgtattgataaccgtctggttcacggtcaggttggcgtgacctggacatccaccatcggtgcaaatctgctggtagtcgtggatgatgttgtcgctaacgatgatattcaacagaaattaatgggtattaccgcggaaacctacggctttggcattcgtttctttactatcgaaaaaaccattaacgtcatcggcaaagctgcaccacatcagaagatcttcctgatttgccgtacgccacaaacggtacgtaaattggtagaaggtggtattgacctgaaagatgtcaacgtcggcaatatgcatttctcggaagggaaaaagcaaatcagcagtaaagtttatgtcgatgaccaggatctcacggacttacgttttattaaacaacgtggcgtgaatgttttcattcaggacgtccctggcgatcaaaaagaacaaatccctgactaaatctaaaatcgccttaatattggtttgaggtaataaaaatgcatgaaataaccctacttcagggattatccctggcggcgttagtttttgttctggggattgatttttggctggaagccttatttttattccgcccgataatcgtttgtaccctaactggcgctattctcggtgatattcagactggcttaattaccggtggtctgacagagttggctttcgccggattaacccctgcaggtggtgttcagccgcccaacccgattatggcgggtctgatgaccaccgtcattgcatggtctacgggcgttgatgccaaaacagcaattggtcttggcctgccgtttagtttgttaatgcagtacgtcattctgttcttctattccgctttctcattatttatgaccaaagccgataaatgcgcgaaagaggcggatacggcagcgttttcccggcttaactggacaacgatgctcatcgtcgcttcagcgtatgcggtgattgctttcctctgtacttacctggcacagggggcgatgcaggcgctggtgaaagcgatgcccgcctggctgacccacggctttgaagtggctggcggtattctgcctgccgttggttttggcttgctgctgcgcgtaatgttcaaagcgcaatatatcccttacctgatcgccggtttcctgtttgtttgctacatccaggtcagcaacctgttgccggttgccgtactgggcgcaggctttgcggtgtatgagtttttcaatgcgaaatcccggcagcaagcgcaaccgcagcccgttgccagtaaaaatgaagaagaggactacagcaatgggatctgaaatcagtaaaaaagatatcacccgtctgggctttcgttcgtcgctgctgcaagcgagctttaactacgaaaggatgcaggcgggcggttttacctgggcgatgttgccgatcctgaaaaagatttataaggacgacaaaccgggcttaagcgcggcgatgaaagataacctcgaatttattaatacccacccgaatctggtcggattcctgatggggttattaatttcgatggaagaaaaaggagaaaaccgcgacaccattaaaggcctcaaagtggcactgtttggcccaatcgccgggattggcgatgcgattttctggtttactttgttgccgattatggcgggaatttgctcatcatttgccagccagggaaacctgctggggccgattctatttttcgccgtttacctgcttatctttttcctgcgcgtcggctggacccacgtcggttattcagtcggcgtgaaggcgatcgataaagtgcgagagaactcgcagatgattgcccgttcggcaaccatcctcgggatcacggtaatcggcgggctgatcgcttcgtatgtgcatattaacgtggtgacatcgtttgccatcgacaatacccacagcgttgcgctgcagcaggatttcttcgataaagtcttcccgaacattttaccgatggcctacaccctgctgatgtattacttcctgcgggtgaaaaaagcgcatccggtgctgttaatcggcgtgacttttgtgctctctattgtttgttccgcattcggcattttgtaaatggaacgaggcactgcgtctggtggtgcctctttacttaaggaatttcatcctgtgcaaacccttcagcaagttgaaaactatacggcgttaagtgaacgtgccagcgaatatttattggccgtgatccgtagcaaaccgaatgccgtgatttgcctggcgaccggagccacgccattactgacgtatcattatctggtagaaaaaatccaccagcagcaggttgatgtcagccagctcaccttcgtgaagctcgacgaatgggtggatctgccattaacgatgccaggcacctgcgaaactttcctgcaacagcatatcgtgcagccgctggggctacgtgaagaccagctcatcagctttcgctccgaagagataaatgagacagagtgcgaacgggtaacgaacctgattgcgcgcaaaggcggtctggatttatgcgttctcggattggggaaaaacggtcatcttgggctgaacgaaccgggagaaagcctgcaaccggcctgccatatcagtcaacttgatgccagaacacagcaacatgagatgttaaaaaccgcgggtcgccccgtgactcgtgggatcaccttaggcctgaaggatattctcaatgcccgcgaagttttgttactggtgactggcgaaggaaagcaggatgcgacagatcgttttctcacggctaaagtctctaccgctatcccggcttcatttttatggctgcacagtaactttatttgtttaattaacacctaaccagatgaaaaatttgctcaaaatgtttaaattaacttatgtaacagtcacgcattatattaaataacatttgactgggttgaacataacgccgatagcaaaaggagttatgttcaacaatttaattttagatatacatataacttgttctattaataaatcacctcgtattctgactcgccccctggcgcagcaaagtcaggcatttatactcttttgaatacatagaaaattgatatcaatataatgaaaatatcaaatatttgcatataaatataatcttaaagttcagtctatttaatgttcaatgaaatatttctgcctgtataatctttaaagatgttgaacatatattcacattaaatatgattatgtacttgttacaaggataaggttatatatgaataaagttacaaaaacagctattgcgggcttacttgcgcttttcgcaggtaatgccgctgcaaccgatggtgaaatagtttttgatggcgagattttaaaatccgcttgtgaaatcaatgactctgataagaaaattgaagttgctcttggtcactataatgccgaacagtttcgtaatattggcgagcgtagcccaaaaattccattcactattcctttagttaactgcccaatgactgggtgggagcacgataacggcaacgttgaagcgtctttccgtctatggctggaaacgcgagataatggcaccgtccctaacttccctaatctggcaaaagtaggctcttttgctggcatagcggcaacaggtgtgggtatccgtattgacgatgcggaaagcggaaacattatgccactgaatgctatgggcaatgataacacggtttatcagatcccggcggaatccaatggtattgtcaatgttgacctcatcgcttactacgtatcaaccgtagttccatcagaaatcaccccaggggaagcagacgctatcgttaacgtaacgctggattaccgttaatacgttagggcgttatctgacctgtcagataacgcccttttccttcctctttctcgttgtatcaggttgaaaaataactatgtcaaaacgaacattcgcggtgatattaaccttgttgtgtagcttctgtattggccaggcgcttgcaggaggaatcgttttacagcgaacgcgagtgatctatgatgccagccgcaaagaggctgcgttacctgtcgcaaacaaaggcgcagaaacgccttatttactgcaatcatgggtagataatatagatggtaaaagccgtgccccatttattataaccccaccgctatttcgtcttgaggctggcgatgactcatcactgcgaattattaaaacagctgataacctgcctgaaaataaagagtcgctgttctacattaatgttcgtgccattccagcaaagaaaaaatcagatgatgttaatgctaacgagttgacgctggtatttaaaacacggatcaaaatgttttatcgccccgcacacctgaagggacgggtaaacgatgcgtggaaatcactggaatttaaacgtagtgaccattcactcaatatatataacccaactgaatattacgtcgtatttgccggactggcagtcgataaaaccgatctcacaagcaaaattgaatatatcgcgcccggagaacataaacagttaccacttcctgcatctggcggaaagaacgtgaaatgggctgcgatcaatgattatggcggcagttccgggacagaaactcgtccactgcaataaaaaatataaaaacacaggtcatcagggaatgccacaacgacaccaccagggacataaacgcacaccgaaacagttggcgctcatcatcaaacgttgtttgccgatggtgctcactggcagcggcatgctttgcactaccgctaacgccgaagagtattatttcgaccccattatgctggaaaccacaaaaagtggtatgcaaacaaccgatctgtcgcgtttttcaaaaaaatatgcacaactaccaggaacttatcaggttgatatctggctgaataaaaagaaggtttcacagaaaaaaattacatttaccgccaatgcagagcaacttctgcagccacagtttacggtagaacaactacgtgagctgggtattaaggtggatgaaatcccggcgctggctgaaaaagatgacgatagcgtgatcaactcgcttgaacaaatcattcccggtacagctgctgaatttgatttcaatcatcagcaacttaatttgagcattccccaaattgcactgtaccgtgatgcaagaggttacgtctccccttctcgttgggacgatggtataccaacgctgtttaccaactactcgtttacaggttctgataaccgttaccgccagggcaatcgtagccaacgacagtacctgaatatgcaaaatggtgctaattttggcccctggcgattacgcaactattccacatggacacgcaacgatcagacatcaagctggaataccatcagtagttatttacaacgtgatatcaaggcgttgaagtctcagttgcttctgggagaaagcgccaccagcggcagtattttttccagctacacctttactggcgtgcaactcgcttccgacgataatatgttgccaaacagccagcgcggatttgccccaacggtacgcggtatcgcaaacagtagtgcaatcgtgactatcaggcaaaatggttatgtgatctatcaaagcaacgtgtcagcgggtgcctttgaaattaacgatctctacccctcttccaacagcggcgatttagaagtcacgattgaagaaagtgacggtacacaacgtcgctttatccagccttattcttcattacccatgatgcagcgacctgggcatctaaagtatagcgcgaccgctggacgctatcgcgctgatgcaaacagtgatagcaaggaacccgaatttgctgaagccacggcaatatatggtttgaataatacttttacgctgtatggcggcctgctcggttctgaagattattatgcgctggggatcggtatcggcggcacacttggcgcactgggcgcgttgtcgatggatatcaacagagctgacacccaattcgataaccagcactcttttcatggctatcaatggcgtacgcagtacatcaaagatatcccggaaaccaacaccaatatcgctgtcagctactatcgctataccaacgatggctattttagttttaatgaagccaatacccgcaattgggactataacagtcgccaaaaaagtgaaattcaattcaacatcagccagacaatatttgatggggtaagtctgtatgcctccggttcgcagcaagactattggggcaataacgataaaaacaggaatatctctgttggggtttccggccagcaatggggagttggttacagcctgaattatcaatacagccgctacactgatcaaaataatgaccgcgcactctctttgaatctcagtattccgttagaacgctggttaccgcgtagccgggtttcctatcagatgaccagccagaaagatcgcccaacccaacatgaaatgcgtcttgatggctcactgctggatgatggtcgcctgagctatagcctggaacaaagtctggatgacgataacaaccataacagtagcctgaacgccagttaccgttcaccttatggcaccttcagtgccggatacagctacggtaatgacagcagccaatacaattacggcgttaccggcggcgtggttatccatcctcatggcgtgacgctctcgcaatatctgggcaacgcttttgcgcttatcgatgctaacggagcatctggcgtgaggatacaaaactatccggggattgctaccgatccttttggctatgcagtggttccttatctcacaacttatcaggaaaaccgtctctcggtagatactacgcagctgcccgataacgtcgatcttgaacaaacaacacagtttgtggtgcccaacagaggtgcaatggtagcggcgcgtttcaacgccaatatcggttatcgcgtacttgttacagtcagcgatcgcaacggtaaaccgttgccctttggcgctcttgccagcaacgatgatacggggcaacaaagtatcgtcgatgagggcggcatactatatctctctgggatatcgagtaaatcacaaagctggactgtacgctggggaaatcaggcagatcaacaatgtcagtttgctttcagtacaccggattcagaacctacaacctctgtattacaaggcacagcgcagtgccattaaggataaaaaaatgaaaagagcgcctcttataacaggtcttttgttgatatccacatcctgcgcttatgcctcctcaggagggtgtggagccgacagcactagcggtgcgacaaattacagcagtgtggttgatgatgttacggtgaaccagacagataacgtgacaggacgggagtttacctctgcaacgctaagtagcactaactggcaatacgcctgttcctgctctgcgggtaaggcagttaaacttgtctatatggtcagccccgtacttaccaccactggacatcagacaggatattacaaactcaatgacagcctggatattaaaaccacattacaggcaaacgacattccaggactcacaaccgaccaggttgtctctgttaacacccgattcacacagataaaaaacaacacggtatattctgctgcaacccaaacgggtgtttgccagggtgatacgtctcgttatggacccgttaatattggtgcgaacaccacctttaccctgtatgtcaccaagccatttctcggctcgatgaccattccgaaaacggatattgccgtcattaaaggcgcgtgggtcgatggaatgggaagcccgtctacaggtgacttccatgatttagtcaagttatcgattcagggaaatctcaccgccccacagtcgtgcaaaattaatcagggcgatgttattaaggttaattttggattcatcaatggtcagaagtttaccacccgcaatgccatgccagacggttttactccagtagactttgatatcacttatgactgtggtgatacttcaaagattaaaaactcgttgcaaatgcgcatcgacggtacaactggggtagtagaccagtacaacctggtcgccaggcgaagaagttcagacaatgtgcccgatgtcggtattcgtattgaaaatctcggcggcggagttgcaaatattccttttcagaacggtatccttcccgttgatccttccgggcatggcaccgtcaatatgcgcgcctggccagttaatctggtcggtggtgagctggaaacaggaaaatttcagggcacagccaccattaccgtcatcgtgcggtaaaagaagacgttgcgttttgattaacgcaacgcttcggcactgttacccctgctgctccagcgcatacttatacagcgcatttttcttcacgccgtgaatttctgcggccagcgccgccgcttttttcagcggcagttctgcctgtagcagcgccagcgtgcgcagggcatcggcgggtaagtcttcttcctgtgctttatgaccttcgacaatcagcaccatttcgcctttgcgacggttttcatcttcctttacccacgccagcagctcgccaacgggcgcgccgtgaatggtttcccaggttttggtcagctcacgcgccagaaccacgtagcgggattcgcctaataccgcaacgatatcttccaggctatctaacagacggtgggtagattcataaaaaatcagcgtgcgcggctccgcttcaatggcttttagcgcatcacggcggccttttgatttggcaggtaaaaagccttcgtaacagaaacggtcagagggtaaacccgctgcgcttaacgcagtgatagcagcacacggcccgggtagcggcaccacgcggatccccgcttcacggcaggtacgcaccagatggtagccaggatcgttaattagcggcgttccggcatcggaaaccagcgcaatgttttgcccctcttgcagcttcgccagcagcgtttcagctttttgttgttcgttatggtcgtgcagcgcaaacaaccgggcattaatcccaaaatgttgcagcaataaaccggtgtgacgagtatcctcggcggcaatcagatcaacggcctgtaatacctctaacgcacgctgggtgatatccgccagattgccgattggcgtcggtacaatgtaaagctggccctgagaattatccgccgattggtgttgtttcattgtgtcgtccgtattgccgatttaatattgagcattgcgtaaaaaaaatatcactggatacattatggtaccctcaacattttctcgtttgaaagccgcgcgttgtctgcctgttgttctggcagccctgattttcgccggttgtggcacccatactcccgatcagtccactgcttatatgcagggcacggcgcaggctgattctgccttttatcttcagcagatgcagcaaagctctgatgataccaggatcaactggcaattactcgccattcgtgcactggtgaaagaaggtaaaaccgggcaggcggttgagttgtttaaccaactaccgcaagaactgaacgatgctcagcgtcgcgagaaaacactgctggcggtagagattaaactggcgcagaaagattttgctggcgcgcaaaacttgctggcgaaaatcacacctgccgatttagaacaaaaccagcaagcgcgttactggcaggcaaaaatcgatgccagccaggggcgtccttccattgatttactgcgcgcgttaattgctcaggaaccgctgcttggcgcgaaagaaaaacagcagaatattgatgccacctggcaggcgctctcctccatgactcaggaacaggcgaatacgctggtgatcaacgccgacgaaaatattctgcaaggctggctggatctgcagcgcgtctggtttgataaccgtaacgatcccgacatgatgaaagccgggatcgccgactggcagaaacgttatccgaacaatccgggcgcgaaaatgctgccaacgcagttggttaacgtaaaagcgtttaaaccagcctcgaccaacaaaatcgccctgctgttgccactgaatggccaggcagcggtatttggtcgcactattcagcaaggctttgaagcggcgaaaaatatcggcactcagccagtggcagctcaggtagctgccgcacctgccgcagacgtagctgaacaacctcagccgcaaaccgtggatggcgttgccagcccggcacaagcctcggttagcgatctgaccggtgaacagcctgcagcccagccggtgcctgtaagcgccccggcgacaagcaccgcagcggtaagcgcacccgcaaatccatccgcagagctgaaaatctacgatacctcatcacaaccacttagccagatcttaagccaggttcagcaggatggcgcgagtattgtggtcggtccgttgctgaaaaataacgttgaagagttgctgaagagcaacactccgctgaacgtactggcactgaaccagccggagaatatcgaaaatcgcgtcaatatttgttacttcgcgctttcaccggaagacgaagcgcgcgatgcagcgcgtcatattcgtgaccagggtaaacaagcgccgctggtgctgatcccacgcagttcattgggcgatcgcgtagccaatgcgtttgcgcaagagtggcagaaactgggcggcggcaccgttctgcaacaaaaatttggttccaccagcgaattacgcgcgggtgttaacggcggttctggtattgctttaacgggtagcccgattactctcagagcgacaaccgactccggcatgacgaccaacaatccaacgctgcaaaccacgccaaccgatgaccagttcaccaataatggcggtcgtgtcgatgcggtgtacattgtggcaacgccgggtgaaatcgcttttatcaaaccgatgatcgccatgcgtaacggtagccagagcggtgcaacgctgtacgccagctcccgcagtgcgcaagggaccgctggcccggatttccgactggagatggaaggcttgcagtacagcgaaatcccgatgctggcaggcggtaatctaccgttaatgcagcaggcactcagcgcggtgaataacgattattcactggctcgcatgtatgcgatgggcgtcgatgcctggtcgctggcaaatcatttctcacaaatgcgccaggttcagggttttgaaatcaacggtaataccggaagcctgacggctaacccggattgcgtgattaacaggaacttatcatggctacagtaccaacaaggtcaggtagtccccgtcagttaaccaccaaacagaccggcgatgcgtgggaagcacaagcgcgtcgctggctggaaggcaaaggactgcggtttatcgccgctaacgtgaacgagcgtggcggcgagatcgatctgataatgcgtgaaggccggaccaccatttttgtcgaggtacgctatcgccgctctgcgctttatggcggcgcggcagccagtgtgacccgcagcaaacaacacaaattattacagactgcccgcttgtggctcgcgcgtcataatgggagttttgatactgtggattgccggttcgatgtggtagccttcaccgggaatgaggttgagtggattaaggatgcctttaatgaccactcataattaaggtttaaggattagcgtgcaagaaagaattaaagcttgcttcactgaaagcattcaaactcaaattgcggcggcagaggcgcttccggatgccatctcccgtgcagccatgacgctggttcagtctctgctcaatggcaacaaaatcctctgttgtggtaatggaacttccgctgccaatgcacagcattttgctgccagcatgatcaaccgtttcgaaacggagcggcccagcttacctgccattgcactaaatactgataatgttgtcttaacggcgattgccaacgatcgcttacatgatgaagtgtatgcaaaacaggtgcgggcgctgggtcatgcgggagatgtattgttagccatttccacccgtggcaacagccgcgatattgttaaagcagttgaagccgccgttacgcgtgatatgaccattgtggcattgaccggctatgacggcggcgaacttgcaggtttgttagggccacaggatgtggagatccgcattccttcgcatcgtagtgctcgcattcaggaaatgcatatgctgacggtaaattgcctgtgcgatctgatcgataacacgcttttccctcaccaggatgattaaggagaatacatgaaggcattatcgccaatcgcagtccttatttccgcgctgctgttgcaaggttgtgttgccgctgccgtagtgggtaccgctgctgtgggtaccaaagccgcaactgacccacgcagtgtcggcacccaggtggacgatggtaccctggaagtgcgcgtgaacagcgcattgtcgaaagacgaacagattaagaaagaagcgcgcattaatgtaacggcctatcagggcaaagtgctgctggttgggcagtcaccaaatgctgaactttcggctcgcgccaaacagattgctatgggcgtagacggtgccaacgaagtgtataacgagattcgtcagggccagccgattggtctgggcgaagcatctaacgatacgtggatcaccaccaaagtgcgttcgcagctcttaaccagcgacctggtgaaatcgtccaacgtgaaagtgaccaccgaaaacggtgaagtgttcctgatggggctggtgactgaacgtgaagcgaaagcggcggcagatattgccagccgggtgagcggcgtgaagcgggtaactacggcgtttacgtttattaaatagcagccccttgtaatgcctgatgcgacgcttgccgcgtcttatcaggcctacaacgatacaaaccgtaggtcagataaggcgtttacgccgcatccgacatgttttccctcaaatcagaacaacagcgccagcccgccgacaatcacaccagacactgccaccatcgcccctgtcagccataaggctttcgccgggaacgctttgcgcagcataatcagtgacggcaaactcactgccgggagcgtcatcaacaatgccagcgccggagcggttcccatacctgccagcatcatcgtttgtacaatcggaatttctgctgccgtgggaatgacaaacaagcatcctgctaccgccatcgccaccacccacatcaggctgttatcgacagcaccatcggcatgggggaataaccagacgcgagcggcacccaacaccagtactgcaaggatgtaaaccgggatcgtactccagaaaagcgtccatagcgccctgccccagcggctaaaaaacccgccctgtgcttccggtatgtcaatttcgaccggtgcctgcgtttgcggtgtttcacgcacccatttttgcaccagcgtcgcaatcagcaacaccatcaccagcccggccaccagacgaatcgccgcaaaaccccagccgaggacaaagcccataaacaccagcgtcgccgggtttaacaccggattgcccatccagaatgccagcgcaccgcccatcgacacctgttggcgacgcattcccgccgcgaccggagccgcacagcaggtacacatcatgcccggcaacgaaaacagcgttcccagcagcgtgccgcgaaagcgcgattgcccaagcgtacgcaacaaccagtcacgcgggatcagcacctgaatcaacgaaccgaggatcacccccagcaccgccgctttccataccgcgaggaaatagatcatcgcgtaatccaacgccgcctgccatgggttagcatccgcctgcgcaaggatagatttaccgatactgtgggtttcggcagcagtaaacgctttgccgtagtaaggttcccatttcacataccagagaccggcaatgacaacgagaaagaaaagcgcgggtttccaccactgaatgggcgttgccgcctgagatgaagactgaccagtcatagcattccccaggaataagttatgataattgagcgcgtgaatattacgctcactatcaattcttgggaataattattcagctcttttgcgtaattctgaagagcttaaaatcgtcacgccttcatgctcaggccgcatcgactctgccagcatgacccgcgccacgtctctcgcatcaatggatttccagttacctggtaacaaacggaacagcggcgcaaaaagcgtttcgttcatccgctgtttgctacgatcgcccagtaacatcgacgggcgagcaatggtcaatttcggccagttctgggcgattaatgcttcttccatctcccctttgacgcggttatagaaaaacggcgagtgggcattggcacccatcgcactgactaccaacatatgctgcgcgcccagtcgccgcccggttaatgcggtatccactaccagcgtgtaatcggcatgaataaacgcctctttgctccccgcttctcgccgcgtggtgccgagacaacaaaacacaatgtcgatgggatcggtgacctgcgccaacgcgtcactcagttgcggatcatggggattaaacaccccgggcatatcgcccaacggacgtcgcgtcggcgcagcaatggcgttaactttcggttcgttaatcaacatccgcagcaggtgaccgcccaccagccccgttgcgcctgtaatcagtacctgactcatcttcgctcctttacagaattgtctgccttgcgctccacggctcatgcaccaggcttaatagaccatgaggtaattatccccgattgtgggaaattcgcctcatccaatgcaacaacgcggaggaagcatgagtaagaaaattgccgttttaatcactgatgaatttgaggattcagaatttacttcacccgcagacgagttccgtaaagccggacacgaagtgattaccattgaaaaacaagcgggtaaaacggtgaaaggcaaaaaaggagaagccagcgtgaccatcgataaatccatcgatgaagtgacgcctgcggagtttgatgccctgctgctaccgggcggccattcaccggattatctgcgtggggacaaccgttttgtcacctttacccgtgattttgtgaatagtggcaaaccggtgtttgccatctgtcacggcccgcagttgctgatcagcgccgatgtgattcgggggcgcaaactgaccgcagttaaaccgatcattattgatgttaaaaatgcgggcgcggaattttacgatcaggaagtcgtggttgataaagatcagctggttaccagccggacaccggacgatctgccagcgtttaaccgcgaggcgttacgcctgctcggtgcctgagtcgcgtagccaaatcatttttttaccaaagcccagcgtgttgtcggtgaatttgatttcatcgagccggatttcccacaccggggccgacagcattctggcaaccggaaagcgacgattgtacgccttgcgcgcgaggtcgctttcctcaccttccagcctgcggatctcacctttaaactgcacaccgcgaattaacgctaccgttttcggctgaccgtttaccgttccggcaaccgcagcctgcggcccactcatctgcgcgtggcgcgttttttcttccgtcaaaatgtagaaggcgactttctgcgcatcaaaaagataaaaggcattagcgcaccagagttccccttcctgctgcacacaccaagtgacaacatgttgttttgccagccaacggctgatggcgatgagtgtttccattgctgttctcttttatactgtgggcctgaccttaacatgcgacgcagacgatgacaccctggtttctttacttgatccgtaccgccgacaataagctttataccgggatcaccacggatgtcgaacgccgctatcagcagcaccaaagcggcaaaggggcgaaagcactgcgcgggaaaggagaactaacgctggtgttttccgcgccagtgggcgatcgttcgctggcgttacgggcggaatatcgcgttaagcaactgaccaaacggcaaaaagagcgtctggtagcggaaggcgcagggtttgcagagctgttaagcagtctgcaaaccccggagattaaaagcgattgaaatgctcgtgatactcaaccaggccggtaacgccattcagcgcgtcatccgctaaacgatgtacctggaaggcgctttcagtgcccggccagcggcaacgcagatcgtgatgcgccgccagttcaaagccgaaacgactgtacagcgccggatcgcccagcgtcaccactgcggcatagccgaactcattaagcgaatcgagtccttcatagaccagttggcgtgccagcccctgtccacggtatttttcatcaaccgccaacggtgccatgccgacccattgcaggtcttcgccctgcacatcaaccggactaaatgccacatagccaatgacctgaccttcgtcatctgtcgccaccagccccagcgtcagaaagccatcttcacgcagatcgtgaaccagcttcgcttccgcatcactttcgaatgagcgacgcagcagggcatcaatacccggcgcatcaatgggaatttctactcgaattagcatggttcacctaccgatgtctgtttggtttcaggcgcggttttcattcccgcctcaacaaaatccgccagttgcagcagcatcatgcgtaaggctttcggcatttgctccagttcaatggcgtccatcaggtttttcacatacagccccagctccgtatcgccttcaatcaccagccgacgctggaagaagagcgtatccggatcttgtttacgcgccgcaatcatcagcagatcgctggcgtcggcactaaaactcacatcagcttgcgcgttctggctaacgaccagtttgccattcaccaccgaggtaaaccattgcaggtcaatatcacgcacatgaatacttaaccagcggccttcaagaaactccagctcgccatcatccagcgcctggcggaattgccagcttaagacctgctcaagaacctggcgttttagcgcaaatggcgtcagttttaccggtacactcaacagagatggccccaaatgcacaatacgggaacgcagtttatccaacacgagttttactccctgtttcaacaatcatcctattttgccatatcagaaaaataacatagcggtataaatcaacaattccatatgaaattgctgctaccaccaatacaactttaactgccttaaatcaaaaattgtcgcagcaaggttaactaaaatcccagttcgttaacatttttgcgttttgatagcgcaaccttcaggaaaaattatggagctgctctgccctgccggaaatctcccggcgcttaaggcggccatcgaaaacggcgcagatgctgtttatatcgggctaaaagatgataccaatgcccgtcacttcgccggccttaactttaccgagaaaaaattgcaggaagcggtgagttttgtccatcaacatcgccgcaaacttcacatcgcgattaacacttttgcgcatccggacggttacgcccgttggcagcgcgccgtggatatggcggcgcagctgggtgccgacgcgctgatcctcgccgacctcgccatgctggagtacgccgccgagcgttatccgcatattgagcgccacgtatcggtgcaggcttcggcgaccaatgaagaggcgattaacttttatcatcgccattttgacgttgctcgcgtggtgctgccgcgcgtgttgtcgattcatcaggtgaaacaactggcacgggtcacacctgtaccactggaagtctttgctttcggcagcctgtgcattatgtcggaaggtcgttgctatctgtcgtcgtatctgacgggtgagtcgcccaacaccataggcgcgtgttctccggcccgtttcgtgcgctggcaacaaacgccgcaggggctggaatcccgcctgaacgaagtgctgatcgaccgttatcaggacggcgaaaacgcaggttatccgacgctatgtaaagggcgttatctggtggacggcgagcgctatcacgcgctggaagaaccaaccagtctcaataccctggaactgctgccggagttaatggcggcgaatattgcttcggtgaaaattgaaggccgccagcgtagcccggcgtatgtcagccaggtggcgaaagtctggcgtcaggctatcgaccgttgtaaggccgatccgcaaaactttgtaccgcaaagcgcgtggatggagacgctcgggtcgatgtccgaaggcacgcaaaccactcttggcgcatatcaccgtaaatggcagtgagaaaagcaatgaaatattccttagggccagtgctgtggtactggccaaaagagacgctggaagaattttatcagcaggccgccaccagcagcgccgacgtgatttatcttggtgaagcggtatgcagcaagcgtcgggcaaccaaagttggcgactggctggagatggcaaaatcgctcgccgggagtggtaagcagattgtgctctccacgctggcgctggtgcaggcatcatctgaactgggcgaactgaaacgctatgttgagaacggtgagtttctgattgaagccagcgatctcggcgtggtgaatatgtgcgctgaacgcaaactgccgttcgtcgccgggcacgcgctgaactgctacaacgcggtgacactgaaaatattgctcaaacagggcatgatgcgctggtgtatgccagtggagctttcccgcgactggctggtgaatctgcttaatcagtgcgatgagctgggcattcgtaaccagtttgaagtggaagtcctgagctacggtcatctgccgctggcctactccgcccgctgctttaccgcgcgttcggaagaccgcccgaaagatgagtgtgaaacctgctgcattaagtatccgaacgggcgcaacgtgctgtcgcaggaaaaccaacaagtgtttgtactcaatggcattcagaccatgagcggctacgtttacaacctcggtaacgagctggcatccatgcagggcctggttgatgtggtccgcctgtcaccgcagggtactgacactttcgcgatgctcgacgccttccgcgctaatgaaaatggcgctgcaccactgccgttgacggcgaacagcgactgtaacggctactggcggcggctggcaggactggagctgcaagcctaagtaaatagctcactttgttaacaactttaactactctttaatgcagtattaaagattaatcggtaacaaagtgagctgttatgactgataaaaccattgcgttttcgctactcgatctggcccccattcccgaaggttcttcagcgcgagaagcattctcccactctctcgatctcgcccgtctggctgaaaagcgcggctatcatcgctactggctggcagaacaccacaatatgactggcattgccagtgctgccacgtcggtattgatcggctatctggcggcgaataccaccacgctgcatctggggtctggcggcgtgatgttgcctaaccactcaccgttggtcattgcagaacagttcggcacgcttaatacactctatccggggcgaatcgatttggggctgggtcgtgctccgggtagtgaccaacggacaatgatggcgctacgtcgtcatatgagcggcgatattgataatttcccccgcgatgtggcggagctggtggactggtttgacgcccgcgatcccaatccgcatgtgcgcccggtaccaggctatggcgagaaaatccccgtgtggttgttaggctccagcctttacagcgcgcaactggcggcgcagcttggtctgccgtttgcgtttgcctcacacttcgcgccggatatgctgttccaggcgctgcatctttatcgcagcaacttcaaaccgtcagcacggctggaaaaaccatacgcgatggtgtgcatcaatattatcgccgccgacagcaaccgcgacgctgaatttctgtttacctcaatgcagcaagcctttgtgaagctgcgccgtggcgaaaccgggcaactgccgccgccgattcaaaatatggatcagttctggtcaccgtctgagcagtatggcgtgcagcaggcgctgagtatgtcgttggtaggtgataaagcgaaagtgcgtcatggcttgcagtcgatcctgcgcgaaaccgacgccgatgagattatggtcaacgggcagattttcgaccaccaggcgcggctgcattcgtttgagctggcgatggatgttaaggaagagttgttgggatagtgtgtcttaacgcgggaagccttatccgagctggcaacgctgtcctacatagacctgataagcgaagcgcatcaggcattgtgtaggcagcagaaatgtcggataaggcaccgctgattactgatacaccggcagtaaattaaagctcgataaaatatgcaccagtgcgttgccgacgccaaacaccagaatcagcgcaatcatcggcttgccaccccagacgcggaatttcgggctgccaaagcgtttacgcgatgcacgggctaacagcgccggaacaattgccgcccagatggtagccgctaaaccagcataaccaatggcgtacaggaatccgttcgggaacaacagcccccccacaactggcggggcaaaggtcagcaatgccgttttcaagcggcccacagccgagtcgtcgaaaccaaacagatctgccagatagtcaaacaaacccagcgttacgccgaggaacgaactcgctaccgcaaagtttgagaacacgaccagcagcagatccagactacggctgttcagtacgccgcttaacgcctgtaccagcacatcaatattaccgcccttctctgcaataccgataaactccggacgcgggatgttacccatcgtcgccagcaaccagatggtatacagcgccagcgccatcagcgtaccgtacaccagacatttcacgatggttttcggatctttgccgtaatacttcatcaggcttggcacgttaccgtgataaccaaacgatgccagacagaacggcagggtcatcaacagatacggtgcataagacgcattgctttcggcgacgttgaacaatgtcgcaggctgcacatgccccagcaggctaccaaaggtgaggaagaaggtaatgactttcgcccccagcacaatcgctgtcatgcgactgacggctttagtgctcaaccacaccacaaacgctaccagcaatgcaaaaccaaaacccgccgcccgtgccgggacgtttagtgacatctctgcgaaggtgtgatgcagaatcgaaccactggcagaaatataggcataggtcaggatatagagcacaaaggcaatggaaatgccgttgaccacgttccagcctttgcccagcaaatctttggtgatggtgtcaaaactcgaaccgattctgtaattcaggttagcttccagaatcatcaagccggaatgcagcatacagaaccaggtaaagatcagcgccgccattgaccagaaaaaccacgccccggacatgaccactggcagagaaaacatccctgcgccaataatggtgccgccgataatcaccacgccgccaagcagcgacggtgacgtttgggtggtggttagtgttgccatgagggcttctctccagtgaaaaatagtgcgactgcgttgttatgcattgcactgtaccagtacacgagtacaaaagacagaaaaaaagccccgatggtaaaaatcggggctgtatatattattttacagattgtgttcgctgttcagcgatgattacgcatcaccaccgaaacgacgacgaccggtagaatcatcacgacgcggagcgcggccttcacgacgttcgccgctaaaacgacgaccatcaccacggccaccttcacggcgttcaccgctgaagttacgaccgccttcacgacgttcgccaccgaaaccacgaccaccgccacgacgctcaccgccagtatgcggctgtgcatcgcccagtaactgcatgttcatcggcttgttgagaatgcgagtgcgcgtaaagtgttgcagcacttcacccggcatacctttcggcagttcgatggtggagtgagaagcaaacagcttgatgttaccaatgtaacggctgctgatgtcgccttcgttagcaatcgcaccaacgatatgacgaacttcaacaccatcatcgcggcccacttcaatgcggtacagctgcatatcgccaacatcacgacgttcacgacgcggacgatcttcacggtcaccacgcgggccacggtcgttacgatcgcgcggaccacggtcatcacggtcacggaattcacgtttcggacgcatcggcgcatctggcggtacgatcagagtacgttcaccctgtgccattttcagcagtgccgcagccagagtttcgagatccagctcttcaccttcagcagtcggctgaattttgctcagcagtgcgcggtattgatccagatcgctgctttccagctgctgctgtactttagcggcgaatttttccagacggcgtttgcctagcagttctgcgttcggcagttctacttccggaatagtcagcttcatagtacgttcaatgttgcgcagcagacgacgctcgcggttctcaacgaacagcagcgcgcggccagcacgacccgcacgaccggtacgaccgatacggtgaacgtaagactcagaatccatcgggatatcgtagttaactaccaggctgatacgctcaacgtccaggccacgggctgcaacgtcggtcgcaatcaggatgtccagacgaccatctttcaggcgttccagtgtctgttcacgcagcgcctggttcatgtcaccgttcagcgcggcgctgttgtagccgttacgctcaagagcttcagccacttccagagtcgcgtttttggtacgaacgaagataatcgccgcatcaaaatcttccgcttccaggaaacgtaccagtgcttcgtttttgcgcataccccagacagtccagtagctctggctgatgtcaggacgggtagtcacgctggactgaatgcgcacttcctgcggctctttcataaagcggcgggtaatgcgacgaatcgcttccggcatggttgcagagaacagagcggtctgatgaccttccgggatctgcgccataatggtttcaacgtcttcgatgaagcccatgcgcagcatttcgtcagcttcatccagaaccagaccgctcagtttagagaggtccagagtgccacgtttcaggtggtccagcagacggcccggagtaccgacaacgatctgcggcccctgacgcagggcgcgtaattgcacgtcataacgctggccgccgtacagagcaaccacatttacgccgcgcatgtgtttagagaaatccgtcattgcttcagcaacctgtaccgccagttcgcgggtcggtgccagcaccagaatctgtggtgctttcagctcaggatcaagattctgcaacagaggtaaagagaatgctgcagtttttccgctccccgtctgggccatacccagaacgtcgcggccattcagcagatgtggaatacactctgcctgaattggagatggtttttcgtaacccagatcgttaagggcttcaaggataggagccttcaggcccagatctgcaaaagtggtttcgaattcagccatgtagtacgtgtgcctcaaaattaatggcggccagtctacataactcatcatgaaattgatcagcaattttcattgaaaagtgtgaaccggctcaaagtaggtgtattaacgaacaacaacgccctcacccgttaaggtgatggcaatcaaaaaagattacgggctgatgtgtacgtcagctattgctggtccgattctgccaggtcatcttggtcctggcccaggagcgataattccaacaatgcgtatcggtgctcaacaaagttatgaacgttgttggcaaccgccagtttgaacagtgccgtggcgctgtccaaatcccccagacttaggtagtacttacctaaatagaagttggtttcactgagatgctcagcgagcgaggtgttatccgttgcgtccgccttgagcctttccattaacgtttgttcgctaatgttgcccaggtagaactcgacaatgttccatccccactgttccttatccgatttttcgaagtgctgtttcaacacttctttagcctgcttctcatcgagcttctgctcggcgagataaagccacagactacggaaaggatcattgggatcgtcttgataaaacgccagcagatcatcttgcgctaacttgtcacgaccgccgtaatataatgcgatcccgcgattcaagtgcgcgtagttgtaagttggatcaagctcaagtacagaatcaaacgcttcataggcagcatcaaaattgcctgcctgcgttaaatatatgcctaagtaattgaatacttcaggcatatccggtcggattgccagcgcttgcgaaaaatcgttacgcgctaatgccctcagaccgagactatcatacaacactccgcgctcatataaaagctgtgcgcgttcgtcatcggttaaagcccgactggcaaggatttgttccatacgtgccagaatcacttcctgctgtaaagtcggttgcaatggtaccgcgaggacttcacttttacgccaggaagtattactgcatcctgcaagcgtaagtgctgtcgcaacgaaacaccagcgcaaaaaaggcttcatttcccactcccgaagaccacggttgaatgaacgtcctgttcccggttgctaacaaggcgtcctgcccggttaaaagccccccgccgcagcggagggcaaatggcaaccttactcgccctgttcagcagccggagcttccggtgctgcagcaggttgagactgctcagtcgcttctttaatgctcagacggatacggccctggcgatcaacttccagaactttcaccggtacttcctgacccatctgcaggtaatcggtcactttctcaacgcgtttgtcagcgatttgagagatgtggaccagaccttctttaccgccgccgatggcaacaaatgcgccaaagtcaacgatacgggtcactttaccagtgtagacgcggcccacttcgatttctgcagtgatctcttcgatacgacgaatagcatgtttcgctttctcgccgtcggtcgctgcaatcttcacagtaccgtcatcttcgatttcgatggtggtgccagtttcttcggtcagagcacggattacagaaccgcctttaccgataacatctttgatcttgtccgggttgatcttgatggtatggatacgcggtgcgaactcagagatatcgccacgcggcgcgttgatcgcctgttccattacgcccaggatatgcagacgcgcacctttagcctggttcagcgcaacctgcatgatctctttggtgataccttcaattttgatatccatctgcagtgcagagataccgtcgcgggaacctgcaactttgaagtccatatcgcccaggtgatcttcgtcgcccaaaatgtcagacagtacaacgtagttgtcgccttctttcaccagacccattgcgatacccgcaacggcagctttgatcggcacacctgcgtccatcagcgccagagacgcgccgcacacggaagccatagaagaggaaccgttggattcagtgatttcagacacaacacgtacggtgtacgggaatttgtccatatccggcatgactgccagcacgccgcgcttcgccagacgaccgtgaccaatttcacgacgcttcggagaaccgaccatgccggtttcgcctacggagtacggagggaagttgtagtggaacaggaaggtatcggtacgttcgcccatcagttcatcaagaacctgcgcgtcacgagcagtacccagcgttgcggtaaccagcgcctgcgtttcaccacgggtgaacagcgcagaaccgtgagtacgcggcagcacgccagtacgcacatccagaccacggatcatatctttttcacgaccgtcgatacgcggttcgcctgccagtacgcggctacgaacaacgtttttctcgatcgcgtgcagaatttcacccagttcgttttcgtccagggtttcgtcttcagcaagcagcgtcgcgatggtttcagatttgatgacatcaacctgcgcataacgctcttgtttgtcggtgatgcggtaagcatcgctcaggcgagcttcagccagtgcagcaacgcgcgcgtttagcgcttcgtttaccggctccggctgccagtcccaacgcggtttaccggcttctttcaccagttcattgatgttctgaataacaacctgctgttgttcatgaccgaacactactgcgcccagcatctggtcttcgctcagcagttgagcttcagattcaaccatcagtacagcggcttcagtaccggcaacaaccagatccagtttgctctctttcagctcgtcctgagtcgggttcagtacgtactggtcattgatgtaacctacgcgggcagcaccaatcgggccattgaacggaataccagacagagacagcgctgcggaagcaccaatcatcgcgacgatatccgggttaacttgcgggttaacagaaaccacggtggcgataacctgaacttcgttgacgaagccttccgggaacagcgggcgaatcgggcggtcaatcagacgcgcgatcagggtttcgccttcgcttgggcggccttcacgacggaagaagctacccgggatacgaccagcagcgtaggtacgctcctgatagttaacggtcagtgggaagaagtcctgacctggtttggcttttttctggccaacaacggtaacgaataccgcggtgtcatccatgctaaccataacagcggcagtagcctgacgagccatcatgccggtttccagagtcacggtgtgttggccgtactggaatttacgaacgatcggattaagcaatgtaatatcctttctctttcttagacagtaccttacggcactggtgttaatacccgatcttctgcgcatcctcgcgactaatgacaaccctaacccagctctatgtgggtaaagcctctcattagccgcgcgaacctctgcaacggaagatcattcatagcaacaatacattagtttccagtgaattgctgccgtcagcttgaaaaaaggggccactcaggcccccttttctgaaactcgcaagaattagcgacgcagacccaggcgctcgatgagctgggtgtaacgtgctacgtctttacgtttcaggtagtcgagcagtttacgacgctgagaaaccatgcgcagcagaccacgacggctgtggtgatcttttttgtgctctgcaaagtggccctgcaggtggttgatctgtgcagtcagcagtgctacctgaacttcggtagaaccggtgtcgtttgcgtcacgaccaaactcagaaacgattttagctgttgcttcagtacttagagacattttaaaactccaaagtatatagaatgaaaggacgccgatctctaattcagcgatcccagtgtacgttacgcaaagtgttaaacaatttacgcgacgttaagcggcagtattctactcgtagcgacctgttatcgcaagacggttaacattacgccgggtattcaaccaccaggcgacgaggcgcaacgcggccttcatcgtcaatttcgcccataccgataaatttgccgttctcaccttccgtgacgcgaaccagtccttccagtggcgcaccagatgtacgaaccgggttaccatttttgaagtaaacagaagacgttaacggaagattcaccaccggatagtccgaagctggactgtccattggcatcagtaatggatcaagtaactccgcggctggaatatcctgctgttcagcttgctcaacaagttcacgcaggtgctccagggtcaccatccgttcaaccggatatttacttaccgccagacggcgcaggtaaataacatgcgcgccacagccgagtttttcacccaggtcatcaatgatggtgcggatataagtgccttttgagcagtgaatttccagctccagctcattgccttcatggcgaataaacagcaattcataaacggtaatcggacgcgcttcacgcggaacttcaatgccctgacgcgcatattcgtacagttttttgccctgatatttcagtgctgaatacatcgaagggatctgttcgatatcgccacggaaagtatccagtgccgctgccagctgctctgcgctaaaggttaccggacgttcttcaacgatctgtccgtcggcatcagaagtatcggtacgctgtccaagacgcgcaatgacccgatagcgtttgtcggagtccagcagatactgggaaaacttcgtcgcttccccgaggcaaatcggcaacatgccggtcgccagcgggtccagcgcaccggtatgcccggcacggttggcgttatatatacgtttcactttttgcagcgcatcgttgctggacataccctgaggtttatccagcaacaaaacgccgttaatgtcgcgaccgcgacgacgaggacgactcattagtcctccttgctgtcgtccgggttaacacgacgttcttcgtcatgtttgaccacgctggtcaccaggtttgacatgcgcatcccttcaaccagagagttgtcgtagaagaaggtcagttccggcacgatacgcaggcgcatcgctttccccagcaggctgcggatgaaaccagaagcttcttgcaacgctttgatgcccgctttaaccgcgtcttcatctttgtcgttgaggaacgtcacatatactttggcatacgccaggtcgcgagacatttcgacaccggaaacggtggtcatcatgcccaggcgaggatctttaatttcacgctgcaggatgagagcgatctctttttgcatttcctgcgctacgcgctgcgggcgaccaaattctttcgccataataaattctcctgacaaaaaaggggctgttagcccctttttaaaattaatttcaggtggaagggctgttcacgttgacctgataagacgcgccagcgtcacatcaggcaatccatgccggatgcagcgtaaacgccttatcccgcatggaaccctaaaaaccttaagcaatggtacgttggatctcgatgatttcgaatacttcgatcacatcgccagtgcggacgtcgttgtagttcttaacgccgataccacattccataccgttacggacttcgttaacgtcatctttgaagcggcgcagggactccagctcgccttcgtagataaccacgttgtcacgcagaacgcggatcgggttgtgacgtttaaccacaccttcggtaaccatacagcctgcgatggcaccaaatttcggcgatttgaacacgtcacgaacttccgccagaccgataatctgctgtttcagttccggagacagcataccgctcatcgccgctttcacttcgtcaatcaggttatagatgacggagtagtaacgcagatccaggctttccgcttcaatcactttacgtgcagaggcatcagcacgtacgttaaagccaaccaggatggcgttggacgccgcagccagggtggcgtcggtttcggtgataccacctacgccagaaccgatgatcttcactttaacttcgtcagtagacagtttcagcaaggagtcggagatcgcttcgacagaaccctgtacgtctgccttcaggacgatattcacttcgtgaacttcgccttcggtcatgttggcgaacatgttctcgagtttagatttctgctgacgcgccagtttaacttcgcggaatttaccctgacgatagagtgcaacttcacgcgctttcttctcgtcacgtacaacggtaacttcatcacccgcagccggtacgccggacaggccgaggatttccaccggaatggacggacccgcttccagcacttcctgacccagttcgttacgcatcgcacgaacacgaccgtattcgaagccacacagaacgatatcgcccttgtgcagagtaccttcacgtaccagaacggtagcaaccggaccacgacctttatcgaggaaggattcgataaccgcaccgctcgccatacctttacgtaccgctttcagctccagaacttccgcctgcagcaggatagcgtccagcagttcatcgataccggtacccgctttcgcagatacgtgtacgaactggctttcaccgccccactcttccggcaggatgccgtactgggagagttcgttcttaacgcgatccggatcagcttctggtttatcgatcttgttcactgcaaccaccaccggtacctgcgccgctttcgcgtgctggattgcttcgatggtctgcggcatcacaccgtcgtcggcagcaacaaccaggactacgatgtccgttgcctgcgcaccacgagcacgcattgaagtaaacgcggcgtgccccggggtgtccaggaaggtgatcatgccgttttcagtttcaacgtggtatgcaccaatgtgctgggtaatgccgcccgcttcgccagaggccactttcgttgaacgaatgtagtccagcagagaggttttaccgtggtcaacgtgacccatgatggtcacaaccggcgcgcgcggttcagccgcagcacccgtgtcacggtcgctcattaccgcctcttccagctcgttttcacgacgcaggataactttatggcccatctcttcagcaaccagctgtgcggtttcctgatcgataacctggttgatggttgccattgcgcccagtttcatcatcgctttgatgacctgagagcctttaaccgccatcttgttcgccagttcgccaacggtgatagtttcgccgatcacaacgtcacggttaacggcctgagcaggcttctggaagccttgctgcagcgaagaacctttacgttttccgcctttaccgccacgtactgctgcgcgtgcttcttcacgatcagcttttgattcagcgtgtttgttgcctttcttcggacgcgctgctttcgcgttacgaccacggccacggccgccttcgacttcacgatcgctttcgtcttctgcctggcgagcatgttgagaagtagtgacgtgataatcgctggaatcttcagtcggttccgcgttatcagtccatttgttttcttccgccatacgacgtgcttcttcagcaacgcgacgtgcttcttcttcgagtttacgacgcgcttcttcttcagctttacgcttgagctctgcagcttcctgctcacggcgggctttttcagcctgggcgtttttagtcatatcgtcttgttgattgctcactttgtctttttccgcagcttcacgtttcgcttgttcagcagcttcacgcttagcttgttctgcggcctcacgttcagctttttgttgcgcctcgcgtttagccgattcttctgcctcacgacgggcttgctcttccgcttcacgctgcgcttgctcttccgctgcaaggcgttcagcctcttgcggatcgcgtttcacaaaggtgcgtttcttgcggacttcgatttgtaccgatttgctttttccaccggtaccaggaatgttaagggtgctgcgtgttttacgttgcagcgtcaatttgtccgggcctgaatttttctgattcaggtggtcaatcaaagtctgtttctcttgtgcagacacagagtcgtcagcagacttccggatacctgcatcagcaaattgctgtaccaggcgttccacggaggtctgtcgctctgcggccagcgttttaatcgttacatctgtcatgctgttccttcctgctacagtttattacgcttcgtcaccgaaccagcaaatattacgggcagccataatcagtgctccggctttttcgtcggtcaacccttcgatatcagccagatcatcaatgccctgttcggcgagatcttccagcgtacaaacgccacgggcggccagtttgaatgccaaatcacgatctaccccttcaaggttcagcagatcgtcagccggtttgttatcaccgaggctttcttcctgggcctgtgcaatggtggccagtgcatttttagcacgctcgcgcagtgcttcaacggtcggctcatcaaggccttcgatttccaacagctctttcatcggcacataggccaattcttccagcgtcgagaagccttcttctaccagaacagtcgcgaagtcttcgtcgatgtcgagatatttggtgaaggtgtcgatcgctgcgtgcgcttccgcctgatgcttagcctgcaggtcgtcaacggtcatcacgttgagttcccaaccgctcagctgcgaagccagacgcacgttctgaccgttacggccaatcgcctgcgccaggttaccggcttcaacggcgatatccatggtgtgtttatcttcatccaccacgatagaagcaacgtctgccggtgccattgcgttaatcacgaactgcgccgggttatcatcccacaggacgatatcgatacgctcgccacccagttcagtagacaccgcctgaacacgcgcgccacgcatacctacgcaagcacctaccggatcgatacgtttatcgttggttttcaccgcgattttcgcacgagaacccggatcgcgagccgctgctttaatttcaatcacttcttcgccgatttctggcacttcaatacggaacagttcgatcagcatttccggcttggaacgagtgacgaacagttgcgcgccacgcgcttccgggcgaacggaatagagcacgccacgaacgcggtcgccagggcggaagttttcacgcggcagcatatcttcgcgcaggatcacggcttcagcgttgttgcccagatccagagagatgttgtcgcggtttacttttttcaccacgccggtgatgatttcaccttcgtgttcacggaactgatcaaccaccatcgcacgttcggcttcacgcactttctgcacgataacctgttttgccgtctgggtagtgatacggtcaaaggtaacagactcaatctgatcttcaacgtaatcgcccaggttcaggctttcatcttcataacgtgcggcttcaagggtgatttccttggtcggctgggtgacttcatcaacaactaaccagcgacggaaagtgtcaaaatcaccgcttttgcgatcgatctgtacgcggacgtcgatctcttgttcatattttttctttgttgctgtcgccagcgcgctttccaatgcttcgaaaatcttctcgcgaggtagcgccttttcattggatacggcttcaactacagccaaaatttctttgttcatcgcgggcttttcacctcatccagactattaaaagtggggaaccaggttcgccttctggatattactcagcgcgaacacttcatctttaccttcgacggtaactgtgatcatttcaccgtctaccgctttgataacgccctgccatttacgacggttttgtaccgccatacggagaaccagagtcacctcttctccgacaaaacgggcgtagtgttcagccgtgaacagtgggcgatcgagacccggtgaggagacttccaggttataagcaacggtgatgggatcttcaacatccagcacagcacttacctggtggctcacatcagcacaatcatcaacattgatgccatcttcactatcaatatagatgcgcagtgtggatgtgcgaccgcgaataaattcgatgccaaccagttcaaaacccagggcctcaactggcgcagtaatcatctctgttaatttttgctctaatgtggacaagcccacccccaagacataaaaaaagggcctaaagcccagttattctgtagtcagataacaaaaaaccccgataaatcggggctttatataactgaaccctataaccgcaactgcggtctggagcactttccagaaggattttttcaaatcccactacgaaggccgaagtcttcacagtatatttgaaaaaggactctaagggaaagtggttgcgggggccggatttgaaccgacgatcttcgggttatgagcccgacgagctaccaggctgctccaccccgcgcctgaaacgtggcaaattctactcgttttgggtaaaaaatgcaaatactgctgggatttggtgtaccgagacgggacgtaaaatctgcaggcattatagtgatccacgccacattttgtcaacgtttattgctaatcatgtgaatgaatatccagttcactttcatttgttgaatacttttgccttctcctgctctcccttaagcgcattattttacaaaaaacacactaaactcttcctgtctccgataaaagatgattaaatgaaaactcatttattttgcataaaaattcagtgagagcggaaatccaggctcatcatcagttaattaagcagggtgttattttatgacgacgattctcaagcatctcccggtaggtcaacgtattggtatcgctttttctggcggtctggacaccagtgccgcactgctgtggatgcgacaaaagggagcggttccttatgcatatactgcaaacctgggccagccagacgaagaggattatgatgcgatccctcgtcgtgccatggaatacggcgcggagaacgcacgtctgatcgactgccgcaaacaactggtggccgaaggtattgccgctattcagtgtggcgcatttcataacaccaccggcggcctgacctatttcaacacgacgccgctgggccgcgccgtgactggtaccatgctggttgctgcgatgaaagaagatggcgtgaatatctggggtgacggtagcacctacaaaggaaacgatatcgaacgtttctatcgttatggtctgctgaccaatgctgaactgcagatttacaaaccgtggcttgatactgactttattgatgaactgggcggccgtcatgagatgtctgaatttatgattgcctgcggtttcgactacaaaatgtctgtcgaaaaagcctactccacagactccaacatgcttggtgcaacgcatgaagcgaaggatctggaatacctcaactccagcgtcaaaatcgtcaacccgattatgggcgtgaaattctgggatgagagcgtgaagatcccggcagaagaagtcacagtacgctttgaacaaggtcatccggtggcgctgaacggtaaaacctttagcgacgacgtagaaatgatgctggaagctaaccgcatcggcggtcgtcacggcctgggcatgagcgaccagattgaaaaccgtatcatcgaagcgaaaagccgtggtatttacgaagctccggggatggcactgctgcacattgcgtatgaacgcctgttgaccggtattcacaacgaagacaccattgagcagtatcacgcgcatggtcgtcagttgggccgtctgctgtaccaggggcgttggtttgactcccaggcgctgatgctgcgtgactctctgcaacgctgggttgccagccagatcactggtgaagttaccctggagctgcgccgtgggaacgattattcaatcctgaataccgtctcagagaacctgacctacaagccagagcgtctgacgatggaaaaaggcgactcggtgttctcgccagatgatcgtattggtcaattgaccatgcgtaacctggatatcactgatacccgcgagaaacttttcggttatgccaaaactggcctgctttcctcctctgccgcttcaggcgtgccgcaggtggagaatctggaaaacaaaggccagtaattcgacatcaaccctgcccttcaggggtggggttaccttgcttatcctctgtaaactcctttctgagcatcacataatcgaaaacatcatggtttgcatccacaacccgtgagtctcctttatagtgtgcaatcacttcctcaagcgtttgcggctgttccggctttgttacccccatccacgcattaataaggtaattattgtaagctgtcgaaaagatgttgttttccgttgtgcgatccacgccatccccaagaacggggctataccagataaacatcgggacatgatatgcctgctggctagcctccctgcctccatgaaaatagacgttcttcttcgtagggtcacgttccaggccgtggtcggcaaaatacatgaccgaggcgcggcgatcttttaataattcaaaaacctgacctagcaaactatctgtgtaatgaatggagttgtcatagcaggcatcctgatcgtcctgcggttgaaacacggcgctggattgcggataggcgctacaagccggttcatggcttccatttaaatgaagaacaatcagtttcttttgctgcgtattttgctgtaatgcttgcgataaatgcggcaacaacaattcatcaaatcctctgacataaactgtttccatggcgcgcatggcgatactggtaactgctgtaccattctgccgaaaagcggattgcgagcttagccagaaagtctgaaatcctgcttgattagccatattaataatgttgtcggggtaattatgaatgtcatgactcaaaacagaatcagcagttaaagaaaggggaaccgacagcgcagtgtaaggtgcgccgcttattgcttgattaaacagtttgatctgttttctttgtgcttcaacttgcggtgtcgtagagcgtgtatatccatacaaagacatattgtcgacacgtacagactcccccacaatcaacacgtaggtatcaatacctgtatccctgactgataattgaaaatacggcaccgtgtttgcaattgagagtaatctttgatgctctttcgctgctaaagcaaaatagttgagattgaaaaacggcgtataggtagcaaatcgcgacgctagtatatatggactgaacgcttttttattttttgcatctttataagcaaattgacaagcggaaaataaactgcccgaaatgacaatcagcaataatattcctgtcactttttttgtcggcaaggaaacatcatattttattattactgccaaaaaaagaagggataaaaaagcaaaggcacatagataagggatatacatccccagcattttgacaacttcatccggatcactctggagcacactaatcgcaaatccatcattgaaagttgtaccaaaggtacaccatgaatagaggctaatactcatgtctgccgcagtcagtaacacaaatggtgcggcaacaagcaggcgaagcggaagggatgatatacgttttacaaccaggatggtcagaacgaagaacagcaagcgctgaaccatatgcgctccggaagaagcgactaagttcgtaataccaaaaacaataacacaaagatacaacaaccaatgagatttaaaagttctagcaaatttgttgaatactgtcatccagaaatccaagttcacaaccaatataaacaattatcaacaatgtttaattttatatcagacatgtttttcaactctgatccatatcagaacgaaacactgttagttttttctttttaaatgatgcggccattgcgttctcagtaattaaataacattatcaatgcgtctctaaacattacgcagaacgtagccatcagtcgttatactgacaggagcaggatggtttatcgagaagtaaacatatccgtattcgtaccggaactggagttgacacaataaagtgccaattatgtcagtagaagggaaaaatttataactaaggcgtaccggcaccatcgtttcaaggtaccagctacgagtaaagcaactggacgagatacagatacctgacaaccattcctcagaccaggaccaaaacgaaaaaagacgcttttcagcgtctcttttctggaatttggtaccgaggacgggacttgaacccgtaagccctattgggcactaccacctcaaggtagcgtgtctaccaattccaccacctcggcacggatactactttttagttcgggatatcgctggtcggcttagccggagcagctggctgagtttgttcggttttcgccggtgcactcagattttcccattcgctacctttattggttttgttgctattgatgttacccagcaccagactgatgatgaagaataacgttgccagcagcgccgtcatgcgggtcatgaagttaccagaaccacttgaaccaaacagcgtagcggaagcgcctgctccgaaggaggctcccatatcagcgcctttaccttgctgcagcatgatcagaccaacaaggccaattgccacaataaggaaaactactaaaagagcttcatacataatcaacctgttccttgcggagttgccgcgtaccaatgcttcaaccaataaagcgggagtttttaatctttcccactgaagcgggtgtgaatactaaccaaagcgaatgaccttcgcaagggcaattttatcgcattgtatcaactgcggaaaaaaacagcaaaaccgatgtgttcgctgagaaaaaaggcgacaatcgccgcctttttagccagttatctaacgctttaaacggcttttactgcatcggcgatgcggtgtgcaaattcagtcacctgcgcttcgtcttcgccttccaccatcacgcgaattaacggttcggtgccggatttacgcagcaacacgcgtccacggttgcccagcgcagcttcaacctctgcggtcacggctttaactgactcatgctcaagtggatcgccgctacctgcggtgtaacgtacgttaaccagaatctgcgggaacattttcatgccgctgcaaaggtcgtgcaggctcatatggttacgtgccatcgccgccagcacctgcaagccagcaacgatgccgtcaccggtagtagttttatccagcaggatcacatgaccggaattctctgcaccgatacgccagcctttctcctgcattttttccagtacgtagcggtcacccactttcgcgcgcgcaaatggaattcctaactgtttcagcgccagttcaagccccatgttgctcatcaatgtacccacagcgccaccacgcagctggccctgacgaagaccttcacgcgcgatgatatacatgatctgatcgccatcgactttattgccttcatggtcaaccataatcacgcgatcgccatcgccgtcgaaggcaataccgagatccgctttttcagccagcacacgagcctggagcgcgcgaacgtcggtagcccccacttcggcattgatgtttacaccgtttggctcacaaccgatagcgataacgttcgcccccagttcgcgcagcacgttcggcgcgatgtgataagtcgcaccgtttgcacaatccaccacaatcttcagttcactgaggctaagttcgttcgggaacgtggctttgcaaaactcgatatagcgacccgcggcatcaacgatacggctggctttacccagttctgccgaatcaacgcagctgatctccttttccatttccgcttcgatggcctcttctaccgcatccggcagtttggtgccgtcgatagagaagaatttaatgccattatcgtagaacgggttatgcgatgcagatatcacaattccggcctctgcgcggaaggtacgcgtcagataagccacggccggtgttggcatcgggccagtgaagagtgcggaaaggcccgctgccgccagacccgcttccagtgctgactccagcatatagccagaaatacgcgtgtctttaccaataataatcttacgggagccgtggcgcgccagcactttacccgcggcccaacccagcttaagcacaaaatcaggtgtgatcggcgcatcccctacacgaccacgaatcccatcggtaccgaaatatttacgattactcatagcgtttgttttcctttgcagacagagtggcttccaccacccgcatcgcttctacggtttctttgacgtcatgaacacgaatgatgtgcgcgccttgcattgcggcaatgaccgcacaggccagactaccgctcaggcgctcggacggccccacgttcagcagctgcccaatcatcgattttcgtgacatacccaccaacagcggcaggttgaaatggtgaaattcagccaggcgcgccagtaatgaatagttatgggagagatttttaccgaaaccgaatccggggtcgagcaacaatttctcttttgcgatacccgcctgctcgcaacgtgctatttgctcaataaagtagcgattcacttctgcaaagacatcgtcatacttcggagcttcctgcatggtttttggatttccctgcatatgcatcagacaaaccggtaaaccggtttctgcagccgcctccagagcgccaggttcggaaagggagcggatatcattaataatgtgagcgccaactttcgctgactcacggatgacttctggtttggatgtatcgactgagatccagacttcgaagcgttgagcaattgcctcaaccacaggaataacacgttgcaactcttcttcaacgctaacttccgccgcccctgggcgcgtggactcgccaccaacgtcaatgatcgtcgcgccagcgttgatcatcagattcgcatgtttcaccgcatctatcagcgagttatgcgtgccaccatccgaaaaggaatcaggcgtgacgttgaggatccccattacgtgaggatggctaaggtccagtgaagtaccctgggcaaagagtttcatgatgttatccctggtatgaattgataagaaaaaaccccggagcacgccccggggttttcggtacaaatacagtcatctgatgcgggaacttacttgtcgcctaactgctctgacatggtgttacccgggttcggcgtacgcggttcatcaaccggacgaggagcctttggactaccattgtcgccagaattgttagaagcgcctggttcttcccagcccgctggcggacgtacatcgcgacgtgccatcaggtcatcaatctgcggtgcgtcgatagtctcatatttcatgagagcatctttcatcgcatgcagaatatccatattgtcggtcagaagctgacgcgcacgattatagttacgctcaatcagtgctttcacttcctggtcgatgatacgtgcagtttcatcggacatatgtttcgctttcgctacgctacggccgaggaacacttcaccttcttcttccgcgtacagcagtggacccaatttctcagagaagccccactgagtcaccatgttacgtgccaggttggtcgcaactttaatatcgttggacgcaccggtagatacatgttccggcccgtagatgatctcttctgccagacgaccaccgtacagcgtagaaatctggctttccagtttctgacggctggcgctgattgcgtcgccctcaggcaagaagaaagtcacacccagcgcacgaccgcgtgggataatcgtcactttgtgcaccggatcgtgttccggcaccaggcgaccgataatcgcatgacccgcttcgtggtaagccgtcgattctttctgcgcttccgtcatcaccatggagcgacgttccgcacccatcatgattttgtctttcgctttctcgaactcaaccatcgacacaacgcgtttgttgccacgagcagcgaacagtgccgcttcgttcaccaggttcgccaggtcagcaccggagaaaccaggagtaccacgggcaatgattgccgcgtcgatatcgggtgccaatggtacgcgacgcatgtgaactttcaggatctgctcacgaccgcgaacatctggcaagccgaccacaacctgacggtcgaaacggccaggacgcagcagggccgggtcgagaacgtccggacggttagtcgcggcgataacgatgataccttcgttaccttcgaagccatccatctcaaccagcatctggttcagagtctgttcacgttcatcgtgaccaccgcccagaccagcgccacgctggcggcctacggcgtcgatttcatcgataaagatgatgcacggtgccgctttcttcgcctgttcgaacatgtcacgaacacgggatgcacccacaccgacgaacatttctacgaagtcagaaccggagatagtaaagaacggaactttcgcttcgcctgcaatcgctttcgccagcagcgttttaccggtacccggaggaccgaccatcaagacgcctttcgggatcttaccgccgagtttctggaagcggctcggctcgcgcagatactcaaccagttcagcaacttcttcttttgcttcgtcgcagcccgcaacgtcagcaaaggtcgttttgatctgatcttccgtcagcatgcgcgctttgctcttaccaaacgacatggcacctttgccaccgccgccctgcatttgacgcatgaagaagatccagacaccaatcagcaacagcatcgggaaccaggagatgaagatagaagccagcaggcttggttcttcaggcggttcaccgacaaccttgacgttcttggtcaacaggttatccagtaatttcggatcctgaaccggaatgtaagtggtataacggttactatctttcttggtaacgttgatttcacgtccgttgatacgcgcttcacgaacctggtcgttattgacctcttgtaggaaggtagagtaatccaccttacggccattagactcgctgggcccaaagctctggaatactgacatcagcacaacggcaatgaccagccagagtattaggtttttcgccatgtcactcaagggattaacctcttattacaactgtgttaaaaacagcgtcaggatactctatatccagcatctttcaaactttcgtctgaaatctcccggttagggtttacgcccggtcgctacaatatacacttcccgcgaacgtgcacgagaagagtccggcttacgaactttgaccttcgtaaacagggagcgaatttcccttagatactcatcgaaaccttcgccctggaacaccttcactacaaaactgccacctggcgctaatacatcacgacacatttctagcgccagttccaccagatacatggcacgggggatatccaccgccggtgttccgctcatgtttggtgccatatcggacatgacaacctggactttgctgtcgccaacgcgctccagcagtgctttcatcaccagttcatcacgaaaatcgccctgaagaaagtccacaccaacgataggatccataggtaaaagatcgcaagcgatgatgcggcctttgccgccaatttgggtgaccacatattgtgaccaaccacccggagcagcaccaaggtcgacaaccgtcattcccggtttaaagagtttgtcactttgctgtatttcatcaagtttaaaccaggcacgggaacgtaacccctttttctgtgcctgttgaacatatttatcgctaaagtgttcctgaagccagcggctggagctggcagaacgcttcttacctgtcatttaactttcccatggggataactcatcgtaaccaattgcgtaaatttttacgcgcctatttggtgatatatgggagatggcggtagaatgacccgttttcaatcccaacgtaagcaaaaaatacgatgaatctgagtactaaacaaaaacagcacctgaaaggtctggcacatccgctcaagccagttgttctgcttggcagtaatggtttgaccgaaggggtgctggccgagattgaacaagcgttagagcaccatgaactcatcaaggtgaaaatcgccaccgaagatcgcgaaactaaaaccttgatcgtggaagctatcgtgcgcgaaaccggcgcctgtaatgtacaggtcatcggtaaaacgctggtgctttatcgcccaactaaagaacgtaaaatctcgctgccacgctaagattatcctaaagttacacacatttgctgtgtaaaacgaggggttttccgcaggcaggagagcaaaatgccacgctctgttcgttgataaaaggccgcatagcggcctttttcctttctttacaatacatcaacatcttgagtattgggtaattcttacaggtattccaccttaattacttcaaattctacttcgccgcccggcgttttgatgaccacaacatcatcttcttctttgccgatcaggccacgagcaataggcgagtttacagaaatcaggttttgtttaaagtcagcttcgtcatcgccaacgatgcgataagtctgttcttcgtcagaatccagattcagcaccgttacggtagcaccaaaaataacgcgcccattgttgggcattttggtgacatcaatcacctgcgcgttcgacagcttggcttcgatgtctttaatacggccttcgcagaaaccctgctgttcacgagctgcgtggtattcggcgttttctttcaggtcgccatgctcacgcgcttccgcgatagcagcaatgatttcaggacggcgcacagatttcagaaaatccagctcttcgcgtaatttttcagcgccgcgtaaggtcatcggaatagcttgcatttgttatacctcttgaatattcctgatagggcaagtcttcacccaccccggctgttcggcctgcccggcataactccttaccgggaccagaagcaaaaaaataccgacccgggtacaagtcccaggtcagctacaattcacattttgatagtcattttaccctgaagttcccgaagggtcatcgtttactttatagggcgttgcgccgtagtatgacggctcgattccaggttgttagcgcgagattatgcgattttccagatttatcatcggattgaccagctgtatagcgttcagtgttcaggccgcaaatgttgatgagtacattactcaactccccgctggtgccaaccttgccctgatggtgcaaaaagtcggcgcgtcggcccccgctattgattaccacagtcagcagatggcgctgcctgccagtacccagaaagtgattactgcgctggcggcgttgattcaactcggccccgattttcgttttaccacgacgcttgaaaccaaaggcaatgtggaaaacggcgtacttaagggtgacttagtggcgcgatttggtgccgatccgacgttaaaacgtcaggatattcgcaatatggtcgcgactttgaaaaaatctggcgtcaaccaaatcgatggcaatgtgttgatagatacctccattttcgccagccacgataaagcccccggctggccatggaatgacatgacacaatgctttagcgctccgcctgccgccgccatagttgaccgcaactgtttctccgtctcgctctacagtgccccaaagcctggtgatatggcttttatacgcgtggcatcttattaccccgttacgatgttcagccaggtacgcaccctcccccgtggttctgccgaagcgcaatactgcgaactggatgtggtgccaggcgacctgaaccgctttacgctgacgggatgcctgccacaacgttctgagccgctcccgttggcttttgccgtgcaggatggagccagctatgccggtgcaattctgaaagatgagttaaaacaggcgggtatcacctggagcggaacactgctgcgccagactcaggttaacgaacctggaacggtagttgccagtaaacagtcggccccgctgcacgatctgcttaagattatgctgaaaaagtcggacaacatgatcgccgatacggttttccgcatgataggccatgcgcgcttcaatgtgcctggaacatggcgggccgggtcggacgccgtgcgtcagatcctgcgccagcaagccggtgtcgatattggaaacaccattattgccgatggttcagggctttcgcggcataacctgattgcccccgccaccatgatgcaggtgctgcaatacattgcccaacacgacaatgaacttaactttatctccatgctgccgctggcgggctatgacggctctttgcagtaccgtgcaggtctgcatcaggcgggcgtggatggaaaagtctcagcgaaaaccggttcgttgcagggggtatataacctggcgggattcattaccacagcgagcgggcaacgaatggcgtttgtgcaatatctttctggctatgcagtagaacctgcggatcagcgtaatcgccgtattccgttagtgcgttttgaaagccgtttgtataaagatatttatcagaacaattagtcaaaaagaaaccccggcacatggccggggcttcagattattgacaaagtgcgctttgtttatgccggatgcggcgtaaacgccttatccggcctacaaaatcgtgcaaattcaacatattgcaattctcttgtaggcctgataagcgtagcgcatcaggctgatttggcgtttatcatcagtgattaacgcttgtaaatgaactcaacgccttcttcgtcgtcttcgtcccagtcgtcatcccagtcttcatcatcctcttcagcaatctcttcaagctgctggcgatgataatcatcccacatgaattcgactttctctggctgtttcgcttcttcagcctgcacgaccgggttttcaatgataaaggtcatcacatcccagcagagatctttcacgcccagtccactcgccgcagagatcagataatatttatcttcccagcccagcgcctcagcgatcgctttcgctttctcttcggcttctaccttatccagcagatcgatcttgttgaacactaaccaacgcggtttcgtcgccagatcctggctgtatttttccagctcgctgataataatacgcgcgttttcaaccggatcggtgccgtcaatcggatcgatatcgatgaggtgcaacaggacgcggcaacgttccaggtgcttcaggaagcgaatgcccagacctgcgccttccgcagcgccttcaatcagtcctggaatatcggcaacaacgaagctcttttcgttgtccattcgtaccacacccagacttggcaccagagtggtaaacggataatccgccactttcggtttagccgccgataccgcacgaataaaggtcgatttacccgcgtttggcatccccaacataccgacgtcagccagcagcatcagctccagcagcagctcgcgcttatcgcccggcgtgccgttggttttctgccgcggtgtacggttaacggacgatttgaaacgggtattgcccagaccgtgccagccgcccttagcaaccagcagacgctgaccgtgtttggtcatatcgcccatggtttcaccagtaccctggtcgattacacgcgtacctaccggcactttaatcgtcacgtctttaccgcgcttaccggtacagtcgcggcttgcgccattctgaccgcgctctgcacggaaagatttttcaaaacgataatcgataagcgtgttcaggttctcgtcggcttccatccatacgtcaccaccatcaccgccgtcgccgccatccgggccgcctttcggaatatacttttcgcggcggaagctcacgcaaccattaccgccatcacctgcaacgaccagaatcgatgcttcatcaacaaacttcattttattctccgtaaatcattcgcctgcgcggggttgcgataccaccgttgtatgcttacgtaatccgccccaaatacgatgaccaatggcggaatacatcgcgcccgcaaccacgacaaacgcaccgagataacctaaaaggtttaacatcggtctggcgaagaaatcgggccaggccagtgataaaagatctgaaaaaaacagcgtaaacagtggggtgagcgtgatgatcgcgctcacctgcgctgcctgccagcgagccatcgcttccgccagggcgccatatcctaccaaggtattcagtccgcaaaaaattaaacatgcgagctgccagtggctaagctgcgctatcactccaggctttgccagagggaagagcgcaattgtacataaagtgtacagtaaaaacaggatctgcggtgaggccagccgacgcaataaaaccttttgcgccacgccataactcacccaaaccgtcgccgcaccgaccccaaagataactccccaggtgtaatcggtgagctttgtaaatatctcgaccagactggtgttaaaaaacatcaccaggccgctcaggagcatcaatgcccctacaacctgagtgctgcgcattttctctttgaggataaatacgctggcaaccatcatgccaactggcgagagttgcccaatcacctgcgaagcggtcggactcaggtattgcaaggatgagctgaacaggatgaagttcccaaacagcccggcggtcgccactgccaacaaaatcaaccagcgtggcttacgaaacacgcgtaatggcggcaacctcttcttcaccgcaagaatggcacccaggccaatactcgccatcaagaaacggtaaaacacgattgtcggaggttccatcacctccagcacctgcttcattgcgattggcaacgccccccagcaaattgctgtggtgagcgccaaaagaatgccaatgcctgcctgctgcttcataccgtattccctgcaaagcgcatttgcggattaacgtcgcaccatgcgcatttttaccggttatcgaatgtaaaaagccccgcaacgtgttgcggggctttcatccgttaccgggacgcgaaaaacttattcagcttcgatgctgataaatttacggtttttcgggcctttaacttcgaatttcactttaccgtctgctttagcaaacagagtgtggtcacgaccgcaacctacgttagcgccagcgtggaatttggtaccacgttgacgaacgatgatgctacccgccagaacggattcgccaccgaaacgcttaacgcccaggcgtttagcttctgaatcgcgaccgttacgtgtggagccgccagcctttttatgtgccatttgaaatctctcctcaggtcttaggcgctgatgccagtaattttcacatcagtgaaccactgacgatggccctgctgcttacgatagtgtttacgacgacgaaacttaacgattttaactttctcgccacgaccgtgagcaacaacttcagctttgattacgccgccatcaacgaaaggaacgccgattttgacttcttcaccgtttgcgatcatcagcacttcagcgaactcaacagtttcgccagttgcgatgtccagcttttccaggcgaacggtctgaccttcgcttactcggtgttgtttaccaccactttggaaaaccgcgtacatataaaactccgcttccgcgcacaccttttcaatgattcagagtgcgctataaatattcacaatagggcgcgaatattacgcaaaacgcacgcctttgacaagtgctacagtcaatacacgaagaaaaaaaacacaacttgtacggtaacgtttatctgtgccattttttcagtacaatcaccctatattcctaaccataaaccctaagttgcctttgttcacagtaaggtaatcggggcgaaaagcccggcttttgcgatgaatttagaaaaaatcaatgagttaaccgcgcaagatatggcgggtgttaatgcggcaatccttgagcagcttaattccgacgtccaactgatcaatcagttaggctattacatcgtcagcggcggcggtaaacgtattcgtccgatgattgctgtactggctgcacgagctgttggctatgagggaaatgcgcatgtcaccattgctgccctgatcgagtttatccacacggcgactctgctacacgacgacgttgtggatgaatcagatatgcgcaggggtaaagctaccgccaacgccgcatttggcaatgccgccagcgtgctggtaggcgattttatttatacccgcgctttccagatgatgaccagcctcggttcgctcaaagtgctggaagtcatgtcagaagccgtaaacgtcatcgcagaaggtgaagttctgcaactgatgaacgttaacgatccggacatcactgaagaaaactacatgcgcgttatctatagcaaaaccgcgcgtctgtttgaggctgccgcgcagtgttccgggattctggctggctgtacgccggaggaggagaaaggcctgcaggattatgggcgctatctcggcactgctttccagttgatcgacgatttactcgattacaatgccgatggcgaacagttaggtaaaaatgtcggcgacgatctgaacgaaggtaaaccgacgctgccgctgctgcatgcgatgcatcatggcacaccagaacaggcacagatgatccgtaccgccatcgaacagggtaacggtcgccatcttctggaaccggttctggaagcaatgaacgcttgtggatctcttgaatggacgcgtcagcgtgccgaggaagaagcagacaaagccatcgcagcgttacaggtgctcccggacaccccttggcgagaagcactcatcggcctcgcgcacatcgctgttcaacgcgatcgttaatcccctcccctcatcccgcgcagcgcgcgggatggttccagtaagttccataaaaacacttattcagctctataacacctgaaaaatagggatgtgcatctttatatattctgaatattcacactctttacaggaactttttagagcaataggccatcaggagtatagtgatgctcgacagaagaagtgttctgaatgaaagcgactaacttaaggagtgaggaaaaatggaaagtaatttcattgactggcatcccgctgacatcattgcgggtttgcgcaagaagggaacgtcaatggcggcggaatctcgcagaaatggtttgagttcctcaacgctggcgaatgcattatcgcgcccatggccgaaaggagagatgattattgcgaaagccctgggaactgacccctgggttatctggccatcacgctaccatgatccgcagacccatgagtttatcgacagaacgcagttgatgcgtagctacactaaaccgaaaaaatgagtggtctggcggtagccccgcgaacggggctgccagctctcagacgattattcgcctttcacacgctcaatatttgcacctaaagcgcgcagtttgtcttcaatgcgttcgtagccacgatcgatgtgataaatacgatcaaccaccgtcgtcccttccgcaatacagccagccagcaccaggcttgctgatgcacgcagatcggttgccataacctgtgcgccagaaagtttttcaacaccgtgacaaataacggtattgctttcgatttcggcgtgcgcgcccatacggctcagctctggcacatgcataaagcggttttcaaagaccgtttcggtgataaacccggtcccttctgccaccaggttcaacagcgtgaactgggcctgcatatcggtcgggaatgccggatgcggcgcggtacgtacgttaacagccttcggacgtttgccatgcatatccaggctaatccagtcttcgccgacttcgatgtccgctccagcgtcacgcagtttcgccagcacggcgtcgagagtatctggctgcgcgttacggcagataattttgccgcgagaaatcgccgccgccaccaggaaagtaccggtttcgatacgatccggcagaacgcgatagacaccgccgcctaaacgttccacaccttcgatgacgatacgatcggtgccctgaccgctaattttcgcacccagcgtaatcaggaagttcgcggtatcgacgatttccggttcacgcgctgcgttttcaataatcgtggtgccttccgccagggttgcagcacacatgatggtcaccgttgcgccaacgctgactttatccatcacgatatgtgcacctttcaaacgaccatcgacggaagctttaacgtaaccttcttccagtttgatggtcgcgcctaattgttcgaggccagaaatgtgtagatcaaccggacgcgcaccgatcgtacaaccgccaggtagtgaaacttgcccctgaccaaagcgcgctaccagcggccccagcgcccagatagaagcacgcatggttttaaccagatcgtaaggtgcgcagaatacattaacgtcgcgggcatcaatatgcacagaaccattacgttctactttcgcacccagctggcttagcagcttcattgatgtatcgacgtctttcagtttcgggacgttctggatctctaccggttcttccgccagtagtgcggcaaaaaggataggcagagcagcatttttagcgccggaaattgtgacttcgccctggagcttcgttggcccctgaacacgaaatttatccatttagtttgttctcagttaacaattcatatccgctaccggcgaatcgcccatagctcaaaagccgttcagtttgcgatcgcgcgcccactccgcaggggtatacgctttgatcgacacagcatgaatgcggttatccgcaatatattccatcagcggaccatagaccgtctgctgttttttaacccgactcatgccgtcaaacaactcacccacggcaataacctgaaagtggctgccatcgccggaaacgtggacttcctggagggagagagcgttcatcaacacgctctgaatttcattattttccatgggatcttcaatcatcagttaataaaccagcgaaacatcttagagcaaagttgcgctggcataaataagcaaaaagcctcgctgataaatcagacaaggctcgacttgcaggcaggtttgccggacaggcggttaacgccatatccggcctgaaaaaatttaacgaggcagaacatcagcaggcaaattatacaatttcgccagggtatacactttgtcgtttaccccctgaagcgtcacattgttgccctgctttttcgccagatcgataagatggagcagcagtgccagtccccccgtatccacgcgggagacacggctaagatcgatgcaggtaatccccttcaccgcttcctcacgcatttcccaaagcggtagcaaaacgtcctgatccagctctccggataacgccagcgtgtcacccgtctgcatccagctcagtgactcgctcattattttttctcttccagagtgattttctgttgagaaatcgatttcagttgcgcagtcaggccgtcgatacctttggtacgcagcagcgttccccactcgttttgtttggtggtgatcatactgacgccttcagcaatcatgtcgtaagcctgccaattgcccgtctgggagtttttacgccactggaagtccagacgcaccggcggacggccattcgggtcaataatggtaacgcgaataggcacaatggttttatcgcccagcggctgttctggcgcaatctgataggtttgaccgtgatacatcgccagcgcctgaccgtaagcctgcttcaggtactcacggaaagcggcaaagtaggcttcacgttgagcaggggtcgcactcttgtaatactggcccagcaccagcgcaccggcgtatttcacctgtacgtatggcagcagttcctgatcaacaatggtacgcagataatccgggttggcccgaatttgcggttgctcattcttcaggcgatcgaacgttttctgcgccgcctcgtccatcagcttatacggattggtctggtctgccgcggttgccgcactcagaggtgcaatcaccagcaaagcgaccatcattaaacgtttaaacatgcgtcggttctcctgaaattatttcgttgtacccacaggttcagtggtttcattattacctggcgcagcagctggcgcatcgccactattcttattgtcatcgcctttactaccgtaaaggaactgaccaatgagatcttccagcaccatcgcagacttagtgtcctgaattgtatcgccatccttcaggatagcagtccccagttccgggtcttcaaaaccgacgtttaatgccagatattgttcccccagcaggccggaagtacgaatgctcagcgaactggtatctggaatgtggttataacgttgttcaatttccagcgttacgcgcggcagataggttttcgggtccagcgtaatatccgccacccgacccacaacaacgccaccaatactgaccggagagcgcgctttcaggccgccaatgttatcgaacgtcgcataaagcgtgtaggtcggttcagtacgtatggacgtcacgttcgccgccttcaggcaaacaaacagcgccgccagcagtgctgctaataaaaagatacccacccaaatttcattttttttcgtttgcatgaactcaattcccaaacatcaatgcggtcagcacaaaatccagccccagaacagccagagacgagtggacaacggtgcgagtggttgcccggctaatcccggcagacgtcgggatggcgtcgtagccgttaaacaacgaaatccacgtcaccgtgatggcgaacaccacgctcttaatcagacagttgaccagatccatacgccagtcgacggcattttgcattgccgaccagaagaacccgctatcaatgcctttccaactgacgccgaccagagatccgccccagatccccacggcgacgaaaataaccgtcaacagtggtaatgaaataaccccagcccagaaacggggagaaataacccgacgcagcggatccaccgccatcatctccatactggagagttgctctgtagcgcgcatcaggccgatttctgcggttagcgccgaaccagcacgcccggcaaacaacaacgcggcaaccaccggccccagttcacgcagtagcgataacgccaccagcatacccagactggtttccgcactataagtggtcagaaccagataaccttgcagccccaacaccattccgatgaacacgccagaaaccacaataatcagcatcgacaggacgccgacattatagagctggcgcaccagcagcggcgcatgtttgcgaaattccggtttgccgaccagcgcattgaataacattaacccggcccgcccgaacgttctcagggttttaatccctttatgtccgagcgacgccagcgcatttaacagcatgagtggcttaactccctggtaaaagatcagcgtgataatcgccggcaggatagcggaacggaacaggcccgtcagctatcccgtccagaaactgacgtacgcgcggatcaggattcgcctgcaacgcctgggcactgccatgagcgacaatttttttgtccgccaggatccaggcgtgatccgcaatacttaacacttccggcacatcgtgagaaaccaccacacaagtcacgcccagcgcgctgttcagctcagaaatcagcttcaccagtacgcccatggtgatgggatcttgcccaacaaaaggttcatcaaacatgatgagatccggctccagcgcaatcgcacgcgccagcgctgcacgccgcgccatcccaccggaaagttcagaaggcattagtttagccgctccacgcagccccacggcctccagcttcatcatcaccgtactatgcaacaatggcgcgggaagttgggtatgttcgcgcagtggataggcgacgttgtcaaatacgttcatatcagtgaacaacgccccggactgaaataacatgctcatccgtttgcgcactgtatacaggcgcgaacgagacatcgccggaatattctcaccatcgaaaaggatctcaccatgatctggtgcgatttgcccgccaatcagacggagtagcgtcgttttaccgatgcccgatggccccatgatcgccgtgatcttccctcgcggcacggtcagggaaatattatcgaagatgcagcgattgccacgcgtaaaactgacatcgcgcatatcgactaaattcgccacagactgctccataattcacccttcgtcttgcgttgattttctaagcatggcgctcaatttaaccttgaacccaacatatttacagaatattacccgccgtggttagcgaaagctggcatttgttttactttttagccgcataaagtcaaaattaagcatccgttacggctttctgaaaatcttcagcggaccggcgagtatacctgaagaaaggacgttagatgcttttagctacggcactgttaattgttggtttacttttggtcgtttacagtgccgaccgcctggtttttgccgcgtctattctttgccgaacctttggcatcccgccgctgatcatcggcatgacggtggtcagtattggtacatcgttaccagaagtcatcgtctcgcttgccgcgtctctgcacgaacaacgcgatttagccgttggtacagccctcggctcaaacattatcaatatattgctgatcctcggtctggctgcgctggttcgtccttttaccgtccattctgatgttctacgccgtgaattacccttaatgttgttggtcagcgtggtggccggttccgtactctatgacggacaacttagtcgcagcgatggtatctttctcctctttctggctgtgctatggctgctgttcattgttaaacttgcacgtcaggctgaacgtcaggggactgacagcctgaccagagagcagcttgcagagctgccgcgtgacggcggattgcccgtcgcgtttttatggctcggcattgcgcttatcatcatgccagtggccacgcggatggtggttgataacgccacggtgctggcgaattactttgccatcagcgagttgacgatgggtctgacggcaattgctatcggaaccagcctgccggaactggcaaccgcaatagcgggggttcgcaaaggtgaaaacgacattgctgtcggaaatatcattggcgcaaacatttttaatattgtcatcgtgttgggtttacccgcgctgataacgccaggagagattgatccactggcgtacagtcgtgactacagcgtgatgttgctggtgagcattatttttgcgttgctgtgctggcggcgctccccgcaaccgggccgtggtgtaggggtattattaactggcggatttatcgtatggctggcgatgttgtactggttatcgccaatactcgttgaataactggaaacgcattatgtcgcacgtagagttacaaccgggttttgactttcagcaagcaggtaaagaagtcctggcgattgaacgtgaatgcctggcggagcttgatcaatacatcaatcagaatttcacgcttgcctgtgaaaagatgttctggtgtaaagggaaagttgtcgtcatggggatgggaaaatcggggcatattgggcgaaaaatggcggcaacgtttgccagcaccggtacaccttcatttttcgtccatcctggtgaagccgcgcatggtgatttaggcatggttaccccacaggatgtggtgattgctatctctaactctggtgaatccagcgaaatcacggccttaattccagtgcttaagcgtcttcacgtaccgttaatctgcatcaccggtcgcccggagagcagcatggcgcgcgccgcagatgtgcatctgtgtgttaaagtagcgaaagaagcctgtccgttagggctggcaccgaccagcagcaccaccgccacgctggttatgggcgatgccctcgctgtcgcgctgttaaaagcacgcggctttactgctgaagattttgcgctctcacacccaggcggcgcactgggtcgtaaacttctgctgcgcgtaaacgatattatgcatacgggcgatgagatcccgcatgttaagaaaacggccagtctgcgtgacgcgttgctggaagttacccgcaaaaatcttggtatgactgtcatttgcgatgacaatatgatgattgaaggcatctttaccgacggtgatttacgccgtgtcttcgatatgggcgtggatgttcgtcagttaagtattgccgatgtgatgacgccggggggaatacgtgtgcgccctggcattctggccgttgaggcactgaacttaatgcagtcccgccatatcacctccgtgatggttgccgatggcgaccatttactcggtgtgttacatatgcatgatttactgcgtgcaggcgtagtgtaaagattcaaggataaacaacaatgagcaaagcaggtgcgtcgcttgcgacctgttacggccctgtcagcgccgacgttatagcaaaagcagagaacattcgtctgctgatcctcgatgtcgatggcgtactgtcagatggcctgatttatatgggcaataatggcgaagagctgaaagcgttcaatgttcgtgacggttatggcattcgttgtgcgctcacctctgatattgaagtcgctatcattaccgggcgaaaggctaaactggtagaagatcgttgtgccacattggggatcactcacttgtatcaggggcagtcaaacaaactgatcgcctttagcgatctgctggaaaaactggcgattgccccggaaaatgtggcttatgtcggcgatgatctcatcgactggccggtaatggaaaaagtgggtttaagcgtcgccgtggccgatgcgcatccactgttgatcccgcgcgccgattacgtgacgcgcattgctggcggtcgtggcgcagtgcgcgaagtttgcgacttattactcctggcgcagggcaaactggatgaagccaaagggcaatcgatatgagtaaagccagacgttgggttatcattgtgctatcactggcggttctggtgatgatcggcattaatatggccgaaaaagacgataccgcccaggtggtcgtcaacaacaatgatcccacctataaaagcgagcatacggacacgctcgtctataacccagaaggggcactaagctatcgattgattgctcaacacgttgaatattattccgatcaggccgtttcgtggtttacgcagccggtacttaccacgtttgataaggataaaatcccgacatggtccgtaaaagcagataaagccaagctgaccaatgaccggatgctctatttatatggacacgttgaagtcaacgcacttgtgccagactctcaacttcgcagaatcacgacggataacgcgcagatcaatctggtgacgcaggatgttacctctgaagacctcgtcacgttatacggaacaacatttaactccagcggtctgaaaatgcgcggcaacttacgcagcaagaacgccgagctgattgaaaaggttagaacatcctatgaaattcaaaacaaacaaactcagccttaatcttgtgcttgccagctcacttctggccgccagcattccggcatttgccgtaaccggagacactgatcagccgatccacattgaatcggaccagcaatctcttgatatgcaaggcaacgtggttacctttaccggtaatgtcatcgtcacccagggcaccatcaaaattaatgccgacaaagtggtcgttacccgtccgggcggcgaacaaggtaaagaagtgattgacggctacggtaaaccggcaacgttctaccagatgcaggacaacggtaaacccgttgaaggtcacgcttcccagatgcactacgaactggcaaaagattttgtcgttctgacgggtaatgcttatctgcagcaggtcgatagcaacattaagggcgataagatcacttacctggtgaaagagcagaaaatgcaggctttcagcgacaaaggcaagcgcgtaacaaccgttctggtgccgtcgcagctgcaggacaaaaacaacaaaggccagaccccggcacagaagaagggtaattaattcgttatggcaacattaactgcaaagaaccttgcaaaagcctataaaggccgtcgcgtggtagaagacgtcagcctgaccgtcaactccggggaaattgtcggtctgctggggccaaacggtgccggtaagaccaccactttctacatggttgtaggcattgtgccgcgcgatgcgggcaacatcattattgatgatgacgatatcagtctgctgcctctgcatgcacgcgcgcgccgcggtatcggctatctgccacaggaagcctccattttccgtcgcctcagcgtttacgataacctgatggcggtactgcaaattcgtgacgacttgtctgctgaacaacgtgaagaccgcgcgaacgagctgatggaagagtttcacattgagcacctgcgtgacagcatggggcagtcactctccgggggtgaacgtcgccgtgtagaaattgcccgcgcactggctgcgaatccgaaatttattctgctcgacgaaccgtttgccggggttgacccgatctcggttatcgacattaaacgcatcattgagcacctgcgcgacagcggcctgggcgtgctgatcactgaccacaacgtgcgtgaaacactggcggtttgtgaacgcgcttatatcgtcagtcaggggcatttgatcgcccacggcacgcctacagaaatcttacaagacgaacacgttaagcgtgtataccttggggaagacttcagactctgatagggtagaagtttgcgacgttttagcaggagagtacgattctgaacatgaagcaaggtttgcaactcaggcttagccaacaactggcgatgacgccacagctccaacaggcaattcgtctgttgcagttgtcgacgctggaacttcagcaggagctacagcaggcgctggagagtaatccgctgcttgagcaaatcgacactcatgaagaaatcgacacccgcgaaacgcaagacagtgaaacgctggacaccgccgacgcgctcgaacaaaaagagatgccggaagagctgccgctcgatgccagttgggacaccatttacaccgctggtacaccatccggcaccagcggtgactacattgacgacgagctgccggtctaccagggcgaaacgacgcagaccttgcaggattacctgatgtggcaggttgagctgacaccgttttccgacactgaccgcgctattgctacctctatcgtcgatgccgttgatgaaaccggttatctgactgtcccgctggaagatattctcgaaagtataggcgatgaagagatcgacatcgacgaagttgaagccgtccttaagcggatccaacggtttgatccggtcggtgtggcggcaaaagatctgcgtgactgtctgctgatccaactctcccaattcgataagaccacgccgtggctggaagaggccagactgatcattagcgatcatctcgatctgttagccaatcacgacttccgcactttaatgcgcgtcacgcgtctgaaagaagatgtgctgaaagaagccgtcaatctgatccagtcgctcgatccgcgccccgggcagtcgatccagactggcgaacctgagtatgtcattccagatgtgctggtgcgtaagcataacggtcactggacggtagaactcaacagtgacagcattccgcgtctgcaaatcaaccagcactacgcctcgatgtgcaataacgcgcgcaacgatggtgacagccagtttatccgcagcaatctgcaggatgccaaatggttgatcaagagtctggaaagccgtaacgatacgctactgcgcgtgagtcgctgtatcgttgaacagcagcaagccttctttgagcaaggtgaagaatatatgaaaccgatggtactggccgatatcgcccaggctgtcgaaatgcatgaatcgacgatatctcgcgtgaccacgcaaaaatacctgcatagtccacgaggcatttttgaactgaagtatttcttttccagtcacgtcaataccgagggcggcggcgaagcttcctccacggcgattcgtgcgctggtgaagaaattaatcgcggcggaaaacccagcgaaaccgttgagcgacagcaagttaacctctttgctgtcggaacaaggtatcatggtggcacgccgcactgttgcgaagtaccgagagtctttatccattccgccgtcaaaccagcgtaaacaactcgtttgacccaaccgataaggaagacactatgcagctcaacattaccggaaataacgtcgagatcaccgaggcactgcgcgaatttgttacagccaaatttgccaaacttgagcaatattttgaccgaatcaaccaggtctatgttgttctgaaagtggagaaagtcacccacacctcagatgcaacactgcatgtaaacggtggtgaaattcatgccagcgcggaaggtcaggacatgtacgctgccattgatggcttaattgataagctggcacgccagttgaccaaacataaagataaactgaaacaacactaattgtccgggcaattagcatgtgcatggcggtctgttgtgcggcacaacgggccatttgtacggttaatgctccgagcctgttccactgtttgagtgggcaggttcttaggtgaaattatgacaaataatgatacaactctacagcttagcagtgttcttaacagggaatgtacgcgaagccgcgtccactgtcagagcaaaaaacgcgccctggaaatcatcagcgagctggcggcgaaacaacttagcctgccgcctcaggtggtttttgaagctatcctgacgcgggaaaaaatgggcagtaccggtatcggcaatggtattgccattccgcatggcaaactggaagaagatactctgcgcgccgttggcgttttcgttcagctcgaaacgcctatagctttcgatgccatcgacaaccaaccggtggacttactttttgccctgctggtgccggcagaccaaactaaaacgcacctgcatactctgtcgctggtggcgaaacgtctggcggacaaaaccatctgccgccgtttacgcgcagcccagagcgatgaagagctgtatcaaatcattacggataccgaaggtactccggatgaagcgtagttattcggtaatgtctcttttagacgttgtgaggagaaacagtacatggtactgatgatcgtcagcggacgttcaggttcaggtaaatctgtcgccctgcgtgcgctggaagatatgggtttttactgcgtggataaccttcccgtagtgttgttacccgatctggctcgaaccctggccgatcgcgagatttctgccgccgtcagcattgatgttcgtaatatgccggagtcaccagaaatattcgaacaggcgatgagtaacctgcctgacgctttctcaccgcaactcctgttcctggatgccgaccgtaataccttaattcgtcgttacagtgacacgcgccgactgcatccgctttccagcaaaaacctgtcgctggaaagtgctatcgacaaagaaagcgatttgctggagcctctgcgttcgcgagcggatctgattgtcgatacctcagaaatgtccgttcacgagctggctgaaatgctgcgtacccgtctgctgggtaaacgtgaacgcgaactgaccatggtctttgagtctttcggcttcaaacacggtatccctatcgatgcagattacgtctttgacgtgcgcttcttgccgaacccgcactgggatccgaaactgcgtccaatgacaggtcttgataaacctgtcgccgcgttcctcgaccgccacacagaagtacacaattttatctaccagacgcgaagctatcttgagctatggttacctatgctggaaaccaacaaccgtagctacttgacggtcgccattggttgtaccggcgggaagcaccgttcggtgtatattgcagagcaactggcagactacttccgctcgcgcggtaaaaacgtccagtcacgccatcgtacgctggaaaaacgtaaaccatgaccgtcaagcaaactgttgaaatcacaaacaagctgggcatgcatgcccggcctgcaatgaagctgtttgaattaatgcagggttttgacgctgaagtgctcttacgtaatgacgaaggcaccgaggctgaagccaacagcgttattgcgctgctgatgttggattctgccaaaggacggcagattgaagttgaagcgaccggtccacaggaagaggaagcactggccgccgttatcgccctctttaattctggttttgatgaagattaatcttcatcactttgacatacaactcccttcaaactccccccgacaataagaaaatcacgtactgaaatcgttctcaatcaacgtcatttgtacattttgtgcgcttttcactttcagaagaaccttaagaaaaccttaagaggcattgtttaggttttgtttaagttaatcgaccatactggagatcgtcagaaaatatttccaggagatggcatgattcgcttatctgaacaaagtcccctgggcaccggaagacatcggaaatgttatgcgcatccggaagatgcccaacgctgtatcaagattgtctaccatcgtggcgatggtggcgataaagagatccgccgtgagttaaagtactacgcgcatcttggtcgccggttaaaagactggagtggaataccgcgctatcacggtaccgttgagacggattgcggaaccggttatgtctacgatgtgattgcagattttgacggcaagccttccattacgctgaccgaatttgctgaacaatgccgttacgaagaagacattgcacaactgcgccagctactgaaacagctgaagcgttatttgcaggataaccgtatcgtgacgatgtcgctgaagccgcagaatatcctctgtcaccgcatcagtgagtcagaggttatcccggtcgtctgcgacaacattggtgaaagcacattgattccactggcgacctggtcgaagtggtgttgtctgcgtaagcaagagcggttatggaaacgatttatcgcccaaccggcgctggctattgccctgcagaaagatctgcaacctcgtgagagcaaaacgctggccctcacttcgcgcgaagcttaatccagctggtgttgttgcataaacggctcaccgcctaactgatacatctgccgtaaaatccacgcctgacggctacgcacgtagcccgatggcgaggagactttgaaacgaagtggattaggtaatacagctgccagtaatgcagcttccgaccgggtaagtttgctcgcgggtttgtggaaataacgttgtgccgcagcttcgacgccaaacacaccgtcgccaaattcggcgatattcaggtaaaccgtcaggatacgctttttgctccagaccgtttctatccccagcgttaatccggcttccagcccttttcgaacccagctacgcccatcccataaaaagagatttttggctgtctgttgagaaatcgttgaagcaccgcgaatacggttttcattgcgctcgttgtgcgccagggctttctcaatggaagcgacatcaaagccccagtgctcaggaaatttctgatcttctgcggcaatcaccgccagtcccatccacggcgagatttgatccatactgacccagtcagaatgtgccacgtaacgaaaattgccatgcagccaggcgctgacctgtcgctcgaccattaccgctgagaagggaacaggcgcaacgctaaacaacgcgatgcccccgccccagaaaacggcgaggacaaccattaaccgcaaaagaaaacggcgaacgaaactaaacaccgttaagcggcttttactcattcagccagaaccagcacgcgggaaaccagcttatcaatgccgctcgccgcttctgcaatgttctgcgccagcatatatgctggggtggtgacaatcttattgtcttcatcaaccacgatatcatcgacaggacacggcacatgctccgcgcccatctcttccagcacttctgcggtatcgatatcagtaccgatggtcaaacgcagcgggaaatcgaaaattttcggcagcatcgccggggcaatacacataaaaccaagcggttttccggcctgatgcatcgcttgtgccagcgcctttaattcacggtcaacggtgcattcgctaccaagactggcaaaattgcttaaattcttcgccgcgccaaacccccccggcacaatcaacgcatccagttcagcggcatcggcctgggccagaggacggatttcaccgcgcgttattcgtgccgcttcaatcagcacattgcgcgtttccgtcatcgcttcgccagttaaatggttgataacatcaacctgctgcttatccggtgcaaagcagaccgcctgcgcaccgctgcgtgaaatagctaacaacgtcaacaccgcttcatgaatttcagaaccgtcatagacgccgcatccgctcagaattacgccaattttcttcattgtgatcatcctttcgcaattgactgaaacacattaatttttttaataaaaatggtacgcatcacacatttaactgattcatgtaacaaatcatttaagttttgctatcttaactgcgtgcggcctgaaaaacagtgctgtgcccttgtaactcatcataataatttacggcgcagccaagatttccctggtgttggcgcagtattcgcgcaccccggtctagccggggtcattttttagtggcttttgccacccacgctttcagcacttctacgtcgtgacgccactcttctttcatctcttcaatccattcaccgacgttatcttcccaggccggaaggtcaggagactgaatttgctgacccagctgttgcagatggcgtaaccccactgaccccgccgcacctttaattttatgtccttcctcaacaatgccttttttatcctgcgccgtcagattcgactccagcacgctgacatagcccggcatcatcttctcaaacaccgctaacccgtcggtgatcagcttcggtcctacaagttcgagatactgttccagcatgggaatatcgagcaatgcttctgatttactgttctcttctgtcgtcaccgtactctcctcatcatcctgggtatcccagaatttcttgatcatcgcggttagcgccggaacagaaagcggcttactcagcacatcatccattccagcattgaggtactcttgtttgtctttcagcacgttagcggttaaggccaccagcggcggtaaatcctcgcgcggataacgtttcgtcagttcacgagagatatccagcccggtcatatctggcaactgaatatccagcaacaccaggtcgtattcgcccggtttaaacatctccagcgccgccttgccggtcatggcgacatcaacgctgttacctaatttttccagcacagaacgcgcaacaatcacgttcagttcaatgtcttccaccagcagcacattcagcgccggtaaaggcatatcgtcttcatcaaacgcatcatcgacctcttctgctaccgacggtgcgtggatcgtcaacgtaaaggttgaacctttgccctgttcgctggtaaccgtaatatcgccgcccatatttttcgccagacgacgagaaacggccagaccaataccggtgccggtggcaggtttaccgccatgactgtctttcacctggtaatacatggcgaaaattttatccagctcatcctgcggaatgccgataccagagtcttccacttcaaaatgcagcatatcgccttcatcgtagcgcacgcgcacggtaacctggccttgctgggtgaatttgacggcgttactgatgaggttccacaggatctgccgtaaacgcgtcccgtcggtaatgacctgatgcggtaatggcagcgtcggctccaggttaaagcgcaatcctttttgttgcgcctgcaatgcggagagattttccagatcggcaaggaagctggtgaaatcaaccggttgattatcaagctggaccttgcgccgttccatcttatccatgtcgataatatcgttaaagatattccccagcgtgacggccgaaacatggatggtcttgagatatttttcctgctcggcggtgagttcggtatccagcagaatgcggctcagaccgacgataccgttcagcggtgtacgcaattcgtgactgatggtggagataaacgtcgttttgtcgcggctggcccgttcaagcgcatcctgataccgcttacgctcggtaatgtcgcgaccaaagcccatcaaaccgtgacgtttacccacgcggtcgtagtacggcactttacggatttcaaagcaggctttgcgcccgtccgggtaatccagccactgttcataggtcagtgacacattatgacggaacactttttcatcggtttcaatgacttttgcggcggcttccggtgagtaaacatcagcaggtttcaggtgaaccagttgtttttcgctttttccggtcagcagctccatcgcgcggttacagccggaaaactctttatcttcgttacgataaaaaaccaggtcgggtgaagcatcaaggaaggaacgtaagaatgaggattgctgctcgagctgaatttgtgtctcttcgcgctctttgatttcaattttcagttggccgaaggtttcctgcagttctgcttccgctttttcacgaacggcaatttcctgatttagctgggcaatattatcttttaactgaacgttgaggctcaaatcgcgctcgcgcatctcctccagtttttgcaccagccgtgacagacgttgtcgtgactcctccagttgctcgacgaccaccgatagaaagtagaccgcccacggcgtaatcagcaaaccaaagaagatagaacgaataacatcaatgctttcgacctgaccatgcagcaccatggttaccgccatttgtaccacaatggcaagaacgacgagggccagcgccagcaacattgagaagcgcaccagacctaacttcatcatcaggtcaacataatactgcgccagcagacgaatttgcttcattagggaattccttcacgacaacctgccccaataatacccaattctgacagttacgttataaattgtgtgagaaatgcggaattcccctcaacgacctactccgttggaggtagccacggacgtcccagcgccgatccctgtacgccatgttcattcagatagcgatccagctcgaccattcccgtccatcgattttcgcaccacagcggagcaagcagcgtcgggcgacgggcgctggcggaaatgcggtggtagatcacttccggtggcgtatggcgaatcatttctccggcagtgagcgtgtaatcctccagttcaataccgttcaaacgccccgcttcccaggctttcgccataatgctgcctttcacaatatgcagcggatgcagctttatgccgtccacgccggtttcaaccactcgctccagcgtttgcaaacattcagcctgcccttcgccaggcaggccgacaattaagtgggaacacaccttcagcccgcgctgacgtgccagctgggttgtacgctgataacaggcaaaatcatggccgcggttgatgcgatgcagtgttttgtcgtgggcggtttgtagccccagctccagccacacttcgtaaccctggtccttatattcgcaaagcagatccagcaccgcatccggcacgcagtccgggcgggtacccacacacaaaccgacaatattggcctggctcaccgcctgctgatacatagaacgcagcacctgaacttccgcaaaggtgctggtatacgcctgaaagtaggccagatagcgtttagcgcggttaactaaattcgcctggtgcgccagttgctcggcaatggaacgatgctgctgcgcttcatcggcaaacgaggcaacattacagaatgtgcagccaccacgcccgatggtaccgtcacggttagggcagctaaaaccgccgtgcagcgtcagcttatgcaccttttgcccataacgacgggtgagatcaccaccaaacatattgactaatttctgtaactgcataatctgatagaccgcgccttgaaaagaggccaaagcctgccatttttagctcaattcggcgatgacctggatcaatcgtcccggcctgcttttatcaactgcataatcaatcaaaattaccgaaatttcatgcataatcacataaatcacttttgcttatcttgtgtcagatttttttatctcctgatggattttaggcaaaaacagtagcatgaaacgtcattaccaattaaggcagtataaaatgctggttttgtcgtcagttcaaggcaggataagggttaacacacctttatgacagtcaggaattgactgtttctctaacgacttcccttttagccttaaagataaaatccattttaatttcagtcatttaataaagaattttgcgctaaagcacatttctgtaccaataagcttgccatttgacctgtatcagctttcccgataagttggaaatccgctggaagctttctggatgagcagcctgctcatcatatttatgcagtaattgagatcccctcttcaccgtattaaccgatgcgaaaaggacaacaagggggcgaatgcgaggcgcgcgtatgacacgcaaaccccgtcgccacgctctttctgtgcccgtgcgcagcggttcggaagtggggttcccgcagagcctgggggaggttcacgatatgttgtacgataaatcccttgagagggataactgtggtttcggcctgatcgcccacatagaaggcgaacctagccacaaggtagtgcgtactgcaatacacgcactggcccgcatgcagcaccgtggcgcgattctcgccgatggtaaaaccggcgacggttgcggcttgctgttacaaaaaccggatcgcttttttcgcatcgttgcgcaggagcgcggctggcgtttagcaaaaaactacgctgtcgggatgctcttcctgaataaagatcctgaactcgccgctgccgcacgccgcatcgttgaagaagaactgcaacgcgaaaccttgtcgattgtgggctggcgtgatgtccccactaacgaaggcgtgctgggtgaaatcgccctctcctctctgccacgcattgagcaaatttttgtgaacgccccggcaggctggcgtccacgcgatatggagcgccgtctgtttatcgcccgccgccgcattgaaaagcgtctcgaagccgacaaagacttctacgtctgtagcctgtcgaatctggtgaacatctataaaggtctgtgtatgccgacggatctgccgcgcttttatctggatcttgcggacctgcgtctggaatcggccatttgcctgttccaccagcgcttctccactaacaccgtaccgcgctggccgctggcgcaaccgttccgctatctggcgcataacggtgaaatcaacaccatcaccggtaaccgccaatgggcgcgtgcgcgtacttataaattccagacaccgcttatccctgacctgcacgacgccgcaccgttcgtcaacgaaaccggctctgactccagttcgatggataacatgctggaactgctgctggcaggcgggatggatatcatccgcgccatgcgtctattagtaccacccgcctggcagaacaacccggatatggacccggaactgcgtgccttctttgactttaactccatgcatatggagccgtgggatggcccggcgggcatcgtgatgtccgacggtcgttttgccgcctgtaacctcgaccgtaacggtctgcgtccggcgcgctacgtcatcaccaaagataagctcatcacctgcgcctctgaagtcggtatctgggattaccagcctgacgaagtggtcgaaaaaggccgcgtcgggccaggcgaactgatggttatcgacacccgcagtgggcgtattctgcactcggcagaaaccgatgacgatctgaaaagccgccatccatataaagagtggatggagaaaaacgtccgccgactggtaccgtttgaagatctgcccgatgaagaagtgggtagccgcgaactggacgacgacacgcttgccagctaccagaaacagtttaactacagcgcggaagagctggactccgtaattcgcgtactgggcgaaaacggtcaggaagcggtcggttcgatgggcgatgataccccattcgccgtgctctccagtcagccgcgcattatttacgactacttccgccagcagtttgcccaggtgactaacccgccaatcgacccgctgcgtgaagcgcatgttatgtcgctcgccaccagtatcggtcgtgaaatgaacgtcttttgcgaagcagagggccaggcgcaccgtttaagctttaaatcgccgattctgctctactccgatttcaaacagctcacgacgatgaaagaggagcactaccgcgcagatacgctggatatcacctttgacgtcactaaaaccacgctcgaagcgacagtcaaagagctgtgcgacaaagccgaaaaaatggtacgtagcggcaccgtgctgctggtgctctccgaccggaatatcgctaaagatcgcctgccggttccagccccgatggcggttggcgcgatccagacccgtctggtcgatcaaagcctgcgttgcgatgccaacatcatcgtcgaaaccgccagcgcccgcgatccgcaccacttcgccgtgttgctgggcttcggcgcgacggctatttatccataccttgcctatgaaacgctgggccgcctggtagacacccatgcgattgccaaagattatcgtaccgtgatgctcaactaccgtaacggcatcaacaaaggcttgtacaaaatcatgtccaaaatgggcatctccaccatcgcctcttaccgctgctcgaaactgtttgaagcggtcggtctacacgatgatgtagtgggcctgtgcttccagggggcggtcagccgcattggtggagcaagctttgaagacttccagcaggatctgctgaatctgtcgaaacgtgcctggctggcgcgtaagcccatcagccagggcggtctgctgaaatacgtccacggcggcgaataccacgcctacaacccggacgtggtgcgcacgctgcaacaagcggtacaaagcggcgagtacagcgactatcaggaatacgcgaagctggttaatgagcgtccggcaaccacgctgcgcgatctgctggcaattacgccgggtgaaaacgcggtcaacattgctgatgttgaaccggcaagcgaactgtttaaacgctttgataccgccgcgatgtctatcggcgcgttaagcccggaagcccacgaggcgctggcggaagcgatgaacagcatcggcggtaattcgaactccggtgaaggcggcgaagacccggcgcgctacggcaccaacaaagtgtcgcgcatcaagcaggtggcttccggtcgctttggggttactccggcgtatctggtcaatgccgacgtcattcagattaaagtcgcccagggcgcgaagccaggcgaaggcggtcagttgccgggtgataaagtcacgccttacatcgccaaactgcgctattcggtgcccggagtgacgctgatctccccgccgccgcaccacgatatctactctatcgaggacttagcgcagctcattttcgacctcaagcaggttaacccgaaagcgatgatctccgtgaagctggtttccgaaccgggagtaggcaccatcgcgactggcgtggcaaaagcttatgcggacttgatcaccatcgcaggctatgacggcggcaccggcgcaagtccgctttcatcggtgaaatacgcaggctgtccgtgggagctggggcttgttgaaacccagcaggcgctggttgctaacggcttgcgtcacaagatccgtttgcaggtcgatggcggcctgaaaacgggtgtcgatatcatcaaggcggcgattctcggcgcagaaagcttcggcttcggcactggcccgatggtggcgctcggctgtaaatatctacgtatttgccatctgaacaactgcgcaacgggtgtagcaactcaggatgacaaactgcgtaagaaccactatcacggcctgccattcaaggtgacgaattactttgagtttatcgcccgtgaaacccgcgagctgatggcacagcttggcgtaacacgtctggtggatctgattggtcgcaccgacctgctgaaagagctggacggtttcaccgccaaacagcagaagctggcgctgtcgaagctgctggagactgccgaaccgcatccaggtaaggcactctactgcaccgaaaacaacccgccgtttgataacggcctgctgaacgcgcagttgctgcaacaggcgaaaccgtttgtcgatgagcgccagagcaaaaccttctggttcgatattcgcaacaccgaccgttctgtcggcgcgtcgctttcaggctatatcgcccagacgcacggcgatcaggggctggcagccgatcctatcaaagcgtacttcaacggcaccgcaggccagagcttcggcgtgtggaacgcgggcggcgtggaactgtacctgaccggtgatgccaacgactatgtcggtaaaggcatggcgggcggcttaatcgccattcgtcctccggttggttccgccttccgcagccatgaagcaagcattatcggcaacacctgcctgtatggcgcgaccggtggtcgtctgtatgccgcaggccgcgcgggtgaacgtttcggcgtgcgtaactccggtgctatcaccgtggtagaaggcattggcgacaacggttgtgaatatatgacgggtggtatcgtctgcattctgggtaaaaccggcgttaacttcggtgcgggcatgaccggcggtttcgcttacgttctcgatgaaagcggcgatttccgcaaacgcgttaacccggaactggtcgaggtcttaagcgttgacgctctggcgatccatgaagagcatctgcgtggtcttatcaccgagcatgtgcagcataccggctctcagcgcggtgaagagattctggcgaactggtcaaccttcgccactaaatttgcgctggttaaaccgaagtccagtgatgtaaaagcactgctgggtcaccgtagtcgtagcgcagctgagttgcgcgtgcaggcgcagtaaggggtagcaacaatgagtcagaatgtttatcaatttatcgacctgcagcgcgttgatccgccaaagaaaccgctgaagatccgcaaaattgagtttgttgaaatttacgagccgttttccgaaggccaggccaaagcgcaggctgaccgctgcctgtcgtgcggcaacccatactgcgagtggaaatgcccggtacacaactacatcccgaactggctgaagctcgccaacgaggggcgtatttttgaagcggcggaactgtcgcaccagaccaacaccctgccggaagtttgcggacgagtctgcccgcaagaccgtctgtgcgaaggttcctgcactctgaacgatgagtttggcgcggtgaccatcggcaacattgagcgctatatcaacgataaagcgttcgagatgggctggcgtccggatatgtctggtgtgaaacagaccggtaaaaaagtggcgattatcggcgcaggcccggcaggtctggcgtgtgcggatgtcctgacgcgtaacggcgtaaaagccgttgtcttcgaccgtcatccagaaattggcgggctgctgaccttcggtattccggccttcaagctggaaaaagaggtaatgacgcgtcgccgtgaaatcttcaccggcatgggtattgaattcaaactcaataccgaagtgggccgcgacgtacagctggacgatctgctgagtgattacgatgccgtgttccttggcgtcgggacttatcagtcaatgcgcggcgggctggaaaacgaagacgccgatggcgtgtacgcagcgctgccgttcctcatcgccaacaccaaacagttaatgggctttggtgaaacccgcgacgaaccgttcgtcagcatggaaggcaaacgcgtggtggtccttggcggtggcgacactgcgatggactgcgtgcgtacgtccgtgcgccagggagcgaagcacgttacctgtgcctatcgtcgtgatgaagagaacatgccgggttcccgccgcgaagtgaaaaacgcgcgggaagaaggcgtagagttcaaattcaacgtccagccgctgggtattgaagtgaacggtaacggcaaagtcagcggcgtaaaaatggtgcgtaccgaaatgggcgaaccggacgccaaaggccgtcgccgcgcggagatcgttgcaggttccgaacatatcgttccggcagatgcggtgatcatggcgtttggtttccgtccacacaacatggaatggctggcaaaacacagcgtcgagctggattcacaaggccgcatcatcgccccggaaggcagcgacaacgccttccagaccagcaacccgaaaatctttgctggcggcgatatcgtccgtggttccgatctggtggtgaccgctattgccgaaggtcgtaaggcggcagacggtattatgaactggctggaagtttaagcgaggtaacaatgaattcgccagactgtgtctggcgaatcaaattactgacgaagtgcgcgttgttttctggcaaatgcggcatgagcgtttgacctttcctataatagggataattttcaataaattgtgctttgttcaccaagtctgatgagtgaagcacatcaagcaatttctcatttacaatccgtctcaattacttgttaacacctctgacaataccgattctgcaagctattcagtcttttcattccatgtaaattgtctcgatattaatatacaaaatatgaatataaaaaaccaatatattatccttaattatctatatattttcctatttttcagcgcaaacattcatgtaatgaataattatcaccacaaaccacctcaccagcaccttattattcacatgatcgtaactataaaattcattaaataaatacatcccagcaagttggctatttctgaacgagttatttatttacattcacaaacagatatatatactgcttcagctttttattttaaaaaataaatttgttattaaggatatgttcatatgtttttcaaaaagaacctcacaacagctgctatttgtgcagcactttctgttgcagcattcagtgccatggcaacagattcaactgatacagaattaactatcatcggcgagtatacccctggtgcatgtaccccagttgttacgggcggcggcattgttgactatgggaaacatcataacagtgcgctgaatccgaccggtaaaagtaataaactggttcaactgggccgcaaaaacagcacattaaatataacctgcacagcaccaacgctaattgctgtaacctccaaggataaccgtcagtcgaccattgtagcgttaaacgacacatcctatattgaaaaagcttatgatactctcgtagatatgaagggaacgaaaaacgcctttggtttaggttctgcgcctaatggacaaaaaattggcgctgcatccattggtattgacaggtctaatggtgggattcacgcggcggacgatacaggtgaaattcctgtcgacctgattcaaactgaccactggtcagcagcgacccccacatggaaagcctcatctaatggcgcattctgctcgctgacaagttgctcagcaatcgagcgcggttattctgttgcaaaaacaggggaactgacacctgttgctattacagcggtcaccttcccgttactgattgatgctgcggtaaatgacaatactattcttggttctgatgaaacgatcaaactggatggtaacgtcactatcagcgttcagtatttataagaacttgtaatacagtttttatttttacgcattaaccagttagctataactcggacagattatgccctatgacatggtctgtcttaatcaatctcatcgcaaacagtgcataacatatattaacaatatgtttctgcgttatttatcattattacaggagttttaatttaaatgctcagacacattacattcactgtatttataacaacatcaatgaataccttagccacagggatggttcctgaaacatcagtattgctggttgatgaaaagcgtggtgaagctagtattaatattaagaatacagatgatcatccttcattgctttacaccaccattgttgatttgcctgaaagcaataaatcaattcgtttaatcccgactcagcccgttattcgtgttgaagccggtcaagtacaacaggttcgatttttacttcaggcgactgttcctctgcaatcagaagagctgaaacgcgtaacgttcgaaggtattccaccaaaagatgacaagagcagcagagttactgtttcaattcgtcaggatctacctgtactgatccacccggcttccctgccggaagagcgagagacctggaaattcctggaatggcgtaaaaatggcgaccaaattgagattagcaaccccagtaattatgtcgttcgtatgaccttacaatttaaaacgctcccttcaggaaaaacgggggctataaataagacctattttctaccacacaccagtacaactactgcattaacaaacgctacggatacaaaagtcgagttttacccagccagccgatatggttatcgcggtaataaatatgtcactgacttaaaataactttgcctggagcgacaaggatgttaaaaaaaacgttactggcctacaccattggttttgccttttctcccccagccaatgcagatggtatagagattgccgctgttgattttgatcgggaaacattaaaatcactaggtgtagatcctaatatatcgcattatttttcccgttcagcccgttttttgccaggtgaatattcactgatagtatcagtaaatggcgaaaaaaaaggcaacattgctacgcgctttgatgaaaatggcgacatttgtcttgatcaggcatttctgcaacaagccggtttaaaaattccttctgaagaaaaaaatggctgttacgactatatattgtcctacccgggtaccacaatcacaccattacctaaccaggaagcgttagatattatcgtttcaccacaggcgatcattcccatagggttggatctcacaaacgcagcaactggtggaacagctgcgctgctaaactactctctgatgagcagccgtgcagaattttctaatgggagttcggactactcccaggctgcacttgaaggcgggattaatattaatgactggatgttacgcagccatcagttccttacacaaacaaatggcacattcagtaaccagaactcgtcaacctaccttcaacgtacctttacagatcttaaaacactcatgcgagcaggtgaagttaacctcaataatagcgtgttggaaggagccagtatttacggtatcgaaatcgcaccggacaacgcattgcaaaccagcggcagtggtgtgcaagttactggtatagccaacacctctcaggctcgtgtcgagattcgtcaacaaggagttttaattcattccattctggttcctgcgggcgcattcactatccctgatgtacctgttcgcaatggtaatagtgatcttaatgtcaccgttgtcgaaacagacggtagttcgcacaactatattgttccctccaccctgtttaatcagcatgtagaaagcttccagggttatcgcttcgcgatagggcgggtagacgatgactatgacgaatcaccttgggtaattagtgcatcgagcggatggaatctgacacgctggagtgcaatgaacggcggcgttatcgtagcagaaaattatcaggcggcatcaatccggtcgagtctggttcccctgcccgatttaacagtgagcagccaaattagtacatcgcaggatacgaaagactcactgcaaggacagaaatatcgtcttgacgcgaactacaatctcccattttcacttgggctaacaaccagcctcactcgatctgatcgccattatcgcgaactgtctgaagcgattgatgatgattataccgatccgactaaaagcacttatgcgcttggtttaaactggtctaactccattctgggtggtttcaacatcagtggctataaaacatatagttacgacggtgacaatgactcaagcaaccttaatattaactggaacaaagcgttcaaacacgccacggtttccgtcaactggcagcatcaacttagtgcttcagaaaataatgaagacgatggtgatctgttctacgtcaacatcagtattccatttggcagatcaaacaccgccacactgtatactcgccatgacgatcataaaacccactatggtactggtgtcatgggagtcgtctcagatgagatgtcctactatgtgaatgctgaacgagatcacgacgaacgtgaaacgagcttgaacggcagtatcagttccaatctccattacacccaagtcagccttgccgcaggagcaagcggcagtgatagccgtacttacaacggtacgatgtcaggtggtattgccgtacatgatcagggagtgaccttttcaccgtggactatcaatgacactttcgccatcgcaaaaatggataacaatattgcaggtgtcagaattacatctcaggcaggcccagtatggacagattttcggggtaatgccgtcattccatcaatccagccgtggcgaacatcaggagttgagatcgataccgccagcttgccaaaaaatgtcgatatcggtaacggcacaaaaatgatcaaacaaggccgtggtgcagtagggaaagtcggattcagtgcgataacacaacgccgtgcattactcaatatcacactttccgacggcaaaaaactgcccagaggcgttgcgattgaagatagtgaaggcaactatctgacaacatcagtggatgacggtgttgtattcctcaataacatcaaaccggacatggtgctagatataaaagatgagcagcaatcatgccgtattcaccttacattcccagaagatgcaccaaaagatgtgttctatgagacagcaacaggagagtgccaatgaaacggataataacaggatgcctgctgctgaacttcgccatggccgctcaggcagagtgtaatatctccagtagcatacaaaatatcgactatggcaaacgaagtgctgccatgcgccaagttgaccggggtaaaacaacacaattagcagacagaacaatcacgctggtaatgcaatgcgatcaggacgctcatattcgtgttcagttgaataccgctaatatttccaacaacggatttggatttggcccgaatggttcattaaatctgatcgccagcgatgcattttcaggtagtaacaatctcgacctggcgttagccagtggcaaaaatgacaatccgggcagcacaggaacagcatcaattagggaaggtgcgaataagcggggaaattcttctcggctgactcagtcatttcatttcttcatgtttgagccgattttttctcccgtaaatgccttgaatcagcctatttagaccgtttcttcgccatttaaggcgttatccccagtttttagtgagatctctcccactgacgtatcatttggtccgcccgaaacaggttggccagcgtgaataacatcgccagttggttatcgtttttcagcaaccccttgtatctggctttcacgaagccgaactgtcgcttgatgatgcgaaatgggtgctccaccctggcccggatgctggctttcatgtattcgatgttgatggccgttttgttcttgcgtggatgctgtttcaaggttcttaccttgccggggcgctcggcgatcagccagtccacatccacctcggccagctcctcgcgctgtggcgccccttggtagccggcatcggctgagacaaattgctcctctccatgcagcagattacccagctgattgaggtcatgctcgttggccgcggtggtgaccaggctgtgggtcaggccactcttggcatcgacaccaatgtgggccttcatgccaaagtgccactgattgcctttcttggtctgatgcatctccggatcgcgttgctgctctttgttcttggtcgagctgggtgcctcaatgatggtggcatcgaccaaggtgccttgagtcatcatgacgcctgcttcggccagccagcgattgatggtcttgaacaattggcgggccagttgatgctgctccagcaggtggcggaaattcatgatggtggtgcggtccggcaaggcgctatccagggataaccgggcaaacagacgcatggaggcgatttcgtacagagcatcttccatcgcgccatcgctcaggttgtaccaatgctgcatgcagtgaatgcgtagcatggtttccagcggataaggtcgccggccattaccagccttggggtaaaacggctcgatgacttccaccatgttttgccatggcagaatctgctccatgcgggacaagaaaatctcttttctggtctgacggcgcttactgctgaattcactgtcggcgaaggtaagttgatgactcatgatgaaccctgttctatggctccagatgacaaacatgatctcatatcagggacttgttcgcaccttccttagtacttcccccaataattggctggtgtttatgcaaaatggtcaagaagtggtaattgatagcggtaaaagcgttagcctcacactgacaatggctccagcttttaaggatgaaggggaactaaccgacatgacagatattacaggcaatctgacggtcctggtggaggcaaaatgaacaatgtaaaattactgattgccggaagtgccttttttgccatgtcagcgcaagccgctgatagagtatcaattgacgttaaggtgactctggaagctgcagcttgtactccaatactaagcaacggcggagttgttaacttcggtagtcattcagtcaatagactttcaacgcagcactacacacagattggaacacgtaatattaatatgactataacttgcgaatccgctaccggcattgcgattaccgctcgtgatacacgaatggatagtatgaccaccggaaaagatagtgggggtcagagtggtgtaaaatataccttaaatggcggaggttatattagccagacaacgcgcttattcggcttagggaaaacaaaagataataaaaatatcggtagttatgccgtgttaattgatagcaacaacattagtgccagcaatggtagccagacgttagctgtatcaatagcaggtgcagatgccgtcataacagggcaaaaaagagcatggcaaacgctcaccgcttatccgcttgcagtcgatcaaagctattattacacctttgtaaaaccaggtgaaacaaccccaactcctgtaacgaacgccattataccgcttcaggtgagcgcatctatcgcgaatgatttaggcggttcagaaaaaatcgaacttgatgggaaagctgtgataagcgtagtctacttgtgataacaatgccggacaggagtactatcaggcattcgttttatacgatcggttaatgtttcaggaaagctcttcgcatatcttggggaaagtaaatgtaatacgctgttcttaattgttcagtgctcaccccccagagtatagctcattccattattcaacttagctccatataaagggacagataatggaatcgctctcagaaggaaccacagcaggctaccagcaaatccacgacggtattattcatctggtcgatagcgcccggacggaaacggtacgtagcgttaacgcgttaatgaccgcgacgtaccaggaaattggccgacgaattgtcgaatttgaacaaggtggcgaggccagggctgcgtatggtgcgcagctaatcaagcgactatcaaaggatttatgtctaaggtataagcgtgggttctctgcaaaaaacttacgccaaatgaggcttttttacctcttttttcaacatgttgaaattcaccagacaatgtctggcgaattaacaccattgggaattccgcagacaccgtctgcagaattcccatcggcaaagatttggcagacgctgtctgccaaatctttccccttgcccaggtccacctacgtccgtttactttccgttaaaaacgctgacgcccgcagcttttatgaaaaagagacgctccgctgtggctggtctgttcgccagctagagcggcaaattgcgacccagttttatgagcggacactactgtcacatgacaaatcagccatgctgcaacaacacgctcctgccgagacgcatattcttccgcaacaggcgatacgcgatccctttgtgctcgaatttctggaattgaaagatgaatattcagaatccgattttgaggaggcgctgatcaaccacctgatggatttcatgctggaacttggggatgattttgcctttgttggtcggcagcgaaggttacgcattgatgacaactggtttcgtgtcgatctgctgtttttccaccgccgtttacgctgcctgctaatcgtcgatctaaaagtgggcaaattcagctatagcgatgccggacagatgaatatgtatctcaactacgccaaagagcactggacgctaccggatgaaaatccgcccatcggtctggttctctgtgcagagaaaggagccggagaagcgcattatgctctggcaggtttgcctaacaccgttctggcaagcgaatataagatgcaactacctgatgagaaacgactcgcagatgaactcgttcgaacacaggcggtgctagaggaaggctatagacgccgttaatttcagcggtttcgaattctgcagacagtgtctgcagaatctttaaaacgaactaagttttaagccattaaatcagccttaaccttcaccacaacctttttaatctctccaggctcgccgacaacgcatcctggtttatgcggttcacctggcataaacacggcgaacattcccggttttaagatgatggcttgctcgttatcaatggtgctgcaaagctgataatcatcctcatggtggaactcttcacactgacgcgcagtgcctgccatgccaaacagaatccgttcctcaccgtttaataacagctggatatcaatgtattgctcgtgcaattccgcttttttctcgacgggcgattgagtgttaaacgtcatgacattcataaagatattgtcgccctgtaattcgtaacgacccggcgctttttcttgcggtctggcagctaatgccagcgttaacgcgtcctgtaacgcaggatgtaacccagcagacggtaatgactgtacttcacccatcatcataatttttctccctgggccaacagcgcagccccaagtaaacctgcatcatggcggtaatgcgccgccagtaaatcaacatgaaatgccgctggctcctgcgccagatacgtttccaccagcgccagatacccttctgccagaccaacgctgccaccgaccaccacgcactggcaatcagttgtggctttaatatcagcgatcagccttgcaagcgtacgtgcggagcggtgaatcagctgctgcgcctgctcgtcaccctgcccggcgcgcgtgaaaatagttttcgcatccgcgccagccaactccccctgcgctgccgctgcaatgccgcgaccagaagcaatcgcttccacgcaacctgtgcgtccacagccgcagactgggccgtgtggatcggcaagcgtatgcccgatatgccccgccagaccgccagggccggtaagcagtttgcagccgctcactacaccgccgccaacgccggtggaaacggtgataaagaccatatcggttatatcgccatccagcgcctgaaactccgcccatgctgcggcctgcgcgtcgttaatggcaatggtcggcaaattggtaagttgttccagcgttttgactaacggaaagtgtagcaatccaccaagattatgcggattaagcgccagcaagctgccgtcacggattatcccggtcgaagcgatggcaacccgctgcgcatgagcttgcaacggagagactaatgcggataaggcatcacgcaaggcttctggtgtctggctggctggcgtaggaagttcacgacgatcgcggatctgcccgtcagcgccaatcagcgcggcggcaagtttagtaccgccgatatcaatcgccagtgtggtcatagcaccgcctttttcatcgctgtgttgtaccactgacaaatgtgctcaagacgcgtgattgcagaaccgaccgtcaccgcccacgcgccgtggcgcatcgcatccgccgcctgagcaggcgtgttgtaacgcccttcggcaatcacccgacatccggcgtcgctcaacgttttcaccagcgccagatccggctcttctggcgtttcaggcgtggtatagccagaaagcgtagtgccaataatttcggctcccagcttttggcatgccaggccgtcttccggcgttgagcagtcggtcatcgccagtaaaccgtgatggtgaatacgtgccagcagcgtttcaacaggcaccggacgcgggcggtcggtgccgtcaatggcgataatgtccgcgcccgcctgcgccagcgcatcaacatcttcaatataggccgtgatgcgtaccggagaatcctccagatcgcgtttcacaattccaataatcggcacgctcaccaccgcacgcgtggcttgcagatttgccacaccttcaatgcgaatggcaaccgcgcccgcctgttctgccgctaatgccatggcggcgacgatttcgggtttatcgagcgggctgtccggaaccggctggcaggagacaatcaggccaccgttagcagcgattttttgatccagttgtgcaagtaacgacatacatcttcccttagcgaaaggcccggtacatagaccgggcaacaggattaacttttggttttgactaaatcgtttttggcgctgccaaacggcacggcaccgctgaatggtttaccgtcgatagcgtcatgagtacgcaacgcttccgggcgcaaccaacgctgaacgcgagaaggcatatccagcccaatcagcaggatcaccacgaacgtcagactgaacgagagcgatgccagcgcagtacccagatccagacgttgagcgatcaacgcgccgatgattggggccagtgcaccgcccaatgcgccaacgttgtaggtaaagcccaggcccgctgcacgctggtcggtatcgaaataaccgccaatcagttttggtaagatcccggcgatcccttgtccaagcatttgctggaagaacagtaacagaccgagcacccagacgtttgcgccgccaatcgcaaataccggaataatcagcagctgcgaggccagcaggctacaaacgtacgctttgcgggttcccagccagtcaccgaggaagccacctacgcagcatcccaccgccgcgccaaagccactaaagaacagcacattggctacagtatgcgggttataagccagatcggttttcagatacgttggcagcagcgcctgaatcggccatgagtagaggaaagcaaacaacacgaccaccatcagcattacgcccgttggccagcgtttgcctgcactctgcaccataaagctgataaagattgcggcgcataacagcccaagaacagcgacgatcgcggcattttgcaggttaccggcgaagcagaaccacagcgcagtagccgccgccagtgtcattacgatattggcaatgcgatgttcaccacggtagagaatatccaccattgtgcgtactggtgctttacctgcgtgtttctctttccagtcttccgcttccgggatgtttttacgcagccagagagcaaagatgattggcaaaatgccgataaagaacagcgcacgccagccccagaccggaaccaccaggctatagacctgagcggcaacgacggcccccacagagaagcctgaaatcaaaaaaccactggctttgttacgcagatgttttggccagctttcaatgacataggtggcgctggaaccgtattcacccgccatccccatgccgatgaccagacgagcgataaacatggtgatgtagcctggcgcaaagccgcaggccagcgtcccggccgagaagagaacgatgctggtgaccattgccagacgacgcccgtagcggtcacccatagcgccgagcatcaggccgccgaaccagcgagagataaaggctgcagagatcagacttgccgcctgcaccgtcgtcagcccgaattcaccttgtacttcggtgagtaccagggcgattaaaacgaaatcaaaaccgtcaagcagatatcccaaccaggcagcggaaaatgcgcgccattgtgcacggttgagatggcgataccacgggatattctgggttgtagtactcattgtgagtctcccgcggtgggcgatgcccacacgctttggtatgaaaattgtagggtacagatgcgtttatttcccctcacccggtaggggcgagcgaggggaaacaactcacccgcgctcttgcatcaactgctgggccagcgccttcagttctggcagatatttttcatctaccggtccaaacggtttgcggcacagcggcacagaaacgacatccatataatggaggacagttttcaggccgcggaatacgcccgttttgatcagtaaatcaatgactttattgcattcagtttgcagtttctgcgcggtctggatatcgccttctttcagcgccttaacgatcccctgatagcgccagcccatgatgttgtaggtactgccgataccaccatcagcgcccgccagcagaccagaggcgaagatttcgtcgtaaccgttatagagcacaagatcaggatgttcacgacggatctgctccatctgatagagatcgccagaggtctgtttcagcgcacctacgccaggcaatgtaacaagtgtgttgatctgatccagggtcagttttaccccactcagggctggaatgttgtacaccaccatcggcaaaccatccgccgaatcaataattgcccgatagtgatcgcagtgttcttcaaagctgaaaggatagtagaacggcgtgacggcggagacggcatcgaagccataacgtttagccgatgccgcaagttgttggctttcggcggtgctgacgcaaccgacgtgggcgatgagtttaatcttacctttcgcctcttcggcgacgatttccagtacctgttcacgctcggaaaggctttgtacaaaggcctcgccggtcgaaccacccacgtataaaccgtcgatgccctgctgaatattgaactgaaccaggcgacgcagactcgctttatccagtgcttgttgttggtcaaaaggagtcaggagtgcagccattacgccacgtaaattcgttgccataaatacctctgaagtgatgcttgtctgataaacgatatacctttatacctgttataccagatcaattaagcaacaccccatacagaaagcttataatgcgatctgcttcactaaagtggcattatttctttttgttggtggtctgaccgaaagcgtgccaggtagcagagacgctgttgagatgcgattgcaacgcacgatcggcttcgtcaggatcatgacggcggatcgcatcaacgatcgcaatatgctgttgataactaacgttgttatgttcgtgcagtgcctgatcggtaaccgttgggcgtgcggcaataagccagtcgagcagggcaacgtggatcgccatgaagattgggttaccggggatctccgccagcacgcggtggaaatcaacgtctgaacgaatgaatgccgcgttgttatccagcgactgactgttgatttccagtgcttttgccagcaaatcgatttgctcatcggtggcatgttcagccgcatagcgcaccagactggattcaaagaacagacgtaattgttcgaaatgggcaatcccaccgggatgagaaaggaaatctttcgccatgccggaaagctcaccgatgatagtgtccgcagaaggacgcgagacgcgagcgcgttcgccgttgtttatttgcaccagacctttgcgttttaacgctgccagcgcttcacgcaccgaaggacgcccgacgttaaagaacgccatcagttcgcgttcagacggtaattgttcaccttcgccaaattcacgacggcggatcatctgttccagctcttcttccaccatttcggagagttttttacgcgccagcgggcggctacgcaagttgcgaccaattgcaggtgaagaatcttcggtttgcgaatcaaatgcgttcataaggcccattctgtaaggtcagtgtgattaacatcatcagtgacatcctatcacaggattgaaagtaggggaaaatggcagggttttctctttgtgcctcatcattaccataattaacggaataattaactattgcgaaaaattaatgtaacgcagataaaaacatcccgtttgaattatttataagactattcacgagcattatgaatattatgaatgtgttcttacaaaataatcataagcgcatattttttaatgaaaaatcacctcacctacaattaaaaacacgacatccgcaccataaatagccttgcaaaaaatataacatcgttgttttcaatctgccgtttatgggattgaccgttttcttttgacacggagttcaacaatgttcggcataattatatctgtcatcgtattaattacgatgggctatttgatcctgaaaaactacaaacctcaggtggtgctggctgccgcaggtatcttcctgatgatgtgcggtgtctggttagggttcggtggtgtactcgatcccaccaaaagcagcggctacttgatcgtcgatatttataatgaaatcctgcgcatgctgtccaaccgcattgccggattggggctgtcgattatggcggtgggcggttatgcccgctacatggagcgcataggggccagtcgcgcgatggtgagcttgttaagccgcccgttaaaactcattcgctcgccgtatattattctgtcggcaacttacgtcatcggccaaatcatggcgcagtttattaccagcgcctccggtctgggtatgttgctgatggtcaccttatttccgacgctggtgagtctgggagtaagtcgtctctctgcggtggcagttatcgcaaccacgatgtccattgagtgggggattctggaaacgaactccatttttgctgcccaggtagcgggaatgaaaattgccacatacttcttccactaccagcttccggtcgcctcttgcgtcattatctcggtggcgatctcccactttttcgtgcaacgcgcttttgacaaaaaagataaaaatatcaatcacgaacaggcagagcaaaaagctctcgataatgtcccgccgctctattacgccattttacctgtgatgccgttaatcctgatgctcggctcgctgttcctcgcccacgtcgggctgatgcagtcagaactgcatctggtggtggtgatgttactgagtttgactgtgacgatgtttgttgagttcttccgcaagcataacttgcgcgaaacaatggacgatgtgcaggcgttttttgacggcatgggtacgcagtttgccaacgtggtaacgctggtggtcgcgggtgaaatatttgcgaaaggcttaacgacgattggcactgtcgatgcggttatcaggggggcggagcattctggtctgggcggtattggcgtgatgattattatggcgctggtcattgccatttgtgccattgtgatgggctctggcaatgcgccgtttatgtcatttgccagtcttattccgaatatcgcagccggactacatgtaccagcggttgtaatgattatgccgatgcattttgccacgacgctagcgcgcgcggtttcgccgattactgcggtggtggtcgttacgtcaggaattgcaggcgtttcgccttttgcggtggtgaagcggacagcgatccccatggcagtcggtttcgtggtgaatatgattgccacaatcacgctattttattaagtcattaaaaagacaaaacaggccgcctgggcctgttttgtattacttcacaacgcgtaatgccggtcgaccaccgcgtggtggctgcggaggttcatcgtcaggatgagtgtcatcatcgtgatctggcttgtcgccatcaataaccgacataacggtttcgttgtctgccgatgcctcttcatcattcatgatgctggtatcttcatcgtaggcagcttcaggctcaaacatcgtgcctgcgccattttcacgggcgtagatagccagcacggcagccagcggcacagaaacctgacgcggaatgccaccaaagcgcgcgttaaagcgcacctcatcattcgccagttccagattgccgacagcacgcggcgcaatgttgagtacgatttgcccgtcacgcgcatattccataggaacctgcacgccagggagcgtcacatccaccaccaggtgcggcgtgagctggttatccagcaaccactcatagaatgcacgcagcagatagggacgacgtggtgttagctgtgacaaatccatacagattaactccggcccagacgcatttcacgttctgcttcagttaaagaagcaaggaaagagtcacgctcaaagacgcgggtcatatagcctttcagctctttcgcacccgggccgctgaactcgatgcccagttgcggcagacgccacagcagcggagcaagatagcaatcgaccaggctgaactcatcgctcaggaagtacggcttctgaccgaagaccggcgcaatcgccagcagttcttcgcgcagttgcttacgtgcggcatctgcttcagaagctgaaccgttgatgatggtgttcatcagcgtgtaccagtctttttcgatgcgatgcatgtacagacggctttcaccgcgagctaccgggtaaacaggcatcagtggcggatgcgggaaacgctcatccagatattccataatgatgcgagattcccacagggtcagctcacgatccaccagggtcggaacgctctgattcgggttgaggtcaatcagatcctgaggcggattgtccttttccacgtgttcgatctcgaaacttacacctttctcagccagcacaatgcggacctgatggctatagatgtcagtaggaccggaaaacagcgtcattaccgaacgtttgttggcagcgacagccatgaaaacctccaggtatagtcagaatttttactgctaccagccaccaggtggccagtcagaagttgtgttacccaataaggaacgactctctttgttcgaaaatcaaacaaaaaatgagcaatacccgacatttgggcagaaaattggatgatagtttaccagattttgcgaccattgtggtgagtcgatgccggaaatggggaaaaagagatgcgctttagtctgaaatagttgacttagtcccttattggcgatgtggtttttgttttacctgtctgtcaggtggcagcaaaaagcaactttccagtttttacgctgattcagattttagctataaaaaaacccgccgaagcgggttttttcgaaaattgttttctgccggagcagaagccaattaacgtttggagaactgcggacgacgacgtgctttacgcagaccgactttcttacgttcaacctgacgagcgtcacgagtaacgaagccagctttacgcagttcagaacgcagggactcgtcgtattccatcagagcgcgggtgataccgtgacggatcgcaccagcctgaccagagataccaccacctttaacggtgatgtacaggtccagtttctcaaccatgtcgaccagttccagcggctgacgaactaccatgcgggcagtttcacgaccgaagtactgttccagagaacgttggttgattacgattttaccgttgcccggtttgatgaaaacgcgagctgcggaacttttgcggcgaccagtgccgtagtattgattttcagccattgcctataatcccgattagatgtcaagaacttgcggttgctgtgccgcgtggttgtgctcgttacccgcgtaaactttcagtttacggaacatagcacgacccagcgggccttttggcaacatgcctttaaccgcgatttcaatcacacgctcaggacggcgagcaatcatctcttcaaaggtcgcttgtttgataccaccgatgtggccggtgtggtgatagtacactttgtcagtacgcttgttgccggttacagcaactttgtcagcgttcagaacgatgatgtaatcaccggtatctacgtgcggagtgtattccgctttgtgcttaccgcgcaggcgacgagccagttcagtagccagacggcccagagttttaccggtcgcgtcaacaacataccagtcgcgttttacggtttctggtttagctgtaaaagttttcattaaaagcttacccaataaatagttacacgttggtgaacacccaaacgtcttcaattgttgaggttcacacgacaaagtccggcaaacctaccccttcgaatagcctatgccagcacacaaaaagttttgggaaaaaaactttcttgtaacgtggggtcgcaggattatagagaagtcggggtcaaagatcgacccctttttgtgatttgtgacaggttttaacccgccaaatgctcgcgcttcagatactcttcgctttgcatctcttgcagacgtgacaggcaacgctggaactcaaacttcagccgatcgccctgataaatttcatacagcggcacttctgcactcaccactaatttgacatggcgctcgtaaaactcatccaccagcgcaataaagcgccgcgcttcgctctccatcaaccgcgtcataactggtacatcaaacaacatgaccgtatgaaagagacgtgagagcgcaatatagtcatgctgactgcgggcgtcgacgcacagcgtagtaaaagagaccgccagcgtctggttctcgacgcccattgttgctaatggccgatggttgatttctaacgtcggtgaattttctcgtttcccccccgccagcgccaaccatagtttatccatttgcgcccgggtttcatcgtgaagtggcgaaagccacagatgcgcctgagtgagtgtacgcagacgataatcaacaccagcgtccacgttcattacatcacaatgctgtttaatggcatcgattgcaggcagaaaacgcgcacgttgcaggccatttcgataaagttcatccggcggaatatttgacgtcgctaccagggtaataccgcgagcgaacagggctttcatcagaccgccaagtagcatggcatcggtaatatcagaaacaaaaaattcgtcaaaacagagcacgtcagtttcggctttaaagcgatcggcaataatttccagcggatcggtctgcccctgtaaggcagttagctcttcatgcacccgcagcataaaacggtgaaagtgcaggcgctgtttccgctctcccggcaggctttgatagaaaaggtccatcagccaggttttcccgcgtcctacaccgccccacatatataagccacgcactggcgtatgctttgtgtcttcgcgtttaccccacagcttaccgacccgcgccattagcccactcgtcctgggggctggtggcgtgctattgatgagttcctgataaataatttccaggcggctgacggcctctttttgaacgtcgtcgggttgatggctgccttcattaagcgccttcaggtattgcgatgttggggtaacgctttgcatgatcttattgttattccttgaataatcggtgcgccgttgttcacggttgacgaaaaaaaggccgttctacactacgcgatatgcagtcgggattccacttctgtggaattaacggttatagtggcataatcagccgcaggcatggagcctgaagccaacaccctacggaaacaaaagacaacgggagatgttcatgacctgggaatatgcgctaattgggttagtcgtcggcatcattattggtgctgtggccatgcgttttggtaatcgtaaactacgccagcaacaggcgttgcagtacgaactggaaaagaataaagctgaactggacgagtatcgcgaagagctggttagccactttgcccgcagcgcggaattactggataccatggcgcacgactatcgccagctgtatcagcacatggcaaaaagctccagcagcctgctgccggaactgtctgctgaagcaaacccgttccgtaatcgtctggcagagtctgaagccagcaacgatcaggcaccggtgcagatgcctcgcgactattctgaaggcgcatccggcctgctgcgtactggcgcgaagcgcgactaatttatttttcgggcgcagccattgcgccctcctcttctctccctccccgactatcatttaatctggtgtctcattgttagccgtctgaaaattcaataacatcaaactgttttgaatctcttttcttatcattcaggtacgagagcaggaataatgaaaaaacaaacccagctgttgagtgcattagcgttaagtgtcgggttaactctctcggcgtcatttcaggccgtcgcgtcgattccaggccaggttgccgatcaggcccctctccccagtctggctccaatgctggaaaaagtgcttccggcagtggtgagcgtacgggtggaaggaacggccagtcagggacagaaaatcccggaagaattcaaaaagttttttggtgatgatttaccggatcaacctgcacaacccttcgaaggtttaggctccggtgtcatcatcaacgccagtaaaggctatgtgctgaccaacaaccatgtgattaatcaggcacagaaaatcagtattcagctcaatgatgggcgcgagtttgatgcaaaactgattggtagcgatgaccagagcgatatcgccctgttacaaattcaaaacccgagcaaattaacgcaaatcgctattgccgactccgataaattgcgcgtcggtgattttgccgtagcggtcggtaacccatttggccttgggcaaaccgccacctctggcattgtttccgcattaggccgcagcgggttgaatcttgaaggtctggaaaactttatccagacagatgcttccattaaccgcggtaactccggcggtgcactattaaaccttaacggtgagttaattggcatcaacactgcaatccttgcgcctggcggcgggagcgtcgggattggatttgccatccccagtaatatggcgcgaacactggcgcagcagcttatcgactttggtgaaatcaaacgcggtttgttaggcatcaaaggcaccgagatgagtgccgatatcgccaaagccttcaaccttgacgtgcagcgtggcgcgtttgtcagcgaagtgttgccaggttctggctcggcaaaagcgggcgtcaaagcgggcgatattattaccagcctcaacggcaaaccgctgaatagctttgctgagttgcgctctcgtatcgcgaccaccgagccgggcacgaaagtgaagcttggcctgctgcgtaacggcaaaccactggaagtagaagtgacgctcgataccagcacctcttcgtcggccagcgctgaaatgatcacgccagcgctggaaggtgcaacgttgagcgatggtcagctaaaagatggcggcaaaggtattaaaatcgatgaagttgtcaaaggaagcccagctgctcaggctggcttgcaaaaagacgatgtgatcattggcgtcaaccgcgatcgggtgaactcgattgctgaaatgcgtaaagtgctggcggcaaaaccggccatcatcgccctgcaaattgtacgcggcaatgaaagcatctatctgctgatgcgttaatgtcgtaaaccgggcatcaggcttacgtgtgatgtccggttaactcgtggtatgctgctgccgttcccttttttaatgacgcctccatcatgtttgtgaagctcttacgttccgttgcgattggattaattgtcggcgctattctgctggttgccatgccttcgctgcgcagccttaacccgctttccactccgcaatttgacagtaccgatgagacgcctgccagctataatctggcggttcgccgcgccgcgccagcggtggttaacgtttacaaccgtggtttgaacaccaactctcacaaccagcttgagatccgcaccctgggatccggtgtaatcatggatcaacgcggttatatcatcaccaataaacacgtcatcaacgacgccgatcagatcatcgtcgccttacaggatggacgtgtatttgaagcattgctggtgggatctgactctctaaccgatctggcggtacttaaaattaatgccactggcggtttacctaccattccaattaatgcacgtcgcgtaccgcacattggcgacgtagtactggcgatcggtaacccgtacaacctcgggcagaccattacccaggggattattagtgccacgggtcgaatcggtctgaacccgaccgggcggcaaaacttcctccaaaccgatgcttccattaaccacggtaactctggcggcgcgctggtgaactcgctgggcgaactgatgggcattaatacgctgtcgtttgataagagtaacgatggcgaaacgccggaaggtatcggctttgcgattcctttccagttagcaaccaaaattatggataagctgatccgcgatggtcgcgtgatccgcggctacattggtatcggcggacgtgagatcgcaccactgcacgcgcagggcggtggtatagatcaactgcaagggatcgtggttaatgaagtgtcacctgacggcccggcggcgaatgcgggtattcaggtcaacgatctgattatttcggtggataacaaaccggccatctctgctctggagacgatggatcaggtggcggaaattcgccctggttcggtgatccctgtagtagtgatgcgtgatgataagcagttaacgctgcaggtcaccattcaggaatatccggcaaccaattaagtcgtgcgctcaaaacaaaaaaccggagtctgtgctccggttttttattatccgctaatcaattacttattaacgaactcttcgcccagggcgatatctttcttcagcgtatccagcataccttccagcgcgttctgttcaaatgcgctcagggtaccgatagatttacgctcttccacgccgtttttacccagcagcagcggttgagagaagaaacgggcgtactgaccgtcgccttcaacgtaggcacattcgacaacgccttgttcgccctgcagtgcacgaaccagagacagaccaaaacgtgcagctgcctggcccatagacagggttgcagacccgccaccggccttcgcttcaaccacttcagtacccgcgttctggatgcgtttggtcagatcagccacttcctgctcggtaaaactaacgccaggaacctgtgacagcagcggcagaatggtaacaccagagtgaccgccaataaccggcacttcaacttcgcctggctgtttgcctttcagttccgcaacaaaggtgttggaacgaatgatatccagcgtggtaacgccgaacagtttgtttttgtcataaacaccggcttttttcagcacttcagcagcaattgcaactgtggtgttaaccgggttagtgataataccaatgcacgctttcgggcaggttttcgcaacttgctgtaccaggtttttcacgatgccggcgttaacgttaaacaggtcggaacgatccatacccggtttacgcgctacgcctgcagagataagaacgacatctgcgccttccagcgccggagtcgcatcttcaccagaaaaacctttgattttcacagcagtagggatatggctcagatcgacagccacaccgggagtcactggagcgatatcatacagagagagttctgaacctgaaggcagttgggtttttaacagtagtgcaagcgcctggccaataccgccagcagcgccgaggactgcgactttcatcctaaactccttattatattgataaactaagatatgttgctccgctgccgcgaccttaatccacaaaattgccgtttacaatgaccacatctcaagaatgtgtagtcacgcaagtttagcgtttatgcatttaattgccgtaatcaggaacctaacttacgtaattaacagtcgcttatgcattagcgcaacattccaacaggtggtgacaatataccctaccgttcagccaaaacaacatcaatttgataacaattaatttacttttaagcagaatttgcatgccgtgacgcaggcatgtttctcaataacgaaatttgataaaatcccgctctttcataacattatttcagccttcttcagggctgactgtttgcataaaaattcatctgtatgcacaataatgttgtatcaaccaccatatcgggtgacttatgcgaagctcggctaagcaagaagaactagttaaagcatttaaagcattacttaaagaagagaaatttagctcccagggcgaaatcgtcgccgcgttgcaggagcaaggctttgacaatattaatcagtctaaagtctcgcggatgttgaccaagtttggtgctgtacgtacacgcaatgccaaaatggaaatggtttactgcctgccagctgaactgggtgtaccaaccacctccagtccattgaagaatctggtgctggatatcgactacaacgatgcagttgtcgtgattcataccagccctggcgcggcgcagttaattgctcgcctgctggactcactgggcaaagcagaaggtattctgggcaccatcgctggcgatgacaccatctttaccacccctgctaacggtttcacagtcaaagacctgtacgaagcgattttagagctgttcgaccaggagctttaatctctgccccgtcgtttctgacggcggggaaaatgttgcttatccctctcaaccccctgctttcccctgcgattaatttaacgaatagtgcgttttactgcgacatgtcattcacacaatgaatacataaggtaaaaaaagcacattatgcaaaattcattatctaattgaaaaaactagaattaacgataaataaccgtatttttaattcttttttgttattaaaattcacatttttaacacttagtatcaactgaaacagttagcgcggtattaattagctcaataattagtgtatacttgattttgtgatatgggtcacgaaacaaaggcccagctaaaagattatgtcgaggtaaaaatcatgaaaatcaaaaccactgttgctgcattaagcgtactttctgttctctctttcggtgcattcgctgccgactccattgatgctgcacaagcacaaaatcgtgaagcaatcgggaccgtatccgtaagtggtgtggcgtcttcgccaatggatatgcgtgaaatgctgaacaaaaaagcggaagagaaaggcgcaacggcctaccagattactgaagctcgtagcggtgacacctggcacgctacggctgaactgtacaaataaaccctcatcgtcttgtccgacgatattgcccccggttcgggggcttttttttgcgctaatgacgaacattaaaacgcaaatgcccttccagctcttcctctgcctcatcaaacagcaatattaacgcgccaaaacggcgacgcgttttctctcccagatgaacaaattcaatctcaagtggtagcggcaggacatcgttcattaacacatcccatagtgagtcgagatcgcgtaccttatctttcgccagaccaaaggtttggctaaagtcacgataaaaatcctcctgactctcaatctcatcaaaatcaaaggtataaatattcatctgttgccaccgtcacgtttcgcggcgagttctgccgtgcatcgctaagtatagccatgaaaaaaccgacgcttttggcgtcggttttgacttaactatcggtcaacgcatgttgatacttatggagcatccccgccagccgatttaccggttccgtcacctgcggtggcgcttgccagatgcgtagcttttcctggtagatttccagttcttccagcaactggccaaagtaccgacgacgtttatcatcgctacgggcagatatcacatggtctgctgtgcggcgcatttgtcggtgaaacgccgataaatcctcgttaaccgggatcggtgcatcacgcaggcgctggtgcgcgataatcatcgtcagcgccaggcgaaatttcggcaaatcccctgggaacttattcatcagcaaaaacagctgctgataaagtgccgggaggtggttctctttacgacgtgccacattggtagtcatcgcggaaacagcggcagaaacaaactgattaagcagtacacgtccggtcctgtcgcgcgatttatcccgcaccagcaaaataacggtgaacgcgagcacacagccgacgatttgccctaatgcgctgtcgagaaactgactgaaatggaaagtcatcgggttatccagcacgataatatttatggtgctggccagtgcccccatcgagcccagtcgccgtttctgtacttctataccgaggaagaatcccagcactgccaggctaatgcacagcagcaacatgctctgttgggtattagggataatcaccaaaaagtagagcagccctaacggcagcgcggccagcgtcccgtagataaagtcgatcgccaccatgcgtggattcggcaaacgcattgccagtgacgtcactaccgcaatcatcaccattgcaccactgccggaagtccagcccgtccacagccagaaaagcgtgcccagaatgcaggaaagtgtggttcgccagaagttaaccattgcatgatgacgttcggctgactctacttttacttccggttcgccttgcaggatctcttcttcggtggcgttgatttttgtgttactgataacgccgcgcttgagaagctgataacgcgttgccgccgcgacccagctataaatggtgacaggcgtttcccgttccccggtccaggcgataactctccgcaggcgtttgagctgcttgtggacgtcctgcgcggtttctaccggcgtgtcaaaaaattcgcggaaagtatcagtgatcaattccgggcgcgtattctgaataagataagtttcgcaggattgggtaatcagcgtcagcgatagcgtattgatcgcttttaaacgtcgattggcccgcgcccagcgggaagattccatattcaggttgctgcgcatgccttgtagcgccgtggtgcgtcgcaccaggtcgccccaggctttatcgacaacttcaccatcgccatgcttgatacagagttgcattaattgatattgcgcgaccagcaaactttccagctctcgatccacttcttgtttgatcgatcgcggagaaaagagcaaatccgccataatcgcacacacaataccgataacgatctcgctacaacgttcgacggcaaactgcggcgtaagcaatggttccggctgaatggtgatcacaatgatcagcgcggtataaccggccagcccccacgcatacgagttttctattcgtaccagcgaggatatccaggtacaaaaaccggcccagatacagcacaccagaatcatcaataatggtgcgcggatcatcgcaatgatgatcaccagtccggcaatacagccaataaatgtgccgatgatgcgcaaaaagccacgatagcgaatagcgccagaatacggttcacctcccgcagcaaaggccgtaccggcggcaacaatcgccgctgtcagtaccgcccagcgtggcgtttccagctggaagtgaaagccaacaaacagcgccagtacaatggcggtcgccagttttaccgcaaagcgaatatgttggttagcaatggagaaaatacccatcgtgattaaccaaactcacgcaggcgatgggccattttacggaagaacgaatcctggctttcgtcgcgatcttgtttgccagtgaccaccactgtagcagtggtgcccgcaggccagatgttctcttgctggttgtcgagacgaatacgaaccggaacacgttgcgcaagacgcacccattcaaggttagagtctatagtcgccatccctttgtcgtcacgcgtgctgctggcgttggtgacccctgcggcaacactatcaacagtccctttcagcactttgttactgccaagcggcgtgatctctgcacgataccccggacgcaccccttccagcttagtttcttccatataggccagtacatagaaggagttctgtttcaccagcgcaaccgccgttgatcctcgagtaataaactcaccggtatagacgttgaggttggtcacccagccatctgctggcgcgcggatcaccgtgcgttcaagatccagttttgccagatcgcgggtcgcctgcgctttcgctaactgatgcagaaccgtttgtagtacgttgttggcctggtcgatctcttcgcgagacatcgcctgcacaccgagacggttacgacgtccggcctcctggcgtttctcctgtgccagtacctgataataagcaacatcggcttgcgcttcctcaagcgccttttgatagcgcggctggtcgatggtgaacagtatctgtccttttttcaccagctggttatcatgaacattcacctgggtaatgagtccagaaacgtccggcgcgatcgcaacgacgtcagcgctaaagcgcgcgtcacgcgtccagggggattcggtgtaatagacccaggcattaaaaattgcgatgaaggccagaatgactaatacgaccgtgatggccgtacgggagaattttcttattagtgttttcacttcaacctcaaacgaacagtcgcgatatcaaataaaacaagcagcaatagagcgcggtgttgaacaacgccggatgccagacaaagtcgtagatacctgttggcacaagtacccggcgcaccagccagaaaatcgccagtgataaaagcaattcaaaaaatatcggtgggaaggacagcccaaacaccacgataacgggaaacagactcatgttgaccttggttgtaaagagagagcaggcgttattattttcagcatctgtcgccgcagagaagggcatggaaagccgggcgagagcaacattgctgtagattgatatttaatatattagcgtaactgttatgctgttatctatattatgtgatctaaatcacttttaagtcagagtgaataatggaacgactaaaacgcatgtcggtgtttgccaaagtagttgaatttggctcttttaccgccgccgccagacagctacagatgagcgtttcgtccatcagtcagacggtatcaaaactggaagatgagttgcaggtaaagctgttaaaccgtagcacacgcagcattggcctgaccgaagccggtagaatttactaccagggctgccgtcgtatgcttcatgaagtgcaggatgttcatgagcaactgtatgccttcaataacacccccatcgggacgctacgcattggctgttcttcaactatggcacaaaatgttctcgccgggctgacagccaaaatgctgaaagaatacccaggtttgagcgtcaatctggttaccggaattccagcccccgacctgattgccgacggtctggatgtggtgatccgcgtcggcgcgttgcaggattccagcctgttttcccgccgtctgggcgcgatgccaatggtggtgtgcgccgcgaaaagctatctcacacaatacggcataccggaaaaacccgccgatttgagtagtcattcatggcttgaatacagcgtgcggcccgacaatgaatttgaactgatcgcaccggaagggatctcgactcgcctgatcccacaaggaagatttgtgactaatgatccgatgacgctggtgcgctggctgacggcgggtgccgggatcgcctacgtgccgctgatgtgggtgatcaacgagatcaatcgtggggagctggagatcctgctgccgcgttaccagtcagatccacgcccggtttatgcgttatataccgaaaaagataagctgccgctgaaggtacaggtcgtgatcaactcgctgacggattattttgttgaggtcggtaaattgtttcaggagatgcacgggcgcgggaaagagaagtaattcatattgtactgttacgttgtacaaacctgtgccaacgggttcccctcaccctaaccctcaccccaaaggggcgaggggaccgttcgtgcacgtagaaagattaattatccttctgaaaatagtgaaattattacgcagtaccgccaacagtcaggttatcgactttcaacgttggctggcccacgccaaccggcaaactttgcccttctttaccgcagacacccacgccgttatccagtttcaggtcgttgccaaccatcgaaatctgctgcatggtttcgataccggaaccaatcaacgttgcgcctttcaccggcttcgttactttaccgttttcaatcagatatgcttctgaagtggagaaaacgaatttgccggaggtgatatccacctgaccgccaccaaagttcggtgcatagataccgtactcaacggattcaataatttcctgcggggtcgatttacccggcagcatataggtgttggtcatacgcggcatgggcagatgggcgtaggattcacggcgaccgttgccagtcggcgtcatccccatcaaacgcgcgttgagtttatcctgcatgtagcctttcagaatgccgttctcaatcagcacgttgtactggcctggcgtaccttcgtcatcaatcgccaccgaacctcggcgatcgaccatcgtgccatcatcaaccacggtacacagttctgaagccaccagctccccgacctgtccactaaatactgaagtgccacggcggttgaagtcgccttccagaccgtgaccaaccgcttcatgcaacagcacgcccggccaacctgcgccaagtactaccggcatggtgcccgctggtgcagcaacggcagaaagattgaccagcgccatacgcactgcttcttttgcccatgcatccgcacggacttcgccgtcgagatcggcaaggaagaattcataaccaaaacgaccgccgccgccactggcaccgcgttcgcgtttgccatcttcttcgacgagaacgctcacggaaagacgcaccagcggacggacatccgccgctagcgtgccgtcggtggccgcaaccaaaattaattcatagacaccactgaggctggcagtcacttcctgtacgcgcttgtccgcttcgcgggcaaccttatcgacgcgacgcaggatatccagcttctcttcacggctcatgctttgcagcggatctaccgaggtatacaacgggctatgctctaccgcgcccagcgtctgtactttaccatcaccactatcacggacgatggtgcgcgccgcttgcgcactctgttccagcgccagcaggctgatttggtcagcgtaagcaaatccggttttttcaccgctgattgcacgcacaccaacgccctgatcgatgttgtaagaaccatctttaataatgcggtcttctaaaacccaggattcgtgatagctcgactgaaaatagagatcgccataatcaaggcgacgttcggccagttgaccgaggatcgcgaacaagtcctgatgtttcaggccgttcgccgctagcaattgttcacttaccaggttaagactcatcgtttttgctactcgttagttactgcagtagaggattttttacggctgccggatgcggcgtgaacgccctatccagcctacggttatgttccggtttgtaggcctgataagacgcacagcgtcgcatcaggcaacggctgtcggatgcggcgtaaacgccttatccgacctacggttatgttccgtttgtaggcctgataagacgcacagcgtcgcatcaggcaacggctgccggatgcggcgtaaacgccttatccgacctacggttatgttccgtttgtaggcctgataagacgcacagcgtcgcatcaggcaacggctgccggatgcggcgtgaacgccctatccgacctacggttatgttctggctcgttggcctttggcaacgattatcctatgagattggggcaattacgcgccctcgtcaaatcattgcgctttttctttacgcggttggcgcaacacttcgttgatttgcggatcgtccagcggacccgaaatgtgatagcgcaaaatggagactttgctccacagcggccccagcactttactggcggcaaacactgccgcgccaacaatggggttaaccgcaaaagccgcagccacgcccaccgtcgcagaaatctctggtgcgacaaccgcttccatattcaggtcgcgacgtaccagatttaccgaccctttcatggcgatatccgcctccaggccatccaccagcgtgtcgtcggtgtgcataacgccgtctttaatccacgcggtgctgcgaatggagtcaaaatagaacccttcgccaaaagtgtctctgaaatcaaaacgcagcttacgcatcagggcatctacgctcaataagcgcagcaattgcccggcatgtccggtattgatttcggtaatttcgcctttacccagttgagtatgaatgatgccattcaacgtcgcttcatctggctgccagggtgctttgcgccagtgtaaatcgtaatccacattaaatgacgactggcgtatgggcgtcgtgacaccaaaaaattctgcggcggcatcaattttctgcccgcgcagttttcctttcagcgaggtacgttcattccccggattattaacccattcaccatcggcagtaagccgcgagaaaccagtatcaatcagtccattggtcagcgttaacgtatcgccagaaatggtgatatcactgtcaatgcgaccgaatttttgcccccagaaccagcactctgtgcatcgtatttgggcgtccggccagccacggaagttaatgcgctccgttgtcgggaaaggtgatgacggcgttgaatcaccacgagttttcgccacgctcgggttgtaataaagatatttgatattcgccagccacggcgcgttattacgcatcgctagcgtggcgttgatttcacgcccttgcgcttcaaccagggtgccatttgccgtcggttgcgaaacaatactcaggttattccattgctgatttcccagtgacaacataggcgtacgtaacgttatgtgttgtgggaaactcgctgcaccaccgacactctccgcagcgcctttctggaacagggccagccactcggcaccattcatcggcggcatattgagttcaacgccactttgttccggcaacggcgggagcgttttactgtctgccgcccaaatagcacgatcgagcgtcagcttttgaccgagcaaccagcggctattgaaatgattatccgcaccagcctgtccggttaattcaaagctgttgagattgccatcaaccttaacgtttaccgctagtggttcacccgcaggtttggctaacggtgaaggtaagtgactgctcacattctttagatcgccgttcagctctatgttataggtcgcaccagcatgataaggcagatcaatgcccactttaccatcccacgccacgctgccactcaatgcttcgttcaccgcttcaggcagaacgccggttttcgccggttgccagttaccgttgaggtttaccgctacctggtaggcttttgccccttctttggtggaaaaatccacgttcaacggctgattaaaccagcttgctgtcagtggttcactttgcagatcgctattgataaagctgaatttaccgctcaaatttttcagggtgctgtcgagtggtttgataaacagactgttattacgcagcgtcacttcacctttcgcggttaccagttcgccgttcagcgggatatcaagatgtaagcgagcattcacatcgccgtcgagctggagttcttgcagggtcgcacccagagaatctttcagcggtgtctcatcaaagtaagggccaacggctttacccggacctttaatgtcagcgtcaatcagcagtttttcttttgagtagtcagggatcactgcggtaagattactcgcgcgcacgccgcccagattaacgccatcggttttcatccataaaccgtcgttaataaagtccagttcaatatcaaggttagttaatgcaggccagtccggctggaaggcaaacttcgcgttgcgcagcggcaccagcacttcaaactgaccttcgttgtgtttataggggaagagttgcggattgccaccataaaccagcgtcgcgttatccgcttcaccgccctgaatcgcgccacttaagtaatcaaccaggtctttacccatcaagttttccgggaaatagcgccaggcttgtgaaccatcatcggtactgatgccagccagaatacccagccagggttcatcgttagcaggttgcaggtaacgaaaaccgccgcgcgcatggacggctttggctttaacgtcaatattacgcccatccagctggaaacctttgttattgttcagccagcttatagttgcctggccgtcggcgatttctagtggcgcacggaataccgtttcgtaaggcatctttgcctgcttcatcgacgcggtaagcaaaccattttcaacgctgccggaaagcgtcccggagaagtgttccgcacccggtaataatttccattgcttccaggccagatcgctccacgatgcctgaaaacgggtcttgtctgccgcctgaagcgggatatccagcgccagagtgttaatcttgccgctcggttgtgtggagcgccaaacatcacccagtgcaggtgaaagtttcgcggccagcgggcgtatgccctccaggcctgccagctccagattactggcgcgaatccggagttcgtcactgcgtttattgtctttgccgccaacgtcctgttccggtatccaggccagcgtcaatgctccgctcggccagggtttgccgtccatcgtgatccgtgtatcgggaatagagaactgccagcccggattttcacgcgtaatatgcgcggtcagattatccaccgacagcgtatgcgtttgcttctcgcccaaccagctggcaccgccctgtttcagccagacgtcaccgccggttacatcgcctttgtcgatcgtcatccagccttcaagggagaactgtgccgtttccagcgcaatattgtcctgcatccatttaccgagccacggcttcaggtcgatgtcatccgcctggagccagacgcgaccattgcttaacaacccctcatcatcgcgcaaatccatgcgcacctgcatcacgccgtgctgtccggtaaggctggagaggcttaccaggccttccgcacggtgtcgacgtggatcgttcagccaggtgagttgtgggatcgccagctcggcgcgctgaccggatggcgtcaggaaactgacttcactgtcgcgaagatcgaaatggtcaaattgacgaagaaacagatcgctgatgtgactggcttccagactgtcatcactaccaccgctggtgataggagtgttggtgcgaaagcgcagctgccagaaagtgaggtcgcgaaactgccagcgcatatgtaacaggctctgccagacatccagcgccagagtaacgcgtttaaccgaaaattcgccgccatcttttagttctgcacggatgtcgtgtgcttcaagcgtcgggccaaaattctgccagctggctgagagctgactggcttctaccggcatgccagtcgcggattctattttgttgaggatttccggacgccaggcgtcaagatgcggtaaagcaatacgcaggccgctaaccagcagggcagcgatcacaacgagcgcggctccagtaagcagtaaaatccccggcaatcgcctcacccgtcactccttgtctgctaaaaatgtgactcaaaaaccctttgccggatggcggcccagcatctgtttacatcattacgacgtcaaactgctcctggttatagagcggttcaatttgtactttaacctgtttgccaacgaaaatttccacttccgccagcgagtgtgactcttcgcctttcaaggcttcagctactgccggagaagcatagaccaggaaacggtcggagtcgtaagcatggtggacacgaacaatctcgcgcatgatttcatagcataccgtttccacggttttcaccgttccgcgaccgtggcaggttgggcattcgttacacagtacgtgctcaatgctttcgcgggtgcgtttacgcgtcatctccaccagccccagcgccgaaaaaccattaacgctggttttcacccggtctttgctcaacgcctgctccagcgagtgcagcactcggcggcggtgatcttcattattcatatcgatgaaatcaataatgataatcccgcccagattacgcaaccgtaactggcgagcgatagcctgcgtcgcttcaatattggtattgaaaatggtgtcgtccagattgcgatgaccgacaaacgctccggtattgatgtccacggtggtcatcgcttcggtctggtcgataatgagataaccaccggatttcagttctactttgcgttccagcgctcgctggatttcgttttcgacatcaaagagatcgaaaatcggctggcgtcctgtgtaatgctccagcttgcttgtcatctcgggaatgtactccgaggtgaactcaagtaacgcttcgtaagtcaggcgtgagtcaacgcgaatgcggtccagttcggcatcggcgaaatcacgcagaacacgctgcgccagcgccagttcgccgtacagctgataacgggtctgcgggcgttttttacgctccataactttggtccagacgcgtttcagataagcggcatcggaggccagttcagcctcgccaaccccttccgctgcggtacggatgataaacccgccctgctcgtcgcaatactctgcgaccacttttttcaggcgttcacgttctgattcgctttcaatacgttgggaaaccccaacgtgagaagcccctggcataaacaccagatagcgagaagggagcgtgatatcggtggtcaggcgcgcacctttagtgccaagcggatctttcaccacctgcaccatcagatcttgcccctgacgaaccagttccgagatgtcgcgcaccgtgaattgcttttgttcttcacccgccacacattcggtgtgcggcatgatgtcggatgcatgaagaaacgcggctttatccagcccaatatctacaaaagccgcctgcatacccggaagtacacgacttacacgacccttgtagatattgcctactattccgcgtcgcgcctcacgttcaatatgaatttcctgcagaataccgccatcaatatacgccactcgcgtttccgaaggcgttacgtttactaacaattcagccgtcatgtttatcccttttctcacgcagtgcgttaaaattacttaataattcatacgtttcaaccagcggtaagccgactacggcgtgatagctgccatttatcttcctgacaaaacagccacccagcccctgaataccgtatgcacctgctttatctaacggttcatcgctggcgacatagcccgcgatgtcttcgtctgttaacgttctgaaagtcacatcggtgaccaccaggcaatcgagaatgtgctggctgtcggccaacgccactgctgtcatcacctgatgggtctgacccgataatttgcgcaacatctgcgccgcatgctctgcgtcgcgcggtttctccagcacttctccgttcaggataacgatagtatccgcacccagcaccgggagatccttcgccgtttgcgcgacacctgcccgtgctttctcgcgcgccagacgcacaacatactgctgcgcgctctcctgcggctgacgctgctcctcaatgcccgtaacaatacgttcaaaggtcacgccaagttgcgcaagtaactcctgacgacgcggagaaccggaagctaaatacagagaagtcatagaaacctttattgcactgcaaactgctgacggactttgcgcatcagcaagaaaatccacggccagagcaccccattgactacactactccagaacacttccggtctgaaagagacgttaatcactaaaaactctgcccagaaaacaataatatccaccaccagcgaaagcaacatgacgaccagcgcctgctgccataatgcgaggttgcggaaaagctggtatttcagcgccaccaggtaagcaatgatgctcatcgccaatacgcgtacgccaagcgtcgagccgctgatcagatccagtatggcacccatcacaaaacctgtgcccacatttacgcgatgaggcaaggccaggatccaatacaacaagatgagtaacacccagtttggccggaaaacaatcaggttatccggccagggcatgatttgcagcaacagcgcaatgaggaaagagagccagattacccagcgtccctggctacgatagctcgccactattgccctcccggcgcacgcgcaggcggttgagcaccactttgcggcggcgtagccctttgtggagagcgattagcagcaggctgtgtcggcgcagcaggcgcagtagctgcatttcctgtcgccggttgctgcggagtcggctgagcgatccccgttgccggttcaggtaactttggccccatcgcgtctggcgaaggcaatacctgcggcatcatctgcatcagacgttcattagcaacacgatgcacctcttccggcgtcatcgggttagcgccgttacgatctgccccccacagcagcagcagataacgcaaacgttgcagccctgcagtcggacgcgcctgaatcacagtataagcgcgctgggtatcgagttttacggaagagacaaccgcgaccggatagccttccgggaaacgaccgcccagaccggaagtcaccagcacatcaccaacacgaatatccgtattcgccggcagatgctcaagctgcaaatcatccgtacaaccgttaccggctgcaattacgcggatatcgttgcgcagcacctggattggcagcgcgtgggtcgcatcacaaatcagcagcacgcgactggtcagtttagcgacggccaccacctgaccaacaacacctttgtcgctgatgaccggctggccttcataaacgccattaacgctacctttatcgataacaacttgatcgctataaggatcgttaaccgtggagataacctgagtcaccattttctgctcatcctgacgcagcggggaacccagcagctcgcgcagacgcgcgttctcctgtttgtattgtccaagcatcagcagttcactgtttttcagcaacagttcctgacgtaacgcccggttttcaagttctaattggtcacgcgaggccagcgtctgcgatacgccatccagcaattcacgaggagcattggaaacaaagtagaaaggactgacggcggtatccatataagtacggatttgactgaacgtccccaggcggctgtcggcaataataatgccgagcgccaccagcaccgccagaataaggcgaatctgtagcgacgggccacggctaaaaattggcttcataagttatgcgtattctcgtatcagaccaggcagggtaaacagacacttcccctgcctgcatccgattactcttcgctgaacaggtcgccgccgtgcatgtcgatcatttccagcgctttgccgccaccgcgcgccacacaggtcagcgggtcttcagcaacaacgactggaatgccggtttcttccattaacaaacggtcaaggttacgcagcagtgcgccaccaccggtgagcaccatgccgcgctcggagatgtcggaagccagttccggcgggcactgttccagtgcaaccattaccgcgctcacaataccggtcagcggttcctgcagtgcttcgaggatttcattggagttcagggtaaaaccgcgtggaacaccttctgccaggttacggccacgaacttcgatttcacggacttcatcgcccggataagccgaaccgatttcgtgcttgatacgttctgcggtggcttcaccgatcagagaaccgtaattacgacgcacatagttgatgatagcttcgtcgaaacggtcaccaccaatgcgcacagaagaggagtaaaccacaccgttcaaggagataacagcaacttcagtggtaccaccaccgatatcaaccaccatagaaccggtcgcttcagaaaccggcaggccagcaccaattgcggcagccatcggttcttcaatcaggaagacttcacgggcaccagcgccctgcgcggattcacgaattgcgcggcgttcaacctgggtcgcgccaaccggcacacaaaccagaacgcgcgggcttggacgcataaagctgttgctgtgcacttgtttgatgaagtgctggagcattttttcagtcacgaagaagtcggcgataacgccgtctttcattgggcgaatggcagcaatattgcccggcgtacggcccagcatctgcttcgcgtcatgacctactgcagctacgcttttcggtgaaccggcacgatcctgacgaatggccaccacggaaggctcattcaatacgatgccttgtccttttacataaatgagggtattcgcagtacccaggtcaatggacaagtcattggaaaacatgccacgaaattttttcaacatactaagggataatcctgaaagctggggcggaaaagaaaatccgcttactttaccaaccacacgcagcagcgacaaggcgcaaaaatcatctgctacggtgaaaattagtgcagttcgtttcctttgttacaaatctctgcctgagtccagaaaggcttaatgcatcagcagcattcctcgcctgtttgcaaccgcgtaaggtcattcatctgcatatgtgctgcaacaatctggcgagcagacaagcacactcccatgagacgcagcgcgcattattctacgtgaaaacggattaaacggcaggttaaaccgagtatctttgtgaatattttttcacgttagtatcaagtggctgtgaggacgcgaaaaaatccccttgcccgcctgtaacaccgcgctgaatcagggtctgccactcgcttcgcgaacgcacgccggtggcgtaaacctgggtgctggtcccggagcaggcttccaccaggctttgaaccagcagctggttctccgttcgcttctcaatgtttctgaccagccccggatggagcttgagtaactcaacattaagttctttgatccaactggtacttaccagcgtcaaaccagcctggttgacggctacccgtacccctaaagcattcactaaacgaataacaggttgtaaacgactgatatgttgacctacatcggcctctgcaagttcaataattatgcgttttcgttgtgatttttcacattgcattaacgtatcgcgcagccaacgctgaaaacgcgggcgaatcagcgactcaacggtaacctgaatcgccagattttcctctggccagtaacgcaatagtggaataagacggctgatttgcagacggtcatactcttccgataagccaaactgcaagaccatcggcatatactccgccgagctaacctcttcattaccatcgaagatgcggcacatgagttcgcgatgatgaacctgaccttcgcgagtaaccgccggtttttgataaaggcgcgggccgccgcgactgagcatttgctcgataagcgtacgccagcgaacattaccgcgtcctttttcaggcaacgagtcatcgtaaatagcccagctattgccgccctgcaatcccgcattacgcgtggcagactctgcatgttccattacctgctcggtatcctgaccactacgccaggcgcagataccaatgtggatcatatcgtcgcgatcgagcattttattgttcggcaaggtatcaacggctttgattaactgaccggcgatgctctctgcctcttttaacgtccggtgcggtaacagcgcagcaaaatcactgcggtggtaacgcgccagcagtgcgccagggtagcgcatcataaatgtcgacagcagattcgtcagagtgaagaactgttcttcaacctggctgtgcccccaggtatcgctcaacatattgaaatccggcagacgaatcatcatcacgatcccgtgggtacctactttctcctgatcttccagtaacgttgctaactgattatcgaaaaagagtcggttattgaggccggttttcacgtcctgggcggcataagagcggatcagcgtatcaagacggctgtgttgttcgcgtgcgttctgaatttcacgaagcagcgtatccagcgcactgctggttctgggcggccattcatagatggttcccaacacattagagccacgctcaccgtttaagatacgagtagcccgggtttccagcaattcttgcccggcaagttgccgttgtaaccagcgtaccgccaggaagagcataacaatgataaagccaatcgcccccgtgagcggcgcggtggtcatcaacgaatggaaatagttgcccatcggatcctgataaaccagacgcaacgacatccccggatgctttatcaacggaacgctcagttcgcgaaacagatcgctggagccaactggacgataactaccatttctggccagggtataaacctgtttatcaccatggagcaggtctacacgaacgatatctgccgacatcattaattcggtaatttgtggccttaatacgctgaagtcattcgacacaaggtgggtatcaatcgccgtcgccaccgcctgaacgcgatgactaaacttatactgaatggcgttgtagaaacttagcgaacagcccagcaaagtcacaaaaattgttaacccggtgagcagcgtaacaaaggccgaaaatttcgtcgttaatctcatccttgtgttaactccgatagtgaggaagcgggcatactagcaaatcagatttatctcgcaatttattgcgcttcatcggctttgcttttccattagcgagtatagtcttcagaaattattttccaatccatcatgcacatgaggaccacttatgcaggcgttacttttagaacagcaggacggcaaaactctcgcatcagtacagactctggacgaaagtcgcctgccggagggcgatgtcacggtcgatgttcactggtcgagcctgaactataaagatgcgctggcgattaccggtaagggaaaaatcatccgtaattttccgatgattcctgggatcgattttgccggaactgtacgcaccagcgaagatccgcgttttcatgccggtcaggaggtgttactcactggctggggcgttggtgaaaaccactggggtgggctggcggagcaggcgcgagtgaaaggtgactggctggttgccatgccgcaagggctggacgcgcgtaaagcaatgattatcggtactgccggttttaccgccatgctgtgtgtgatggcgctggaagatgccggtgttcgcccgcaggacggggagattgtcgtgacgggtgccagtggtggcgtcggcagtaccgccgtggcgctgctgcataagttgggttatcaggtcgttgccgtttccggtcgcgaaagtacccatgaatatctgaaaagtttaggtgctagccgtgttctccctcgtgatgagtttgccgaatcccgtcctctggaaaaacaagtctgggctggggcaattgacaccgttggcgacaaagtgctggcaaaagtgctggcgcaaatgaattacggcggctgcgtggcggcctgtggtctggcgggtggttttactctgccaaccacggtcatgccatttattctgcgtaatgtccgtttgcaaggggtggattcagtaatgacgccaccagaacgccgcgcacaagcctggcagcgactggtcgccgatttaccggaatcattctatacccaggcggcaaaagagatatctctgtcagaggcaccgaactttgccgaggccatcattaataaccagatccagggtcgcacgctggtgaaggttaactaaccatttagcagggaataataagagagggaactcattttgaaatcattattcaatcggttaacgggaaaagcggttagccggacagctttcgtcgaacaccttggtcaggaagttatacaacatcatccaaactggaaagtcatgatttcgactgaccacaaattgatgcgcattgatactccactaaacagctattattgatacgcctccgtcgcctgttaggtttatgttgctttgcctgggcgacgctacgcttagccccttacttatttctggtaccatggggtgaataatctgattttgtttgactacaaattaatcactcgaacctatttaatgctgagcattgtcaatcggttaattttgcgtgctttagcattcacatctatccagacgatgcagtgaaaattgggtaatccccagcaaccgctgcgtaatgtcgtctatcttgtcgcgatcctggcatccctacattatttgtggtctgtgaagattatctcattgcagcccctcatcttcgcagggctggcttttcagcttttcaccttacgttataagaagttccgtcgatgatggcgctaatttcgtgaattgtgcggcttgttgcaaattacacggtgttgaaggttatttacatgttagctgttgattatcttccctgataagaccagtatttagctgccaattgctacgaaatcgttataatgtgcgacctcgtcctccctgacgcagtttttgcgctgcggaaaaggtgacattggcgcaacgaaggtatattttgttttttgccggaggatagcagcagatcgctgcacaatgtccgtcaagtctaacattgacactctggggcaaaatagaccggcgtcccggcctgctggaatttatcgctatgcatacagctgtcggggcatacgctttacagacggcggtgaaacgcctgtcacaatcacactaaacaaagagtacggaacccactcatggatattcgtaagattaaaaaactgatcgagctggttgaagaatcaggcatctccgaactggaaatttctgaaggcgaagagtcagtacgcattagccgtgcagctcctgccgcaagtttccctgtgatgcaacaagcttacgctgcaccaatgatgcagcagccagctcaatctaacgcagccgctccggcgaccgttccttccatggaagcgccagcagcagcggaaatcagtggtcacatcgtacgttccccgatggttggtactttctaccgcaccccaagcccggacgcaaaagcgttcatcgaagtgggtcagaaagtcaacgtgggcgataccctgtgcatcgttgaagccatgaaaatgatgaaccagatcgaagcggacaaatccggtaccgtgaaagcaattctggtcgaaagtggacaaccggtagaatttgacgagccgctggtcgtcatcgagtaacgaggcgaacatgctggataaaattgttattgccaaccgcggcgagattgcattgcgtattcttcgtgcctgtaaagaactgggcatcaagactgtcgctgtgcactccagcgcggatcgcgatctaaaacacgtattactggcagatgaaacggtctgtattggccctgctccgtcagtaaaaagttatctgaacatcccggcaatcatcagcgccgctgaaatcaccggcgcagtagcaatccatccgggttacggcttcctctccgagaacgccaactttgccgagcaggttgaacgctccggctttatcttcattggcccgaaagcagaaaccattcgcctgatgggcgacaaagtatccgcaatcgcggcgatgaaaaaagcgggcgtcccttgcgtaccgggttctgacggcccgctgggcgacgatatggataaaaaccgtgccattgctaaacgcattggttatccggtgattatcaaagcctccggcggcggcggcggtcgcggtatgcgcgtagtgcgcggcgacgctgaactggcacaatccatctccatgacccgtgcggaagcgaaagctgctttcagcaacgatatggtttacatggagaaatacctggaaaatcctcgccacgtcgagattcaggtactggctgacggtcagggcaacgctatctatctggcggaacgtgactgctccatgcaacgccgccaccagaaagtggtcgaagaagcgccagcaccgggcattaccccggaactgcgtcgctacatcggcgaacgttgcgctaaagcgtgtgttgatatcggctatcgcggtgcaggtactttcgagttcctgttcgaaaacggcgagttctatttcatcgaaatgaacacccgtattcaggtagaacacccggttacagaaatgatcaccggcgttgacctgatcaaagaacagctgcgtatcgctgccggtcaaccgctgtcgatcaagcaagaagaagttcacgttcgcggccatgcggtggaatgtcgtatcaacgccgaagatccgaacaccttcctgccaagtccgggcaaaatcacccgtttccacgcacctggcggttttggcgtacgttgggagtctcatatctacgcgggctacaccgtaccgccgtactatgactcaatgatcggtaagctgatttgctacggtgaaaaccgtgacgtggcgattgcccgcatgaagaatgcgctgcaggagctgatcatcgacggtatcaaaaccaacgttgatctgcagatccgcatcatgaatgacgagaacttccagcatggtggcactaacatccactatctggagaaaaaactcggtcttcaggaaaaataagactgctaaagcgtcaaaaggccggattttccggccttttttattactggggatcgacaacccccataaggtacaatccccgctttcttcacccatcagggacaaaaaatggacactcgttttgttcaggcccataaagaggcgcgctgggcgctggggctgacccttttgtatctggcagtttggttagtagccgcttacttatctggcgttgcccccggttttaccggctttccgcgctggtttgagatggcctgcatcctgacgccgctgctgtttattggactgtgctgggcgatggtgaaatttatctatcgcgatatcccactggaggatgacgatgcagcttgaagtaattctaccgctggtcgcctatctggtggtggtgttcggtatctcggtttatgcgatgcgtaaacggagcaccggcaccttccttaatgagtatttcctcggcagccgctctatgggcggtattgtgctggcgatgacgctcaccgcgacctatatcagtgccagttcgtttatcggcgggccaggagctgcttataaatacgggctgggctgggtattgctggcgatgattcagcttcctgcagtctggctttcactcggtattctcggcaagaagtttgcgattcttgcgcgccgctacaatgcagtgacgctgaacgatatgctgtttgcccgctaccagagtcgtcttctggtgtggctggcgagtttgagtttgctggttgcgttcgttggtgcgatgaccgtgcagtttatcggcggtgcgcgcctgctggaaaccgcggcgggtattccttatgaaaccgggctgctgatttttggtatcagcattgcgttatataccgcctttggtggctttcgcgccagcgtgctgaacgacaccatgcaagggcttgtgatgctgattggcaccgttgtgctgcttattggcgtagtacatgccgctggcggcttaagtaacgcagtacagaccttgcaaaccatcgatccgcaactggttacgccacaaggcgctgacgatattctgtcgcctgcctttatgacgtcgttctgggtactggtgtgttttggcgtgattggcctgccgcatactgcggtgcgctgtatctcttataaagacagcaaagccgtacatcgggggatcatcatcggtacgattgtggtcgcaattctgatgttcggtatgcacctggccggagcgttaggtcgggcggtgatccccgatctcaccgtaccggacctggtgatcccaacgttaatggtaaaagtgctgccaccgtttgctgccgggatcttcctggctgcaccgatggctgcgatcatgtcgacaattaacgcccaactgctgcaaagttccgctacgatcattaaagatctctatctgaatatccgtccggatcaaatgcaaaacgagacgcgtctgaagcggatgtcggcggtaattacgttagttctcggcgcgttgctgctgcttgccgcctggaagccgccagaaatgatcatctggctgaatttgttggccttcggtgggctggaagccgttttcctgtggccgctggtgctgggtctttactgggaacgcgccaacgccaaaggcgcgctaagtgcgatgatcgttggcggcgtgctgtatgccgtactcgcgacgctgaatattcagtacctgggcttccaccctatcgtgccctcgttactactaagtttgctggctttcctggtcggaaaccgtttcggtacatccgtcccgcaagctaccgttttgactactgataaataaagagttttgccatgccttggatccaactgaaactgaacaccaccggcgcgaacgcggaagatcttagcgatgcgctgatggaagcgggtgccgtttctatcacttttcaggatacccacgatacgccagtatttgaaccgctgccgggcgaaacgcgcctgtggggcgacaccgatgtgattggtctgttcgacgctgaaaccgatatgaacgacgtggtggcgattctggaaaaccatccgctgctcggcgcaggcttcgcgcataaaatcgaacaactagaagataaagactgggagcgcgaatggatggataatttccacccgatgcgctttggtgaacgactgtggatctgccctagctggcgtgatgtgccggacgaaaacgccgtcaacgtgatgttagatccagggctggcgtttggtacgggtacccatccaaccacctctctgtgcctgcaatggctcgacagcctcgatttaaccggtaaaacagtcatcgactttggctgtggttccggcattctggcgatcgcggcgctgaaactgggtgcagcaaaagccattggtattgatatcgatccgcaggcgattcaggccagccgcgataacgccgaacgtaatggcgtttctgaccgtctggaactctacttaccgaaagatcagccagaagaaatgaaagccgacgtggtggtcgctaacatccttgcaggcccattacgtgaactggcaccgttaatcagcgtcctgccggtttcaggcggtttgctgggcctttccggtattctggcaagccaggcagagagcgtttgtgaagcttatgccgatagcttcgcactggacccggtcgtggaaaaagaagagtggtgccgtattaccggtcgtaagaattaaccttcgcatcgccgtagggtgacgcggggcgaagtgcgagcaagctcacaaaaggcacgtaaatttgccgattatttacgcaaatttgcgtgccaaaattttcattcataaagaaaaattgagaacttactcaaatttctttgagtgtaaattttagtcactattttctaatatgatgatttttatgagtaattatcgcaccacgctcattttaaatgcaattctttgatccatctcagaggattggtcaaagtttggcctttcatctcgtgcaaaaaatgcgtaatatacgccgccttgcagtcacagtatggtcatttcttaactcatgcgcatcggacaatatcagctcagaaatcgcctgatcgcagcgcccatggctggcattacagacagaccttttcggacgttgtgctacgagatgggagccggattgacagtatccgagatgatgtcttctaacccacaggtttgggaaagcgacaaatctcgtttacggatggtgcacattgatgaacccggtattcgcaccgtgcaaattgctggtagcgatccgaaagaaatggcagatgcagcacgtattaacgtggaaagcggtgcccagattattgatatcaatatgggttgcccggctaaaaaagtgaatcgcaagctcgcaggttcagccctcttgcagtacccggatgtcgttaaatcgatccttaccgaggtcgtcaatgcagtggacgttcctgttaccctgaagattcgcaccggctgggcaccggaacaccgtaactgcgaagagattgcccaactggctgaagactgtggcattcaggctctgaccattcatggccgtacacgcgcctgtttgttcaatggagaagctgagtacgacagtattcgggcagttaagcagaaagtttccattccggttatcgcgaatggcgacattactgacccgcttaaagccagagctgtgctcgactatacaggggcggatgccctgatgataggccgcgcagctcagggaagaccctggatctttcgggaaatccagcattatctggacactggggagttgctgcccccgctgcctttggcagaggttaagcgcttgctttgcgcgcacgttcgggaactgcatgacttttatggtccggcaaaagggtaccgaattgcacgtaaacacgtttcctggtatctccaggaacacgctccaaatgaccagtttcggcgcacattcaacgccattgaggatgccagcgaacagctggaggcgttggaggcatacttcgaaaattttgcgtaaacagaaataaagagctgacagaactatgttcgaacaacgcgtaaattctgacgtactgaccgtttctaccgttaactctcaggatcaggtaacccaaaaacccctgcgtgactcggttaaacaggcactgaagaactattttgctcaactgaatggtcaggatgtgaatgacctctatgagctggtactggctgaagtagaacagcccctgttggacatggtgatgcaatacacccgtggtaaccagacccgtgctgcgctgatgatgggcatcaaccgtggtacgctgcgtaaaaaattgaaaaaatacggcatgaactaattcaggttagctaaatgcttgattaaaaaggcgctactcggcatggggaagcgccttttttataggtgtcacaaagggagtgaccatgagaacaggatgtgaaccgacccggtttggtaatgaagctaagaccattattcacggtgatgcgcttgccgaacttaaaaagatccccgccgaaagtgtcgatctgatctttgccgacccaccatataacatcggtaaaaattttgatggtctgatcgaagcctggaaagaagatctgtttatcgactggctgtttgaagtgattgcagagtgccaccgcgttctgaaaaagcagggcagcatgtacatcatgaacagtacggaaaacatgccctttatcgatctccagtgccgcaagctttttaccatcaaaagtcgcatcgtctggtcatatgacagttctggagtgcaggcgaaaaaacactacggctccatgtacgaacccatcctgatgatggtgaaagacgcaaagaactacacattcaacggtgatgctattctggtagaagccaaaaccggatcgcagcgcgcgttgatcgattatcgcaaaaatcctccacagccttacaatcatcaaaaagtaccgggtaacgtttgggattttccgcgcgtgcgttatttgatggatgaatatgaaaaccacccgacgcaaaaaccggaagccttactgaaacgcattattctcgcctcttccaacccaggcgatatcgttctcgacccgtttgctggtagctttactaccggtgccgtagccatcgccagcggacgaaaattcattggtattgagatcaacagcgagtacatcaaaatggggcttcgacggctggatgtcgcgtcgcattactctgcggaagaactggcgaaagtgaaaaaaagaaagaccggcaacctgtcaaaacgaagccggttaagcgaagttgaccccgatctcattacaaagtaaaggatgtgtaagcctggttttcagattattcatttcgtgtatatttcctgccagacttggttaaacatgcacaggctcaggtaatgattcgcaagtattggtggctcgtcgttttcgctgtcttcgtttttctgtttgatactttactgatgcagtggattgaactgctggcaacagaaacagacaaatgccgcaatatgaactcagttaatccactaaaactggttaactgtgacgaactgaattttcaggacagaatgtgaatttacatgacacttaattcattcgtttgatgaattaatttcgttatgttttcatctggcatgaacattcttaatacgttatcgaccagagcgggggcttgtttataaagatcataacccgccatattcattaaccagttttgaacaattccgctgaaggcaccatcaataataatcatcacaacatctaaatcgaggttatttgctacacaaccttgttgctgacacgcctgcaatacttcgcggagagtctgcggattaaagcccatcttttcgcgtatcactccctcggccagcatctcatcattaaattcacatttgtgatataagattttcagcaacgcctgctggcggggaattttggcaatatattgcaagccgacaatcaatttttcacgcaattgttgaaacgggtcatgctctaatccagccgtcaagtgttcctggattaactcccgcaatgaaggctgttgcaaccacatctcattaaacagttgagtcttgttttcgaagtgccagtagatagcgccacgcgtaacgttagcggcgtcggcaatgtcgttgagcgtcgtcttgcttacgccatgctgcgcaaactgggcgatggcagtttcaatcagttcttgccgggtcttcagagcttcggctttggttctttttgccatgattaattattcaggaaataaatatattcgacacagagtgagaaaatagcgaaggttaatctatcacctaatgtgtatttatacgagaggctaatattgagttgctataaatcgttaaataaataatatatattatttacctaagatacattcactacatcaatatatatttcaatttacgaggttttaattctgcctctttcaacccgcgtcaaaataaaacagtagaatattaatctttttttgtgtttatgtgccttgagatgcctgtattcataactattccttacatcgacgaatgataatttgtaggatagcgaactgtatttttctttctgcgagttaacgcgttgcctttttgggtaaataacgcgcttttggttttttgaggaatagtaatgacgaaacatgccaggtttttcctcctgccctcctttattctgatctccgcggctttaatcgccggttgtaacgataagggagaagagaaagctcacgtcggtgaaccgcaggttaccgttcatattgtaaaaacggccccgttagaagttaagactgaattaccaggccgcaccaatgcttatcgtatagccgaagttcgcccacaggttagcgggatcgtactgaatcgcaatttcactgaaggcagcgatgtgcaagcaggccagtccctgtaccagatcgatcccgcgacctatcaggcaaattatgacagcgcgaaaggcgaactggcgaaaagtgaagccgccgccgccatcgcgcatttgacggtaaaacgttacgttccgctcgtgggtacgaaatacatcagccagcaggagtacgaccaggccattgctgatgctcgtcaggccgatgccgccgtgattgccgcaaaagccacagtcgaaagcgctcgcatcaatcttgcttataccaaagtcactgcgccaattagcggacgtatcggcaaatcgactgtgaccgaaggcgctcttgtcactaatgggcaaacgactgaactggcgactgtccagcagctcgatcctatctacgttgatgtgacccaatccagcaacgattttatgaggctgaagcaatccgtagagcaaggaaatttgcataaggaaaacgccaccagcaacgtagagttggtcatggaaaacggtcaaacctatcccctgaaaggtacgctgcaattctccgatgtgaccgttgatgaaagcaccggctccataaccctacgtgctgtcttccctaacccgcaacatacgcttttgccgggtatgtttgtgcgtgcacggattgatgaaggcgtccaacctgacgccattcttatcccgcaacaaggcgttagccgcacaccgcgtggtgatgcaaccgtgctgattgttaacgataaaagtcaggttgaagcgcgccctgtcgttgccagtcaggcgattggcgataaatggttgattagtgaaggactgaaatctggcgatcaagtcattgtcagcggcctgcaaaaagcgcgtccgggagagcaggttaaagccactaccgatacccccgcagatactgcatcgaagtaaggtaatctgacatggcaaacttttttattcgacgaccgatatttgcatgggtgctggccattattctgatgatggcgggcgcactggcgatcctacaattgcccgtcgctcagtatccaacaattgcaccgcctgcggtttctgtttcagcaaactatccgggcgctgatgcgcagaccgtgcaggatacggtgacgcaggttatcgaacagaatatgaacggtatcgataacctgatgtatatgtcctccaccagcgattccgccggtagcgtgacaattacccttaccttccagtccgggaccgatcctgatatcgcgcaagtgcaggtgcagaacaaactccagctcgccacgccgttgctgccgcaggaggttcagcagcaggggatcagtgttgaaaagtccagtagcagctatttgatggtggcgggctttgtctctgataacccaggcaccacacaggacgatatctcggactatgtggcctctaacgttaaagatacgcttagccgtctgaatggcgtcggtgacgtacagcttttcggcgcacagtatgcgatgcgtatctggctggatgccgatctgctaaacaaatataaactgacaccggttgatgtgattaaccagttgaaggtacagaacgatcagatcgctgccggacagttgggcggaacgccagcgttaccagggcaacaattgaacgcctcgattattgctcagacgcggtttaaaaatccggaagaattcggcaaagtgaccctgcgcgtaaacagtgacggctcggtggtacgcctgaaagatgtcgcacgggttgaacttggcggtgaaaactataacgttatcgctcgtatcaacggaaaaccggcggcgggcctggggattaagctggcaaccggcgcgaatgctctcgataccgcgaaagccattaaggcaaaactggcggaattacagccattcttcccgcagggaatgaaggttctctacccttatgacaccacgccattcgtccagctttctattcacgaagtggtaaaaacgctgttcgaagccattatgctggtgttcctggtgatgtatctgttcttgcagaatatgcgagcaacgctgatccccaccattgcggtacccgtggtgttgttagggacgtttgccatcctcgccgcttttggttactccatcaacacactaacgatgttcgggatggtgcttgccatcgggctgctcgtcgatgatgcgatagtggtggtggagaacgtcgagcgcgtgatgatggaggataagctcccgccaaaagaagcgacggaaaaatcgatgtcgcaaattcagggcgcactggtgggtatcgcgatggtgctgtcagcggtatttattccgatggcattcttcggcggttctactggggcaatttatcgccagttctctatcaccatcgtttcggcaatggcgctttctgttctggtggcattgattcttacccctgcgttatgtgcaacgctgcttaaacccgtctctgctgagcatcacgaaaataagggcggtttcttcggttggtttaataccaccttcgatcatagcgttaaccactacaccaacagcgtcggcaaaatcctcggatccacaggacgatatttactgatctatgcgctgattgttgcaggaatggtggtgttgtttttacgtcttccgtcttccttcttacctgaagaggatcagggtgtctttctgaccatgattcagttacccgctggcgcgacgcaagagcggacgcaaaaagtgttggatcaagttacggattactatctgaagaacgagaaagcgaacgttgaaagtgtctttacggttaacggctttagcttcagcggccaggcacaaaacgccggtatggccttcgtcagtctgaaaccgtgggaagagcgtaatggtgacgaaaacagtgcggaagcggtaatccatcgtgccaaaatggaattgggcaagatccgcgacggttttgtcattccattcaatatgccagccattgttgaactgggcacggcaacgggtttcgactttgagttaattgatcaggctgggctgggtcacgatgccctaacccaggcccgtaaccagttgcttggtatggcggcgcaacatcctgccagcttagtcagcgtgcgccctaatggcctggaagacaccgcgcagtttaaactggaagttgaccaggaaaaggcgcaggcattaggtgtttcactttctgacatcaatcagaccatttcaacggcgctgggtgggacttacgttaacgacttcatcgaccgtggccgcgtgaaaaagttgtatgttcaggcggatgccaaattccgtatgctgccagaagatgtcgataaactttatgtccgcagcgccaacggcgaaatggtgccattctcggcctttaccacttcacattgggtgtatggctctccgcgactggaacgctacaacggtctgccgtcaatggagattcagggggaagccgcgccaggaaccagttccggcgatgccatggcgttgatggaaaaccttgcgtcaaaattacctgcgggcattggttatgactggacgggtatgtcgtatcaggaacgcttatcgggaaaccaggctcccgctctggtagcaatttcctttgtggttgttttcctgtgccttgctgcactctatgaaagctggtcaattcctgtctcggttatgttggtagtgccgttagggattgtcggcgtgctgctggcggcgacactctttaatcaaaaaaatgacgtctactttatggtgggcttgctaacgacaattggcttgtcggccaaaaacgctattttgatcgttgagttcgctaaagatctcatggagaaagagggtaaaggtgttgttgaagcgacactgatggcagtacgtatgcgtctgcgtcctatcctgatgacctctctcgcctttattctcggcgtattaccgctagctatcagtaacggtgccggcagtggcgcgcagaacgctgtgggtatcggggtaatgggaggaatggtctctgcaacgttgctggcaatcttcttcgtaccggtgttctttgtggtgatccgccgttgctttaaaggataaatcagaaacataaaggcgctttcgggtgcctttattatttccagtgaaacccataaaaattaataagatattcttctgctcactctttaaaagctttctatagttcccgctcccttcactatttttacaattcacataatttgtcattattcattccgcaagatttataacctccggtgataaaatggcattcagctcgttaataagagagttaacttattaagcgttagcgtttattactgaggtaacaccatgaaaagattaattcctgtggcattgctcaccgcattgctggcgggctgtgctcacgattcgccctgcgttccggtttatgacgatcagggtcgtctggttcacaccaatacctgtatgaaaggcacgactcaggataactgggaaacggctggggctattgccggcggggcagctgctgttgctggcctgacgatggggatcatcgctctatcgaaataactgaacagggcgcggagttccgcgctctttttaacgatacagtatctctccataagataaaatattgctatattctgctgggtaattccctgctgatttagcatgttacatcgcgttatttcgctgctttcgaaataacgcatcaatttaattttcacacttcccaccagaaatatactcacgctaacaatcattattctgcttagtaaaacacgcgtaaatattttgcgccaaaatgtggcgcatgtttcattttcgcaccattgcggggcgctgtttttattatttcctgtctacactcagcttattgcgacgcgaaatcgtgcgcaaaagctggcactacttttgcttataagaggatggccacagacaggtaaaagacgtttcccaaacgtcctataacgataattttcgcctcacaggaagcattatgaaaaagatgatgatagccacactggctgccgccagcgtgctgcttgccgttgcaaatcaggcgctgctggcgcgacgcttgatgccgttcagaaaaaaggttttgtgcaatgcgggatcagtgatggattacctgggttctcttatgccgatgctgacggtaagttttcaggtattgatgttgatatttgtcgtggtgttgccgctgctgtatttggtgacgacacgaaagtgaaatataccccgctcactgcaaaagaacgcttcaccgctttacagtcaggggaggtggatttgctctcccgtaatacgacctggacttcatctcgcgatgccgggatgggaatggcatttaccggcgtcacttattacgacggcattggcttcctgacgcacgataaagcggggctaaaaagcgcgaaagaactggatggcgctaccgtctgtattcaggcgggtactgataccgaactcaacgtcgccgactacttcaaggcaaacaatatgaagtacacaccggtgactttcgatcgctctgacgaatcagcgaaggcactggaatctggtcgctgcgatacgctggcctcggatcaatcacaactgtatgccctgcgcatcaaattaagcaacccagctgaatggattgtcttaccggaagttatctcaaaagaaccgcttggtccggtagttcgtcgtggcgatgatgaatggttctcgattgtacgctggacgcttttcgccatgctgaatgctgaagagatgggcatcaattcccagaacgtcgatgaaaaagcggctaatccagcaacgcctgatatggcacatctgctgggtaaagaaggcgattacggcaaggatctgaagctggataataaatgggcctataacatcatcaaacaggtgggtaactactcggaaatttttgagcgtaacgtaggttcagaaagcccgctgaaaattaaacgtgggcaaaataatctctggaataacggcggtattcagtacgcaccgcccgtgcgttaagtcggtgtgaggtaacgagcgtcgctacggcggcgctctcttcagcgttatgctttccgaggtttctatgtctcatcgccgctcaaccgttaaaggctcactctcttttgccaaccctacggttcgcgcctggttattccagatccttgccgttgttgctgttgtcggcattgttggttggttatttcacaacactgtaacgaatctcaataatcgtggcattacttcaggttttgcctttctggatcgcggcgctggcttcggtattgtccagcatttgatcgattaccagcagggcgacacctacggacgcgtttttattgtcggcttactcaatacgctactggtttctgcattgtgtattgtgttcgcttctgttttgggcttctttatcggtctggcgagactttcggataactggctgctacgaaagctttccacaatttatattgagatcttccgtaatattcccccgctgctgcaaatcttcttctggtactttgccgtgttgcgcaatttgcccggaccacgccaggctgtgagcgcgtttgatctggcctttttgagcaatcgtgggctttatattccgtcaccgcagctgggagacggatttattgcgtttatcctggctgttgttatggctatagtcctttctgttgggctattccgctttaataaaacataccagataaagaccggacaactgcgccgcacctggccgatcgccgcagtgttgatcattggtttgcctttactggcgcaatggctttttggcgcagcactacactgggatgtcccagccctacgaggctttaacttccgcggcgggatggttttaattcctgaactggcagccttaacgctggcactttcggtttatacatctgcatttatcgccgagattatccgcgctgggatccaggcagtgccttatggtcaacatgaagcggctcggtcactgggattacccaacccggttacgctacgccaggtcattattccccaggcattgcgggtgattattccaccgttaaccagccagtatctcaacatcgtcaaaaactcctctcttgccgccgctattggctatcccgatatggtttcgctgtttgccggcaccgtgctgaatcagacggggcaagccatcgagacgatagccatgaccatgtcggtctatctgattatcagcctgactatctcgctgctgatgaatatctataaccgccgcatcgcgatcgttgaacgctaaggagtcatgatgacaaaagtattgctgtctcatcccccgcgcccggcgagccataactcaagccgcgcgatggtgtgggtgcgaaaaaatctgttctccagctggagcaatagcctgctgactattggctgcatatggttgatgtgggaactgatcccaccgttgctgaactgggcatttttgcaggctaactgggttggctcaacgcgtgccgactgcacaaaagccggtgcctgttgggtcttcatccacgaacgatttggtcagtttatgtatgggctttacccacacgaccaacgctggcgaattaacctcgcattactgattgggcttgtgtcgatcgcaccaatgttctggaaaatactcccgcatcgcggtcgctatattgcggcctgggcggtgatttacccactgattgtctggtggctgatgtatggcggtttttttgctcttgagcgggttgaaacccggcaatggggcgggctgacgctaactttaattattgcatcagttgggattgcgggggcgctaccgtgggggatcttactggcgttaggtcgccgctcccatatgccgattgtgcgtatcttatcggtcatttttatcgaattctggcgcggcgtgccgctgattaccgttctgtttatgtcttcggtcatgctgccgttgtttatggcagaaggcaccagtatcgacaaattgatccgcgcgctggttggcgtgatcctgtttcagtcagcatatgttgcggaagtcgtgcgaggtggattacaggcgctgcctaaagggcaatatgaagcggcagagtcgctggcgttgggttactggaaaactcaggggctggttattctgccacaggcgttgaagctggtaattcctgggctggtaaataccatcatcgcactcttcaaagataccagcctggtgatcattatcgggttgttcgatcttttcagtagcgttcagcaggcaaccgttgatcccgcctggttgggtatgtcgacggaagggtatgttttcgccgcgctgatctactggatcttctgtttcagcatgtcgcgctatagccagtatctggaaaaacgttttaacaccgggcgtacaccgcattgaggacactatgagccaaattttactgcaacctgctaacgcgatgattacgctggaaaacgtcaataaatggtatggacaattccatgttttgaaaaatataaatttaaccgtgcaaccgggagaacggatcgttctgtgtggcccttcaggttccggtaaatcgacaaccattcgttgtattaatcatctggaagaacatcaacagggacggatcgtggtagatggcatcgaacttaatgaagatatccgcaatattgagcgcgtcaggcaggaagtgggaatggtctttcagcatttcaatctcttccctcatctgaccgttttacagaactgtaccctggcaccgatttgggtacgcaagatgcctaagaaagaggctgaagatctggcggtgcattacctagagcgggtgagaattgccgaacatgcgcataagtttcccggacagatttcaggtggtcagcagcaacgcgttgccattgcgcgttcgctgtgtatgaagccgaaaattatgttgtttgatgagccaacgtcggcgctcgatcctgagatggtgaaagaggtgctggatacgatgattgggctggcgcagtcgggtatgacaatgttgtgtgtaacacatgagatggggtttgcacgaaccgtcgctgaccgggtaatttttatggatcgtggggaaatagtggagcaagctgcacctgatgaattttttgcgcatcctaaatcagagcgtacgagggcatttttatcgcaggtaatccattaattgaatgttagttcgaaaagcaaaaaggccatcctttcggatggcctttcgcttgatttgatgtctggcagtttatggcgggcgtcctgcccgccaccctccgggccgttgcttcgcaacgttcaaatccgctcccggcggatttgtcctactcgggagagtgttcaccgacaaacaacagataaaacaaaaggcccagtcttccgactgagccttttgttttatttgatgtctggcagttccctactctcgcatggggagaccccacactaccatcggcgctacggcgtttcacttctgagttcggcatggggtcaggtgggaccaccgcgctactgccgccagacaaattcttttctaatctgccgaactttaacctaaaaagtggtgctgatacccagagtcgaactggggacctcacccttaccaagggtgcgctctaccaactgagccatatcagcacgctaaatttgatgcctggcagttccctactctcgcatggggagaccccacactaccatcggcgctacggcgtttcacttctgagttcggcatggggtcaggtgggaccaccgcgctacggccgccaggcaaattctgttttatcagaccgcttctgcgttctgatttaatctgtatcaggctgaaaatcttctctcatccgccaaaacagcttcggcgttgtaaggttaagcctcacggttcattagtaccggttagctcaacgcatcgctgcgcttacacacccggcctatcaacgtcgtcgtcttcaacgttccttcaggacccttaaagggtcagggagaactcatctcggggcaagtttcgtgcttagatgctttcagcacttatctcttccgcatttagctaccgggcagtgccattggcatgacaacccgaacaccagtgatgcgtccactccggtcctctcgtactaggagcagcccccctcagttctccagcgcccacggcagatagggaccgaactgtctcacgacgttctaaacccagctcgcgtaccactttaaatggcgaacagccatacccttgggacctacttcagccccaggatgtgatgagccgacatcgaggtgccaaacaccgccgtcgatatgaactcttgggcggtatcagcctgttatccccggagtaccttttatccgttgagcgatggcccttccattcagaaccaccggatcactatgacctgctttcgcacctgctcgcgccgtcacgctcgcagtcaagctggcttatgccattgcactaacctcctgatgtccgaccaggattagccaaccttcgtgctcctccgttactctttaggaggagaccgccccagtcaaactacccaccagacactgtccgcaacccggattacgggtcaacgttagaacatcaaacattaaagggtggtatttcaaggtcggctccatgcagactggcgtccacacttctaagcctcccacctatcctacacatcaaggctcaatgttcagtgtcaagctatagtaaaggttcacggggtctttccgtcttgccgcgggtacactgcatcttcacagcgagttcaatttcactgagtctcgggtggagacagcctggccatcattacgccattcgtgcaggtcggaacttacccgacaaggaatttcgctaccttaggaccgttatagttacggccgccgtttaccggggcttcgatcaagagcttcgcttgcgctaaccccatcaattaaccttccggcaccgggcaggcgtcacaccgtatacgtccactttcgtgtttgcacagtgctgtgtttttaataaacagttgcagccagctggtatcttcgactgatttcagctccacgagcaagtcgcttcacctacatatcagcgtgccttctcccgaagttacggcaccattttgcctagttccttcacccgagttctctcaagcgccttggtattctctacctgaccacctgtgtcggtttggggtacgatttgatgttacctgatgcttagaggcttttcctggaagcagggcatttgttgcttcagcaccgtagtgcctcgtcatcacgcctcagccttgattttccggatttgcctggaaaaccagcctacacgcttaaaccgggacaaccgtcgcccggccaacatagccttctccgtccccccttcgcagtaacaccaagtacaggaatattaacctgtttcccatcgactacgcctttcggcctcgccttaggggtcgactcaccctgccccgattaacgttggacaggaacccttggtcttccggcgagcgggcttttcacccgctttatcgttacttatgtcagcattcgcacttctgatacctccagcatgcctcacagcacaccttcgcaggcttacagaacgctcccctacccaacaacgcataagcgtcgctgccgcagcttcggtgcatggtttagccccgttacatcttccgcgcaggccgactcgaccagtgagctattacgctttctttaaatgatggctgcttctaagccaacatcctggctgtctgggccttcccacatcgtttcccacttaaccatgactttgggaccttagctggcggtctgggttgtttccctcttcacgacggacgttagcacccgccgtgtgtctcccgtgataacattctccggtattcgcagtttgcatcgggttggtaagtcgggatgacccccttgccgaaacagtgctctacccccggagatgaattcacgaggcgctacctaaatagctttcggggagaaccagctatctcccggtttgattggcctttcacccccagccacaagtcatccgctaatttttcaacattagtcggttcggtcctccagttagtgttacccaaccttcaacctgcccatggctagatcaccgggtttcgggtctataccctgcaacttaacgcccagttaagactcggtttcccttcggctcccctattcggttaaccttgctacagaatataagtcgctgacccattatacaaaaggtacgcagtcacacgcctaagcgtgctcccactgcttgtacgtacacggtttcaggttctttttcactcccctcgccggggttcttttcgcctttccctcacggtactggttcactatcggtcagtcaggagtatttagccttggaggatggtccccccatattcagacaggataccacgtgtcccgccctactcatcgagctcacagcatgtgcatttttgtgtacggggctgtcaccctgtatcgcgcgcctttccagacgcttccactaacacacacactgattcaggctctgggctgctccccgttcgctcgccgctactgggggaatctcggttgatttcttttcctcggggtacttagatgtttcagttcccccggttcgcctcattaacctatggattcagttaatgatagtgtgtcgaaacacactgggtttccccattcggaaatcgccggttataacggttcatatcaccttaccgacgcttatcgcagattagcacgtccttcatcgcctctgactgccagggcatccaccgtgtacgcttagtcgcttaacctcacaacccgaagatgtttcacttcagagttgcgaaaatttgagagactcacgaacaactttcgttgttcagtgtttcaattttcagcttgatccagatttttaaagagcaaaacttcgcagtgaacctttgcaggtacactctgaagtattttttatttaatcactacagagatggtggagctatgcgggatcgaaccgcagacctcctgcgtgcaaagcaggcgctctcccagctgagctatagccccataacatgtagttaaaacctcttcaaatttgccgtgcaaatttggtaggcctgagtggacttgaaccaccgacctcacccttatcaggggtgcgctctaaccacctgagctacaagcctgtagaggttttactgctcattttcatcagacaatctgtgtgagcactgcaaagtacgcttctttaaggtaaggaggtgatccaaccgcaggttcccctacggttaccttgttacgacttcaccccagtcatgaatcacaaagtggtaagcgccctcccgaaggttaagctacctacttcttttgcaacccactcccatggtgtgacgggcggtgtgtacaaggcccgggaacgtattcaccgtggcattctgatccacgattactagcgattccgacttcatggagtcgagttgcagactccaatccggactacgacgcactttatgaggtccgcttgctctcgcgaggtcgcttctctttgtatgcgccattgtagcacgtgtgtagccctggtcgtaagggccatgatgacttgacgtcatccccaccttcctccagtttatcactggcagtctcctttgagttcccggccggaccgctggcaacaaaggataagggttgcgctcgttgcgggacttaacccaacatttcacaacacgagctgacgacagccatgcagcacctgtctcacggttcccgaaggcacattctcatctctgaaaacttccgtggatgtcaagaccaggtaaggttcttcgcgttgcatcgaattaaaccacatgctccaccgcttgtgcgggcccccgtcaattcatttgagttttaaccttgcggccgtactccccaggcggtcgacttaacgcgttagctccggaagccacgcctcaagggcacaacctccaagtcgacatcgtttacggcgtggactaccagggtatctaatcctgtttgctccccacgctttcgcacctgagcgtcagtcttcgtccagggggccgccttcgccaccggtattcctccagatctctacgcatttcaccgctacacctggaattctacccccctctacgagactcaagcttgccagtatcagatgcagttcccaggttgagcccggggatttcacatctgacttaacaaaccgcctgcgtgcgctttacgcccagtaattccgattaacgcttgcaccctccgtattaccgcggctgctggcacggagttagccggtgcttcttctgcgggtaacgtcaatgagcaaaggtattaactttactcccttcctccccgctgaaagtactttacaacccgaaggccttcttcatacacgcggcatggctgcatcaggcttgcgcccattgtgcaatattccccactgctgcctcccgtaggagtctggaccgtgtctcagttccagtgtggctggtcatcctctcagaccagctagggatcgtcgccttggtgagccgttaccccaccaacaagctaatcccatctgggcacatccgatggcaagaggcccgagggtccccctctttggtcttgcgacgttatgcggtattagctaccgtttccagtagttatccccctccatcaggcagtttcccagacattactcacccgtccgccactcgtcagcgaaacagcaagctgtttcctgttaccgttcgacttgcatgtgttaggcctgccgccagcgttcaatctgagccatgatcaaactcttcaatttaaaagtttgatgctcaaagaattaaacttcgtaatgaattacgtgttcactcttgagacttggtattcatttttcgtcttgcgacgttaagaatccgtatcttcgagtgcccacacagattgtctgataaattgttaaagagcagttgcgacgcggctttcagctcactgtcgcgaggtggcgtatattacgctttcctctttcagagtcaaccctgaatttcaggatttttttctcttcgttgttccgaccatcctgtgaagtgtttcacgttgtcgtctcaacggaggcgcattatagggatcccaattttttgcacaagtatttttttgatctttttttctgtttgttgttttttcaccctttttgctgcaatcgcacacaaaacggtgcttttttgcatactaaaagacttgcacaaggccaataatgcccccaaagtcattagtaaatcatttattgctgaggtaagtatgtctgatgttttacgcccataccgcgatctttttccacaaatcggtcagcgcgtaatgatcgacgatagcagtgtcgtgattggtgacgttcgtctggctgatgatgtggggatctggccgctcgttgtgattcgtggagatgtacattatgtacagatcggagcacgcaccaatatccaggatggcagtatgttgcatgtcactcataaatcctcgtacaacccagatggcaacccattaaccattggcgaagatgtcactgttggtcacaaggtgatgctccacggctgcaccattggcaatcgagttttggttgggatgggctcaattttacttgatggcgcaatagtagaagatgatgtgatgattggtgcgggtagtctggtcccacaaaataaacggctggagagcggatatctgtatctcggtagccccgtcaaacagatccgcccgttaagtgatgaagagaaggctgggttacgctattccgcgaataattacgtgaaatggaaggacgaatatctggatcagggtaaccagacccagccttgatcatcttcactttgttcctgaattaagttttccgcttcttcttccaggtcccagcgatgctgacgaaaactcgctaaccactgttctggcgtatctccagtaaagcgatacgccagactctcgccagagatcgcgcatgtcagttgcataccattcacgagagcgggaaaacatacacattttttattctcgtcccactcttccctgtccggaaactggatggcctgattcacgcggacaattcctcctgcaattgctttataactggttctacgtcaggcagaacaccgtgccagagaagaaaggcatgagccgcctgtgccaccagcattcctaaaccatcagcattacgctttgagcctcgctgctcacaccatgccagaaaaggagtttttcctttctgatagaacatgtcatagcaataaatgcctggatgaatgagcgatgacgggatcgccggaatatcaccactgatgccactggatgttgcattaataatgagatcaaactcatgaccttccagttcgtccatactcaacgcctgaatactgccagtgtgcgcaaacaatttagccaactcttccgcgcgggataccgtccgattagttattgtcaccgcacagtccagggaaaggagtggcagtagtacgccgcgagatgctccaccagcgccgataagcagaatacgtaaaccagggcggataaaagacagacgttccagatcgcttaacaagcctacaccatcggtattgtcacccagcaggcgtccatcttctaaccgcatgagggtattaacagcaccagccaacgctgcccgttcagtaagctcatccgctctggcaaaagcctcttctttaaaaggcaccgtcacattcgcacctttaccaccagcactaaagaaagcgttcagtgtgttgatgaaatcattgatgggtgccaacacgcgcccatagggatgttcaatattcagttgctgagcaaattgctgatgaatgaatggcgatttgctgtgggctatcggattaccaaaaacagcataggtttccattatgttacccctgtcgaaacagttcacccgtcagggcatcgcggatttctgaaggatttaaacgcccccccgtttcaccaggcacaaccgggaacgccgcgccaaattgtgcgcgaacttcgtctactgttcgacaaggtggcaatccactcaagttggcactggtagaaaccagcggtttaccataagcctggcacaaagcaaccaccaacggatggtcggtgactcgtacagcaagcgaatcaaagcggcccgtcaaccagcgcggtgttgtcgcaggcgcgggaaagacaaaggtgacaggacctggccagcgggaaaaaatggtttcacgctgcacgtcagtcaacatggtgtcatcaatatagggtttaagctgctcgtaatttgctgcgattaaaatcagccccttatcaaccggacgctgttttaactccaacagtcgcatcactgctgtttcgctatcaggatcgcacccaacaccgaaaacggcttccgttggataggcgatgacacgttcttcattgagaacatctatcgcagctgcgatagcgtctctttgcaggttattattcacgttattattccgccgaaaccggctttccacattgtttactggcacaaaagtgttttacaccctgcgcggttttcttttcgatgagtagcggataatgacactcagggcattctccagctatgggtttgaagttaatggcaaattgacactccgggtagcgatcacaagagtgaaatgttttgccataacgggagcggcgctggaccagatggcccgtccgacattgggggcatgtaattgctgtttcgtccggtttatcgataagttcggtatgttcgcattcagggtagttaatgcaaccaataaacataccaaagcgtccctggcgtaataccagatttgcgccacatgcagggcaaacctgcccctccagaactttgacgatatgtccatccgctgaagatttcagaggacggacgtagtcacacgccggatactgtgagcatccaagaaacggaccgtgtttcccggatcgaataaccagttcagccccgcactttgggcaggactcattattacgcaccgtgaacagtgctgatttcgccataacaacttatgctgaattaaagaaatgattaatgcagcataccttcattcacttcaaagagtaattcttccatttgctggtacgcattttcgcagcccggaatattgaacaacaccatcaggatcacccatttcagatcatccagttcgaactctgcgttatccagcgcgagcactcgctctatcaccatttcacgagtttcaaggttgagcacctgaatctgctcaaggaaaagcagaaacccacggcagctggcatccagtcgttcacactcttccggtgtataaatacgcatggagagaggatccgaggccagttgcatcggttctgccaacccttcctgataatcagcaagtttttccagccatagcagggcattgtagatatcttctcgctcaaaacctgcgtcggtaagatcctgttcaagtttgtcttgatccacacgcaactcagcttctgtgtgaatataggtttcaaacaaatacattagtacgtcgaacatggcatgccctcctcaatcggacatagccgccgggtacagctgcgatccatcctgctaactccagttcgagtagttgagtaactacctctggcacaggttggccggcacgttcagcgacgacgtcaacaggtgttacctcatctcctacgttagccaggagctcaggaaatggcaatgccacgtcttgctgatctggtgaataaaatgaattttcaggggcgtctggcaaccagtgcaatccaaattgcaagttttccagaatttcttccggttccgtcacaagaatcgcaccttgttttattaaccagtgaggcccttcgcttcccggattccctattggacctggcaaggcaaaaacttctcgcccctgctcaagcgcacaacgtgctgtcaccagcgaaccactacgcaaagccgcttccaccaccagtacacctttacttagaccactgataatgcgatttcttcgtgggaaattgtaagcaaggggtggaacatcgaggggaaattccgagacgagagcgcccccctgttcaagcagactggcagccagtcgggcatgacggcggggatgaatggtattaagtccattccccaatacagcaatgctgacgccatttacctgtaaggctgctttatgcgctacaccatcgattccacgcgccagtccactcgtaattgtcactccacgcgtcgccagagtttcgcaaaataatcgtccccatcgctcgccataccatgaatgcgcccgactccccactacggcaagctgaaatgaatgcagcgcgtgcagttctccttcaacaaacagtgcgccggggtaatctgtcgtcgccagaagttgaggaggataaaattcgctgtccgcaggaattaaatgatggttgggttgctccaaccaacaaagtgagctttcgatactctttcgtggaaatgaaagaaagcgttgtgcctgccgcaatgtaagccctgtttgctgcaatacaaccgcatcaatatgcgactgttttgccacccagtgagcgatacggaccatatcatcgccgtacaagctgctgatactcattaaacgcagccaaatttctgtatcgaccatccttatctccctgccataagcagccttagcaatctttgcgattggtcagtgatgctgtcaatcagagggggatttgtctagaatagaagaaataatctttctaactcctgaacacatctctggagatttatgtcagttttgcaagtgttacatattccggacgagcggcttcgcaaagttgctaaaccggtagaagaagtgaatgcagaaattcagcgtatcgtcgatgatatgttcgagacgatgtacgcagaagaaggtattggcctggcggcaacccaggttgatatccatcaacgtatcattgttattgatgtttcggaaaaccgtgacgaacggctagtgttaatcaatccagagcttttagaaaaaagcggcgaaacaggcattgaagaaggttgcctgtcgatccctgaacaacgtgctttagtgccgcgcgcagagaaagttaaaattcgcgcccttgaccgcgacggtaaaccatttgaactggaagcagacggtctgttagccatctgtattcagcatgagatggatcacctggtcggcaaactgtttatggattatctgtcaccgctgaaacaacaacgtattcgtcagaaagttgaaaaactggatcgtctgaaagcccgggcttaaggataagaactaacgtgtcagaatcactacgtattatttttgcgggtacacctgactttgcagcgcgtcatctcgacgcgctgttgtcttctggtcataacgtcgttggcgtgttcacccagccagaccgaccggcaggacgcggtaaaaaactgatgcccagcccggttaaagttctggctgaggaaaaaggtctgcccgtttttcaacctgtttccctgcgtccacaagaaaaccagcaactggtcgccgaactgcaggctgatgttatggtcgtcgtcgcctatggtttaattctgccgaaagcagtgctggagatgccgcgtcttggctgtatcaacgttcatggttcactgctgccacgctggcgcggtgctgcaccaatccaacgctcactatgggcgggtgatgcagaaactggtgtgaccattatgcaaatggatgtcggtttagacaccggtgatatgctctataagctctcctgcccgattactgcagaagataccagtggtacgctgtacgacaagctggcagagcttggcccacaagggcttatcaccacgttgaaacaactggcagacggcacggcgaaaccagaagttcaggacgaaactcttgtcacttacgccgagaagttgagtaaagaagaagcgcgtattgactggtcactttcggcagcacagcttgaacgctgcattcgcgctttcaatccatggccaatgagctggctggaaattgaaggacagccggttaaagtctggaaagcatcggtcattgatacggcaaccaacgctgcaccaggaacgatccttgaagccaacaaacaaggcattcaggttgcgactggtgatggcatcctgaacctgctctcgttacaacctgcgggtaagaaagcgatgagcgcgcaagacctcctgaactctcgtcgggaatggtttgttccgggcaaccgtctggtctgatagtccactcttctaagcccggtcttgccgggcgtttttatacttatgaaaaaacaacgtaatttacgtagcatggcggcccaggccgttgaacaagtcgtcgagcaagggcaatcattaagcaacattctgccaccgctccagcaaaaagtttccgataaagacaaagcacttcttcaagagttgtgctttggcgtactgcgtacgctttcgcagttagactggctgattaataagttaatggcccgtccgatgaccggcaaacagcggaccgtgcattacctgattatggttggtttgtatcaactgctttatacccgcattccacctcatgctgcgctggctgaaacggttgaaggcgctatcgcaattaagcgtccgcaacttaaagggttgataaacggtgtattacgccagttccagcgtcagcaagaagagttattagccgagtttaatgccagtgatgcacgttatctgcatccttcctggttgctgaagcgtctgcaaaaagcgtatccagagcagtggcaatccatcgtcgaagccaataaccagcgtccgccaatgtggctgcgtattaatcgtacgcatcattcccgcgacagctggcttgcattgctggatgaagcaggaatgaaaggtttcccgcatgcggattaccctgatgctgtacgtctggaaacacctgcacctgttcatgcgctacctggttttgaagacggatgggttaccgttcaggatgcatcagcacaaggttgcatgacctggcttgcgccacaaaacggtgaacacattttggatctttgtgccgcccccggcggtaaaacaacgcatatccttgaggtggcaccagaagcgcaggttgttgcggttgatatcgacgaacagcgcctctctcgggtttacgacaatttaaaacgccttggtatgaaggcgaccgtgaaacaaggtgatggccgttacccttctcaatggtgtggcgagcaacagtttgatcgcattttattagatgcgccttgttcagcaaccggtgtgattcgtcgccatccagatattaaatggttacgtcgcgatcgcgatatcccggaactcgcgcaattgcagtctgaaattctcgacgccatttggccgcatttaaaaaccggtggaactctggtctatgccacctgttcggtgttaccggaagagaatagcctgcagattaaagcctttttgcaacgtaccgctgatgccgaactttgcgaaacaggaacaccagagcaaccgggtaaacaaaatctacctggtgccgaagagggcgacggcttcttttacgctaagctaatcaaaaagtgatgagataacgggtcgcgactgatgaaaattatcattctgggtgccggccaggttggcggcacactggcggaaaacctggttggcgagaacaacgatattactgttgtcgataccaacggtgagcgtctgcggaccttacaggataaatttgacctgcgggtcgtgcaggggcatggctctcatccacgcgtattgcgggaggcaggtgccgacgacgccgatatgctggttgctgtaaccagttcagatgaaaccaatatggttgcctgccaggtagcctactcacttttcaacacccctaatcgcatcgctcgtatccgctcaccagactacgtgcgcgatgccgataagctatttcattcagatgctgtgccgattgatcatctgatcgcaccagagcagttggttatcgataatatttaccgactgattgagtatcccggcgcattgcaggtggtgaacttcgctgagggtaaagtcagcctggctgtggttaaagcctattatggcggcccgctgattggtaatgcactttcgaccatgcgcgaacatatgccacatatcgatactcgtgtggcagcaattttccgccacgatcgccccattcgtccgcaaggttcgaccattgttgaagctggtgatgaagtgttctttattgccgcttcacagcatatccgcgcggtgatgagtgaattacagcgactggaaaaaccgtataagcggatcatgctggttggtggcggtaatatcggtgcagggctggcgcgtcgtctggaaaaagattacagcgttaaactcatcgaacgtaatcagcagcgcgctgccgaactggcggaaaagttacagaatacgatcgtcttttttggtgatgcgtcggatcaagaactactggccgaagaacatatcgatcaagttgatctgtttattgccgtcaccaacgatgacgaggccaatatcatgtccgccatgcttgccaaacgtatgggtgcgaaaaaggtgatggtattgatccagcgtcgcgcttatgtggatctggttcaggggagcgttatcgatattgcgatttcaccacaacaagcaactatttctgcgttgcttagccatgtgcgaaaagcagatattgttggtgtttcctcattgcgccgcggcgtagcagaagctattgaagccgttgctcacggtgatgaaagcacctcacgcgttgtcggcagagtcattgacgaaatcaagctaccgccaggaacgattattggagcggtggtacgtggaaacgacgtgatgattgccaatgacaatctgcgcattgagcaaggcgatcacgtaattatgttcctcacagataaaaagtttattaccgacgtcgaaagactcttccagccaagccctttcttcttgtaattaataaggcgtctaatgacgccttattatttccctttgattatcaaggattaattaaattcattcctggcaggaaaatggcttaacatttgttagacttatggttgtcggcttcatagggagaataacatgagcattattaaagaatttcgcgaatttgcgatgcgcgggaacgtggtggatttggcggtgggtgtcattatcggtgcggcattcgggaagattgtctcttcactggttgccgatatcatcatgcctcctctgggcttattaattggcgggatcgattttaaacagtttgctgtcacgctacgcgatgcgcagggggatatccctgctgttgtgatgcattacggtgtcttcattcaaaacgtctttgattttctgattgtggcctttgccatctttatggcgattaagctaatcaacaaactgaatcggaaaaaagaagaaccagcagccgcacctgcaccaactaaagaagaagtattactgacagaaattcgtgatttgctgaaagagcagaataaccgctcttaacaagcgcctgaaagcagaagaccagtggtaaaaaagtgatttactttcttgccactggcctcccagttcccccgattgccatgttttccttttcgcatgtaactgcctttccccttcttatttttctctacgcgctgtcggaataagggatcatgtagtaatgcttctatcgcattatcctttatctgccctttagtatgctgatatcgactcataaaaactccagttggttatttaacggcgcgagtgtaatcctgccagtgcaaaaaatcaacaaccactcttaacgccactcgccccttgttcaagagcttcaagaatcgaacaataaacactgctatgagcagtcccacaacaggcatcgttaaggcgttgcaaggaacgctgcatactctgcaactcggctatccgtgcttcgacttcctgcaatctttcctgcacaatgccttttgactcctgacaggtatggtgttcaggatcgatgcggatcgacagcaactcgcggatcgactccagactgaaacctagttgtctggcatggcggataaatttcaatcgctggagatcgctttcggtatataggcgaaacccaccttcagtacgcacttcatgctccatcatctgctgtttttcgtaataacgaatcgtgtcgggtgttacttccgccatttttgccagctcaccaatgcgatacatacatactccactagttatcgttgattttgtccaacaacttgtcagcataatcgccgcgtaaaaaatcggtactcaatccagcttgtcgcagcttcaattccagtaatgacaatcgacggctaacctcttgatattgcggatcatcgtgacggatacctttgagaatatccagaagctgaattgcttctctccgttgctcaagttctggcggtaagcaaccggcattcttcagcaagcgataccccgcacgtaattccggtggcacgtgagaatcatcatccagtatcaatggttcgccgctacctgccaggttatcaaactcacctttcgcttgcgcttctgctatatggcgctctgcccactggtcaagtaaccacataaatactccaggggatgaacaaaaagagtacagctattgtagataagtggggatactacgggtataaaaaaacccgccggggcgggtttttttacgttgcttcagattactctgcagcagcttctgctttctctgaacgatcaaccagctcgatgtaagccatcggcgcgttgtcgcctgcacggaagccacacttcagaatacgagtgtaaccaccggcacggctcgcgaaacgcgggcccagttcgttaaacagttttgccacgatctcgttatcacgagtacgggcgaatgccagacgacgattagcaacgctatcagtcttggcaagagtaatcagcggctcaactacgcggcgcagctctttcgctttaggcagagtcgtcttgatgatttcatgacgaaccagtgaacctgccatattgcggaacatagcctggcgatggctgctgttgcggttcagttgacgaccactcttacgatggcgcatgaccttatccttctcagtaaaaccttaacctgtgatccggttactcgtcagcgatgcttgccggtggccagttttccaggcgcatgcccagagacagtccacgggaagccagcacgtctttaatctcagtaagagattttttaccaaggttaggcgttttaaggagctcaacctcggtacgctgtaccagatcaccgatatagtggatagcttctgctttaaggcagttagcagagcggacagtcaattccagatcgtcaacagggcgcagcaggatcggatcgaactctggtttctcttctttcacttcaggctgacgtacatcacgtaagtcaacgaaagcttccagttgttcagccagaatggttgccgcacgacgaatcgcctcttcaggatcgattgtgccgttggtttccatttcgatgaccagcttgtccaggtcggtacgctgttctacacgcgctgcttcaacattgtaggcaatacgctccacagggctgtagcatgcgtcgaccagcagacggccgattgggcgctcatcttcttccgaatgaattcgggtagaagccggcacataaccacgaccgcgctgaactttgatacgcatgctaatagacgcgttctcatcggtcaggtggcagatcacgtgctgcggcttgacgatttcgacatcaccgtcgtgggtgatatcggctgcagtcacagggccaatgccagatttattcaaggtaagaataacttcatctttgccctgaactctcaccgccagccctttcaggttgagcaggatttccaggatatcttcctgaacgccttctttggtgctgtactcatgtagtacaccatcaatctcaacctcggtcaccgcgcaacccggcatcgatgagagcagaatacggcgcagtgcgttacccagagtatggccaaagccacgctctaaaggctcaagggtcaccttggcgtgcgtcgaactcacttgctcgatatcaaccaggcgcggttttagaaactctgtcacagaaccctgcattgtgtcctctctttggtactaagctttacttggagtaaagctcgacgatcaggtgttcgttaatgtccgcagacagatcagaacgctccggcttacgcttaaacgtaccttccatcttgccagcatcaacttccagccaggttggcttttcacgctgctcagccagctccagagcggctttcacgcgagactgcttcttcgctttctcacgaatgcttacaacgtcattcggactaacctgataagaagcgatgttaacaacacgaccgtttaccataattgctttatggctaaccagctgacgtgcttctgcacgagtggcaccgaagcccatacggtatacaacgttgtccagacgaccttccagcagagccaacaggttttcaccggtgttgcctttcagacgtgctgcttctttgtagtagttacggaactgacgctccagcacaccatagatacggcgaactttttgcttttcacgcaactgcacaccatagtcagacagacgcggtttacgcgcaccgtgctggccaggagcttgttcaattttacacttggtatcgatcgcgcgaacgccagacttaaggaataagtcggtgccctcacgacggctcagcttgagcttaggacccaaatatcttgccattttctttctccaacaaacctggaaaacgaggcgttatacgcgacgttttttcggcggacgacaaccgttatgagggatcggagtcacatcagtaatgttagtgatgcggaaacctgcggcgttcagagcacgaatagtagattcgcggcctggacccggacctttaaccataacttccagattcttgatgccgtattctttcacggcgtcagcgcaacgctctgctgcaacctgagctgcaaacggagtggatttgcgagaaccacggaaaccggaaccaccggctgttgcccaacccaacgcgttaccctgacgatcagtgatagtcacgatggtgttgttgaaagaagcatggatatgagccacgccgtcagagacttgttttcttacacgtttacgtgcacgaattggtgcctttgccattattcaatcaccccgattatttcttgatcggtttgcgcggacccttacgggtacgtgcgttggtcttggtacgctgaccgcgaaccgggagaccacgacgatgacgcaaaccgcgatagcaaccaagatccatcaggcgcttgatgctcatgctgatttcacggcgcagatcaccttcaacgacaaatttggcaacttcgtcacgcagcgtgtcgatttgtccttcagacagctcactgatcttaacatcttcagcgatacccgctgcagccaggatggctttagaacgggtcttgccgacgccataaatcgaagttaatgcgattacggcatgcttatgatcaggaatgttaatgcctgctatacgggccactatgcactcctactatttaatatgtacgttccatgctgaaaagcccgttttcaggatactcaaatggaaacgcacagacatacaaaagattggctggctaatctagccagctcaacccaactttgcaagaaaaatatgcgaaaaaatcagccttggcgctgtttatgcttcggctcggcactgcaaatcacacggatgacaccatcacgcttaacgattttgcagttacggcataatttcttgacggaagcacgaactttcatttttactctccgtaacttctcgggcgaccaattatcggccgtagcctttcaggttcgccttcttcaatgcagactcatactgactggacatcatcagagtttgcacttgagccataaagtccataatcacgacaacaacgataagcagtgaggtcccaccgaagtagaacggtactttcattgcatcacgcatgaactccgggatcaggcagataaaggtaatatacagcgcaccaaccagggtcaggcgggtcattactttatcgatatacttcgccgtttgctctcccggacgaattcctggtacaaatgcaccggacttcttcaggttatctgctgtttcacgcgggttgaaaaccaacgccgtgtagaagaaacagaagaagatgattgcagacgcatagagtaacacataaagcggttgcccaggctgcaaatacagcgaaattgttgtcagccagttccaaccagtaccgcccccgaaccatgacgcgatggtcgccgggaacagaataatactggaagcgaagattgccgggattacccccgccatattcactttcagcggtaaatgtgtgctctgtgcagcatagacacgacgaccttgctgacgtttcgcgtagtttaccacaatgcggcgttgaccacgctcaacaaatacaacaaagaacgtcactgcaaatactaatactgcaaccaacagcaacacgaggaagtgcaggtcgccttgacgcgcttgctcgatagtatgggcaatggctggcgggagtcccgcgacaataccggcgaagataatgattgaaataccgttgccgatacctcgttcagtaatctgttcgcccaaccacatcaggaacatggttcctgtgaccagacttacaacagcggtgaagtagaatgcaaagcccgggttaatcaccaggccttgcataccaggcatattcggcagaccggtagcaataccgatcgactggaatattgccagcaccagagtaccgtagcgggtgtactggctgatcttacgacgaccagactccccttctttcttaatttctgccaacgttgggtgaaccaccgtcagcagctggataatgatcgacgccgaaatatacggcatgatccccagagcaaagatagaagcacggctgagagcaccaccagagaacatgttaaacatctcaatgatggtgcctcgctgttgctcaagcagtttggcaagtacagcggcatcaataccagggatcggaataaaagagccaatacggaacacaatcagcgcaccgataacaaacagcagtctgcgtttcagctcgcctaagccacctttggcactttgaaaatctaatcccggttgtttagccatctgctacttattcctcgattttaccgccagcagcttcgatagcagcacgagcgcctttagtaacacgcaggccacgaacagttaccggagtcgttacttcgccagccaggatcactttcgcgaactcgatctggataccgataatgttagccgctttcagcgtgttcaggtctactacaccgccttctactttagccaggtcagacagacgaatttcggctgtaatcgctgctttacgagaagtgaagccgaatttcggcagacgacggtacagaggcatctgaccaccctcgaaaccgcgacgtacgccaccgccagaacgagacttctgacctttgtgaccacgaccaccggttttaccgaggccagaaccgataccacgacccaggcgtttacccgcctttttggagccttcggccggagacagagtatttaaacgcatctcttactcctcaactttaaccatgaaggaaaccgcgttgatcataccgcgaatagcaggagtatcctcgcgctctacggtgtgaccaatacgacgcagacccaggccaagcagcgttgccttgtgtttcggcagacgaccgattgcactgcgggtttgagtaattttaatagtctttgccatggtttatttccccagaatttcttcaacggatttaccacgcttggcagcgaccatttctggagaattcatattttccaggccatcaatagttgcacgaaccacgttgatcgggttggtggaaccataggctttagccagaacgttatgaaccccagcgacttccagaacggcgcgcattgcaccaccggcgatgataccggtaccttcggaagccggctgcatgaatacgcgagaacccgtgtgaacacctttaacagggtgttgcagagtgccgttattcagcgcgacgttaatcatattgcgacgggctttttccatcgctttctggatcgctgctggaacttcacgcgctttaccgtaaccaaaaccaacgcgaccgttaccatcgccaactacagtcagagctgtgaaggagaaaatacgaccacctttaacggttttagatacgcggtttaccgcgatcagcttttcctgcagttcgccagcttgtttttcgatgtgagccatcttacacctctaccttagaactgaaggccagcttcacgggcagcatctgccagtgcctggacacgaccatgatattggaacccggaacggtcaaaggatacatctttgatgcctttttccagagcgcgttcagcgacagctttacccacagctgcagccgcgtctttgttaccggtgtacttcagttgttcagcgatagctttttctacagtagaagcagctaccagaacttcagaaccgttcggtgcaattacctgtgcgtaaatgtgacgcggggtacgatgtaccaccaggcgagttgcgcccagctcctggagcttgcggcgtgcgcgggtcgcacgacggatacgagcagatttcttatccatagtgttaccttacttcttcttagcctctttggtacgcacgacttcgtcggcgtaacgaacacccttgcctttataaggctcaggacgacggtaggcgcgcagatccgctgcaacctggccgatcacctgcttatcagcgcctttcagcacgatttcagtctgagtcggacattcagcagtgatacccgcaggcagctgatggtcaacaggatgagagaaacccagagacaggttaatcacattgcctttaaccgctgcacggtaacctacaccaaccagctgcagcttcttagtgaagccttcggtaacaccgataaccattgagttcagcagggcacgcgcggtaccagcctgtgcccaaccgtctgcgtaaccatcacgcggaccgaaggtcagggtattatctgcatgtttaacttcaacagcatcgttgagagtacgagtcagctcgccgtttttacctttgatcgtaataacctgaccgttgatttttacgtcaacgccggcaggaacaacgaccggtgctttagcaacacgagacattttttcctccgattaggctacgtagcagataatttcgccaccaagaccagcctggcgcgctgcacgatcagtcataacacctttagaggtagaaacaactgcgatacccagacccgccataactttcggcagctcatctttacgtttatagatgcgcagacctgggcggctgacacgctgaatgctttctacaacagctttgccctggaaatacttcagagtaagttccagttcaggcttggtgtcgccttcaactttaaaatcttcaataaaaccttcttccttcagcacgttggcgattgccactttcagcttggaggaaggcatggtgaccgcagctttgttcgcggcctgaccgttacggatacgggtcagcatatccgcgatcggatcttgcatgctcatctgtctttactcccgtgattcaattggtgacaattaccagctagcctttttcagacccgggatttcaccgcgcatagcggcttcacggaccttaatacggctcaacccgaacttccgcaggaaaccatgcggacgacctgtttgacggcagcggttacgctgacgagacgggctggaatcacgcggcagagtctgcagcttgagaacagcgttccaacgatcttcgtcggaagcgttcacatcagagatgatcgctttcagttcagcgcgtttcgcgaagtatttatcagctaaagctacgcgttttacttcgcgtgctttcattgattgcttagccatttagtaaccctaccttacttgcggaacgggaagtcaaaggcagccagcagagcgcggccttcttcgtcagatttcgcagtagtggtaatggtaatatccaaaccacgaacgcggtcgactttatcgtagtcgatttctgggaagatgatctgctcacggacacccatgctgtagttaccacgaccgtcgaaagacttagcggacaggccacggaagtcacggatacgaggtacagcaatagtgatcaggcgctcaaagaactcccacatgcgttcgccacgcagagttactttacagccgatcggatagccctgacggattttgaagcctgcaacagatttgcgtgctttggtgatcagcggtttttgaccggagattgctgccaggtctgctgctgcgttatccagcagttttttgtcagcgatcgcttcaccaacacccatgttcagggtgatcttctcgacccgagggacttgcatgacagaattgtagttaaactcagtcatgagttttttaactacttcgtctttgtagtaatcatgcagtttcgccatcgtactactccaaattacttgatagtttcgctgttagacttgaagaaacggacttttttaccgtcttcgaatctaaagcctacacggtcagccttgccggttgccgcattgaagattgctacgttggaaacctgaatagcggcttctttttcaacgatgccacccggttggttcagggccggaaccggcttctgatgtttcttaaccaggttgataccttcaacaatgaccttgccggaagacaggacattcttaactttaccgcgtttacctttatctttaccggttaacacgataacttcgtcatcacgacggattttcgctgccatgattcgctccttagagtacttctggtgccagagagataattttcatgaacttctcactacgaagctcacgagttaccggcccaaaaatacgcgtaccgataggctgctcgctgttgttgttcagaagaacacaagcattaccatcgaagcgaatgacagaaccgtccgggcgacgaacacccttcttggtgcgcaccactaccgccttcagcacatcaccttttttgaccttaccacgcggaattgcttctttgatggtgatcttgatgatgtcgcctacgcctgcgtagcgacggtgcgagccacccagaaccttgatacacattacgcgacgtgcaccggagttgtcggcgacgttcagcatagtctgttcttggatcattttagtgctccgctaatgtcaactactactgagacccgaaaatcaggtcgttaaaaatccccatatcgagggcgcggcattataacaccgcttcaaggatatgggtagaaaaaataaacggctcatttctgagccgtttattcgtattgagagagtgtactgtattacagaaccgctttctctacaacgcgaaccagcgtccaggatttagtcttggacagcggacggcattcgcggatttcaaccacgtcaccgataccgcattcgttgttctcgtcatgtacgtgcagtttggtcgtacgcttgatgaatttaccgtagatcgggtgtttcacaaaacgttcgatagcaacaacaatggatttctccattttgtcgctaacaacgcgaccttgcagagtacggattttatcggtcattacgcacccgccttctcgttcagtaaagtcttaacgcgtgcgacatcgcgacgcacttgcttcaacaggtgagactgttgcagctggccacttgcagcctgcatacgcaggttgaactgctcacgcagcaggttcagcagctcggtgttcagctcttcaacgctcttctcacgcagctcttttgctttcattacatcaccgtcttagttacaaaggtggttttaatcggcagtttcgctgctgccagcttgaatgcttcacgggccagctcttccggaacaccgtccatttcatacaggactttacccggctgaatcaaggcaacccaatactccacgttacctttacctttacccatacgcactgccagcggcttttcagtgatcggtttgtccgggaacacacggatccagatcttaccttgacgcttaactgcacgggtcatagcacgacgtgctgcttcgatctgacgggcagtcagacgaccacggccaacagctttcagaccgaagctgccgaagctaacatccgtaccctgcgccagaccgcggttacggcctttgtgcattttacggaattttgtacgctttggttgtaacatcagcgacgctccttatttacggcctttacgctgctgctttttaggctgagcagccggtttttccggttgttcaacagcagccataccacccaggatctcgcctttgaagatccacactttaacgccgattacaccgtaagtggtgtgcgcttcagaggtgttgtagtcgatgtcagcacgcagagtgtgcagcggtacgcgaccttcgcggtaccattcggtacgtgcgatttccgcgccgcccagacggccgctaacttcaactttaatacctttagcgcccagacgcattgcgttctgtacagcacgcttcatagcacgacggaacataacgcgacgttccagctgagaagtgatgctgtcagcaaccagttttgcgtccagttcaggcttacgaacttcggcgatgttgatctgtgcaggaacgccagcgatgtccgctacgaccttacgcagtttttctacgtcttcaccttttttaccgataacgatacccgggcgagcagtgtgaatggttacacggatgctcttagccggacgctcgataacgatacgagatacggacgctttagccagttccttagtcaggtactgacgtactttaaaatcgctgtccaggttgtcagcgaattctttggtgttcgcaaaccaggtagagttccatggttttacaatacccaggcgaataccattaggatgtactttctgacccattgctagtctccagagtctcagcgatcggacacaaccacagtgatgtggctggtgcgcttcaggatgcgatctgcacgaccttttgcacgcggcataatgcgcttcatgctcgggccttcgtctacgaaaattttcgtaactttcagatcgtcaatgtcagcgccatcgttgtgttcagcgttagcaatggcagattccagaactttcttgaccagtacagccgctttcttgttggtgtaggtcaaaatatccagagcctgcgacactttcttaccgcgaatcaggtcagcaacaaggcgaaccttctgagcagaagaacgagcatggcgatgtttagcgatagtttccatctcttcctcctaccttatttcttcttcgcttttttatcagcagcgtggccgcgataagtacgagtcggtgcgaattcacccagtttgtgaccaaccatttcgtcggttacaaataccggaacgtgctgacgaccattatggacagcgatggtcaaaccgatcatgttaggaaagatcgttgaacgacgggaccaagtgcgcaggggcttcttgtctccgctttccaccgctttctctaccttcttcagcaagtgcaggtcaataaaaggacctttcttgagagaacgtggcatggcttatcctctaaaattatttgctacggcgacgtacgatgaatttatcagtacgcttgttgctgcgggtcttcttacctttggtctgaacgccccacggagttaccgggtgcttaccaaagttacgaccttcaccaccaccatgtgggtggtctaccgggttcatcgcggtaccgcgaacggtcggacgaacaccacgccagcgtgcagcacctgctttacccagaacgcgcagcatatgctcagcattgccaacttcgcccagagttgcacggcagtctgcttctactttacgcatttcaccagaacgcagacgcagggtgacataagcaccatcacgagcaacgatctgaacgtaagtaccagcggaacgtgccagctgaccgcctttacctggtttcatttctacgttatgaacagtagaaccaaccgggatgttgcgcatcggcagggtgttacctggtttgattgcagcatcaacgccagactgaatctggtcgccagctttcaggcctttaggggccaggatgtaacggcgttcaccgtctttgtacagaaccagcgcgatgttcgcggaacggttcggatcgtactcaagacgttcaacaactgccgggataccgtctttgttgcgtttgaagtcaacaatacggtaagcctgcttgtggccaccaccgatatgacgagtggtgatacggccattgttgttacgaccaccggatttgctgtttttttccagcaacggagcaaaaggtttgcccttgtgcagctcagggttaaccactttaactacgtggcgacgacccggagatgtcggtttacatttaacaactgccattgtattactcctccgacttactcagcgccgccaacgaagtccagattctggccttctttcagggtgacgtaagcttttttccagtcgctacgacgaccgatacgctgtccgtgacgtttaactttccctttaactaccagggtgttaacgacttcgacttcgacttcaaacagtttctgcacagcagctttgatttctgctttggtcgcgtctttagcaactttgagtacgatggtgttggatttttccatcgcagtagacgctttttcagaaacgtgcggtgcacgcagcaccttcagcagacgttcttcacgaatcatgccagcatctcctcaacttgcttaacagcatcagcagtcattacgactttgtcgaaggcgatcaggctaaccgggtcgataccagttgcatcgcgtacgtcaaccttgtgcaggttgcgcgcagccaggaacaggttttcgtccagctcaccggtgatgatcagcacatcttccagagccatgtctttcagtttctgtgccagcagcttagttttcggcgcttctacagagaacttctcgacaacgatcagacgatcctgacgtaccagttcggacaggatgcttttcagcgcgccgcggtacatcttcttgttaactttttgactgtggtcctgcggacgagcagcaaaggtcacgccaccagaacgccagatcgggctcttgatagaaccagaacgcgcacggccggtgcctttctggcgccacggttttttaccggaaccagttacttcagcacgagtcttctgagcacgagtaccctgacgagcaccagctgcataagcaacaacaacctggtgaaccagcgcttcgttgaaatcacgaccgaaggtagtttcggaaacagtcagcgcgctctgcgcgtctttcaatactaattccattgctatctccttacgccttcacagctggtttaacgatcaggtcgctaccggttgcacccgggacagcacctttaaccagcagcaggttgcgctcagcgtcaacgcgtactacgtcaaggctctgaacggttacacgttcgttacccatctgacctgccattttcttgcctttgaacactttgcccggagtctggttctgaccgatagaacccggaacgcggtgagacaaggagttaccgtgagtagcgtcctgggtacggaagttccagcgcttaacggtacctgcgaaacctttacctttagaggtgccagttacgtcaacttttttaacgtcagcaaacagttcaacgctaatgctctgacctacagtgaactcttcgccttcagccaggcggaattcccacagaccacggccagcttctacgccagctttagcgaagtggccagcttcaggcttggtcacacggttagcttttttagcaccggtggtcacctgaatagcacggtagccatcgttagccaggtctttaacctgagtaacgcggtttgcttcaacttcgattacggttactgggatagaaacgccgtcttctgtgaagatacgggtcatacccacttttttaccgactaaaccaatcattgtttcaacctctcaatcgctcaatgacctgattaacccaggctgatctgcacgtctacaccggcagccagatccagacgcatcagagcatcaacggttttctcggttggctcaacgatgtcaaccagacgcaagtgagtacggatttcgtactgatcgcgcgcgtctttgttgacgtgcggggagatcagaacagtgaagcgctctttgcgtgtcggcagcgggatcggaccacggacctgcgcaccagtgcgcttggcagtctcgacgatttccgcggttgcttgatcgatcagacgatgatcaaacgctttcaggcggatacggattctttggttctgcatgagaccagagctccaattattttataaacgaaaatgattactcctcagacccattacgattgatgggagagtgtaaccgttcttacgtagctccccgattgggagcattgttaggtagccaaattcggctaactgaggttcagattgaacctgctgtcaactacgacaagcccgcgcattatacatacttaaccaccgaacgcaagcgtattgctagtaaagtaaacagccttcgggttatctctcaagttcgttcagtgcatttttgacacgctctcttaaaccggctttctcttcgctttcttccacagtattttcttcgtcttcagaagaagagggggcattctcaaccgcgacgcctgggtcatcttcctcctcgacggattcgacgacggggagtggctgttttttgaagaaatagtgttgtgttgattgtttaaaagcgggcgtttcagcctctacagtgacttcggcttttactatccaaagcacccatagctgcctggcatacccaccaaccagcaccattcctgcaaaccacaggcaaatcagtaataaacaaattacatatattatggtgctgtgtttttgtcgggagaagataccagggtgacctgtttctttctgctcacgcgcggcgatatagaattcaaacatgtcatttccccttcactgttgtttccggggaaatatttgcttcatcccgatataagtaggcactctcccctgccacctgccagagatgtactaacgttgaaaagccaacaacaccgtcagttttcaagtggtggcttttttgaaattgctttattttttctaccaacaagggacgccactccgccgaaggttctgtcgaaatatgcaatgcgcggtttaacatcgtttccagccagagaatctcttcctcgctgctatcacgcgtaatggtactctccccttccggcgacattttccacaacagaagataatcacccgtccataccgactcaaaccatttatgtgtcagcgtccacgtttgctgacctacgaggacatcaacgctagcctcaccgacgcgaacgaccacaacaggcaattttttgtccccgactttaagcgatgcgatccagggcaaattctgatctaccaatgtttgtaaagaagcattcccacttttacatgccagccccgctcttactgcctgatcgcaccaggccgaatcagctgggacctcgtacccccatacgccgtataacacgcttagcgcctcactatcgcgcatcaccacatgagcaatatccttagtcatatcttgtttaactactggcgttacgggtatcagccacgcaggaacgggtaacgtagctgtaaaagaggacagcagtagccaaccacaggtaagagcgataatggttccactcatcaccacggcaagctgcattttccgggggcggttatcacccaatatgcggtaaatcattcgccattgttttgctgtgaaaacgctggtctgctcggcttgctgtaataagcgaattgtttcgccggcaagcgccagctttctgcgatcgccccgacataataaagctatccgtttcagaactctggcggttaaaaggagatcgggttggtcaatattctgaccttcaaggatgcttgccttaagttcgtgctccgtcagacgtcctatcgagacaagttcaatgccctgttttttaaaatcacgttcgacttttcgatcgggtctgccgatcagcaaaaattgaccgtcaggaataagagatattgcgcgttggagatcatcaagtatgcggcggtgattcaggtgagcattttcaataataataagagggcagcgactatcagttcgatgaagcgcatgcagtaattgccccgccatctcatctcgcgtccaggcgctgtcacggcagccctgttcagccgcgttatcgtcggtaacgatccatgcggccttaccttgccaggaaacaacgaggcttaaagtaatcacacggcgatgtttatctttttgcagttgctgcgccagccaggtttttccacttccagcctcacccaacaaatagcatagacgccaggtttgacgtttctcacacaaccaggaaagaataacttctcttctcgtagacatagaacttcctgttttaattattgattatccttaatcataaaaataatgtatgtatttattaattaaatacatattactaatataaataaattttgcttgattcatgcaagcggcattaatactatttatactaacgtcaatatacaacccacccaatctattttattagaacatacatcgtgcccacactacgtttccccttccatctggcgaatcataataaagatgctgccatcaatatattgattatatttataagcatagggtcgattatttttaatgtgaattatttccatacaactatagttaaaaatggacagatcattaatcaaccaacaaacgcatttcagtctgatttcagccttgccgctttatggcgtaacgaaaatcatgctggggtaaaagatgcaaatcccgtggcagttaatcaggaaacacctaagctctctatagcgcttaatggcattgtactcacatcgaatgatgagacttcttttgtcttaattaatgaggggagcgaacaaaagcgatactccctcaacgaagcccttgagtcagcgccgggaacgtttattagaaaaataaataaaaccagcgttgtgtttgaaactcacgggcattacgaaaaagtaactctccatccagggctacctgacatcatcaagcagcctgattcagaaagtcaaaatgtactcgctgattatattatcgccacgcctatacgtgatggagaacagatatacgggcttcgattgaaccctcgtaagggcctcaatgcatttaccaccagcttgctacaaccaggggatatcgccctcaggatcaataatctttcgctgacccaccctgatgaggtttcacaggcattaagtttactgctaactcaacaaagtgctcagtttacaattcgtcgcaacggcgtaccccgcttgataaatgtttccgtcggggaacttacaggaatgaatggactgcgtcatgaaaggactcaataaaatcacctgctgcttgctggcagcactactcatgccttgtgcaggacacgctgagaacgaacaatacggcgcgaacttcaataacgccgatatccgccagttcgtggaaatagtgggtcagcatcttggcaaaacgatcctgatcgacccttcggtacagggaaccatttccgtacgcagtaatgatacgtttagccaacaggagtactaccagttctttttaagtattcttgatctttacggttattccgtgatcacgctggacaatggttttctgaaagtggttcgctcagctaatgtaaaaacatcgccagggatgattgctgacagttctcgtccaggcgtaggtgatgagttggtcacccgaattgtaccgcttgagaacgttcctgctcgtgacctggcccccctgctccgccagatgatggatgcgggtagcgtcggtaatgttgtgcattatgaaccctccaacgttcttattctgaccggtcgtgcctccaccattaataaactgattgaagtcataaagcgcgttgatgtcatcggcacagagaagcagcaaattattcatctggaatatgcgtcagcggaagatctcgccgagattcttaatcaattaatcagcgaaagccacggtaaaagccagatgccagccctcctctccgcgaagattgtggcggataagcgaaccaactctcttatcatcagtggaccggaaaaagcacgccagcgcatcacttcattactgaaaagccttgatgtcgaagagagcgaggaaggaaatacccgggtttattacctgaaatatgctaaagccacgaatctggtggaagtgctaaccggtgtttccgaaaagctgaaagatgaaaaagggaatgcgcgtaagccctcctcttctggcgcgatggataacgtcgccattaccgccgatgaacagactaactctctggtcattaccgctgaccagtccgtccaggaaaaactcgccacggtaattgcgcgtctggacattcgccgtgcacaggtgctggttgaggcaatcatcgttgaagttcaggatggaaatggactaaacctcggcgtgcaatgggcgaataaaaacgttggcgcacagcaatttaccaataccggattaccgatttttaacgctgcgcaaggtgtggctgattataaaaagaatggtgggatcaccagcgcgaatcctgcctgggatatgtttagcgcctacaatggcatggccgcaggcttcttcaatggcgactggggagtactgcttaccgcgctggccagtaacaataaaaatgacatcctcgccaccccaagcatcgtaacgctggataataaactcgcgtccttcaacgtggggcaggatgtgccggtgctatccgggtcacagaccacttcaggggataacgtctttaataccgtcgaacgcaaaacggtggggacaaaactcaaagttactccgcaggtcaatgaaggcgacgcggtgttgctcgaaatagagcaggaagtctccagcgttgactcttcctctaactcgacgctcggcccgacgtttaatacccgtactattcaaaacgccgtgctggtcaaaaccggtgaaacggtggtcctgggcggattgctggatgatttttctaaagagcaagtgtcaaaggttcctctgcttggcgatattcctttagtggggcaactcttccgctatacctccaccgagcgcgctaaacgcaacctgatggtatttatccgtccgacgattatccgtgacgatgatgtttatcgctcactgtcaaaagagaaatacacccgttaccgtcaggagcaacaacagcggatcgacgggaaatcaaaagcgctggttggctcggaagatttgccggtgctggatgaaaacacgttcaacagtcacgcccctgcgccatcgtcacggtgaggcattcatatgagaattcactcaccgtaccccgccagttgggcgctggcacaacgaattggttatctctattcagagggcgagattatttatctcgccgatacgccattcgagcggttactcgatattcaacgtcaggttggccagtgccagaccatgaccagcttgtcacaggctgattttgaagctcggctggaagcggtattccatcagaataccggtgagtcgcaacagattgcgcaggatatcgatcaatccgtcgatcttctctcgctttcggaagagatgcccgcaaatgaagatctcctgaatgaagattcagcggcaccggttatccgcttgatcaatgcgattttgagtgaggccatcaaagaaaccgcctctgatatccacattgaaacctatgaaaaaacaatgtcgatccgttttcgcatcgacggcgttttgcggacaattttacagccaaacaaaaaactggcggcactgcttatctcccgaattaaggtcatggctcgtcttgatatcgccgaaaaacgtattccacaggatggaagaattagtttgcgtatcgggcgacgtaacatagatgtccgcgtatccacactgccgtccatctatggtgaacgcgccgtactccgcctgctggataaaaacagcctccagctttcattgaacaacctggggatgacggcagcggataagcaggatttagaaaatctcattcagcttccgcacggtattatcctggtgacagggccgacaggctccggtaaaagcaccacgctctacgccatcctttcggcgctgaatactcccggccgcaatattctgacggtagaagatcccgtggaatatgagctggaaggcattgggcaaacgcaggtgaatacccgtgtggatatgtctttcgctcgcggcctgcgcgccatacttcgccaggacccggatgtcgtcatggtgggggaaattcgtgatacagaaaccgcgcagattgcggttcaggcctcgctcaccggccatctggtactctcaacactccacactaacagtgcatcaggcgcagtgacccggctccgcgacatgggcgtcgaatcattcctgctttcgtcttccctggcagggattatcgcgcaacgtctggttcgtcgcctgtgtccgcaatgccgacaattcacgcccgtatcaccccaacaagcgcagatgtttaaatatcatcagctcgcggtgacaacaattggcactcccgtaggctgccctcattgccatcaatccggctatcaggggcgcatggcgatccacgaaatgatggtggtgacgccggaattacgggccgctattcatgaaaatgtggatgaacaagcactggagcgactagtccggcaacaacacaaggccttaatcaaaaatggcctgcaaaaagtgataagcggtgacacctcctgggatgaggttatgcgcgtcgccagtgccacgctggagagcgaagcatgaattatcgctatcgcgccatgacccaggatggtcaaaaattgcaagggatcattgatgctaacgatgaacgtcaggcacgactgcggctgcgtgaagaagggcttttcctgctggatattcgcccccaaaaaagttcgggagtaaaaacacgtcgcccgaggatcagccatagtgaactgacgcttttcacccggcagttggcaaccttaagcgcagcggcattacccctggaagagagccttgccgtaatcggtcaacaaagcagtaataaacgactgggtgacgtgttaaatcaggtacgcagcgccatccttgaagggcatcccctttccgatgcattacagcattttcccacgcttttcgattcgctctatcgtaccctggtaaaagcgggcgaaaagagcgggctgctggccccggtgttggaaaagctggctgattacaatgaaaaccggcagaaaatccgcagcaagctcattcagtcactgatctacccctgtatgctcactacggtggcgattggggtcgtgattattctcctcactgctgtcgtgcccaaaattaccgaacagttcgtgcatatgaagcagcaactgccgctgagtacacgcattcttttaggtctgagcgacacgttgcaacgtaccggcccgacattattagcgacagtgtttattgtcgctgtaggtttctggctctggttaaaacgcggcaataaccgccaccgttttcatgccatgttgctgcgcgttgcgctcatcggcccgctgatttgcgccattaacagcgcacgctatctccgcactttaagtattttgcaatccagcggcgtccctctgctggatgggatgaatttgtccaccgaaagcctcaacaacctcgaaattcgccagcgtctggcaaatgcggcagagaacgttcgccagggtaacagcattcatctttcgctggaacaaaccgcaattttcccgccgatgatgctctacatggtggcctctggcgaaaaaagcgggcagctcggcacattaatggtcagagccgcagataaccaggagacactccaacaaaatcggatcgccttaacgctctccatcttcgagccagcactcattattacgatggcactgatcgtcctgtttattgtcgtgtcggtactccaacctcttcttcaacttaactcaatgattaattaaggaaagcatatgcgcgcaacggataagcaacgcggttttacattactggaaattatggtggtgatcgtcattatcggcgtacttgccagcctggtggttcctaacctaatgggcaataaagaaaaggcggataagcaaaaagccgtcagcgatattgtggcgctggaaaacgcccttgatatgtacaaactcgacaatcatcactatccaaccacaaatcaggggcttgaatccttagtagaagcgccgacactgccaccgctggccgcaaactataacaaggaaggttatatcaagcgtctgcctgccgatccctggggcaatgattatgtcctcgttaatcctggtgaacatggtgcatacgatctgctttcagcagggcccgatggtgaaatgggaaccgaggacgacatcaccaactggggtttgagcaagaagaaaaagtaagtcagcgatgaatcagcaacgcgggtttaccctgctggagatgatgctggtgctggcgctggtcgctatcacggcaagcgtggtgctcttcacatatggccgggaggatgtcgccagcactcgtgcgcgcgaaacagcggcgcggtttaccgctgcacttgaattagccatcgaccgcgccacgctcagtggtcagcctgtcggtatccatttctctgattcagcatggcgcattatggtaccgggcaaaacaccatcagcctggcgctgggttccattacaagaagatgccgcagacgagagccaaaatgactgggatgaagaactctcaattcatcttcagccatttaaacctgatgacagcaaccagccacaggttgtgattctggccgacggacaaatcacgcccttctctttgttgatggctaacgccgggaccggtgagccgctcctgacgttagtctgttcaggctcatggcccctggatcaaacgctcgccagagatacccgcccatgaacaaacaatcagggatgacactgcttgaagtcttactggcgatgagtattttcaccgctgttgctctgactttaatgagcagtatgcaagggcaacgaaatgccatcgagcgaatgcgtaacgagacgctggcattgtggatagcggataaccagcttcagtcacaagattcattcggcgaggaaaacacgtccagttctggcaaagagttaataaatggcgaagagtggaactggcgcagcgatatccactcaagcaaagacggcacgcttctggaacgcaccataacggtgacattacccagcggtcagacaacctcgcttacgcgttatcaaagcatcgataataaatccgggcaggcacaagatgattaatcgccagcagggtttcacattgctggaggtcatggcggcgctggcgattttctcaatgcttagcgtgctggcgtttatgattttttcgcaagcttccgagttgcatcaacgctcacagaaagaaatccagcagttcaatcagctacagcgcaccatcaccattcttgataacgatctcctgcaactggtcgcccggaggaatcggagtacggacaaaatcatggtgttgggtgaagaagctatttttaccacgcaaagtcgcgatccgctggctcctctcagtgaagcacaaaccttactcactgttcactggtatctgcgaaatcatacgctctaccgtgctgttcgtacttctgtggatggcaggaaggatcaacccgcccaggcgatgctggaacatgtcgagagctttcttctggaaagtaacagcggggaaagccaggaacttcctctctcagtcacgttacatctgcagactcagcaatatggggggttacagcgccgttttgcattacctgagcagttagcgagagaagagtcgccagctcagacgcaggccgggaataataaccatgaataatgaacaacgcggcgtcgcgctgctcattgtactcatgttactggcgctcatggctgctctggcagcagacatgacgctcagttttcacagccagcttcagcgaacccgccaggtaaaccatcatctgcaacggcaatatgatattgaactggcggagaaacttgcgcttgccagcctcacccaggacgttaaagataacgacagacagaccacgttgcagcagtactgggcacagccacaacagttgcagctggaagatggcaatacagtgaagtggcagttacgcgatgcccagcactgttttaatctcaatgcgttagcaaaaatctctgacgacccgctggcttcccctgatttccccgcccaggtattcagtgcgctgctgattaacgccggtatcgatcgcggaaacaccgatgagatcgtgcaatcaatcgctgactatattgatgtcgatgactcaccacgctttcacggcgcagaagatagcttttaccaaagccagacgccgccccggcatagtgccaatcagatgctttttctgactggcgaattacgtcagataaaaggcataaccgaaaacatctatcagcggcttatcccgtatgtctgcgttctcccgaccacggaacttagcatcaatcttaatatgctaacggagaacgatattccgctcttcagagcgttattcctcaataacatcacggatgctgacgctcgggtcttattgcaaaaaaggccgagggaaggctggctaaccacggatgcatttctttactgggcgcagcaggatttctccggtgtgaagccactggttgctcaggtgaaaaggcatctctttccctatagccgctattttacgctgagtacggaaagtatcagcgacgaacaatcccagggatggcaaagccatatttttttcaaccgtaaacagcagagcgcccaaatctatcggcgtacgctgcaactctactaatcataaggatcgtgatgcctgaatcgttgatggtcatacgttcttcctcgacgctgcgtaagcattgggaatggatgacgttctccgcagatagcgtatcttcggtacatacgctcacggacgatcttccgctggagtcgctggccgatcagcccggtgccggaaatgttcatcttttgatcccaccagagggccttttatatcgttccctcacgctgcccaacgccaaatacaaactcaccgcacaaacattacaatggctggcagaggagacgttacccgacaacacccaggactggcactggacggttgtcgataaacaaaacgaaagtgtcgaggtgataggcattcagtcggagaaactcagtcgctatcttgagcgtttacatactgccggactcaacgtgacgcgggttttgccagatggctgctatcttccctgggaagtagatagctggactctggttaaccagcaaacaagctggctcattcgcagtgccgcacatgccttcaacgaactggatgaacactggttacagcatcttgctgcccagtttccgcctgagaatatgctttgttatggtgtagtacctcacggcgttgcagcggccaatccacttatccagcatcctgaaataccatcactgagtttgtattctgccgatattgcattccagcgctatgacatgctgcatggtatttttcgtaaacagaaaactgtaagcaaatcgggaaaatggctcgcccgcctggcagtaagctgtctcgttctcgccattctttcttttgttggcagccggagcatcgcgctctggcatacgcttaagattgaagatcaacttcagcaacaacagcaagaaacctggcaacgttatttcccgcagatcaaacgcacccacaattttcgtttttactttaagcagcaactcgctcagcaatatcctgaagctgtgccgttgctctatcatttacaaacacttctgctggaacaccctgaactgcagttaatggaggcgaactatagccagaagcaaaagtcgctgaccttaaaaatgagtgctaagagtgaagctaatatcgatcgtttctgtgagttaacacagtcctggcttccgatggaaaaaacagaaaaagatccggtcagtggtgtatggacagtaaggaactcagggaaatgattaaatcatggtgggcagaaaaatccacatcggaaaaacagatcgttgcggcactggcggttctctcgctcggcgttttttgttggcttggggtgataaaaccgatagatacctacattgcagagcatcagtcccacgcgcaaaaaattaagaaggacatcaaatggatgcaggatcaagcgagcacccatggtttactcggtcatcctgcgcttacgcagcccatcaaaaatatccttctcgaggaagcaaaacgtgagaatttggctatcacgctggaaaacggcccggacaatactctgacaattcatcctgtcacagctcccctcgaaaacgtctcccgctggctcactacggcacaggtaacatacggtattgttattgaagaccttcagtttactcttgccggaaacgaagagatcaccctcaggcatttgtccttcagggagcaacaataatgacaatgctactgccgctcttcattctggttggttttattgcagattattttgttaatgccatcgcctatcacctctcgccgttggaggataaaacggcgttaacgtttcgccaggtattggttcatttcaggcaaaaaaaatatgcctggcatgatacagtgcccctgatactttgtgttgctgctgctatcgcctgcgccctggcacctttcacgcccatcgtgactggcgcactctttctctatttctgtttcgtactcacgctcagtgttattgattttcgcactcagctcctgcccgacaaactcaccttaccgctgctctggcttggcttggtatttaatgcgcagtatggattaattgatttacatgatgcggtttacggcgcggtagcgggctatggggtgctgtggtgtgtttactggggcgtctggttagtttgtcacaaagagggattgggctacggtgatttcaagctactggccgctgcaggcgcatggtgtggctggcaaacgttgccaatgatactgctgattgcctcgctgggtggcattggttacgccatcgtttcacaacttctgcaacgccggactataaccactatcgcattcggcccgtggcttgcgctcggcagcatgataaacctggggtatctggcctggatctcttattaaccgggagggttctccctcccgacacggctcaaccttcttcgcggatctgtgcttgcagataattttgcaggcccatcttctgaatcagatcaagttccgtttccagccagtcgatatggccttcttcatcacgcaaaatttctatcatcatatcgcggctgacgtaatcatgaacgctatcggcataaccaattgcctcacgcaaattcttcgcgccatccagctcaagtgccagatcagaacgcagcatttcctcaacatcttcaccaatgttcagtttgcccaggtcctgtaagtttggaagaccttccagaaaaagaatgcgctcaatataacgatcggcgtgtttcatctcatcaatggattcatgatactccacatcattgagacgtttgagaccccagtttttaaacattcgggcatggagaaagtactgattgattgcgacaagctcatttcccaacagtttgttgagataatttataactttagtatcacctttcattttttgactccttcgcttccactctttgaagagtagaacggcttacgagtaagtcaaaaaacacactccgtttatgcggactccttaaactccggcagctgcattaattcatcctccatcacttcacgcgcggcccggacacatttaccgcactgattgccgaccggaataaatttttttaattgctggaacgagtgaggggaaaactggcgcacagcctgacgaatttttttatcgctgataccattacaaagacaaacgtacatagagactcccgtatactttcttcaaaaataaatgaaaatagttcttatttcaattacggaaagactcttttttaagcaaagaatagaaatatgaataaaaataatgggctaccaaaagtagcccattgacaaaaaatgcggcgatactggaaggtatcgccaacacatttattgcttagtaaacggcgcgaagatttcgctaaatgcgtacttcggtgcctgttctttagtcaggccgtggaattccggagacaggttagtgccgcccggcaggtcgcgcgcgattgaccagataccaaccataccgagattacgcttctgcgcatcctgcatgaccagacgagcatcagagagatagaacacctcgccctgaacgtcgttcacgccaaccatcggcgtggtacccatcatagcgtcaatttctgcatcgctcttattgggatggaggcctttcaattgtgaatgcaggttggcaatcgcagacgttgcacacttaccgtgaatgttctggccttcggtatttgcagactgacaaatcgcgttaccgtagtccattgtcatcacgttcacacccgccagctcaacacctttcgctttggcatcgctcaggacattcatcccttccggcgtcaggccagtcggcagaattggcaaggtgtaccagatagcaatatctttgccttctgacttccatttatcctgcactttcttcacagcaaggttacgacgttcaatagatgcctgatccgcaacccaggtgccttcgatatcgaagtccaggactttgaggttcaggttatcaacgatgtcataataatgctgcatcagatcgtctacgttcttacaggaagcagccagcggagcgttgttagcaccaccgatagacagcatcacatcgccgccagcctcacgcagagctttgattttgctgtactgagcgtaattctgcataccgtaagcggtaccccatgtcggcagacaggtgttcgcatctttactcaccacaaacgccagcgtgaagtggttgacgttatgattcttagccagcgcagccagatccgggatcgtattcagcgtaaagtcgacatacggtgcataaacgtgtttcggccacgctttcttcggcgtacctacgcgctctttggttccggtccagtcaacaaaaacacgccacgggttgctgtcagaaggagaaactttctgcactttactctgagaaatgtagttcacaccgttaaagcgaatcagcgtatcgctggcataaagcgtttctggattaaactgcggcgcattattcagctcttcgttgctatagctctgagccttacctaacggcttccacgggcggctattgctaccggtggcgttttggttcgccaccagagcagggttgtcactttgcgtccagaacagcgcttcataagcctgcccatcaacaacaacgcgatcacctttcacgtacacagtggatgcggaccatgctttcgccggttcgtatttcttccacgggttatcgccgcccgggacaaagccccatgcgtcttgatcgacagaagttttataatgtgcatcgttataatctacgatgctgtccgcgctgtacgctttgctggcctggaaaccatccgcaacaatgacgccgccgttatcaatttcacaggtagtcgggttaccgtactgactcaattccgcagcggtagctgtacgctcgagacgccatgggttattggagttttcagcgctggtaccccgtgggcaatctttagacccaacccaccaggcgttcttgtaaacattaccattgaaaataacatggtaaatttcgctaccttcctggccgctccacgcttgcaatgagtaatcgttaacgctatccgctggtgttgatggctcgctgttatccggagttggggtcaccggtgtttccggagttggatcaaccggagtcacagcaccgccattattatccggcttaacggaacaggagccagggttaccatactggctgatttctgttgccgttgccgcgcgaacataacgccatgggttactggcatcgttttctttcgcatcgcctgggcaatttgccgcgcctacccaccaggcgttcttataaatgccgccgttatagataacgtaccatgtagaagaaccttcctgacctttccaggctactacagcatagttgtcgtttgacttatcagctggggctggctgaacatcaggagccggtttaacgtccggtgccggtttcacatccggtgaaggctgtggtgctgaagtacaggactgtggattactggtttctgagatttccgttgccgtagcggcacgaacataacgccatgggttgctggcatcattgcttttcgcatcacccggacagttagaagaggctacccaccaggcatttttatataccgcaccattaaagacgacataccaggtctgaccgccctgctgtttattccaggcaactacagaagaattagacggaacagtgccctgtgctggtgtagccgaaccgccattagccggcgtattggatgcaggcgtatttgaatttgaagaagatgagctgccgctcttttcgcaggaaagtgtattgccaaactgactaatttcagcagctgttgcggtacgctttaaacgccacgggttagttgcatcatttgctttcgcttttcccgggcaatttgtagaagaaacccaccaggcattttcataaattttgccatcgaaaataacctgatatttattaccaccttgttggttattccatgcttccattgccaatgctggcagagcggaacacaccagccccataccaatcatagatttagtaaatatatttaatttcattataatcccttgtgacgtaaaaactgcaaaacaaaagtcctacgcaggaattatttacgttttacgagaacccttcaatatgaattaaattacggcattaaaaataagaaaaaagcctgacaaatgaagcattttaaaaacagaaacattcatatttaaaatgttaaattgaattgatattttaaatatgaataatttattcgttctgacagtacgaataagatatgccgtcaacaaatgcaaaaagggcgccgaagcgcccttttcaattcaaaactaattaacgtgtaattagcccagaactttagcaacaacgcccgcgccaacggtacggccgccttcacggattgcgaaacgcagaccgtcgtccatcgcgatcgggtggatcagggtaacaaccattttgatgttgtcgcccggcattaccatctctacgccttccggcagttcgatggtaccagtcacgtcagtagtacggaagtagaactgcggacggtagcctttgaagaacggagtatgacggccgccttcatctttggacagaatgtacacttcagattcgaacttggtgtgcggcttgatggtgcccggcttagccagtacctgaccacgttcgatttcttcacgtttgataccacgcagcagaacacctacgttctcaccagcacggccttcgtccagcagtttgcggaacatttcaacgccagtacaggtagacttctgagtctctttgataccaacgatttcaacttcttcaccaactttgatgataccgcgttctacacgaccggtaacaacggtaccacgaccggagatggagaatacgtcttcgatcggcagcaggaacggcttgtcaatcgcacgctctggttccggaatataagaatccaggaagccagccagttccaggattttcgcttcccactctgcgtcgccttccagcgctttcagagcagaaccacgaacgatcggagtgtcgtcgcccgggaagtcgtactgagacagaagttcacgaacttccatttcaaccagttccagcagctcttcgtcatcaaccatgtcgcatttgttcaggaacacgatgatgtacggaacgcctacctgacgacccagcaggatgtgctcacgagtctgcggcatcgggccgtcagtcgcagcaactaccaggatcgcgccgtccatctgagcagcaccggtgatcatgtttttaacatagtcggcgtgccccgggcagtctacgtgtgcgtagtgacgggtcggggtgtcgtattcaacgtgagaagtgttgatggtgataccacgagctttttcttccggcgcgttatcgatctggtcgaatgcacgagcagcaccgccgtaggttttagccagtacggtggtgattgcagcggtcagagtagttttaccgtggtcaacgtggccgatagtaccaacgttaacgtgcggttttgtacgttcaaatttttctttagacacggctatattccttactatagtgctctccccttcaggagagagcacgggactttggtattaacccttaggcttatttaccacgggcttcaattacggcctgagcaacgttactcggcgcttcatcatacttcaggaattccatagtgtatgatgcacgacctttggtcagagaacgcagctgagttgcgtatccgaacatttcagacagcggtacttcagcgtggatcttaacgccagtaacttcagattcctgacctttgagcataccacgacgacggctcaagtcaccgataacgtcaccggtgttctcttccggagtttctacttcaaccttcatgatcggctcaagcagaactggtttcgctttcttaaagccttctttaaaggcgatagaagcagccagtttaaacgccagttcagaggagtcaacgtcatggtaagaaccgaagtgcagacgaatacccatgtctactaccgggtagcctgccagcggacctgctttcagctgttcctggatacctttatcaacggccgggatgtattcgccagggattacaccacctttaatgtcgttgatgaactcgtagcctttcgggtttgaacccggctccagcgggtacatgtcgataacaacatgaccatactgaccacgaccaccagactgtttcgcgtgtttaccttcaacatcggtaactttctggcggatagtttcacggtaagcaacctgcggtttacctacgttcgcttcaacgttgaattcacgcttcatacggtcaacgatgatgtcgaggtgcagttcgcccatacccgcgatgatggtctggttagattcttcgtcagtccatacacggaaagacgggtcttctttagccagacggcccagagccagacccattttttcctggtcagctttggttttcggttcaactgcgatggagattaccggctcagggaattccatacgttccagaatgatcggcgcatccgggtcacacagggtgtcaccagtggttacgtctttcagaccgatagcagcagcgatgtcgcccgcgcgaacttctttgatctcttcacgtttgttagcgtgcatctgaacgatacgaccgaaacgctcacgtgcagctttcacggagttcagtacggtatcaccagagttaaccacaccggagtaaacacggaagaaggtcaggttaccaacaaacgggtcggtagcgattttgaacgccagtgcagagaacggctcgtcatcacttgcgtgacgttcagccggagtgtctttaccgtcgtccaggataccgttgatcgcaggtacgtcaaccggggatggcaggtaatcaattaccgcatccagcatcgcctgaacacctttgttcttgaacgcagaaccacaggttaccaggatgatttcgttgttcagaacgcgctgacgcagagcacctttgatttctgcttcagtcagttcttcaccacccaggtatttttccatcagctcttcagaagcttcagctgcggattcgatcaggttctggtgccattcgttagccagttcaaccatgtctgccgggatatcttcgtattcgaaggttacgccctggtcagcgtcgttccagttgatagctttcattttcaccaggtcaacaacaccggtgaaatgttcttcagcaccaatcgccagctgcagcggaaccgggttcgcgcccagacgggttttgatctggttaacaactttcaggaagttcgcacccatgcggtccattttgttaacgaacgcaatgcgcggaactttatatttgtttgcctgacgccatacggtttcagactgcggctgaacaccaccaactgcgcagtaaaccattaccgcaccatcgagaacacgcatggaacgttctacttcgattgtgaagtcaacgtgccccggggtgtcgatgatgttgatgcgatgcggctcatactgcttagccataccagaccagaatgcagtagtcgcagcggaagtgatggtaataccacgttcctgctcctgctccatccagtccatggttgcagcgccgtcatgaacttcaccgattttatggtttacaccggtgtagaacagaatacgttcggtagtagtggttttaccggcgtcgatgtgcgcactgataccgatgttacggtagcgtgcgatgggtgttgtacgagccatttgtttcctcgtttatcttttaggcgttcaatttaagtagcccaaagcgggctgcttactggaagcgcccgcctggtgactaaaactccgaagggataaccaacggtagtgtgcgaacgccttgttggcttcggccatacggtgaacgtcttcacgtttcttaactgcagtacctttgttttctgcagcatcagaaagttcgttcgccaggcgcagagccatggatttatcaccgcgtttacgagcagcttcaacgatccaacgcattgccagagcattacgacgaaccggacggacttcaactggtacctgataagtagaaccaccaacgcggcgagacttaacttctacagtcgggcgcacgttttcgagagctacttcgaatgcttccagttcagatttaccagagcgctgagccagggtctccagcgcgctgtatacgatagattcagcagtagattttttaccatctaccatcaggatatttacaaatttagccagcagttctgatccgaacttcggatccggcagaattttacgctgaccaatgacgcgacgacgtggcatggaaatactccgttgttaattcaggattgtccaaaactctacgagtttagtttgacatttaagttaaaacgtttggccttacttaacggagaaccattaagccttaggacgcttcacgccatacttggaacgagcctgcttacggtctttaacgccggagcagtcaagcgcaccacgtacggtgtggtaacgaacacccgggaggtctttaacacgaccgccacggatcaggatcacggagtgctcctgcaggttgtgaccttcaccaccgatgtaggaagtcacttcgaaaccgttagtcagacgaacacggcatactttacgcagcgcggagttcggttttttaggagtggtagtatatacacgagtacatacgccacgtttttgcgggcatgcttccagcgcaggcacgttgcttttcgcaactttgcgagcacgtggtttgcgtaccagctggttaactgttgccattaaatagctcctggttttagcttttgcttcgtaaacacgtaataaaacgtcctcacacaatatgaggacgccgaattttagggcgatgccgaaaaggtgtcaagaaatatacaacgatcccgccatcaccaggccatctggctggggtgcttaaccgtaagtctgacgaaatcagtatagtcaatgagaatgatgtcgttcgaaatttgaccagtcaaaccgcgggcaataaggtcttcgttcagggcatagaccttaatgggggcattacgcagactttcaaggtagcggttaccgtcaactgcggcagttacgccatcttgcaataatagcagttcgtctccttcactgagcagacgcagcagcgcagcaaaatccgtcagccagggtgagcgatgtaatgtgtgcagcataaacgcctcaaaacctcaaaataacatcgtagttggcgagttcgcggcgtaaggcatctgcttcgagcggcgtggcttcgacaacaaagggtgtctgcggatctaacccgcgttcgcgcagtgaagccgcacaaacccagcactgttcaatgtcgtacagacccaacaatttaaaagtggcaatgtaatcacgcgccagcactgcatcgggcttttgtcctggcagcagctgaaaaacgccatcagctataaagaagacagccagatcgtcagttaatgcggaagttgccagtaaagcatctaaaccttcccggcctgcggctgtaccatgaggtgcagtagaaaaaacaaacgcaattcgtttcatcagaactgtaccaccctgtcacaggtcagcgaggcttccgccagcgccccaagtccgcttaaggtaaatccctgctgaaggtttgacgaagccagccccagtcttccggcctccgtttcatcaacaacgccacggcgtaatgctgccgctacgcagatattcagcgccacaccatgttgcgcattcagttgttgccaggcccgtacgaggtcaaattcgtcacttgccggagaggtcaattggttagcgttatagaccccttcccgatagaaaaagacgctgcttaactcatggccatctgctatcagcgcctgcgcaaactgaaaagcactactcgcctgttgcgtaccgtatgctggcccggtcaccacgatggcaaaacgcattacttatcttgcccctggaaatcaccgctcttgaactggcggatgtagagatagacagtgtgtttggagatgttcaggcggtcagcaacctggttgatcgcatctttaatatcgaagatccctttctcgtagagattcagcacgatctgacgatttttggcgttattagaaacattgcgatcggcattcacttcttcgatggtgaactccagcgtttgggtaaccagatcttcaacagaagaggcaaagttgacgcttgaaccgacatccggggtttctggcggcacaaaggtgctcataatctgcgagaagggaacatcaagattcatattgatgcacagcagaccaattacacgctgttcgcggttacgaatcgcgatagtcagggacttcattaatacgccgcttttggcgcgagtaaagtagcatttagaaacgctgctatccgctcccgtcatatcgtgcagcatacgtagcgccaggtcagtaattggcgaaccaatcttccggcctgtatgttcaccgttagcaatgcgaatggctgaacattttagatcctgcaaagagtgcaaaacgatttcacagtgggagccaataagcatcgctaacccgtccaccaccgcttcgtaggatttcagaatatcaaaatcggtctggtcgaaaggacgttgatccagtaaatccaactcactggtttcgttggttaaaagcgacctggacatgaaaaaaaacactccttttcaggagcctgtcgttaacttttcagggcaggctcattaatgatgcgggtaactaaattaatacagcggaggttccgctttccagcactaattatatccggcctgtaataaaaaaaccgccgcctggtcaggcggcggttcttaatgcttattttttagcagaatctgcggctttcgcatcagcttccggctttgcatcagccttcggcgctggtttcacatccagcagctctacgtcaaacaccagggtagaattcggtgggatccccggaacacccgctttgccgtaagccagttctggtggaataaccagtttgatcttaccgcctttcttgatgttcttcagaccttctgtccaacccgggataacaccgtccagacggaaagaaagcggttcaccacgggtgtaagagttgtcgaactctttaccgtcgatcagcgtacctttgtagttcactacaacagtatcgctgtctttcggtgcttcgcctttaccggcttctactacctgataaaccagaccagttgaagaggttttcacacctttctctttggcaaatttctcgcggtactctttaccttttgcttcgttatcagccgcgtctttttccatcttcgcctgagcagaagacttcacgcgagcttcgaatgcttgtagagtctgttcgatctcttggtcggagagtttgctcttatcagcaaatgcatcctgaacaccagcgatcagctgatctttatccagtttgatgcccagtttttcttgttcttttagagagttttccatgtaacgacccagcgaggcacccagtgcataagctgatttctgatcgtcatttttgaacgctgctttgctgtcagcagctgtagcaggttttgcagcttcagcagcaaaagtgattggtgcatgcagggcaacggccattgtggtcgccagcagcgttactttaaacagtgatttcatccatatctccaggatcggggcatctcaccccagggttaactattatcagaagggtactataaagcgttgtcgaacaaatctacatacagacacgccctattatcatctattttcagactctttttgtttaaattagtttcgatgaccgcgaaatgagtgctgtctcgggcagcaaagttaagtagaatccgcggcgaccattcgacaaaagaggtgaatcatgcaggatttatcattggaagcacgcctggcagagctggagagccgactggcttttcaggaaatcaccattgaagaactgaacgtcacggtgaccgctcatgaaatggagatggcgaaactgcgcgatcatctgcgtctgctgaccgagaagttaaaagccagccagccgtcgaacatcgcgtcgcaggctgaagaaacgccaccgccacattattgaggcgtaaaaaaagcggggattccccgcttttttgtcactttttcggtattagtggcaaccgcaaccgccgttgcctttaccgccacagcagccttcgccaccgtgttcatgaccgtgatcgtggccatgaccgccgcagcaaccgtcgtggtcgtgatcgtggtggtgatcgtgcgcgccgtgaacgtgaccatgagccagttcttcttcagtcgcttcgcgaatcgccacaacttcaacgttgaatttcaggttctgaccggccagcatgtggttaccatcaaccacgacgtgatcgtcttcaaccgcagtgatttcaaccggtaccggaccctggtcggtttcagccaggaaacgcatacctacctgcagttcatcaacgcccataaatacgtctttaggaacacgttgcaccaggttttcgtcgtactgaccgtaagcgtcgttcgcgccaacagcgacatcaaatttgtcgccaacttcatgaccttccagcgccgtttccaggccagagatcagggaaccgtgaccatgcaggtagtccagcggcgcactcaccggagactcatcaaccaacacaccgtcttctgtacgtacctgataggccaggctgaccaccaggtcttttgctactttcatgatatctcctgagcatgggaagaatagtggcgcagattgtagcggaattctgcagccgtgtactcactagcttaaaaaaactcggcgcatatcgctagtccggatgaaaaatcccgatcacttgctcatctttgcgaacgtgatcgcgggcttctttgtctgcttctcgcatctgatgtccgcacttaacacattcaacaatatcaatattattttcgcgccacatcgccattgaatcctgcgcctgacaggccgggcattttgcgcccgcaataaaacgttttcggattgccatctttaccctctactcaaattcatcccagccgtccagctggcgtcgttcttgttgcatttcacgctggaaaatctcttccagttcgcgtcgggcttccctggcgcgagaaatttgtacggtatcggcatgcattgggatgagctctcgcagcatccgcatatccaggcggcgaaaatgcagttgcgctcgctgtgcctgatgcggatgcatgccaagcgtgaccagcgtcttgcgccccagctctaacgcactggagaatgtttcacgggaaaactgcgtcacccctgcctgtaataactcatgcgcttccacacgtccgcgcgctcgcgcaagaatatgcaaatgcggaaagtgctgttggcatatttccaccagcttcatggtgtcttccggctcgttacaggtaatgacgatagactcagcggcctctgcacccgcagaacgtaaaagatcgacctgcgtggcgtcgccgtaataaactttgtagccgtatttacgcatcaggttaacggcgctgatatcccgctccagcacggtaatgcgcattttatttgccatcagcaaacgaccaatcacctgaccaaaacgcccgaagcccacgacaatgacctggggtttatcatcgttgacccacggtttttcgtcttcttcttccggtccgttaaactggcgggatagccatttatccaccagcttcatcagcaacggcgtggtcatcatggaaagcgtcaccgtcaccagcaacaacgccatctggtcgccctggaataagcgttgtgaagaagcggtagaaaagaggacaaaggcaaactcaccaccctgactcaacacgccagcaaactgcatccgctctgagctacgcacgccatacaatcgcgccagcagatacagcacgagaattttcaccgccaccagcacaaccacgcttatcactacccacaacagatgggtataaagcaccccgaggttgagtgacatgccgacagagataaagaacaaaccgagcagcaagcctttgaagggatcgatagccgtttccagttcatggcgatattcactttccgccagcagcacgcccgcaataaatgtaccgagcgccatcgacagccccagcgcatccataaacaatgcggaacccaacaccagcagcagcgtcgcggcggtgaacacttcccgcacgccagaagctgcaataaagcggaataccggacgcagtaaatagcgcccaccaatcagcatgccgacaaacgccagcaccttcatgccgaccttcatccagtcgaaatgttcgtctgccgaccccgccaacaacggcactaacgccagtgctgggattactgccagatcctgaaacagcagaaccgaaaacccgagctggccggattcgctgcgattcatccctttctcacgcatcaattgcaacgccattgcagttgaagacatcgcaaggccaatgccaccgaccaccgccgcctgccaggcgaaatccgtcagcatcaataatcccgccagcaacgccgcgcttaacagcacctgtgccgcgcctacgccaaaaatcgaacgccgcagttgccaaagtttggagggattcaactcaaggccgatgataaacatcaggaataccacgccgagttccgaaaagtggaggatctcatcgacgtcgctaataaaccccagcccccacgggccaattgcaatccctgccagcaaatatcccaacacagcgccaatacccagccgcgatgccagcggcaccgcagccaccgccgcgaagagaaacagcactcctgcgagtaaaaaatcggaaccttccatcagcggcctcctggagacagcggatttgccagccagtcaccgtaggctctggcgtggctcgccagctcctgtgcgctttgccgtctcgcccagtaaataatgatgggacttaaccaatgcatccggcacatgcccgccgccagttcaaaggggcgcagcacatcgctcatcgggtagcgattcagcgcgtcataacggtaagcactttccggctcgccggtggtaatcacgctacgccagtactttcccgccagttggtttcctcccggcccgctggcaaaaccacgacttaatacccggtccagccactctttcagtagcgccgggcagctataggtataaagaggatgctgaaagacaatcacctcgtgctcgcgcagtaatgcctgctcacgggggatatcaataaaaaaatcgggatagtgcgcgtaaaggtcgtgcacggtaacattgctgagctgcgtggccggtttaagcagtacccggtttgccaccgagtcctgagattccggatgggcatacagcagcaaaactttcgctggctgagacatcatccccctcccggtatggtttttgtgtatagtcgctgttttgggctaccattgcgcccggtgcggcagctcgcccatacattacattatcataatgataagttaacatagtctgaacatacggcaccttatgattgttttctcctcgttacaaattcgtcgcggcgtgcgcgtcctgctggataatgccaccgccaccatcaaccctgggcagaaagtcggcctggtgggtaaaaacggctgtggtaaatctaccctgctggcattgctgaaaaatgaaatcagcgccgacggcggcagctacacctttccgggaagctggcaactggcgtgggtgaatcaggaaacgccggcgttaccgcaagcggcgctggaatatgtcattgacggcgaccgtgaatatcgtcaactagaagcgcagctacacgacgccaacgaacgtaacgacgggcacgccattgcgaccattcatggcaagctggatgctattgacgcatggagtattcgctcccgtgctgccagcctgctgcacggcctcggtttcagcaatgaacaactggagcgcccggtaagtgatttttccgggggctggcgtatgcgtcttaaccttgcccaggcgctgatttgccgttcagacttgctgctgctcgacgaaccgactaaccacctcgatctcgatgccgttatctggctggaaaaatggctgaagagctatcagggcacgctgatcctgatctctcacgaccgcgacttcctcgatccgatcgtcgataaaattattcatatcgaacaacaaagcatgttcgagtacaccggcaactacagttcgtttgaagtacagcgcgccacccgtctggcgcagcaacaagcgatgtacgaaagccagcaggaacgcgtagcgcatctgcaaagttatatcgaccgtttccgtgccaaagccaccaaagcgaagcaggcccagagccgcattaagatgctcgagcgtatggagctaattgcccccgcgcacgtcgacaacccgttccgctttagcttccgcgcgccggaaagcctgccaaatccgttactgaagatggaaaaagtcagcgcgggctatggcgatcgcattattctcgactcgattaaactgaacctggtgcccggctcgcgtattggtctgttaggccgcaatggcgcgggtaaatcgacattaatcaaactgttagccggtgaacttgcgccagtcagcggtgaaattggtctggcgaaagggatcaaactcggctacttcgcccagcatcaacttgaatacctgcgcgccgacgaatcacctattcaacatctggcacgtttagcgccgcaggagctggaacaaaaactgcgtgactacctcggcggctttggtttccagggcgataaagtaaccgaagaaacgcgccgcttctccggtggggaaaaagcccgcctggtgctggcattaattgtctggcagcggccgaatctgctgctgctcgacgaaccgactaaccaccttgacctcgacatgcgtcaggcactcaccgaagcattaatcgagtttgaaggcgcgctggttgtcgtttcgcacgaccgtcatttgctgcgttccaccactgacgatctctacctggttcacgatcgtaaagtcgaaccgttcgacggcgatctggaagattatcaacagtggttgagcgacgtacaaaagcaggaaaaccagaccgacgaagcgccaaaagagaatgcgaacagcgcccaggcacgtaaagatcagaagcgtcgggaagctgagctgcgtgcgcaaacccagccactgcgtaaagagattgcccgtctggaaaaagagatggagaagctgaacgcgcaactggcgcaggcggaagagaaactcggcgacagcgaactgtatgaccagagccgtaaagcggagttgaccgcctgcctgcaacagcaagccagcgccaaatccggcctggaagagtgcgaaatggcatggctggaagcccaggagcagcttgagcagatgctgctggaaggccaaagcaactgatggcgcagataacgacgaccgatgccaatgaattcagcagcagtgctgaattcatccccatgcgcggctttagcaattgtcatctgcaaaccatgctgccgcgtctgtttcgtcgtcaggtgaaattcaccccgtactggcagcggctggagttgcccgacggcgattttgtcgatcttgcgtggagtgaaaaccctgcacaggcgcaacataaacctcgtctggtggtgtttcacgggctggaaggcagtctcaacagcccttacgcccacggtctggttgaggcggcgcaaaagcgcggctggctgggcgtggtgatgcattttcgcggatgcagcggtgaaccaaaccgtatgcaccgcatttaccattcgggcgaaaccgaagacgccagttggtttttacgctggctgcaacgcgaatttggtcatgcgccaacggctgccgtcggctattcgctcggcggtaatatgctggcctgtttgctggcaaaggaaggcaatgatctcccggttgatgcggcggtgattgtctctgcgccgtttatgctggaagcctgtagctatcatatggaaaagggcttttcccgcgtttatcagcgttacttgctgaacctgttaaaagccaatgccgcgcgcaagctggcagcctaccccggaacgctgccgattaatctcgcgcagttaaaatcggtacgtcgcatccgtgaatttgacgatctcatcaccgccagaattcacggctacgccgacgctatcgactattatcgtcagtgtagcgccatgccgatgctgaaccggatcgccaaaccgacgctgattattcacgccaaagacgatccgtttatggatcatcaggtgatcccgaaaccggaaagtctccccccgcaggtggagtatcaactgactgaacatggcggtcatgttggctttattggcggtacattacttcatccgcaaatgtggctggagtcacgcattcctgactggttaacaacgtatctggaggcgaaatcatgttgattccgtggcaagacctctcccccgaaacgctggaaaatttaattgaaagctttgtgttacgtgaaggcaccgattatggtgaacatgagcgtacacttgaacagaaagtcgccgacgtcaaacgccagctacagtgcggagaagcggtgctggtatggtcggagctgcacgaaacggtcaatattatgccgcgcagtcagtttcgcgaataacctgcaaccgtcggcggacgagataataatgatagctaagtcatggagttactatgtctgccaaacatccggtcattgcggtaacaggatccagcggcgcggggaccaccaccaccagcctcgcgtttcgtaaaatattcgcgcagttaaatctgcatgcagctgaggtggaaggcgacagttttcaccgttacacccgcccggaaatggacatggcgatccgcaaagcgcgcgacgccgggcggcatatcagctacttcggccccgaggctaacgacttcggcctgctggaacaaaccttcattgaatacggtcagagcggcaaagggaaatctcgcaaatatctgcatacctacgacgaagccgtaccgtggaatcaggtaccggggacattcaccccctggcaacctttaccggaacccactgatgtactgttttatgaaggtttacacggcggcgtagtcacgccacagcataacgttgcgcagcatgtggacttactggtcggcgtggtgcctatcgttaaccttgagtggattcaaaaactgatccgcgacaccagcgagcgcgggcactcacgagaagcagtgatggactcagtagtgcgttcaatggaagactatatcaactacatcacaccgcagttttcccgcacccatcttaacttccagcgcgttcccaccgtcgacacttcaaacccgttcgcggcaaaaggtatcccgtcgctcgatgaaagctttgtggtgatccattttcgtaatctggaagggatcgatttcccctggctgctggcgatgttgcaaggctcattcatttcccacatcaatacgttagtggtaccgggcggcaaaatgggtctggcaatggaattaattatgctgccgctggtgcaacgattgatggaaggaaagaaaatcgagtaactctgctattacgccggataaaatactatccggcttcacaacgggatagttaagtcacgcggcaaccacttcatacgagtgagtaatattcaccgctttttccagcatcaacgccactgaacaatatttctcggcagagagatcaaccgcacgcgcaaccgctgcgtctttcaggtcgcgaccggtgacgataaaatgcagattaatgtgcgtaaacaggcgtggtgcctcttcgcggcgttcagaggtcaattttacttcacaatcgaccacatcctgacgccctttttgcaggatcgaaaccacatcgatggcactgcaaccacccgccgccatcaacaccatttccatcggacttggtgctttatcgcctgagttgccgtccattaaaatctgatgaccagaggcggattcgcccagaaaagttaacccttcgacccacttcactcgcgcttgcatttttgctactccactgcgtcaattttcctgacagagtacgcgtactaaccaaatcgcgcaacggaaggcgacctgggtcatgctgaagcgagacaccaggagacacaaagcgaaagctatgctaaaacagtcaggatgctacagtaatacattgatgtactgcatgtatgcaaaggacgtcacattaccgtgcagtacagttgatagccccttcccaggtagcgggaagcatatttcggcaatccagagacagcggcgttatctggctctggagaaagcttataacagaggataaccgcgcatggtgcttggcaaaccgcaaacagacccgactctcgaatggttcttgtctcattgccacattcataagtacccatccaagagcacgcttattcaccagggtgaaaaagcggaaacgctgtactacatcgttaaaggctctgtggcagtgctgatcaaagacgaagagggtaaagaaatgatcctctcctatctgaatcagggtgattttattggcgaactgggcctgtttgaagagggccaggaacgtagcgcatgggtacgtgcgaaaaccgcctgtgaagtggctgaaatttcgtacaaaaaatttcgccaattgattcaggtaaacccggacattctgatgcgtttgtctgcacagatggcgcgtcgtctgcaagtcacttcagagaaagtgggcaacctggcgttcctcgacgtgacgggccgcattgcacagactctgctgaatctggcaaaacaaccagacgctatgactcacccggacggtatgcaaatcaaaattacccgtcaggaaattggtcagattgtcggctgttctcgtgaaaccgtgggacgcattctgaagatgctggaagatcagaacctgatctccgcacacggtaaaaccatcgtcgtttacggcactcgttaatcccgtcggagtggcgcgttacctggtagcgcgccattttgtttcccccgatgtggcgcagactgatttatcaccccgatatcaactatgcacttcgacaaacgctggtgctatgtttgcccgtggccgttgggttaatgcttggcgaattacgattcggtctgctcttctccctcgttcctgcctgttgcaatattgcgggccttgatacgcctcataaacgttttttcaaacgcttaatcattggtgcgtcgctgtttgccacctgtagcttgctgacacagctactactggcaaaagatgttcccctgccctttttgctgaccggattaacgctggtacttggcgtcactgctgagctggggccattgcacgcaaaattgcttcctgcatcgctgctcgccgccatttttaccctcagtttggcgggatacatgccggtctgggaaccgttgctcatctatgcgttgggcactctctggtacggattgtttaactggttttggttctggatctggcgcgaacaaccgctgcgcgagtcactaagtctgctgtaccgtgaactggcagattattgtgaagccaaatacagcctgcttacccagcacaccgaccctgaaaaagcgctgccgccgctgctggtgcgccagcaaaaagcggtcgatctaattacccagtgctatcagcaaatgcatatgctttccgcgcaaaataatactgactacaagcggatgctgcgtattttccaggaggcgctggatttacaggaacatatttcggtcagtttgcatcagccggaagaggtgcaaaagctggtcgagcgtagccatgcggaagaagttatccgctggaatgcgcaaaccgtcgccgctcgcctgcgcgtgctggctgatgacattctttaccatcgcctgccaacgcgttttacgatggaaaagcaaattggcgcactggaaaaaatcgcccgccagcatccggataatccggttgggcaattctgctactggcatttcagccgcatcgcccgcgtgctgcgcacccaaaaaccgctctatgcccgtgacttactggccgataaacagcggcgaatgccattacttccggcgctgaaaagttatctgtcactaaagtctccggcgctacgcaatgccggacgactcagtgtgatgttaagcgttgccagcctgatgggcaccgcgctgcatctgccgaagtcgtactggatcctgatgacggtattgctggtgacacaaaatggctatggcgcaacccgtctgaggattgtgaatcgctccgtgggaaccgtggtcgggttaatcattgcgggcgtggcgctgcactttaaaattcccgaaggttacaccctgacgttgatgctgattaccaccctcgccagctacctgatattgcgcaaaaactacggctgggcgacggtcggttttactattaccgcagtgtataccctgcaactattgtggttgaacggcgagcaatacatccttccgcgtcttatcgataccattattggttgtttaattgctttcggcggtactgtctggctgtggccgcagtggcagagcgggttattgcgtaaaaacgcccatgatgctttagaagcctatcaggaagcgattcgcttgattcttagcgaggatccgcaacctacgccactggcctggcagcgaatgcgggtaaatcaggcacataacactctgtataactcattgaatcaggcgatgcaggaaccggcgtttaacagccattatctggcagatatgaaactgtgggtaacgcacagccagtttattgttgagcatattaatgccatgaccacgctggcgcgggaacaccgggcattgccacctgaactggcacaagagtatttacagtcttgtgaaatcgccattcagcgttgtcagcagcgactggagtatgacgaaccgggtagttctggcgatgccaatatcatggatgcgccggagatgcagccgcacgaaggcgcggcaggtacgctggagcagcatttacagcgggttattggtcatctgaacaccatgcacaccatttcgtcgatggcatggcgtcagcgaccgcatcacgggatttggctgagtcgcaagttgcgggattcgaaggcgtaatgcaggctaaaccatcggataaggcattcacgccgcatccgacatcttttgcctgatgcttcgtatttacgccccaaccaccttcgccaccgcgtgggcgaaacgttgcatcccttcatcgatatccgcatcttccaccaccagcgacggtgcaaaacgcatcacatccggtccggcattcagcaccattacgccagcctctgcgcccgcatacaggaaatcacgcgcccgacctttgtactgtggtttcagctctgcgccaatcaacagccccataccgcgaatatcgctaaatacatcgtactgctgatcgatcttctgcagatggtcaacaaaacgctggcgtttcgcctgaatgccttccagcacttcaggggtattgatgatatcaaacgccgcccccgctactgcacaggccagaggattaccgccgtaggtggaaccgtgagaaccaggatgaaacgcagaagcaatttccgccgtggtcagcatggcgctaatcgggaagccgccgcctaacgctttcgcagaggtcagaatatccggcgtaacgccgtagtgcatgtaagcaaacaaatcgccggtccgccccatcccgcactgcacttcatcaaacaccaataatgcctgatgttgatcgcacagctcgcgcaagccctgcaaaaactctggcgtcgctgccgtcacaccgccctcgccctggatcggctcaaccaccaccgcacaggtgtgatcatccatcaccgctttcactgcatggagatcgttaaagggaacgtggatgatgtctgccggtttcggcccaaagccgtcggaatattttggctgcccacccaccgaaacggtaaacagcgagcgaccatgaaaagcgttatggaaggcaataattttggttttgaacgggctatgacgcacacaggcgtaatggcgtgccagtttaaaggcggtttcgttagcttccgtgccggagttcataaacaccacgcgttcggcaaacgttgcctcaatcagtttacgcccaagacgcagcgccggttcattggtgaaaacgttactgatatgccacagagtttcgccctgggtttttaacgcgttcaccagcgcaggatggcaatggcccaacgccgtaactgcaatgccacccgcgaaatcgacatactccttgccttgctgatcccagattcggctgccctgaccttttaccggaataaactctgccggagcataaatcggcaggatcacttcatcgaaagtcgcgcgtgtaattgctgtttgttcaattgccatctcatgatcaccctgttacgcataaacaaatgtgaaattataaccacaaaatatgcataaaaaatcactaaatggcaatcagaaatcagcgatgcaggaaattagccagcagttgatgtccttgttcgctaagaatactttctggatggaactgcacaccttccagatcccactggcgatggcgaatccccataatctctcgggtttcgctccaggccgtcacgtcaaagcacgctggtaatgagtcaggttccaccaccagcgaatggtagcgtgtcacggtaagtggatttgccagcccccgaaatacgccctcaccgttatgtgtaatcggcgaggttttgccgtgcatgacctttgcggcgcgcacaactttaccgccaaatgcctgcgccattgcctgatgaccgaggcagacgccaagaatcggcaagcgcccggcatagtggcgaataacgtcaagggagatcccggcttcatctggcgtacaggggccaggtgagatgacaattttttgtggtttaagggcgtcgatatccgccagcgtcaacgcatcgttgcgcttaaccagcacatccgcccccagttcacaaaagtactggtagaggttccaggtaaaagaatcgtagttatctataagcaggatcatggcggctccggtacaaaagaaccgcgctattttactcagattccccggcttcgcttaccactttgctaaatatcatctgcagtgcggtgagatcccccattgccccactctgatttgcctgattccaggcctctttttcgataccctgccagctcagttgatatccggcatgaatcgccagttgctcgaagaagatccgctgtgccagaccacttcccacccggaagggatgcagcacgttgatttcacaatagtaatgcgccagccgctcgacgaacttcgctttctccaggccaaccagataaccttcttcctccagatcctgcatcagggcattgccctctttttcgatataagcaaagtggcagaacggcgtatcaccctgataaatatcaacttcacgcagttgccctgcccagtcgaaaatatcctgatacagctggcgatggatagttcgcaaatgcggtaaaccgcgcaccagcggaccaagctcaatggtcgcagcacgcagcgccgtcatttcgtaagcggcctgttccagccgctgctgctggcggatgttcagccggttacgcatgatatcaaggcctggataaagatacggatcgcgcccttcgccgaatttatcgctcatagtgactcctcagctcttcaaggcgcgctaaagcctctgcggcagtaagagtgactaaaggcatctcgacgccttcaagacggcgactggcctgaaaattacgattacgctgaagctcccagagacgggacttttgcttatcggtgagtttcttcacttgatgcctccctgaacgtgtccatttgccacaagtataagcggcaaatccgggttacgccgggagagcagaagcgcgggcaagattgcccgcgcgagaaatcattacggcaggactttagcggaaaggataactaccggttttgacggcacattctggtacggaccaacgtcatgagtcggcacctgggaaatcttatcggcaacgtccatgcctttcaccactttaccaaataccgcgtaaccgaaatcacgctgaccatggtcaaggaaggcgttatcggcaacgttgataaagaactggctggtggcgctgtctttgtcagcggtacgtgccatcgcgatggtgccacgcgtgttgcgcaggccgttatcggcttcatttttgattggcgggtttggttttttctgctgcatctgctcggtgaaaccgccgccctgaatcataaagccaggaatgacgcggtgaaaggtagtgttgttataaaaaccgctgttcacataatcgacaaagttttgcacagacactggcgctttttgtttatccagctccagttcgatgttaccagctgaggttgtcaacaatacgtgcgggtcccctttcgctgccattgctgcgggagaaagagcagaaagagcgaaaacagcagccatcgccgccagggtcgatttgaacatgagatttccttaacaaacagagcagaaaaaaagcaagtgaagagattctaaatagccttcaagaacaaggccatccctttacctaattttacgtatctgaaatatatgtaacctgacgatcactttttattccgtgatcaaaatcacctcttaaaatgcaatttagcaaccgattgcaataaaacatttaaacagatcacaaaatcacctaaaatcgcccgctcgcggcatatcccgctatgccattttatttttgaacgcaggccaatcatgactaacagcaatcgcatcaagctcacatggattagctttctctcctacgcactgactggtgcgttggttattgtcaccgggatggtgatgggaaatatcgccgattatttcaatctgcctgtttccagtatgagtaataccttcaccttcctcaacgccggcattttaatctctatcttcctcaacgcctggctgatggaaatcgtcccgttgaaaacgcagttacgttttggctttctcctgatggtgctggcggttgccggtttgatgttcagccacagcctggcgctgttctcggcggcgatgttcattctcggggtggtcagcggcatcaccatgtcgattggtacattcctggtaacacaaatgtatgaagggcgtcagcgcggttcccgcctgttatttaccgactccttcttcagtatggctgggatgattttcccaatgatcgccgcgtttctactggcgcgcagcattgagtggtactgggtttatgcctgcatcgggctggtgtatgtcgctatttttattctgaccttcggctgtgagttcccggcgctgggcaaacatgcgccaaaaacggatgctccggtagagaaagaaaagtgggggatcggcgtactgtttctctctgttgcggcgttgtgctacatcctcggtcagttaggttttatctcctgggtgcctgagtatgccaaaggcctgggcatgagcctgaacgacgcgggcacgctggtgagtaacttctggatgtcatacatggtcggcatgtgggcgttcagctttattcttcgcttctttgatttgcaacgcattctgaccgtactggctggtctggctgcgattctgatgtacgtctttaacaccggaacaccagcacatatggcgtggtcaattctcgctctgggcttcttctccagcgcgatctataccaccatcatcaccctgggttcacagcagaccaaagtaccgtcgccaaaactggttaactttgtcctgacctgcggaaccatcggtactatgttgacctttgtggttaccggcccgatcgttgaacatagcggtccgcaggcggcactgcttacagcaaacggtctgtacgctgtcgtctttgtgatgtgcttcctgttaggtttcgtcagccgtcaccgtcagcataacaccctgacctctcattaattgctcatgccggacggcactatcgtcgtccggccttttcctctcttcccccgctacgtgcatctatttctataaacccgctcattttgtctattttttgcacaaacatgaaatatcagacaattccgtgacttaagaaaatttatacaaatcagcaatatacccattaaggagtatataaaggtgaatttgatttacatcaataagcggggttgctgaatcgttaaggtaggcggtaatagaaaagaaatcgaggcaaaaatgagcaaagtcagactcgcaattatcggtaacggtatggtcggccatcgctttatcgaagatcttcttgataaatctgatgcggccaactttgatattaccgttttctgtgaagaaccgcgcatcgcttatgaccgcgtacacctctcgtcttacttctctcaccacaccgccgaagagctgtcgctggtgcgcgaaggcttctacgagaaacacggcatcaaagttctggtcggcgaacgcgctatcaccatcaaccgtcaggagaaggtgattcactccagcgccggacgtaccgttttttatgacaagctgatcatggcaaccggttcctacccgtggatcccgccaatcaaaggttctgatactcaggactgctttgtctatcgcactattgaagacctcaacgccattgaatcctgcgcccgtcgcagcaaacgcggtgccgttgttggtggcggcctgttaggtctggaagccgcaggcgcgctgaaaaacttaggtattgaaacccacgttatcgaatttgcccctatgctgatggcagaacagcttgatcagatgggcggcgagcagctgcgtcgcaaaatcgaaagtatgggcgtgcgcgttcacaccagcaaaaacacccttgagattgtgcaggaaggtgttgaagcgcgtaaaaccatgcgttttgccgacggcagcgaactggaagtcgactttatcgtcttctctaccggtatccgtccgcgcgataagctggcaacccagtgtggtctggacgttgctccgcgtgggggtattgtcattaatgattcctgccagacttccgatccggatatctacgccatcggtgaatgcgcaagctggaacaaccgtgtatttggtctggtagcacctggctacaaaatggcgcaggtcgccgttgaccatattctcggtagcgaaaacgcctttgaaggtgctgaccttagcgccaagctgaaactgctgggcgtagacgtaggcggtattggtgatgcgcacggtcgcacgcctggcgcacgtagctacgtttacctcgacgaaagtaaagagatctacaaacgcctgattgtcagcgaagacaacaaaaccctgctcggtgcggtactggtgggcgataccagcgactacggtaacctgctgcaactggtgctgaacgctatcgaactgccggaaaacccggattccctgatcctgccagcacactcgggtagcggcaagccgtctatcggtgttgataaactgccggacagcgcgcaaatctgctcctgcttcgacgtcaccaaaggtgatctgattgctgccatcaacaaaggctgccacacagttgcggcgctgaaagctgaaaccaaagcgggtactggctgcggtggctgtatcccgctggtcactcaggtactgaacgcggaactggcgaaacagggcatcgaagttaacaacaacctgtgcgaacactttgcttattcgcgtcaggaactgttccatttgatccgcgttgaaggcattaaaaccttcgaagaactgctggcgaaacacggcaaaggctacggttgtgaagtttgtaaaccaaccgtcggttcgctgctggcctcctgctggaacgaatacattctgaagccggaacatactccgctgcaggattctaacgacaacttcctcgctaacatccagaaagacggcacctactcggtgatcccgcgttctccgggcggtgaaatcaccccggaagggctgatggcggtaggtcgtatcgcgcgtgaatttaatctctacaccaagatcactggctcccagcgtctggcgatgtttggcgcacagaaagacgatctgccggagatctggcgtcagctgattgaagccggcttcgaaaccggtcatgcctatgcgaaagcactgcgtatggcgaaaacctgcgtgggtagcacctggtgccgctacggcgttggcgacagcgtcggcctcggcgtggaactggaaaaccgctacaaaggcatccgtacgccgcacaaaatgaagttcggtgtctccggctgtacccgtgaatgttcagaagctcagggtaaagacgtgggtattatcgccactgaaaaaggctggaacctgtatgtttgcggtaacggcggcatgaaaccgcgtcatgcggatctgctggcggcggatatcgatcgcgaaacgctgatcaaatatctcgaccgcttcatgatgttctacatccgtactgccgacaaactgacgcgtaccgcaccgtggttagaaaacctcgaaggcggcatcgattacctgaaagcagtgatcattgacgacaaactggggctgaacgcacatctggaagaagagatggcgcgcctgcgtgaagcggtactgtgtgagtggactgaaacggtcaatacgccgtctgcgcagactcgcttcaaacacttcatcaacagcgacaagcgtgacccgaacgtgcagatggtgccagagcgcgaacagcaccgtccggcaacgccgtatgaacgtatcccagtaactctggtggaggacaacgcatgagccagtggaaagacatctgcaaaatcgatgacatcctgcctgaaaccggcgtctgcgcgctgttaggtgacgagcaggtcgcgattttccgcccgtatcacagcgatcaggtgtttgcgatcagcaacatcgacccgttcttcgagtccagcgtgctgtcacgcggactgattgcggaacaccagggcgagctgtgggtcgccagcccgctgaaaaaacagcgttttcgcttaagcgacggcttgtgcatggaagacgaacagttttccgtcaaacattacgaagcgcgagtgaaagacggcgtggtgcagctgcgcggttaatgttttaacgggaggcgcaatgcctcccctttttgcatggtcctgtaataatcttcggtatattgcaggacattttttaaactttttgttttattttttgtttttattttttaaaggataatcaaatgtttacagacactattaataagtgtgcggctaacgctgcgcgcattgcacgcctgtcggcaaataacccgctcggcttttgggtcagctccgccatggcgggcgcgtatgtgggtcttgggatcatcctgattttcacgctcggtaatttgctcgatccatccgtacgccctttggtgatgggcgcgacctttggtatcgccttaacgctggtgattatcgccggttctgaactgttcaccggacacaccatgttcctcacctttggggtaaaagcgggcagcatcagccacgggcaaatgtgggcaatcctgccgcaaacctggctgggtaacctggtcggttccgtcttcgttgccatgctctatagctggggcggcggtagcctgctgccggtagataccagcatcgttcactccgtcgcgctggctaaaaccactgcaccggcaatggtactcttcttcaaaggtgcattgtgtaactggctggtttgcctggcaatctggatggcgctgcgcactgaaggggcggcgaaatttatcgctatctggtggtgtctgctggcatttatcgcgtccggctacgagcactctatcgctaacatgacgctgttcgcgctctcctggttcggcaaccacagcgaagcctacacgctggcgggtattggtcataacctgctgtgggtgacgctgggtaatactttatcaggtgccgtattcatgggattgggttattggtatgctacgccgaaagcgaatcgtccggttgcggacaaatttaatcaaactgaaacggctgccggttaattactaaggggtttttacgtggatcatttgcctatattttgccaattacgcgatcgcgactgtctgattgtcggcggtggtgatgtcgcggaacgcaaagcaaggttgctgttagacgcaggcgctcgcttaacggtgaatgcattagcgtttattccacagttcaccgcatgggcagatgcaggcatgttaaccctcgtcgaagggccatttgatgaaagccttctcgacacctgctggctggcgattgcagcgacggatgatgacgcgcttaaccagcgcgtcagcgaagccgctgaagctcgtcgcatcttctgtaacgtggtcgatgcgccgaaagccgccagctttattatgccgtcgattattgaccgctcaccgctcatggtagcggtctcctctggcggcacctctccggttctggcacgcctgttgcgcgaaaaacttgaatcactgctgccgttacatctgggccaggtagcgaaatacgccgggcaattacgcgggcgagtgaaacaacagttcgccacgatgggtgagcgtcgccgtttctgggagaaattgttcgttaacgaccgcctggcgcagtcgctggcaaacaacgatcagaaagccattactgaaacgaccgaacagttaatcaacgaaccgctcgaccatcgcggtgaagtggtgctggttggtgcaggtccgggcgatgccgggctgctgacactgaaaggactgcaacaaattcagcaggcagatgtggtggtctacgaccgtctggtttctgacgatattatgaatctggtacgccgcgatgcggaccgtgttttcgtcggcaaacgcgcgggataccactgcgtaccccaggaagagattaaccagatcctgctgcgggaagcgcaaaaaggcaaacgcgtggtgcggctgaaaggtggcgatccgtttatttttggccgtggtggcgaagagctggaaacactgtgcaacgcgggtattccgttctcggtggttccgggtattaccgcagcttctggttgctctgcctattcgggtattccactcacgcatcgcgattatgcccagagcgtacgcttaattaccggacacttaaaaaccggtggcgagctggactgggaaaacctggcggcagaaaaacagacgctggtgttctatatggggttgaatcaggccgcgactattcagcaaaagctgattgaacacggaatgccaggcgaaatgccggtggcaattgtcgaaaacggtacggcagtcacgcagcgcgtgattgacggtacgctcacacagctgggagaactggcgcagcaaatgaacagtccatcgctaattattattggtcgggttgttggcctgcgcgataaactgaactggttctccaaccattaatttaacccgggccagagaattctggccttcttaatgactctttttatatattcagcaaataaaacatagccccttaataaatattatctgctaatgggttatattcaccgttacagcgacttacaaaattaagtcattcgctcactgacgccaattaaatattcctgtatcgttcttaacgagcagtctgcttatattcatataatcaatgaatattaattaatatataatacatagggaatgtaaatgaacaaatttattaaagttgcactggtaggtgcagtactggctacgttaactgcatgtactggtcatattgaaaaccgtgataagaactgctcttacgactacctgctgcacccggcaatttctatttctaaaatcattggcggttgcggtcctactgcacagtaagtctctgacagaaatcggctaacaccggtttaattgcccgacgccctctggattttccgagggcgtatttgtttctatgtccttcttgcccccgcccgtaaaaatattttcactttaaattcaatttgataactacatccattagccacagcgcgatcctgtgcgaaattttgtgatcttcctccacattacataacatcatatgttgttatattcatcatgcattgtcatgttaccttttaaatgactgcaaactctcccctacaacgtattggacaagaaaaaggtatcgctatgggaagccaggaactccaacgcaagctcggattttgggccgttcttgcaatcgccgtcgggacaaccgtcggctccggtatttttgtatctgtgggtgaagtggcaaaagcagcgggcacgccgtggcttacggtgctcgcgtttgtcattggcgggttaattgtgatcccgcaaatgtgcgtctatgcggaactatccaccgcttatccggaaaatggcgcagattatgtttatctgaaaaatgccggaagccgaccgctggctttcctctccggctgggccagcttctgggccaacgatgcgccgtcattgtcgattatggcgctggcgattgtcagcaatcttggctttttaacgcctatcgatccgttgctcggtaaatttatcgccgccggattaattatcgcctttatgttgctacacctgcgctccgttgaaggcggcgcagcgtttcagacgctaattaccatcgccaaaattatcccgttcactatcgtcattggccttgggatcttctggtttaaagcggagaattttgccgcccctaccaccactgcgattggcgcaacgggcagctttatggcgctgctggcggggatctctgccaccagttggtcgtataccggcatggcctctatctgttatatgaccggcgaaattaaaaaccccggaaaaaccatgccacgagcgctgattggttcctgtctgctggttctggtgctctacaccctgctggcgctggtgatttccggcctgatgcccttcgacaaactcgccaattctgaaacgccgatttccgacgccctgacctggatccccgcactcggcagcaccgctgggatctttgttgccatcacggcgatgatcgtcattcttggttcgctttccagctgcgtgatgtaccagccgcggctggaatacgcgatggcgaaagacaacctgttctttaaatgcttcggccatgtgcatccgaaatacaacacgccggatgtctccatcatcctgcaaggggcgctggggatcttcttcatcttcgtttccgatctcaccagcctgctgggttatttcaccctggtgatgtgtttcaaaaataccctcaccttcggctccatcatctggtgtcgtaaacgcgacgattacaaaccgctgtggcgtactccggctttcgggctgatgaccaccctcgccattgcgtcaagcctcattctggtcgcctcaacctttgtctgggcaccgattcccggccttatctgcgccgtcatcgttattgctactggtctgcctgcttacgccttctgggcgaagcgtagccgccagctcaacgctttgtcgtaatgttatctggagaaaataaaatgttggatattgataaaagcaccgtggactttctggtcaccgaaaatatggttcaggaagtggaaaaagttctcagccatgacgttccgctggtgcacgccatcgtggaagagatggtgaagcgcgacattgatcgtatttatttcgttgcctgcggatcgccactcaacgcggcgcaaacggcgaaacatctggcggatcgcttttccgatcttcaggtctacgccatttccggctgggagttctgcgataacaccccgtatcgcctcgacgatcgttgcgcagtaattggcgtttctgactacggtaaaaccgaagaggtaatcaaagcgctggagctgggccgggcctgcggcgcactcactgcggcgttcaccaaacgcgcggatagcccgattacctcggcggcggaatttagcattgattatcaggccgactgtatctgggaaattcacctgctgctctgctacagcgtggtgctggagatgatcacccgcctcgcgccgaacgcggaaatcggcaagatcaaaaacgatctcaagcagttgccgaatgcgctcggtcatctggtacgcacctgggaagaaaaaggccgccagcttggtgaactggccagccagtggccgatgatttataccgttgctgcgggtccgctgcgtccgctgggttacaaagaaggcattgtaacgctgatggaatttacctggacgcacggctgcgtgattgagagcggagagttccgccatggcccgctggagattgtcgaaccgggcgttccgttcctgttcctgctcggcaatgatgaaagtcgccacaccaccgaacgcgccattaactttgttaaacagcgtactgacaacgtgatcgtcatcgattacgccgaaatttcgcaagggctgcacccgtggctggcaccgttcctgatgttcgtgccaatggagtggctctgctactacctgtctatttacaaagatcacaacccggatgaacgccgctattacggtggtctggtggaatattaatccctctcccggcccggcaacgggccggatttacgcaaggagttacccgatgaaaacaggtatgtttacctgcggccaccagcggctgcctattgaacacgcatttcgtgatgcaagcgagctgggttacgacggcatcgaaatttggggcggtcgcccgcacgcgttcgcgccggacttaaaagcgggcggcatcaaacaaatcaaggcgctggcgcagacgtatcagatgccgattatcggctatacgccagaaaccaacggctatccgtataacatgatgctgggcgatgaacatatgcgtcgcgaaagcctcgacatgatcaagctggcgatggatatggcaaaagagatgaacgcgggttatacgctgatttccgcggcccacgcgggctatctcacgccacctaatgttatctggggacggctggcagagaacctaagcgaactgtgtgagtacgcggaaaacatcggcatggatctaatcctcgaaccgttaacgccgtatgaatcgaacgtcgtgtgtaatgctaatgatgtgcttcatgcgctggcgctggtgccttcgccgcgcctgttcagcatggtcgacatttgcgcgccgtatgtccaggcggaaccggtgatgagttatttcgacaaactgggcgataaattacgtcatctgcatattgtcgacagcgacggggccagcgacacgcattacattcctggagaaggcaaaatgccgctgcgggaactgatgcgcgatattattgagcggggctatgagggttactgtacggtggagctggtgacgatgtatatgaacgagcccagactctatgcccgccaggcgctggaacgctttcgcgcgctgctgccggaggatgagagatgaaaaccctggcgacaatcggcgataactgcgtcgatatctacccgcaactgaataaagcgttttctggcggtaatgcggtcaatgtggcggtgtactgcactcgctacggcatacagccgggatgcattacctgggtgggtgacgatgactacggcacaaagctgaagcaggatctcgcccgcatgggcgtcgatatcagccatgtccatacgaaacacggcgttaccgcacaaactcaggtggaactgcacgacaatgatcgcgtttttggcgactacaccgaaggcgtgatggccgactttgccctgagtgaagaggattacgcctggctggcgcagtatgacattgtgcacgcggcaatctggggacatgcggaagacgcattcccacagctgcacgctgcgggcaaacttaccgctttcgacttctccgacaagtgggacagcccgctctggcagacactggtgccgcatctcgattttgcctttgcctccgcaccgcaagaagacgaaacgctgcgtctgaagatgaaagcgattgttgcccgtggcgcaggaacagtgattgtcacgctgggtgaaaacggcagcattgcctgggatggcgcgcagttctggcgtcaggctcctgaaccggtgacggttatcgacaccatgggtgccggagattcgttcattgccggattcctttgcggctggtctgcggggatgacattaccgcaggcgatagcgcagggaacggcgtgcgcggcgaaaaccattcagtaccacggtgcctggtaggtataacgttggcgtgagcatcttcacgccaacgtgctgttacttgccggaaaacgaccctataatccgagtaattcattctttatttcagggtcgattatgtcagctacggaccgctactctcatcaactcctctacgctaccgtccgccagcgactgctggatgatatcgcgcagggggtttaccaggccgggcaacagatccctaccgaaaacgagctttgtacacaatataacgtcagccgcattaccattcgcaaagccatcagcgacttagtggcagacggcgtactgatccgctggcagggaaaaggcacctttgtacaaagccagaaagttgaaaacgccctgcttactgtcagtggttttaccgattttggcgtctcacaaggcaaggcgacgaaagagaaagtgatcgaacaggaacgggtcagcgccgcgccgttttgcgaaaagctgaacatccccggaaacagcgaagtgttccatctctgccgggtgatgtatctcgataaagagccgctgtttattgatagttcatggatcccgctgtcgcgttatcctgactttgatgagatttacgtcgaaggaagctccacctatcagttatttcaggagcgttttgacacgcgagtggtcagcgacaaaaagaccatcgatatctttgccgccacccgcccgcaggcaaaatggctgaaatgcgaactgggcgaaccgttgtttcgcatcagcaaaatcgcctttgatcagaatgacaaaccggtgcacgtctccgaactcttctgccgcgccaatcgcatcaccttaactattgataataaaagacattaaccgtaggccggataagatgcgccagcatcgcatccggcgatgctggcgcgttgaattttacatcccgtacgttcccctcaccctaaccctctccccaaaggggcgaggggaccgttcagtacggaatttagcttgacggtgctatccagcattaaatactggcaatactctcacgcaaaatccgcagcaccgtctcttcaccgctgcgattcgggttaatgcgaatcgcacaatgttctgattgtggattcgcctggcgaaacgttccggaaaggcgataaaagagcggcgggatttcatatttcgactctgcacccaccgggtaaggcaaggcaccgcgcttttgcgcctcttccagcactctggcggcaatcggctgatgaaactcgacaatcaacaccttcgactgcgcattagcaatcaccgcgcttttcacttccggcaccgcaccaccgttaagcaaagccagcaaccgttcagatacccctgcctgcaccgcgtgcatcactggcgcaaacaccagaccacgcaatacttccagcgcctgtgcgccctggatctggctaccgccggagtaaagcgtggcgcgaatacggttgataacatcagcatcgccgaccactgcaccaacaccctctggcccaaatagcttgaagcaggaaaatgtcgagacattcgcgccgcattcacagccgattcgagccaccttcatcaccgcatagttgtcatcggttaacgctggaacacctgccgcgcgcaacgttgccagcacatctgccagcacgtagctgtcctgcggctgctggcgcgtatgctgcaccagcgccgcatccggttgttgctcgtcgacgacctgcttcagtgccgacaggtcattgaaatcaacagtaataagcgtcagccccatctgctcaataataacccgtgtcgtcgggtaaacaggcgcgtcatgcaccagaagacgctgccccggtttgagcaaagccgccagcccggcgcgaatcgcgccagtccccgcgccctgcaccagcgccgcagcctgtgcgtgaaatgcatcagccagcacctgttccacacgctgggtaacgcgcggttgattcagtcctggcgttaagcctaaatcaccgccagtaagaaactcgctgccggggaaatggcgacaaatgctatccaccagcgcaaactgcttttgctgcgcctcaataatcgtcaggctttgcagaggaaacgtcttcataggtgccttccttaagccggaacgaacaggccaagccagtaaagaacattcagcagaataccggtgatcattactgccacgaccggtgccgccattttctgtaccggacggcccagggattcgttgaggaagtaaatggcaaccgcgatagagaatccggtataacccgccatcttaattgctgcgaaaatcgaaccgaccagcagcgccacttccatcagcatattcatggcgttacggatgttatccgacgcattacgcaccgacgggtagcgtcccagccatttgccgatcgaacgaagcagcaagacttccgccgaaataaccactgcgcctaataccgctgcaaccatcggattcggcgagagatagtccaccgcataaacaaaggtaaagcccgcaactgcatacacacccgttgctaacgcggtggtggcaatcaacggcacaaaccccagtccgcgcataaattctgccagagccgcctgattaatcagcgtttgcgattgttccggcgttacgcctgcggaatatgctttctccagtgtgaagatcgacacttcactgccagcaaaaatcttcatgctggcaacggcggcaatcaatgctcccacgatggcgatatagggtaagtttttgataatccgtgacgtgcgttcttcaaacaccgaaagcccgctggcatcaatgtcattttcatcacgatgacgcaggtcgtgagttatcgcgatccccagcagcatcaccatgccaataaagatttcgatggattcagggttaagatgtgggaaatagcgcacgactaccacacgggtcatcagtaccaccacggcggcgatcagactttgcttccagccaaactggtagaaaatcgccaccagcgggaacagtgcaaaagctgaaaccaccggcgagcttaattcccccaggctacctaatacatccaccggcagcgcggtcagcagctggtttactggcaacaggcaagtaaggatcaacacgccccagatagcgccaagaccaaacgccatcaggctgtttatcgccaggacgccgaggatatcggtaggaagaaagagtaaccatgcgttgagcagcccggttttcagggtaaaagagatccccaccgaggccacaaaaccaatgctcagaccaaaagcgatactccccgcctcgcgacggttcatatagccttcaatcagttgcggcaggatcgggcggatgccgtcatgaaaaacagccgccgagcgatgcgccagaagcgatgtcatacccgtcaggcacgccaccacgataatctgaatatacagatccatagtcgtgccttttatttcagatggttaatcagcatcggaatcgcgtgttcgacgtgctcaacggaaaggccaaacgccacttttccttcagcgatcattttggcgatatgctcgtctttcgctttaatgcctggtttggcaatggtgcaacttttgttatagcctatcaccgcgatggcaatcgacaatgccgcgcccgcaccggtattacacgcgccgatgtaataatccagttgcccggatttcaccttcattgccgcttccatgtcgttgtgaatgaaaacttcaaaacagccaggagccgtcgcttcaatagtttttttaatctgctcacgctgtaagcctgcaacgccaatctttttcatgagtctgtccttattggaaaaattgagagggattttcacgtaacatcacatccacatcggcctgactgaatcctgactggcgcaattgcggaataaaggtggttagtaaatagtcatagccataaccaccgttggcttttaaatgggagcggcgcgtaatatccatcgacagcatgacgcggttcagcaacccacggtcgcgtagcgcatgaagcatcgcaatacgcttttcgtccgggtagtaactgttcttgccgatggtgtcgaactgcacgtacgcgccgagatcgatcatcttcaaaatgttgtcgaggttgtctttcagatcgcagtgaccaacggtgacgcgcgaaagatcaaccccgtgggcttgtagcaacgccagttgctccagccccatcgtgctgaacgacgtatgcgtggagatcgggcgtccggtctggttatgcgccagcgcagcggcaataaataccttctcttccagcggcgtaatctttccttcgctggtgccgatctccgcgatgatcccggctttcagctccgtgccatcgataccctgttcaatttcatcgaccatctcctgcgccagttcctgcacgctgcgggtcgccacatgttccgggaaaaacgcgtcctggtaataaccggtacaggccaccacgttgatccccgtctcgcgcattacatcaagcataaattgcgcattgcgccccatgtaacggttggtcatctcaatcacattacgcacgccccgggtcatcaggtcgttcatctcctggcaaatgaacgcatactgatcaaggcggcagtccacgttgtttttaaagccggagagatcaatatgcagatgctcatgggcgagggtgtaacccgtcggatcaaaactcatagggtgtctcctgcaaaccggagggaggaaagaaaagagcgaccattttgtggcggtggcgcgcggaaaaattcacacacggtagcccccacatcagaaagcgtggtgcgcacaccgagctgcgtagcgatcatcccttgctgataaaccagcactggcaccacttcgcgggtatggtggctgtgaccaatggtcggatcgttgccgtgatccgccatcacgaccaggcaatcatctggctgcatcgcctcaacaagccgggcaaggttacggtcaacgacctgcaaacgttcggcataacgtgcgacgtcttctgcatgaccagcgaggtcggtttcctgaatgttggtgcaaataaacgccgtcggatgggtgttaaattcgttgagggtgatatccataatccgctggctatccaccagattttgccagctcacgccataaggattgttgacgatatctgccaccttacccaccagcacggttggcacgcctgcttcatacagtttttgtggcacctgcactttttcatcgacgccatagcccatatgcacgacctggaaaccgttgtcataagcgccagaacgcggcgcattgataccaataaagcgcccttctttgctttctgcggcatcgagaatgcgttgactgtcggttaacaggccaccaaatgtaatgacccgaccgacctgtacctgctcacgcacgatacgaccaattttgattgcgtcgtcaaaagagatcacagagagattggcggtaatgttatagacctggcctaaatccgcctcgagattatcgccaatcgcaaccgcctgattgacccacagaaattgcagatcatcgccacggcgctccacctgccagccagcggaaactaatgcctgctcaacacggtcaatcacatcgcgaaaaggcatccgcagcggcggtaacgggcgcgtgcctaaaatttcctgatgccccataaaggtatcgccaccttcatgttgcagctctgccacgccccaggttgcggaatctgacggctgcatatcgcctggcgcataacccaatgcgttgattagccccagcgtctccagcgttggtagctgcaaatgcggcaactggctcaggatgtgaccacatgtattcgctcccgcatcttgcggacgcaccagcgtgacatctttcattgcccctacgccaaagctatcaatcactaacaccacaaatcgcgccattacgcccccagagagtttccaagactgtcataacgaccgacgatttccggttcgccacgatgaataccggacaccagcaccacatcgctacgggtgacaaaaatctgcgtgcgaaaacagagcaccactgcactgcttaccggaaactcgcctgccagcggcagggtgtagtcgatactgctgtcatccacagttttgagattggtttcagtaatcttttgattttctggcgtaaacaccaacgcatgttgcgcatgaccacgacgatagtaaccgccgccgtagcagtagctgtcgccacggaaatgatgggagatttcacttaaccagagcatcgcgatacgttcaggctgatcgccctgctggtttgccggaatagtgcccgtcagcgcatgaccgggttcggcatgagtcacaccgtattgcgccagtaatggcagcgaagtgcagctggtcgctgaaggcgcgttcagttgctcaagtgcaataccagatttcgccagttgatcccgtgcctgtatcagcgtgtgaagattcggtgtcggcaaaacttttccgacagcctcatcccaaagcaggcaagggaaatgggtaagtccggctaaatgcagccctggcagattctggatttcggcgacaatctccggcaacaccttgagggcaaaaccgctctcctggcccggataaagaaaatcatcgtcgctataaactttaagcagcacagactggattcgcccggccttcaccgccgccgcagaaacttcccgcgctttgtcgagagtaaacacggtgatgacgtcggtgccctgttcaacggcgtcagcaacctgatgacaagggatttgtaccagatgcccctgatgcgccacaggcaaaccagcgcggcgcatgactcgcgcctctttgtaatccaccgccacaatgccgctgtagcctaatgccagcaatttttccgccagccacggattacgaccaaactgcttggtcatcagatacagttcaatgccgtaaagccgcgccgtctcaatcagccgcttaccgttttccagtatctgatccacgtcgatcacccagctgtccggggcgatcttgccctgctgccacaggcttagtgcggcggaaatcagcgccgggttctggcgtttcaatgcttctacaaacatcttgttgcctcgtttctgttccttgaattaaatattcatttttttgaatatttaggttgtgcgacgtggatttgtcgggagcttcaaacctcttcgttagcagccatccataatccataaaggttggccagcaaatagccttcttcacacgggttaacttccagtgcgaattccttcaacaacacctgatgcaattgcacaacggcttgccagtggctggattgcgccagttctgccagcaactcgttatccagcggctctatttcttcaccacggcgactgcgcatcagtgcactcgccatatgtgtcatcgccatcgttccttgctcactgcgcaccggcagatggcactctgtttccagtacgttgacgacctgcatcatgcctttgcagatgtccttatcaataacgcctgcctcgcaaagcaggttgagtctggtttccatatcagatgcctttcgtttaataactcggttcctgttccccactcactacccgttgttgatgggcgagcagggcgtgtttatctacaacggcacgcagcagttgttgcattgggtaatcatcgactcgcgtcaggaccacggcttcggtggcctgtaaaaatcgcggatcgtctgtgagcggcgtcgcctctaatcccagcatggtcagttcgttttccgccaccacgttccagatcaccgcatcgacatcgcctttaacaatgcgttgtaaactctcgtgataagagagatcgactcgttccacatcactaccgccaaaaaaaacatcggtcatgattttctgatccgccgaacggttatccagccccacgcgcttcacgtttgcggactcgcctttacggcaaatcaactggtgctcgccaacgtaggtgtgcggccccaactccagcgcgaggcataagcctttttgcgtgagataactttccgccgctagtcgcgaaaccaccgccatgtcatacacgccattaagcagacactccacgcgaatatccgcgccacgcatgtgcgcatagtaaaaaggaatgccatcaaactgggctttcaatccgctcgccaggccttcgtacaaacgggtatagggcaagggcattgcacataccacgttgttgatatccacatgagtcagcaatgctttgttatccatctcgaccagataactgccattgcgcccacggcgttcaatccgtatcgctccgcttgattccagcgttttcaacgcggcctgcgtcaggccaacggatgaacggcattcatttgccagctcatctatggttttcaatcgattaccgcacttttcacccaacaaataacgggccagcgtcgtgatgacgacgccttcttttttgataaacgttcgacgcataataaattttcagtaaattgaatatttatatcttcaggaatttgaagataaggcgcaacagcgagatgtggaaacggcgaggcacttcacattttttcggattattgcaaatgaggataaaaaaaccgggtttccccggtttcagagtgatgataaaagcaaaattgcctgatgcgctacgcttatcaggcctacatttccttgcaatatgtgcattactttgtaggccggataaggcgttcacgccgcatccggcatgaacaaagcgcaatttgccagcaatagtgaattacggcttcgccacaaaaccaatcgcttcgtacaccgcttttagcgtacgggaagcgtgcgcgctggctttttccgcgccatctttcatcacctgttgcaggaaggcttcatcgttgcggaaacggtgatagcgttcctgcaattcagtcagcataccggaaacggcatcagccacttcacctttcagatgaccatacatcttgccttcgaactgtttttccagttctgggatgctctggcccgttaccgctgaaaggatatccaacaggttggaaacgcccgctttgttctgcacatcgtagcgaactaccggcggctcgtcggagtcagtgaccgcacgtttgattttcttcactaccgatttcggatcttccagcaggccgataacgttattgcgattatcgtcagacttggacatcttcttggtcggctccagcagcgacattacgcgcgcgccagatttcggaataaacggctccggcaccttaaagatctcgccatacagcgcgttgaaacgctgggcaatatcgcggctcagttcgaggtgctgtttctggtcttcacccaccggtaccagattagtttgatacagcaggatgtccgctgccatcagcaccggatagtcaaacagaccagcgttgatgttctcggcataacgcgcagatttatctttaaactgcgtcatgcgactcagttcgccgaagtaggtatagcagttcagtgcccagcctaactgtgcatgttccggcacgtgggactgaacaaaaatggtgcttttctcaggatcgataccacaagccagatacaaggccagcgtatccagcgtcgctttacgcagcttctgtgcatcctggcgcacggtgatcgcgtgttggtcaacgatacagtaaatgcaatggtagtcatcctgcatgtttacccactgacgcagcgcacccatgtagttaccaatggtcaattcacctgagggctgtgcgccactaaaaacgatgggcttagtcatttttcgattcctgattttcgctatgcggaagccctaatgcgggcagaaggtcatttatagactgataaattacatcaggctggctgagatcgatagcctcgccgtagttatatccgtaggttaagccaactgatgggcaacctgccgcttttgccgcctgaatatcattgcgtgagtcgccgacaaacagcatctgttgtggggcaattcccatccgctcagccaccagtaacagcgggtccggatgcggttttttgttttgcacatcatcaccaccaatcaccacgctgaagtatttggcgatatctaaggcttcgagcagcggcgcgacgaacggcgtcggtttgttggtgaccaggcctagcggcaggcctttagcctgcaacgcgcccaacgtatcggcaacgtgcgggaacaaaaacgtcccctcttcggcaacctcgccatagtagcgatcgaacagtttacgcagaatacgtacctgttcttctgccggaatgtcgtcatcaacgggcggtttacccattgttttacgctgagtcgcacgttcctgacgcgcccaggtcaatgcgcgctccatcagaacatctgcgccgttaccaatccaggtaataacgcgttcttcacctgcgacgggcaactccagcgcatacagcgccatatctaccgcagcagcaagaccaggagcactgtcgaccagcgtaccatcaagatcaaaagcgacgccgcgaatatcttcaaacttattcatgacttacctttgccagttcactgcgcatttcatcaatgacttttttgtagtctggctggtcgaagattgccgaaccggcgacgaacatatccgcgcccgccgcagcgatttcgccaatgttgttcaccttcacgccaccgtccacttctagtcgaatgtcaaagccagactcgtcgatacggcgacgtacttcgcgcagtttatccagtgtttgaggaatgaaagactgaccgccgaaaccagggttgacggacatcagcaggatcacatccagcttatccatcacgtaatccagatagctcagaggtgtcgccgggttaaataccagacccgctttacagccattttctttaatcagttgcagcgtgcggtcaacatgctcggaggcttctggatgaaaggtaatgatgctggcaccagcggcagcgaaatcaggcacaatgcgatcgacgggtttcaccatcaggtgtacgtcgataggggcggtaatgccatagttacgcaaggatttcagcaccattggcccaatcgtcagattgggaacatagtggttatccatgacgtcaaaatgcacgacatcagcgccagctgccagggcttttgcggtatcttcacccaggcgggcaaaatcagccgacagaattgagggggcaatcaaatactgtttcatccgcttctccttgagaattattttttcgcgggtgaaacgactcctggtttgtacaaagccagcagttcgtccacctttttacgtgtgccgccgttgctgcttatactgcgtcgaactttgacgacatgcaattttgcgcgctgataccactcacgcgttaacatcgtatcgtgattggagatcagcactggaatatggcgctcaaccagaccttcggcgatctccgccagatgcgcttgttgttcaagcgtaaaactgtttgtgtgatacgccgtaaagttggcggtcgcagacagcggtgcataaggcggatcgcaatagacgacggatgcatcatctgcgcgcgccatgctatcggcgtaagactcacaatagaaaaaggcattctgcgctttttcagcgaagtgatacaactctgcttccgggaaatagggttttttgtagcggccgaacggcacgttaaactcaccgcgcagattgtaacgacacaggccgttgtaaccgtagcggttcaaatataaaaacagtaccgcccgacggaacggatcctggcttttgttgaactcttcgcggaactgatagtaaacctcggcgcaatttgtttcgggaacaaacagctcgcgtgcggcctgtacgtactcatcagtacgcatcttcacaatgttatagagactgatcaggtcgctattgatatcggcaaggatataacgagaaaagtcggtgttgagaaacaccgacccggcacctacaaaaggctcaaccagacattcgcccttgggcaaatgccgtttaatatcatcaagcaggggatacttgccccctgcccacttcaaaaaagcgcgatttttcttcatgctgactaactaattacaccttctccggctgtggagaaagctccgacagcatccagcgcttcaggcaactcccgcaacgataaaccattgcgggagataaccttgattacttcagatcggcctgtacctgacgcagcggtttcgcccacgggtttttggcctggacatctgctggcaatgtagataccgcttttttcgcctcttctttcgaagcgtacacgccagaaaccaggacataccacggctgaccattacgcgtcgtttcatagacaacgtagtttttcagattctctttcttcgcccaaccgttcaggttgtcgtagttagaggaactgctcagctgcagagtgtaatggctggacggtgccgatttcaacgaaccaacattacctgcggtcttcgccccagcagcgggtgttgctgtggtttgcgccggggatgccgtctgtactggagccgtagtcgccgtctcttttggtgctggcgtagaagtcgcagccggtgccttcgtgctcgccacaggggcagctggttcagtacgcttcggcgtctgtgctaccggcttcggctccgttttcacggttgcttgcggttttttcggttcaatcaccgcctgctgacgagctgggcgcgtagtggacggacgttcagcggtttgcgttttcgccgtgtcacgcgatgcattgccattgcgaacaggcgcaaccgttgcgggttcagtcggcaacgtggaattgaccgccacattgttcagctgttgctgattttgtggctgggtcagcgcattgttcaggtcaccctgcacttcaacacgttgttgaccatccgttgccaccggggtttgcccttgagtcggcgtagaagagatcggtggcagagaaacatcctgctgagtattttccgcagacgtggttcccggcgctggctgcacgccattcgcctgatcggtcgcattgccagcaagatcaatactcttctcgccagacgcggtttgatcgctggaagtggtcgagggggcttttagcgcagaaccgataccgatgatcaacagcagtagaaccagaatgccgacgcccatcatcatatactgacgagaagcgggtttactggctgcttttttgcgcttacgcggacgacgctctacgcgctcttcatccacggtttcatcttcggattcgtcaatttcttcttcgatttccggttcctcattgcgctctttttgcgcacgagtcggacggcgatcgtcagtgtcatcaagttcaatatcatcaaaattgatctgcggttcgccacgttcagtacgctcagaacgttcagaagattgacgagaacgaccagtacgacgatcgctgggatcgggtttcagctcgtcttctggtttgaattcatccatttaacaccccactaaaaggttaatgcttaccacgttgcaattaacctgaagctaatagaccgcttgataagcggcctgacctttcttgttgttacgctgattgacaatcggcaatggcgttaagaacaagctcgtgcgaaacgccgctgcgaacttcactcttaccaattgccaacggaagaattaagcgcatctctcccgcaaggactttcttgtcacgcagcatatgcggtaaatacgcctgcgcggacatttcgcgcggcccattgaccggtaacccagcccgcttgagcagggttataatacgctgcgtttcggcagaactaaactgcccgagacgttccgacgtccgcgccgccatcaccatacccgcagcgaccgcttcaccatgtaaccaattgccataccccatttcagcttcaatggcatgaccaaaggtgtgtcccagattcagtaaagcacgtaacccggtttcgcgctcgtcggcggcgacaacttctgccttcagttcacaacaacggcgaatacagtacgccattgccggaccgtccagacgcaacaacgcatccagattctcttccagccagttaaaaaacgcaccgtcaagaataatgccgtatttgatgacttctgccagccccgacgctaactcacgcgggggaagcgttttcagacagtcgagatccaccaccactgaagcaggttggtagaacgcgccaatcatgtttttaccgaggggatggttgaccgcagttttgccgccaacggaggaatcgacctgcgacagtaacgtcgtcgggacttgaatgaaacggacaccgcgctgataactcgccgccgcgaagccggtcagatcgcccactacgccgccgccaagcgccaccagcgtagtatcgcgaccatgcggtttttgtaacaacgccgtaaagacggtatcgagtacagccaggcttttatactgctcgccgtcagggaggataacgctatcgacgttaacacccgcctgttcaagtacgccgcggaccttatcgagatacagaggagccagggtttcgttggtgaccaacatgacctgctcgcccgatttcagcggtaagaatgaagctggttcattaaacaaaccagatgcgatggtaattgggtaactacgttccccgagagtaacgacaatcctctccataacgcgacatccaccttaattactgtacccgcagacgagtgtatataaagccagaattagttgctttccagcatgtgaataatctggtttgcaaccactttagcgctttgatcatcagtacgaatggtcacgtcggcaatctcttcatacagcggattgcgttcattggccaacgcttccagaacttcacgcggcggtgtttcaacgtgcagcaacgggcgttttttatcacgctgcgtgcgtgcaagttgcttttcgatggtcgtttcaagataaacgacaacgccacgagcggaaagacggttacgcgtttcacgggatttcacagagccgccgccagtagccagcacaataccctgtttctcggtcaactcattgatgaccttttcttcgcgatcgcggaagccttcttcgccttctaaatcgaaaacccagcccacatcagctccggttcgtttctcaatctcttgatcggaatcgtaaaattccatattgagttgttgagctaactggcgcccaatagtgctttttccggcacccataggcccaaccagaaagatattgcgtttctctgccattttttcggtactactaagactattcgttaatgataaacccgcttcgctcagagagcgccgcaggacatgaactgaaacctcataagatattgcgagagtcagactgaaaattatctcaatactccagcgggtttggcaactgaataaatcacccatccctctgcatatctggtcgctgcaagcgcgctgccttgctaccaccgctctggcgataaatcaccgggtaagattagcgtaaaaaagacagcaaaatgccgcctgaatgataaatcatcatcatggaacgcaggcagcgaagagcaccaactctcaaatcggtactccttgtatgctaaatacctgcgcgcgtcaaatagatgaaacacgttcagcgtaaaaacattaccgcttttacggctgtttactcactggaaaccagtcgtggcgtgataaacaccactaactcgcgtcgttcatcttcttttccgtcatgacgaaataattgcccgaaccagggaatgtcgccaagcaacggtacgctatcctgacccgatttatttttacgggtaaaaatgccgcccagcgccaacgtttctccgcttttgacctcgacctgcgtttcgatctcctgcttatcaatcgccagcacttcgccatcggcctgctgtagcacctgccccggaacgttctggctgatgtgtaatttcagccggatgcgacctttttgtaacaccgtgggcgtgacctccatccccaggacggcctctttaaattccaccgacgtcgcgccactttccccgctggaaacctgatatggaatttcgctcccctgtttaatgctggcaggctgaagatgtgaggccagcagacgcggactggcgataatatccagctgctgtttttgttcgagcgcggaaagctcaagatccagcaagcgtccgttgatgcgcccaatgttaaaaccgacatgcgttgtcgccgtcgctacggagaggtcgctaccaagcgtggtgacttgcccaacgccaccagcgtgttgcgcatcggccagcgtccatttcacgcctaactcacgcaaacttttttcattaatggtgacaatatgcgccgacagctcaacctgcccgaccggcagatccatttgcgctacccactgttcaagcgcgcttaacgccgttttgttatctcgtagcaaaaggcgattggtgcgtttatcgacggtcatactccctttggcactcagtagcttctcccccgctttcgccagttctcccgcgtcggcgtattgcagggttatactgcgattttccagcggcagatttgcctgcgcccgcgcctgctccgcctcctggcgggcgatattgttattctgccaggcaatggaatgcactgagagaatgttgccttcctgccgcgttatcagtccggcgcttttcactacagtttgtagtgcctgcttccagggaacatctgttagatgtaacgacaccgtaccgctgacgtctggcgacacgaccaggttcaacttctcctgttcagccagcgcctgcaacacctgagctaccggaacgtcatccaccatcagcgtcactttttgcggctttgccgcctgtacgccgggtatcagcatcaacagtagtgcggctatccattgcttcatttgtatctccttgccgttgccacaaccattgtggcggttcgcagtttgtcccggtacccagcgttagtacgtctggcgtcagctgtaaaattgtccagccgttttccagcacatcgttttgctgcacccgtcgccatttcttttgcccgtcttttattacaccgatgatgcgctcgcctcgccctaccatcccctgatagcgccactggctaagttcgctaatccggcatagatcttccggcggtttaaaagggtcacgcataccggttaaaaggcacaatgcaatacctgccaacaaccagcgtttaaccctcatgcggcgtctccagttgtagcgtgaacaaaagatcatcaccttccacgcttaacgaaaaacggctcacgctgacgttgcgctctgccagccgtgtaaatgccgacggcactgcttcccacagcgttttcaacgccaactcgcctccctgcgcggatggatgccaggaaaccagttgcgcgccggataactgaaaatccagtggcgaaaagggcagcgttttttcctcgctgaagggagcggtgtctaccaggcgatacagtgcggcccactgctggtgatgacttgcccgtagtcgaattaatgcgtcgcgctcttcatggtgtgtcgatgacagaaaaatgagcgtaactaacatcagcaaccagaatgcccagcaaagctggcggaggcggggtgatgtggcgaaccaccagtcaaagaacatgttcatcgctaaccttccttgttaactgatactcaaattgccagcgtccctgcgcatcctgctgcgtggctccccgctgattgagatgaaaagatgcatcctggcggagtgacgtttctagtgcgtttaacgcggtaatgcttgttgtcagccccttgatctccagcgttccctgctgccagcttatcgttgtcagccaggcgtgctcgggtaaaagcgccgccagtgcttccagcgcagattgccagtcgcgggtaaattgtcgctggcgctgccgttgcgaacgctgttcgcgtaactgctgttgctccagcaaacgtggcttcgttatctgtaagctgcgggcgagttgttgttccgcctgaagcaaaactgcgtctatgcgcgcttcggcgctgcctgtcagacgcagtattagcgttatcccgacggccagcagcagaggcgcaacgaacatcagcaaccagaaacgcagaaaagcggtccggcgttgctgtcgccagggcaaaaaattaattggcgggttcatcagtacgccttcccaagcgccagccccagcgcgatggcaaagtctccacctggcggcggtagcggcggctgacgaacagaaacggcctcccagggatcaaatccgccttcgccacatatcgcgacgctttcgggatcaacggataacgctgccgccagctccttcgcgctagtcatccccaccgccagtttgcgcccccagctatagcgcgtcgcccacagccactgttcgttatcacgccaggccagacattgctgatgagaaggtaaaaaaggcaggaatcgctgtaatgcactggcatccggggtgatcgcgctcacatgaacacgcaacctttctgccagagtaagcagcgttgccagctctttgctttgcgcggcagtcacgttataggcgggactgagtgagtcttcgctgtaatcgaagcgcagggagtccggatccatatccagctcgcgggccatcgtccctgacagccaggccgtttgctcccgctcaccaagggacatcgacgggcgcggaaatgaccgctgtaatgtgcgactggcgggaaacgccaacataatgtgatgacgctgcggcagttcgcgactccacggtaacaacgttttagccagctgctgcgcatcaacaatccgcccatctttgataatgtcgttctccagcggcaaccgccaccagcgttgcaaaaagcattcttttgcgccccgcacgatcgcaaccgctaccgcttcttgctgttgtaaatgcaaaccaatttgccagatcttaaatgccattgtgatgatctccttatcacccgtcactctgacgggtatatcaatgcgtctggcttgcctttatactaccgcgcgtttgtttataaactgcccaaatgaaactaaatgggaaatttccagtgaagttcgtaaagtattttttgatccttgcagtctgttgcattctgctgggagcaggctcgatttatggcctataccgctacatcgagccacaactgccggatgtggcgacattaaaagatgttcgcctgcaaattccgatgcagatttacagcgccgatggcgagctgattgctcaatacggtgagaaacgtcgtattccggttacgttggatcaaatcccaccggagatggtgaaagcctttatcgcgacagaagacagccgcttctacgagcatcacggcgttgacccggtggggatcttccgtgcagcaagcgtggcgctgttctccggtcacgcgtcacaaggggcaagtaccattacccagcagctggcgagaaacttcttcctcagtccagaacgcacgctgatgcgtaagattaaggaagtcttcctcgcgattcgcattgaacagctgctgacgaaagacgagatcctcgagctttatctgaacaagatttaccttggttaccgcgcctatggtgtcggtgctgcggcacaagtctatttcggaaaaacggtcgaccaactgacgctgaacgaaatggcggtgatagccgggctgccgaaagcgccttccaccttcaacccgctctactcgatggatcgtgccgtcgcgcggcgtaacgtcgtgctgtcgcggatgctggatgaagggtatatcacccaacaacagttcgatcagacacgcactgaggcgattaacgctaactatcacgcgccggagattgctttctctgcgccgtacctgagcgaaatggtgcgccaggagatgtataaccgttatggcgaaagtgcctatgaagacggttatcgcatttacaccaccatcacccgcaaagtgcagcaggccgcgcagcaggcggtacgtaataacgtgctggactacgacatgcgccacggctatcgcggcccggcaaatgtgctgtggaaagtgggcgagtcggcgtgggataacaacaagattaccgatacgctgaaggcgctgccaacctatggtccgctgctgcctgccgcagtcaccagcgccaatcctcagcaagcgacggcgatgctggcggacgggtcgaccgtcgcattgagtatggaaggcgttcgctgggcgcgtccttaccgttcggatactcagcaaggaccgacgccgcgtaaagtgaccgatgttctgcaaacgggtcagcaaatctgggttcgtcaggttggcgatgcatggtggctggcacaagtgccggaagtgaactcggcgctggtgtcgatcaatccgcaaaacggtgccgttatggcgctggtcggtggctttgatttcaatcagagcaagtttaaccgcgccacccaggcactgcgtcaggtgggttccaacatcaaaccgttcctctacaccgcggcgatggataaaggtctgacgctggcaagtatgttgaacgatgtgccaatttctcgctgggatgcaagtgccggttctgactggcagccgaagaactcaccaccgcagtatgctggtccaattcgcttacgtcaggggctgggtcagtcgaaaaacgtggtgatggtacgcgcaatgcgggcgatgggcgtcgactacgctgcagaatatctgcaacgcttcggcttcccggcacaaaacattgtccacaccgaatcgctggcgctgggttcagcgtccttcaccccaatgcaggtggcgcgcggctacgcggtcatggcgaacggcggcttcctggtggacccgtggtttatcagcaaaattgaaaacgatcagggcggcgtgattttcgaagcgaaaccgaaagtagcctgcccggaatgcgatattccggtgatttacggtgatacgcagaaatcgaacgtgctggaaaataacgatgttgaagatgtcgctatctcccgcgagcagcagaatgtttctgtaccaatgccgcagctggagcaggcaaatcaggcgttagtggcgaagactggcgcgcaggagtacgcaccgcacgtcatcaacactccgctggcattcctgattaagagtgctttgaacaccaatatctttggtgagccaggctggcagggtactggctggcgtgcaggtcgtgatttgcagcgtcgcgatatcggcgggaaaaccgggaccactaacagttcgaaagatgcgtggttctcgggttacggtccgggcgttgtgacctcggtctggattggctttgatgatcaccgtcgtaatctcggtcatacaacggcttccggagcgattaaagatcagatctcaggttacgaaggcggtgccaagagtgcccagcctgcatgggacgcttatatgaaagccgttcttgaaggtgtgccggagcagccgctgacgccgccaccgggtattgtgacggtgaatatcgatcgcagcaccgggcagttagctaatggtggcaacagccgcgaagagtatttcatcgaaggtacgcagccgacacaacaggcagtgcacgaggtgggaacgaccattatcgataatggcgaggcacaggaattgttctgattaaaaaggcgcttcggcgccttttcagtttgctgacaaagtgcacttgtttatgccggatacggcgtgaacgcgttatccggctaacaaaatcgtgaaaactcaataaattgcagaaaccccataagcctgataaacattgtgcatcaggcaaacttcacgcatttacactcgcccctgccctttcaaccattcgcgcacgaggaacagcgcactgacattgcgcgcttcattgaagtcagggtcttccagcaaatccatcatatgcgccagcggccagcgcacctgtggtagcggctctggctcatcgccttccagtgattccgggtagagatcttgcgctaccacgatattcattttgctggaaaagtaagacggtgccatgctgagcttcttcaaaaaagtcagatcgttcgctccaaatccaacctcttcttttagctcgcggttagcggcttcgtagacgctttcacccggatcaattaatcctttcgaaaaacctaattcgtaggattcagttcccactgcgtattcgcggatcaggatcaggtgatcgtccacaatcggcacaatcatcactgcttcccggttggttggacgcattcgttcataaacacgccgcacgccattgctgaactccagatccacgctctcgacggtaaacagtcgggaacgggctacagtttcaacattcagaatggtgggtttttgtaatgatttgctcatcgtgggatctatgctgtgaaatcagcggttattgtgcgatatcggacacgctttcggcaatgtgaattgcatgttatttacatttatgtaacttaataaataatcgtcctcaaatcaaattaaaagtcaataggttgaaataactccaggaatttgctgatattccgccttcagagggtttgctatgatcagcggttactgtgatgtgcttaatgatgctcaagttaaactccacgcttgccgatagccaaccgcagaatcatgtattgtgtccggtgcgactgaccacgcctgacagactaagtaagatggggaaagcatgagcaccattgtgatttttttagctgctttgctggcctgctcactacttgcgggatggctgataaaagtgcgatccagacggcgtcagctgccctggaccaacgccttcgcggatgcgcaaacgcgtaaactcacacctgaagaacgtagcgccgttgaaaattatcttgagagcctgacgcaggtattacaggtgcctggcccaacgggagccagcgcggcaccgatctctctggcgctgaatgccgaaagcaacaacgtcatgatgctgacacacgctatcacgcgttacggcatctctaccgacgatccgaataaatggcgttactacctcgattcggtagaagtccacctgccccctttctgggaacagtacatcaacgatgagaataccgttgaactgattcataccgattcgctgccgctggttatttcactcaacggtcatacgctgcaggagtacatgcaggaaactcgcagctatgccttgcaacctgttccgtcaacgcaggcgtcgattcgcggggaagagagtgagcaaatcgagctactcaatattcgcaaagaaacgcatgaagaatatgcgctgagtcgtccgcgcgggctgcgtgaagcgttgctgatcgtcgcctccttcctgatgttctttttctgcctgattaccccggatgtatttgttccgtggctggcaggcggcgcgttactgctgctgggcgcaggtctgtgggggctattcgcgcccccggcaaaatcctccctgcgggaaattcattgtctgcgcggtacaccccgtcgttggggattgtttggcgaaaacgatcaggaacagatcaacaatatttcactcggtattatcgacctggtctatcccgcacactggcagccatacattgctcaggatctcggtcaacaaaccgatatcgatatctatctcgaccgccatgtagtgcgtcagggacgatatctttcgctgcatgatgaagtaaaaaactttccgttacagcactggctgcgcagtacgattatcgctgcgggctcgctgctggtgctgtttatgctgttattctggatcccgctggatatgccgctgaaattcactctctcatggatgaaaggcgcgcagaccattgaagccaccagcgtaaaacaactggctgacgctggcgtgcgggtaggcgatacattgcgtattagcggtacgggaatgtgtaatattcgaacttccggaacctggagcgcgaaaaccaattcaccttttttaccgtttgactgctcgcagatcatctggaacgacgcccgctcattgccattaccagaatctgaactggtcaacaaagcgacggcattgactgaagcagttaatcgccagctgcaccctaaaccggaagatgaatctcgcgtcagtgcctcattacgttcagcaattcaaaaatccggcatggtattgcttgatgattttggcgacattgtactgaagacagcggatttatgttctgccaaagatgactgtgtgcgactgaaaaatgcgctggtcaatctcggcaacagtaaagactgggacgcgctggtaaaacgcgccaacgccgggaagctcgatggcgtgaatgtgttattacgcccggtgagtgcggaatcgctggataacctggtggcaacctccaccgcgccgtttatcacgcatgaaacggcgcgagcggcacaatcactaaacagtccggcccccggcggattcctgattgtcagcgacgaaggcagcgattttgttgatcagccctggccttcggcatcactttacgactacccgccgcaagaacagtggaacgctttccagaaactggcacaaatgctgatgcatacgccgtttaacgccgagggtatcgtcacaaaaatcttcactgacgccaatggtacgcagcatattggccttcatccgatcccggatcgttccggcctgtggcgctatctcagcaccacattgctgctactgacgatgctgggtagcgccatttacaatggcgtacaggcctggcgtcgttaccagcgtcatcgcactcgcatgatggagattcaggcctattatgaaagctgcctgaacccgcaactgatcaccccttcagaaagccttatcgaataacacgtttgcgcggcaggttatgctaccctgtcgcgcaaattgcttcactctggagatttccctcatgcatatcaacattgcctggcaggacgtagataccgttctgctggatatggacggcacgttgctcgacctcgccttcgataactatttctggcaaaagctggtgcctgaaacatggggcgcgaaaaacggggttacgccacaggaagcgatggaatatatgcgccagcaatatcacgacgtacagcatacgctaaactggtactgtcttgattactggagtgagcaactgggtctggatatctgtgcgatgaccaccgagatgggaccgcgtgccgtactgcgtgaagataccattccgtttcttgaggcactgaaagccagcggtaagcagcgaattttgctcaccaatgcgcatccgcacaacctggcggtaaaacttgagcataccggtctggacgcacaccttgatttattactttccacccacacatttggttatccgaaagaggatcagcggttatggcatgcggtggccgaagctacgggtctgaaagctgaaagaacgctgtttattgatgacagcgaagcgattctcgatgctgccgcgcaatttggtattcgttactgcctcggcgtgactaatcctgattccgggattgccgagaaacagtatcaacgccatccgtcactgaatgactaccgccgcctgatcccctcgctaatgtgaaggagacgccatgaaagagaaacctgctgttgaggttcgactggataaatggctatgggctgcccgtttttataaaacccgcgcgctggcccgtgaaatgattgaaggcggtaaggtgcattacaacgggcagcgcagcaagccgagcaaaatcgtcgagctgaatgccacgctcactctgcgccagggaaatgacgaacgcacggtgattgtaaaggcgattactgaacagcgtcgccccgccagcgaggcagccttgctgtatgaagagactgcggaaagtgtagagaaacgcgaaaaaatggcgctggcacgtaaacttaatgccttaaccatgccgcacccggaccgacgcccggacaaaaaagagcgccgcgacctgttacgatttaaacacggcgacagtgaataactgtcacctgcaagagagatgattatgccgcaacatgaccaattacatcgctatctgtttgaaaactttgccgtgcgcggcgaactggtaaccgtttcggaaaccctgcaacagatccttgagaaccacgattatccgcagcccgttaaaaacgtgctggcagaactgctggttgcgaccagcctgttaaccgctacgctgaagtttgatggtgatatcaccgtacagctgcagggcgacggtccgatgaatctggcggttattaacggtaacaataaccagcagatgcgcggtgtggcgcgcgtgcagggcgaaattccagaaaatgccgacctgaaaacgctggtcggcaatggttacgtggtgatcaccattaccccgagcgaaggcgaacgctatcagggcgtagttggtctggaaggtgataccctggcggcctgcctggaagattactttatgcgttctgaacagctgccgacgcgcctgtttattcgcaccggcgacgtagacggcaaaccggctgcaggcggtatgttgttgcaggtaatgcctgcgcaaaatgcccagcaggacgactttgaccacctggcgacgctaaccgaaaccatcaaaaccgaagaactgctgaccttaccggcaaacgaagtgttgtggcgtttgtatcacgaagaagaggtgacggtttacgatccgcaggatgtggagttcaaatgcacctgctcgcgtgaacgttgcgccgatgcgctgaaaacgctgcctgatgaagaagttgatagcatcctggcggaagatggcgaaattgacatgcattgtgattactgcggtaaccactatctgttcaatgcgatggatattgctgaaatccgcaacaacgcgtctccggcagatccgcaagttcattaatgagtatgtccggcagagagggctctgccggattttacgactaatacacctgatgcgctttgtcactcattcagattcacattcagcctttcaccatccactacaagatcgcgccacgctttaggcttcgtccccagttttccatccttcgcagctgtgagtaatttttctttcgttatttcgttcggaagtaaactcatatcaagcgcgtcccattcttttctgtctgagtcaaagccatagacaatgactctgtcatcattaaaagcaaacaggatccgctccgcctgaccatcactattcagatcttgctcgaccaggacgcaggcgtctttttcaatacaggtcatcacgttatagcgatcctggattaaggccgaccagaatgtcgcatcaggtttaacagaaccaggggcaattaacacattatcggctaatactttttccgatacctgttgctgaagatgttgctctccatctaacgccatcagcagatcccgcgcgcgtttcgggtctttcataaacccggcatcgcttttcagcgactcaagcgcagcacgtccatagcgaccgctctgctcgagcatgtagatagttacctggtctgacgtgtttttgccgctctgataacgcgccatatggctgttcacgctaatgcgcatactgtccagcaccggcgaattaagaagcaccagtatcaccaacaccaataacgaaaccgcaaggttcactttgccctgaagaacaacgggattttgccctttacgccagacgatgctgacaaaataccccagcgaccacaccagtaacaccagcaccgccagcacgccctgcaagcggtcgacagtccagccgtactgagcgacccgcagccataacgcccaggcggcgacgaacacatacagcggagcaaccagcaaagcggttttaatcaggcaacgcaacggccctgtccagggaagtgacgctttttgcggatcgcggacaatagccattaagatcaattgcaaaaaggccagcgtcaacagcaacccggcggcggagatgtggcgagaaatcgcgctcaggcccgtaaacggcagggtgatgataaacatcagggttagcaatgatactaacggcagcaaccccgtggcgattaacgtgaacaacttttgaatagagtcgattaaacgtgactgtgttcgcgcgaggatcaccgccagcgcggtaaccagacctaacgtgagataaataaaccagtcggttgcaaaaaagagcgtattgaaaaacgtgatgccaacaagtttaaacaactcactccacagtaaaagcaccagccacgtcaagccattggcgagaaaaatcaccagtaatataagtacgttatgccatactgactggtaaaaatagcgatagcggctactgtcattgcggatgcgaaggctttgttgtatccacggtagcaacaacattgccatcaacagcagatagcaaccaaaatcccaaagcgccttttcagctctccaggggttcatgccatcagtttgccacttcagccagccgctcatccccagcgtggcaataaacactagcgccagccatccccaaaggcgcttctgtttaaaagagatcacggagaagagtaaaacggatgaaaacgcgacggtcgcaggcacgccataaacaatccaactgtgattttttccggaaagccaggcgatcagcaggtagcaaaccagaccctgaagtaatccggtagcaatcatcccccagcgtgttgcgggtgaaagttcaacgttatccatgttggttatccagaatcaaaaggtgggttaattatcgcatccgggcagtagtattttgcttttttcagaaaataatcaaaaaaagttagcgtggtgaatcgatactttaccggttgaatttgcatcaatttcattcaggaatgcgattccactcacaatattcccgccatataaaccaagatttaaccttttgagaacattttccacacctaaaatgctatttctgcgataatagcaaccgtttcgtgacaggaatcacggagttttttgtcaaatatgaatttctccagatacgtaaatctatgagccttgtcgcggttaacacccccaaaaagactttactattcaggcaatacatattggctaaggagcagtgaaatgcgcgttaacaatggtttgaccccgcaagaactcgaggcttatggtatcagtgacgtacatgatatcgtttacaacccaagctacgacctgctgtatcaggaagagctcgatccgagcctgacaggttatgagcgcggggtgttaactaatctgggtgccgttgccgtcgataccgggatcttcaccggtcgttcaccaaaagataagtatatcgtccgtgacgataccactcgcgatactttctggtgggcagacaaaggcaaaggtaagaacgacaacaaacctctctctccggaaacctggcagcatctgaaaggcctggtgaccaggcagctttccggcaaacgtctgttcgttgtcgacgctttctgtggtgcgaacccggatactcgtctttccgtccgtttcatcaccgaagtggcctggcaggcgcattttgtcaaaaacatgtttattcgcccgagcgatgaagaactggcaggtttcaaaccagactttatcgttatgaacggcgcgaagtgcactaacccgcagtggaaagaacagggtctcaactccgaaaacttcgtggcgtttaacctgaccgagcgcatgcagctgattggcggcacctggtacggcggcgaaatgaagaaagggatgttctcgatgatgaactacctgctgccgctgaaaggtatcgcttctatgcactgctccgccaacgttggtgagaaaggcgatgttgcggtgttcttcggcctttccggcaccggtaaaaccaccctttccaccgacccgaaacgtcgcctgattggcgatgacgaacacggctgggacgatgacggcgtgtttaacttcgaaggcggctgctacgcaaaaactatcaagctgtcgaaagaagcggaacctgaaatctacaacgctatccgtcgtgatgcgttgctggaaaacgtcaccgtgcgtgaagatggcactatcgactttgatgatggttcaaaaaccgagaacacccgcgtttcttatccgatctatcacatcgataacattgttaagccggtttccaaagcgggccacgcgactaaggttatcttcctgactgctgatgctttcggcgtgttgccgccggtttctcgcctgactgccgatcaaacccagtatcacttcctctctggcttcaccgccaaactggccggtactgagcgtggcatcaccgaaccgacgccaaccttctccgcttgcttcggcgcggcattcctgtcgctgcacccgactcagtacgcagaagtgctggtgaaacgtatgcaggcggcgggcgcgcaggcttatctggttaacactggctggaacggcactggcaaacgtatctcgattaaagatacccgcgccattatcgacgccatcctcaacggttcgctggataatgcagaaaccttcactctgccgatgtttaacctggcgatcccaaccgaactgccgggcgtagacacgaagattctcgatccgcgtaacacctacgcttctccggaacagtggcaggaaaaagccgaaaccctggcgaaactgtttatcgacaacttcgataaatacaccgacacccctgcgggtgccgcgctggtagcggctggtccgaaactgtaatgatttgaagctggagaatatctatccagtatcttatagaaagcaaaacgggaggcaccttcgcctcccgtttatttacccttcttttgtcgtgccctgcgcccgcgttaccggcactggcagccaggcgcgaatggaaagcccgccccgctcgctggtgccaagctccagcatcccgttatggttatccacgatacgctgcacaattgccagccctaatcccgtgccgctaatggtgcgcgcactgtcgccgcggacaaacggctggaacaggtgcttacgttgttccggcgcaattcccggaccgtcatcttccacctggaaccaggcgcgattcggctccgttccgctgctgactttgatccagccattgccataacgggcggcgttgaccaccatattcgccaccgcgcgtttgatcgacagcgggtgcattttcacttcaatgctgccggggtaaagcgcggtttcaatttcccgctcatagccactttcggcagcaatcacctcaccgagtactgcattaagatccgccatttccatcggcatctcctgcccggtgcgcaggtagtcgataaactgctcaatgatggcgttgcactcttcgatatctttattgatcgattctgccagatagccatcctgctcgctcatcatctcagtcgccaggcgaatacgcgtcagcggcgtgcgcaagtcgtgacttacccccgccatcagcagcgtgcggtcatccgccagttgcttaacaccagccgccatatggttaaaggcacgggtaacggaacgcacctccgaagcgccatactcacgcagcggcggcggaataatccctttaccaacctgcaaggctgcgtgttcgagatcgaccaacggtcggttctggatacgaataaacagccacgccccgcctatcgccaatagcataatcgccagcgtatagcggaacagcggagagaaatcgccctgatgaatttcggtcagcggcacgcgtacccagatattgggcgacagccaggttttcagccagacgacaggcgaacttttgttgacctcaacgcgcacttccgtcgggccgcccagttgctgcgccatctgatggcttaagaattcatagtgttgcgcccaacgcagacctgcctcttcggcagcctcgttggagtagagagagatccccagctcacggtagatctcccgacggaaagcgggaggcacaaccaactgcgtgccgtcctccagttgcagtttgtcggtcatcaacatacgcacttcgtacgcgaggactttattaaactgctggaggctcggcaaaatcgcgaagttcagcaccaccagataagtcgtcaccaggctggcgaacagcaaggtgacgatgagcaataacgtacgggcaaatgaacttcgtggcgagaagcgcaatcgcctcatgctttagagccgtccggtacaaagacgtagcccagaccccagacggtctgaatgtaacgcggatgcgctggatcttcttccaccatgcggcgcagacgcgaaatctgcacgtcgatggagcgttccattgcggaatattcacgaccacgggcaaggttcatcagcttatcgcgggagagcggctcacgcggatggctgaccagtgccttcagtaccgcaaactcaccgctggtgagcggcatcggctcgtcttcgcggaacatttcgcgcgtaccgaggttaagtttgaacttaccgaaagcaattaccgcctcttcctgtgacggtgcgcctggcagttcgttcgcctgacgacgcagcaccgcacggatacgggccagcagttcacgcgggttaaacggttttggaatgtagtcgtcagcgccaatctccaggcctacgatacggtccacttcttcccctttcgccgtcaccataatgatcggcatcgggttgctctgactacgaagacgtcggcaaatcgacaagccatcttcaccaggtaacattaaatccagtaccataagatggaaagattcacgagtcagcaggcgatccatctgttctgcattagcgacgcttcgaacctggaagccttgttcggtgagataacgttccagcagcgcacgcaggcgcatgtcgtcatcgaccaccagaatcttgtagttctcttgcattgtttgtactcccaaaggttcgcaacaatttgtaagcgtgtattcttaaaaaagctcacgttcgtcaccagctaaatctggtatgaatttcagcctaaattgttacaaagcatattaaacagcagcttaagtatacaatttattcggcgaaacattattgattctgttgatatgatcacgttatacccaatgtgcgcattatcaaacagacaaagggaatcaacgagatgaaaacgcccctggttacccgggaagggtatgaaaaactcaaacaagagcttaattatctctggcgtgaagaacgcccggaggtcacaaaaaaggtgacctgggccgcaagtctgggcgaccgcagcgaaaatgctgactatcagtataataaaaagcgtctgcgtgaaatcgaccgtcgcgtgcgctatctcactaaatgcctggaaaatctcaaaatcgtcgattactcccctcagcaggaaggcaaagtcttttttggcgcgtgggtggagattgaaaacgacgatggcgtgactcaccgtttccgtattgtcggctacgatgaaatttttggccgtaaagattacatctctatcgattccccgatggcccgcgcattgctgaaaaaagaagtcggcgatctggcggtggtgaatacccctgccggggaagcgagctggtatgttaatgctatcgagtacgtgaaaccgtaaggaagagtcttaacctcctgccgatggctggcatttttgccagccagtccgtataactatcccctgatttttgatccgaaaagatgaactcaaaccatgatgaatgattcgttctgccgcattattgcgggtgaaattcaggcgcgcccggaacaggttgacgctgccgttcgcctgcttgacgaagggaataccgtgccgtttatcgcacgttatcgtaaggaaatcaccggcggtctggatgacacgcagctgcgtaatctggaaacgcgtctgagctatctgcgcgagctggaagagagacgtcaggcgatcctcaagtccatttccgagcaaggcaaactcaccgatgatctggcgaaggccatcaacgccaccctaagcaaaaccgaactcgaagacctctacctgccctacaaacctaaacgccgcacccgcgggcaaatcgccattgaagcagggcttgagccgttggctgacctgctgtggagcgatccgtcacacacgccagaagtcgccgctgcacaatatgtttatgccgataaaggcgtggcagataccaaagccgcgctggatggcgcgcgctatatcctgatggaacggtttgccgaagatgccgcgctgctggcgaaagtgcgtgattatctgtggaagaacgcgcatttggtttctacggtggtgagcggtaaagaagaggaaggggcgaaattccgcgactatttcgatcatcacgaaccgttgtccacggtgccttctcaccgcgcgctggcgatgttccgtgggcgtaacgaaggcgtacttcagctttcgctgaatgccgatccacagttcgatgagccgcccaaagagagctattgcgagcaaatcatcatggatcaccttggcctgcgcctgaacaatgccccggcggatagctggcgcaaaggcgtggtgagctggacgtggcgcatcaaggtgctgatgcatctggaaaccgaactgatgggcaccgtgcgcgaacgtgcggaagatgaagcaatcaacgtctttgcccgtaacctgcacgatctgctgatggcggcccctgccggactgcgtgcaacgatgggcctcgatccgggtctgcgtactggggtaaaagtggcggtggtcgatgccactggcaaactggtggcgaccgacaccatttacccgcacaccggacaggccgcaaaagcagcgatgaccgttgctgcgctgtgtgaaaaacataacgttgaactggtagcgatcggtaacggtacagcttcccgcgaaactgagcgtttctatctcgatgtgcagaagcagttcccgaaagtgaccgcgcagaaagtaatcgtcagcgaagcaggcgcgtcggtttactcggcttccgagctggctgcacaggagttcccggatctcgacgtttcgctgcgtggcgcggtgtctatcgcccgccgtttgcaggatccgctggcggagctggtgaaaatcgatccgaaatctatcggcgtaggtcagtatcagcatgacgtcagccagacgcaactggcccgcaaactggacgcagtagtagaagactgcgtaaacgccgttggcgtcgatctcaacactgcttctgttccgctgttaacccgcgtggcgggcctgacgcgcatgatggcgcaaaacatcgttgcctggcgcgatgagaacggtcagttccagaaccgtcagcaactgttaaaagtgagccgtctggggccgaaagccttcgagcagtgcgcgggcttcttgcgcattaaccacggtgataacccgctggacgcgtctaccgttcacccggaagcctatccggtggtggaacgcattctggcagcaacacagcaggcactgaaagatctgatgggtaacagcagcgaactgcgtaacctgaaagcgtctgactttactgatgagaaattcggtgtgccgacggtaaccgacatcatcaaagagctggaaaaaccgggtcgcgatccgcgtccggaatttaaaaccgctcagtttgccgatggcgtcgagacaatgaacgacctgcaaccgggtatgatcctcgaaggcgcagtgaccaacgtcaccaactttggcgcgtttgtcgatattggcgtgcatcaggacggcctggttcacatctcttcattgtcgaacaagtttgtggaagatccgcataccgtggtgaaagcgggcgacattgtgaaggtgaaagtgctggaagtggatcttcagcgtaaacgtatcgccctgactatgcgcctggatgagcagcctggcgaaaccaacgctcgtcgcggcggcggtaatgaacgcccgcaaaacaaccgcccggcagccaaaccacgcggtcgtgaagcgcagcctgccggtaatagcgcgatgatggatgcgctggcggcggcaatgggcaaaaaacgttaaacgcccgtactggcctacggttcgaatttgcacgaaatcgtagggcagataaggcgttcacgccgcatctggcaacgaacgccttgcctgacataaaagtgccggagaatatctccggcatttttattccacagccaaactcataatatattccggcaatatttatcatttcattaacaactgaaaccttaattaaacattagccagtccgggtaattcactattcgaattatattttcgctgcgatataaccttgagccacatcaacattgagtcagattattattcaaaccaacattcgcacacattttaagtattgctgatagaaaccattctcattatcattgtgttgttgattatttaatctctcctttgttggcaaatcatctggtctcatgtcgctgtcaaacgccccatgaggtagttatccagttaatgagaaacaagtaggcacctatgcaatacactccagatactgcgtggaaaatcactggcttttcccgtgaaatcagcccggcatatcgccaaaaactgctttctcttggcatgttacctggctcctcttttaatgtggtgcgcgtcgctccactcggcgaccccattcatatcgaaacccgtcgtgtgagcctggtattacgcaaaaaagatctggccttattagaagtggaagcggtttcctgttaatacggtgataacaacaatgaaaaaattaaccattggcttaattggtaatccaaattctggcaagacaacgttatttaaccagctcactggctcacgtcagcgtgtaggtaactgggctggcgttaccgtcgaacgtaaagaagggcaattctccaccaccgatcatcaggtcacgctggtggacctgcccggcacctattctctgaccaccatctcatcgcagacctcgctcgatgagcaaatcgcctgtcactacattttgagtggcgacgccgacctgctgattaacgtggtggatgcgtctaaccttgagcgtaacctgtacctgacgctacaactgctggaactcggcattccctgcattgtggcactgaacatgctcgacattgccgagaagcaaaatattcgtattgaaattgatgctctgtcggcgcgtctgggctgtccggtgatcccgctggtttcaacccgtggtcgcggtattgaagcgctcaagctggcgattgatcgctataaagctaacgagaatgtggaactggtgcattacgcacagccgctgctcaacgaagcagattcactggcaaaagtgatgccttccgacatcccgctgaaacaacgtcgctggctgggcctgcaaatgctggaaggcgatatctacagccgcgcctacgccggtgaagcgtcgcagcatctggatgccgccctcgcccgtctgcgtaatgagatggacgatccggcgctgcacattgccgatgcgcgttaccagtgcattgctgccatctgtgatgtggtaagcaacaccctgacggcagaacccagccgtttcaccactgcggtagataaaatcgtgctcaaccgtttcctcggtctgccgattttcctctttgtgatgtacctgatgttcctgctggctatcaacatcggcggggcgttacagccgctgtttgacgtcggctccgtggcgctatttgtgcatggtattcaatggattggctacacgctccacttcccggactggctgactatcttcctcgcccagggcctgggtggcggcattaacaccgtgctgccactggtgccgcagattggcatgatgtacctgttcctctccttccttgaggactccgggtatatggcgcgtgcggcgtttgtgatggaccgtctgatgcaggcgctgggcttgccggggaaatcctttgtgccgctgatcgtcggtttcggttgtaacgtaccgtcggtaatgggtgcacgtacgcttgatgcaccgcgtgaacgtctgatgaccatcatgatggcaccgtttatgtcctgcggcgcgcgtctggctatcttcgcagtattcgcggctgccttcttcgggcagaacggtgcgctggcggtcttctcgctgtatatgctgggtattgtgatggcggtgctgactggcctgatgctcaagtacaccatcatgcgcggtgaagcgacgccgtttgtcatggagttgccggtctatcatgtaccacacgttaaaagcctgattatccagacctggcagcgtctgaaaggcttcgttctgcgtgctggtaaagtgatcatcatcgtcagcattttcctgagcgctttcaacagcttctcgctgagcgggaaaatcgtcgataacatcaacgactcggcgctggcgtccgtcagccgggtgatcaccccggtcttcaagccaattggcgtgcatgaagataactggcaggcaacggttggcctgtttacaggtgccatggcgaaagaagtggtagtgggtacgctcaacaccctctacaccgcagaaaatattcaggacgaagagttcaatccggcagaatttaacctcggtgaagagctgttcagtgcgatagatgaaacctggcagagcctgaaagacaccttcagccttagcgtactgatgaaccccattgaagccagcaaaggcgacggcgaaatgggtaccggggcgatgggcgtgatggatcagaaattcggtagcgcagcagcagcttacagctacctgattttcgtcctgctgtatgtaccatgtatctcggtgatgggggctatcgcccgtgaatcaagccgtggctggatgggcttctccatcctgtgggggctgaatatcgcttactcactggcaacattgttctatcaggtcgccagctacagtcagcatccaacttacagcctggtgtgcattctggcggttatcctgtttaacatcgtggttatcggtctgctgcgccgcgcgcgtagccgggtggatatcgaactgctggcaacccgcaagtcggtaagcagttgctgcgcagccagcaccaccggtgattgccattaatggcttcacttattcaggtgcgcgatttgctggcgttacggggccgtatggaagcggcccagataagccagacattgaacactccacagccaatgattaacgccatgctgcaacaactggaaagtatgggcaaagccgtgcggattcaggaagaacctgacggctgcctctctggcagttgtaaaagctgcccggaaggaaaagcctgtctgcgcgagtggtgggcgctgcgttaaccttactccatcgcctgttttggaaagcccggtatgcgtctgcatccgggcttttttgcgtgcggctttccataaaaatgcaactcttgcagcacggcgtaagttcctttgaaagcatctcgcagggatgaaaactcgctaatacacaggtgtggagtggcgcgtagagtcgcggcattcaaacaacaggtgaaggaacgccatgagcaaaaagcagagttccaccccacacgatgcgctgttcaaactctttttacgccaaccggacacggctcgtgattttcttgcgtttcatttaccggcacccattcacgcgctttgtgatatgaaaaccctcaagctggagtcgagcagctttattgatgacgatctgcgtgaaagctattccgatgtgctgtggtcggtgaaaacggaacaaggaccaggatacatctattgtctgattgaacatcaaagcacctcaaacaaactgatcgcatttcgcatgatgcgttacgctattgccgcaatgcaaaatcaccttgatgctggatacaaaacgttgccgatggtggtgccattgttgttttaccacggtattgaaagcccctatccctattcgctgtgttggctggattgtttcgccgatcccaaactggcaaggcagctttatgcctccgcatttccgctgattgatgtcaccgtcatgcctgatgatgaaatcatgcagcaccgacgtatggcgctgctggagttaattcaaaaacatattcgtcaacgcgacctgatggggctggtagagcaaatggcctgcttattaagtagtggatacgctaatgacagacaaatcaaagggctgtttaattacatactgcaaactggcgacgctgtacgttttaacgattttatcgacggcgttgccgaacgttcaccgaaacacaaggagagtttaatgactattgcggaaagattgcggcaggagggggaacaatccaaagccctgcatatagccaaaataatgcttgaatccggagttcctcttgcagacatcatgcgctttaccgggctgtcagaagaagagttggctgcggcgagtcagtaaagttctgtctcgccatttcaaaagccacctacaccctctgcttcaacgccaccagcaggtgacaaaactcggccggatgcgaaataaatggcgcatgggccgctttggcgaagatatatgattcgctgtgaggccaaagtttatccagcatcggcaccactttgcgcggcaccagaccgtcgagatagccatacaatcgcaaaaacggcatggacacgttttgcagcggctgacggagatcgaccgttttcaggatttccagcccgccattaagcacgtcaacctccggcatcggtaacgccagaacggttttcttcaacgcccgcgcatcctggcgcgccgtttcagtccccatggtttgtaacgccaggaaccgctccactgtacgctgaaaatcatcactgagttgctgctgaaatcccgccagcacgtccggttttatccccggccactcgtcacgagcactaaaacaaggtgacgacgccacggtgaccagcgcctgaacacgctcgggatgggttaacgcaatctggcttgccaccagcccgcccagactccagcctaaccaaatggctttatcaggtgcctgttgcagcacggcttcggccatatcagcaagtgacagcgcaccaaatccccggctacgcccgaagccgggcaggtcaacaaggtgcagcgtaaaatgcgagctaagttcctcgtcaatgcaacgccacacttcggcattcagtccccatccgtgcagcagcacaagatgaacattcccctgacctttggtctgccaccagatgttattcatccgctattgttctcttttgacttacaaggatgaacatatgctaacagtaccgggattatgctggctatgccgaatgccactggcgttaggtcattgggggatttgttcggtctgttcacgcgccacccgcacagataaaacgttatgcccacaatgtggattacccgccacacactcccatcttccctgcggtcgctgcctgcaaaaaccgccgccctggcaaagactggtcacggttgccgactatgcgccgccgttaagtccgcttatccaccagcttaaattttcccggcgcagtgaaatcgccagcgccctgtcacgtctgttactattggaagtcttacacgctcgtcgcaccaccgggttgcaattgccggatcgcatcgtcagcgttccgttatggcagcggcgtcactggcgtcggggatttaatcagagcgatttgctgtgtcagccgttatcacgctggttgcactgccaatgggatagcgaagccgtcacacgtacacgggccactgcgacccagcattttctcagtgcccggctgcgcaagcgcaacctgaaaaatgcctttcgtcttgaattgcccgtgcaaggtcgccatatggtgattgtggatgatgtcgttaccaccggaagtaccgtcgcagagattgcgcagttgcttttacgcaatggtgcggcggctgtccaggtctggtgcctttgtcgaaccttgtagagcctcgatgatgggcgtattataaccaactaaaatagtcaactattaggccattactatgatccgtatttccgatgctgcacaagcgcactttgccaaactgctggcaaatcaggaagaagggacacaaatccgcgtatttgtgattaaccctggcacgcctaacgctgaatgtggcgtttcttattgtccgccggacgctgtggaagccaccgacacagccctgaaatttgacctgctgaccgcgtatgttgatgagttaagcgcaccatacctggaagatgcagagatcgattttgttaccgaccagttgggttcccagttaacgctgaaagccccgaacgccaaaatgcgtaaagtggcagacgatgcaccgctgatggagcgcgtggagtatatgctgcagtcgcagatcaacccacagcttgctggtcacggtggtcgcgtttcgctgatggaaatcaccgaagacggttacgccattctgcaatttggcggcggctgtaacggttgttccatggtcgatgtgacgctgaaagaagggatcgagaagcagctgctgaacgaattcccggagctgaaaggtgtgcgcgatctcaccgaacaccagcgcggcgaacactcctactactaagttatcccctcttttgtagattgcccgatgcgacgctaaagcgtcatttcgggcctacgttgaacatgtgccagacgttggcgcagcattgctttgtcaaatcctcggttcgtttccccgcgataatatgaccaacctctcataatttaaatttaccccgctctggtgattctcaaacgccagatgttacccgtatcattcacatgggtaccaaacatactcctgacatctgactacaataattagttttagtgggtatcagtcgtggtgccgcaatatctctgttcccgattgggataattagagtttgtcgtcagaaaattgacgttacccataacaaatgaaaggccaggtaaatcatgccattagtcattgttgctatcggtgtaatcttgttgttgctcctgatgatccgcttcaaaatgaacggcttcatcgctctcgtcctcgtggcgcttgctgttggattaatgcaaggaatgccgctggataaagttattggctccatcaaagccggtgtcggcgggacgctcggtagccttgccctgatcatgggttttggcgcaatgctgggcaaaatgctggcagactgcggtggcgcacaacgtatcgccaccacgctgattgccaaatttggtaaaaaacacatccagtgggcggtggtactgaccggttttaccgttggttttgccctgttctatgaagtgggctttgtgctgatgctgccgctggtgtttaccatcgcggcttctgcgaatattccactgctgtatgttggtgtaccaatggcggctgcactgtctgtgacccacggcttcctgccaccgcatccgggtccgactgcgattgccaccattttcaatgccgatatgggtaaaaccctgctgtacggtactattctggcaatcccgaccgtgattctcgccggtccggtttacgctcgcgtgttgaaaggtatcgataagccaattccggaaggtctctacagcgcgaaaaccttcagcgaagaagagatgccgagctttggcgtcagcgtctggacctctctggtgccggtagtactgatggcgatgcgtgcgattgccgaaatgatcctgccgaaaggtcacgctttcctgccggtagcggagttcctcggtgacccggtaatggcaacgctgattgccgtgctgattgcgatgttcacctttggtctaaaccgtggtcgttcaatggatcagattaacgacacgctggtttcttccatcaaaatcattgcgatgatgctgttgatcatcggtggtggcggtgcgttcaagcaggtgctggtagacagcggcgtggacaaatacattgcttccatgatgcacgaaaccaacatttctccgctgctgatggcctggtcgattgctgccgtactgcgtatcgcgctgggttccgcaaccgttgcggcaatcactgcgggtggtatcgcggcaccgctgattgcaacgacgggtgttagcccggagctgatggttattgcggttggttccggtagtgtgattttctctcatgtgaacgatccgggcttctggctgttcaaagagtactttaacctgactatcggcgagaccatcaaatcctggtcgatgctggaaaccattatctcggtgtgcggtctggtaggctgtctgctgctgaatatggtgatttgataacactgactgccggatgcggcgtgaccgccttatccggcctacgattcgggatgaattagtaggccggataagacgcgtcaagcatcgcatccggcatcaaccgcactctacttcttcttcgctgcagctctgcgccgtctgtccaaatccttcagcaacttgttcacgccatcatcggcaaacatcgactcaagcgttgcggaaagcttgcgtcgccagtttttatactggtaactggtgccaggaatattcaccggttcggccatatccagccagtcttccggctgtagtcctaacagagcactgttactgtcggcaatgtagcgctgcaaaccacggttcagcgtcggcgtcatcgacatcaacgatgccttatgcccggcacgtttcggcagacaaccatatttatgcagtgcatccagcagcccttgcttcgccagttcgcgatcctgatacagaccgcgcagtaccacttcatccggatacagccccagggttttgcccagcgttagatccccgcactcccagtaaccgcgcagcgttggcaggtcatgtgtcgccgcaaccgccatcgactgctccggatacgctttcggtgcacggaacgtcttctcgtggtcgttttcgaaatagagcactttgtaagagtacacaccgctgctgcgcagcttaccgacaatctctaccggtacggtaccgagatcttcaccaatcaccatacagcgatgacgtttactttcgagtgccagaatcgagagcagatcatccaccggatagtgaacatacgcgccctgatctgccgtctcgccatacggtatccaccacaaacgcagcatcgacatcacatggtcaattcgtaatgcgccgcagttttgcatattggcacgcaacagctcgataaacggttcataggcacgcgcggtgatgatatgcgggtccattggcggtaatccccagttctgccccaacgggccgaggatatccggcggcgcgccaaccgatgctttcaggcaatatagttcacggtcacaccaggtttccgccccaccttccgctacgccaaccgccagatcacgatacaagccaatcggcatttcatagccctggcttatctcccagcaggcggcaaactggctgtaagccagccactgcaaccagagataaaaatcgacgtcatcacgatgttcttcgcagaactgacgcacttctggtgaatccacgttctgatacatctctggccatgcaggccagccccagcgcatttcgtcctctttcacttgctgggcatgtagcgcatcaaaggctgcctgccagaacaggctgtcgccctgctctgcaacaaactggcgaaacgcggccatctgctcatcatcacgttgcgcgaaacctttccacgccattcgtaatgctgtcatttttagggcggtaaccgtggagtaatcgacccagtcggcatcgcgcgcctgttgcagcgtctgttgcgtggtcggcaactgccaccaggcctgagcctcttcgctaagatggaaatcttcaacggcgttaacgtcgatataaatcacattcagccaacggcgagaagacgggctgtatgggctggcgctctccggatttgccggatagagcgcatgaatcgggttcaggccaatgaacgacccgccacgttttgccacatccaccagcatcgctttgagatcgccaaaatccccaataccccagtttttttccgatcgcagcgtataaagctgaacgcaggcaccccacagcttttgtttattcagcaacgcctgcggttcgtaacagcgtttcggggcgacaatcacccggcaatgcgcgcgctggtcgtcctgggtgagtgtcagcgtgtgataaccttccggcagcttcgtcggtagattgaacgctttgccccccgttacatggcctttgtactgcgttccttcttcggtggtcagcagccagctatattcgccgctgccctccaccaccatcggcatttttttgccgctggtataaaccatgacattcgggactggcgttaccgccactttcgtggcggtacgttgatgcatcgcgtcaagcaaacgccgtttggtttcggcgctaatcgactgcggtttaccgtgggcattgatgtaattggggctaatccccgccgccagcgcggcattatccagacgtttgctttccatcgagcttccttagcgttttgcctgccagatacgagcctgataatcgcgaatagagcgatccgagctaaacataccgcagcgggcggtattgaggatcgccgcgcgagtccaggcctcctggtcgcggtacagcacatccacctgcttttgtgcctctacataggctgcgaaatccgccatcaccagatacggatcgccgccctgtttgccgatactgtgcagcatctggtcgaaggcatgcttatcgccgtcgctgtatttaccgctttccagctctttcaatactgcgtccagcaccttatctttcttccgccatttcaccgggtcgtagcctttggccagaattgccttcacttgttccacggtatgaccaaaaataaagatattttcttcaccgactttctcggcgatttcaacgttcgccccatccagcgtaccgacagtaagcgcaccattgagcgccagtttcatattgccggtaccggaagcttctttacctgcagtcgaaatttgttcggagatatccgccgccgggatcagtttttccgccgccgaaacgcaataatccggcaggaacaccaccttcaacttatcgccaaccagcggatcgttgttgatcacgtcagccactttgttgatcgcaaagataatattcttcgccaggtagtagcccggtgccgctttcgcgccgaagaggaagacgcgcggtacgcgatcagcctgcgggttttcacgaatttctttgtacaacgccagaatatgcagcagattcaggtgctggcgtttgtactcatgcaaacgtttgatctgaatatcgaaaatcgcctgtggattgatctcaataccggtacgaactttcacaaactccgccagacggactttattcgcctgcttgatctcgcgatattgctgacggaatttcgcatcatcagcgaatttttccagattgatcagctgatcgagatcgttagcccactctttttgcagtgatttatccaacagagccgccagtgccgggttgcactgtttgatccagcgacgtggggtaataccgttggtgacgttatggaatttgttcggccatagctggtgatattccgggaacagatctttcaccaccagatccgagtgcagcgccgcaacaccgttcaccgcgaaaccgccaaccacacacaggttcgccatatgcacttgtttgtcgtgcaccaccgccagtttggcccacactttttcatcgcccggccaggttttctctaccagcgttttaaagcgagtattaatttcgttaataatctgcatgtggcgcggcagtaagcctttcaccagtttcacatcccagcgttccagcgcttctggcatcagggtatggttggtgtaagcgaaagttttgctggtaatggcccaggcgtcatcccagctcatctggtgctcatcgatcagcacgcgcagcagttctggaatcgcgatagttgggtgggtatcgttcagctgaataacttcgtaatccgccagttcgtgcagtttacgccccgccagatgatggcgacgcaaaatatccgctaccgaacaggcacactggaagtattgctgcatcaggcgcagctttttaccggcagtatggttgtcgtttggatagagaactttggtcagtttttccgcattgatgccctgctgttcggcacgcaagaaatcaccgtcgttaaatttagtcagatcaaacggatgcgcgtgcgtcgcctgccacagacgcagcggctgcgccacgccattacgatagccgacaacggggagatcccacgcttgaccggtaatggtaaactccggctcccagcgtccgtctttcgtcactttaccgccaatccctacctgcacatccagtgcttcgttgtggcggaaccacgggtagttactgcgatgccagtcatccggcgcttcaacctgtttgccatcgacaaaagactggcggaacaaaccatattgatagttcagaccgtaacccgtcgcagactgaccgacagttgccattgagtcgaggaagcacgccgccagacgtcccagaccaccgttacccagcgccgggtcgatctcttcttccagcaggtccgtcagattgatgtcataagccttcaacgaatcctgtacatcctgataccagccgagattcaacaggttgttgcccgtcaggcgaccaatcaaaaactccattgagatgtagttaacatgtcgctgattcgccaccggcttggcgaatggctgagcacgcagcatttcggccagtgcttcactcactgctagccaccactggcgaggagtcatttcagccgcagaatttaagccataacgctgccactgacgtgaaagcgcttcctgaaattgcttatcgttaaaaataggttgtgacataggagttccacttttcttagattttcaacacaacgttatcgctagtttgccaggctcgatgttgaccttcctcatcctgcgggggattaggcagggaggagttgcggggatgagcaaggaaatgtgatctcaaccacttaaagctagtgcaaaccacaggattagcatcaaatcaatgcaatacagcgcagaaaatctgtatctaagtgcaaaaaatggccgttgcgtattttcaaaaagcggaaggtaactctataaattaagtaaaggagtgaaacagtttcataagtaaaatatccagtgtgctccatctcattcttaatagatttattaagatcatctttttagatggcactttcatcaggaatgaagaagaaacccttgcttaaatgaatctgatgaacataagggaaaccagtattcacgctggatcagcgtcgttttaggtgagttgttaataaagatttggaattgtgacacagtgcaaattcagacacataaaaaaacgtcatcgcttgcattagaaaggtttctggccgaccttataaccattaattacgaagcgcaaaaaaaataatatttcctcattttccacagtgaagtgattaactatgctgattccgtcaaaactaagtcgtccggttcgactcgaccataccgtggttcgtgagcgcctgctggctaaactttccggcgcgaacaacttccggctggcgctgatcacgagtcctgcgggctacggaaagaccaccctcatttcccagtgggcggcaggcaaaaacgatatcggctggtactcgctggatgaaggtgataaccagcaagagcgtttcgccagctatctcattgccgccgtgcagcaggcaaccaacggtcactgtgcgatatgtgagacgatggcgcaaaaacggcaatatgccagcctgacgtcactcttcgcccagcttttcattgagctggcggaatggcatagcccactttatctggtcatcgatgactatcatctgatcactaatccagtgatccacgagtcaatgcgcttctttattcgccatcaaccagaaaatctcaccctggtggtgttgtcacgcaaccttccgcaactgggcattgccaatctgcgtgttcgtgatcaactgctggaaattggcagtcagcaactggcatttacccatcaggaagcgaagcagttttttgattgccgtctgtcatcgccgattgaagccgcagaaagcagtcggatttgcgatgacgtttccggttgggcgacggcactacagctaatcgccctctccgcccggcagaatacccactcagcccataagtcggcacgccgcctggcgggaatcaatgccagccatctttcggattatctggtcgatgaggttttggataacgtcgatctcgcaacgcgccattttctgttgaaaagcgccattttgcgctcaatgaacgatgccctcatcacccgtgtgaccggcgaagaaaacgggcaaatgcgcctcgaagagattgagcgtcaggggctgtttttacagcggatggatgataccggcgagtggttctgctatcacccgctgtttggtaacttcctgcgccagcgctgccagtgggaactggcggcggagctgccggaaatccaccgtgccgccgcagaaagctggatggcccagggatttcccagcgaagcaattcatcatgcgctggcggcaggcgatgcgctgatgctgcgcgatattctgcttaatcacgcctggagtctgttcaaccatagcgaactgtcgctgctggaagagtcgcttaaggccctgccgtgggacagcttgctggaaaatccgcagttggtgttattgcaggcgtggctgatgcaaagccaacatcgctacggcgaagttaacaccctgctagcccgtgctgaacatgaaatcaaggacatcagagaagacaccatgcacgcagaatttaacgctctgcgcgcccaggtggcgattaacgatggtaatccggatgaagcggaacggctggcaaaactggcactggaagagctgccgccgggctggttctatagccgcattgtggcaacctcggtgctgggtgaagtgctgcactgcaaaggcgaattgacccgctcactggcgctaatgcagcaaaccgaacagatggcacgccagcacgatgtctggcactacgctttgtggagtttaatccagcaaagtgaaattctgtttgcccaagggttcctgcaaaccgcgtgggaaacgcaggaaaaagcattccagctgatcaacgagcagcatctggaacagctgccaatgcatgagtttctggtgcgcattcgtgcgcagctgttatgggcctgggcgcggctggatgaagccgaagcgtcggcgcgtagcgggattgaagtcttgtcgtcttatcagccacagcaacagcttcagtgcctggcaatgttgattcaatgctcgctggcccgtggtgatttagataacgcccgtagccagctgaaccgtctggaaaacctgctggggaatggcaaatatcacagcgactggatctctaacgccaacaaagtccgggtgatttactggcaaatgaccggcgataaagccgccgctgccaactggttgcgtcatacggctaaaccagagtttgcgaacaaccacttcctgcaaggtcaatggcgcaacattgcccgtgcacaaatcttgctgggcgagtttgaaccggcagaaattgttctcgaagaactcaatgaaaatgcccggagtctgcggttgatgagcgatctcaaccgtaacctgttgctgcttaatcaactgtactggcaggccggacgtaaaagtgacgcccagcgcgtgttgctggacgcattaaaactggcgaatcgcaccggatttatcagccattttgtcatcgaaggcgaagcgatggcgcaacaactgcgtcagctgattcagcttaatacgctgccggaactggaacagcatcgcgcgcagcgtattctgcgagaaatcaatcaacatcatcggcataaattcgcccatttcgatgagaatttcgttgaacgtctgctaaatcatcctgaagtacctgaactgatccgcaccagcccgctgacgcaacgtgaatggcaggtactggggctgatctactctggttacagcaatgagcaaattgccggagaactggaagtcgcggcaaccaccatcaaaacgcatatccgcaatctgtatcagaaactcggcgtggcccatcgccaggatgcggtacaacacgcccagcaattgctgaagatgatggggtacggcgtgtaagtttagccggataacgcgccagatccggcttacatctctgcatcattcaatgctcacccgcgttacgccatctgtttctatcaaactaaaccgcaccggcaagaaacgctccaccaccgcgatattggtcagcagatggcatgagggatgggcgaccgtaaattcccccgcgcccgccagcgccatcggtagcaccagttggtcagcaagatattcccccaccgccgccgtgcttgccaggtagcgtttcacctctttcaccaactgtgccgcaaccacctcggcactgacgcgcttttcaccgacgacaaaaaagcgttcggtgatattttcactttcgacttcaagcgagacggtattacccggcccctggtcgcgcggcaggttatgaatattctgttcatgcagggaaaaactccccgccagtgtagcgatttcacgctcagcaacatggcgcggcacaccagctaatagaacttctccacgcatctgcacaatgttcccgcgctcgccaagttgcaaggtgttaaacgatgccacgggcgagacttccgttgccaccacaccgcctccggcagggtaaaaaccgtggcgtaacagcgtggtttgctgatgaattcctattttcgccagcagcggctccagcacccggcggataaaatccgcaggcggcgccgacgggttatcggtgccgccgctcacttcaacacgcgaaggtccatcggcaaaccacagcgcgggcagcaccgtttgcagcaccagcgtacaacttccggcgctaccgatagcaaagcggtaatcgccgccgcgcacggtgccgggccggaagagcagacgctgcgaccccagctccgcgccttccacggttgctccgcaaatttccgtcgccgcctttaccgcggtcagatgctggcgcaacagccccggtttcgcccgcccggcacgaatgctggtgatggtaaatggctggccggttatcatcgacaggctcagcgccgagcgcaggatctgcccgccaccttcgccctgtgcgccatccagcgcaatcatccttttcatcatttatccttttacgcacaccacctgacgcagggtatagataacttccaccagatcgctttgtgccgccatcaccgcatcaatatctttatacgccatcgggatttcgtcgatcacttcggcatctttacggcattccacatgcgcggtggcacgaatttgatcttccacgctgaacagttttttcgctttagttcggctcattacccgcccggcaccgtggctgcacgaacagaacgactcttcatttcccagcccacggacgataaagctttttgctcccatcgaaccgggaataattccatattgaccagcacgcgcagacaccgcgcctttacgcgtcacgtagatctcttcaccaaagtgctgttctttttgcacatagttgtggtgacagttgatctcttccatcgccagcgtttgtggctgtctgaccgttttctgcgtaatgctctgcaatgccgttaccacgttttccatcatcgcatcgcggttaaggctggcaaaaagctgcgcccaggccacggctttcaggtaatcatcaaagtattccgtaccttccataaagtacgccagatcacgcgacggcaacgtctcaagcgtttcctgcatctctttttgtgccagatcgataaagtaagtcccgatggcgttaccaattccgcgtgaaccggagtgcagcataatccacacctggtccgactcatcaaggcagatttcaataaagtggttaccggttcccagcgttcccaggtgtttatagttattggtattcaggaaacggggatatttttgcgttaaccactgataaccggcttcaagctcagcccatttagcatcgacgttaacaggtggattttcccaggcacctttatcacgtttacaacggccagtggtacgcccgtgcggcacggccgtttcaatcgcctgacgcagctctgccaggttttcaggcaggtcttccgccgttaacgcggtacgcagcgcgttcattccacagccaatatccacgcccaccgccgccggaataatcgcccctttggtcgggatcacgctaccaatggtggaacctttacccaggtgtacatcaggcattaccgcaatatgtttgaaaataaacggcatcttcgccgtattaataagttgctgacgcgcatcggcctctaccggcacgcctttggtccacatttttaccggggcattttcagtggtcagtaattcgtaattcattttgtttttctcttttcgttgtttgctgtcctgataattgcaaccgtcgtgccagaaaattaaataagcagcttaattttttaattcattgttttaaaaaagattatatctttacgtccgtaaccggagatttcccgcaaagccaatttaccgataatgaaatatcgtcttttataaggatatctaagatgcgtaaaacagtggcttttggctttgtcggtaccgtactggattatgccgggcgcggcagtcagcgctggtcaaaatggcgtccgacactctgtttatgccagcaagaatcgttggtcatcgatcgactggaattgttgcacgacgcccgctcgcgctcgctatttgaaacgcttaaacgcgatatcgccagcgtttcgccagaaacagaagtggtgagcgttgagattgaactgcataacccgtgggatttcgaagaggtctacgcctgcctgcatgatttcgcccgtggttacgagtttcagccagaaaaagaagactatttaattcacatcaccaccggtacccacgtcgcgcagatttgctggtttctgctggcagaagcgcgttacctgcccgcccggctgatacaatcttcacctccgcgcaaaaaagaacagccgcgcggcccaggtgaagtaacgattatcgatctcgatttaagccgttataacgccatcgccagccgctttgccgaggaacgccagcaaacgcttgattttcttaagtccggcattgccacgcgtaacccccacttcaaccgcatgattgagcagatcgaaaaagtggcgatcaaatcccgcgcgccgattctgcttaacggtccaaccggcgcgggcaagtcatttctggcgcgacgcatcttagagttaaaacaggcgcggcatcagtttagcggcgcgtttgtggaagtgaactgcgccaccctgcgcggcgataccgccatgtcgacgctgtttggtcatgtaaaaggcgcgtttaccggggcgcgggaatctcgtgaaggtttattacgcagcgccaacggcggaatgttgtttcttgatgagattggcgaactgggcgcagacgaacaggcaatgctgctgaaagccattgaagagaaaaccttttacccgtttggcagcgatcgccaggtgagcagtgattttcagcttatcgccggaacggtgcgcgatttgcgccagctggttgccgaaggcaaatttcgcgaagatctgtacgcgcggatcaatctctggaccttcaccctgccgggtctacgccagcgccaggaagatattgaaccgaacctggattatgaagtggagcgccacgcctcactcactggcgacagcgtgcgttttaacaccgaagcgcggcgcgcctggttggcttttgcgacctctccccaggcaacatggcgcggtaactttcgcgaactttctgccagcgtcacgcggatggccacctttgccactagcggacgcatcactctggacgtggttgaagatgagataaaccgtctgcgctataactggcaggagagccgcccctccgcgcttacggcgttgctgggcgcagaggcagaaaacatcgatctcttcgaccgtatgcaactggaacacgttatcgctatctgccgccaggcaaagtcgctttccgcagccggacgccagctttttgacgtttcgcgccagggcaaagccagcgtcaatgacgcggatcggctacgcaaatacctggcgcgttttggtctgacgtgggaagccgtgcaggatcagcacagctccagttgaatatggtggtccgtcagcacctgcatcacgcttactggcggcggggcgtcggtgtagacggcatctaccatgctgatgctgcccatattgaccatcgcgttacggccaaatttcgagtgatcgacaaccagcataacgtggcgcgagttctcaataatggcgcgtttggtgcgaacttcgtggtaatcgaactccagcagcgagccgtcgctatcgatgccgcttatccccagaatgccgaaatcaaggcggaactgggagataaaatcgagcgtcgcttcgccaatgatcccgccatcgcggctgcgtaattcgccaccggcgagaatgatgcgaaaatcttcttttaccatcaacgtgttagcaacgttgagattgttggtgacaatgcgcaaattgctgtgattgagcagtgcgtgcgctaccgcttccggcgtggtgccgatatcgataaacagcgtcgagccattggggatttgctccgccactttgcgggcgatgcgctctttttcttcggtctgggtggccttgcgatcgtgccacggcgtgttaaccgaactggaaggcagcgccgcaccgccatgatggcgcaggatcaggttttgctccgccagctcattgaggtcgcggcgaatagtctgcgggctgacggagaaatgctctaccagctcttcggtactgacataaccctgctgtttaaccagttcgataataccgttgtgacgttgtgtttgtttcatttataaatccctggaattattttcgttttcgcgcattgagcgaatcaacaaaagccatcgctaaacccacggctaacccggcgatgtgtgctccgttcgccatcgacatcccaaacaaatcaaaccatccggcgacaatccagatcagcgcaaagataattaacccacgttgcaggtaaatgccactttgcggatcgcgttcgccacgtagccagacgtagcccatcagcgcatacaccacgccagaaagcccgccaaaccacggcccgctgaatttttgctgcacatagccgcttaacagggcgctgataagcgtaatgacaattagcttaccgctaccgaggcgtttttccaccgcaccgccgagataccaccaccagagcaggttaaagaggatatgcatcagcgagaagtgcattaacgcgtgggtgaagtaacgccagaactcaaatttcagtgttggatcgaatggccaggccagccataacatcacttcctgatcgccgagaatttgcatggcaataaacaccaccacgcaggcgatcatcatcacccaggttaccggacctgcgcgttcacgcaaggcggcaaagaaaggataacggcgataatgcaggccactgccggtatggcctgcctgccagctcgccgccagataacgcggatctgccgggttttcgagaaaacgcgccagctccgcccgtacgcgctcggcctgggactcatccgccagccagacatcgctttggttatgttgttgaatcgtgaggataacaccctgcgtcgccatgtaatcaacaaacgcctgcgccacgcgggggttagcaaaagaggtaatcatcaacatcgttgctgtcgcttattccacacaaaaggggacagtataaagcgttacgcgccgtacgccacctctgcgggaaactgacgttgccaggcttcaaagccgccgtcaatgctatagaccacatcgtagccctgttgcagcagatactgcgccgcgcctttgctgctattgccgtgataacacatcaccatcaccggagtgtcaaagtcgttatcacgcataaaagcgcccagcgtgtcgttggttaaatggaaagcctgcaccgcatgtcccattgcgaaactctgtggatcgcgaatatcgaccagcaccgcctctttttcctgcaacttctggtgcgcgtcggcaacgttaatacattcgaactgatccatgcgtctctctttctttacaaacaagtgggcaaatttaccgcacagtttacgtcgaagcggcagataaacgccataatgttatacatatcactctaaaatgttttttcaatgttacctaaagcgcgattctttgctaatatgttcgataacgaacatttatgagctttaacgaaagtgaatgagggcagcatggaaaccaaagatctgattgtgatagggggcggcatcaatggtgctggtatcgcggcagacgccgctggacgcggtttatccgtgctgatgctggaggcgcaggatctcgcttgcgcgacctcttccgccagttcaaaactcattcacggtggcctgcgctaccttgagcactatgaattccgcctggtcagcgaggcgctggctgaacgtgaagtgctgctgaaaatggccccgcatatcgccttcccgatgcgttttcgcctgccacatcgtccgcatctgcgcccggcgtggatgattcgcattggtctgtttatgtacgatcatctgggtaaacgcaccagcttgccgggatcaactggtttgcgttttggcgcaaattcagtgttaaaaccggaaattaagcgcggattcgaatattctgactgttgggtagacgacgcccgtctggtactcgccaacgcccagatggtggtgcgtaaaggcggcgaagtgcttactcggactcgcgccacctctgctcgccgcgaaaacggcctgtggattgtggaagcggaagatatcgataccggcaaaaaatatagctggcaagcgcgcggcttggttaacgccaccggcccgtgggtgaaacagttcttcgacgacgggatgcatctgccttcgccttatggcattcgcctgatcaaaggcagccatattgtggtgccgcgcgtgcatacccagaagcaagcctacattctgcaaaacgaagataaacgtattgtgttcgtgatcccgtggatggacgagttttccatcatcggcactaccgatgtcgagtacaaaggcgatccgaaagcggtgaagattgaagagagtgaaatcaattacctgctgaatgtgtataacacgcactttaaaaagcagttaagccgtgacgatatcgtctggacctactccggtgtgcgtccgctgtgtgatgatgagtccgactcgccgcaggctattacccgtgattacacccttgatattcatgatgaaaatggcaaagcaccgctgctgtcggtattcggcggtaagctgaccacctaccgaaaactggcggaacatgcgctggaaaaactaacgccgtattatcagggtattggcccggcatggacgaaagagagtgtgctaccgggtggcgccattgaaggcgaccgcgacgattatgccgctcgcctgcgccgccgctatccgttcctgactgaatcgctggcgcgtcattacgctcgcacttacggcagcaacagcgagctgctgctcggcaatgcgggaacggtaagcgatctcggggaagatttcggtcatgagttctacgaagcggagctgaaatacctggtggatcacgaatgggtccgccgcgccgacgacgccctgtggcgtcgcacaaaacaaggcatgtggctaaatgcggatcaacaatctcgtgtgagtcagtggctggtggagtatacgcagcagaggttatcgctggcgtcgtaaattaacgtaaggtgatcaggtcagatttcaatctggcctgagactgatgacaaacacaaaactgcctgatgcgctacgcttatcaggcctacgtggtttatgcaatatattgaatttgcatggtcttgtaggccagataagacgttcacgtcgcatccggcatgaacaaagcgcactttgtcaaaaatctaacctactttttaattcagggaattaccgcaaagcccacgccatcatacccaacgtaacaaaactcaggcacgttccccactcgccccgagaaaaatagcattaatgcgcccagcgccagcataaaaattttgagcagaaggtaaattgttggcgtgataaggatattacaaacttcaataataccggcaagtccgacacccagcatggcaataaccaccgccaaaaattgcgccagtatggggatgccgaaaaaagtcattaccagcgaggtcaaaatccattttctgttttgcattattctttccattctttttgaatggtgaaattatactccccgagtccccttgccccttctggacacttttccgaaatgatggcggaaaaaaacgggaccctttggccccgttctatttattggtgaacttacaatctcaccggatcgatatgccagatatgatcggcgtactctttgatagtacggtcagaagagaagtagcccatattggcaatgttcagcatcgcttttgcggtccactcttcctgaagctcgtagagttcatcgactttatcctgacaatcgacatagctgcgataatccgccagtacctggtagtgatcgccgaagttgatcagcgaatcaaccagatcgcgatagcgacccggatcttccggactgaatacaccgctgccgatttgcgtcagcacctgatgcagctcctcatctttctcgtagtattcacgcggtttgtagccctgacgacgcagttcttccacttcttccgctgtgttaccaaaaataaagatattgtcagcaccgacatgatccagcatctcgacattcgcaccgtccaacgtaccgatagtcagcgcaccgttaagcgcaaacttcatgttactggtgccggaagcttccgtccctgccagcgaaatctgttcagacagatctgccgccggaatgatcaactgcgccaggctaacgctgtagttcgggatgaacacgactttcagcttatcgccaatctgcggatcgttgttgatcactttcgctacgtcattgatcaaatgaataatgtgcttcgccatgtaataggccgaagccgccttaccgccaaaaatattcacgcgcggtacccacttcgcatccgggtcggccttgatgcggttatagcgggtaatcacatgcaacacattcatcaattgacgtttgtattcgtgaatacgtttgatttgtacatcgaacaacgcctttggattcaccaccacattcagctgctgggcgatatactctgccagacgctttttgttctccagcttcgcctgatgcacagcgtgattaaccattgggaaatcacagtgttgttgcagctcattaagcaggctaaggtcggtgcgccagttacggcccaggtgttcgtccagcacggctgaaagcgatgggttcgctaccgccagccagcgacgcggcgtcacaccgttggtgacgttggtgaaacgacccgggaagattttcgcaaagtcggcaaacaacgattgcaccatcagattagagtgcagttccgatacaccgttaactttgtggctcacaacaaccgccagccaggccatacgcacacgacgaccgttggattcatcaatgatcgacgcccgtcccagcagatcggtatcgttcggatactgttcctgcaaggttttcaggaaatagtcgttgatttcaaagatgatctgcaggtgacgcggcagaattttacccagcatatcaaccggccaggtttccagcgcctcgctcatcagcgtgtggttagtgtaggagaagacctgacaacacacctcaaacgcgtcgtcccagctaaattggtgctcatcgatcagcagacgcatcatctcaggaatcgacagtaccggatgggtatcattgagatgaatcgcgattttatccgccaggttatcgtaggttttatgcaactgataatggcggcttaaaatgtcctgaatggtcgaggaaaccaggaagtattcctgacgcaggcgcagctcacgcccggagtaggtggagtcatccggatacagtacgcgagatacgttctcggagtggtttttatcttccactgccgcgaagtagtcaccctggttgaatttaccgaggttaatttcgctactggcttgcgcactccacaaacgcagcgtgttggtcgcgtcggtgtcgtaaccagggattatctgatcgtaagcgactcccagaatctcttcggtttcaatccagcgcgtttttttaccttcctgctgaatgcgaccgccaaaacggactttatagcgcgtgttgtggcgtttgaattcccacgggttaccgtattccagccagtagtctggcgactctttctggctaccgttaacgatgttctgcttgaacataccgtagtcatagcggatgccgtaaccgcgccccggcaaccctaacgtcgccagagaatcaaggaagcaagccgccagacgtcccaggccaccgttaccgaggcctgggtcattttcttcatcaatcagctcttcgagatttaaccccatcgcttccagtgcgccctgtacatcttcgtaaattcctagcgacaacatggcgttggagagcgtacggccaatcaaaaactccatcgacaggtagtaaacctgacgagtttcttgcgacaactgggcacggtttgaacgtaaccagcgctccacgagacgatcgcgcacagcaaataacgttgcgttcagccattcatgtttattggcgacgaccgggtcctttccaatcgtaaacatcagcttgtaagcgatagagtgcttaagagcttctacgctaagcgtgggcgatgaatatgtaaacggagcattcatataggcgtttcctgaaaactatttcaagcgatagtaaagctcacggtacgacttcgccgcgacctgccagctaaaatccattgccatagcctgacgttgcacaaaccgccacagtgaaggacgggaccacagtacaaaagcacgtcgaatagcccgtaacagcgaccaggcattactatcttcaaagacaaacccactggcgacgccatctgcaaggttctcaagagaacagtcagaaaccgtatcagcaagcccaccggtgcgccgcactaacggcagcgtaccgtacttcaatccataaagttgcgttaagccgcacggttcaaaacggctgggcaccagaatgacgtccgcgccgcccataatgcgatgcgaaaatgcttcgtgatagccaatctgaacgcccacctgaccggggtattccgctgccgccgcaaggaaaccttcctgcagcaccggatcgcccgcgccgagtagcgccagctgcccgccctgctccagaagacccggtaaggcttccagcaccaggtcgagacctttctggctggtcagacggctcaccactgcaaaaagcggcactttatcgtcaaccttaagccccattgcgatttgtaactggcgcttattttccgctttatcttccaacgtatcgcgggtgtaacgcgaggccaacagtaagtccgtctctggactccagattttctcgtccacgccgttcagtacgccggaaagacgcccttcacggtgacgctgttgcaacagaccttccataccgtaggcaaactgcggttcggtgatctcgcgagcgtaggttggactgaccgccgtaatgtgatcggcatagtacagaccggccttcaggaaagagatttgtccgttgaattccagcccatgaatattaaagaatgaccatggcaattggatgtcattcatgtgatgtgcataaaacatgccttgataggccaggttgtgcacagtaaacaccgacttcgccggacgcccgcgcgccgccagatacgcaggcgcaaggcctgcatgccagtcgtgcgcatgcaccacatcaggacgccagaatgggtcaagcccgctggccatttctgccccaacccaccccagcagcgcaaaacgcaatacgttgtcggtataggcaaataagttggtatcgtgatacgggcttcccggacgatcatagagatgcggcgcgtcaatcaggtaaatgccaaccccgttgtaatgaccgaacaacagcgtgatatgtccggcgaaggtatcacgacgggatactacctgcgcatcggtcacgccacggcgaatatcgggaaatgcaggcaacagtacgcgagcgtcaacgccgtctgcgatttgtgctgcgggtaatgccccaataacatcagccagaccgccggttttaagcagcgggaacatctctgaacatacatgtaaaacctgcattatcgctcctgtttatgccctaacttccgtagcatttcgcgcgttaccagcacgatgccttcttctgaacgatagaaacgacgtgcatcttcctctgcgttttcaccaatcaccatgccttccggaataacacaagcacgatcgatgacgcagcggcgcagacggcacgagcgacctacccatacttccggtaacaatacggcggaatcaatgttgcagaatgaattcacgcgaacgcgcgagaacagaacggactgcaccaccaccgaaccggagatcacacaaccgccggaaaccagtgagttaagggtcatcccgtggctaccggagcgatcctgcacgaatttcgctggcggtaatgattcattgtaggtgcgaattggccaattgcgatcgtacatatccagttccggcaccacagaggccagatcgaggttcgctttccagtaagcttccagcgtacccacatcgcgccagtacggctcggcatccgggtcggattgtacgcaagagagcgggaacgggtgcgcataggccagaccggcttcggtgatcttgggaatcaaatctttgccaaagtcgtggctggagttctcatcgcgatcgtcttcttccagcagttcatacagatagtcggcgtcaaagacgtagatacccatactcgccagagatttgctcggatcgttcggcattgacggcgggttagcaggtttttcaacgaattcgataattttatcgttctcatcaaccgccataacgccaaatgcggaggcttcttcaatcggtactggcatacaagcaacggtgcaacgtgcgcctttttcgacgtgatcgataagcatacgcgagtagtcttgcttgtagatatggtcgcccgccaggatcaccacgtattccgctttataacggcggataatgtcgaggttttgggtgaccgcatctgcggtgccgcgataccagttttcccctttcattctctgctgtgctggcagcagatcgacaaactcgttcatttcttcattgaagaatgaccagccgcgctgaatgtgctgcaccagagtgtgggactggtactgggtgatcacgcccatacgacggatcccggagttgatgcagttagacagcgcaaagtcgataatgcggaacttaccgccgaagtgtacggccggttttgctcgcttattggttaaatccttcaggcgggtaccacgtcctcccgccagtatcagggcaacagatttcaatggcagctggcgcgccaacattaagtgatcgttcttctctaaactaaccatgactaactccttttttatcatctctggaacacacacaatccgtgtgcaggtccctgccagacagccgtaatcactgggttatcctctccagcgaatgggggaatggcgtgccactccccagcaggtaaaacaatctctgttacctcaagcgtggcgttaattgcgatcaaaaagcgatccgagagcagaatttgcagctgtttcggcccgttttgccactcatccgtgcttaaaggttgagcatatcgatttagccaacggacattgccgtcgccttcttcccaccagcgattctccaccaaagcgggaatgcgcttgcgcagatggattaacgcggcggtaaatgcggttaaaccactgcttgcctgcgaccagtccaaccaggttaattggttatcctgacagtaggcattgttattgccatgctggctgtgaccatgttcgtcaccggccagtaacatcggcgtaccctgggagagcaacaacgttgttaacagggcgtgaatgctgtcgcgccgccgttcaaccaggtcaagagaaccgcctaacccttctttaccatgattgttactgtaattgttgttggtcccgtcgcgattttcttctccgtttgcttcattgtgtttatggttgaagcaaacgcagtcgcgaagcgtaaaaccgtcatgcgcggtgacgagattaatcgcggcactcggcagacgaccattacgtttaaaaacatcgctggaggcagcaaaacgcccggcaaacgcccccagaggcaaatcataatgtagccagaaacgacgggcagcatcgcggaaatgatcgttccactcggcaaacagcggcgggaaatttcccacctgataaccaccaggagcgatatcccacggttcagcaattaacttcacctgcgagagcaccgggcagttctggatagcggtaaacaacggcgcatcctgacggaactctggcgtacggcccatgactgccgccagatcaaagcggaaaccatcgacgtggcaggtttctacccaataacgcaggcaggcgctggcataatccaccaccgccggatgactcaaattgagcgtgttgccgcaaccggtccagttgtgataatcgccgtcttctcttatccaataatagctacggttatcgatcccacgcagcgagaataacgggccgtcgaggtccagttccgcactatggttgagcacgatatcaagaatgacttcgatacccgctttatgcagtgctttgattgcatcgcgaaactcatccagcgccgtttctggcgagcaggcatacgccggatgcagcgcaaacatcgccaccgggttgtaaccccagtagttacttagccccatgcgttgcagacgtggttcactggcaaactgcgccactggcagcagttccagcgcggtaatgcccaattgtttcaaatagttgatcatcaccggatgcccgagggctttataagtgccacggatctcgaccgggatctccgggtgcaagtacgttaatcctttgacatgggcttcataaatgatggtgctgccccacggcgtgcgcggcggggcatcatcttcccagtcatagtgatcaaccaccactacgcatttcggcgcaatggcggcgttgtcgcgatagtcaggttcattatgaccggcgtgcagcagcgggttatctttaaactccccgtcaatttgccgcgcgcaaggatcaatcaacaacttcgccgggttaaagcgatgcccctcggcgggttgccaggggccatgaacgcgataaccataacgcaaacccgggcgcgcatccggcagataaccgtgccaaatgtcgccactgtgccctggcaagtcatagcgatgttcctggccattggcgtcaaagacacacagttctacccgctcggcatgagcggagaaaagtgtgaagttgacgccctgaccgtcgtaatgcgcgccgaggggagcgggtttgccaatggcgagttgtgtcattctgcctcccgaaccagccagatagtggccagcggtggtagcgtcaggcttagtgaatgctgacgaccgtggctggcaatctcatcgctgtgtaccgtgccgccattgcctgcattactgccgtgatagtgcatggaatcggtattgaggatttcacgccatttgcccggctggtttatgccgaagcgataatcatgacgcggtaccggcgtaaagttactggcaacgatgatttcgttaccctctttatcgcgacgcacaaagatcagcaccgagcgttctttgtcatccaccaccagccattcaaagccgtacgggtcaaaatccagttcatgcattgctttatggtggcggtaggtgaggttcagatcgcgcaccagacgctggacaccgtggtgccagttatcgccgccttccaacagatgccagtcgaggctggcgtcatggttccactcgcggccctgggcaaattcgttacccatgaacagtagtttcttgcccgggaatgcccacatccagccatagtaggcgcgcaggttcgcgaatttctgccatgcgtcgcccggcatgcggtcgagaatcgattttttaccgtggaccacttcatcatgcgacaacggcaggacgaagttttcagtgtagttgtagagaatcccgaaggtcagtttatcgtgatgatactgacgataaaccgggtcgagcttcatgtagtccagggtgtcatgcatccagccgaggttccacttgtaccagaagcccagaccgcccatatcctgcggacgagaaacgccagggaaatcggtagactcctcagccattgtcaccgcaccggaaacctgctcaccaagaatacggttggtattacgcaagaattcaatcgcttcaagattctcgcgcccgccaaattcgttcgggatccactccccctctttacggctgtagtcgcgataaatcattgacgccaccgcatcgacgcgcagcgcatcaataccaaaacgttcaatccagtaaagcgcgttaccgacgaggaagttactgacttcacggcgaccatagttgtagatcagcgtgttccagtcctgatgatagccttcacgcggatcgctgtgttcatacaagttcgtgccatcaaattcggcaagcgcaaagtcatcagtcgggaagtggcctggcacccagtcgagaatcacgttcagaccagctgcgtgtgcggcatcaatgaaataacggaagtcgtcgcgagtaccaaaacggcgggttggcgcatacaggccggttggctgataaccccaactgccatcgaagggatgctcgttaatgggcagtagttcgaggtgggtaaagcccatccatttagcataaggcaccagttgatcggccagctcgcggtagctcaaccagaaattgttgtcggtgtggcgacgccaggaacccaggtgaacttcataaatagagattggcgcatcaaactgattcgcttttttgcgctcttcagtctgtacaaccttttccggcagcccgcaaataagagacgcggtttccgggcgcatttgcgcttcaaaggcataagggtcggacttcagacgcaagttgccattggcatcaatcatctcgtatttatagagctgaccgttatgcgccccagggataaacagttcccagatgccgctctctttacgcaggcgcatcgggtgacggcgaccgtcccagtagttgaattgcccaaccaccgagacccgacgggcgtttggagcccagacagagaaacgcgtacctgtgacgccatccatagtatctgcatgcgcgcctaaggtttcatacgggcgcaggtgagtaccttcagataatagccaggcatccatttcctggattagcggaccaaaacggtaaggatcatcaatcaggttttgctgaccatgccagacaacagccaactgatagcggaaaaaattcttacgtcgcggaatgacgccgctaaagaatccccgtgagtcgagacactccagttttgcgagtttgcgcccggttttcggttcaatcacccacacatcggtagcgtcgggtaaaagggcacggacttccagtcccgcggtggttttatgcattcccagtacggaaaaaggatccgcaaaatggcctgcaattagcgcgttaatcacgtctctatcgatacgatcggacatgcttgtcttcctgttttattgtgtcaccccatccaattggatttttgacttctggttgtgacatttttttgacctgaacggcgcagcactctgtgcatcctctctgcgtcgtcctcacttcaggtaaggctgtgaatactcatgtattcagccacccttaaagaatagccaatgctctatttaactcccggtaaatcatgaaacatctgcgcttactcctgtattacgcactaacaggggcggcatcgcgccccagatttaatgaataaagattacgccagttgacgaagcatccgacgcagcggctccgcggccccccacagcagctggtcgcccacggtaaaggctgacaggaactctggtcccatattcagcttacgcaggcggcctaccggcgtggtcagcgtgccggtaacggcagctggggttagctcacgcatagtgatttcccgatcgttcggaacgactttcgcccacggattgtgcgcagccagcagttcttccacggtcggaatagacacatcttttttcaatttaatagtgaatgcctggctgtggcagcgcaatgccccgacacgcacacataaaccatctaccggaattacggaagatgtgttgaggatcttgttggtttccgcctgccctttccactcttcgcggctctgaccgttatcgagctgtttgtcgatccacggaatcaggctacccgccagcggcacgccaaagttatccaccggcagctcaccgctacgggttaaggttgtgactttgcgttcgatatcgagaatagcagaggacggggtcgcgagttcatctgccacatggccatacagatggcccatctgggttaataactcacgcatatgtcgcgcaccaccgccggaagcggcctggtaggttgcaacggacacccaatcaacaagatcattggcgaataaaccacccaacgacatcaacatcaggcttacggtacagttaccgccaacaaaagtcctgatgccattatttaatccgtcggtaatgacgtcctgattgacggggtcaagaatgatgatggcgtcatctttcatgcgcagagacgatgctgcgtcaatccagtaaccttgccatccgctttcacgaagctttggatagatttcgttggtataatcgccgccctgacaggtcacaatgatatcgagggcctttagcgcctccagatcaaaggcatcctgaagtgtgccagtggttccgccaaaagacggcgcagcctggccaagctgagaagtagaaaagaagacagggcgaatggcgtcgaagtcgcgctcttcaaccatgcgttgcatgagaacggagccgaccataccgcgccagccgataaaaccaacatttttcataagcgtttttttcctgcaaagatgtgtgctgtataaatgtgccggtctcctcttggcacatctttcaccatacaaaaagcagccaaagtcgcaagtgaaattaatcaatgatagcgaagccatcagtaatgcgacttatcctgctttgttagcacgcagaaagtccgcggcaattatcagggaatttgagttatgaatgaaatcatttctgcagcagttttattgatcctgattatggatccgctcggaaacctacctattttcatgtccgtactgaaacatactgaaccgaaaagacggcgggcaatcatggtgcgagagttgcttattgctctcctggtgatgctggtgttcctgtttgcgggtgagaaaattctggcatttcttagcctacgagcagaaaccgtctccatttctggcggcatcattctgtttctgatcgccattaaaatgattttccccagcgcttcaggaaatagcagcgggcttccggcaggtgaagagccatttatcgtgccgttggcaattccgttagtcgccgggccgactattctcgccacgctgatgttgttgtctcatcagtacccgaatcagatggggcatctggtgattgctctgctgctggcctggggcggcacctttgtcatcctgctacagtcttcgctatttttacgtctgctgggcgagaaaggggtgaacgcacttgaacgcctgatgggattgattctggtgatgatggcaacccagatgttcctcgacggcattcgaatgtggatgaaggggtaacgaggagagtttttcgaaaagaacccggtagcgtcacaactaccgggcgaacaaacttaactcaacagctggaacgcaatcatcccaacgatggcaccgacagtgccgaggatggtttccatcatggtccaggttttcagcgtttcggcttcggtcgcgccggtaaatttaccgaacaaccagaaaccggcgtcgttaacgtggctgacaacaatcgaaccaccagcgatacaaatcgacagcgccgccatttgcgcaccggagtagttcagttgttcaataaccggcatcaccagtcctaccgccgttaaacaggctacggtggcagaaccctgaatgatgcgcactgcagctgccagcacgaagcaggtgatagcaatcggcaggcccatgccggttaacgcttcgcccagtgccggacctacgccagagtcaaccagcacctgtttgaacacgccgcccgcaccaatcaccagcagaatgatccccgccggttgcagcgcgtgaccgcaaatctccatcactttgtcttttggcatgccctgacgcattgccagaccgtaaatcgccaccagacaagcaaccagaatcgcggtaaacggatgaccgataaactcaaaccattcgtaagcagttgatccttccggcacaaaacgcgcggcaatggttttcagccctaccagcaccagcggcagcaggatcagcgacaggctgaatccgaaagatggcattttgccttcgccgagatgcggttcgctgatgtcgtcaggaatatgcagctcaacgtaacggctgatgaagttaccccacagcggcccggcaataatcattcccggaattgccgcacacaggccaatcaggatcatccagccaaagtcggcattcatctgcgatgccagcagcatcggcgctggtccaggcaccagaaatgccgccgctgccgccacgcctgcaaataatgggattaccagcttcaccaggttcgtaccggtgtggcgcgccattgagaaagcaacgctaatcagcagaactatcgccacttcaaagaacagcggtagcgcacagaccagccccgcaaggccgatggcataatgcgcgcggctgtgaccgaaggatttgagcattttgacggcaatctgatcgactgcgccggtttcatgtaagatcttgccaaacatagctcccagggcgacaaccaccgccaggaagccgagggtgcctcccatccctttttccatcgtcgctgcgattttatcgagcggcataccagaaaaaaggccagcccccatggacaccaccattaaagccaggaaagcgtgcatacgcgccttcatgactaaaaacagcagcagtaaaacagaccctactgctgttaaaacaagcgttaatgtagtcactacttatttgccttttttaataacctcaatggtgcttgccacaacaccttccagcggttgatcgatatccaccaccagtacatcggtttcgtccgcacccggctcctgcagcgtttcaaactgcgtcaccaacatttgggttttaaagaaatggcctttgcgcgctttcaggcggctttcaatcacatcaaaatcgcctttcaaatagatgaaagagagattcggattaccttcacgcagcaagtcgcgatagtgttttttcaatgcagaacagacgatcagcgacactttattagtgcgctgcatagcaaacgcggcgtcgttcagcgcctgcaaccacggtttgcgatcgtcgtcattcagtggttcgccagacgccattttttcgatattgcgccgtggatggaggaaatcgccatcaagaaacgcggcatgaagttgatgcgccacttcactggcgaccgcagatttgccgctgcccgatacgcccatcaagacgtaaatgtggtgatcatggttagtcgtgctcaaagtggtgcccccacaatacaagaattaaaaatgttacgggtaactgttatcggtaacattgtccagccggacaatatcagaagcaatatccatccatgccttaagtgtataagtgtgagctacttcaaatttgtgggcttaaatagatccgcccggtgacaaggtgaaacctaaatctaacattttcggtgtcacagattcgccacgaatacgcgccagcaggcgttcagcgccaatactgcccatccgctcacgcggcgtcagcacgctcgcaagtcgtggctccatcacctgaccaatgtcatgaccgtggaaaccggcaatcgccatatcgtcaggaacttttaaccccagacgctgacattcaaacgccgcgccgaccgccaggtcatcattcgtacagaacacgccatccagctgcggatattcccgccgcgcctggcgaatcagttcaataccggaagagtaagaagaagattgctcaaccatcacgctatatggcaccaggcctgcatccagcatcgcctgttcgtatcccttctgtttgatgatagtacgttcgtcgagacgtgcgccgagataggcaatgtggcgatgcccgcgagcaataatggcagtggtcatctggcgtgctgcttcaaagttatcaaaaccgacggcgatatcaaggcatggcgacttgctgtccatcagttccaccacgggaatacccgccacttcaatcatctttaaggtgcgcggcgtgtgggtacgttcggtgaggatcaggccgtcgatattccaggagagcatggattcgaggcgttcttgctccatttccggtttataaccgtagtgcgccagcatggtctgataaccgtgcgcgtcggtgacgctttcgattccgcgtaatacttccgcgaaaacctggttggtgagagaaggtaacaggacgccaatcgcccggctggtggcgttagagaggatatcgggcgcacgattgggaatatagcccagttcatcaagagccgcggcaatcttgccgcgtagagcgacggaaacctgctccgggttgcgtaaaaaacggctgaccgtcattttggtcacgcctacacggtcagccacatcctgaagtacgggtcttttctttttcatcgtcctgaaggtacaaaagagatagattctcttagtttaacacggacacatcagaaccttcccggggaaaacagtgcttgtttacaattattagatatacactaaatcaattgcatcgcattgtgctaacgacgcggcaaaaccccggaagcgtacatcagcacgcgaccggagcgagcgaggaagcctgcaaaaaggcaggcttcaaagatgccgttgagttttaaaccggcggcagatcgaacagtaacacttcgctgtcgctatccgcatggatggagattgcctgctcatcccagattgccagaccatcgctggtcgaggctttcacgccgttaatggtgacattgcctttcaccacctggatccagacgcggcgttcagcggcaatctgatgcaccgactgctcatctttcagcaacgcccagcggtacagttccatatcctgatgcactttcaatgaaccatctcgcgcatccggcgagagcaccagctgtttgccctgtacggcatcgaagcgacgctgttcataacgcggcgtaataccgttttcttcaggcatgatccagatctgatacagatgcagacgctcggtgctgcttgggttgtactctgagtgacgaatacccgtaccagcactcataatctggaactcacccgccggaacctgctctttattgcccatgctgtcctgatgctcaacagtaccttccagcacgtaggtcaaaatttccatatctttatgcgggtgagtgccgaagccctgccctgcttcaatcacgtcgtcgttaatcacgcgcagcgcggagaagcccataaagttcggatcgtaatagttggcaaaagagaaagtatgccaggagtccagccagccatgatttgcatgaccacgttcatttgctttgcgtaagtagatcatttgtattcgccccctgaatgatttcgatgggcttagtgtggacccgatctgcctgggatgatagagggtgaaaattgacccctctgttcaaaaaaattgaactattcgaggggccatcaaacttacttagcgagagttactgtggagggagaggcttgctcaaatccgcgttcaaggatttccagattggtaagaacttcagattccttgacgtaatttggcgcaccgtgggtgatggtttgatacaacgcatcataaacgcgcccgtaatcgcccatctccggcttcatctcttctctgaccgtcacgccctcgtcattgacatactccagcacaccgaccgaatcatccgctgcgaatcccggttcgcccggcataatattagccttcaggctggtttcctgctggtcgataccgtatttaataaacgaacctttcttaccgtgaacgataaatttcggataatcgattttcaccagatggctggttttgacgatggctttcaggtcgccataaaacagttgcgcttcaaaggtgtcgtcaggattggctttattacgcaggctgcggatgtcataagcgacgtgatccgggcgaccgaacagagaaataatctggtccatcgtatgcacaccaaggccataaaacgcgccatcctgcggcagcccaggtttggtttctgccaccgggcggtaatagtcaaaatggctttccacttcaacaatctctcccaacttgccactttcaatcgcttttttcgctgtcaggaagcaggagtcaaagcgacgattctgatacggcgtgacggtcagccctttgcttttcgccaacgcaaacagctctttcgcctgcgcaagtgtcggagtgaacggtttttcgaccagcacatttttcccggcttccagcgcgcgtttcgcgtactcgaaatggctgtccgcgtgggtgcagacaacaaccagcttaacatcgggatcgtttagtacttcgtcgagatcgctggtgaaatggatatgggaataaatgggagcctgttcttccggcttcgcatggcgacgaaaaatatgcgcgacatgccagctatccttgcggttaagtacatacggcagatggtaacgggtggtgcttttgccgaagccaataaaggcgcagttgatgaccatgatttcgtcctttttaaggtggttatttacaccttagcgcaaagcggacgtggttcctactggagtgcgcataacgaacacaagcactcccgtggataaattgagaacgaaagatcaaaaaaaaagccagcacccggctggctaagtaatactggaagcaatgtgagcaatgtcgtgctttcaggttctccgcgagggtcttcctgatcgcgagacaataataatcattctcattcgcacttgtccaacactttttgcaaaaaaatgcatttgactcgcatttgaaagtcaatgatgttgaaagggacatttaccccaaagaggacaaaggaatgagtgagatagtaatacgccacgcagaaacacgggattacgaggccatcaggcagattcacgcccagccggaggtgtattgcaacacactacaggtgcctcatccttccgatcatatgtggcaggagcgactcgccgatcgtcccggcatcaagcaactcgtcgcctgtattgatggagacgtcgtgggccatctcaccattgacgtgcaacagcgcccacgccgcagtcatgttgccgattttggtatctgtgtcgactctcgttggaagaaccgcggcgtcgccagcgccctgatgcgagagatgattgaaatgtgcgacaactggttgcgggtagatcgcattgaactaaccgtgtttgtcgataacgccccggcaattaaggtctataaaaaatacggctttgaaattgaagggactggtaagaagtacgcattgcgtaatggtgaatatgtcgatgcatattatatggcgcgggtgaagtaagatagtgccctttttctgagatggaaaaagggtgtcattcaaaatcgacataccttcctttaaggtatttatttgcccaatacatatattgagatttaactcataattacttcctaaagtgtaatattttattttttaatatatacgcctacaatttcctggagtaaataaataacaattaacaagcataatattgccattgataaaatagcatgccataaaaggacttttcagggatgagtaatattgtttacctgacagtaacgggagaacaacaaggaagcatctccgcaggttgtgggacttctgagtctacaggtaatcgttggcagagcgggcatgaggatgaaatatttacattctcactcttaaataatattaataatacggggcttggttcacagttccatggtataacattttgtaaattaattgataaaagcactccattatttattaattccattaacaataatgaacaattatttatgggatttgacttctatcgaataaatagatttggtagattggaaaagtattattatatacaactaagaggcgcttttttatcggctattcatcaccagatcattgaaaaccaactggatacagaaacaataactattagttatgaatttatcctctgtcaacatcttatcgcaaataccgagttcagctatttggcactccctgaaaattataaccgtttgtttttaccaaattcaaaaaaccaaacaaataatcgtttcaaaacgttaaacagcaaagctattggcaggctacttgctgctggtggcgtatacaatgggaacattgaaggattcagagatactgcggaaaaactgggtggagatgcaataaaaggctatgatcaaatactaaatgaaaaaacagcgggcatagcgatagcaacagcatctattcttttaacaaagcgttctaatgttgatacatatacagaaataaatagttacttaggcaaacttagaggtcaacaaaaacttcttgatggtatagacataatagaaataatatacattaagagaccttcaaaagacttagctaacttacgaaaggagtttaataaaactgtaagaaaaaattttcttatcaaacttgcaaaaacctccgaagcatctggaagattcaacgccgaagaccttttaagaatgagaaagggcaatgttcctctaaattataatgttcaccataaactatctctagatgatggtggtactaatgatttcgaaaatttagtattaatcgaaaacgaaccatatcataaagtttttactaacatgcaatcacgaatagctaagggaatattagtaggtgaaagcaaaatcactccctgggccattccatctggctcaatttatcctcccatgaaaaatattatggaccacacaaaatgatgactaaaacccaaataaataaattaataaaaatgatgaatgatttagactatccatttgaagcaccgctcaaggaatcatttattgaaagtataatccaaatagaatttaattctaattcaactaattgcctggagaagttatgtaatgaagttagtattctttttaagaatcaacctgattatcttacttttttaagagcaatggatggattcgaagttaatggattacgattatttagcctctcgattccagaaccttcagttaaaaacctttttgccgtaaatgaattttatagaaataatgatgatttcataaaccctgatctacaagaacggttagtgatcggggattatagcatttcaatatttacttatgacattaaaggtgatgctgccaacttactgatttagtgtatgatggtgtttttgaggtgctccagtggcttctgtttctatcagctgtccctcctgttcagctactgacggggtggtgcgtaacggcaaaagcaccgccggacatcagcgctatctctgctctcactgccgtaaaacatggcaactgcagttcacttacaccgcttctcaacccggtacgcaccagaaaatcattgatatggccatgaatggcgttggatgccgggcaacagcccgcattatgggcgttggcctcaacacgattttacgtcacttaaaaaactcaggccgcagtcggtaacctcgcgcatacagccgggcagtgacgtcatcgtctgcgcggaaatggacgaacagtggggctatgtcggggctaaatcgcgccagcgctggctgttttacgcgtatgacagtctccggaagacggttgttgcgcacgtattcggtgaacgcactatggcgacgctggggcgtcttatgagcctgctgtcaccctttgacgtggtgatatggatgacggatggctggccgctgtatgaatcccgcctgaagggaaagctgcacgtaatcagcaagcgatatacgcagcgaattgagcggcataacctgaatctgaggcagcacctggcacggctgggacggaagtcgctgtcgttctcaaaatcggtggagctgcatgacaaagtcatcgggcattatctgaacataaaacactatcaataagttggagtcattaccgacattaaaagtaacttttttgaaattagagataatattggcacagaaaatatattcagttcgtttagtgatttctcttcattcttaaacgaaatcatggacagttgttcataataatcaaaaggaaacaaaaatcattgtaaaccatgccatctttttagagattaccagcagaaaattccttgttcgaaatttagcagtgcaagctatggaaaaacttacaacggaactacactccttaagtgagatggaccgaagacatgtagtctctattttagccgaaatagctaatggctatgatgattttaatgacatgttgatttatttagaattttacccgaatcataagattctgatatcttaaataagaaaatcccgttcgacgttctgaaaaagaaatcataaaatattagcagatacttatttcgtgactatatcttatccgatgaacttttttcaaaaccagcatttaataatatctttgacgaagatgaacgcgtctttgctcaatgtatcacacaggaataataatataacactcaacaataatatttattataattatgattacttatcacgacgcattcgcgaaagcgaaccattaccttgatgatgcagatctcccggtcgtcattactctacatggacgctttagccagggctggtatttctgtttcgaagcacgagaatttctcgaaactggagatgaggccgcgcgcttagctggtaacgcaccttttattattgataaagacagtggtgaaattcattctctgggaacggcaaaaccgctggaagaatatctacaggattacgaaataaaaaaggctaccttcggcttgccctgacaaaatagccctcttcccacgaagagggccgctaaccttagtaccccgccgttaaatcatccaccgagcgcgggtcggatgcgccgtacaactcaccgtccggcccaaccataatgctttgtgtactgcccatcgcctctttcagcgccactttctgaccttttgcttccagcagcttgagcgtatccgggctaaaccctttttcgacacgcagctcgtccggcaaccactgatggtggaaacgcggcgcattggtcgcttcggcgacgttcaagccataatcgatgctattcaccaccatttgcagcactgtagtgatgatccggctaccgcctgggctaccggtaaccagccaggttttaccgtctttcaccacaatggtcggcgacatcgacgacagcgggcgtttgttcggcccgacggcgttggcatcaccgcccaccagcccgtaaacgttcggtacgcccggtttggcggagaaatcatccatctggttattaagcagaataccgctctcgcccgcgacaatgcccgtaccgaaggtggtgttcagcgtataggtcaccgccaccgcgttaccatctttatccaccactgagtaatgggtagtttgattactctcataaggcgcaagcttgccggggcgaatttcgctggatggcttcgctttattgatatcaatttgatcggcaatagatttggcataggctttattggtcagcgcctgccacggtactttgacaaaatccgggtcgccaagatattccgagcggtcggcgtaggcgtatttctccgcttctgccatgatttgcatcgcatcggcgctgccaaagccgtatttcttcatatcgaagttttccagaatattgaggatttgtacgatatggatcccgccggaggatggcggtggcatggagtaaacctgatacccgcgataatcgccgcttatcggagtgcgttcgaccgctttataggctgctaaatcttctttagtgatcaagccaccgtttttctgcatctcctgggcgatctgttccgcaatcgtgcctttatagaattcgtccgggccgttttcagcaatcatctccaggctctttgccaggttcgcctgcaccagcgtgtcgccctttttcagcggctcgccctctttccagaagatagctttactgttttcgtgattcggcaacacttcgctaccgtaggttttgagatcgtcagccagcgcgtcgttaacgataaaaccatcgcgtgccagtttaaacgcgggctgcacgactttgttcagcggcatggtgccgtatttatccagcgccagcgagaaacctgctaccgtacccggtgtgccggaagccagatgcgaagtgagtgattttttgctgtccgggttgccctgatcatcgaggaacatatcgcgggtcgctttggcgggtgccatttcgcggaaatcgatagccgtggtattgccatttttcgagcggattaacataaaaccaccaccgcccagattccctgcctgcggatgcgttaccgccagcgcgtagcccaccgccacggcggcatcaacggcattcccgccctccttgagaatatccacccccacctgagtggcagtggcgtccacagacgctaccattccctgtttcgcgcgtaccgggtggaagacatcttcctccacaccatacgagacgggcggcgcaggaggcgcggcggcggcgctaaaacaacttcctgagagcagagcagcaatggccacccggcgtaaaaacgtcggttttatcatcgttattctccagagattaaggggcaaccccagctaagcctggtatataactctgaattaatcatcgttttgtcgggaagcgagtaaacttaaaggatatcttcagaggaggatacgcgatgaaacgacttctgattcttacggcactcctgccgtttgtcggctttgcacagcccattaatactctgaacaaccctaaccagccggggtatcagatacccagccagcagcggatgcaaacccagatgcagactcagcaaatccagcaaaaagggatgctgaatcagcaactgaaaacgcaaactcagttgcaacagcagcatttagaaaaccagataaacaataattctcagcgggtgttgcagtcacagccgggggagcgaaatcccgcccggcagcaaatgctgcccaacaccaacggcgggatgttaaacagcaaccgtaatccggatagttcgttgaatcagcagcatatgctgccggagaggagaaacggcgacatgctgaatcagcccagcacgccgcagcctgacattccgttgaaaactattgggccgtaaagttcggaccaatcacgtcaatcgcatcggtacagatgcaatccacaccccagcgcagcaactctgctgcgcgctggggtttattgacggtataaaccagaatccgcagtccggcgtctttcaactgcatcactcgcgctttattgagtaacttatgattgagatgaatagagacgcagcccagccgcgcggtcagttcgcgccagtcgtcgcgccactcatccagcaacaaaccgcgcggcagttccggtgccgcctgttgtgcagcttctaaagcatcaatctcaaacgatgacagcagcggcggcgtcataccggcccacagctcgcgtgccgccagcgccaccattttgcccgttaatggcccggtgccggtggtgggtttgatttcgatattcgccatcatcccgtgttcgcggcaacgttccgccacctgcgaaagcaacggtagcggctcacctttaaacattttgctgtaccaactgcccgcatccacgcgcagtaaatcctgccagttcagttcacccgcgacgccccagccgttgctggtacgttcgagattgtcgtcatggagcaggaagatctcgccatctttcgataacttcgcgtcaaattcgatcatcttatgaccgtattttgccccgacgtcgattgacgccagggtgttttccggggccagcttaccgccgccacgatgagcgacgatgcggggataaggccagttactcatactcgttgtcctgtttcaccatcaaaaagatgcagctgattttccgccagatgcagccacagcgtgctgcctgccgtcgggcgctcctgatgcgccagtcgcaccaccagcttctgctcgccccagcgtccgtgcgccaggttatctgcgccgaggatctccagcgtgtccatcaccatcggtacgccgccttctgcctgcgagcttagcgcaatatgttccgggcgaatgccgagagtcattttacgcccggcatactgacggtagccaccgtttagcggcagctcaataccgccgtccagttcgaaatgcgtgccttcgttattcacgcggcctgtcagcaggttcatcgccggactgccgataaaactcgctacaaacaggctggcgggcttttcgtagacttcaactggtgtgccaatctgttcggcaacaccgccgttcatcaccattactcgctgggcgagcgtcatcgcttcaacctgatcgtgagtaacgtagagtgaagtcgttttcaggcgacggtgcaactgttgcagttcaagacgcatctgcacgcgcagcttggcatcgaggttagagagcggctcatcaaacaggaacaccgccggatcgcgcacaatcgcgcggcccatcgccacacgctggcgctgaccgccggaaagctcgcgcgggcgacgtttgagcagaccgtccagctccagaatgcgcgccgcttctttaacgcgctcggcaatttgctgcttgcccatgccgcgaattttcagcccccacgccatgttttcttcgacactcatatgcggataaagcgcgtagttctggaacaccatcgcaatcccgcgatcttttggctccatttcagtcacgcgctggtcgttgatccagatatcgccttctgtcacccgctccagcccggcaaccatgcgcagcagcgtcgatttcccgcagccagacggcccgaccatcacgataaattcgccatccgccacatcaagggtcagcggtttaatgacctgggttttaccatcccagcttttggttactgcctgtaatttcagtcctgccatcttatttctcactatcgaccaggccgcgcacgaaggcacgctgcatcactaaaacaatcaccaccggagggataagcgttaacaacatcgccaccatcactgagttccattccgtggtgccttcgcctgtagcgatcatccctttgatccctgccacggtggtgccgagatccacatcggtaataatcaacaacggccacaaatactgattccagccgtagataaaggtgatcacaaacagcgccgccagattagttttggagagcggaaaaacgatgtcgcaaaagaagcgcattggcgatgcgccgtcgatccgcgcggcttccaccagctcatccggcagcgtcataaagaactggcggaacaggaaagtagcggtcgccgaggccatcagcggcagcgttaaaccggcgtagctgtcgagcatctgcaggttggcgatgacttccaccgtcgggaagatacgtacttcaaccggcagcatcagggtgataaaaatcatccagaagaagaggttacgtagcggaaaacgaaaccagacaatggcaaatgccgagagcatcgagacggtaattttgccgagcgtaatgctgaacgccatcacaaagctgttaagcaacatccgccagaacggcgcgctattcgtgcctaccccgttcacccagatgttgtggatgttttccagcagatgtgtgccggggatgagcgtcatcggcgcggcatagacggcctgtttatccagcgtcgccgcgacaaacgccacgtacagcgggaagaggatcaccgcgatcccgaggatcagcatggtatggctgaatatcgtcagccacggacggttctcaatcattggtaacgcaccttgctttcaacatagcggaactgcaccaccgtcagcacgatgacgaggaacatcaacaccaccgactgtgcggcagacgaagccagatccagtccggtaaaaccttcgcggtagatcttataaatcagcgtcgtggtggcctgaaccggcccgccggacgtggcggcgtcgatcaccgggaaggtgtcgaagaaggcatacaccaggttcactaccagcaggaagaaactcaccggggcgataagcggcagcgcaatcttaaagaagcggcgaatcggccctgcaccgtcgatggctgcggcttcgatcaacgaacggggaatggattgcagcgcggcatagaagaacaggaagttgtagctgatttgcttccatactgaggcaaacaccaccagaaacattgcctgaccgctgttttgcgcgtggttccagtcgtagccgaactccgcgagaaaatgggtgatcagcccgcgaccggggttaaacaggaagatccacaatacggcggcaacggcgggagccacggcgtaaggcagcaacattaaggtttgatagaaacggctgccgcgcacgatgtactccaccagcgccgcaaagaacagcgataccagcaaaccgctgacggtgacaaaggtgctgaattttatcgtcgtccagaaggagtcgagatagtagctgtcatggaacagcgtgacgaagttatccaggccgacaaactggctggagaaaccaaacggatcgacgctttgtagcgagtaccacaacgcttcgcccgcaggccagataaaaaagataacggtgatgatgagctgcggcgcgaccagcagataaggcagccagcgcgagcggaacaccggacgggatgatgacattacggttaattcctgaactgtgccggatgcgcttcgcttatccggcctacacgcgatgccaggtcagataagcgaaacgcatccgacattacactgattaagacttcgtcgatttctcaaagcggcgcagcaactgatttccacgctcaacggcggtatccagtgcctgctgtggtgtcttcttaccggtccacacgctctccagctcttcatccacaatcacgcggatctgcggcatgttgcccagacgcagccctttggtgaacggcaacggcggcttattcagcatctgacgcgtcgcggtatccgcccctgggtttttctcataaaagccctgctcacgggtcaggtcatacgctgctttggtgattggcagataaccggttttctgatgccactcggcagcgttttctggcttcgcgaggaaatcgaggaacttcgccacaccggtatacgtttctttatctttaccctgcatcacccacaggctggctccgccgataatggcgttttgtggcgcatctttcgcatcggcgtcgtaaggcatcatgcctacgccgtagttaaatttggcgtactcgcgaatgttggcaagagaaccggaagaggcggtggtcatcgcgcaatcaccgttatagaacttctcggtggattcatccttacgaccgacgtagctgaagtcgcccttcttgttcatctcctcgagcatggcgatgtgtttcacctgctccggcttattgaactccagcaccgcgtccgtgccgtcaaagccgttgtttttgctggcaaacggcagaccgttccaggcgctaaagttttccagttggatccagccctgccagccgctggcgtagccgcacttcatgccggaggctttcagtttcgcggcatagtccgccagatcctgccaggttttcggcggctgttccgggtctaatcctgctttcttgaaggcgtctttgttgtaatagagaacgggggtcgagctgttgaatggctgggagagtaagtggcccgttttgctgtcggagtagtaacctgaaaccgtcggcacaaactgcgactcatcgaactgaatccctgcctctttaaacacgtcatacaccggtttaatggctttcgacgccatcatggtggcggtgccaacttcataaacctgcaaaatagccggcgcgttgccggtacgaaatgcggcaatccccgcgcttaaattctgttcgtagttgcctttataggtcggtacaattttgtaatccgggttttcggcgttaaaacgttgggccagagaatccacctctttacccagttccccttccatagaatgccagaacggaatggtcgtcactgcctgtgcattccccattaacgccagtccgagcgccagtgctgaagctgtataatgtaacggtttcatcgtttatctctcttgttgtaccgaatgcgcgaattcacgcgttttatgctcgcggggtaacatgacatgctcgaattacagaaaaataacttttttgttacatttgtaagatagtaaggtgtcagaaagatgacaaggcggtgacggcgtgggtgagggaaaatgggagatggggcacggataagcgggaaaatatagaaggtctgaatcaaactctacagattgctcatcgtttcatgccggatgcggcgtaaacgccttatcaggcctacaagatcgtgcaaattcaacatattgccactcacccagtaggcctgataagcgcagcgcatcaggcaattttacatttgtcacctgtctcaaaggagtcttttgactccctatcaatcaacgtgttattacccgcctaaatacgcacttctcaccgcttcattcgccagcagcgcatcaccagtatcggaaagcactacatggccgttttccagcacgtagccgcgatccgccagctttagcgcctggttggcgttctgctcgacgagaaagatagtcatcccctgctcgcgcagctgctcgatggtgtcgaaaatttgctggatgataatcggcgcaagaccgagcgatggctcatcaagcagtagcaaacgcgggttgctcatcagcgcacgaccaatcgccagcatctgctgttcaccgccggacatggtgcccgcccgctgaatacggcgctcatgcagacgtggaaacagctcatacacccactttatgcgctcctggaactggtcgcgttcagcaaaaaaaccgcccatcgccaggttctcttccaccgtcatccgcgagaagacgcgacgcccttccgggacaatcgccaccgcttcgcgcatgattttcgctgtctgccagtcggtaatgtctttatcatcaaacacaattcgcccgctggtggcacgcggatcgccgcataacgtgccgagcaaggtggttttccccgccccgttcgcgccaatcagcgtgacaatctcgccctgattgatatgcaggctcacctcatgcagcgcctggattttgccgtagtgggcgctgactttgtcaaaggacaacatgactttttccatcttatgcctcacctaaataggcacggatcacgtccgggttattacggatctgctccggcgtaccgtttgccagcggcgtcccctgattgaccacgtaaattcggtccgaaattcccatcaccagcttcatatcgtgttcaatcaacaagatagtggtgttgtgatgattgcgcagttcggcaatcagctcatccagctctttcgtctctttcgggttaagacctgccgcaggttcgtcgagcattaaaatctccggctgcgtcaccatgcagcgggcaatctcaagacggcgctggtcaccataggccaggttactcgcctgacggttggcgtgttccagcaaaccaatgcgctcaagccaggtcgcggcgcggtcgagcgcttcgctctgggcgcgacggaaggatggcgttttcaacaggccagagaacagcccggttttcagttgctgatgctgcgccaccagcaggttttcaattaccgtcatttcacggaacagacgcacatgctggaaggtgcgcaccacgcccatgcgggcaatttgctgccccggtaaaccttccaggtgctgatcgcgcagtaaaatggtgccgccggtgggtttgtagaatccggtcagacagttaaaaaccgtggtttttccggcaccgttagggccgattaacgagacgatctcctgcgggtacagttcaagattgacgttgttcaccgccagcaggccgccgaagcgcatcatcaggccgttaacagataataatggctgactcatgcctgctctcctttcgctgcgccgtttttcagcttcagttgcgggcgcgtcatgggcagcaagccctgcggacgccagatcatcatcagcaccatcaaaccaccgagcattaacatgctgtattcgttgaaatcacgcatcaactcgcgcgacaccaccagcaaaattgccgccagaatcaccgcaaattgcgagcccataccgccgagcaccactatcgccagcacaaacgccgattcggcaaaggtgaaggattccgggctgacaaagccctgacgcgccgcaaacagcgttccggcaaaaccggcaaacgcggcacttatggtaaaggcagtcagcttgatacgacgcgggcttaagcccagcgaacggcaggcgatttcatcttcacgcaacgcttcccacgcacgccccagcggcatccgcagcaggcggttaatgacaaacaggcttagcaccaccagcagcaacgccaccaggtagaggaagatgacacgatcggagggatcgtatttcaggccaaagaaattactgaacgtgtcccagccgccttcacgagcggtacggctgaactcgagtccgaagagtgtcggtttcgggatctgactgattccgttcgggccgccggtaatttcggtgttattgagcagcaatatgcgcacaatttcgccgaaaccgagggtaacgatcgccagatagtcaccgcgcaaacgcagcaccggaaaaccgagcaggaagcccgccgccgctgccattaatccagcaatcggcaggcaggtccagaagcccaagccgtaatagtgattgagcagcgcaaaagtgtaagcgccgatggcgtaaaaaccgccgtaccccagcaccagcagaccagaaagaccaacaaccacgttcagcccgagaccgaggataatgtagatcatggtcagggtggcaatatccaccgtcccgcgtgaaaccataaacggccacgccaccgcaagcaccaacagcgccacgaggaacagtttctgcttcaccgtggagccatcaatggcgggcagaataaacttcggtccggaaacgcttttcaaccctttctggaaagccggtcgcaaaagctggaagaaaaagaccaccgccgtgccgataaacacccactgccaacggacatccgaagccgtgtcgaccaccagtttggtgccatccagctccagttgcacgcccataaagacgcccgccagcacaaagaacatcgcggcagagagcagcgccattgcaatatgcatcggtttcatactttctctacctccgggcgacccagaataccggtcggcatcaccagcagcaccagaatcagcagggcgaatgagaccacatctttatattccgtactcagataggcagaagagagcgcctccgcaatccccagaatcaggccgccaatcatcgctcccggaatgctgccaatcccaccgagcaccgccgcggtaaaggctttcatcccggccataaagccgatgtaggggttaatgacgccgtagaactgaccgagcagcacacccgccaccgccgccatcgccgcgccaatcacaaaggtcagcgcaatcacccggtcggtgttaatgccaagcagactcgccattttcagatcttccgcgcaggcacgacacgcgcgacccatgcgggaatagcgaatgaaaatcgtcagcgccagcatggcgaggaaggtaacaatccagatcaccgcctgcatggtggtaatagaggcagagaagttttcgctatgccccaccacccactgaccgttaaacaggctcggcagcgccacgtcgcgcgaaccttcggtcaggctgacgtagttttgcaggaagatggacataccgattgcagagatgagtgcaatcaggcgcttagagttacgcaccgggcggtaagccacccgttcgatactccagccgtaggcgctggcaatgacgattgcgccgacgaatcccgcagctaccagcagccagccggtatcaatgcccatcatcatcagcgcggcgatgatcataaatgagacgtagctgccaatcatataaacctcgccgtgggcgaagttgatcatgccgataatgccgtaaaccatggtgtagccgatggctatcagcgcgtaggtactgcccagcgtgacgccgttaaacatctgctgcaagaaatacaaaaactgctcagacataaggtaacctttctaaacccgcccgcattttacgggcggtgggatgatcacttggctgccgtggatgaaccgtcggcgtgccactggaagacaccaaaatcaaatcccttaagatcgcctttttcatcccagttcagcggcccaatcacggtgtttgcaccgttagcttttaaatctttcaccagcgccagcggctcatcgctgccggtacgctcaagggcagtcgccagagattgcaccgccgcgtaggtgatccagacataaggcccggacggatctttcttgtctgctttcagcgcatcaacgatgccctggtttgccggatcctggtcatagcgttttggcatagtgaccaacatgccttcggcggcatcaccggcaatgttcgacaacgacgcattacccacaccttccggccccataaactgggttttcaggccaacggaacgggcctggcgcagcatctgccccatttccgggtagtaaccgccgtagtaaacgaagtcgatgttttcttttttcaggcgggcgatcagcgcggagaaatctttctccccggcggtaataccgtcgaagaagacgacgttggcgttagccgctttcagcccgtcctgcaccgaacgcgccagcccttcgccatactgttgtttgtcgtgaatgatggcgatgcgctggggcttcaccgtctcaagaatgtattttgccgccgttggcccctgggaagagtccagcccggcagtacgcataatgtgttgataaccgcgttgggtcagctccgggttggtcgctcccggcgagatcatcagaataccttcgtcttcatagatatctgacgcaggctgggtagaagaagaacacagatgaccaataacgtatttaatgccgtcattaacgattttgttggcgaccgcaacggcttgtttcgggtcgcatgcgtcgtcatattccacgccaaccagtttatcgcccttaattccccctttggcattaatgtctttaattgcctgacgcgcgccgttaaattccatatcgccccactgggcaatcgggccggacatcgcgccgacaacggcgactttaatatcgtcagccatagcggtgtgtgaaattgccagtgcaatcatccctgcgatgatagttttcgcattccgtttcatagtcaaaaatccccattcgtgatgttgtgttgctttgtttttatgtgttaacaaatcagactgttctttttttatactgcactgtttttgcctgtctgattaaggggttagcgcagtattttgtgataatagcgattaaaatccctatttttcagtcgattaagaacagataatattctgaatttattgatagataaacagaaaaaagtgcctttgtcagcataaaataacggcacaaagggcggaataattcactatcattcaggggattatgctggacatttttcattctctaatgttttaattttgtaattattgctgttaaaaaattaatcacctgccaaaagaaataaaaaagagaaagcctccgattaaattatttcgctacactggttccacttttgtgatttacacgggttacccatgaagctgaccatcattcgattagaaaaatttagcgaccaagaccggattgacctgcaaaagatctggccggagtattccccttcctcgttacaggttgacgataaccaccgtatctacgccgcgcgttttaacgagcgcctgctcgctgccgtgcgggtaaccttaagcggcaccgagggagcactggattccctgcgcgtgcgggaagtcacccgccgtcgcggtgtggggcaatatctgctggaagaggttttgcgtaacaatcctggcgtttcatgctggtggatggcggatgcaggcgtggaagatcgcggtgtgatgacggcgtttatgcaggcgctggggtttacggcacaacagggcggctgggagaagtgttaatcgtcaagtttgatttcaaaagtgatattgcctgatgcgctacgcttatcaggcctacaatgtgtgttgcaatttactgatttctttggatcttgtaggccggataaggcgtttacgccgcatccggcatgaagcaacgtactcgatattagcaatttggcggcaacccaaagttgccgattaatgattacttcgcatcggtcgccgtgccgttggcgtgccagtcaaatacgccgaactcaaagcctttcagatcgcctttctcatcccaggtcagcggtcccattacggtatccacggagttcgctttcaggtatttggcgatttcagccggatcgtcagactgattcaggcccgcctgcaaagattgcagcgcggcgtaggtggtccaaacgaatgcgccacttgggtcctgttttttcgctttgatcgcgtcaacaatgggtttgttcgccggaacctgatcgtagttcttcggcttggtcaccagcagcccttccgctgattcgcccgcaatgttagacagcgaaacgttagccacaccttccggccccataaactgagttttcagccctgccgcgcgtgcctgacgcaggatttgccccatttccgggtgataaccgccgtagtaaacgaagtcgatattctcttttttcagacgcgccaccagcgttgagaaatctttttccccggcggtgatgccatcaaagaacaccacgtttgcattgcctttcttcaggccgtcctgcaccgctcgcgccagaccttcgccgtattgctgtttgtcgtgaacgatagcaatacgctgcggtttcactttctcaagaatatatttcgccgccgtcggcccctggtcggagtccaggccggtggtgcgcaggatcagctgatagccacgggcggtcagctccggcgcggttgccgctggggtgatcattaaaatgccttcgtcttcgtagatgtcagacgcaggctgcgttgatgaagaacagaggtgaccaatcacatatttaatgccgtcgttaacgactttgttcgccaccgcaaccgcctgtttcgggtcacaggcatcgtcatattttacgatttgcagtttgttgcctttaatgccgcctttagcgttgatatccgcaaccgcctgctctgcgccggtaaactcctggtcaccgtactgcgcaaccggaccggacattgcgcccacgaccgcgactttaatatcttctgccagagccatattgctgaatgccagcgcgatacatcctgccagtaacgctttaccctttatgttcatcctgagaatccccattcttctggttattacgtgtgttgtgatgttgtttttcagcactttatttcgttttatgcatgactacccgtgctttagcagcatactctgctaaaacatacccgatttttatgatattggaatagctattttgacagtttattaacaatctgcgtggggattggcgttttgccggaggggaaattgattattacagaggcccaaaaaacaaaaaccccggactctcatccagggttctctgcttaatagcggaaattacgcttcaatggcagcacgcaattttttcatcgcgttcttttccagctggcgtacacgctcagcggaaacgccgtaacggtcagccagttcctgcaacgtggacttgttgtcttcgtccagccagcgcgcacggatgatgtcctggctgcgttcgtccagaccctgcatcgcgtcggtcagacggtttgccgcctgctcttcccagttatcatcttcaatgccgtcggcaaagttagatgatttatcctgcagatagagcaccggagccatcggctggctgtcggaatcgtcgtcggaagacaggtcaaaggtcatgtcctgtgccgccatacgtgattccatctcacgtacgtctttgctggttacgcccagttcacgggccaccatttcgacttcatcctggttaaaccagcccagacgctgcttggttttacgcaggttgaagaacagtttgcgctgcgctttggtggtcgcaactttgacgatacgccagttacgcagaacgtattcgtggatctctgctttgatccagtgaacggcgaaggagaccaggcgcacacccacttccgggttgaaacggcgcactgctttcatcaggccgatgttaccttcctgaatcaaatccgcctgtggcaggccatagcccgcataattacgagcaatatgaacaacaaaccgcaggtgagacaggatcagcgttttagctgcttccagatcgccatggtaatgcagcttttcagccagcgcccgctcctcgtcagccgacaacatcggccacgcgttagctgcccggatgtaggaatccaggttgccaactggggctaaagctaaactttgcattttgtcagtcattcaaatcctctcaatcgatatcttctggcgcttcagtggtagcaacaactgtgccagagcttaagagcaacgaggttatcattcactgttttatcagaccgtgattttatccacaagttcaatgcaagcttgtgaataaattacgcacaaaatgtgacatagagatgaaataccgggaagagacaacggggtctctttccctgctacggaacccattgcagggaaagagtataacacgcttttattattcaggcgtaaagtggcgtaaatgttgtaccgtggcaagccacgctgccacccagccaatcatcgagcataccagcagcaatagcaggcattcatcgaatgataagccattgatatcaaacttcgttccgaaaacctgtgccacttccgcaaccgccgatgacaatcgcagcaccagaatttctgacaaaattaatgacaacaatgcgccagaaaatcccagcagtgcgccaccatacaggaacgggcgcaggatgaatccatctgtcgcaccaatcagtttctgtacgttaatggagtcacggcgagcaaagatactcagacgcacactgttaccgatgacgaggaacacggccgccaccatcaacacgccgatcatcgccgaaacgcgcccgaccagcccggtcaacgccgccagacgggcaaaccagctgtcatccatccgcacttcgtcaatgccgttaatctgcgtgatacgatcacgcagcgtattcagtgattccgtcccctggaaatcgagtttcgggatcaccaccgccactgccggaagcgggttttcttccagcatatccagcgcaccaccaaaaccagaccagttacggaactcacccagtgcgtcttcacgagaaagatagttcactttctccacgccttgctcggcctgcaactgtgccaccacgcccgcagcagcgtcatcgtccagcgttttttgcagataaacagtgatttgcggtgacggataatactgcgtcgccgcctggttaacgtttttgtacaccatataacagacgctgggcagcgtcagagaaatggcgataaccatcaccgttaaaaacgtggcgaacggtttgcttttcagatcctgcaatgcgccgtggaaggcatagcgcacctgttcgttgaaaacgttggttttgcgatttaccggttttggcgaggatttcgcgcgttttggtgcgttacgaccgccgtcgcctgagccgccgaccgatttacggaagcgatcaagacgcccgccaaactgccgaatatgattgattgcatcgcgcttattcatggcccacgcctccatgcaagtgaccatcgctcagggtgagcatgcgataggaacgccgcgagatcaggttgatgtcgtgcgttgccatcaatacggttaccccaacgcggttaaactcttcaaacagacgtaaaatgccttccgacagcgcgtcgtccaggttaccagtcggttcgtccgccagcagtaccgcgggcttgttcaccaccgcgcgggcaatgccaacacgctgttgttcaccgcccgaaagctgaatagggaagttcttcgctttgtccagtagcccgactttatccagcgccgccgacacccggcgacgaatatcgtcaccgctggcaccggcgataatcagcgggatcgccacgttatcgtagacagtacggtccatcagtagatggtgatcctggaaaatcatgccaatctggcggcgcagaaacggaacttcacggtttttcagacgcgtgatgtcatggccgctaaaccagattttcccggcgctgggccgctcaatcccacagatcagcttcaggagggtacttttccctgcgccggaatgaccggtcagaaacgccatctcacccggctgcatatggaacgtaacgccctgcagcgcctgtctcccaccgagataagccttgctgacatgttcaaagcgaatcattgttaatcctctcgggcaaaaagtgcctctataaagtcgtccgccttaaacggacgcaaatcctcaatacgttcgccgacaccaatgtagcggatagggataccaaactggtcagccaccgagaaaattaccccgcctttcgccgtgccgtccagtttcgttagcgtgatgccggttaagccaacggcttcatggaacagtttggcctggcttaccgcgttctgcccggtgctggcatcaatagtcagcataacttcatgcggcgcttcaacgtcgagtttcttcatcacgcggacgattttcttcaactcttccatcaggtgcgatttgttctgcaggcgtccggctgtatcggcaatcaggacgtcgatattacgcgctttagctgcctgaatggcgtcgaagataacagaggcggaatccgccccggtatgctgggcaatcaccggaatattgttgcgctgaccccagacctgaagctgttcaaccgcagctgcacggaaagtatcacccgccgccagcatcaccgatttaccctgctgctcaaactgacgcgccagcttaccaatcgtcgtggttttacccacaccgttgacgcccaccatcaggatcacaaacggcgctttgccttcaacattcagcggctcatcgactttcgccagaatctcgcccatctcttctttcagcaggccatagagcgcctcggcgtcacgaagctgcttgcgggatgcgccttccgtcagattggtgataattttacgtgtggtttccacacccacatcggcgatcaaaagctgctcttccagctcctcaaacagatcatcgtcgatttttttaccgcggaacaggctgataaatccggaaccgagattttctttggtttttaacaggctgcgtttcaggcgcgcgaaaaaaccttctttggtcggtttttcctgctcctgagcgatttcttccaccggctgctcttcttctgccggaggaaccaccatcaccgcctcttctgccgcttcggcagccagcgccgtttccagctcttcgtcggtaatttcttctttagccgcttcttcttccgccgcttcgacaatctctacggtttccgcttcagcctgccactcttctggcgaaaccgcttcggcgttgacgtcttccggcaacggcagctcttcacgttcgatagccactggctccggcgtttcttctacgaccggttccggctgtgcaacgacttccgcttcaggctgcgctttttcactttcagcaacctgttcagtgacttccacaacgtcggcagcaaaagtttccgcctcggcttcagtatgcgcttgcggctgctcttcaacggcttgttcagaggccttcacaggctcttgcgcctgaacgatttcttctacaaccggttgttcattctgaacttctgtctctttttccggggtctgctctttttgaccaaagcccagccaggaaaaaaagccacgttttttttctttcgccatttgcgactacactcctcgctgttgcttcatggcacagcgttaacgctatgtacatagcagctaaaaaaatgatgaaatagtctatcacttaacttaattcacatcaccgcctgcaagtatgtgttatctggcggattgagcaatttatcatgaaaaaaccgaatcattccggcagcggccaaatccgcattattggcgggcagtggcgaggccgtaaactcccggttcctgatagcccaggtctgcgccccaccaccgaccgcgtacgcgaaacgttgtttaactggctggctccggtcattgttgacgcccaatgtctggattgcttcgccgggagcggcgcgctggggctggaagcgttatcgcgctacgctgcgggggcaacgttgattgagatggatcgcgcggtttctcagcagttaattaagaatctggcgacactaaaagcaggcaatgcacgcgtggtgaacagcaacgcgatgtcattcctggcgcaaaaaggtacaccgcataatatcgtgtttgtcgatccaccgttccgccgtggcttgttagaagagacgataaatttactggaagataacggctggctggctgacgaagccctgatttatgtcgaaagcgaagtcgaaaacggtctgcccactgttccagcaaactggtcattacatcgggaaaaagtggcgggtcaggtggcttatcggctgtatcaacgcgaagcacaaggagaaagtgatgctgattaatattggtcgtttgttaatgctctgcgtttggggatttttaatcctcaacctggtgcatcccttcccacgcccgctgaatatcttcgttaacgtggcgctgatttttaccgtgctgatgcatggtatgcagctggcgctattgaaatccactttaccgaaagatggcccgcagatgaccaccgccgaaaaggtacggattttccttttcggcgtgtttgaactgctggcctggcagaagaaatttaaagttaaaaaataaccttattgttcgcctacaaagctgacaaagcgcgttcctttatagctcagcgtacctttatcgcccactgtcagggcgtggtactgctgggcgtcgaggcgaaacgtctgctccattcctccgctttgcggtttgaagcttgcctcatagcgtatactggtgcctgccggagtcacttcctgctggcgcgaacggcgatcgttaatcggtttttcccgcttgttgctcaccaccaccagcttttgctggagcggagccatatcattatcagctttttcccgtcgctgttgcataaaacgaaacgatgcggcgacgacaattaagccaatgataacaataaagaaaagaggtggtttgctcatctttatccctcatcggaaaatgcggaaataagcataccctgccagttatggtgttgtcatccgtccaccctcgccactaaactggaagcaagaccgtaggcattccgcttacgaaaaaataacgaattcaaggaactaagatgctttggtcgtttatcgctgtctgtctttccgcatggctatctgtggatgcatcgtatcgtgggccaacctggcaacgctgggtgtttaaaccgttaacccttcttctcctgctgttactggcctggcaagcgccgatgttcgacgccattagctatctggtgctggcagggctgtgcgcctcactgctgggcgatgcgctaaccctgttgccacgtcaacgtctgatgtacgccatcggcgcgtttttcctctcgcacctgctgtacaccatctatttcgccagtcagatgacgctctctttcttctggcctctaccactggtgctgctggttctgggtgcgctgttactggcgattatctggacgcgcctggaagagtaccgttggcctatctgcacgtttatcggcatgacgctggtgatggtgtggctggcaggtgaactgtggttcttccgtccgaccgctccggcgctctctgcgtttgttggcgcttcgttgctgtttatcagtaactttgtctggctggggagccactatcgccgacgcttccgtgcggataacgcgattgctgcggcctgctactttgccggtcacttcctgatcgtccgctcgctgtatctctgataaaacttgactctggagtcgactccagagtgtatccttcggttaatgagaaaaaacttaaccggaggatgccatgtcgactcctgacaatcacggcaagaaagcccctcaatttgctgcgttcaaaccgctaaccacggtacagaacgccaacgactgttgctgcgacggcgcatgttccagcacgccaactctctctgaaaacgtctccggcacccgctatagctggaaagtcagcggcatggactgcgccgcctgtgcgcgcaaggtagaaaatgccgtgcgccagcttgcaggcgtgaatcaggtgcaggtgttgttcgccaccgaaaaactggtggtcgatgccgacaatgacattcgtgcacaagttgaatctgcgctgcaaaaagcaggctattccctgcgcgatgaacaggccgccgaagaaccgcaagcatcacgcctgaaagagaatctgccgctgattacgctaatcgtgatgatggcaatcagctggggtctggagcagttcaatcatccgttcgggcaactggcgtttatcgcgaccacgctggttgggctgtacccgattgctcgtcaggcattacggttgatcaaatccggcagctacttcgccattgaaaccttaatgagcgtagccgctattggtgcactgtttattggcgcaacggctgaagctgcgatggtgttgctgctgtttttgattggtgaacgactggaaggctgggccgccagccgcgcgcgtcagggcgttagcgcgttaatggcgctgaaaccagaaaccgccacgcgcctgcgtaagggtgagcgggaagaggtggcgattaacagcctgcgccctggcgatgtgattgaagtcgccgcaggtgggcgtttgcctgccgacggtaaactgctctcaccgtttgccagttttgatgaaagcgccctgaccggcgaatccattccggtggagcgcgcaacgggcgataaagtccctgctggtgccaccagcgtagaccgtctggtgacgttggaagtgctgtcagaaccgggagccagcgccattgaccggattctgaaactgatcgaagaagccgaagagcgtcgcgctcccattgagcggtttatcgaccgtttcagccgtatctatacgcccgcgattatggccgtcgctctgctggtgacgctggtgccaccgctgctgtttgccgccagctggcaggagtggatttataaagggctgacgctgctgctgattggctgcccgtgtgcgttagttatctcaacgcctgcggcgattacctccgggctggcggcggcagcgcgtcgtggggcgttgattaaaggcggagcggcgctggaacagctgggtcgtgttactcaggtggcgtttgataaaaccggtacgctgaccgtcggtaaaccgcgcgttaccgcgattcatccggcaacgggtattagtgaatctgaactgctgacactggcggcggcggtcgagcaaggcgcgacgcatccactggcgcaagccatcgtacgcgaagcacaggttgctgaactcgccattcccaccgccgaatcacagcgggcgctggtcgggtctggcattgaagcgcaggttaacggtgagcgcgtattgatttgcgctgccgggaaacatcccgctgatgcatttactggtttaattaacgaactggaaagcgccgggcaaacggtagtgctggtagtacgtaacgatgacgtgcttggtgtcattgcgttacaggataccctgcgcgccgatgctgcaactgccatcagtgaactgaacgcgctgggcgtcaaaggggtgatcctcaccggcgataatccacgcgcagcggcggcaattgccggggagctggggctggagtttaaagcgggcctgttgccggaagataaagtcaaagcggtgaccgagctgaatcaacatgcgccgctggcgatggtcggtgacggtattaacgacgcgccagcgatgaaagctgccgccatcgggattgcaatgggtagcggcacagacgtggcgctggaaaccgccgacgcagcattaacccataaccacctgcgcggcctggtgcaaatgattgaactggcacgcgccactcacgccaatatccgccagaacatcactattgcgctggggctgaaagggatcttcctcgtcaccacgctgttagggatgaccgggttgtggctggcagtgctggcagatacgggggcgacggtgctggtgacagcgaatgcgttaagattgttgcgcaggagataaggcaaaccgatcgcaacattgagcgcgatcggtcccctcgcccctctggggagagggttagggtgaggggaaaaggcggcatcgaagccaatcagcccctatcaaccgcctttacgaatcaaataacgataaggcagtccatccgtctctttagcaaccagttcgtgttccataaaggtacaaaacccaggaatatcgcgggtagtggccggatcgtcggcgataatcagcaacgtttcgccaggctgcatattgcgcacggttttgcgcaccatcatcaccggttccgggcagcgcaggccaagcgcgtcgagtgtgtggtcagggctggaaaagagatcggtcattttcttctcatcacttaaaaaaacggcgctagtttacgccctgtgagtccgtaagcaaactaggttaacgattgcgtgaaaattaaccattgcattgtcaacgtaaagcagtatcatgcggcggctcgaaaaaagggtaagcacgttattatgttaaggtaacagacgtgtcgtacgtattgggttccctcaccccaatggttaatcaaaaaggtacaatatgaacgttttctcgcaaactcaacgctataaggcgttgttctggttatcgttatttcatctgctggtgatcacctccagtaactatctggttcagcttcccgtctccattttgggtttccataccacctggggcgcgtttagctttccgtttatttttcttgctaccgacctgaccgtgcgtatttttggcgcaccgctggcccgacgcattatcttcgcggtaatgatccctgcgttattaatctcctacgtcatctcgtcgctattctatatgggttcctggcagggattcggcgcactcgcccacttcaacctgtttgtcgcccgtatcgccaccgccagtttcatggcctacgcgctggggcaaatcctcgacgtgcacgtttttaaccgcctgcgtcagagtcgccgctggtggctggcaccgacagcgtccacactgttcggtaacgtcagcgacacgctggcctttttcttcattgccttctggcgtagcccggatgcctttatggctgaacactggatggaaatcgcgctggtcgattactgtttcaaagtgttaatcagtatcgttttcttcctgccaatgtatggcgtattactcaatatgctgttgaaaagactggcagataaatccgaaatcaacgctttgcaggcgagttaaaggttcgttatcagagttgtgataagatggatgaatgagccgttatggccgtttatcgaaaggaagaagtcaatgcgcaatctggttaaatatgtcggaattggcctgctggttatggggcttgcggcctgtgatgataaagacactaacgctacggcgcagggttcggtcgcggaaagtaacgctaccgggaatcccgtcaacctgcttgatggcaagttaagtttctcgctgccagcggatatgaccgaccagagcggtaagctgggaacgcaggccaataacatgcatgtctggtccgacgccaccgggcagaaagcagtcatcgtcatcatgggcgatgatccgaaagaagatctggcggtgctggcgaagcgtctggaagatcagcaacgtagccgcgatccgcagctgcaagtggtaaccaataaagccattgagctgaaaggtcacaaaatgcagcagttagacagtattatctccgcgaaaggccagacggcgtactcttccgttattctgggtaacgtgggtaatcaactgctgaccatgcaaattacgctgcccgctgacgatcagcaaaaagcgcagaccaccgcagaaaacatcattaatacgctggttattcagtaagttttaagatgatgaggcggcctcagggacgtgttccggaggccgtttttttaatcgccacgtcagtaataacgcgattgcgaccagtcccgccgccgccagataaatcaccggtacgcccgcccagctcatcaccagcccagccagtggtccagtcacgccaagcgataaatccataaatacggtgtaagttgccagcgccgccccctgattttgctgcggaaccgcttttaccgccactacacccaatgccgggaacaccagcgaaaacccggcccccgccagtaagacgccgattttcgccatccacggcatagtcgccacgccaaccagtagcaggccgattatctcaacgctaaagcaaatcatcgctacgtttaagccaccgatacggttaatgccgttagggaataacaaacgcgtaccgacaaacgcacagctaaacagcgtcagcgcgaaagccgcaccgtcccaacctttagcgtcataaaacagcgtgataaaggtggcgatgacgccaaatccggcggaagccagtgccagcgccataccgtacagccagacgcgcccaagcaccgcgcgaaacggcagcggtttgcctttactggcttttaccgtcggacgcgggatcgccaacaaaatggccaccagcgccacgcccataatgattaacgctaacgcctgcaagccgccccagtgataaaacacgacgcctaacggcgcacccatcgccatcgccccgtaagtgacaatgccgttccacgaaatcacccgcccgatatgcagcgagccaaccacgccaacgccccatagggtcgatcccgttccggcaaaactttgcccaatcccaaggatgacgcgccccaggcaaagtaataacaggctgatgacaggcagactggcggttaatcctgccgtcagataccccagaccgctcaaaaagcagccgcataaaccgaagacgacaatctttttgggtcccagcgaatcggcgtaacgtccggcatgagggcggctcagcaaggtggcgaaatattgcaggctgataaccaatcctgcccagaaggcgctaaagcccatcacatcatggacatagcccggtaatacagcgagcggcaacccgatggtgaggtagctggcgaagttaaacatgactatagagacaatgcgcaaattcaggcgcaatccgtttagcgcgggttcggctacgggttcgggcatgaggatcaccacatttttacaacagtgtttcatttttaccacgtgctgacgtgaaaatcagcagtaagaatcagaatattgctggcgtgactcccgctacacttaatacaaaaagtcacaaggaagccccaatggaaacccctcaacccgataaaacgggcatgcacattctgctcaagctggcctcgctggtagtgatcctcgcgggcattcacgcagcggcagatatcattgtgcagctgttactggcgctgttttttgccatcgtcctcaacccgctcgtcacctggtttattcgtcggggagtacaacgccccgttgccattacgattgtagtggtggtgatgctgatcgcactaaccgcgctggtcggcgtactggcggcatcgtttaacgaatttatctctatgctgccgaagtttaataaggagctgacgcgcaaactttttaaattgcaggagatgttgccttttcttaatttgcatatgtcgccggagcgaatgctgcagcggatggactcggaaaaagtggttaccttcaccacagcgctaatgaccgggctttccggggcaatggcgagcgtgcttttgctggtgatgaccgtagtttttatgctgtttgaagtgcgccacgtcccttacaaaatgcgttttgcgctgaataatccacagattcacatcgcgggattacaccgcgcacttaaaggcgtttcgcactatcttgcattgaagacgctactcagtttatggacaggtgtcatcgtctggctggggctggagctgatgggggtgcagtttgcgctgatgtgggcagtactggcgtttttgctcaactacgtgcccaatatcggcgcggtaatttccgccgtaccgccaatgattcaggtgctgctgtttaatggtgtttacgaatgtattctggtcggcgcattgtttttagtggtccatatggtcatcggcaatattttagaaccacggatgatgggccatcgcctggggatgtccaccatggtggtatttctttcattgttaatttggggatggctgctcggcccggtagggatgctactttcggtgccattaaccagcgtgtgtaaaatctggatggaaaccaccaaaggcggtagcaaactggcgattttactggggccgggcagaccgaaaagtcggttaccgggatgaggcgacaagtgatacgatacgcactttcattttccattaaacgttggccctgatatgtatcggatagttctggggaaagtttcgaccttaagcgcagctccactgccaccgggtttacgcgagcaagcaccgcaaggtccacgacgcgaacgctggctggcggggcgtgcattgctttcgcacacgctttccccgctaccggagatcatctatggcgaacaaggcaaacctgcatttgcgccggaaatgccgctatggttcaacttaagccatagcggtgacgatatcgccctgctgttgagtgatgaaggcgaagtcggctgcgatatcgaagtgattcgcccgcgcgccaactggcgctggctggcgaacgccgtattcagcctcggggaacacgctgagatggacgccgtgcatcctgatcagcaactggaaatgttctggcgcatctggacgcgcaaagaagccatcgttaaacagcgtggcggcagcgcctggcaaatcgtcagcgtagacagcacctatcactcctcgctgtcagtcagccattgtcagcttgaaaatttaagccttgcgatctgcacccctactccctttacgctcaccgccgacagtgtgcaatggatcgattcagttaactgatccgcccacccgactgcccatctattgatccagaacaggtaatcagtatgacgaatacttaaaatcgtcatacttatttccgccatctattttaatccattggggttaccatgctctccacactccgccgcactctatttgcgctgctggcttgtgcgtcttttatcgtccatgccgctgcaccagatgaaatcaccaccgcctggccggtgaatgtcgggccactaaacccgcacctttacacgcctaaccagatgttcgcccagagcatggtttatgaaccattggtgaaatatcaggcagacggttcggtgatcccgtggctggcaaaaagctggactcattcagaagatggtaaaacctggaccttcaccctgcgtgatgacgtgaaattctccaacggtgaaccgttcgatgccgaggcggcggcagaaaacttccgcgcagtgctcgataaccgtcaacgtcacgcctggctggagctggcaaaccagattgttgatgttaaagcactcagtaaaacagagctgcaaattaccctgaaaagcgcctactatcctttcctgcaagaactggccctgccccgtcctttccgttttatcgctccctcgcagtttaaaaaccatgaaaccatgaacggaattaaagcgccgattggcaccggaccgtggattttgcaggaatcgaaactgaatcagtacgatgtcttcgtccgtaacgaaaactactggggcgaaaagccagcgattaaaaagatcacctttaacgtcatcccggacccgactacccgcgcggtggcgtttgaaactggcgatatcgacctgctgtacggaaacgaagggttattaccgctcgataccttcgcccgctttagccagaatccggcttaccacacccaactgtcacagccgatcgaaaccgtgatgctggcgctcaataccgccaaagcccccaccaacgagctggcagtacgtgaagctcttaattacgcggtaaacaaaaaatcgctgattgataacgcgttgtatggcacccagcaggtcgccgacaccctgtttgccccttctgtgccctacgccaacctcggcctgaaaccgagccagtacgatccgcaaaaagcgaaagcgttgctggaaaaagccggttggacgctgcctgcgggcaaagacatccgcgagaaaaatggtcagccgctgcgcattgaactttcgttcatcggcaccgatgcgttaagcaaatcgatggcggaaatcattcaggctgatatgcgccagattggcgcagatgtctcgctgattggcgaagaagagagcagtatctatgctcgtcagcgcgacggtcgttttggcatgattttccaccgcacctggggcgcgccatatgatccacacgccttcctcagttcaatgcgcgtaccgtcacacgctgacttccaggcacagcaaggattagccgacaaaccgctgattgataaagagatcggcgaagtgctggcgacccatgacgaaacgcaacgtcaggcgctgtatcgcgacattctgacccgtctgcatgacgaggcggtttatctgcctatcagttacatctcaatgatggtggtatcaaaaccggagctgggtaacatcccctacgcgccgatcgccaccgaaattccgttcgaacagattaaaccggtgaaaccttaatgttgcgttacgtattacgccgctttctgctgctgatcccgatggtgctcgccgcctcggtgatcatttttctgatgctgcgcctcggtaccggcgacccggcgctcgattatttgcgtctgtctaacctgccgccgacgccggagatgctggcctctacccgcaccatgctgggactggatcagccgctgtacgtccagtacggcacctggttgtggaaggcgctgcatcttgactttggtatctcattcgccagccaacgcccggtactggacgatatgctgaacttcctgcccgccacgctggaacttgcaggtgcggcgctggtattaattctgctcacttccgtaccgctcggtatctgggcggcgcgccatcgcgaccgtctgccggatttcgccgtacgtttcatcgcgtttcttggcgtgtcgatgcctaacttctggctggcgtttttactggtgatggcgttttcggtgtatctgcaatggctacccgcgatgggttacggcggctggcagcacatcattttgcctgcggtttccattgcctttatgtcgctggcgattaacgcgcgtttactgcgcgccagtatgctggacgtcgccggtcagcgtcacgtcacctgggcgcgtctgcgcggcctgaacgacaaacagaccgaacgtcgccacatcctgcgcaatgcctcgctgccgatgatcaccgccgtggggatgcatatcggcgaactgattggcgggacgatgattatcgaaaacatctttgcctggccgggcgtcgggcgctatgcggtgtcggcgatttttaaccgtgactatccggtgatccagtgctttacgctgatgatggtggtggtttttgtggtctgtaatttgattgtcgatttgctcaacgccgcgctggacccgcgcattcgtcgtcatgaaggagcgcacgcgtgaactttttcctctcttcccgctggtcggtacgcctggcgctgatcattatcgccctgctggcgctgattgcgctcaccagccagtggtggctgccgtatgacccacaggcgattgatttgccgtcgcgcctgctttcgccggatgcgcagcactggctgggcaccgatcacttaggtcgcgatattttctcgcggctgatggcagcgacccgcgtgtcgctcggttcggtaatggcctgcctgctgctggtgctgacattagggctggttattggcggcagcgccgggttgattggcgggcgcgttgatcaggccaccatgcgcgtcgccgatatgtttatgaccttcccgacctcgattctgtcgttctttatggttggcgtgctcggcaccgggctgaccaacgtaattatcgccatcgccctgtcgcactgggcgtggtatgcacgcatggtgcgcagcctggtgatttcactacgccaacgcgagtttgtgctggcgtcacggctttccggtgcgggccatgtgcgggtgtttgtcgatcatctggcaggcgcggtgatcccttcgctgctggtgctggcaacgctggatatcggccatatgatgctgcacgtcgcggggatgtctttccttggcctcggtgtgaccgcgccgaccgccgaatggggcgtgatgattaacgacgcgcgccagtatatctggacccagccgctgcaaatgttctggccggggctggcgctgtttatcagcgtgatggcctttaacctggtgggtgacgcactgcgcgatcatctggaccctcatctggtgacggagcacgcacactaatgccgcaacagattgaactacgtaatatcgcgctacaggccgcgcagccgctggtacacggtgtatcgttaaccctgcaacgcgggcgcgtgctggcgttagtcggcggtagcggcagcgggaaatcattaacctgcgccgcaacgctgggcattttgcccgctggcgttcgccagacggcgggggaaattttagccgatggcaaaccggtttcgccttgcgccctgcgcggcatcaaaattgccaccatcatgcagaacccgcgcagcgcctttaatccactgcacaccatgcacacccacgcgcgggaaacctgcctggcgttagggaaacccgccgatgacgctacgcttaccgctgccatagaagcggtggggctggaaaacgccgcgcgcgtgctgaagctgtacccgttcgagatgagcggcggcatgttgcagcgcatgatgattgcgatggcggtgctgtgtgaatcaccgtttatcatcgccgatgaaccgaccaccgaccttgacgtggtagcacaggcgcgcatcctcgatctgctggaaagcattatgcaaaaacaagcgccgggaatgctgctggtgacccatgatatgggcgttgtggcgcgtctggcggatgacgtggcggtgatgtctgacggtaagattgtcgaacagggcgatgtagaaacgctgtttaacgcccccaaacatacagtgacgcgcagcctggtttccgctcatctcgccctctacggtatggagctggcatcatgactttacttaacatctccggcctttcccatcactatgcgcacggtggatttaacggaaaacatcaacatcaggcggtgctgaataacgtttccctgaccctgaaaagcggcgaaaccgtcgccctgctggggcgcagcggctgcgggaaaagtaccctcgcgcggttgctggtgggtttagaatcgcccgcgcaggggaatattagctggcgtggcgaaccgctggcgaaactcaatcgcgcccagcgtaaagcgttccgccgcgatattcagatggtatttcaggactccatcagcgccgtgaatccgcgcaaaaccgtgcgcgagatcctgcgtgaaccgatgcgccacctgctatcactgaaaaaatccgaacaactggcgcgcgccagcgaaatgctgaaggcggtcgatctcgatgacagcgttctcgacaaacgcccaccgcagttaagcggcggccagctccagcgcgtctgcctggctcgcgcgctggcggtcgaaccgaaactactgattctggatgaagccgtttctaaccttgatctcgtgttacaggcgggtgtcattcgcctgctgaaaaagctacaacaacagtttggcaccgcctgcctgttcatcacccacgacttacgcctggtagaacgcttttgccagcgggtaatggttatggacaacggacaaatcgtcgaaacccaggtggtgggagagaaattaaccttttcctctgacgccggacgtgtgctacaaaacgcggtattacccgcattccccgtgcgccgtcgcaccacagaaaaggtttaacgcaaatgcaacgagtcaccatcacgcttgatgacgatttactggagacgctggacagcctgagccagcgtcgtggttataacaaccgttccgaagctatccgcgacattctgcgtagcgccctggcgcaagaggccacccagcagcacggcacgcaaggtttcgcggtgctgtcgtatgtgtatgaacacgaaaaacgcgacttagccagccgcattgtctccacccagcatcatcaccacgacctctccgtcgccacgctgcatgtgcacatcaaccacgacgactgtctggaaatcgccgtgttgaaaggtgacatgggtgacgtgcagcattttgccgatgacgttatcgcccagcgcggcgtgcggcacgggcatttgcagtgcttgccgaaggaagattgagtctattattgggtcctttggtgaacgatcaacaaagggccactagcacacctgattcctctctaaataccctatccgaaccttctcttttgtaacgttctaaatatattcctaaaaatcttcaattcattgtgaccacaagtttttcttcgctttttcgtatgaagatactgtcattaaaataatagaaaaggattttacgatgagcggaaaaccggcggcgcgtcagggtgacatgacgcagtatggcggtagcattgttcagggttcagccggggtacgtattggtgcccccaccggcgtggcctgttcggtgtgccccggcggagtgacgtccggccatccggtcaatcccctgctcggtgcaaaggtccttcccggtgaaaccgacatcgccctgcccggcccgctgccgttcatcctctcccgcacctacagcagttaccggacaaaaacgcccgcgccggtggggagcctcggccccggctggaaaatgcctgcggatatccgcttacagctgcgcgataacacactgatactcagtgataacggcggcagaagcctgtattttgagcacctgtttcccggtgaggacggttacagccgcagcgagtcactgtggctggtgcgcggcggcgtggcgaaactggatgaaggtcaccggctggccgcactctggcaggcgctgccggaagaactccgcttaagtccgcatcgttatctggcgacaaacagtccgcaggggccgtggtggctgctcggttggtgtgagcgggtgccggaagcggatgaggtgctgcctgcgccgctgccgccgtaccgggtactgaccgggctggtggaccgcttcgggcgcacacagacgttccaccgcgaagccgccggtgaattcagcggcgaaatcaccggcgtgacggatggtgcctggcgtcacttccggctggtactgaccacgcaggcgcagcgggcagaagaagcccggcagcaggccatttccggcgggacggaaccgtccgcttttcctgataccctgccgggttacaccgaatatggccgggacaacggcatccgtctgtctgccgtgtggctgacgcacgacccggaatacccggagaatttacctgccgcgccgctggtgcgctatggctggacgccacgcggcgaactggcggtggtgtatgaccgtagtggcaaacaggtgcgcagctttacttacgatgataaataccggggccggatggtggcgcaccgtcacacgggccggccggaaatccgttaccgttacgacagcgacgggcgggtgacagaacagctaaacccggcaggcttaagctacacgtatcagtatgagaaagaccgcatcaccatcaccgacagcctggaccgccgtgaagtgctgcacacgcagggcgaagccgggctgaagcgggtggtgaaaaaggaacacgcggacggcagcgtcacgcagagtcagtttgacgccgtgggcaggctcagggcacagacggatgccgcaggcaggacaacagagtacagcccggatgtggtgacgggcctcatcacgcgcataaccacgccggatggcagggcatcggcgttttactataaccaccacaaccagttaacgtcagccaccgggcctgacgggctggaattgcgccgggaatatgatgaattgggccgtctgattcaggaaactgcccctgacggcgatatcacccgctaccgttatgataatccacacagtgacttaccctgcgcaacggaagatgccaccggcagccggaaaaccatgacgtggagccgttacggtcagttgctgagcttcaccgactgttccggttatgtaacccgttatgaccatgaccgcttcgggcagatgacggcggtgcaccgcgaggaagggctgagtcagtaccgcgcatacgacagccgtggacagttaattgccgtgaaagacacgcagggccatgaaacgcggtatgaatacaacatcgccggtgacctgaccgccgtcattgccccggacggcagcagaaacgggacacagtacgatgcgtggggaaaggccgtccgtaccacgcagggcgggctgacgcgcagtatggaatacgatgctgccggacgggtcatccgcctgaccagtgaaaacggcagccacaccaccttccgttacgatgtacttgaccggctgatacaggaaaccggctttgacggccgcacacagcgttatcaccacgacctgaccggcaaacttatccgcagcgaggatgagggtctggtcacccactggcactatgacgaagcagaccgcctcacgcaccgcaccgtgaagggtgaaaccgcagagcggtggcagtatgacgaacgtggctggctgacagacatcagccatatcagcgaagggcaccgggtggcggtgcattacaggtatgatgagaaaggccggctgaccggtgagcgtcagacggtgcatcacccgcagacggaagcactgctctggcagcatgagaccagacatgcgtacaacgcgcaggggctggcgaaccgctgtataccggacagcctgcccgccgtggaatggctgacctacggcagcggttacctggcaggcatgaaactcggcgacacaccgctggtggagtacacccgcgaccgcctgcaccgggaaacgctgcgcagcttcggccgttatgaactcaccaccgcttatacccctgccgggcagttacagagccagcacctgaacagcctgctgtctgaccgcgattacacctggaacgacaacggcgaactcatccgcatcagcagcccgcgccagacccggagttacagctacagcaccaccggcaggctgaccggcgttcacaccaccgcagcgaatctggatatccgcatcccgtatgccacagacccggcaggtaaccgcctgcccgacccggagctgcacccggacagcaccctcagcatgtggccggataaccgtatcgcccgtgacgcgcactatctttaccggtatgaccgtcacggcaggctgacagagaaaaccgacctcatcccggaaggggttatccgcacggatgatgagcggactcaccggtaccattacgacagtcagcaccggctggtgcactacacgcggacacaatatgaagagccgctggtcgaaagtcgctatctttacgacccgctgggccgcagggtggcaaaacgggtgtggcggcgtgaacgggacctgacgggctggatgtcgctgtcacggaaaccgcaagtgacctggtacggctgggacggcgaccggctgaccacgatacagaacgacaggagccgcatccagacgatttatcagccggggagcttcacgccactcatcagggtcgaaactgccaccggtgagctggcgaaaacgcagcgccgcagcctggcggatgcccttcagcagtccggcggcgaagacggtggcagtgtggtgttcccgccggtgctggtgcagatgctcgaccggctggaaagtgaaatcctggctgaccgggtgagtgaggaaagccgccgctggctggcatcgtgcggcctgaccgtggagcagatgcaaaaccagatggacccggtgtacacgccggcgcgaaaaatccacctgtaccactgcgaccatcgcggcctgccgctggcgctcatcagcacggaaggggcaacagcgtggtgcgcagaatatgatgaatggggcaacctgctgaatgaagagaacccgcatcagctgcagcagcttatccggctgccggggcagcagtatgatgaggagtccggcctgtattacaaccgccaccgctattatgacccgctgcaggggcgatatatcactcaggatccgattggactgaaggggggatggaacctgtatggatatcaattgaatccgatatcagacatcgaccccctgggtttatctatgtgggaggatgcaaaatcgggggcatgtactaatggtctttgcggcacactatccgctatgataggtccagataaatttgattctatagatagcaccgcatatgacgccttaaataaaataaatagccaatctatttgcgaagataaagagttcgctggtttaatatgtaaggataatagtggcagatatttctcaacagcacctaaccgaggagaaagaaaaggatcatatccattcaatagcccttgccctaatggtactgagaaagtatcagcttatcatactcatggtgcagatagtcatggagaatattgggacgaaatattttcaggtaaagatgagaaaatagttaaaagtaaagataacaatatcaagtcattttatttaggtacgcccagtggtaattttaaagcaatagataaccacgggaaggaaataacaaacagaaaaggattacctaatgtctgcagagttcatggtaatatgtaaaaaaatattgtttaggaactgtgtcattgtatctttgtttgtttttacatacaacacatgggcgcagtgtaataataatattaaaataatgcgcaagtatgaaagtgaaggtaaatataccgttagaaatttggttaaaaataaagctatagcattggaattagctgagatatatgttaagaatcgttatggacaggatgccgcagaagaagaaaaaccatacgaaatcactgagttaacaacaagttgggttgttgaaggtaccattcactcagaccaaattgctggtggggtttttattatagaaataggcaaaaatgatgggagaattctgaattttggccacggaaaataagtatgtaaggataatcaaacatcgtgtgcgctgatggcagagtaggtggaggactccagacagtcaaacgatagaaaaagatagcctttatggaggttcctgcaatgtcaaatacataccagaaaagaaaggcaagtaaagagtatggtttatataataaatgtaagaaactaaatgatgatgaattatttcgcttacttgatgatcgcaattccttgaaaaggatttcatctgccagagtattacagttaagaggggggcaagacgctgttagattggcaattgaattctgcactgacaaaaattatatccgtagagatatcggagcatttatactcgggcaaatataaatttgcaaaaaatgcgaagataatgtttttaatattttgaacaatatggcattgaatgataagagtgcttgcgttcgagctacggcaatcgagtcaacggccagggaaagatcatcaaaagttcactttttgcactaaataattcgcattttatgtttaaaaattgagatattccttattacctgaagctgttttttattgcttatacatgatcaaatactccttacctaattaaggagaacaaaatggaacttaaaaaattgatggaacatatttctattatccccgattacagacaaacctggaaagtggaacataaattatcggatattctactgttgactatttgtgccgttatttctggtgcagaaggttgggaagatatagaggattttggggaaacacatctcgattttttgaagcaatatggtgattttgaaaatggtattcctgttcacgataccattgccagagttgtatcctgtatcagtcctgcaaaatttcacgagtgctttattaactggatgcgtgactgccattcttcagatgataaagacgtcattgcaattgatggaaaaacgctccggcactcttatgacaagagtcgccgcaggggagcgattcatgtcattagtgcgttctcaacaatgcacagtctggtcatcggacagatcaagacggatgagaaatctaatgagattacagctatcccagaacttcttaacatgctggatattaaaggaaaaatcatcacaactgatgcgatgggttgccagaaagatattgcagagaagatacaaaaacagggaggtgattatttattcgcggtaaaaggaacccaggggcggctaaataaagcctttgaggaaaaatttccgctgaaagaattaaataatccagagcatgacagttacgcaatcagtgaaaagagtcacggcagagaagaaatccgtcttcatattgtttgcgatgtccctgatgaacttattgatttcacgtttgaatggaaagggctgaagaaattatgcgtggcagtctcctttcggtccataatagcagaacaaaagaaagagccagaaatgacggtcagatattatatcagttctgctgatttaaccgctgagaaattcgccacagcgatccgaaatcactggcacgtggagaataagctgcactggcgtctggacgtggtaatgaatgaagacgactgcaaaataagaagaggaaatgcagcagaattattttcagggatacggcacattgctattaatattttgacgaatgataaggtattcaaggcagggttaagacgtaagatgcgaaaagcagccatggacagaaactatctggcgtcagtccttgcggggagcgggctttcgtaatcttgccctgaatacaggactgagtatcaaaaagccggttaactgaaactgtccaggttttgggggtcagttcataaacgccttatccggcctaaaaacaactaaaattcaataaattgcaccgatgcgtagtccctataagcttacgcatcgggcaattgtatttacgccattgtcccaatcgtcttcctgaatcgcagcagcgcaatggtgaaaaatgcgccgccaattgccatcagcgtcagaaactgcggccagacgatttcgaatccggcaccccggtagaggatggcctgcgcgaggctaacaaagtgtgtcgtcggcatggtcagcataatgtcctgcaccatctgcggcatactttcgcgcggcgtggaaccaccggaaagcatttgcagcggcagcagcaccagaatcaccagcagccccagttgcggcattgaacgcgctatcgtccccataaaaatgccgattgacgtggtggcaaacagactgagcgccacgcccagcataaacagcgggatcgagccttcaatcggtacgcccagtacacctttcaccatcagcaccagcgataatcccgataccaccagcaccaccagccccatcgaccagatcttcgccatcatgatctcaaacggcgttatcggcatcaccagtaagtgttccaccgtgccgtgttcacgctcgcggatcagcgccgatccggtcaatacaatcgccagcatggtaatgttgttgatgatcgccatcaccccgccaaaccacgcgggatcgaggttcgggttaaagcgcatccgggtttccagcgataccaacggttcgctgttatcacggtagcgcgcgacaaagctgttcacttcaccgttgataatattctggatatacccattgccggtaaatgcctggctcatgcgcgtggcatcgacgttcacctgaatatccggctggcgtccggcgaggacatcacgctgaaaattaggcggaatatttatcgcgaaggtatagcgtccggcgtccagtccggcatccatctcatcggcggtgatcatctccggtggcaaaaaccacggacgatagaagctgttaacgatccggttcgataactgcgattgatccatatcggcaatggcgatcggcgcgaggttcaacgatcctggcgtaacggtcgctgacgaatacaccgacaccgtaaacgagaagacaatcagcgtcagcatcgctttatcaccgagcagactgcgcaactctttgatacccagattaaaaatattgcgtaaatggcgcatcatccctcctgttttttcagcagcaggatacttaagcccatcaccagcgggatggctatcagtaacgggataaaaagttgccacaaatcagtcagatccagcgctttcgagaacgtcccgcgggcgatagtcagaaaatgactggtcgggtaaacctcgccgatccaacgtccaggcccttccagcgaagctaccggatcgatcatcccggaaaactgtgtcgccgggatcaacgtgataatcgccgttccgaaaatggcggcaatctggcttttcataaaggtggagatcagcagccccattccggtggcaatgatgatatacagcagcgccgccagggtgagcgtcaggaaactgcctttatgcggtacgccaaacacaaacaccgacaggccgcagagcaggaaaaagttcagcatccccagcgcgatgtatggcaactgtttaccaagcaaaaattcactacgcgtggtgggggtcacgtaaaggttgataatcgacccaagctctttttcccgcaccacgctaagggcgcttagcattgacgggatcatcatcagcagaagcgggatcaccgccggaacaatcgctggcaggctttttacgtccgggttatagcgatagcgcgtctcaatattcatcagcccgctttggctggcgggtgtcgattgtcggctcgccacatcctgtaaccagctctggtgcatggcctgcacgtaaccttttaccgtttcagcacggctcggcatcgctccgtcgatccagacgccgagttccacaggcgtaccacgcgcgatatcgcgcccgaaattgggcgggatctcaatcgccaccgtgatatcgcccgcacgcatccgacgatcaagctcgtcataactggtgagcggcggctgttcgataaagtaacgggaaccggagaggttgagtgtccacgcctggctactgacggtctggtcgcggtcgagcaccgcaaagcgcaggttttccacatccatactgatgccgtaacccattatcagcatcaggatcaccgttcccatcagcgccagcgtcgaacgtactggatcgcgtcgcagttccagcgcttcgcggcggctgtagctaaacagacggcgcaggctaaatccctgacgcggcgcgtgggtggtgtcgtgtaccacgggcggcgcttcggcttcgttgctctgccctgccgcttcctgcaaataggcgataaatgcctcttccagactggcggctccgcgtttctcaaccagttcctgcggtgtaccgctggcaagcacttttccggcgtgcatcagtgagatgcggtcgcaacgttccgcttcgttcataaagtgggtggagatgaagatagtcactttgtcctggcgcgagagatcgaccatcaactgccagaacatatccctcgccaccggatcgacaccagaagtaggctcatcgaggattaacatctccgggcgatgaatcaccgccaccgccagcgaaagccgctggcgaatgccgagcggcaatgactccggcagaatatcttcaacgtcgttgagcttaaaacgctcgctcatttcagccactcttgcgggaatttccgcttccgggatgtgaaacaaacgggcatgtaactcaaggttttgccgcacggtgagttcgttatagagcgaaaacgcctgcgacatatagcccacccgacggcgggtatcgatatcttttggatcaaccggttgcccgaacagccacgcctcaccttcgctggcgggcagcagtccggtgagcattttcatggtggtggatttaccgcagccgttcgaaccaagaaaaccaaaaatctccccgcgtggaatgcggaaattaacgtgatcaacggcaacgaaggaaccaaaacgcatggtcagatcgcgcgcttcgatggcaatctctgcgttttcaggttgatacggtgggatcactaccgcctgatgcgcctggcgttgcgcttgcggtaacagatttataaatgcttcttccagcgtagcgctttgcgtttgctgccgtagctcttcggcgctgccagttgccagcacttctccggcattcatcgctaccagccagtcgaagcgttcggcctcttccatataggcggtggcgaccagcacgctcatattgctctgccgctggcgaatactgtcgatcagatcccagaactgggagcgggagagcgggtcaacccccgttgttggctcatcaaggatcaacagttccgggtcgtggattaacgcgcagcacagcccaagtttttgcttcatcccgccggagagtttccctgccggacgatcgcgaaacggtgctaacccggtgctggtcagcagctcattgattcgcacttcccgctccgctttgtcgtgaccgaacaggcgagcgaaaaaatcgacgttttcatacaccgacaaggtgtggtagaggtttttgcccagcccctgcggcatccaggcgatgcgcgggcagacgtcgcggcgatgcttcgggtcgcgcatatcgccgcccagcaccatcacattgccctgttcaatgacgcgggcaccggaaatcaacgacaacaagctcgacttcccgacgccgtccgggccaatcagcccgaccatacagcgggccggaatatcgagagtgatattgttcagcgcaacggtttttccataatgctggctcacgcccgccagttgcgcgacaggcgggacgggaaccagttccagatgcgtcattgcggcaacctcaccacgaggtcgtcaggccacggaagttcttcattcacccgcacccacgctacgcccggcaaaccggttttgacatattccagatgctgctggagtaattccggtgggatacgcgctttgacgcggaacatcagtttcagccgttcatcgctggtttcgacggtttttggcgtgaactgggcgacactggcgacaaaactgatggttgcaggaatacgcagatctggcgcggcatcgaggatcagccgggcttcaccgcccagtttcagcgtgcccgcctgttcggttggcaggaagaaagtcatatagacgtcgctgagatcgaccatattcagcacccgaccgcctgccgccagcacttcgcctggctcggcaacccgatactgcacgcgtccgtcacgcggggctttcagttcgctgtcatcgatatctgcggcaatgcgccgttcagtggcttgtgccgcttcgacgcgggtttgcgcctgaatgatattggtgcgtgccgcttctatagccgctttagaagccgatacctgagctttcgccgattccagcgcagctcgggcgctctcagcggcggcgcgatcgtcatccagctgttgcgcagaaatagcccctcgttgggccagtgaacgggaacgcgtatgacgttttgctacggagtccagttctgcctggcgttgattaaccagcgactgtgcggcacgagtttcgctttgtcgttgctccagcaaagcctgcgcggcagcaacggcgctttgtgcctctttgatttgcgcgatggcttccagtcgctgttcctgcaacacgcgagtatccatcttcgccagcacttcaccttcgcgaacaaacttgccttctttcaccagaatggtgtcgatacgcccggcaattttgctggcaatatccacttccgtcgcttcaatgcgcccattactgacagcaaagccttccggcacacctgccgggcgcaacagccaccacgccacgatagccgccaccgccagtaacccgacaacccaccacgccagatggcgcttactcttatccataatcgacccgccataatccctgtaagcaaacgacgcgtgttacaactgccgccgaacgacgttcagcggattcttccatccgggataagaaggaaacggcaaatacgaccagcgcgcagagcattgagcgccaacggggaaggcttagtgaaaacgggtagtaatgttgtcatcatcagcattcctggccgtaaatgaaacacgcatactcataagtgtgatctataaaactggctgacaaaacggtatccatcctgttggatagcgtttcacgcctgttcagttgcaggaacagagcattcctttttacgttttatcaacagtctcaaccagatagtaacattaatattcatgttgtctatggttcagagctgtaacattgtgcgccttctaatcaaaggcataagtccatttctgtttttttcatgctggtaagacttccagggagtggttatctcaggccctgcaccagggttaatttggcaattatgcatgctgaacattcttccagcatgtttactgtcacgggcgttaagacctaaaactgtccccgtttcgcctatgcgttctcttccaccatttccgttatgtgcaacaacttgatttatacctaacatttgtgaacatgctaatagtgcttcaagtttaggtctgtaatctgtcgaaacagaaaaataacgattaaaggatcgacaagagatagcccggctagttttaaactttttgccattaattatagcatgatgctttttattgataattgccgctaattcgaccggatcgagagcattggtcatttcatcaatagagactgttatcggtcctataatgtaacgttttcgctgatcatcaaaagttatcccatgatgatttgccattattttgtatttggggtcatagaaacatacaggataatcttttatcccagagtaggtatcctcatcgagtggtttcatacgcgtgaagttctgcatatagttaccattgcaattcgtttcatgatttccagctaatacatgaacattttcattgatactcattatgcgttttaacaaatcgatgataaattgatcaccacagatattgctaaatcgatcgccggtttggtcgcccagaaacgtacatggcgtcacagcgtctttattaataactaaataaggctgaagactttctaaaataatgtctcttctgttcaggatactgattattgtattaacattagtgttaagttgctcattaaagttctcccttagcaatacgttgagaacttcatcttctatattaagcaactggctaaggaaattttctccttcagccatgattcccaaatgtcccgttgcgaaaagcgcgaacaaaactgcaccgactgagccatcggtatcaccaaaataggttggtctggtacttgtgggatcaacgggtaaacaattggagaaatagattctgtcagcgaactggggttttatcattgtttcgaatttaatatcagatacattatattgcgatattttccagttccagatgggtttgtacgactcagtaactgcaacatcattagcattatcatttactgtcatattattaagtaaataaacaatactgcaccaattaatatcggtattatcaagagagcaaccgtaatttttgctattaattgtcacaataaactgataattattattcctacgtagaatatgagcacgcatgcccgatagcatactatatttttctgaatgatccgtttgtatggtaaatgaaattttgtcatcttgaatagattgttggaaccgttctatttgccaatcatctattttttccacaacctcaccgagcattgtcctggcaatacttgatatatcatcacctataccatttgcaatatacccaaacagttctttagtgaagttggtaacatgctcttgcaccatatcatttgttgcgattgtcgttgtactgtcgttagtgcctgccacagttccaattttcatattttacctcatattatttaccgcgaggaatacatagttaacattttatcttatgacatacacctcatgttcgatgggaaaataattatattttgcacaaatcattcagcctcaaagcataatatgaaatttcttatctcatagcagagaaagtccctaaagattgtagaggcgtcatcagaacatgcctctacaatcgattaagaaaacctatgaaatactggcaggattaaaaagacataccaccgtattcatggagttttaatgtagttgaaaacaactaagccctgaggaataaattattttattatttttatcacgtgcttccttcagggaatttagccccataataccattatcaaattgttgattatgatctaccccgggcccatgatgcccatatttttgtctaatgtatttgctggggtcttcacctttgagtgtctccccacatatgaagatacgttcacgtgctggtctgaaatcagtagtgttatcaaaataattagcatatacaggtgtgggtttcaaagtattgcttcggattagatggaatagaggatcatccatgtgttctttatgttttttattaaaaatattggctaattcctcaggatcagtaggatttttcatctgattaaatggaacctgcaaagcaccgagacaataacatttttttcttcatctcttattattccgtgatgactggttaaaacttgcctttctgagtcataattacaaacatcgagcgttttaattaagttatacgtatcaccggcagagagtttatgatttgctagtcgtgcagtatagttaccattaaaattgatttcatgatttccagccagaacgacgacatttttattaatacggctatctttattaccctccatatttcgcatagaatttagcaaagtaaggatatatttatcaccaaaaatagtactaaatctatcgcctgtatgatccccaaggaagatacaaggggttatcgcatcgtcctttaaaaaaacatgttgatgcaactcattcaagatcatgtctctcgtatttaataaatcgtagagcactttattatttttatgtttgtatgcagatgaagccatctcttcgtgttttaataattcacataataaactccaacccttttccctgatgcctatatgccctgaaacgagcaatgcataaagtacagcgcctactcttccatctgtatcgccaaaataagccgtgttggcattttgtgggttaatcacaccacactgtttatagaagtctatttttgaaaacacagatttaacatagctatcaaacttttccttagtaaacgtctctttagagacatcccaacgccagtcaggtttgaaattaccactaagaagagtaaagaaatttctcgctatgatagaaagcccatcaactttataaattatatctgatttatctccagaggaattaataaaataataaccgcccttacactcaacagtaacggtaatgggagacgataattttaacacatggttattgtctggtataattgtaaagataaacgtatcagtagtattgtcggcgaatctattatattcttgaatatctatagaaggttcactattataaaaccatactttctccatctggtgactacgatcatttaccttccagtgaccatgttgcaggaaatagatgatatgcaggccaaaatcgttatctatttgcgaatcattatccagtttatcaaattcaactatctttgcacgatgtgttttatcaaccttgccatggtgttgatgactgttaactttatctgaatgcttatcttgatggcttgaagagatgtttctaatctgattgtcaattgctttcataaataacctgtgatatttttgaattgtttgtaacaaaataaatgatacttgtctgaaaaacagatttacgacgatataaaataataatacttatatgttcgctgattttaagcaccgagactatccggtcttttaccaaataatgaagaataatccctccctggaagataattgtaaaaaacaacagcataagaattaatcttaggataaatttttatttatcatggccttttgaacgctgaaaagtagcgctctgcaaagtaaaccccgctatagttatgctatgcatttgtctttaatgatatctcgtcattatattaacaggatgaaattatcattaatgcatatttcaatattagcagggatacctgaggagtttaaagtgaacatatatatcgggtggcttttcaaattaatccctttgattatgggcttaatttgtatcgcgttaggtggctttgtgctggaaagttcagggcaaagcgagtatttcgtcgcgggtcatgtgctgatttctctggcggccatatgcctggcattattcactaccgcatttattatcatttcgcagctcacgcgcggcgttaatacgttttacaatacattgttccccattattggctatgcggggtcaattatcaccatgatatggggttgggcactgttagcaggcaatgatgtgatggcagacgagtttgtcgccggccatgttattttcggcgttggtatgattgccgcctgtgtatcgacggtggcagcgtcatccggtcactttctgctcattcccaaaaatgcagcggggagcaagagcgacggaacaccggtacaggcttattcttcattaatcggtaactgcctcattgccgttcccgttttactcaccctgctcggtttcatttggtctattacgctgttacgtagtgctgacataactccgcattatgtcgcgggtcacgtattgcttgggttaaccgcaatctgtgcctgtctaattggccttgttgccacaattgtccatcaaacacgtaatacgttttcaactaaagaacactggctgtggtgttattgggttatttttctcggctcaatcacggtactgcaggggatatacgtcttagtcagttccgatgcaagcgcccgactggctcccggcattattcttatttgcctcggaatgatctgttacagcatattctcaaaagtctggctactggcactggtatggagacgtacctgttcgttagccaacagaataccgatgattcccgtcttcacctgcctgttttgccttttcctggcatcgtttcttgcggaaatggcgcagaccgacatgggatattttattccttcgcgagttctggtcggtttgggagcggtatgctttacgttgttctcaatcgtttcaatattagaagcgggttctgctaaaaaataattgcaacgtaccggataaaaccagcgttgaccatttgcgtaacgctggtttttcttaggcatcatgaaataacgcagcattaatgcatagtggttaagtataaaaaacagcaaagttactgtttttttcaacctgttcatatttcataaagatctggccactgagtgagttttcaatcacctttccatccaccttatattaagcatggagggtttcagttcacgggctcattagaaaataatcacaagataaccactatcaaaattagctcatttttaatgcgactctaataattttcatctttaggaaataggtcaggacgactttgctgcaatcaaatcctgcgcacaagcccacgcactcgaccacgcccactggaagttatagccccccagccagccggtgacgtccatcacttcgccgatgaagtacagcccaggcactttgcgcgcttccatcgtccgtgaagagagttcgttggtgtccacgccgccgagcgtcacttcggcagtgcgatagccttcagtgccgttgggttgtacgcgccagtcggtcaatgtgctaatcagtgcctgttggtcacgcacgttgagctgttttagcgaaacatccgggatttgcccgagttgctgtaagcgttcaaccaaccgcttcggtagatgaaccgccagtgtgtttttcaggctttgattcggatgtgcgttacgctgctcattcaggaaggtttcgaggtccacatccggtagcagattgatgctgacaaattcccccggttgccagtagcttgaaatctgcaacaccgccggtccagacaagccgcggtgggtgaagagtaagttctcacggaaaacggtgccgttttcagcggtaatcacggaaggcaccgccacgcccgccagcacctgtaactcttcgagcaacggtttatgcagagtgaatggcaccagacccgcgcgggtcggcagcacgttgaggccaaattgttcggcaatcttataaccaaacggcgacgcgcccagccccggcattgacagcccaccagtcgcgatgaccagcttttcgcaaccgacagtcatgccgttcagatcaagcgtgaagcctgtttcatccttcgccacactcagcacttcgctacgcaatctgaaggtcacattgcccttctcgcactcatccaccagcatgtcgacaatctgctgcgcggagtcatcgcagaagagttgccctaacgttttctcgtgccaggcgatgccgtgtttattgaccagatcaatgaaatcccactgggtaaaacgtgcgagtgcagacttacaaaaatgcggattctggctcagataagcgcctggttcgacataaaggttggtaaagttgcagcgcccaccgccagacataaggattttgcgccctggttttttaccattatcgatcagcagaacccggcgtcctgcctgacctgccagcgcagaacagaacatacccgccgcaccagcgcctataataatggcatcaaacctttccacgttgcgctcctcttagaaaaaacgggcgtgaattgtaaagattcctcagtggtcgcaccagcatcaatattactaaaaggaagtatttgcctgaattatataagataattattttttgagtgaaatccatacagggggcaaatcaaaaaaagtctatatttcactttgcccgcgccgcgaaagtcactgataatgcgccgcgttcatgtcctcaaaatggcgtaacgtcctatgctacatttgtttgctggcctggatttgcataccgggctgttattattgcttgcactggcttttgtgctgttctacgaagccatcaatggtttccatgacacagccaacgccgtggcaaccgttatctatacccgcgcgatgcgttctcagctcgccgtggttatggcggcggtattcaactttttgggtgttttgctgggtggtctgagtgttgcctatgccattgtgcatatgctgccgacggatctgctgcttaatatgggatcgtctcatggccttgccatggtgttctctatgttgctggcggcgattatctggaacctgggtacctggtactttggtttacctgcatccagctctcatacgctgattggcgcgatcatcgggattggtttaaccaatgcgttgatgaccgggacgtcagtggtggatgcactcaatatcccgaaagtattaagtattttcggttctctgatcgtttcccctattgtcggcctggtgtttgctggcggtctgattttcttgctgcgtcgctactggagcggcaccaagaaacgcgcccgtatccacctgaccccagcggagcgtgaaaagaaagacggcaagaaaaagccgccgttctggacgcgtattgcgctgatcctttccgctatcggcgtggcgttttcgcacggcgcgaacgatggtcagaaaggcattggtctggttatgttggtattgattggcgtcgcgccagcaggcttcgtggtgaacatgaatgccactggctacgaaatcacccgtacccgtgatgccatcaacaacgtcgaagcttactttgagcagcatcctgcgctgctcaaacaggctaccggtgctgatcagttagtaccggctccggaagctggcgcaacgcaacctgcggagttccactgccatccgtcgaataccattaacgcgctcaaccgcctgaaaggtatgttgaccaccgatgtggaaagctacgacaagctgtcgcttgatcaacgtagccagatgcgccgcattatgctgtgcgtttctgacactatcgacaaagtggtgaagatgcctggcgtgagtgctgacgatcagcgcctgttgaagaaactgaagtccgacatgcttagcaccatcgagtatgcaccggtgtggatcatcatggcggtcgcgctggcgttaggtatcggtacgatgattggctggcgccgtgtggcaacgactatcggtgagaaaatcggtaagaaaggcatgacctacgctcaggggatgtctgcccagatgacggcggcagtgtctatcggcctggcgagttataccgggatgccggtttccactactcacgtactctcctcttctgtcgcggggacgatggtggtagatggtggcggcttacagcgtaaaaccgtgaccagcattctgatggcctgggtgtttacccttccggctgcggtactgctttccggcgggctgtactggctctccttgcagttcctgtaatcgtacgcaccaaaacgagcgggtcagctggcccgcttcagattgtgacatagtgcgctttgttcatgccggatgcggcgtgaacgccttatccggcctacaaaaacatgcaaattcaatagattgcagagattatgtaggcctgataagcgtagcgcatcaggcaattttgcgtttgtaatcagtctcgagcgggtcagtttactggcccgctttttttatgcgttattattgctgaagtgcttaatgccaaatcatcaatgcaatcaggctgaccaccaccagaccacacaatgcgctggtcagaataaactgccgacgcacccgctcacagcggcgaataaattcatcatcgtgatgatcgcgataacgttgggcatagatataccaaacgagacgcacctgtttgttgggttggccatgtgaggtaaaaaagccccctccatcaacatattgatagagcaatggatcgcagttacgcagtaccactaacaacgcgcgtagtgatgagaaatagcgcgccatgttaacaatgcaaacgacacataaagcccaaaataatgcgacggtgcttatcatacctcctccccggcgacctgcccgcggagttccaccccggggctaccgctcccgatacgctgccaatcagttaacaccaggtcctggagaaaccgcttttgtggtgaccaacatacgagcggctctatagatagtgtaggagatcaggttgttttttttccagaaggttaaccactatcaatatattcatgtcgaaaatttgtttatctaacgagtaagcaaggcggattgacggatcatccgggtcgctataaggtaaggatggtcttaacactgaatctttacggctgggttagccccgcgcacgtagttcgcaggacgcgggtgacgtaacggcacaagaaacgctagctggccagtcatcgacaactttatggaaggagtaacactatggcttataaacacattctcatcgcggtcgacctctccccggaaagcaaagttctggtagagaaagcagtctctatggctcgcccctacaatgcgaaagtttctctgatccacgtagatgtaaactactctgacctatacaccgggcttattgatgtgaatctgggtgatatgcagaaacgcatctctgaagagacacatcatgcactgaccgagctttccactaatgcaggctacccaatcactgaaaccctgagcggcagcggcgacctgggccaggttctggtcgatgcaatcaagaaatacgatatggatttggtggtttgtggtcaccaccaggacttctggagcaaactgatgtcttccgcacgtcagctgatcaacaccgttcacgttgatatgctgattgttccgctgcgcgacgaagaagaataatcttccctctacgacgtgttcctgaacgcccgcatatgcgggcgttttgctttttggcgcgccttgttacctgatcagcgtaaacaccttatctggcctacggtctgcgtacgcaatcaaaatccccagccaatacaacatttaacaccatcatattttccatcattagtgtgatcatctggttattttctgttgtaatagtgtattaatctattcaccgcatcaatattaagaatctctgacagatgtaaactttttcgcgcgttatcccttacgcgttcatacttttcaggatggtattggaaggttaataaatatgaatacaacaacacccatggggatgctgcagcaacctcgcccatttttcatgatcttttttgtcgagttatgggagcgattcggctactacggcgtgcagggcgtactggcggttttcttcgttaaacagcttggattctcgcaagagcaggcttttgtcacttttggtgcttttgctgcgctggtctatggcctcatttccattggcggctatgtcggcgaccacctgctggggaccaaacgcaccattgttcttggagcacttgtgctggcgattggctacttcatgaccggcatgtcgctacttaagcctgacctgattttcatcgccctggggactatcgctgtcggtaacggcctgtttaaagctaacccagccagcttgctttcgaagtgctatccgccgaaagatccgcggcttgatggcgcattcaccctgttctatatgtcgatcaacatcggctcgttgatagcgttatcgctggcccctgtgatcgctgatagattcggttattcagtcacctacaacctgtgcggggcggggttaattatcgcattactggtttacatcgcctgtcgtggaatggtgaaagacattggttctgaacccgacttccggccaatgagcttcagcaaactgttgtacgtgttacttggcagcgtggtgatgatcttcgtatgcgcatggctgatgcacaacgtagaagtcgccaatctggtgctgattgttctctccatcgtcgtcaccatcatcttctttcgtcaggcattcaagctggataaaaccgggcgcaataaaatgtttgtcgcctttgtcctgatgctcgaagcggtggtgttttacattctctacgcccagatgccaacatcgctgaacttctttgccatcaacaacgtgcatcatgaaattctcggtttttccatcaacccggtcagcttccaggcgcttaacccgttctgggtggtactcgccagcccaatactggcaggcatttacacgcatctgggtaacaaaggcaaagacctctcgatgccgatgaaatttactctcggcatgtttatgtgctcactgggctttttgacggcggcagctgcgggaatgtggtttgcggatgcacaagggctgacatcgccatggtttatcgtgctggtgtacttattccagagcttaggtgaactgtttattagcgcccttggcctggcgatgattgctgccctggtgccgcagcatttgatgggctttattctcgggatgtggttcctgacgcaggctgccgcgttcttgctgggcggctatgtggcaacatttaccgcggtgccggacaacattaccgatccgcttgagacgttgcccgtctataccaacgtgtttggtaagattggtctggtcacgctgggcgttgcagtagtgatgctgttgatggtgccgtggctgaaacgcatgattgcgacgccggaaagccattaattattcttgcagaaagcagggtagcgttatcgctaccctgttttagttttacactggcgtacctgcatagatatcaaagcgatgccctttagtgactaccgcgtttggcgtggcgacattcgccagcggtggcgcgtagtccgggcgctttaccaccacgcgtttggtcgccagcaagcgtgcaggctccagtaatccatcggcatcaagatccggtcccaccagcgactgaaagacacgcatctcttttttcactagcgcgcttttctgcttatgcgggaacatcgggtcgagataaaccacctgcgggcgcggggtaatatcagtcagcgccgtcaggctggaggcgtgaattaactgcaaccgctcctgcaaccagccgccgatttccgcatccgcataaccacgcgccaggccgtcgtcgagtagcgcggcaaccactggattacgctccagcatccgcacgcggcagccgactgaagccagtacaaaggcatcgcgcccaagtcctgcagtggcatccaccacatccggcaaataatcgcctttaatgcccaccgctttcgccaccgcctcaccgcgaccaccgccgaatttgcgtcggtgcgccatcgctccgccaacaaaatcaacaaagatgccgccaagttttggctcatcacgcttgcgcaattccagatgttccggcgttaacaccagcgccatcaggttgtcttcatcgtgctccagcccccagcgggccgccagaacagataaggcaccgtctccggtgcctgtttcatcaattaagcagattttcactgaatgatcagcccttaatgccgtaatgctccagcatcgcatccagctgcggttcacgaccacggaagcgtttgaacagatccatcggctcttctgaaccgccacggctcagaatgttgtcgaggaacgactgcccggtttcacggttgaaaatgccctcttcctcaaagcgcgagaaagcatctgccgccagtacgtcagcccacaggtagctgtagtaacctgcggcataaccaccggcgaaaatatggctgaaagcgtgcgggaaacggccccaggacggagatggcaccacggcaaccagtttcttgatttctgccagagtttcgaggatttttgccccctgatccgggcggaactcggcatgaaggcggaaatcaaacaggccgaactccagctgacgcagaataaacagcgccgcctggtagttcttcgccgccagcattttatccagcaactctttcggcagcggttcgccggtttcatagtgaccagagataaacgccagcgcctccggctcccagcaccagttttccataaactgactcggcagttcgaccgcatcccacggcacaccgctgataccggaaacaccagcggtttcgatgcgggtcagcatatggtgcaggccgtgaccgaactcgtggaagagggtgatcacttcgtcgtgagtgaacagcgccggtttaccatttaccgggcggttgaagttacaagtcaaatacgcgaccggtttttgcaaagaaccatcagctttacgcatctggcctacgcagtcatccatccacgccccgccgcgcttgttttcacgggcatacagatcgaggtagaagctaccgcgcagttcgttattttcgtcatacagttcgaagaaacgtacatccggatgccagacatcaacatctttacgctctttagcggtgatgccgtaaatacgcttaaccacttcaaacaggccgttaaccgctttgttttccgggaagtacggacgcagctgttcgtcactgatgctgtagaggtgctgtttttgtttttcgctgtagtaagcgatatcccacggctgcaactcatcgacgccaaattcggctttggcaaaggcacgcaattgcgccagctctttttcgccttgtggacgcgcgcgttttgccagatcggttaagaaatccagcacctgctgcgggttttctgccattttagtggcaagggatttaaaggcgtagttttcaaagcccagcagttgcgccagttcgtgacgcagcgcgaggatctcttccatcaccttgctgttatcccatttaccggcgtttgggccttgatcggaggcgcgggtgctgtaagcgcgatacatctcttcacgcagagcctggttgtcgcagtaggtcattaccggcaagtagcttgggatatccagcgtcagcaaataaccttccagctctttcgcttcggcctgggcttttgccgcagccagcgcgctttctggcatccccgccagctccgcttcgtcggtaacgagtttggtccagcccattgtcgcatcgaggacgttgttgctgtactggttgcccagttcagaaagacgggtcgcaatttcgccgtaacgctgctgtttctctttcggcagacctatgccagagagttcaaagtcgcgcagtgcgttatcaaccgctttcttctgcgccgtgttcagcgtggcgtaatgatcgccatcgcgcaggtcgcgatacgctttatacagcccttcatgttgccctacccaggtgctgtattccgacagcagcggcagggtttgttcgtaggcttcacgcagttccgggctatttttcaccgagttcaggtggctgaccggggagaagatacgccccaacacatcgtccacttccgccagcggctggcagagattttcccaggtgtacggtgccccttgcgctactacgcgctccacgttttcgcggcagtcgttcaatgccttagtcacggctggaacgacatgttccgggagaattttagaaaacggaggcaattcaaagggagtcagtaacggattcgtcattcgcgcagtcctggttaaagaggttaaggaagcgctcaacaggcgctttacataatgtgtgtagcatggggttaagtgtagtgaatttcaatgagaaacgttacgctttcgcggcggcggcctcttttcggtatactgtcctgatacgcttttgtgcgccccgaatacgggccgatttttacttaccggaacacctttacccatgctcagttatcgccacagctttcacgctggcaaccacgccgacgtccttaaacataccgttcagagcctgatcatcgagtcgctgaaagagaaagataaaccgtttctctatctcgacacccacgcaggggccgggcgttatcagttaggcagcgaacatgccgagcgtaccggcgaatatctcgaaggcatcgcccgtatctggcagcaggacgatttgcccgcagaactggaggcgtacatcaatgtggtaaaacacttcaaccgtagcggtcagttgcgttactaccccggttcgccgttgattgctcgcctgctactgcgtgaacaggacagcctgcaactgaccgaactgcacccgagcgattacccgttgttgcgttctgaatttcagaaagatagccgtgcgcgtgtcgaaaaagccgacggtttccagcagcttaaggccaaactgccgccggtttcccgccgtggtttaatccttatcgacccgccgtatgaaatgaaaactgactatcaagcggtggtcagcgggatagcagaaggttacaaacgtttcgccactggtatttacgcactgtggtatccggtggtgctgcgtcagcaaattaagcgcatgatccacgatctggaagcgaccggtattcgcaaaattctgcaaattgaactggcggtactgccagacagcgatcgccgtggcatgaccgcttccggcatgattgtgattaacccgccgtggaaactggaacaacagatgaataacgtgctgccgtggctgcacagcaaactggttccggcaggcaccgggcacgccaccgtaagctggatcgtgccggagtaattgcagccattgctggcacctattacgtctcgcgctacaatcgcggtaatcaacgataaggacactttgtcatgactaaacactatgattacatcgccatcggcggcggcagcggcggtatcgcctccatcaaccgcgcggctatgtacggccagaaatgtgcgctgattgaagccaaagagctgggcggcacctgcgtaaatgttggctgtgtgccgaaaaaagtgatgtggcacgcggcgcaaatccgtgaagcgatccatatgtacggcccggattatggttttgataccactatcaataaattcaactgggaaacgttgatcgccagccgtaccgcctatatcgaccgtattcatacttcctatgaaaacgtgctcggtaaaaataacgttgatgtaatcaaaggctttgcccgcttcgttgatgccaaaacgctggaggtaaacggcgaaaccatcacggccgatcatattctgatcgccacaggcggtcgtccgagccacccggatattccgggcgtggaatacggtattgattctgatggcttcttcgcccttcctgctttgccagagcgcgtggcggttgttggcgcgggttacatcgccgttgagctggcgggcgtgattaacggcctcggcgcgaaaacgcatctgtttgtgcgtaaacatgcgccgctgcgcagcttcgacccgatgatttccgaaacgctggtcgaagtgatgaacgccgaaggcccgcagctgcacaccaacgccatcccgaaagcggtagtgaaaaataccgatggtagcctgacgctggagctggaagatggtcgcagtgaaacggtggattgcctgatttgggcgattggtcgcgagcctgccaatgacaacatcaacctggaagccgctggcgttaaaactaacgaaaaaggctatatcgtcgtcgataaatatcaaaacaccaatattgaaggtatttacgcggtgggcgataacacgggtgcagtggagctgacaccggtggcagttgcagcgggtcgccgtctctctgaacgcctgtttaataacaagccggatgagcatctggattacagcaacattccgaccgtggtcttcagccatccgccgattggtactgttggtttaacggaaccgcaggcgcgcgagcagtatggcgacgatcaggtgaaagtgtataaatcctctttcaccgcgatgtataccgccgtcaccactcaccgccagccgtgccgcatgaagctggtgtgcgttggatcggaagagaagattgtcggtattcacggcattggctttggtatggacgaaatgttgcagggcttcgcggtggcgctgaagatgggggcaaccaaaaaagacttcgacaataccgtcgccattcacccaacggcggcagaagagttcgtgacaatgcgttaaatgttaaagggctaagagtagtgtgctcttagcccttaattacgtttccgctatcagttcagaagctgaagcagaaagcggatcagttccagcagcgcaattaacgcccctagaacgatgattgctttatcaatcacccgttttctccatgcgatggagtgagaatgcatccgcttactcatccactgcctgtcacggcgcatgtctcattgttagataagaactctctcactccggccagagcatcagttaacggcaccacccgtacttctgaccaggactttgaaagcgtttatgcgcattgccagagtgaaaatgcctcagagctaactggataatcatacagtacatgcaggttataaaaccagcacgtccttgcaatagtttcagtatggtattagcattgatgcgttagatgatggctatctcactccagtcagagccaccaactcagggctggaaagtaaaaaaccgacgcaaagtcggtttttttacatccggattcggacaaggcttaatatgacgatgacccagtgaaagtatataaatcgtcactgcgatatataccgaagtgctccctccgccagctgaagaaatcgctaattcttgcaatgttagccactggctaatagtattgagctgttagataagaactctctcactccagccagagccaccaactcagggctggaaagtaaaaaaccgacgcaaagtcggtttttttacgtcctgattcagacctcctttcaaatgaatagccaactcaaaattcacacctattaccttcctctgcacttacacattcgttaagtcatatatgtttttgacttatccgcttcgaagagagacactacctgcaacaatcaggagcgcaatatgtcatttctgttacccatccaattgttcaaaattcttgctgatgaaacccgtctgggcatcgttttactgctcagcgaactgggagagttatgcgtctgcgatctctgcactgctctcgaccagtcgcagcccaagatctcccgccacctggcattgctgcgtgaaagcgggctattgctggaccgcaagcaaggtaagtgggttcattaccgcttatcaccgcatattccagcatgggcggcgaaaattattgatgaggcctggcgatgtgaacaggaaaaggttcaggcgattgtccgcaacctggctcgacaaaactgttccggggacagtaagaacatttgcagttaaaaatttagctaaacacatatgaattttcagatgtgttttatccgggaggcattatgttactggcaggcgctatctttgtcctgaccatcgtattggttatctggcagccgaaaggtttaggcatcggctggagtgcaacgctcggcgcagtactggcgttagttacgggcgtggtccatccgggtgatattccggtggtgtggaatatcgtctggaacgcgacggctgcgtttatcgccgtcattatcatcagcctgctgctggatgagtccggcttttttgaatgggcggcgctgcacgtctcacgctggggtaatggtcgtggtcgcttgctgtttacctggattgtcctgctcggtgctgccgttgccgccctgtttgccaatgatggcgcggcgcttattttgacaccgattgtcatcgccatgctgctggctttagggttcagtaaaggcactacgctggcgttcgtgatggcggccggattcattgccgataccgccagcctgccgcttattgtctccaacctggtgaatatcgtttccgctgatttctttggcctcggctttcgcgaatacgcctcggtgatggtgccggtggatatcgccgcgattgttgccacgctggtgatgttacatctctattttcgcaaagatattccgcagaactacgatatggcgctgctgaaatctcccgcagaagcgatcaaagatcctgctacgttcaaaactggctgggttgttttactgcttctgctggtgggatttttcgtcctggaaccgctcggcattccggtgagcgccattgcagctgtgggcgcgctgatattatttgtcgtcgctaaacgcggtcatgcgattaatacgggtaaagtcctgcgcggtgccccctggcagattgtcatcttctcgctcggcatgtatctggtggtttatggcctgcgcaatgccggattaacggaatatctttctggcgtactcaacgtgctggcggataacggcctgtgggccgcgacgctcggcaccggattcctcaccgccttcctctcttctattatgaacaatatgccgacggtactggttggcgcgttgtccattgatggcagcacggcatctggcgttatcaaagaagcgatggtttatgccaatgtgattggctgcgatttgggaccgaaaattaccccaattggtagcctggctacgctactctggctgcacgtactttcgcagaagaatatgactatcagctggggatattacttccgtacagggattatcatgaccctgcctgtgctgtttgtgacgctggctgcgctggcgctacgtctctctttcactttgtaatgagatactgatatgagcaacattaccatttatcacaacccggcctgcggcacgtcgcgtaatacgctggagatgatccgcaacagcggcacagaaccgactattatccattatctggaaactccgccaacgcgcgatgaactggtcaaactcattgccgatatggggatttccgtacgcgcgctgctgcgtaaaaacgtcgaaccgtatgaggagctgggccttgcggaagataaatttactgacgatcggttaatcgactttatgcttcagcacccgattctgattaatcgcccgattgtggtgacgccgctgggaactcgcctgtgccgcccttcagaagtggtgctggaaattctgccagatgcgcaaaaaggcgcattctccaaggaagatggcgagaaagtggttgatgaagcgggtaagcgcctgaaataaagcggcgatatcccccccacaggttgttagaaaagtgcgctttatttatgtcggatgcgacgctggcgcgtcttatccgacctacaaagttatgaaaattcgatgaatagtatgttatttgtaggcctgacaggcgtagcgcatcaggcgattttgctatttacacagtactccctgcgtgagattccaattatcgcgtccagcatggtgtatcagtgagctgcttagttatcagcgatacagcgcagtagtttaaagacgtactggattatgatttatcagtggtttacacaacaaattattaaataattataagataccttaacccattttattattacacatctaaaacatcacaaaaaaaatcacttcacacactatcagagaacataataactttttaaaatgagcgcattttgatagttgttaacgatttcctttacgatactatcactaccctttttttacacacaaatattaccgggtggagataaaagggaaatcaaaggtaattatatcaggaagatataacgcattacatttattgtgtgtagaagaaaatccattcctgttctaattatccaatttaaacatcttagcataaaacaaatgatgaataaggaattttatgtcaattgactttaccccaggtataataaatacatatcacggcgatatttataactgcacaacaaataccgataatgctaaaacgccagacacaccgaagtggccttgcgataattgggaagaacaacaacccattaattccacattctctggagaaggatatatctctgatcaatatgatttagcgcaacaccaacttcaacaaattaatgcgtgccacacgaacactacatatacaaatgcagactactcaaaagttgtggctcaacttgtaagtcttattactaacattgaaacgataagttcgacacaacttacgcaacagacacaatcaatacttaatcagattaataacattagatatgaaaaaaacaaaagtgctgaatgtcgaatcattgttatcgctaatcctaaacccgacaaggcaatcataactaaaattagcgtagaagagggaatacccataacattcagtgtccaaaccatgttttcagatactaattttattgctgaacaacgagctgacttaccaactaatataaaagatattcaaagcctgtatcaaaaaatgacgaagttatatattgagcacagtgaaaataaaaacaggatgaaagtctttgccggaaccaactttattgatttcaatatgacaggacagaacctgtccgggttcgttctaaccttgtcaaggttttatttcgaagatctacttaatataaatttcactgacgcaaatttagggaaggtgcgaataagcggggaaattcttctcggctgactcagtcatttcatttcttcatgtttgagccgattttttctcccgtaaatgccttgaatcagcctatttagaccgtttcttcgccatttaaggcgttatccccagtttttagtgagatctctcccactgacgtatcatttggtccgcccgaaacaggttggccagcgtgaataacatcgccagttggttatcgtttttcagcaaccccttgtatctggctttcacgaagccgaactgtcgcttgatgatgcgaaatgggtgctccaccctggcccggatgctggctttcatgtattcgatgttgatggccgttttgttcttgcgtggatgctgtttcaaggttcttaccttgccggggcgctcggcgatcagccagtccacatccacctcggccagctcctcgcgctgtggcgccccttggtagccggcatcggctgagacaaattgctcctctccatgcagcagattacccagctgattgaggtcatgctcgttggccgcggtggtgaccaggctgtgggtcaggccactcttggcatcgacaccaatgtgggccttcatgccaaagtgccactgattgcctttcttggtctgatgcatctccggatcgcgttgctgctctttgttcttggtcgagctgggtgcctcaatgatggtggcatcgaccaaggtgccttgagtcatcatgacgcctgcttcggccagccagcgattgatggtcttgaacaattggcgggccagttgatgctgctccagcaggtggcggaaattcatgatggtggtgcggtccggcaaggcgctatccagggataaccgggcaaacagacgcatggaggcgatttcgtacagagcatcttccatcgcgccatcgctcaggttgtaccaatgctgcatgcagtgaatgcgtagcatggtttccagcggataaggtcgccggccattaccagccttggggtaaaacggctcgatgacttccaccatgttttgccatggcagaatctgctccatgcgggacaagaaaatctcttttctggtctgacggcgcttactgctgaattcactgtcggcgaaggtaagttgatgactcatgatgaaccctgttctatggctccagatgacaaacatgatctcatatcagggacttgttcgcaccttccttaggtgacactatttttttacataaagaacaccctacccccaaattatataaagatggacaatatcttgacaaacaaatcgaaggtttattttcaacattattaaccattaatgacaaccttttacgagcaaaagcggaaattgcttcgacaataattaaatttttagaggccaggataaccaatctttcatacaatgacatattaaaatatcagcaagaattccaaagacaatgttataagcaagttaaagcctttacgacactctcccgatacaataaaattcaaacatgggcagaaatgtctgaatatcaattcgaagtatttcaatacgagacgcttaacccaaaaaaaatgtcacacacgccttatttaaagaggccactgcctaatgaaaaagatataaattatggggtggaaatagaaataccatctggtaaaagaattcgcttatcaaatcattaccagaatataataccataatattgattattagcactttataatcattgaataaaaatagattttatgtacttttaaaacaatgcactatattatggggtgatggatattcatgtcacgccccaaaattaactgagttcacctaaacagaaaggatataaacatcagacaggtttacgttactatcaggcatatcacctcagaatcagatgaaaactataaagaaatatctattatggttttaatatttgttgataaggatagtaacatgaacatgacaaaaggtgcactcatcctcagcctttcatttttgcttgccgcatgtagttcaattccgcaaaatatcaaaggcaataaccaacctgatattcaaaaaagttttgttgctgttcataaccagccggggttatatgttggtcaacaagcgcgctttggtgggaaggttatcaacgttatcaatggcaaaacggatacgttgttagaaatctctgtattaccgttggatagctatgcgaagcctgatattgaagccaactatcagggccgactgctcgccagacaaagcggcttccttgatccagtgaactatcgtaatcactttgttaccatcctcggcaccattcagggtgaacaacctggctttatcaataaagtcccgtataacttcctggaagtgaatatgcagggcatccaggtgtggcatttgagagaagtggttaataccacctataacctgtgggattacggctatggtgcattctggccggaaccgggctggggtgcgccttactacaccaatgcggtgagtcaggtaacacctgagctggtcaaataacaccaccgaaagatgcagatgctttctcagcatctgcatcatgcattacatcaaattaatacacagtaagctaactattattattataagccctgtcctgttaattacctttggcaaactgattataaagttaatgtccgcaccaggagtcggttatgtttcttataattaccagggatacgatgttcttcaccgcgatgaaaaacattctgagtaaaggtaatgtcgttcatatacagaacgaagaagagatcgacgtaatgttgcatcagaatgccttcgtcattattgatacattaatgaataatgtatttcattctaattttctcactcaaattgaacgattaaaacctgtccatgtcattattttctccccctttaatattaaacgctgcctggggaaagtgccggtgacctttgttccgcggactatcactatcattgattttgtcgcactcatcaatggcagttactgctctgtgcctgaagcggctgtgtcactttcgcgcaagcaacatcaggttctgagctgcattgcgaatcaaatgacaacggaagatattctggagaaactgaaaatatcgctaaaaacgttctactgccataaacacaatatcatgatgatcctcaatcttaagcggatcaatgagctggtacgccatcagcatattgattatctggtgtgaatttcaggcttacggtgagtctggctacgctgccacacagattagctaattgaaacgcctttcacccctgccataccttttaataatcgcaacaggtcttctatcgacgttgtggcatgaagctggatatcaatggcgaccacttcatgatcttcattttcctgcaacgaaactaaatcagtttttattttttgctgcttaaaccagtcgagcattgataccgtattaccgttcactaatgtcagctgtaaatggtaatttttgttcatcaggcggaaggttaattgatggaagacttccagcaccaacaaggtcatcactgaaccataaatacccagttcgtacataccgctgccaataaccatacctatggcggcggtcacccagatatccgctgccgtcgtcagacctacaatattttggttacgaacgagaatgttacctgcaccgataaacccgacgcccgtcaccacctgagcagcaatacggctggggtcgagtccgacgtgatctaaagacagcacgtcagcaaaaccatatttcgaaacaatcataaacagggcgcttcccatgccaattaatacatgtgtgcgtaaccctgctcctttgccgcgcatttgcctttccatgccaatagcgccacaggcaattgccgcgagtataagacgtataataaattctgctgtcatataaaaatgcaaaaaggagcagcaagatggctcaacttgctactcctttttacttgcacctcattaattcggcaagtcattagatgcttgatttttgaaggtatacaaatttttctgcgggtttttcttacagtattcgatcactttaggaatttgagtgagatcggtttcatttaaagtaacggtatcgccacctttatatactgtttcttcatgcagcatccaccatgcaaccggggtcattgcttttggattcagatcaataaattcctggcaggtcatatctttagcggattcattggctgccaacgcagattgtgcgttcaccagtgacaaagccgctacagcgcccataaaaataaacgctttacggagagatgaaatattcattttgtaacccattcaatatagagattatatatgaacaggaggaatagctgcttttaaagaagatattccggcctgttcaatatgcaaggaagtacgatgtaacgcattcccggaattacatatctttcttaattttgtcccattcgcctttaactttatctttaaagttggcttgtttatcctgagtacaagcctgaacgatagctggggttacggttgcaataccctgaacatctaaaaccgcatcttctggtttatctttgttgttcagcgcttcagcaaaaccaactgcagttggctggaaggattcgtccacagccaggaaatcttcacaggtccaggagttgaccggttttttgttatcagctgctttttgcgcatccgctgcattgctcacaactggcagaagaagcagaccaccaagaataacgcctaatacttttttcatcgtaatatcctcaactataaagtgaaagagccgtcacgaatcaatttcgacactgaggttataacctggttttctgtatatgtcatgttgatggaaaatatcaaaatcagatatttttatttcaatacaatgagttacagatgcatcagatactgcaattaggaaatttttattaaatcgactgcattcttagacgcgtttttggcatagattgatagcaggggattttcttcttaattttatagggtggttctatgttatatatagataaggcaacaattttgaagtttgatctggagatgcttaaaaaacatcgcagagcaatccagtttattgccgtgctgctgtttatcgtcgggttgctgtgtatcagtttcccgttcgtctctggcgatattttaagcacagtagtgggtgcattattaatctgctcgggtattgcgcttattgtcgggttattcagcaaccgcagtcataatttctggccggtattatccggtttcctcgtcgcagtcgcctatttattgatcggctatttcttcatccgcgcaccggagctgggcatttttgccattgcggcatttattgccggtttgttctgtgttgcaggggttattcgcctgatgagttggtatcgtcagcgttcaatgaaaggcagctggctacagctcgttattggtgtgctggatatcgtcattgcctggatattccttggtgcaacgccgatggtgtctgtaacgctggtttccacactggtgggaattgaactgatatttagcgccgccagcctgttcagcttcgccagtttgttcgttaagcagcaataattaccccggttgtcacccggatcatagtcacttgatgtgactatgatccgattaatactctctccgctacgcagtgttgtagatcaattgcgcactatcattgaaataattacctgctagtgattatttcaacctactgaatttcatctaatttttttcactctatggcaaattagccatttcaaacattatcatggctgatattttccgtagtcaggtttaatgttttaaaagtgctgtgggaaagtgaacaaagagttccgtaagcgttgatgctatgggcggttaaataagtaatccgggttcatttttttgcaactggcgttgattacattgcataaatatccgtgtctccagacgctatataaaaacctgaagacatgaatgcgttatttactcaggtaatttcaatgcgttaaaagaaagctggcaatccaattgccagcttaagtcgaaacaaggagactcgatatttaaatcggattacattttaactttagtaatattcttcagagatcacaaactggttattgataacttattcttgggcagtaatccgcaaacgttaactttttgtttgctatttacaagctgataacaaccaggaatcttacttaggatcaatatatggagtgcgtgatggataaatctgaagtattgattagtgttaatagacgtattagttcacgaagggtaaagttcttataggcgtttactatattgaacaacgattcggacaaggatgtaaataatgaaaaggatgacatattcgaaacgataacggctaaggagcaagttatgatttttctcatgacgaaagattcttttcttttacagggcttttggcagttgaaagataatcacgaaatgataaaaatcaattccctgtcagagatcaaaaaagtaggcaataaacccttcaaggttatcattgatacctatcacaatcatatccttgatgaagaagcgattaaatttctggagaaattagatgccgagagaattattgttttggcaccttatcacatcagtaaactaaaagctaaagcgcctatttattttgttagccgcaaagaaagtatcaaaaatcttcttgagattacttatggtaaacacttgccccataagaattcacaattatgtttttcacataatcagttcaaaattatgcaactgattctgaaaaataaaaatgaaagcaatatcacgtcgacgctcaatatttcgcaacaaacattaaagattcagaaattcaacattatgtacaagctgaaactaagacgtatgagcgacatcgtcaccctgggtatcacatcttatttttagtcaggacataagcaactgaaattgatggctggcatgacgagggatgcagatgctgatttcattacccccggtgattactaaaggagaggctaaaacgactttattcccctggtatgtgtatccaccagtagaacccttcgttgcccgaatgctggcaggaactgttggcagaacggcaacattttttttgtcgttgacctcaccatgtcgatcactgtgcctgtatcccaccttactggctgacaaccccactatgccgctggtctgtaaatccctcatatctctcctcgcgcgcaatttaaagaaccgttatttctcaagaattttcagggactaaaatgaacagaagaagaaagctgttaataccgttgttattctgcggcgcgatgctcaccgcctgcgatgacaaatcggcggaaaacgccgccgccatgacgcctgaggtcggtgtcgtcacactctcccccggttcggtcaatgtgttgagcgaattgcccggtagaaccgttccttatgaagttgccgagatacgtccccaggtgggcggtattatcattaaacgcaactttatcgaaggcgataaagtgaaccagggcgattcgctgtatcagattgatcctgcacctttacaggccgagctaaactccgccaaaggctcgctggcgaaagcgctctctaccgccagcaatgcccgcatcacctttaaccgccaggcatcgttgctgaagaccaactacgttagccgtcaggattacgacaccgcgcgcacccagttgaatgaagcagaagccaatgtcaccgtcgccaaagcggctgttgaacaggcgacgatcaatctgcaatacgcgaatgtcacctcgccgattacgggcgtcagcgggaaatcgtcggtgaccgtcggcgcactcgttaccgctaatcaggcagattcgctggttaccgtacaacgtctggacccgatttatgtcgatctcacgcagtcggtgcaagatttcttacgcatgaaagaagaggtcgccagtgggcaaatcaaacaggttcagggcagtacgccagtacagctcaatctggaaaatggtaaacgctacagccagaccggcacgctgaaattctccgacccgacagtggatgaaaccacgggctccgtgacgttacgggcgattttccccaacccaaatggtgacttgctgcctggcatgtacgtcacggcattagtggatgaaggtagccgccagaatgtattactggtgccgcaggaaggcgtcacccacaacgcccagggtaaagcaacggcgctcattctggataaagacgatgtcgtgcagctacgcgaaattgaagccagcaaagccatcggcgaccagtgggtcgtcacctctggcttgcaggctggcgatcgggtgatcgtttccggtttgcaacgcattcgtccgggtatcaaagcacgagcaatttcctccagccaggaaaacgccagcaccgaatcgaaacaataacgttgcaggcttaaggggactttcatggctaactattttattgatcgcccggtttttgcctgggtacttgccattattatgatgcttgcaggtggtctggcgatcatgaacttaccggttgcgcagtatccgcagattgcgccaccgaccattaccgtcagcgctacctatccaggtgccgatgcgcaaacggtagaagactcggtcactcaggtgattgagcaaaatatgaatgggcttgatggcctgatgtacatgtcttcaaccagtgatgcggcgggcaatgcctctatcactctgaccttcgagactgggacatctcctgatatcgcacaggttcaagtgcaaaataaactgcaactcgctatgccttcattacctgaagcagtgcagcagcaggggattagcgtcgataagtcgagcagtaatatcctgatggtagcggcgtttatttctgataacggcagcctcaaccagtacgatatcgcggactatgtagcgtctaatatcaaagacccgctaagccgtaccgcgggcgttggtagcgtacaactctttggttccgagtatgccatgcgtatctggctggacccgcaaaaactcaataaatataacctggtaccttccgatgttatttcccagattaaggtgcaaaacaaccagatttccggtggtcaactgggtggcatgccacaggcggcagaccagcagctaaacgcctcgatcattgtgcagacgcgtctgcaaacgccggaagaatttggcaaaatcctgttgaaagttcagcaagatggttcgcaagtgctgctgcgtgatgtcgctcgcgtcgaacttggggcggaagattattccaccgtggcacgctataacggcaaacctgctgccgggatcgccatcaaactggctgccggagcaaacgccctggatacctcgcgggcagtcaaagaggaactgaaccgcttatcagcctatttcccggcaagtctgaagacggtttatccttacgacaccacgccgtttatcgaaatttctattcaggaagttttcaaaacactggttgaggctatcatcctagtcttcctggtcatgtatctgtttttgcagaatttccgtgccacaatcatcccgacgattgccgtaccggtggttattctcgggacgtttgcgatcttgtcggcggtcggtttcaccatcaacacgttgactatgttcgggatggtgctggcgatagggttactggtggatgacgccatcgtggtggtggagaacgtcgagcgtgtcattgcggaagataagctaccgccgaaggaagcgacgcataaatcgatggggcagatccaacgtgcgctggtcggtattgccgttgttctttccgcagtgtttatgccgatggcctttatgagcggtgcaaccggggagatctaccgccagttctccatcacgctgatctcctccatgctgctttcagtatttgtggcaatgagcctgacccctgccctgtgcgccaccattctgaaagccgcgccggaaggcggtcacaaacctaacgccctgttcgcacgcttcaacacgctgtttgaaaaatcaactcaacactataccgatagcacccgctcgctgttgcgttgtaccggtcgctacatggtggtctacctgctgatttgcgccgggatggcggtgctgttcctgcgcacgccgacctctttcttaccagaagaggatcagggggtatttatgaccaccgcgcagttaccttccggtgccaccatggttaacaccacgaaagtgctgcaacaggtgacggattattatctgactaaagagaaagataatgtccagtcggtgtttaccgttggcggctttggcttcagcggtcaggggcaaaacaacggcctggcgtttatcagtctcaagccgtggtctgaacgtgtcggtgaggaaaactcggttaccgcgatcattcagcgggcaatgattgcgttaagcagtatcaataaagccgtcgtcttcccgttcaacttacccgcggtggctgaactgggtaccgcgtcaggttttgatatggaactgctggacaacggtaacctggggcacgaaaaactaacccaggcgcgaaacgagctgttatcactggcagcgcaatcaccgaatcaggtcaccggggtacgcccgaacggcctggaagatacgccgatgttcaaagtgaacgtcaacgctgcgaaagctgaagcgatgggcgtggcgctgtctgatatcaaccagacaatttccaccgccttcggcagcagctacgtgaacgacttcctcaaccaggggcgggtgaaaaaagtgtatgtccaggcaggcacgccgttccgtatgttgccggataacatcaaccaatggtatgtacgcaacgcctctggcacgatggcaccgctttctgcctactcgtctaccgaatggacctatggttcaccgcgactggaacgctacaacggcatcccgtcaatggagattttaggtgaagcggcggccgggaaaagtaccggtgacgccatgaaatttatggcagacctggtcgctaaacttccggcaggcgtcggctactcatggaccggactatcgtatcaggaagcgttatcctcaaatcaggctcctgcgctgtatgcgatttcactggtcgtggtgttcctcgccctcgccgcactctatgagagctggtcaattccgttctcggtgatgttggttgttccgttaggcgtcgttggcgcattactggccaccgatctgcgcggcttaagtaatgacgtctacttccaggttggtttgctgaccaccatcgggctttccgccaaaaacgccatcctgattgtcgaatttgccgttgagatgatgcagaaagaagggaaaacgccgatagaggcaatcatcgaagcggcgcggatgcgtttacgcccaatcctgatgacctctctggcctttattctcggcgtgctgccgctggttatcagtcatggtgccggttctggcgcgcaaaacgcggtaggtaccggcgtgatgggcgggatgtttgccgcaacagtgctggcaatttacttcgttccggtctttttcgttgtagtggaacatctctttgcccgctttaaaaaagcgtaacgtgtaaatgagagtaaggttgaacatgaaggttcagccttactctttcctgctaaccattcaccactcaacaaccagctaaccgtcaggaataccaggcttagtacacagcactgaaagtagaaaccactccagccattcgtcatcaatttgaacaacacaatactgacccacattcccgtaatcgtatgaattgtcagcttaataatcccaaacatgccgagtcttttcctcctgaaaataccgataccgcctggcaaactgcgaaagagaactagccggtagcccggcagaaatcatcagggaagagtttcacatgaagcaggtgtgagatcctgaccaatattcaaatgcgaaatatgtcaggaaaaggtacctggcgaatgttgcgcaaactgatgtggcgttacaccataatattgtcgaaatgtgtttataaagtacgatgtactgctatagccacatttttccgcaatagtatgcagaggaatttgacgtaactcgagtaatcgtctggccatcgacatcctggaggcgagtaatattttactgaaacaggtattttcatcctgcaacttttttttgattagactctcgctggtatacattctttccgcgatatcgcgcagataccaacgtttggcgatatcaaagctaataaggcgttcaacttttcctgaaacagtgctgatgctattgaaaagtaaggggatcagttctttcttatgagaaaacatcgataaacaggaaaggtagagcatattgctcagtatcggtgaatttaccccggattcattgaagctatcaaaaatcgccgtcaccagcggcatggggggtgactggttaattaacaaacggtctttgctgtgtaaccctaaattgcgtggtagctgacgaatattttgtaagtaatggcaaactgtcagctcatcgatatccagtcgtcgcgtatccggtgaacaaaacgcaaaatcgtctgccaaatttttctccagcagcagaatactctcgttatgcagcgatattttttgctgttcatgataaatatcgaatgaacgacgaatgaggatcaccgagcagacatgagtcatgattatcccttatatttcatactgcgattatttcaatttcagtatactaatgaaatgatgccagactgtttcttagcgcaaaaactgccagatttggtaggaccaaaatttatccacaaagtagttttgcataacagttaattgataataagtaaatgcagcacgaatatattttcgcacagcgtatagcttatgtttataaaaaaatggctgatcttatttccagtaaaagttatatttaacttactgagagcacaaagtttcccgtgccaacagggagtgttataacggtttattagtctggagacggcagactatcctcttcccggtcccctatgccgggttttttttatgtctgagtaaaactctataatcttattccttccgcagaacggtcagtgccgtaaaaattcccttgcgcaacaatacttgccgccgagtcacggttcgacaatctctgcgccgatcgctcctgatactctgtgggcgtcatcccataataatttcgaaagacgtaaatgaaatacgacacgctgtgatatccacaggatactgcaactcgcttaattgaaaaaccatgtataacaataagttgcaaagcacgttgcattctacactcagtaagcaactgtgaatatgatgtctcttcttcgcgcaattttttctttaacagacttggactcatcaacagctcgctggcgattcgggctagtgtccactcatgggcgatattattattgataaccgtacaaactcgtgttcgcatgttcggttgtaaaacgttcagaagcagcggtataaagtgctcatcctcaagaaaaacagataacaacgcaaagattaatgctcttttacgtagcatttctgcatagcgaagattcttattctgcgatagttgcgcaacttcctgaaaaacaggaatatctctactacagtgatgaacgagtaatgaagaaacttttttatgtgcatgaagatttaatgcctcctccttgagcatcgggagaaataatgaaagcgtgtcccttgacacgaatacaaaattttcaacacacttatctactcgaatttggcttgcatccgcaaaaaccaggtcaccgccattaaaatagcgatattcaccattaaccatggtgagaatatatttatgtcttgcatacgcaattagacaattcccatgtagtgattgcatagttgacttaatattacataaacatattactgtttattaatgtagcacgccgccctcttaagtcaaattgattgataaataaatttaaacgaagcgggagaacaggatgataatgtgtgatgttctacgggcaggatgactggatttataatacaaaaacgtgtttaagaacacagggaaattaatagtaagcaaataatcccttttcgtgacattaaaggtaatcgctacatttaataaacattcatataacatatatcttatcaacacgatgaatagacagccaatatattattgcgattaataagcaaccgaatgcccagctgtttttttaaaggctgggcattcggtttttacaacgttatgttatcaggtgtgtttaaagctgttctgctgggcaataccctgcagtttcgggtgatcgctgagatatttcagggaggctttgtagtcttccagcaacagttcagcaaagtccatttcgaagccgcgacgacacataatgcgcatcaccacgatgtcggtggcttcaccgccgagagtgaaggccggaacctgccagccgcgcagacgcagacgttcagagaggtcgtacagggtgtatcccggatcttcaccatctttcagtttgaagcaaaccgccgggatgccttcgtccgggcgacccgtacagatgaactcatacggccccagtttggcgatttcatccgccagataagcggcaacctggtaagaggcgttctgtactttggtatagccttcacgaccgaggcgcaggaattcatagtactgtgcaattacctgacccgccgggcgggagaagttgatggcaaaagtaccaatttgaccacccaggtagtcaacgttgaacaccagttcctgcggcagcgcttcttcgtcacgccagataacccagccgcagcccagcggagccagaccgaatttatggcctgaagcactgatcgatttcacacgcggcaggcggaagtcccagacgatatccggggcgacgaacggtgccaggaagccaccgctggcagcgtcgatgtgcatgtcgatgtcgataccggtgtcggcctggaatttatccagcgcatcgtgcagcggttgtgggaactcatagttaccggtgtaggtcacgccgaaagtcggcaccacgccgatggtgttttcgtcacaggcttcaatcatgcgtttcgggtccataaacaactgaccggggcgcatagggatctcacgcagctccacatcccagtagcgggcgaatttatgccagcagatttgtaccggaccgcacaccaggtttggtttatccgttggtttgcctgcagcttccatacgcttgcgccaacgccatttcatcgccatcccgccgagcatacaggcctcggaagaaccaatggtgttggtgccaacggcctgaccatttttcggcgcaggcgcatgccacagatcggcaaccatatttacgcaacgcaggtcgatggctgcggattgcggatattcttctttgtcgatccagtttttattgatcgacaaatccatcaatttatggacgttttcgtcgtcccaggtctggcagaaagtggccaggttctgacgagcgttgccatcaagatataattcatcattgataatctgaaatgcgacatcatcgcgcatttcgtgcagcggaaatcgttttgactccgcgatagtagaaatggcctttgcgccaaaacgtgaatcgagtagttctgagcggaaatccgttaacagcttctggtccatttcgaactccttaaatttatttgaaggcaataaaaaagtaggatttatccgcaatggaagcaaggcattacaggcttaatttaaataacaaaatcctaagcagaaaaacgactttttataatataaacatttaacatgataatattaaaaacagactttattatcgtaataaaaatcgcccaaacattgctgttcgggcgatcaaattaattattgtttatcctgcatatacggcgtgtacaccccgttcagactgtgcaggaaagctacgatatcatccacatcctcctgcggcagctctttgcctacctgatagcgcagcatcagtttcaccgccccgtccagcgtcggcacgtcaccgcgatggaagtacggtgccgttaaagcaacgttacgtaaaccgggtactttctgacgcaatttatcacgctcttctttagtcacattcatacgaccaatatccgccgccgtaatttccccaaagttaaagtcttttttcagccccaacggttcaaaggaacgtccgccgagaataataccaccatgacaagttgcacatttattatctttaaataattgatagccttttttctgttgcgccgtcagcgcattttcatctccgcgcaaccatttatcaaatggggaatccggcgtaattaatgttttctcaaattcagcaatggcatcagtaatattttcgccactgaaaccttgcggatagacttcgaggaactgcgttttaagctgcggatctttttccagcttagcaataatttcgtcccaggatttcgacgccatttcaatcgggttcaacggcggtccaccagcctgatcctgcaatgttgccgcacgaccatcccagaactgctcaacgttaaatactgagttaaataccgtcggcgcgttaatcggcccaactgcgccaccaacaccaatcgatgtttttctgccatcgacgccccccgcattcaacgcatggcaatgagcgcatgaaatggtgctatcagccgataaacggggatcgtgatacagcgcaaaacccaacgccactttttgcgcatcggtaggcagtttttgcgggatgggctgcaccggttcattgcgatgttccggagcagtatcattgctggcgtaatattccgcgcgctgttttgcaatccaggccagtatttccgcccgctcttcatcactcaccttacccgcccagtgtagcgcggtataacgcgttggtggcatagtttcatactgcatcacccattcaatcttattcaaatcgctttgcgaaacgggtttatcagccagcagtgccgcacgcacggcctcaaggttaaaagatttatatccaagcttaatgtcgtaatccatcaactgtttcgcgccaggaatataataataggcgggtaattctgccgaaggcgtgtggcaatagtcgcatcctttttcgcggagaaagcctaaaaccttattattttcactgacagcagatgcctgaacatcggcctgtttactgcgtttattatcgtggtaccacacataaccagataaccctaaatagcaaatcgcgacgccagccaggccgatcgcggtaatacgtgagaccattttcattattcttccctcacggtggtgagttattgtgacccagaaaattttccagaatgctgcaaacgtctctgcgagacaaagccatcataaaaaacagggagatacgctttttgataggaatcaatcaattacatgaatataaactatcaataagatagcctgtgcctattacccagatcaggaatggcatatcatgattgcggcgagagcaggattgaatgttctgaaaatgaaaaacaacaccaaatcggtatttttataaattccattgatattagtgcgttatattttttgacaggttaataaacgtgatccaccgcacgctttgtcgcccaccaggcggagcgaatgactacccttaaagaaaagccgataattagcgacgaatttcggaggttggatccttatgctcaatcagaaaattcaaaaccctaatccagacgaactgatgatcgaagtcgatctctgctatgagctggacccgtatgaattaaaactggatgagatgatcgaggcagaaccggaacccgagatgattgaagggctgcctgcctctgatgcgctgacgcctgccgatcgctatctcgaactgttcgagcatgttcagtcggcgaaaattttccccgacagtaaaacctttcccgactgcgcacctaaaatggacccgctggatatcttaatccgctaccgtaaagtgcgccgtcatcgtgattttgacttgcgcaagtttgttgaaaaccacttctggctgccggaggtctactccagcgagtatgtatcggacccgcaaaattccctgaaagagcatatcgaccagctgtggccggtgctaacccgcgaaccacaggatcacattccgtggtcttctctgctggcgctgccgcagtcatatattgtcccgggcggccgttttagcgaaacctactattgggattcctatttcaccatgctggggctggcggaaagtggtcgggaagatttgctgaaatgcatggccgataacttcgcctggatgatcgaaaactacggtcacatccccaacggcaaccgcacctattatttgagccgctcgcaaccaccggtttttgcgctgatggtggagttgtttgaagaagatggtgtacgcggtgcgcgccgctatctcgaccaccttaaaatggaatatgccttctggatggacggtgcagaatcgttaatccctaatcaggcctatcgccatgttgtgcggatgccggacggatcgctgctcaaccgttactgggacgatcgcgacacgccgcgtgacgaatcctggcttgaggacgttgaaaccgcgaaacattctggtcgcccgcccaacgaggtgtaccgcgatttacgcgcgggggcggcctccggttgggattactcttcccgttggctgcgtgatactggtcgtctggcgagcattcgtaccacccagttcatccccatcgatctgaatgccttcctgtttaaactggagagcgccatcgccaacatctcggcgctgaaaggcgagaaagagacagaagcactgttccgccagaaagccagtgcccgtcgcgatgcggtaaaccgttacctctgggatgatgaaaacggcatctaccgcgattacgactggcgacgcgaacaactggcgctgttttccgctgccgccattgtgccactctatgtcggtatggcgaaccatgaacaggccgatcgtctggcaaacgccgtgcgcagtcggttactgacacctggcgggattctggcaagcgagtacgaaaccggtgaacagtgggataaacccaacggctgggcaccgttacaatggatggcgattcagggatttaaaatgtacggcgatgaccttctgggtgatgaaatcgcgcgaagctggctgaagacggtgaatcagttctatctggaacagcacaaactgatcgaaaaataccatattgccgatggtgttccccgcgaaggcggcggtggcgagtatccgttgcaggatgggtttggctggactaacggtgtggtacgccgtttaattggtttgtacggcgaaccataatatttttacagccagccgctaacttcctgctggctgtaaaattatcctcttcaggaggagatatttaacatcattgccgcctgggtgcgatttttcacttccagacggcgatacagggattccagatgcgcttttaccgttccggtactgatattcagcgctctgccgatctccttatttgattcgcccgccgctaacatggttaaaatctcccgctggcgggcgcttaacgatttgagatctttaatgtccttttccggcgtcgtccgccagtctccaggcagaaacatcatccccatcgccgcactatttaccgccaacgcaaatgtctcgacggttgaatcacgaggcacaatggccagcacattaaaatggataacttcctgtaaccaccgtttattgcaatccgtcgccgtaattaacaccttaacctcaggaaattgcaccacggttttttgcagcaaccagtagcaaaactcaccatcctgatcgccatcgagcataactaaggcttcagggtaactttccagcttttgccataactcgtctgcctgactggccccctgaatactcactcctggaatacgctgctgtaaactgattttcattccatgaataaatattgactgcctgtcaaacatgactatttgcataactgaatctccacctgaatacgttaaaaagacttaagtagtggaagggtattacccgcgagaaaaaataagaattcgccatttggcggtggccattctacagagatgacgtgtagaaaatagttaccgatataaatagttacagctaaacgcctgaaattacatgtcgagggcactatttaaaacaattttgaggatttccttatattggtggttagtacgcatgcaattaaaaatgaaattccgcgaccacaagccaaaataacaaacggcaaggagacaaaaataagcacaaatagccaacacgtcctctgttcactttaaagggaatcgctgaaaaatacgctctgtttaaggggattcacctttctcagaaagctattccgcccttttcctgctgagaaatcgccacattcggcatgacaacattgtgaaacccggcattagatgttagaaaaaacaataaacaatgcgatatgcgcgttactgtttcgctgtgaacaacaatcggtcaaagaaatggataaaattcacgcaatgcagttgttcatcaaagtcgcggagctggaaagtttttcccgcgcagcggatttctttgctttgccaaagggaagtgtttcgcgccagatacaggcactggaacatcaacttggcacccagcttctccagcgcaccacgcgacgggtcaaactcacgccagaaggcatgacctattatcaacgagcaaaagatgtgttgagtaatctcagcgaactggacggtctgtttcaacaggatgccaccagtatcagcggtaaattacgcatcgacatcccgccaggaatcgcgaaaagcctgttactgccgcgcctgtcggaatttctctatctgcatccgggaattgagctggaactgagtagccatgaccgtccggtagatattcttcatgatggttttgattgcgtgatacgcactggcgcgttaccggaagatggcgttatcgcccgtcccctcggcaaactgaccatggtcaactgtgccagtccgcactatctgacgcgctttggttatccgcaaagccccgatgatctgacttcacacgcaatagtgcgttatacaccgcacctgggtgtacatccgttaggttttgaggttgccagcgttaatggcgtccagtggtttaagtctggcggcatgttgacggtaaacagtagcgaaaactatctcaccgccggtcttgccggtctggggattattcagatcccgcgcattgccgtgcgcgaagccctgcgtgccgggcggcttattgaagtattacctggctaccgtgccgagccgctctccctttcgctggtttatccgcagcgtcgggagctttcccggcgtgtaaacctgtttatgcagtggctggctggcgtaatgaaagagtacctggactgaccgactatactttttaagaatgaccacgacagaaggacaaaagagcggatgacgcaggaaaacgagatcaaacgtcccatccaggatctggagcacgagccgattaagccgttggataatagcgagaaaggcagcaaagttagccaggcgctggaaaccgtcaccaccactgccgaaaaagtccaacgccaaccggttattgcgcacctgattcgcgcgacagaacgctttaacgatcggctgggtaaccagtttggtgcggctatcacctatttctcatttttgtcgatgataccaattttgatggtgtcgtttgccgcagggggctttgtgctggcctcccatccgatgttgctacaggatatcttcgacaaaattctgcaaaacatcagcgatccgacgctagccgccacgttgaaaaacaccatcaacaccgccgttcagcagcgtacgactgtagggcttgtcggcctggcggtggcactttattccggcatcaactggatgggtaacctgcgtgaagcgattcgtgcccagtcgcgcgatgtctgggaacgctcgccgcaagatcaggagaagttctgggtaaaatatctgcgagattttatttcgctgattggtttgttgattgcgctgattgtgacgctttcgatcacctcggttgccggttcggcgcagcaaatgattattagcgccctgcacctgaacagcattgagtggctgaaaccgacgtggcgattgattggcctggcgatttccatcttcgccaactatctgcttttcttctggatcttctggcggttgccgcgccaccgtccgcgcaaaaaagccctgattcgcggaacatttctggctgctattggttttgaagtgattaaaatcgtgatgacctacaccctgccatcgttgatgaaatccccctctggcgcagcatttggttccgtgctggggctgatggcatttttctacttcttcgcccgtttgacgctgttttgcgcggcgtggattgccaccgccgaatataaagacgacccgcgaatgccggggaaaacgcagccttaaaataggccggatgcggcgtaaacgccttatccggcatacgattttattcggcctggctccccgtaggccggataagatgcgccagcatcgcatccggctataatgcgcacataacctcttgaaactcgtccccagagcctcttcagccatctatttgggagcaaacaatttcattccaactcataaccccagcatataaatccagttggtaacttttatttaacctgaaaccagttttatccactatttataaaattatgtgaagcatttcatagaagaaaaatcactggcctaaacattatcccctttttgcctgatttttgaccatttccgcgatttgttacacattgaaatatcacttttgctgtgcgtaatatggctattcgttagccaaaaaataagaaaagattatgcaagcaacagccacaacactcgaccacgagcaagaatacacgccgatcaactcgcgtaataaagtccttgtcgcctctctcattggcacagccattgagttcttcgacttttacatttacgccactgcggccgttattgtgtttccgcatatcttcttcccgcagggcgatcctacggcagcaacgctacagtcgctcgccaccttcgccatcgccttcgtcgcgcgccccattggctctgccgtttttggtcattttggcgatcgcgttgggcgtaaagcgacgctggtcgcctcgttgctaacgatggggatttcgaccgtggtgattggtctgctgccgggctatgccacgattggtattttcgccccgctgctgctggcgctggctcgatttggtcagggtctgggcttaggcggtgaatggggcggcgcggcgctgctggcgactgaaaacgccccaccgcgcaaacgtgcactgtatggctcctttccgcagctgggcgcaccgattggcttcttctttgccaatggcactttcttgctgctttcctggctactgaccgacgagcagtttatgagctggggctggcgtgtgccatttatcttctcggcggtgctggtcattatcggcctgtatgttcgcgtgtcgctgcatgagtcgccggtgtttgagaaagtcgctaaagcgaaaaaacaggtgaagatcccgctgggtacgctgctgaccaaacatgttcgcgtaaccgtactgggtacgttcattatgctggcaacctatacgctgttttacatcatgacggtctactctatgacctttagtaccgccgccgcgccagttgggcttggcctgccgcgtaacgaagtgttgtggatgttgatgatggcagttattggttttggcgtgatggtgccagtcgctggattactggctgatgcctttggtcgccgtaaaagcatggtaatcatcaccacgctgatcatcctgttcgcgctgttcgcctttaacccactgctcggttctggcaacccgattctggtttttgccttcctgctgctggggttaagtctgatgggtctgaccttcgggccaatgggtgcgctgttaccagagctgtttccgacagaagtgcgttacaccggagcatcgttctcttacaacgtagcgtcgattctcggggcttccgttgcgccatatatcgcagcctggttgcagactaactacgggctaggtgcggtggggttatatctggcggcgatggctggcttgacgttaatcgccctgctgctgacccatgagacgcgacatcagtcgttgtaataagagtgaaaagcctgatgcgctacgcttatcaggcctgaatttccatacaatatattgaattcgcaaggatttgtaggccggataaggcgttcacgccgcatccggcatgaacaaagcacactttgccaacaatctaaatctgtttaattgccggatgtcagacatccggcaattatcatcacttcttcatctgcgacaaaatcgtccgacactgattagcctccccttcggaaggtgagatcagtgccagtaacgccgccgccggtgttaccagcgttgccagtgccgcagcaacagcaccacgggcaatcagcggtccggctttcaccccagcctgcggatttttaaacgtcccccgcacatacagcggcgaacgcagtgtgataatccgaattcctttactctccggatcaatagtcaaatccagctgttccgaagcaaaacttgccgtgccggtaacattaatcaacgcgttctcagtatcgaaagcaaaaatctgcgggcgcgccacgccgttggcaatattcagattcgccgccgcgcagttcacccgcacctcatcatcaccaaatatcgcaccgacaatgtagttgccgacattcagcccaacaatctccatcaggttgcggctcaccagcccgtcattcatcaacagtttcaggttgccgttactgttgcctaaaagtgccgccaccgagttaccgctaccgcgtagttccgcgtcaccgttcatttcccccagcgtcttctgcatcagttccacatcgggcatcagttctttcagtttcagtcgacgagcctgaatatctgcccgcccctgcatcggctttttatcgccttccagatgaatattcgccgcaatgctgccgcccgccatgccaaatttcagcggttgcaggcgcaggtcagcatttttgaggatgatatgagtagaaagatcgctaatcggcaggctactgccatgctcaatgcgccgccctttgaagcgaacatcggcatccataacgtcccatttatcggtttcgaagcggtcataaggcagcactttgcccgcaggctgaacgcttttttcgcccttcttctgttcagaccgtttcgacttttctgcccctttcccggaatcaacgccaatcaacggtcccaggtccgccagccgcaattgccgcgactcgacatcaccttccagttttggtcgtggctttccggtggtgtagaccagagaaccgtggatatcgctatcaccaattcgcccattaaaaccgcgataatcaaagaccgacgatttttcagtgtcgattttcgctaccagccgaccatccgtttcaaacggcggggtatcgggcagcagaacgcccgtcagttcatagagatcacccagtgaatcgccagaaaatttaagccgtaaatcgacaccgcccatcttcattgggtcattcacgacgccatcaaaagcaacacgggtgttaccagagcggaaatcagcctgtaccggaaacggcgtcccttcgccacgcagcgccagcataccgcctatttttcccgtacccgtgagcggttcaccgttatatcgtccctgcgccttcaggccaaaaacgtaatcgcccaccttttctttatccgctttacctttcgatccagtaacttcgctgaacggcagcggcttgcctaagggatcaacaaaaatctccagatccgctttgcttactttgtcatcaatggcgatccgcccttgatcgaaaagaatattatccagccgaaacgaccatgccgacggctttgcattcgcgtctttgttatcatcgttggcaagattaaacgtccagttattgttcttttcagagaggcgaatcaggcgcgcgtcgggcttttcgagcttgatccacggcagccagaccgttttggtcagcagcgccagcggggccagcgttgcctctacgcgtggcaaatgcaccatcgtgacttcgggaatatccggtggattgccaagaatgatgtcttccgcgtgtacatggggccacggcacccagctgcgccagccagtttcttgtttttgccgctcccacaccacgcccagatcgccacggatagcgaacggacgattcaactccgcagagactttctggttgatagtcggtttgagtcgattccagtcaaaagttgcaatcaaaatgatcgccacgacaatcaacaacaagaaagcccctgaaatcgcagcggttattttgcctgccttgctcatcgttcgcttcctcatattcttcctgtgccagtcctaaagatagtccagccaggcggaaaatgaggcagcttatagcgccagaaccgccgtattcagcgtttctatcggtgccgggcgtgaaagaaaccagccttgtgcggcgaatgcgggcgagttctgaacatcacgccactcttccggcgtttctacgccctcgacaatcaccccgcgacaatagcgattcattagatgtaaaagctgagaaaagagtgtgcgtccttccggcgactgacgcagcatcacaaacagttctcgcgcgattttgatgtagtcataacgcacttcacttagcgcagagaaatttgccatcccggtaccaaaatcatccagccacagcgggccaaattcacacatcgaggcaaaggttgaatctttcggcagacggatatgctccaccagttcgaaacgcagccagggaagacgctcaatctggcgcaggatttttggttgctgacgcagggcgatgagcgtagggccatcaatattgaccgatgccagcaggccgtgctctataaagaagtcggctttttgcgccagcaaatcaatctgctctttcacaacctccatccgatggctgacggtgatttcagtaaaatagcgatccggcggcaggcgttgcgaagggttcaagggatgcgtgaccaccgttaatagctccacggccattaaccgcccgcatgtttgatagatcggctgccaggtgtaagcacgctcacactgcaaccaaaaacgccgttcctgcaagctctcgatgcttgcttcagggttgcttattcgctggataacctgccttatcatcaaagatgtcctgtgtttaaaagtgatgctgcccggactcgacaaagattatcggcgcgtaagggcagaactttaccgcctggccggggtaaatttcctcactccacaacggaatctttcaggaatacgttctggctcaaaaaaataatggaacactgttttaatatggttgaccagcaaaccaccacagcgcaaactaacgctaattttttacagatcaggttcacgactatgtccaaaaagattgccgtgattggcgaatgcatgattgagctttccgagaaaggcgcggacgttaagcgcggtttcggcggcgataccctgaacacttccgtctatatcgcccgtcaggtcgatcctgcggcattaaccgttcattacgtaacggcgctgggaacggacagttttagccagcagatgctggacgcctggcacggcgagaacgttgatacttccctgacccaacggatggaaaaccgtctgccgggcctttactacattgaaaccgacagcaccggcgagcgtacgttctactactggcggaacgaagccgccgccaaattctggctggagagtgagcagtctgcggcgatttgcgaagagctggcgaatttcgattatctctacctgagcgggattagcctggcgatcttaagcccgaccagccgcgaaaagctgctttccctgctgcgcgaatgccgcgccaacggcggaaaagtgattttcgacaataactatcgtccgcgcctgtgggccagcaaagaagagacacagcaggtgtaccaacaaatgctggaatgcacggatatcgccttcctgacgctggacgacgaagacgcgctgtggggtcaacagccggtggaagacgtcattgcgcgcacccataacgcgggcgtgaaagaagtggtggtgaaacgcggggcggattcttgcctggtgtccattgctggcgaagggttagtggatgttccggcggtgaaactgccgaaagaaaaagtgatcgataccaccgcagctggcgactctttcagtgccggttatctggcggtacgtctgacaggcggcagcgcggaagacgcggcgaaacgtgggcacctgaccgcaagtaccgttattcagtatcgcggcgcgattatcccgcgtgaggcgatgccagcgtaaacgcagcatatgcaaaaggctggataaagtgttacccctctatccagctcatccataaatacctgatggttgtgctaactcatcaccatcaggcattactgtgcaggtggaatatccgtcacttcaggatgtacgtcatccgtggcgacagaggtggtcgcagcggcggtagatggggccatgatttgatcccagaccgcctgcaacgctttcatgttaaattccggctcgcctttcggctgcagcagtattaacgccatatcattcgacaactgttgacgcagatcctgatttaacatctctaccgtcaggctattaaggaaatcctgccgcagtttctgatattgctccggcgcgatatcgacaacctgattttgcaacgaacgcatccgctgacccatcagaatatcggtatcagctcgtgcataggcggcaaacagtttctgcagctccagtttcttttgcgccactaacgcattgaactcttcttccggcagacctttatcgcgaaccttcgccagttcacgcgccaccagattaaggttgctgttcagcttgtcgtttggtgattcgatgttgatggcacactgcgcacgcagatacagcacacggcagtcaaatccaagaccgatgtctttgctgttactggcacttaacgcttgctgaacatgccagaacagcgcctcgcgggccaggtccgcacgccagtagcgcagcagtgcggctgattcacgaatcggctgccacggcgtatcccacatgatagataaccggtcctgacgcaccgcgtcagtcataatactcaccgcttccgcacgcagcggagaaagcgtcggcaccggagctggcgtttcacgtttgcctttcagttcgccaaacgttttgtttatttggtcgacaaccgagcgcgcatccacgtttcccaccaccagtagcgtcattgcatccggggtgtaccatttctgatagaaatctttaattttttccgcttcaacgggttgtttcagcggatcggcaggatcgtgacctaacaaggttgaccctttcagacgatagcgccaccagccctctttagtatcggcaggccaggttgccaccatgtcctgactttgcagcgcgtggttgatggtttctggtgtgatggtcaatttgccagtggcatttgccagataagagagcgcttctttcagcaaatcgttacggttattgggcaaactcagattaaacagcgtggtgtcataagagacaattaccggcggcatcgggcgtttagggtcgatcccctgctgccacaatgaacgcgcctgtgctgcgtcaaggccaccgctttgcgttagcgcaatacgagggatggcgtgactgtaaccgctctgttgtgtactttcggcgagcgaaccggtattaaccagcaggcgaatttcaacacgatcgctgggacgctggggggtggtcagcacttgccactgtaaaccgttggaaagcgtcccctgttgccatgctggatcaggctggagcgcatctgcctgcacatagccagcagtggccatcatcagcaaaccgcccgctaaaagtcgaatttttgtgccctgcatgtgaacccctgatcaactatcctggtaataaaaaaactgcccgttgtcggtcagtctaaatgacgttaaaaacacttcgtgttagaccgcaagaacatgaaaatgtcacggaagaagtgaaataaacctgaactcacccaggtggtaagttcaggcacaggggtcaattatgcgcaaacacccgcactcggggaagggagtgcgggcataagtgatgagattaagaggataattcgtgcgttttgccatccggcgcacgattattcagcacatcgtccagttttttgtggtccagttctttcacccacttagcaacgacaatggtcgctacgccgttaccgaccaggttagtcagcgcacgagcttctgacataaagcggtcgataccgaggatcagcgccagacccgctaccggcaaatggcccaccgcagagagcgtcgccgccagcacgataaagccactacccgttacccctgccgcccctttagaagaaagcagcaacacgattaacagcgtgatttggtggacgatatccatctgactgttagtggcctgggcgataaacaccgccgccattgtcaggtatatcgatgtgccatcaaggttaaacgagtagcctgtcgggatgaccagccccaccaccgatttacggcagccgagtttctccatcttgtcgagcatacgcggcagcgccgactcggaagatgaagtccccagtacaatcagcagttcttcacggatgtagcggataaatttgaagatactgaaaccagtcgctttagcgattgaacccaataccagcaccacaaacaggatacaggtaatgtagaaacagataatcagctgccccagttgcaccagtgtgccgacgccgtatttaccgatggtaaacgccattgccccgaacgcaccaataggtgccagacgcatgatcatattgatgatgccgaagatgacctgcgagaaactttcgatgacgttaaaaatcagttggcctttgctgcccagacggtggagcgcaaaaccaaacagtacggcaaacagcagcacctgcagaatgttaccgctggcaaatgcgccaatgacgctcgccgggatgacatccataatgaaggcgacaatgccctggtctttcgcctgatcggcgtaaaccgctaccgctttcgcatcaagcgttgccggatcgacgttcattccggcaccaggctgcacgacgttaacgatgataagaccaataatcagcgcgatggtactgacaatttcaaagtaaagcagtgcgactgcgccggtacgaccgaccgccttcatgctttccatgcccgcaatgcccgttacgacggtacaaaagatgacaggagcgatgatcatcttaatgagcttaacgaagccgtcgccaagcggtttcatttgctcgcctatttcaggatagaaatggccaaggagaataccaatggctatcgctgtcaggacctgaaagtaaaggcttttaaacagagaggttttcatagggtgtcctttagtaaaaccacaggtcttgtaaggttatggggtacctgcggccttaaaataacacccagacaacatcacagaaatgtacctggatcataattgaaacaaaaaggttaaaaagtttgagctggctcgcacaaaccagcactttttaaagttttgtaatcagtttggggtagctacttttcttccaggtaactctcttcgaagatttcaatagggagtgggcgagcaaaaaggaagccctgggcaataccaacgcccgcttttgccagccagtcgcgttgtgcttcagtctccacgccttcggcaatcatttgtaagttcaggctctgcgccagcatgataattgcagcaatcatgctgctatctcccggcaagccttcaacaaacattttgtcgattttcagtacgtcgattggcaacgatttcatatgctgcagctgacgcagccctgcgtagcccatgccgaaatcatccagcgccacccgaactccggcattgcgcagcggacggaggattgccaccgcagcatgagggtcgtcaatacgtcggctttctgtcacttccagaatcagtgttcccggctgaatgcgatagcgggttaacagttccagcatatccgccaccatattcgggtgcatcagttgcagcgcagagaggtttaccgacaagggcagcataatgccgcgctcttgccaggctgcaagcaatcgacaggactcttccagcacccagtgaccgacggtaaccatcagcccacagcactcaatgcgatcgattaagccatccggcaggtcccaactgccatccggttgctggatacgcagtaacacttccgcactgaccagtttaccgctggtcatctcgacctgtggctgtaaccaaatagcaaactgatgattttccagtgcattaaggatatcgctctcttccgtcaaccgcttctgggcggcttccatctgctgcggatcaaagaactgaatctgattcttgcctttatggcgagcggtaaatgccgcagaaatagcgcgactgtaaagctgttcggcggtgagatcgccgtagaacatcgccacgccaatgctacagtgcggacggagttgaatacgttcaatcggcaggcgctcgctcatgatagtgagcacttgctgacctaaggtgattgcgtgccacggttcctgtacaccgttggcaatgacagcaaagtcataaccgctaatctgcgcgaggatcatacgtggcgacagtaccgatttgagtttttccaccagcgtcagcagcagaatttctcgttgcgcctctttcagcacgcccgcagtatcacgcagggtttcacaggtgatgatcatcagcgcggtggtttgtttacgcgcgacaacctgctccagcatctccatcagcaaggctttgttcggcaaatccgacaccgggaagcgcatcgcattttcgttctgttcttcataatggcgctgcagcaattgctggttgaggttgtaactgcgcaccaacataccgatttcatcgtcctgatgcagacgcggtaatgccagttggtgaccaacaagctccttggctgggatggcgttaagttcgcgagcaatattgcgtaacggatgcaaaatcaggcggttaatgcaccagctgatggcgacggtcaggataagcgacaaaagtaagtaaatggtcactaacgttgagagggtgctcatcacgaacttatacatacggaaggaatccgcctgtagtaccagataggcaattggctgcgggtttgccggacgttcgagcgagtaaacgcccagcgagatttgaaccggtagctcaaacaggcgagtaaccattaccggcaccgggcgctctggaataaaacttttacgcagcgcctggaactggttaggcagcactacatcggcacggctgaccacgcctgccggtttaatgctggcaagaatagcttccgcttcgggaatatcgcctttcaaaatagctgaagataagggttcgcggacagagcgagcaatgctttccagttgcgtagccgtgttatagcgattctgctggaccagatggaacagcaaaacggtgcaaaaaataaaaacgaacaccaggacaacggctgccaccattgccatctgcttgattgttaacgagcgacttacgcgcaaattgtctccccccggaaatcccagattgccgcccgagtatacccgatcgcagcggcattaagagaggcgctatctgaaaacttaccagtcggcgtaaggtatcagcggctgcggcggtaaatccatgtcaccctgccatccggcggcggaataacgtacgtagagcaggaaatggctgggtgcgtaatctttcgcctgctggatatcaattgccgtgccaacaaaccagttggaagtaacacgtcgttcaagtaatgcccgcgccgtgtagccgaagccctgactgctgccgccatcgttggattgccgcgcagcttcttcctgccagtcggtcgggatcagattcatcagcggataacgcggcatggttttggtgcgtgaatgcgaccacgagccagacgcacccagctcccacgaccagttttccgtgcgctcccgccacatcaccggtatggcaaacgacaggtattcctgcggactgtagtaaccgccctgaccgagtgagtagccactcagatctttgtcgtaatgccagatcatgttgttcaggccgattgtgacgcggcgattgttctggttaatgaccttatagtaatagcccgtcatccagcgcacgcgccagttatcttcgacatttttaccggttaactggtcgccactaagcgatgcccagacgccgtttgcttcacctttatcgtagctcagacttagccccacaccgtcggcacgtacgccaccccattttttcccggtattgctcggggagtctttttgcccaccaaaggccagcaaagaactggagatgggccgacggtgggcgttaacggtgtaacccagcggcccgatatcatcgctgtaactgatgccgccgaccacatccaccacgttgaagcccatcggcgtggtaccgatatcccagctccagacgtcatttcgccagccgaccgccacgctggcaccggaatccgactggctgcggttgccgctacagtcctgtaatgtacaggtgccccagttgtcatcccatttgccatcggcattagtggagaaactgccgacgttcatattgacgaaatcactgcgaaagaacatccgcccgtcagaatacggcgcatccacctgcaacatggtagtgtgcgctttcagatcggagtaaccaccggtgccgctcgaaccccagtaatcgtgctcaagggtgacgttaagatcctgctggcgatagaggtccgccgcatcgctgcgcacgccacgtttcagccagtcatctttctcgtcgttacgggtcagtcgggtaaaggtgtcgttatcctgcggacgcgtcgtagtcacaccggatgcgaccatggcgtctttgtaggtttccagcgcctgcgttggatcgcccgcctgcgcttcaaacttcgcaccatcacgcagcaccatcgcgctttccatcgacggtggctgagattttgcctgcgggatcaacttattaaacgtccgctgcgctgctgcggtatcgccaagctgcgcctgtgccagcgccacgcgccgctgtgtgttcagcgaggcgttatcggtagcgggcagtttcgccagctggctacgtgccgccgctttgtcaccggcagcaatatccacttccgtcagaccaagaatggcgtcggcgttagctggctcccgcgtcaggacattctgatatgcagcgcgggcggcggtgtaatcacgtcgttgttgcgcccagtcagccagcgtgaggtcaatacgcgtggaaggtggttgctggcgcagcatcgcttccgcttctgcctctttgccgctttctcgcaggcggttagcggtttccagcacctgatcgctttgcagtcgattaaccagctcctgaatattgctgttccactgcgcacgcggcaggctattgatatgcgccagcgccgctctgtcctggtcatgaccagagaggtacagcccgtaagcgtaaacctgctccgggtcgttcgacttctgctgcgccagattgcgcattaacgtatcggcctggctgcgttgtccggcctgccagagatcctgcgaaagtcggtaagtaatccatacgctgccggggtccagcgccagtcgttgccgctgaagtgctgccgcctgcgcccatttgccctggttttccagtgcctctgcctgctgtgccagacggtcgttttgcaggctgcgttcgatatcatcaatgctacgccgctgactggcagagagcgaggcgataaacgcttcagctttttctggcgattgctggcggtaaatatttgccagcccgcgcacggcgttagtgttgccgctgtccatacgcaaggtctgctgataataacgttcggcggcgggataatcttttcgcgccatcgccacatcgcccagccccagcactgcataactgtcggtgttatcgacattacgcgcctgctggaacaggcgttctgcccggtcaggattattggctttcagcgcagcatcgccctgctggatcgccagccagtagcggtttactttcagcagactgttccatttgtcgttgttgctgctgtgcgggtccagtgcgagggctttttccagattcgccactgcattggcgcgatcgcctttctgagaatacgcctggcccagcgcccccagagcttcactgtctttcgggttcgcccgcaccgcctgttgtagttcgggaatggctttacccgccataccagagtccaccgccgctaaaccttgcgcacgagcgcggaaagcaggatcggccagctgtttttgctgttctgccagttgcgattgcgcagccgccacgctatcgccatcactaaagatcgagagatattttttcagcgccgacacactggcatcactgacgggcatgtctttaatctgcccgtaccagattttagaggccccttcgcgcccggcgttcgattttgccatctgttccaggacggcaaaaccttcgtcacggcgatcgctactaaacagcaatagcgccagattgttttgcaggcccgtattgcccggtgcatccgcattgatgcgttttaactgattaatcgcttcgccacggcgagccggaattttcgccaccgtactccagtactcgacagcaatgtcaccttccggcggcgcaccgttgaacagtttgttgtaactcgccacagcttcttctgcatgaccggtcgtcgcctgcaatcgtgcctgttgcagtgcctgacgaccatccggcgtggaaagtagcatcgtagtccgcgacgatttatacgcatttgaactcggcgctaactgcgacagccgatcgagctgtttttgcgcgccatcaatatcgccctgacgtaacaaagaacggaaacgggcggcaacgacgtccgggttattcggatcaataagttccagccgatataacgactgttgcaccagatcttcacgatgggtcgcttcgcctaaccgaacttgctccagcaactgttgctgagcggttggtgctgcctcgaccatcggcatgacggccagaccgagggaaagcgtgaatatgtttagtgtgaatttgcgcattcctggccccagtcaggtaataactcaccttttgtcgagaagcggaaacggtgttgatcccagccttgtccaaacagggtcagcacatagttgtaataggcatcgctgccgggaaagttatcggccacgcgctggcgctgaacggcctgcgcatcgcggttttgtaaaaagggcagcatggcggcagaaaaaccgactggtcctttaccctgcgctttccccgtagccacatccactttttccggcggataaccgtttttctcagtgaatgtcgccatcggtttaaaccggttgagcatccgcgctttttgcggatcgctgtcaggcatcatgcctacccacatgtaaacgcggatagcgtcgtagctgctgatcaatgttttttcggcttttagctgccagcctttgtctttctcatagcgcacccagtctggcgaaaaacctttcggggcggtttccagcaataaacgttgattggtttcgcgcagcgtggtccacggcgcgccaaagcgggtgaaatactgcgccagcgtcggcggcaggtagctggggttaaaacgccagctgttatcctcagcaaaacccactttgcccggtaacaacatggaacccagcccaggcaccgtcaccacttcctcccgcgcgatacgttttagcaacgcgctgccgatgtcggtataacgctgctctttccacaaacgccccgcctccagcaacgaccaggccatccagacatcaccatcggaggccgaattgctgtccagcacttcccacttactgttctctttcttgccccacagccaggcgggcaaacgttcttttaaagaaccctgagcgagattgttctgcgtccagtcgagaatattatcgaaagctgcacggtcgttagccgccagggcagagaacatgccgtaactttgcccttcggaggtggtgattttgcgcgcgtcgctggggtcgatgacgcgcccttcctgactgatgtaatcctttttaaactgctcccaggcaggccaggtacaggctgcctgaacactaaaggcagccagcagcagcatcgtcacgattccactacgcaacacattcatcttcaattactcgttatccgggttaagacgacgacgactaataattcgcagcagacgccacagtacccatgccagcaatatcacactgatagccgccagcaccgccagcagaatcggatggtttgccagcgcataccacacgcgctcgaaccacggcagatgacctacgtaataaacgtcgccaacacgtaggctgttgataccggactcgcggatcaccgcgaccgaaccgaacatggtggcgcgtttgccgctatcgttcaccgcatcgttaagcatttcataaccgcgtgggctatctgccaacagcgcaatcacgctgcgctggtcgttatacggcgactggaagccaatcaccgccgccatcgcaccggaagaggtcagcgttgaccgggtttctgccgcgcgatcgctctcgtccggcacaatgccggggaacggggtctggcgcatcggtgttttcacccagctttcggtcgcctgcaccaataggtcgatctgcttatcgtctttcagtttgtccgggataccaccgatgatcatgatgtcggcatctttgccctgaatggtgctgccatcatcggtcaccgtcagattaatcgccgggaagcccgtctgtgcgccgataaaaccaacagtattcagcaacgtttccatctgtgcttcgttaggcgctttcggcatcacggtgatggtttgcgacagatccgccatccggctgaatgggaagcccgcgttagcaaaggcgcgtagatccggcatcgggatgaagtggtaatacttcgagaagtcgatggtggagtcgtcaccaatcaccacatgattctgcaccggctggaaggtaatacagttatccaccgaaccgcccggcatcgggttcatatactcaaagtcgaagcgcagctggttggtcgcgcccagtttcagcgccggaatagagacatctgttttgccatccagcaaaccttgtaataccggaatccgcagcagcaggcggttcgcctcctgtttgctgctcaggttgaaggattgcaggaactggttattcaggctgatatccatccgcgaactgtctttcaccggcggcatggtgtagcggtaattaatatccatatcaatgccggtactgcgcatcaggtagagatccggcggcaggtttagcgaaacgttaatcgctgctggctcaagaccgctggattgtaactgttcttcataggttttcagttcgccaaatgtgaccggacgatcggtacgtacccagttcggcgcatcgtacggcttacgcggtagcagcggtttcacttcattcactaccacgctttcaccacggaacagaatgttaccctgagcgatacctttcgctgcctgcaacaggtctttgtcgtcacgaccaaacaccaccagcagtttgacgtaaggattctgcggatggttaatcatctcaatcaccggggcttttaccgccggatgatcgcgcaggaagtccggccgtttgtcgttggttgcaaagacaatggcattgcgatccggcagttggttatagagtaccgggaagttctgcccacgccagccagaacgcgaaccaaaccacgaggcgacaatggcagaggcttgttgcagcccaacatccggcgcacccgcaaagaccatcggcaaggtgttggtgcggttatcgctcgggtcaaagaatggcaccgggaagtgtgacaggtcattcttcacattcagggtctgataggtcagatccagtccactgctccgcccaacatccagccaaagcgtggtgctggccggtttttcgcacacgtcctgataatggccgacaaactccagccgtacacggttgaagtcgctaataaacagtgggttaatgggcatttgcgccagcgtttttttacccaactgttctttggtcactggcagcacgcccatcagttcatcattgagataaacctttaactgcgactggacaggcagtaacgatggcgatggggtgtattcgaggttgagcatcgccttcgtcaccacttcatcgctgcgcataccaaactcaatgctgccgttcgggttaatgccacgtagcaccatgctgcccggcggcggtgcaatttgcgcaaaggtcagcttcacatcacgcgaaggaccgttctgcgccacgactggcgcatcagcgccctgcacgcccggcatcacttgccccacctgcggattttgttccgtctgggcggctacagctggctcagcattgatcagtggttgcgttgctggcgtcgcctgcgtcatgaaagaggggaacgcactcatccccatagccactgcacaaatccagaatagttttcttttcatcgcgttatcatcattgttgagccaaagcctgatccgatggttgtgccgtttcgctccgctccgggcggcgcggaataaacgatacaacccaggaaaccagagaagtcagcacacggaatatgcccttcaccgaagaaggcgcaaactccgccagatggcggtagccacggaagccgagcttcagaatatccagcagactttccagcggcttatcttccgggtagctgtcctgccagagcgcccatgtatccgcacgggcaaacgtacactgcacaaaatcgatatgttgctgggtggtgagcggcattaatttcagcccaacttcattacccatcacgcgcgccacctgggtcgggaagacgtattcctgctgaccgcgtttaagcaacagattcactttctgcccttccagaatctgcgcctgaccgttgatcttgatccccaaaccaccgtcggagaaatcctgaacggtacacgagaagaggtgaccatcttcgcgggcaattgccgcgggcatcgtcatctccacgcggtgcgatcggcgtacctgtttgctttctaccgataccgcaactgcgccgccaagaacaatcaggttgtagaacacccacaccatactgacgaccacggtgagcatctcggttggcgggccatagaagtagcgccagatgcctaccgcaacgcccaccaggttgagcaggacaaggaagatgtagggccgcgagatcacccagtcgacgtactcttcttccaccagtccacctttggcggtgacgttaaatttgcctttgtgcgggttaatcagcgccaccagcgtcggtggtgcgatataccacgccagcaccgtttcgtagatttcactccagaaagagtggcgatatttgccctggatcttggagttggtcaggctggcatggatcatatgcggcagcacgaatagggcgatcatcaacgctggcgcatagatgatgtaggcatgaagcagcaggaacgccagcggcgcagtcaggaagatcagccgtggaatgcccgacaagaagtggaacatggcgttgacgtaacatagccgctgagcaaacttcagccctttaccggtgagcgggttatcgagacggaagatttgtaccatcccgcgcgcccagcgaatacgctgaccgatatgcgccgacagactttcggtcgccagccccgccgcctgcggaatacgcatatacgcggaggtatagccacgacggtgcaaccgcagagaagtatgcgcatcttcagtcacggtttcgacagcaatgccgccaatttcatccagcggcttacgacgaatcaccgcacaggaaccgcagaagaaagtggcgtcccacatatcgttgccatcctgcaccagaccatagaacagcgtgccttcgttcggcgttttacggaaacgccccaggttgcgttcaaacgggtccggtgagaagaagtggtgcggcgtctgcatcatcgccagctgtttttctttcaggaaccagcccatggtcatttgcaagaacgatcgcgttggtacgtggtcgcagtcgaaaatcgacacgaactcgcctttggcatatttcagcgcattgttgatgttgcctgctttcgcatgttcatgagtggtgcgggcgatatatttcacccccacgttttgcgcaaactggcgaaactcttccctgccgccgtcatcaaggatccagatattcagcttatctttcggccagtcgatacccagcgaggcgtaaatggtatttttcaccacgttgagatcttcgttgtaagtcgggacaaagatatccaccgacggccacagcgacatatctttcggcaatggcaccggctgacgattcagcggccatactacctggaagtagccgagcaccagcacaatccacgcgtacgtttcagcgaagagcagaataagcccgcacaccaggctgaccggatcgtcccagttcagcgtagaggtgtaacgccaccagatataacggcaagaaacggtcagcgacagcacaatcaacattagcgccgagaagcgccccggcatccgccgtacgatcagcgctaccccccacagcagcatcaggaagataaactgcgccagcgggttaaacggctgagtaacgcagattaacgccagaatcagcgagaaggtgacgatgataccgaggatcaaccgccgcgccccggcactcaaatgaccgagctcttttttctcatccagatgctgtgttttatggctaacgcgctcaggcagctcgttcatccattgatggtaacgtccacgaatattttgcagacctgaaaatgcccgcctgcgcggtttcggcgtttctttgcgcgatgcaccgatcaataaccagcatgtttgaatgagataacggaccgggtccagcggacgcggacgcgaggcgttgatatgcggatacaggtttttatgttctgcgcgaatacgctgccagcgcgggtgctccagcggaataaaaatccaggccaggatcatccagaaacagccgagcgtcgcgctgaaagccgacgcaccgtgacgacgataatcgcgataacgcccgataagccgcgcgttgaccggcgggataagcaaccaccgggtcaggatactcatgatgcactcccgactggcgttttcagcccggagtagttcaacaggcaccagttcgccagcgtcagtatctcttcagccgccagcgcatcactgcgatattcacctactggttgcttagccgccaggcattcagccatcgcttcatcacgatgaatgagcatcggcagtaatcggcgctggctttgcaaccaaagctggtaaatatcgtcctgaacctgactgccaatacggaagtcattaatcaaaatatgtgcgccatccggcagcgcttgctgatgcagtcggatatggcagttggcatccacattgacgattgccagcgagtgatcgcacaaactcagcagctggtgggttatctgcgaggcatcacgcggtaagtcgattaaaatccactggtaacgcccgctggcttttagttgctgtaagccggagcaaatatcgctcagccgggtttgccagtgctgtggattttcttgttcttcaatggataactgaccaaaaggcagcaaatcgagctgcgaggtgtagcgcaacccagcgtcacgccagtcctggccatccagcatcgctctggcccagccctgacggtgggtaaaatcaacattaaatgacaggcgcaacaagttgtccgggcaggcatcgaccaccaggacattttctcccaacatttgtaatgaccaggctaatgcggcggtgatggttgttgtccccacgcctccccgcaccccctgctatcccagtacggccattcaccaatcccctacttttgttgcgcaaactctgccagcaacggccagcgttttaatgccgcggccaactgttcgcgttgggaaatatcggcataatcaatatcaggcagtgaaaatgcctgctttaacgccacaatatcattctggaagatatagcctatcgcgggatcaggcagagtatctggttcattgttattcattttgcttgatccctatgaaataaccgtaccgttcatgagacaattctaaccgtgagcatttcgccggtttattgtttacggcgagacgggaatttgctcactttttgactttccgttacgcaacagaaaaagttaaaaacgaaaagactaaaatcacacgtcttgtgaccttctaaattgattcacatgctaaatctgataagttttaatttcaatggtaggtttatttcttagctttcgctagtaaactgataatcagacaaaatggtgacatgagggacattgtggaccctgtattctctatcggtatctcatcattatgggatgagctgcgacatatgccagcaggcggcgtctggtggtttaacgtcgatcgccatgaagatgctatcagtctggcgaatcaaacaattgcatcccaggctgaaaccgcacacgtcgcggtcattagcatggacagcgatccggcgaaaatctttcaattagatgattctcaagggccggaaaaaataaaattattttcaatgctaaatcatgaaaaaggtctatactatttgacccgtgatttgcagtgttctattgatccccataattacctttttattcttgtttgcgcaaataacgcatggcaaaacattcctgccgagcggcttcgctcatggttggataaaatgaataaatggagcaggttaaaccattgttcgcttttggtaattaatcccggaaataataacgataaacaattttcattgttgcttgaggaataccgttcactttttggtcttgccagtttgcgttttcagggtgaccaacatttgctggatattgccttctggtgcaacgaaaaaggggtcagcgcccgtcagcagcttagcgttcagcaacaaaatggtatctggacattagttcaaagcgaagaggcggagatccaaccacgcagcgacgaaaaacgcattctgagtaatgttgctgtactggaaggtgcgccgccgctatcggaacactggcaactgttcaacaataacgaagtcctgttcaatgaagcccgtaccgctcaggcggcgacggtggtcttttctttacagcaaaatgcgcaaatcgagccactggcccgcagcattcataccctgcgtcgccagcgcggtagtgcgatgaaaatcctcgtgcgggaaaataccgctagcctgcgcgccaccgatgaacgtttgttattggcctgcggtgcaaatatggttattccgtggaatgcgccactctcccgttgtctgacgatgatcgaaagcgtgcaagggcagaagtttagtcgctatgtgccggaagatatcactaccttgctgtcaatgacccagccgctcaaactgcgtggtttccagaagtgggatgtgttctgtaatgccgtcaacaacatgatgaataaccctctattacctgcccacggtaaaggcgttctggttgccctacgtccggtaccgggtatccgcgttgaacaagccctgacgctgtgtcgccctaaccgtaccggcgatatcatgaccattggcggtaatcggctggtgctgtttctctcattctgtcggattaacgatctggataccgcgttgaatcatattttcccattgcctactggcgacattttctcaaaccgtatggtctggtttgaagatgatcaaatcagtgccgagctggtgcagatgcgcttgcttgccccagaacaatggggcatgccgctgcctttaacgcaaagttctaaaccggtcatcaatgccgagcacgatggtcgccactggcgacgaataccagaacccatgcgactgttagatgatgctgtggagcgctcatcatgatgaccatcagcgatatcattgaaattattgtcgtttgcgcactgatatttttcccgctgggctatctggcgcggcactctttgcgacgcattcgcgacaccttacgtttgttctttgctaaacctcgttatgttaaaccggccgggacgttacgccgcacggaaaaagccagggcaaccaaaaaatgactcaatttacgcaaaataccgccatgccttcttccctctggcaatactggcgcggcctttccggctggaacttctattttctggttaagttcggcctgttgtgggcgggatatcttaacttccatccgctcctcaatttggtgtttgccgcgtttctgctgatgccccttccgcgctacagcctgcatcgcttgcgccactggattgccctgccgatcggctttgctttgttctggcatgacacctggttgcctggcccggaaagcataatgagccagggttcgcaggtggcggggttcagtaccgattatttaatcgaccttgtcacacgctttattaactggcagatgattggggccatttttgttttattagtggcctggttattcctgtcacaatggattcgcattaccgtttttgtggttgccatactgctatggctgaacgtacttaccctggcgggaccaagtttctccttgtggccagccggacaaccgacgaccactgtaacaacgacgggtggtaacgcagcggcaaccgttgcggcgacgggtggcgcaccggtagtgggtgatatgcccgcacaaactgcaccgccaacaacggcgaaccttaacgcctggctgaataatttctataacgcggaggcgaaacgtaaatcgaccttcccgtcttcgctgcccgctgatgctcagccatttgaactactggtgattaacatctgttcgctttcctggtcggatatagaagccgccgggttgatgtcgcatccactgtggtcgcatttcgatattgagttcaagaactttaactccgccacctcctacagtggcccggcggcgatccgtttactgcgcgccagctgcgggcagacttcgcacactaatctgtatcaaccggcaaataacgactgctatctgtttgataacctttcgaaactgggctttacccagcacctgatgatgggacataacggccagttcggcggttttttgaaagaagttcgcgaaaatggcggcatgcagagcgaattgatggatcaaacaaatctgccggttattttgctgggctttgatggttcgccggtttatgacgataccgctgtgcttaaccgctggctggacgttaccgaaaaagataaaaacagccgtagtgccacgttctacaacacgcttccactgcatgacggcaaccattatccgggggtcagcaaaacagcggattacaaagcgcgggcgcagaaattctttgatgaactggacgccttctttactgaacttgagaaatcgggtcgtaaagtgatggtggtcgtggtgccggaacacggcggcgcgctgaagggcgacagaatgcaggtatctggcctacgtgatatccctagcccgtctatcaccgacgtccccgttggggtgaaattcttcggcatgaaggcaccgcatcagggggcaccgattgtcatcgaacaaccgagcagcttcctggctatctccgatctggtggttcgcgttctcgatggcaagattttcaccgaagacaatgttgactggaaaaaactcaccagtgggttgccacaaacagcaccggtctccgagaactcaaatgcagtagttattcaataccaggataaaccgtacgttcgcctgaacggcggcgactgggtgccttacccgcagtaagaacgaaaaaggccgcagagtttcccccctgcggcctggtccgggcgcaaattgccattacggcagcctgacgcccgcatgacacgttacttccgcttgttcagccagttcacgatcatactggcaagaatgccagcaatgaccggagccgctaaatcatgccagaaggccatgcccagctctgcgaacgtcatatagccgcctgtgttgtaatgacaacgtttcgcggctattcttgagtggtctagagtcaagattagcccccgtggtgttgtcaggtgcatacctgcaacgtgcgggggttttctctctccagcaaccaatgccaccagggataaagcccccgcaacattgcgcctcaccggaacctttccggcttgccgctgattctacgattgctttttactgtcagcacccggcaatcttcctcattgcgcgatgccttccagcttaatttctttatttgcaatagttgcagttcatatccgggctgactccagactggtagtgaaatgcgcaattttgtagaattgcgcctcctcgcgacctccccagtgaatctgttgcctcattttttacatactgcgtattcgacttctccacctgttgcgcaagagaaactgggtttattcatttttgcgaggccgacttctttctggacaggactttatgcagcacaacacactatcgaaacacaatcagaaattgccgtttacacgctacgacttcggctgggttttattatgcataggcatggcgattggtgccggaaccgtgctgatgccagtacaaattggcttgaagggaatttgggtatttattaccgcagcgatcattgcttatcctgccacctgggtagtgcaggacatttatttaaaaaccctttctgaaagcgattcctgtaatgactacaccgatattatcagtcattacctggggaagaactggggaattttcctcggggttatctactttttgatgattatccacgggatttttatctactctctctccgtggttttcgacagcgcctcgtacctgaaaaccttcggtttaaccgatgccgatctttcacaatctctactttataaagtcgctattttcgccgtactggtggcgattgcgtctggtggtgaacgattactgtttaagatttccgggccaatggtggtggtcaaagtagggattattgtcgtgttcggttttgcgatgatcccgcactggaatttcgccaatataaccgccttcccgcaagcctccgtctttttccgcgatgtcttgcttaccattccattttgcttcttttctgcagtatttattcaggtacttaacccaatgaatattgcctatcgtaaacgggaagcggataaagtactggcaacccggctcgcgctgcgtacccaccgaattagttatatcacgctcatcgcggtgatcctgttttttgccttttcgtttaccttctcaattagccacgaagaagccgtttctgcctttgaacaaaatatctcagcactggcgctggccgcgcaggtgatccctgggcatatcattcatatcacctctacggtgcttaatatctttgccgtactgaccgcattctttggcatttatctcggtttccacgaggccattaaaggcattattctcaatctgttaagccgaattattgataccaagaaaattaactcacgcgtgctgactctggcgatctgcgcttttatcgtcattacgttgacgatttgggtttcgtttcgtgtatcggtgctggtgttctttcagttgggaagcccgttatatggtattgtgtcgtgcctcattccgtttttcctgatctataaagtcgcacaactggaaaaacttcgcggatttaaagcctggctgattctgctgtacggcattttgctatgcttgtcgccactgttgaagctgattgagtaaaccggagcgcatggccccggttttgtgagttaacgctgcggattttcatcctgatcaacagcaaaacaagctaccagttgaccgccgtagtcttttagctgcggctgcaactgggtgcaggggccgaagcgccgacgacagcgggcgttgaaggcgcaacccggcggtggattcagtgggcttggtagttcaccgctgagcttgatgcgctcgcggcgatcgtccgggttcaggcgcggcgtcgcggaaagtagcgcctgagtgtacggatggcgcgggttattgaagatttggtctttcgttcccttctccacgcagcggcccaggtacatcaccatcacttcatcagcaatgtgctccaccaccgacaggtcgtgggagataaagacataagacagccccaactcctgctgcaaatccatcatcagattcagcacctgcgcgcgcactgaaacatccagcgcggaaaccggttcatcggcaatcaccacatccgggtcgagcatcagaccacgggcgatggcgatacgctgacgctgaccgccggagaacatatgcggatagcggtcatagtgctcggttttcaggccgactttcgccatcatcgacagggctttttcccgacgctgttctttgcttaagctggtgttgatcagcagcggctcttcaagaatttgcccgacttttttacgcggattcagcgaaccgtaagggttctggaagacgatctggattttctgccgacgcagcttctgcgcctgcggatcgtgcttaagcagatcctgcccctggtaatacagctcgccaccggtgggcatttcaatcatcgtcagcaaccgaccgagggtcgatttaccgcagccagattcgcccactactgccagcgttttgccacgttcaaggttaaacgaaacgccatccagcgctttaaccagacgttccggcgcgaacatgcctttcttcaccggataatgttttttcaggtcgatagcctgcaacagcggttgttgcagggtggcctcttgcgtactcatagtgtcggcctcccggcatcatcaagtgggtaatggcatttggactgacgcccgtcagcgagcatattcagcgccggttcttcagcgcgacatctgtcagtggcataggggcagcgcgggttaagcaggcagccgttcgggcggtcgtacttgccgggaacgacacctggcaacgacgccagacgttctttgtcctgagcaaattctggcagcgcacgcagcaatgcctgagtatacgggtgacgcggcgcatggaagatggcgtgcgcatcaccggtttccaccacctggcctgcatacatcacgatgattttatgtgccgcttccgccaccagcgccaggtcatgggtaattaacaccagcgccatgttctctttctgctgtagctccagcagtagttcgatgatttgcgcctgaatggtcacgtccagcgcggtggtcggttcatcggcaatcagcagttttggccgacaggcaatcgccatggcgatcatcacgcgctggctcatgccgccggaaagctgatgcgggtaaacatccagacgcgatgccggatcgggaataccgacctgattcagcaggtcaatcgctcgctgacggcgggtacttttgttgccgccctgatgcaccttaatcgcttccataatctggaaacccacggtgtagcacgggttaaggctggtcatcgggtcctggaagatcatcgccacttcggcacccaccaggttgcggcgctctttttctgagatacgctgcaaatcctggccgttaaactccagtttttctgccattacgcggcccggataatcaatcagccccataatcgccagtgaactgaccgacttaccggagccggactcacccacaatcccgaccacttcgccctgttttacgctgtagctgatgcggtctacggcgcggaacggcgcgctttcgtcgccgaaatgcaccgataatttatctacatttaataacgccatctcgaacctcttactgcttcagtttgggatcgagcgcgtcacgcagaccgtcacccatcaggttaaatgccagcaccgtcagcaggatcgccagacccgggaaggtcacgacccaccaggcgctttgcgcgaactgcaacacgtcggagagcatggtgccccactcaggcgttggcggctgtgcccccatgccgaggaaaccaagagcagccatatcgagaatggcgttagagaaaccgagcgacgcctgaacaatcagcggcgcaaggcagttcgggaagatgttaataaacatctgacgcatcgccccggcacccgccacgcgagacgcggtgacgtaatcgcggttaacttccaccagcacggcggcgcgggttaagcgcacatagtgcggcaaggcaacgaaggtcagtgccagcgcggcgttaccaatcgacgggccgaaaattgccaccagcaccagcgccagcagcagacttggcagcgccagcatgatatcgaccacgcgcataatgatgttatcgaccaggccgccaaagtaaccggcgatcaggccgagaataacgcccataatcagcgataacacaactaccagacagccaaccagcagcgacaggcgcgcaccgtacatcaggcgcgacagcacatcacggcctacgtcatcggtgcccagcaagtgcgccatgctgccgccttcctgccaggctggcggggcgagcagtgcatcgcggaactgttccgccgggttatagggtgcaatccagttggcaaagatcgcgatgaacagcacgatgacgacgtaaaccagcccgacgaccgcgcctttgttgcgtttaaaatagtgccagaactcctgtaacggggtcatcggcaccggtgcgctaatcactttattttcagtaacctgtgacatgatgtccccttacttcttatgacgaatacgcgggttcaccacgccgtacagcagatcgaccagcaagttgacgaggataatcatcgtcgccaccagcaatacgccgccctgcactaccggatagtcgcggcgttgcagtgcgtcaatcaaccagcgtcccagaccgggccacgagaagatggtttcggtcagaatcgcccccgccagcaatgttcccacctgcaggccgataacggtcaccaccggcagcatcgcgttacgcagcgcatggacgataatcacccgcatgcgggttagccctttggcgcgcgcggtgcggatgtaatcctcgcccagcacttccagcatcgaggagcgtgtcatacgcacaatgaccgccagcggaatagtacccagcacaatggcaggcaagatcatatgggcgacggcatcgataaagttgccgtcttcaccccagatggcggtgtcgattagcataaaaccggttaacggattggagtcatcgaggaacaccatatcgctcacgcgaccggagacgggcgtcaggttccagtgcaccgaaaccagcatgatcagcatcatgccccaccagaagataggcattgaataacctgtcagcgccaggccaaccgctgtgtgatcgaaaatggaaccgcgtttaaccgcagccagcacgccgaccggaataccgactgccgtagcaaaaatcatcgcgcagacgccaagttccagcgtggcctggaagcgcggcacgaactcttcccaaaccgggatgcggcttttcattgaaatgcctagatcgccatgcataacgccccaaatgtaatggagatactgctgccacatcggtttatctaagccgagttcagccagcagctgcgcgtgacgctctggggagatcccacgttcgcccgccatgatcatcaccggatcgcccgggatcatgtggacaaaggcaaatgtgagaagggtaataccgataaacgtggggatgacgagtcccaaacgtcggagaataaactgcaacataacccggattctctatagtgacccgcagcctggaactgcgtgtctgtattgctcacaaatcaattcccgcccttatcggacagggaatgaagtattgctgccggatggcgctgcacgcagaggcacagcgccaccgggtatacagattgttgacaaagtgcgctttgtttatgccggatgcggcgttaacgccttatccggcctacaaaatcgtgcaaattcaatacattgcagaattttcgtaggcctgataagcggagcgcatcaggcatttttgcctttgccatcagtcttgtatggcttttaattattcgatagagacgttttcgaagtgatgtttgcctaatggatcaaccacatagcctttaacttctttacgtaccggttcaaacacggtggagtgagcgatgatcagtgccggagcctgatcgtgcatcaccacctgcgcttgtttgtacagttcaacgcgtttattgtggtcgtcggtagcacgcgccggttgaatcagatcttcaaacggtttgtagcaccattttgagtagttggagccttgttcagaggcggcgcagctgaacagggtggcgaagaagttatccggatccccgttatcgccagtccagcccatcattaccgtctggtgctcgccatctttcgcacgcttgaggtactcaccccattcgtaggtgacaattttggcctgcacgccgactttcgcccagtctgcctgaatcatctccgccatgcggcgagcgttcgggttatacggacgttgtaccggcatcgcccacaggtcgatggagaaacctttttccagacccgcttctttcagcaaggctttcgctttttcaggatcgtaggtgtagtcctgaacgtcgtcgttatagccccacatggttggcgggatcaggtttttcgctgatacgcccgcgccctgataaaccgctttgatgatcgcgtctttgttcaccgcgtaggtcagagcctggcgaactttcacgtcatcgagtggttttttctgcacgttatacgagagataaccgacgttcagccccggcatttccatcagattgatggatttatcctgcttcatgcgagcgatatctgccgggttcgggtacggcatcacctggcattcattcttctgcaatttcgcgtaacgcacggaagcgtcaggggtaatagagaaaaccagcgtatcgatctgcggtttggtgccccagtagccatcaaacgctttgtagcggatacgggaatctttttgatactgctgtaactggaacggaccggttccgattgggttgaggtccagtttttccggtgtaccggctttcatcatcgcatcagcatattcttttgacagaatagaggcgaagtccattgccaggtcagcgaggaacggcgcttccgggcgagtcagcacaaactgaacggtgttgtcgtccacctttttcacttcactgatcagctctggcaagcccatgccttcgaagtattcgtagctgccgccagaaactttatggtacgggttttgcgcgtttttctgacgatcgaacgagaacaccacatcatcggcgttcagttcacgcgtcggtttgaattctttattgtcgtgccacttcacacctttacgcagatggaaggtataggttttaccgtcttcgctgacttcccacttttcagcgaggcccgggatcacttcggtggtgccgattttaaattcaaccagacggttataaagcgggacggaagaggcgtcataggtggtgccggaggtaaacagctgcgggttaaacccttccggagatccttctgagcaataaaccagagttttagcctgaacacttgctgcgacggtcatagccaccaggctgagaccaagcttcagcatccctgactttttcaaggaaatacgcattattctgctccaattgtgatgtttgttgttttaaccctttgcagtgggttgtcgctgcctgaccttttttgttttttgcccggtcgggtcaacgttatgaggtggggatgccgtactaattaacatcagtgtaacagtgcggatcctccataaaatgcccctcgtgacctacaatctgtcaacagaatgtgaaaacgtcaatacagccaaccgggatttacaccaacggtgagaatccacacacaaagattaaaaaaacttcaaacagctatttgcagcagagaaatttgtgctactccaacatgaccagaacaatcagcttaatatttagcaacatttggtgattaagttttatgcatttaatgaaaaaaatctgaggaaaaggtggatatctgagcgattaataccatgaacgctaaaacgcacagcggaaaatgccagggccagccataagtaacgcaaaaaaagatttaagcaaatataaaaaaagacaatggtttctgtcacaaatccgttaatggatagtgagatatggggcgcaaatttggcagggaaatgtgtgtcgtgtaggtcgaataaggcggtcgcgccgcatccgacaatggccggcacatttgcctgatgcgacgctgacgcgtcttatcaggcctacgtcgagtcgaacctccctgcccccggaggttctcatcctcatgagctgcagatgcaaaaaagcctgctcgttgagcaggcttttcgaatttggtcggtgatagaggattactcgccacttcgtggctcgccctgcgggccgttgctggcgcaacgttctctcgcttcgctcgagtcgaacctccctgcccccggaggttctcatcctcatgagctgcagatgcaaaaaagcctgctcgttgagcaggcttttcgaatttggtcggtgatagaggattcgaacctccgaccccttcgtcccgaacgaagtgcgctaccaggctgcgccaatcaccgaatgcggggcgcatcttactgcgcagatacgccctcgtcaatcccttaatagcaaaatgccttttgatcggcgagaaagtcagcaggccgcttagttagccgctgcctcttttgcctgcgggatgtgacaccagttgttgttttcgttaattccaccatccggtgaagtatagccaagacaacccatgatggtatcgtacagctctacgtgacggcgtggcactttcatgtcggcttcttttttcagctgcgcaaacgcctgcgcattggccggattttccagatatttatctgacatccagaccatcatcggtacgcggaactgctccggcggtgccagttcacgcggcgtgccgtgcaggtgctcgcgttcattaattgactcaccgtggtcagctgcgtagaacacaatcgctttcttatcgcgaacctgatcaatcacgctggagataaagtgatccacataggtcaccgagttgtcataggagttgatcatctgcgctttggtacagccgctatcaacaccaatacattccggcttccactgcgcgaagctacgcggataacgctgggtgtagttaaaatgcgaacctttggtatgcagaatgatcagatgcttaccatccgggttgcgccctagcgattgctgcatttcgtctaccagcaacatatcatctaccggcttgccacgattacgtggctccgcaccaatctgctcacgataagcaatgttgtccgccatcgtgttgctgtagaaccacatttcgctctgcatagcgtagaggtcagaactgaatcctaactgcttcagaaccgcgaaaatgttctgttcttttaatgtgcgctgcggattatcttccgcgcccccctgacgtacaaacatgcaacgcagtgagagtttggttgcggtatcacaggagtaaccacggaacgccgccagatttttctcctgggccagtttcggcgtggtattacgctcatagccgaaaatacccatatggtcccaacgcgtggtttcaccgatgataaacacgacataagtgtcatcaacgttttgcggtgcctgataagtgaatttcttcgccggattaagcaatgaattattatcggaagattcatcgacccgcgcccaggcatacagccccaacgcagaaagccagtttgatggcagataagagttcgctacgacaccgccataactcggcaaatcaacgccggtcgccctctccactttcttctgctggatatccagcaaacgaatcggtgcccaaaccataatacccgccagtacgacgaccgccaggctgcgaatacgctgccctggggttcgcagttgtcggagcaaggtgtagcgacagcggttattccagataaggataagaggcaatgcactaacggcgattaaccagagaataaagttcagaccaacaacttcttttgacaggtcgatatcggtggtcatgacggaagcgatgatgccataaccaatgaccacattaaggaaggtcatgtaatagctggcacctgcggaaaagagcaccaccagcgatgccagaatacgccagctgcggcggccaaacagcgaaagaagacgtagtaaaaagaaggtcaccagtacggtggcggccagttcaacaacagcagaaatgcctttccagacggtaaaatcgtgcgcatagctgccgaagcggcggtaaaaaaccgcgccattcataaaaaggccaatatagattgcaagcaaaaagctcagcttctgctgtgtaatcgatttgatgtatctcatgcaaacaaaccctggacaaacaggtgataacaccctgcttagtggcttttcaggcccggcagggaaaaagtgcggaggtagtcagataagtaaaatctacacgcgcgaataagtagaccacagcaaagggaaaaagtgtggggaaagagtgtgcatgaagcacaaatttacaaaaatgcaagtttgaaaagagactttagcgttacaaaaagcagtaaaaagggccagttaattggcccaaattttacgagtcattgtttatacatttcgttgatgcgtttgatgcacacggaagctgaagcccagtagctcgcggctgagcattaaagggagccatgcgcctcacgcaacattttctgctctggctgacgaatcgtcgtagaaagcgccaatgacagaatcagcagggcgaaaatcacgtagaaggtcacatagaagccgccaaacagtgaggcgataatcgaaccacaaatgctaccgataccgaaaccgagataaatcacaccgtagtttttcgccaggttattgaggccaaagaactcactgaccagtgacggaaagacggtaatagtgccgccaaagttaaatgccacgcaggcaatcgctgcaaagaacgtcactgcattcaatggtgcaaacagcagggccgccatacccaccagcgatatcacctgaccaatggtaataacacggatacgggcgattttgtcagacagaatacccagcaccagacgacctgaaaggttggcgatggaaataacagtgactgcattggctgcggaaaccacatcaaggtgtgccagactttgggcgatatctttcgctaccccaatcacgtacaggccgctcatgcaggcggtcaggaacattaccgctaacatccagtactgcggtttacgcatcgactctgccagcgtgtaatctttctccaccacaccattgctggttttcacttcctgttttggtgcgtctttcattaacgttgcgccgaaaacaatcatcaacagcgcaatcgctccccaaatcacaaaggttttttccagaccgaccgtttccagcagctgcgtgtcgataaatttgaaacccaggctacccagaccataagaaccgatagcgaacgcggagatcagacctttacgctccgggaaccacttcacacagttagagagcgtcagcagataacccgcgccatctgccagtcccaccagcacaccggcgcttaaccacagcatcatcaggttgtcagaatgcgctgtcaggaagaagcctaatcccagcaaaatgccggaagccatggtgacgcgtttaacgccaaaacgttcctgtaatttgcccgcaacagaagacgaaattgccagccccagacttaacaagccgaaagagaaagcgacctggcttaccggcgcatccagcttggcggaaagcgcgccattaaacaggctccaggtataaaccgaccccagcgcaaactgggtaatgatagtaccgatgagtgtcagccagcgggtacgctgataatttgaaggtgtcatggcagtattcctgcagtaataaaaaggaaaaatctctgccgacaaccataacgaagtgcactttatgcctggggaaaaacggcatgaaatgccatcagaacggaatgaaatgccttagttcaggaatgaatgacgcgacaattattcaccaaatttattatttggtaagttagcacccactatcgccacaactattgttatttaatggtttcaattgtgactgttacgttaaaatctggcgctaacccccatcgtatacagatagtcgctattattagtggtattttctgcctgagttagcgcggcataggcggcaatattttgattgagcaacatatcagcgcctacggtgacatccagccagttgccgttctggtttgtcgccgtcatccggctcaggcctgattgcgccttccagatattctcgccaaattgctggttatagctgatttgcgcccagggtcggagatcgccaagccgggagtcaacacgccagcctaaggtactcacgctggcatgccataacggatcggtcagcgtggtagtactgtcgccaaactcgttatacatcgaggtggttgtgccatcgtaatgtaatgccgcgaccgggccggttgtaacctgttcatataaaggaaaattccagcccatactcatactgctggtcacatccacaggggtttcttccgccagattgacttccagtcccagcgccctttggctactttgaatacgttgcgacaaaatatcgttgtaatcaggttgatgatcactatcccaggtgtaacgctctgtggaaagtccgggttgcgtatcaacgatatattcttgttgccaggcgtaagctgtgttgagaaaaaaggcactgattaccacgctcgccagcaggcttagctgccagcgaccaccgcttttttttatgatcattaacacgactccagggaagagccgaattcggcaatattattgtcattgtatgaaggatatcgggcatagtagccctgtattaaatattgactttttcaccgatgcgtcaagaaaagcggctgaaatttttacgatcgggtacatagcgagggaaagtatggaacgttgcggctgggtgagtcaggacccgctttatattgcctaccatgataatgagtggggcgtgcctgaaactgacagtaaaaaactgttcgaaatgatctgccttgaagggcagcaggctggattatcgtggatcaccgtcctcaaaaaacgcgaaaactatcgcgcctgctttcatcagttcgatccggtgaaggtcgcagcaatgcaggaagaggatgtcgaaagactggtacaggacgccgggattatccgccatcgagggaaaattcaggcaattattggtaatgcgcgggcgtacctgcaaatggaacagaacggcgaaccgtttgtcgactttgtctggtcgtttgtaaatcatcagccacaggtgacacaagccacaacgttgagcgaaattcccacatctacgtccgcctccgacgccctatctaaggcactgaaaaaacgtggttttaagtttgtcggcaccacaatctgttactcctttatgcaggcatgtgggctggtgaatgatcatgtggttggctgctgttgctatccgggaaataaaccatgattcgggaagcgcaacgttcagaactccccgcgatcctcgaactgtggctggaaagtacaacctgggggcatccctttataaaagcgaattactggcgtgactgcattccgctggtgcgggatgcctatcttgccaacgcgcaaaactgggtctgggaagaagacggtaagcttctcggttttgtcagcattatggaaggccgatttctggcagcgatgtttgtcgcaccgaaggccgtcaggcgcggtattggtaaggcgctgatgcagtatgtgcagcagcgccatccccacctgatgctggaggtttatcaaaaaaatcaaccggcgataaatttttaccaggcacagggttttcacattgtcgattgcgcatggcaggatgaaacccaactacccacatggattatgagctggccggtggttcaaacgctgtaagtgtcagttccggaccgttgtatttttccagccatgccagcgccgtattacccgcacagccattccccagccgcgagctggggagatctttggtcagcacgttcactgcgccgtttttacaaataccgtcagcggttaaatccagatccggccatgccccttcgtgaatgcaaatcacgccaggtttaattccctcgctaatgaccgctccggcaagaatttgcccgcgtgcgttccacaaccgaacagtatcgccatcttgtatgccgcgctcctgggcatcgtcaggatgaatggtgacaggctcacgatttgccaccgcgtacaattcgcgcagagaactgtaattcagctggctgtgcaggcggtgcgccggatgggcagaaagtacctgcaactgttctggttcggcattgccctgccattcgtccggctccagccacattggatgcccagggcaatccgggtaaccgtaatcggcaatacgctgtgagaagatttcaatcttgccgctggcggtttttaacggatgcgccagcggatcgcggcaaaaatcagcgaagcgaataaaccgctcgctgtccgggttttccggcatctcaattaactggttggcttgccagaactcagcaaatggcggcaattcaacctgctggcttgccccgcgctgtcgggcaacgttataaaacgtttccagccattgcagctcactttttccttccgtaaaacgtgcataaccgcccttctcccagcgttcacttaactcggcaaaaacatcaaaatcattacgcgcttcatagcgtggcggcaccacttgcttcatcggcaccagatgctgattactgtaatcaccggtcatggtgagatcattacgctcaaaagaggtagtcgcaggcagaacgatatccgcgtgttttgccgccgccgtccagaagcattcagagatcaccaccagctccggtttttgccaggcacggatcaggcgattggtatcctgatgatgagtaaagttggcaccgcccgcccaccagataaaacgaatatccgggaaatgtcggttcataccgttgtgttgatatgcgccaccagggttttccagtgcttcaacaatgcgggcaacagggattttatccaccgcatcgcagccacccggcaagctgccctgcatggaagagagcaccgcagaacgccgcgtggggttaccaccattggcaaaatggtaagaaagaccaaaaccgccgccgggtgtgccgatttgccccaacattgctgccagcgtgacgatcatccagtgtttttgctcaccaaactgttggcgctgcattccccagcctgccatcagcatggtggtattttggtggaaaatagccgccagctcgcggattttcgctgcgccaacaccacaaatctctgctgcccattcggcggttttcgctattccgtcactctcgcccagcaaataagaggcgaagacggcataacctgtggtgcaacgcgccagaaacgcttcgtcgtgccaaccattttccaccagcgtatgggcgatccccagcatcagcgcaacatcggtgcccatgtgcggtgccacccactccattttatcgccaaagaaatcgacggtttccgatcgcattggatcaatgcagatcagctttttcccgctgtcacgcagtgcagaaaagtaagaaagcccctgctcatcggatgcattccacgcaattttcagcgtattgagtgggttagcactccacagcaccacgacatcgctatgttccagcaccagcggccaactggtctgctgttgataaacttcactaccacccacgacatacggcatgatcgcctgtgccgcgccggtcgaataatcccccagatgcccggtataaccgcctgccagcgccatatagcgttgtaataatgtcgaggccttatgcagcacgccgtttgaacgccagccgtaggaaccagcaaaaatcgatgccggaccataagcctcacgaatgcgtttatgttgttggtgaataagatccagcgcctcatcccaactcacgcgaacaaattcatcctgcccacgaatgccttgcgggttttccggtgacgcaagaaagccttttcgcaccattggaaatcgtacccgcgtattgctgtgaacctggtcgcgaaccgcgctctgcaaggagttttccattcctgtggctaacgcgccacgcgagctaaacacggtttcgccgtcggtttcaaccagcatgggcccccaatgggcggcagtcagaacggaatatcgtgaggatgagttggccaaaccgaagactcctgaaaggttagatgtattgagcagttaaatattacttacaaatttccgagtattcccaggaataatcttcatgttcacgcggcataatctcccgccacggaacccgtggcaaagaataaaaaggttattaaggattaacaatgaagaaacgtgtttatcttattgccgccgtagtgagtggcgctctggcggtatctggctgcacaactaacccttacaccggcgaacgcgaagcaggtaaatctgctatcggcgcaggtctgggctctctcgtgggcgcgggtattggtgcgctctcttcttcgaagaaagatcgcggtaaaggcgcgctgattggcgcagcagcaggcgcagctctgggcggcggcgttggttattacatggatgtgcaggaagcgaagctgcgcgacaaaatgcgcggcactggtgttagcgtaacccgcagcggggataacattatcctcaatatgccgaacaatgtgaccttcgacagcagcagcgcgaccctgaaaccggcgggcgctaacaccctgaccggcgtggcaatggtactgaaagagtatccgaaaacggcggttaacgtgattggttataccgacagcacgggtggtcacgacctgaacatgcgtctctcccagcaacgtgcggattccgttgccagcgcgttgatcacccagggcgtggacgccagccgcatccgtactcagggccttggcccggctaacccaatcgccagcaacagcaccgcagaaggtaaggcgcaaaaccgccgtgtagaaattaccttaagcccgctgtaatccctttcatgccaggtgatgcagaaatcacctggcattcttcagttttccttcatcatatttcaggctaaggtgatcgccttatcagtgaatggagagaagcatgaagccgtccgttatcctctacaaagccttacctgatgatttactgcaacgcctgcaagagcatttcaccgttcaccaggtggcaaacctcagcccacaaaccgtcgaacaaaatgcagcaatttttgccgaagctgaaggtttactgggttcaaacgagaatgtaaatgccgcattgctggaaaaaatgccgaaactgcgtgccacatcaacgatctccgtcggctatgacaattttgatgtcgatgcgcttaccgcccgaaaaattctgctgatgcacacgccaaccgtattaacagaaaccgtcgccgatacgctgatggcgctggtgttgtctaccgctcgtcgggttgtggaggtagcagaacgggtaaaagcaggcgaatggaccgcgagcataggcccggactggtacggcactgacgttcaccataaaacactgggcattgtcgggatgggacggatcggcatggcgctggcacaacgtgcgcactttggcttcaacatgcccatcctctataacgcgcgccgccaccataaagaagcagaagaacgcttcaacgcccgctactgcgatttggatactctgttacaagagtcagatttcgtttgcctgatcctgccgttaactgatgagacgcatcatctgtttggcgcagaacaattcgccaaaatgaaatcctccgccattttcattaatgccggacgtggcccggtggttgacgaaaatgcactgatcgcagcattgcagaaaggcgaaattcacgctgccgggctggatgtcttcgaacaagagccactgtccgtagattcgccgttgctctcaatggccaacgtcgtcgcagtaccgcatattggatctgccacccatgagacgcgttatggcatggccgcctgtgccgtggataatttgattgatgcgttacaaggaaaggttgagaagaactgtgtgaatccgcacgtcgcggactaagccgcgactgcgtagagtaaagcccgataatcgctcgggcttttactctttattgggttgcagtaactgctgtagtccaggcctgattaaacgcctgatgctgtgccggtaatggcgcaatcagtttgttatattcacttgcctgctgtgaagtcgggaactggatgccatttgcgacaaagctcacctgagtaccttgctgagcaatgtagtctccaaccatcaccagttgttgcgtgaaagtttgtgccgccggaatcaacggttgcaatgcatcagctggcgtcgttaccactttggtgaatgcctgatcaaagaccggtttcaaatcatcgctctgttttagcgcagagtgcgcagcatcggcctgcaacttcgcattttgcagttgttgcgccagcacacccagcgaaccgttcatttcacgcagcggaccgctttgcgtaacgtaatcctgcggtacgcgaattgcgttaacgctgtctacaaccgggcgcagaccggaatccatcgcctgattcacctgctgagaataaccatacagaatcgcgtaatcagagacaaaaggaccaaactgttttttctgatcggcagtcagggttggtagacgttcaccgctacgcatcactgtattctgcaggaagtcgataaacgctttacgctgatcgccttctttatcaaaacacccactcaggctaactaccattaataacgccgcaagaggcgcaaaccagcgagagcaggactttcctgtcgccattttcttactcctttcacccaaaaaaagcgcacaacgacacacgcgtgtctgacgtgacaaggatagtccaggacaggcttgcaggataccctttctacgtaatcttcctggtaaaatcatggagaaaatgaaacaaggttaatttgttgtttcattgttaaaaaatgatagtgccgttgccttttttgtagccagagatttacgccttcgcagaaggttagattttcgaaatctttacaaaacaggagtggtaagagatatatcggcatttatcagatcgttaggtggctataagtcacgctaaatgacaggctgaatcgaatcatagccagagcatgccctgacttcaccccgctgtgtctgcttttcccgactattcttaatgagcttcgatgcaattcacgatcccgcagtgtgatttgaggagttttcaatggaatataaagatccaatgcatgagctgttgagcagcctggaacagattgtttttaaagatgaaacgcagaaaattaccctgacgcacagaacaacgtcctgtaccgaaattgagcagttacgaaaagggacaggattaaaaatcgatgatttcgcccgggttttgggcgtatcagtcgccatggtaaaggaatgggaatccagacgcgtgaagccttcaagtgccgaactaaaattgatgcgtttgattcaagccaacccggcattaagtaagcagttgatggaatagacttttatccactttattgctgtttacggtcctgatgacaggaccgttttccaaccgattaatcataaatatgaaaaataattgttgcatcacccgccaatgcgtggcttaatgcacatcaacggtttgacgtacagaccattaaagcagtgtagtaaggcaagtcccttcaagagttatcgttgatacccctcgtagtgcacattcctttaacgcttcaaaatctgtaaagcacgccatatcgccgaaaggcacacttaattattaaaggtaatacactatgtccggtaaaatgactggtatcgtaaaatggttcaacgctgacaaaggcttcggcttcatcactcctgacgatggctctaaagatgtgttcgtacacttctctgctatccagaacgatggttacaaatctctggacgaaggtcagaaagtgtccttcaccatcgaaagcggcgctaaaggcccggcagctggtaacgtaaccagcctgtaatctctgcttaaaagcacagaatctaagatccctgccatttggcggggatttttttatttgttttcaggaaataaataatcgatcgcgtaataaaatctattattatttttgtgaagaataaatttgggtgcaatgagaatgcgcaacgccgtaagtaaggcgggaataatttcccgccgaagactcttactctttcaatttgcaggctaaaaacgccgccagctcataactctcctgtttaatatgcaattcacacagtgaatctcttatcatccaggtgaaaaataaaagcgtgaaacaaatcactattaaagaaagtaatctatatttctgcggcattcccagcctcctgtgttgatttccaacgagtatgtactgcacccattttgttggacgatgaaatggaatagcccctaatatgtcaaagccaaaatacccttttgaaaagcgccttgaagtcgtgaatcactacttcacaactgatgatggttacaggatcatctcggcacgttttggtgtcccccgaacccaggtcaggacatgggttgccctctatgaaaaacatggagaaaaaggtttaattcccaaacctaaaggcgttagtgctgatccagagttgcgtattaaggtcgtgaaagctgtgatcgagcagcacatgtcccttaatcaggctgctgctcactttatgcttgctggtagtggttctgtagccaggtggctgaaggtctatgaagagcgcggagaagctggtttacgcgcgctcaagattggcaccaaaagaaacattgcaatatcagttgatccagaaaaagcggcatcagcattggagctgtcaaaagaccgacgcattgaggatcttgaaaggcaagttcgatttcttgaaacgcggcttatgtatctaaaaaagctgaaagccttagctcatcccacgaaaaagtgaaagtactcaacgagctaaggcagttttatcctcttgatgagcttctcagggctgcggagataccgcgcagtacgttttattatcatctaaaggctctcagcaagcctgacaagtatgcggacgttaaaaagcgtattagtgagatttatcacgagaatagaggccgatacggataccgtagggtaacgctgtctcttcatcgagaagggaaacagattaaccataaagctgttcagcgcctgatgggaaccctctcacttaaagcagcgattaaggtcaagcgataccgctcttacagaggagaggtagggcaaaccgcccctaatgttctccaaagagatttcaaggctacgcggccaaacgagaagtgggttaccgatgttactgaatttgcagtcaatgggcgcaagctgtatttgtctccagtaatagatctcttcaacaacgaagttatttcttacagcctttcggaaagaccagtgatgaacatggttgagaatatgctcgatcaggcattcaaaaagcttaatcctcacgagcatcctgttctgcactctgaccagggatggcagtatcgtatgagaagatatcaaaatatccttaaagaacatggtattaaacaaagcatgtccagaaaaggcaattgtctggataatgctgtggtggagtgtttctttggaaccttaaagtcggagtgtttttatcttgatgagttcagtaatataagcgaactgaaggatgctgttacggaatatattgaatactacaacagcagaagaattagcctgaaattaaaaggtctgactccaattgaatatcggaatcagacctatatgcctcgtgtttaactgtccaactttttggggtcagtacaaactttgatttatagtcaggtggggcttttctctgtctgcctttcggtgaatacctgagacaaacagtctcaagcacccgtggctattctagcttaataagtttgtttcttctccttgatataatcctaaaaaaatctcataaaattaatatatgagataatctttattcagcagaagattattaaaggttgctgtattatttagcgataaaaaaagcctgccagatggcaggctatttaataacggcgttattattgcaacagcgaaatatccgcaacgcgcaggaacagttcgcgcagtttctccagcatggtcagacggttgatacgcaattctttgtcatcaaccatgaccatcactttatcgaagaaagcatcaaccggttcacgcagctcagccagttcgaccagcgcatcctggtaacgaccttccgtaaagtacggctccagcttgtcacgtagcaccacaacctgcatcgccagtttaatttcttccggctctttcagggtagaggcattcacgcggtcgctcagcacttcgtcagatttcgccagaatgttagatacacgtttgttcgccgccgccagtgcagcagctgcatccagggtacggaaatgcgataccgctttcatacgggcatcgaaatcagccggacgagtcggacgacgcgccagtaccgcctggatggtgtcaacggtataaccttcgtcctgataccaggcgcggaagcgaccgagcataaagtcgataacatcatcaactacgttggcattagtcagcttatcgccatacagacgcaccgcttcttcggtcagcgtttgcagatcaaggttgaggttcttctcaacgataattcgcagcacgccaagcgcggcacgacgcagcgcaaacgggtctttgtcgcctttcggatgctgaccgataccgaagatacccgccagggtatccatcttgtcagcaatcgccagcgcacaagctactgggttggacggcaggtcatcaccagcaaaacgcggctgatactgctcattcagcgccaccgcgacatcttccgcttcgccatcgtgacgcgcatagtgcatccccataacgccctgggtgtcggtgaactcgaagaccatgttggtcatcaggtcgcacttagacagcagacccgcacgggtagcgtggttaacgtcagcgccaatctgttcagcaatccagccagccagcgcctggatgcggtcagttttgtcgcgcagcgtccccaactgttgctggaacaacacggtttgcaggcgcggcaggttatcttcaagacgttttttacggtcggtgttgaagaagaactcggcatccgccagacgcggacgaacgactttctcgttaccggagataatctgctgcggatctttcgattcgatgttggcaacgaagataaagttcggcagcagtttgccgtcgttcgcatacaccgggaagtatttctggtcacctttcatggtgtaaaccagcgcttcagccggcaccgcgaggaatttctcttcgaattttgcggtcagaacgaccggccactccaccagcgaagccacttcttccagcaggctttcgcttaagtcagcgttaccgccaatcttacgcgctgcttcttcggcatcggctttaatcttcgccttacgttcttcgtaatcggcgatgactttcccacgctcacgcagaatttccggatactgatcggcgttatcgatggtgaattccggctcgcccataaagcggtggccgcgaatcacgcgatcggactgaatgcccagaatggttgccggaatgactttgtcgcccagcagcagggtcacggtgtgcaccggacgcacgaagtgcacgtcgcttgcgccccaacgcatcagtttcgggatcggcagtttcgccagagaagtcgcaaccatattcggcagcagtgcttcggtgctttcgcccttcacatgggcgcgatacagcagccattcgcctttatcggtagtcagacgctcagcctggtcaacggtaataccgcaaccacgcgcccaaccttctgccgctttgctcggtttgccttcagcgtcgaacgcctgggcaatcgccgggccgcgtttttcgatttcacgatccggttgcgcttccgccaggttagctactttcagcgccagacgacgcggagcagcaaaccattgaacggtgccgtgtgcgaggccagcgttatccagctccgcagtaaagttcgcagcaaaggactcagccaggctgcgcagtgcttttggtggcagctcttcagtgccgatttccaccagaaaagttttctcagacatagccgcctcttacttatctttgttgcacatcgggaagccgagggcttcacgggaagcgtagtatgcttctgccactgctttggtcagggtgcgaatgcgcagaatgtagcgctgacgctcggtgacggagatggctttacgcgcatccagcaggttgaagctgtgggcggctttcagaatacgctcgtaggctggcagcggcagcggattttccagcgccagcagctgctgcgcttctttctcgtactgctcgaagcaggtgaacaggaagtccacatccgcgtattcgaagttgtaagtggactgctccacttcgttctgatggaacacgtcgccgtaggtggttttacccagcgggccgtcgctccagaccaggtcgtaaacgctgtctacgccctgaatgtacatggccagacgttccagaccgtaggtgatctcgccggtaaccggtttacactccagaccaccaacctgctggaagtaagtgaactgcgtcacttccatgccgttcagccacacttcccagcccagtccccaggcacccagcgtcgggttttcccagttatcttccacgaaacggatgtcgtgaatagtcgggtccatgcccagctctttcagagaaccgaggtacagctcctgaatattgtccggcgatggcttaatgaccacctggaactgatagtagtgctgtaaacggttggggttttcgccgtagcgaccatcggtcgggcgacgagaaggctgaacataagcagccgccatcggttctggccccagctcgcgcagacaggtcattgggtgagaggttcccgcgccgacttccatgtccaatggttgaacaatggtgcagccctggcgagcccagtaatcctgtaaggtcaggatcaagccctggaaggtcctggtatcaaacttttgcatattatttcgtgctggatacgtgtggatttaaaggaagggatcagtatacccgctggatggaagatatacagtacgaaacgggaaaaagcagggcttaacgcatggaaagatgcaaaaaatggccatccgcgtcaaaagaacagacaaactgctctttacggaaggtataaccgcgcatttcatagcttccctggaactgttcgaaggcggtgacgtcgattttttgctcgccggtgttataacgttttgccgcctgatccttgcataacgcttccatattcaacgaacgcagaggatcaacctttacccgttgtgctttctgcacgggtgacggtatagaacaacccactagcaccataagcgccattgccggaaagaaagcgttcatcatcattaaattaccgtctggtttgcaggtgagtcttattatttatatcggtatagtggctgatatcttacgaatttccttaagcctctataagctgtagtgataaaactcagattattccagtgcgccaaccaaatgatttatcggtcagactttttttaaccagatacagagacacagatgcagcccaaaatttactggattgataacctgcgagggatagcgtgtttaatggtggtgatgattcacaccactacctggtatgtgaccaatgctcatagtgttagccccgtcacatgggatatcgccaatgttctgaattctgcctctcgtgtcagcgtgccgctatttttcatgatttccggctatctcttttttggcgaacgcagcgcccagccgcgccatttcttgcgtatcggcttatgtctgattttttatagcgcaatcgcactgctctacattgcgctgtttacctccatcaatatggagttagcgctgaaaaacctgctgcaaaagccagtgttttaccacttgtggtttttcttcgcgattgcggtgatttatctggtttcaccgctgattcaggtgaagaacgtcggcggaaaaatgttgctggtgctaatggcggtgattggcattatcgctaacccaaacacagtgccgcagaaaattgacggttttgaatggctgccaattaacttatatatcaatggcgatactttttactacattctgtatggcatgttgggccgcgctatagggatgatggacacacagcataaagcactgtcgtgggtgagcgccgcgctgtttgcgacgggggtttttattatctctcgcgggacattatatgaattgcagtggcgcggaaattttgccgatacctggtatctttactgtgggccgatggtttttatctgcgcaatcgcgctattgactctggttaaaaacacgctggatacgcgtaccattcgcggacttggcttaatctcccgccattcattgggtatatacggattccacgccttgattatccatgcgctgcgcacccggggaattgagcttaaaaattggccaatactggatattatttggatcttttgcgcgacgttggcagcgagtttgttactttctatgctggtacaacgaatcgacagaaacagattagtgagttaagtaaaagcccggtcacattggactgaccgggcttacgtgagttattcgctgtattcttcctgggtaacctgtgtttcttttggtgggtttattccggcatcacgaatatttttctgcaccgctactgcaccaaacaagcttaagaagaaagccagtccataaaaacctttttcgctgagtaataatgtcgcattccacagacctaccatcagtaatgcaacagagataataaagacagtcaggcaggtcatataataaatggaagtggtcggtatgccttcatacttgtcccgaacggtcttttgataagacgccgcagaaaacagtcctaataccagtacggcaaaataatatcctttttcatttaactgcatctctgcattccatagccctaacagataggtaacgataccaccaacgagagctatccatgacacaatactaaaggccggtgaataggttgatattttgttgtccatcacagtattcctttcattcctgaatatgtaagagctttatgttgctcatgccgagcgaaacaaacgcatttgaccaaacaagcagacaaaaaaggcgatgggatagatcaccatttcataagtattgataggtgcgtttaaaacaccgataaacaagagaccgatagtgattaacgcaactaactggcagatatgggtaaaaaaatcatccagttgcccgagtttttctgcgcgaagatatgcatagttgccaaaagttgctgtcattaacacgccaagaaaatagccttttccacttaacaatgggcatgagatccatagcccaaccagataaaccagcgccccgacaacaaataatagttttgccacagtctttgaggttttcataacgatctccatatctaccagcgatacattacgagtaaccaacgaaagacaaaactgaaaaatgccattaacaaatgattttcagaataaattcatactaaatattaattaattactgagatatatagatgtgaattatcccccacccggtcaggcaggggataacgtttacgccattaatggcagaagttgctgatagaggcgacggaacgtttctcgtcgtggctgataagcggcataacgctgcgcatctggtagatgcgactgttctaacggtagttgcggcaacaattcaatgagcgatttctctggattcgccgcgatctgcgccagccttgctgcgcccagtgctggccccacatccccccccgtacggtaatcgagctgctgaccgctgatatccgccagcatctgacgccagtactcactacgcgccccgcccccaatcaacgtaacactttgcggtttaataccgcaggcatgcacgacatccatgccatctgccagcgcataacccacgccttccagcactgctcgcgccagttcattggggccatgttgatgagtcaaaccaaagaaaacccccttcgcctggggattattgtgtggcgtacgctcgccggaaagataaggcagaaaccaaactggctcggcactttcatcagcctgttgagctgcagcgattaaagctgggacattgctcaggccggttaatttcgcggcccaatccagacacgacgctgcactcagcatcacagacattaaatgccaacgttgcggtagcgcatggcaaaagctatgtacggcgctttctggcttgcttaagaacccttcgctgacagcaaaatagacccccgacgtccccagcgataacattgcctgattagcatcaaccattcccacaccaactgcaccagctgcattgtcgccaccgcctgcgacaactggcaccgtcgccataccccacgctttcgcaacttcaggtaacaaagcaccagtaatttcgctgccttcgtataatgcgggcatctggtcacgagataagtcgcaagcctgcagcatgacgtcactccagtcacgctttgcgacatccagccacatggtgccagctgcgtcagacatatcgctggcaaactcccccgtcatacgcagacgcaagtaatctttcggtaataatactttgtcgatttgacggaatatctccggctcatgccgctgaacccatagcaatttaggcgcagtaaatccgggcatcatcaggttgccggtaatcacccgcgattgcggaactcgcgcttccagcaaagtgcactcttgcgcacagcgcccgtcgttccacaaaatggcagggcgtaacacccgttgctgagcatccagcaaggttgctccgtgcatctggccggcaatacccaatgctttaacgtcctgcagagaatgctgatcgcccagagctttcattgcgcgatcagttgcctgccaccactgttccgggtcttgttccgaccagagtggatgcgggcgcgaaacggtcagcttttccgtttgcgcagcaaccacctcaccctgctcgttgagcaaaataacttttacgcccgaggtgccaagatctatcccgatatacatatcgatcgttccttaaaaaaatgcccggtatcgctaccgataaccgggccaacggactgcacagttagccgttatttgtcgaacagataatggtttaccagattttccagttgttcctggcgaccactctgatgcaccggagacaaatgatgttcctgagcatatttggctaaatctgccagtgacatttggcctttcaggatttgctggcccaattcgctattccagccggaataacgctgcgcgatgcgtttatccagctcgccatcttcaatcatgcgcgctgcaattttcagcgccagtgccatcgtatccatcgcgccgatatgaccgtaaaacagatcatatttatcagtactttgacgacgtactttggcatcgaagttcagaccaccggtggtgaaaccgcctgctttgagaatttcatacatcaccagcgcattctcttccacactgttcgggaactggtcggtgtcccagcccagttgcgcatcgccacggttggcgtcgacagaaccgaacaggccaagcgcaatggcggtggctatttcatgatggaaagagtgacctgccagcgtcgcgtggttagcttcaatgttcagtttaatctctttttccagaccaaactgtttcaggaagccatagaccgtcgcggcatcgtaatcatattgatgtttggtcggttcttgcggtttcggttcgataagcaacgtgccctggaaaccgattttatgtttatgctcaaccaccatctgcataaagcggcccagttgttcacgctcctgacgcaagtcggtatttaacagcgtttcgtaaccttcacgaccgccccacaggacatagttttcaccgcccaatttatgggttgcttccatcgctgtaacaacttgcgttgccgcccagctgaagacttcaggatctgggttcgtcgccgcacccgcgccgtagcgagggtttgtaaagcagttggccgttccccacagcagcttcacgccgctctcttcttgcttgcctgccaggacatcaaccatttgcgcaaaattattgatgtactcttttaacgacgcgccctcaggggaaacatccacatcgtggaagcaataaaatggcacatgtaacttgtggaaaaactcaaatgcgacatctgctttacgcttcgccaacgccagtgcctcaccaggctgctgccacggacgattaaacgcccccacaccaaacatatccgccccgttccagcagaaggtgtgccagtagcaggcggcaaaacgcaagtgctcttccatacgcttacccaacaccagttcgtcgggattgtagtgacggaatgctaacgggtttgaggattttgagccttcataacgaacgcgatcgagctggtcaaaataggcttgcatattgaactccataatcaggtaatgccgcgggtgatggatgatgtcgtaatattgggcactccctttcagttgctcaattatgttatttcacactgctattgagataattcacaagtgtgcgctcgctcgcaaaataaaatggaatgatgaaactgggtaattcctcgaagagaaaaatgcaataagtacaattgcgcaacaaaagtaagatctcggtcataaatcaagaaataaaccaaaaatcgtaatcgaaagataaaaatctgtaattgttttcccctgtttagttgctaaaaattggttacgtttatcgcggtgattgttacttattaaaactgtcctctaactacagaaggccctacaccatgaaaataaagaacattctactcaccctttgcacctcactcctgcttaccaacgttgctgcacacgccaaagaagtcaaaataggtatggcgattgatgatctccgtcttgaacgctggcaaaaagatcgagatatctttgtgaaaaaggcagaatctctcggcgcgaaagtatttgtacagtctgcaaatggcaatgaagaaacacaaatgtcgcagattgaaaacatgataaaccggggtgtcgatgttcttgtcattattccgtataacggtcaggtattaagtaacgttgtaaaagaagccaaacaagaaggcattaaagtattagcttacgaccgtatgattaacgatgcggatatcgatttttatatttctttcgataacgaaaaagtcggtgaactgcaggcaaaagccctggtcgatattgttccgcaaggtaattacttcctgatgggcggctcgccggtagataacaacgccaagctgttccgcgccggacaaatgaaagtgttaaaaccttacgttgattccggaaaaattaaagtcgttggtgaccaatgggttgatggctggttaccggaaaacgcattgaaaattatggaaaacgcgctaaccgccaataataacaaaattgatgctgtagttgcctcaaacgatgccaccgcaggtggggcaattcaggcattaagcgcgcaaggtttatcagggaaagtagcaatctccggccaggatgcggatctcgcaggtattaaacgtattgctgccggtacgcaaactatgacggtgtataaacctattacgttgttggcaaatactgccgcagaaattgccgttgagttgggcaatggtcaggaaccaaaagcagataccacactgaataatggcctgaaagatgtcccctcccgcctcctgacaccgatcgatgtgaataaaaacaacatcaaagatacggtaattaaagacggattccacaaagagagcgagctgtaagcgttacgccccagcgcggagcgggggcgtgatttctctccatgccgcgtgaatgaattggcttaggtggagtcgttatgccttatctacttgaaatgaagaacattaccaaaaccttcggcagtgtgaaggcgattgataacgtctgcttgcggttgaatgctggcgaaatcgtctcactttgtggggaaaatgggtctggtaaatcaacgctgatgaaagtgctgtgtggtatttatccccatggctcctacgaaggcgaaattatttttgcgggagaagagattcaggcgagtcacatccgcgataccgaacgcaaaggtatcgccatcattcatcaggaattggccctggtgaaagaattgaccgtgctggaaaatatcttcctgggtaacgaaataacccacaatggcattatggattatgacctgatgacgctacgctgtcagaagctgctcgcacaggtcagtttatccatttcacctgatacccgcgttggcgatttagggcttgggcaacaacaactggttgaaattgccaaggcacttaataaacaggtgcgcttgttaattctcgatgaaccgacagcctcattaactgagcaggaaacgtcgattttactggatattattcgcgatctacaacagcacggtatcgcctgtatttatatttcgcacaaactcaacgaagtcaaagcgatttccgatacgatttgcgttattcgcgacggacagcacattggtacgcgtgatgctgccggaatgagtgaagacgatattatcaccatgatggtcgggcgagagttaaccgcgctttaccctaatgaaccacataccaccggagatgaaatattacgtattgaacatctgacggcatggcatccggttaatcgtcatattaaacgagttaatgatgtctcgttttccctgaaacgtggcgaaatattgggtattgccggactcgttggtgccggacgtaccgagaccattcagtgcctgtttggtgtgtggcccggacaatgggaaggaaaaatttatattgatggcaaacaggtagatattcgtaactgtcagcaagccatcgcccaggggattgcgatggtccccgaagacagaaagcgcgacggcatcgttccggtaatggcggttggtaaaaatattaccctcgccgcactcaataaatttaccggtggcattagccagcttgatgacgcggcagagcaaaaatgtattctggaatcaatccagcaactcaaagttaaaacgtcgtcccccgaccttgctattggacgtttgagcggcggcaatcagcaaaaagcgatcctcgctcgctgtctgttacttaacccgcgcattctcattcttgatgaacccaccaggggtatcgatattggcgcgaaatacgagatctacaaattaattaaccaactcgtccagcagggtattgccgttattgtcatctcttccgaattacctgaagtgctcggccttagcgatcgtgtactggtgatgcatgaagggaaactaaaagccaacctgataaatcataacctgactcaggagcaggtgatggaagccgcattgaggagcgaacatcatgtcgaaaagcaatccgtctgaagtgaaattggccgtaccgacatccggtggcttctccgggctgaaatcactgaatttgcaggtcttcgtgatgattgcagctatcatcgcaatcatgctgttctttacctggaccaccgatggtgcctacttaagcgcccgtaacgtctccaacctgttacgccagaccgcgattaccggcatcctcgcggtaggaatggtgttcgtcataatttctgctgaaatcgacctttccgtcggctcaatgatggggctgttaggtggcgtcgcggcgatttgtgacgtctggttaggctggcctttgccacttaccatcattgtgacgctggttctgggactgcttctcggtgcctggaacggatggtgggtcgcgtaccgtaaagtcccttcatttattgtcaccctcgcgggcatgttggcatttcgcggcatactcattggcatcaccaacggcacgactgtatcccccaccagcgccgcgatgtcacaaattgggcaaagctatctccccgccagtaccggcttcatcattggcgcgcttggcttaatggcttttgttggttggcaatggcgcggaagaatgcgccgtcaggctttgggtttacagtctccggcctctaccgcagtagtcggtcgccaggctttaaccgctatcatcgtattaggcgcaatctggctgttgaatgattaccgtggcgttcccactcctgttctgctgctgacgttgctgttactcggcggaatgtttatggcaacgcggacggcatttggacgacgcatttatgccatcggcggcaatctggaagcagcacgtctctccgggattaacgttgaacgcaccaaacttgccgtgttcgcgattaacggattaatggtagccatcgccggattaatccttagttctcgacttggcgctggttcaccttctgcgggaaatatcgccgaactggacgcaattgcagcatgcgtgattggcggcaccagcctggctggcggtgtgggaagcgttgccggagcagtaatgggggcatttatcatggcttcactggataacggcatgagtatgatggatgtaccgaccttctggcagtatatcgttaaaggtgcgattctgttgctggcagtatggatggactccgcaaccaaacgccgttcttgattttgataaaaattttctcaaagccggttacgtattaccggttttgagtttttgcatgattcagcaggaaaagaaccatgtttactaaacgtcaccgcatcacattactgttcaatgccaataaagcctatgaccggcaggtagtagaaggcgtaggggaatatttacaggcgtcacaatcggaatgggatattttcattgaagaagatttccgcgcccgcattgataaaatcaaggactggttaggagatggcgtcattgccgacttcgacgacaaacagatcgagcaagcgctggctgatgtcgacgtccccattgttggggttggcggctcgtatcaccttgcagaaagttacccacccgttcattacattgccaccgataactatgcgctggttgaaagcgcatttttgcatttaaaagagaaaggcgttaaccgctttgctttttatggtcttccggaatcaagcggcaaacgttgggccactgagcgcgaatatgcatttcgtcagcttgtcgccgaagaaaagtatcgcggagtggtttatcaggggttagaaaccgcgccagagaactggcaacacgcgcaaaatcggctggcagactggctacaaacgctaccaccgcaaaccgggattattgccgttactgacgcccgagcgcggcatattctgcaagtatgtgaacatctacatattcccgtaccggaaaaattatgcgtgattggcatcgataacgaagaactgacccgctatctgtcgcgtgtcgccctttcttcggtcgctcagggcgcgcggcaaatgggctatcaggcggcaaaactgttgcatcgattattagataaagaagaaatgccgctacagcgaattttggtcccaccagttcgcgtcattgaacggcgctcaacagattatcgctcgctgaccgatcccgccgttattcaggccatgcattacattcgtaatcacgcctgtaaagggattaaagtggatcaggtactggatgcggtcgggatctcgcgctccaatcttgagaagcgttttaaagaagaggtgggtgaaaccatccatgccatgattcatgccgagaagctggagaaagcgcgcagtctgctgatttcaaccaccttgtcgatcaatgagatatcgcaaatgtgcggttatccatcgctgcaatatttctactctgtttttaaaaaagcatatgacacgacgccaaaagagtatcgcgatgtaaatagcgaggtcatgttgtagcgatgatgagaattgtcggcgtcacatcaggtaacgctgcgtggttgtcggatgcggcgtgaacgccttatccgacctacccgccaggcatgataaaacgcaccaacaacgcttcaggctcgtagctcaactgcctgagacaaagtaaaaagccttatccgactgacaagtcggataaggctcaaggaaatgcaattacatatgcgccgcgattaaccgttggttatcctggtacattgcgaacaggtagttgttataactcttccctttggtcgagtagcccttcagcttgtgaatcatcgctgtggcagtcacttcctgatccgctttacgcagctgcgcacgcgatttacggaacgaagagtaagccgggtgcgtattcaggttagtgacataggcgctcaccgattctttgacagaactaaactgtgagtaccctttcactttacctggcgcattggtacaacgtcctttcatgcatttcatgccgaacaggttgttgttgttgcgcgccagcttcgacgttccccaaccgctttctgctgcagccatcgtcgccaccatactggtggggataatgtctacgcgttcaagcaaggtattccacgggatttttcgcgtattaccggaccacttcaccttgtagcgtttggcgatgtctttcagacgcgcacgctcagcaggtgaccattggccctgatactgttttgaaatgagccagttacgttccgcagtaatggccgcattttggctggtaatgtaaggcattacggtccggagaaacgcctttttccttggtgttccggaagggtattttcgcaaatcaggaagtgaactactctttgcactattgcgagaatactcttgtttactgcttacctgtttattactagctttagttaagtgggacttttgactcgctgttgttgtgtgcgtcttcgctaacacctcactcgaaaacaccagagtgagtaacataagaatcatcgccccatatcgtcgtatgggagtcaaaatcatcaggtctcctggtcggatttaatcattccaacaccttatatttttcacaaatttgagagttgaatctcaaatcatatcaaaaatagctgtcaagagcaccccaaggaatagtccaaatctgaaactatgtcacgtgttaacgattcagattggcgctaaatcgcagaaaatgtgggggttatcgcaaaattcagccgttttttgcgcgagatcgctcacccttgcttctcatcctgtggacttaccgctcagggatgagttttgtttggcttatcgctggcaaactgtctgaaatcgcagcaataaggactcatccgccatgaaactcgccgcctgttttctgacactccttcctggcttcgccgttgccgccagctggacttctccggggtttcccgcctttagcgaacaggggacaggaacatttgtcagccacgcgcagttgcccaaaggtacgcgtccactaacgctaaattttgaccaacagtgctggcagcctgcggatgcgataaaactcaatcagatgctttccctgcaaccttgtagcaacacgccgcctcaatggcgattgttcagggacggcgaatatacgctgcaaatagacacccgctccggtacgccaacattgatgatttccatccagaacgccgccgaaccggtagcaagcctggtccgtgaatgcccgaaatgggatggattaccgctcacagtggatgtcagcgccactttcccggaaggagccgccgtacgggattattacagccagcaaattgcgatagtgaagaacggtcaaataatgttacaacccgctgccaccagcaacggtttactcctgctggaacgggcagaaactgacacatccgcccctttcgactggcataacgccacggtttactttgtgctgacagatcgtttcgaaaacggcgatcccagtaatgaccagagttacggacgtcataaagacggtatggcggaaattggcacttttcacggcggcgatttacgcggcctgaccaacaaactggattacctccagcagttgggcgttaatgctttatggataagcgccccatttgagcaaattcacggctgggtcggcggcggtacaaaaggcgatttcccgcattatgcctaccacggttattacacacaggactggacgaatcttgatgccaatatgggcaacgaagccgatctacggacgctggttgatagcgcacatcagcgcggtattcgtattctctttgatgtcgtgatgaaccacaccggctatgccacgctggcggatatgcaggagtatcagtttggcgcgttatatctttctggtgacgaagtgaaaaaatcgctgggtgaacgctggagcgactggaaacctgccgccgggcaaacctggcatagctttaacgattacattaatttcagcgacaaaacaggctgggataaatggtggggaaaaaactggatcagaacggatatcggcgattacgacaatcctggattcgacgatctcactatgtcgctagcctttttgccggatatcaaaaccgaatcaactaccgcttctggtctgccggtgttctataaaaacaaaatggatacccacgccaaagccattgacggctatacgccgcgcgattacttaacccactggttaagtcagtgggtccgcgactatgggattgatggttttcgggtcgataccgccaaacatgttgagttgcccgcctggcagcaactgaaaaccgaagccagcgccgcgcttcgcgaatggaaaaaagctaaccccgacaaagcattagatgacaaacctttctggatgaccggtgaagcctggggccacggcgtgatgcaaagtgactactatcgccacggcttcgatgcgatgatcaatttcgattatcaggagcaggcggcgaaagcagtcgactgtctggcgcagatggatacgacctggcagcaaatggcggagaaattgcagggtttcaacgtgttgagctacctctcgtcgcatgatacccgcctgttccgtgaagggggcgacaaagcagcagagttattactattagcgccaggcgcggtacaaatcttttatggtgatgaatcctcgcgtccgttcggtcctacaggttctgatccgctgcaaggtacacgttcggatatgaactggcaggatgttagcggtaaatctgccgccagcgtcgcgcactggcagaaaatcagccagttccgcgcccgccatcccgcaattggcgcgggcaaacaaacgacacttttgctgaagcagggctacggctttgttcgtgagcatggcgacgataaagtgctggtcgtctgggcagggcaacagtaacttttccggcttcccgttcgtcagtacctcgggaagccgccaaccaggataaaatgtcagccctaatcagcgttgcaggataaagcaccgctcactcttcaacagaccgatttgcaccccagcaaatgtagcgttattgttaccttccttgctacagagttcgacagatatcccgctatgacattctccctttttggtgacaaatttacccgccactccggcattacgctgttgatggaagatctgaacgacggtttacgcacgcctggcgcgattatgctcggcggcggtaatccggcgcagatcccggaaatgcaggactacttccagacgctactgaccgacatgctggaaagtggcaaagcgactgatgcactgtgtaactacgacggtccacaggggaaaacggagctactcacactgcttgccggaatgctgcgcgagaagttgggttgggatatcgaaccacagaatattgcactaacaaacggcagccagagcgcgtttttctacttatttaacctgtttgccggacgccgtgccgatggtcgggtcaaaaaagtgctgttcccgcttgcaccggaatacattggctatgctgacgccggactggaagaagatctgtttgtctctgcgcgtccgaatattgaactgctgccggaaggccagtttaaataccacgtcgattttgagcatctgcatattggcgaagaaaccgggatgatttgcgtctcccggccgacgaatccaacaggcaatgtgattactgacgaagagttgctgaagcttgacgcgctggcgaatcaacacggcattccgctggtgattgataacgcttatggcgtcccgttcccgggtatcatcttcagtgaagcgcgcccgctatggaatccgaatatcgtgctgtgcatgagtctttccaagctgggtctacctggctcccgctgcggcattatcatcgccaatgaaaaaatcatcaccgccatcaccaatatgaacggcattatcagcctggcacctggcggtattggtccggcgatgatgtgtgaaatgattaagcgtaacgatctgctgcgcctgtctgaaacagtcatcaaaccgttttactaccagcgtgttcaggaaactatcgccatcattcgccgctatttaccggaaaatcgctgcctgattcataaaccggaaggagccattttcctctggctatggtttaaggatttgcccattacgaccaagcagctctatcagcgcctgaaagcacgcggcgtgctgatggtgccggggcacaacttcttcccagggctggataaaccgtggccgcatacgcatcaatgtatgcgcatgaactacgtaccagagccggagaaaattgaggcgggggtgaagattctggcggaagagatagaaagagcctgggctgaaagtcactaaaaattgcctgatgcgctacgcttatcaggcctacatgatttctgcaatatattgaatttggaagaatttgtaggccggataaggcgtttacgccgcatctggcataaacaaagcgcactgttccggcgttgagaaacgccggaaaacgtttcaaacaggctgctgccgtagccgatgccgctgcactttctcgacatccatgcactgcaacgcctttgtcgggcaggcttcaacacaggccggtcccgtctcccgatgccagcacagatcgcacttaatcgccctcgcctttttgcgcgaagaaacgacctccatcgcaccaaacgggcaagccagcatacagcttttacagccaatgcaacgtgtttgttcaacgaaaatatgcccatgttcgcggcttatcgcgtcaacagggcagacattcgcgcacggtgcatcttcacactgatgacaggctactgccgtggtccagcagtggtctttaatgacacgaatacgggaaataaactcgtctggtgacaacgcagcgcaatcctgattctcatgatgcgacactgcgcaagccacttcacaggtacggcaaccgatacatttcgtcgcatccgcaataataaaccggttcatgatcactcctttgcactaaaacagcagagtgccagagagcgcgtccctactgctttgatccaacgaaggaaatgttaaagttttggcacttgtccaaagcgttatgtgatcgcgcccaggtcatccctgacagtaaatcccagttcattagaaatagcctgcgcggtttcacgcagtggtttcaggagatttttctctcccacctgtttcagacgtgatgtcgaaagcgaaatcgacacggcgtacggcacccgcccatgaatatcaaacaccggaacagcaatacaggagacgccgagttcgttttcttctctgtccatcgccgctccgctttcacgaatgtgcgccagttcgtcgaacatcgcgggcagctcggtaatggtattgcgggttaacggctggatctcatgctgatggctttcccagtatgacttcacgtagtccgggtgaccaaacgccatgtagatcttgcccattgcggaacagtagagcggcatatgctggccaatataggcacgggttcgcagcatcccggttgtgggttccagcttataaatcaaaatagcgtgatcgtcttcgcggctggagaagttaatggtttcaccagtggcgatgttcagtgcctcaagatgcggagcggcgatatgaatgatattcagcgaagacagcgccttctgcccgacggcaataaatttggtggtcaggcgataactccctgcggcaggcgcggtggtcacatagccgcaggactgtaatccctgcaataagcgatggacggtactcttatttaaaccagccagctccgaaagatgcgccaacggacaaccgtttggatagttgctcaaaatctcaatcagcatcaacccgcgaaacagactctggcttccggctggacgctctttttcctgcgccatctcgttctctttttttcccatcacttctttccccattttgtcgcgtcctgatggtagcgcaaagtgtgccgtagttcacgatctcgacagataatttataaccaattgatttttatgtcttttgaaattcatcaatcagattgccttgttaaaaagtgatcgatatatttgaaatcaagtttcgcatattgaaattttaagccaaaaaagcgatcaaaaaaacaaggaagcctgggatgaaagtgacatttgagcagttaaaagcagcctttaatcgggtcttaatttcacgcggcgttgacagcgaaacggctgacgcctgtgcagagatgttcgcccgcaccaccgaatccggcgtttattctcacggcgttaatcgtttccctcgtttcattcaacaactggaaaacggcgatatcattcctgatgcccaacccaaacgtataaccagcctcggcgcaattgaacagtgggacgcccagcgttcgatcggtaacctgacagcgaaaaagatgatggatcgcgccattgaactggctgccgatcacggtattggtctggtggcactacgtaatgccaaccactggatgcgcggcggcagctacggctggcaggcggcggaaaaaggctatattggcatttgctggaccaactccatcgccgtaatgccgccgtggggcgcaaaagagtgtcgcataggcactaacccgctgatcgtcgccattccttccacgccgatcaccatggtcgatatgtcgatgtcgatgttctcttacggcatgttagaagttaaccgtctggcaggtcgtcagctcccggtcgatggtggctttgatgatgagggcaatttgaccaaagaacctggcgttatcgagaagaatcgccgcattttgccgatgggctactggaaaggttctggcatgtcgattgtgctggatatgatcgctactctcctttccgacggcgcatccgttgccgaagtcacccaggacaacagcgacgaatacggcatttcacaaatttttattgccattgaagtggacaagcttatcgacggtcccacccgcgatgccaagctgcaacgcatcatggattacgttactagtgccgagcgtgctgacgaaaatcaggccattcgcttacccggccatgaatttactaccctgctggccgaaaaccgccgtaacggcatcactgttgatgacagcgtgtgggccaaaatccaggcgttatgaggagataagtcatgatttttggacatatcgcgcagcccaatccgtgccgtttgcccgccgccattgaaaaggcgctcgattttctgcgcgctaccgatttcaacgccctggagccgggcgttgtcgaaatcgacggcaaaaatatttatacgcaaattatcgatttaaccacacgcgaagcggtggtaaaccgtccggaagtgcatcgtcggtatatcgatattcagtttctggcgtggggcgaagagaaaatcggcattgctattgatacgggaaataataaagtcagcgaatcactattagagcagcgcaatattattttttatcacgacagtgaacatgaatcatttatagaaatgataccgggcagctacgcaattttctttccgcaggatgttcaccgaccaggttgtattatgcaaacagcctctgagatacgaaaaattgtggttaaagtcgcattaacggcgctgaattaatcgaataatcgtctacgccagaacgcctgggtaatgttattgctctaactatattaataattcaggttgctgcacatgcgacttgaattatgacagacatagcctcaaggaatagctatgaaaaaaatactcgaagcaatactggcgattaatctcgccgtactttcctgtattgtatttataaacattattttaagatatggttttcagacaagcattttatctgttgatgaattgtcacgttatttatttgtctggttaacgtttattggcgcgattgtagcttttatggataacgcccacgttcaggtcacctttctggtggagaaactctcccccgcatggcagcgacgagtcgctctggttacccattccttaatcttatttatttgtggcgcactggcctggggcgcaacgctaaaaacaattcaggactggagcgattattcaccgatcctcggtttacccatcggcctgatgtatgccgcttgtctgcccaccagcctcgttatcgcattctttgaactgcgtcatttatatcaactcatcacgcgtagcaattctctaacgtcgccaccgcaaggagcttaatcatggctgtgctgatttttctgggctgtctgttgggtggtattgctatcggtttgcctattgcctgggcactgttgttgtgcggggcggcgttaatgttctggctggacatgtttgatgtccagatcatggcacaaacgctggtgaacggagccgatagcttctccctgctggcgattccgttctttgtgctggcgggtgaaatcatgaatgcgggcggcttgtcaaaacgcattgttgacctgccgatgaaactggtggggcataaaccaggcgggctgggctacgtcggcgtgctggcagctatgattatggcgagcctttctggttctgccgttgcggataccgccgccgttgccgctctactggtgccgatgatgcgcagcgccaactatccggtcaaccgggcggcggggctgattgcctctggcggcattatcgcgccaattattcccccttccattccgtttattatcttcggcgtttccagcggattatccatcagtaagctgtttatggcgggcattgcccctggcatgatgatgggcgcaacgctgatgcttacctggtggtggcaggccagtcgccttaatttaccccgccagcaaaaagcaacgatgcaggaaatctggcactcttttgtctccggtatctgggcgctgtttcttccagtcatcattattggcgggtttcgctccggcctgtttacccctaccgaagccggggccgttgctgctttctatgcgctgtttgtcgccacagttatttaccgtgaaatgaccttcgccacactttggcatgtactcattggcgcggcgaaaaccacctcagtggttatgtttctggtggcctcggcacaagtttccgcctggctgattaccattgctgaactgccgatgatggtttctgatttactgcaaccgttggtcgattcaccgcgtctgctgtttatcgtcattatggtggctatcctgattgtcggcatggtcatggatttaacgccgacggtattaattcttaccccggtattaatgcctttagttaaagaggcaggaatcgatccgatttatttcggtgtcatgtttatcattaactgctcaatcggcttaattacaccgcctatcggtaatgtacttaacgttatttcaggggtggcaaaactcaaattcgatgatgcagtcagaggcgttttcccttacgtcctggttttatattcattattagtcgtatttgtttttattcccgatctcatcatcctccctttgaaatggattaattaaaaggaaaatattatgaaattacgctctgtaacctacgcattattcattgctggcctggctgcattcagcacatcttctctggcggcacaatctttacgtttcggttatgaaacatcacaaaccgactcgcaacatattgcggcgaaaaaattcaatgatttattgcaggagagaaccaaaggcgagctgaaattaaaactgttcccggacagcactctcggtaacgcgcaggcgatgatcagcggcgtacgtggcggcaccatcgatatggaaatgtccggctcgaataactttgccgggttatcaccagtgatgaacttgcttgatgtccctttcctgttccgcgataccgctcacgcgcataaaacgctcgacggcaaagtcggtgatgatctgaaagcctcacttgaaggtaaaggactgaaagtactggcctactgggaaaacggctggcgcgatgtcaccaactcgcgcgcaccggttaaaacccccgccgacctgaaagggctgaaaatccgcaccaacaatagcccgatgaatatcgccgcattcaaagtctttggcgctaacccgatcccgatgccgtttgccgaagtctataccgggctggaaacccgcactatcgacgctcaggaacacccgatcaacgtcgtctggtcagcaaaatttttcgaagtgcagaagttcctttctctgacgcaccacgcctattccccgcttctggtggtgatcaacaaagcgaagtttgatggcttaagtccggagttccagcaggcgctagtttcatctgcacaagaagcgggtaactatcagcgcaaactggttgctgaagatcagcaaaaaatcatcgacggcatgaaagaagcgggcgtggaagtcatcaccgatctcgaccgcaaagcctttagcgacgcactggggaatcaggttcgcgacatgtttgttaaagatgtgccgcagggagctgatctgctgaaagccgtggatgaggtgcaataaaccatgacgcaatactggctggggttagattgtggcggtagctggctgaaagccgggctgtatgaccgcgaaggccgggaggcaggcgtgcagcgcctgccgctgtgcgcattaagcccgcagccaggctgggcagagcgcgatatggcagaactgtggcaatgctgcatggctgtcattcgcgccctgcttactcattctggtgttagcggggaacaaattgtcggtatcggcatctccgcacagggaaagggcttgtttttgctggataaaaacgacaaaccgctcgggaatgctattttgtcctcggaccgccgggcgatggaaatcgttcgtcgctggcaggaagatggcatcccggaaaaactctacccgctgacccgacaaaccttgtggaccgggcatccggtgtcgctgttacgctggctgaaagagcacgaaccagaacgctacgcgcaaattggctgcgtgatgatgacgcacgactacctgcgctggtgtttaactggcgtcaaaggctgtgaagagagcaatatttccgagtccaacctctacaacatgagtcttggggaatatgacccgtgcctcaccgactggctggggatcgctgaaatcaatcacgccctgccgcctgttgtcggatctgccgaaatctgcggggagatcaccgctcagacagccgccctgaccggtctgaaagcgggtacgcccgttgttggcggcctgtttgatgtggtttccaccgcactctgcgccgggatcgaagacgaatttaccctcaatgcggtgatggggacctgggcggtgaccagcggcataacccgcggtttacgtgacggtgaagcgcatccgtatgtctatggtcgctacgttaacgatggtgaatttatcgttcacgaagccagccctacctcttccggcaacctcgaatggtttaccgcacagtggggagaaatctcgtttgatgagatcaatcaggccgttgccagcttgccgaaggctgggggcgatctctttttcctgccgttcctgtacggcagcaacgccggactcgagatgaccagtggtttctacgggatgcaggccattcacacccgcgcgcacctgttgcaggccatctatgaaggggtggtgttcagccatatgacccacctcaaccgaatgcgcgaacgttttactgatgttcacaccctacgcgtcactggcggcccggcgcactccgatgtctggatgcaaatgctggcggacgtcagcggtctgcgtatcgagctgccgcaggtggaagaaaccggctgctttggtgcggcccttgccgcccgcgtcggcaccggggtttatcacaacttcagcgaagcccaacgtgacttgcgacacccggtgcgcaccctgctgccagatatgaccgcccatcagctttaccaaaaaaaatatcaacgttatcagcatctcattgccgcacttcagggctttcacgcccgcattaaggagcacacattatgagccgaccacttctgcaactggccctcgaccactcatcacttgaagccgcgcagcgcgacgtgacgctgttaaaagacagcgtcgatatcgtcgaagcgggcaccattctctgtttaaacgaagggcttggcgcggtgaaagccttgcgcgaacagtgcccggacaaaatcatcgttgctgactggaaggtcgccgacgctggtgaaacgctcgcgcaacaggcgtttggcgcaggcgctaactggatgaccatcatctgcgccgcgccgctcgcgacggtagaaaaaggccacgcaatggcacaacgctgcgggggtgaaattcagatagagctgttcggtaactggacgctggacgacgcccgcgactggcatcgtattggcgtgcggcaggccatttatcatcgcggtcgtgatgcacaggccagcgggcaacagtggggcgaagccgatctggcacgcatgaaggcgctttcagatatcggccttgagctttccattactggcgggattacccctgctgacctgccgctgtttaaagatatccgcgtgaaagcgtttattgccgggcgggcactggcaggcgcggcaaatccggcgcaagtggctggcgatttccatgcgcaaatcgacgctatctggggaggtgcgcgtgcgtaatcatcagttagggatttatgaaaaagcgctggcgaaagatctctcctggccggagcggctggtgctggcaaaaagctgcggttttgattttgtcgaaatgtcggtggatgaaaccgacgaacggctctcacgtcttgactggagcgccgcacaaaggacttcgctggttgccgcgatgatcgaaacaggtgttgggatcccgtcgatgtgcctgtccgcacatcgtcgctttccctttggtagccgtgacgaggcagtgcgcgaacgggcgcgggaaatcatgagtaaagcgattcgcctggcgcgcgatctcggcattcgcaccatccagctggcaggttatgacgtctattacgaagaccacgacgaaggcacccggcaacgttttgctgaagggctggcgtgggcagtcgaacaggcggcggcatcacaagtaatgctggcggtggagattatggataccgcgtttatgaactccatcagcaaatggaaaaaatgggacgagatgctcgcctcaccgtggttcaccgtctacccggacgtcggcaacctcagcgcctggggcaatgatgttcccgccgaactgaaactgggcattgaccgtatcgccgcgatccacctgaaagacacccagccagtcaccgggcaaagtcccggacagttccgcgacgtgccgtttggcgaaggctgcgtcgatttcgttggcatcttcaaaacgctgcataaactgaactatcgcggttctttcctgattgagatgtggaccgaaaaagccaaagagccggtgctggagattattcaggcgcggcgttggattgaagcgcgtatgcaggaggctggatttatatgttagagcaactgaaagccgacgtgctggcggcgaatctggcgcttcccgctcaccatctggtgacgttcacctggggcaatgtcagcgcggtagacgaaacgcggcaatggatggtaatcaaaccttccggcgtcgagtacgacgtgatgaccgccgacgatatggtggtggttgagatagccagcggtaaggtggtggaaggcagcaaaaaaccctcttccgatacaccaacgcatctggcgctctaccgtcgctatgccgaaattggcggtattgtgcatacccactcgcgccacgccaccatctggtcacaggccgggctggatctccccgcctggggcaccacccacgccgattatttttacggtgccatcccctgcacgcgacagatgaccgcagaggagattaacggcgaatatgaatatcagaccggcgaagtgatcattgaaaccttcgaagaacgtggcaggagtccggcacaaatcccggcggtgctggtgcattctcacggcccgttcgcatggggtaaaaacgccgccgatgccgtgcataacgccgtagtactcgaagaatgcgcctatatgggtctattctcgcgccagcttgcgccgcagctccctgcgatgcaaaacgaactgctggataagcactacctgcgtaagcatggggccaatgcctattacgggcagtaatccctcacgccggggcttcatcgccccggcactacgaattgatatgttccttgctgtaacgccgcttccacgctgctggcgttaaaccagtatgtttctgaaaaatctgccggaaatagccaacgtcattaaaccgtattgcatggagcaggccgacaacgtcgagtcactgcataacctgttgctgcccgccgatgcgccatttacgacatttgaaggcaagggattgttcagccataagatcctgattcagacgccaggttcccggtatgaacagagcaatccagagcaacaacctttgtggcattacgacggagcaccagccgcaccgacatccaccggtgaattaaaaacgccagctcaccccggtgacaaaggtaaaactctcattacgatcaatcatcgggctgtcggtaatctcttccggcagctcgctgtatcctgcgctcgccatcaatacgacgtgctctcctatcgggtattttgccgtcaggctgacatagggcacccaggcatcctgcgcggaataacttgccagaccgctacgacgggactcactctctgaaatgccatagtaatagtcactgaaattctcgtcataatagagaacgcccagcgcaggtgtcagcgacagacgacctatctgcattttgtggaataccgatagctcccccacccagccgttgctgttatccagaacgtccgcagctgcagaggctttcacggttccccaacgctcgtggtgataccaggcaacccccgccatagccgtactatcacgcttatcaagctgttgcatggcataatcgtcattatcggtagggtcaaattccagcggcatccaggatgcggtcaggctaagttcatttttttcactttgcgacagaataaaacctaacgtggtctgacgaacataaaaagtatcaccttcataactaatcagcggaattgccttcgtattttcattataaccgcgataaggcgattcattataagccgcaccagcaccaatggataattcagaagcagttgcgcttgccataaaaggcaacgcaaataacgccacaatattgcgattaattaacatgtccggtattccattttaaaataagataaaaaagagtcggcataataatgcttacaatttctccggtgcaagattcatatttatatagtaatatataaaattatatataattgggctgttgcgatgacaaaattacaacttaagtaccgggagttaaaaattatctcggtaatcgctgccagtgaaaatatcagccatgccgcgactgtacttggcatcgcacaggccaacgtcagcaaatatcttgctgattttgaatcaaaagtgggtttaaaagtctttgaccgaaccacccggcagctgatgctcacaccttttggcaccgcgctgttaccgtacatcaacgacatgctggacagaaacgagcaacttaataattttattgcagattataagcatgagaaacgtggtcgggtcaccatctacgccccaaccggcataattacctatttatccaaacatgtaatcgataaaattaaagatatcggtgatatcaccttatcgctaaaaacctgcaatcttgagcgtaatgccttttatgaaggcgtcgaatttcctgatgattgtgatgttttaatcagctacgctccaccaaaagatgaatcgctggttgccagttttattacccaatatgccgtaaccgcttatgccagccagcgctatcttgagaaacatcccattagccgtcctgacgaactcgaacatcactcctgtattttgatcgactcgatgatgatcgacgacgcgaatatctggcgcttcaacgtcgccgggagtaaagaggtgcgggattatcgcgtgaagggaaattacgtttgcgacaacacgcaatctgcgctggagctggcacgaaatcacctggggattgtgtttgcgccagacaaaagtgtgcagagcgacctgcaagacggcacgctggtgccctgctttcagcaaccctatgaatggtggctggatctggtggctatcttccgtaaacgggaataccagccctggcgggtccagtatgtgctggatgaaatgctgcgtgaaattcgccaccagcttgctcagtcgcagcaactgcggcctgaacaagcggcggaaagcgaagattaatgatcgagataaaggtaatgcacccagctggtcatgcgtaatagcactttgcgcatcaccgagacatggctgaaatgatcagagtaaaccgccacctgggcgtaaataccgtctggtaaagcgctcaaatcagtgtgctcatccagttcaatggtcgcgataacgccatctgaacccggcgctgtgtttaacgtctgtaaggtgccggtcgactgataagctccgccgggaacggctggactaatggctgccagcttaccgctgaataccttacctggcagagcattaaacaccacttccgcatcgtcgccaggagccagtcgcagcaaggagttctgacggaactgcgccacgatttgtcgtttctgatcgggtataaacaccatcaccggacgtagcggcagcgacgcggcataggtacccggacgaatcagtacctgggtcacataaccatcgctcggcgcacgcactatcgtctgctcaaggttatattttgcttccgcgagctgtgctttcaggctggcgatttgagaatgttcacccaacaccaggctatccagctggctctggatctgtttttgttccgccgccgatgacttcacggaggcttcctgcgccagataattttgccgcgccacatcgatatcgcgttctgaaaacgggtttactttcgcctggctgccacgtgcgtaacgctgatactctttagcgaatttatcccgcgtggcctttgcctgctgagtattcgccgccatctcatctaactctgcgcccaacgcccgctgtttatgttctgcggtaacgatatccgccatcagccgatccacccgcgcctgataacgcgtcgggtccagtcgaaatagcacctcaccttttttaatcagcgtatttttcttatccgtcacttcaatcaccacaccagtcacctgtgggacaacaggaatagaaataaccgctttttgcgctttaaaggtatacggatggttatagttcattaacagaattagaccgctgacaataaatattccacccagggccgctgtgggaatggtccatttatttacgggaattttgaagatcttaaacattgcccatgcaaaagccacataggtcaaaataatcagtaaatccataagtattactcggcagaagaggatttgatgtcggcgagctgtttctccagcccggcaatgcgctgttgcagttgcataacggatgaatcatggctttgcattccccatccccgctccgggcggtaaagcgtggcccaaatccacaaaaacggccagataacatgtaacgtaaaaagactcacccaaccagcaacatgaatggcgtcggcatgaggatgattacgttttttggcaatcaggtagggaatatcatgtaaaataatgatcccatagaagatcaccagaaatacaaaaataagcactcccagtgcaaaatagtccaggaacatatttccctcaaagaatataaaaaagaacaattaacgcatattatgaaatgccatgatgcagtgcaatttccttatttatataacgacatattgttttttatatactttcttaaatgtgctgtctggtttttcaacaggacgaggtttatcatattgaaatagtggaactattggccaaactaatgaataactccagtaaaacatccacagtacagattaagcgtattaaaccttcaattatctaccgtttattgctgattggcctcggatcaccaatggtgatttacggcctggttcgcccgctcaccatcgaaacgcgagattaaactcctgacaaaacacgccccagaaacgtacttctgttggcgtagtctgggttattgcgcacgtaggtttaaaacgtaaattgtaacaacgtgcgctttgtttatgccggatgcggcgtgtacgccttatccggcctacggtcaggttcccgtaggcatgataagacgcgtaagcgtcgcatcaggcaatgaatacccaatgcgaccagcttcttatatcagaacagccccaacggtttatccgagtagctcaccagcaggcacttggtttgctggtaatgctccagcatcatcttgtgggtttcgcgaccgatacctgattgtttgtagccaccaaacgccgcatgtgccgggtaagcgtgataacagttggtccacacgcgcccagcctgtatgccgcgccccatcttataggccagattaccgttgcggctccagacgcccgcgcccaggccatattgcgtatcgttcgccagctccagcgcttcttccatcgttttgaaggtggtcaccgccagcaccgggccaaaaatctcctcctggaacacccgcatattgttctgaccaaacagaatcgtcggttcgaggtagtagccgtctttcagttcaccttccagcagcttgcgccgcccgcctgtgagcacgtcagcgccctcttttttaccgatatcaatgtagttgaggatggtttccagttgcccgtgagaaacctgcgcgcccatttgcgtcacgctgtcgagcgggttaccgctacgaatgctttcgacacggcggatggcgcgttccataaagcgttcgtagatagattcctgcactaaagcacgactcggacaggtgcaaacttcgccctggttaaaggcaaacagtgcaaagccttccagcgctttatcgaaaaaggcatcttcttcatccatcacatcagcaaagaagatatttggcgacttaccgcccaactccagcgtcaccggaataatgttttgcgttgcgtattgcataatttgttggcccacttccgttgagccggtaaacgccactttggcgatgcgtttcgaggtcgccagatattcgccaattaccccacctgcgccattgaccacgttcaccacgcccggcggcagtaaatcaccgacaatttccattagcagcagtacagaaagcggggtaagacgtgcgggtttcagcaccacacagttgcccgccgccagcgcgggagccattttccagctcgccatcagcagcgggaagttccacgggataatctgccccaccacgcctaacggttcatggaaatgataggccacggtttcgctatcaacttcactgatcccaccttcctgcgcccgaatacacgaggcgaaatagcggaaatggtcaatcgccagcggtacatccgcagcactggtttcgcgaatgggtttgccgttatcccaggtttcagctgtcgctaacagctcgaggttttgttccattcgatcggcaatcttaaacagaatcgccgcacgatcctgcaccgaggtgtgcgcccatttatctttcactttgtgcgcagcatccagcgccagatcgatgtctcgtttgcccgaagacgccacttcgcacagcagctgcccggtcaccggcgtcagattctggtaatactcgccgtcggcaggggctacccattcgccgccaataaagttgtcatagcgggcttttaacttgagggggaaaccatactcgccgggcttaatctgtgctgaagggggattattggtcatgatcgtctccttgcggtgtgaggtataacaagggtagacgtgactggcgaaatcttcgccagtcggtaacagctttacgacagctatcacgaatttacgggcaagggttacagagatagttgaaaaagcggctaacaatttgccagccgttgtggaaatgatgattacatcgctgcgcgataaatcgccacaatttcttcgtgagttgcctggatcgggttagtaaagccacaggcatctttcagggcattagtcgccaataccgcgaaatcttcttctttcacgttcaggtcgcgtaggcctgccgggatatccactttcttcgccagttcacggatggcgttaatgcaggcttcagcaccttccgcgtcgtttttacctgtcacgttcacgcccattgcagcggcacagtcacgcagacgtgcagcggcgactttgctgttgaatacctgaacgtgcggcagcaaaacggcgttacatacaccgtgtggcaggttgtagaaaccgcccagctggtgcgccatcgcatgaacataacccagagaagcattattgaacgccataccggcgaggaactgggcataagccattgcttcacgcgctttcgcattactgccatcttcaacggctaacggcaggttttcggcaatcatggtcacggctttcagtgcacaagcgtcagtgatcggcgtggcggcaatagaaacatatgcttcgatagcgtgcgttaaggcatccatacccgttgcggcggtcagtgacttcggcataccaatcatcagagaggagtcattgacagaaagcagcggagtgacatgtttatcaacaatcgccattttgatatgacgcgcttcgtcagtgatgatgcagaaacgggtcatttcagaggccgtacccgccgtggtattgatggcgatcatcggcagctgcggttttgcagagcggtcaacgccttcgtaatcgcgaatatcgccgccattggctgccaccagcgcaataccttttgcgcagtcgtgtggagaaccaccgcctaaggagatcacgctatcgcaattattctctttaagtaatttcaaacctgcggcgacgttttccgtggtggggttaggttgggtgccatcataaataacgctaaaaatattgcgttcttccagtgctttttgcacatcgcccgccatacctaatttcgttaacatattgtcagtgacaattaaggtacgggtaaatccataatctgccatcatattcattgcatcagtcaatgaatcagcgccgatgacattcacagaaggaataaagaacgttgaagctgccataacacactcctgaaagtgtaaaaaagggcgggcagcttactgaggattttcattcgaaaatatgatcagtattattgattatcaaaattaatctaataaaaagcacattgtattcattaaacaatgtgctttttttaaattcataagaattttgtattaatttattttaaaacttaattaatcatttccttatttttccggaaataataatgcgtcgcgcaataaatgatcatttccacgacgacgcgtaaagccaatgcggtcaaaatattccagaatctgaattgccagctttcggcctacgcctaagcgatcgcggaaatccgccgcgcaggttgaaccacactcctgatcgagatcgcggatcatattggcaaactcgacaatccgatcgttacggtaataacgatctttaacgatcgcggtaattattccttgctgcgccgcctggcgtagagtcaggcgcattgcctgctcgtcggttcccgtctcttttgccaggtcacgcacccaccacggttcgtcaccaaacagtggctctgctttttgccagatggcctgctgctcttcgctgaagcccgctttgtgatctggcagatgcagccagccgtgatggctgtggatgtcgccgctttcgcgcatcttttcaatcagcaacagtaccagcgcttcatcttccattggcaacgccatacgtcgcagacgttcgcgcccagggccaggttcatcgcgatgttgctcatgataagtcgctaatgtgtcgagaattttccgctgccagcgggcggcaaccggcgcattcaacaagctataaccagcctgaatataaccaggctgttgcagcaattcgcgcatcccttcgccgttgagctggcgcgcccaggcgaaatccgcaaggttaaccgcgccgcgttccagatgaacagataacgcatcggcatcgctctgcgcccgtgcaagagacgccagccattgcagatattccggcttacgtttaccgcgacgcggcgggttaagcatcacgacgcgcgctccggccagcgtgttgcgggcagagatatcgcgcaataccaggcggtcgttatctgccagccataacggggtgtcgaagaccagttcagcaaggttatcttccagcagtgaaacgcgtcccgtgacgtggctggcggcgtggtgaatatgcagcggctgccactgggtcagcggtgtatgggtttgaagctcgacaatcacccgtgtgaacggctctggcggcacatcggcaagcagccagtcgccacggttaatctgctctttttccgcatcacccgcgatgttaagcgcgatacgctgcccggcattggcggtttctgttggctggttttgcgcatgcagcgcacgtacacgcatcggtttatttacaccagtcagccagagtgaatcgcctaccttcacttccccgcttaacgccgtaccggtgacgaccagcccggcaccttttacggtaaatgcgcggtcaatcgcgaggcggaaactatgttggctggcgtgctcgcgttccggcaactgaagcagatgctcgcgcagggcatccattccccgaccttcggttgctgcggtgataaacagttttgcctcagcaaaaccgtattcccgcagaacctcctttacctggcgttcaacctcatcaacacgcgcttcgtccacgcgatcggctttggtcagcgccactgtcagcatcgggttaccggtcagctgcaaaatcgccagatgctcacgggtctgtgccatcacgccgtcatcgcacgccaccaccaacagcgcgtgatcgataccaccaacgcccgccagcatgttggaaagaaacttttcatgaccgggaacgtcgataaaaccaggcacgcgaccatccggctgcggccagtaggcatagccgagatcgatggtcatgccgcgctttttttcttccggcagacggtcagcatttacgccagtaatcgcctgcaataaggttgttttgccgtggtcaacgtgtccggcagtcgcaataatcatttcaacaacatctccaaaaaccgttgctcatcttcaaggcagcgtaaatccagccacaatcgtccgtcataaatacgaccaatcaccggcactggcaattcacgccagcgggcggctaatgactcaaggtggctaccgcgtccatcatggggtgtaaacgttaatgccgcgctcggcaggcgatcaaccggcagcgaaccactgccaatctgcgaaagacatggcataacctgtaccgcaaactccgcgccgtaatgtgcggcaaggggggcctgtaaacgttgtgcctggatttgaatgacctctgcgctgcgggtaagcaggcgcagggtcggtaatttttcactcagagcttcagggtgtaaataaagacgcaacgtggcttccagcgccgcgagggtcattttatccgcgcgtaatgcacgcttcagcgggtggctttgcaggcgggcgatcatctcttttttaccaacaataattcctgcctgcggcccgcctaacaacttgtcgccggagaaactcaccagactgacgcccgccgcaatcaactcctgcggcattggctctttcggcaaaccgtactggctaagatcgaccagcgagccactgcctaaatcagtcactacgggaacatccagctctttgccgagcgccaccagttccgcttcatctatcgctttggtgaacccctgaatgctgtagttactggtatgtactttcatcaacagtgcggtattttcattcaccgcctgacgataatcattcgcgtgcgtgcggttggtggtccctacttcgtgtagggtgcagcctgcctgacgcataacatcgggaatacgaaacgcgccgccaatctccaccagttcgccgcgagataccaccacctcttttccgctggcagtggccgccaacatcaataacaccgccgccgcattgttattgacgatacaggcatcttccgcccccgtaatacggcacagcagctgcgccagcgcccgatcgcgatgtccgcgtccggcgtcgtccagatcatactcgagggtcactggcgaacgcatagcctgcgcaacggcttccaccgcggcttccgcctgtaaagctcgcccaaggttggtatgcagcacggttcccgtcaggttgatcaccggacgcagcgcgctctgcgcttctttcgtcaaccgggcatcgacttcttgcgcccagttttcacaccacgcaggcagcgtctggctgccacgaatcacttctcgcgcttcgtcgagcatctgacgcaacaattccaccacgcgggtgtgaccataagtatcacgcaaagaaaggaaggagctatcgcgcaataagcgatcaatagccggaagttgactatagagggaacgcgtttcggttgtcataggaaacctggctgatcaaggccctctcacacggagaagggcgtttaacataaccacggattgtaacgtgagatgggtcaggaggacatatcgcgcatcaagcctttggcggttcggtgcgagcaaaactttcgcggctaaacaggttttcgaccagtttgactaagtgtgggcggtcgacacaccaacctggcgcaacgcggcggaaattgagatatccgacggcacaggcaatggcgatagtcgccagattgaccgtatcggttttgagtgtgccatcgaccagatatccttccagcacatccagactgcggttgattttctcccgctggcgtaacaattcatcttcagactgctgcgccgctggacgcgcctgttcacgcaccgataccagcccggcatccataatgccatccgccagtgcctcaattttgcgcacccgcaacgactccagcggatcgcgcggcaacatcgccggagcgacattcattaattcaatatattcagcgatgatcggcgaatcaaaccagcattcgccctcttcggtcaccagcaccggcacttttcctaacgggttaaattgcgccacgccgttgtccgcgttatagggcagttcattaataaattcgaaagttatgcccttttctaacaacagaatagaaagtttgcgtacaaacgggctggtgtagctaccgacgagtttcatgccgagtcctttgtgcgaggaaaaatatcagtatggcctggtgatgggaaaaagggcagaaaatgttgatggtttgttacttccaaataaatcacatatttatcatggtgatataaatattttcctaattatttcactctgatggatatctcacttcaggctttcttataaatctgtagggtttcgcctgtcagcagacaaataacccgataaaacaaggatgagaaatgagcggaaaaccggcagcgcgtcagggcgacatgacgcagtatggcggtagcattgttcagggttcagccggggtgcgcattggtgcccccaccggcgtggcctgttcggtgtgccccggcggagtgacgtccggccatccggtcaatcccctgctcggtgcaaaggtccttcccggtgaaaccgacatcgccctgcccggcccgctgccgttcatcctctcccgcacctacagcagttaccggacaaaaacgcccgcgccggtggggagcctcggccccggctggaaaatgcctgcggatatccgcttacagctgcgcgataacacactgatactcagtgataacggcggcagaagcctgtattttgagcacctgtttcccggtgaggacggttacagccgcagcgagtcactgtggctggtgcgcggcggcgtggcgaaactggatgaaggtcaccggctggccgcactctggcaggcgctgccggaagaactccgcttaagtccgcatcgttatctggcgacaaacagtccgcaggggccgtggtggctgctcggttggtgtgagcgggtgccggaagcggatgaggtgctgcctgcgccgctgccgccgtaccgggtactgaccgggctggtggaccgcttcgggcgcacacagacgttccaccgcgaagccgccggtgaattcagcggcgaaatcaccggcgtgacggatggtgcctggcgtcacttccggctggtactgaccacgcaggcgcagcgggcagaagaagcccggcagcaggccatttccggcgggacggaaccgtccgcttttcctgataccctgccgggttacaccgaatatggccgggacaacggcatccgtctgtctgccgtgtggctgacgcacgacccggaatacccggagaatttacctgccgcgccgctggtgcgctatggctggacgccacgcggcgaactggcggtggtgtatgaccgtagtggcaaacaggtgcgcagctttacttacgatgataaataccggggccggatggtggcgcaccgtcacacgggccggccggaaatccgttaccgttacgacagcgacgggcgggtgacagaacagctaaacccggcaggcttaagctacacgtatcagtatgagaaagaccgcatcaccatcaccgacagcctggaccgccgtgaagtgctgcacacgcagggcgaagccgggctgaagcgggtggtgaaaaaggaacacgcggacggcagcgtcacgcagagtcagtttgacgccgtgggcaggctcagggcacagacggatgccgcaggcaggacaacagagtacagcccggatgtggtgacgggcctcatcacgcgcataaccacgccggatggcagggcatcggcgttttactataaccaccacaaccagttaacgtcagccaccgggcctgacgggctggaattgcgccgggaatatgatgaattgggccgtctgattcaggaaactgcccctgacggcgatatcacccgctaccgttatgataatccacacagtgacttaccctgcgcaacggaagatgccaccggcagccggaaaaccatgacgtggagccgttacggtcagttgctgagcttcaccgactgttccggttatgtaacccgttatgaccatgaccgcttcgggcagatgacggcggtgcaccgcgaggaagggctgagtcagtaccgcgcatacgacagccgtggacagttaattgccgtgaaagacacgcagggccatgaaacgcggtatgaatacaacatcgccggtgacctgaccgccgtcattgccccggacggcagcagaaacgggacacagtacgatgcgtggggaaaggccgtccgtaccacgcagggcgggctaacgcgcagtatggaatacgatgctgccggacgggtcatccgcctgaccagtgaaaacggcagccacaccaccttccgttacgatgtacttgaccggctgatacaggaaaccggctttgacggccgcacacagcgttatcaccacgacctgaccggcaaacttatccgcagcgaggatgagggtctggtcacccactggcactatgacgaagcagaccgcctcacgcaccgcaccgtgaagggtgaaaccgcagagcggtggcagtatgacgaacgtggctggctgacagacatcagccatatcagcgaagggcaccgggtggcggtgcattacaggtatgatgagaaaggccggctgaccggtgagcgtcagacggtgcatcacccgcagacggaagcactgctctggcagcatgagaccagacatgcgtacaacgcgcaggggctggcgaaccgctgtataccggacagcctgcccgccgtggaatggctgacctacggcagcggttacctggcaggcatgaaactcggcgacacaccgctggtggagtacacccgcgaccgcctgcaccgggaaacgctgcgcagcttcggccgttatgaactcaccaccgcttatacccctgccgggcagttacagagccagcacctgaacagcctgctgtctgaccgcgattacacctggaacgacaacggcgaactcatccgcatcagcagcccgcgccagacccggagttacagctacagcaccaccggcaggctgaccggcgttcacaccaccgcagcgaatctggatatccgcatcccgtatgccacagacccggcaggtaaccgcctgcccgacccggagctgcacccggacagcaccctcagcatgtggccggataaccgtatcgcccgtgacgcgcactatctttaccggtatgaccgtcacggcaggctgacagagaaaaccgacctcatcccggaaggggttatccgcacggatgatgagcggactcaccggtaccattacgacagtcagcaccggctggtgcactacacgcggacacaatatgaagagccgctggtcgaaagtcgctatctttacgacccgctgggccgcagggtggcaaaacgggtgtggcggcgtgaacgggacctgacgggctggatgtcgctgtcacggaaaccgcaagtgacctggtacggctgggacggcgaccggctgaccacaatacagaacgacagaacccgcatccagacgatttatcagccggggagcttcacgccactcatcagagttgaaaccgccaccggtgagctggcgaaaacgcagcgccgcagcctggcggatgcgcttcagcagtccggcggcgaagacggtggcagtgtggtgttcccgccggtgctggtgcagatgctcgaccggctggaaagtgaaatcctggctgaccgggtgagtgaggaaagccgccgctggctggcatcgtgcggcctgaccgtggagcagatgcaaaaccagatggacccggtgtacacgccggcgcgaaaaatccacctgtaccactgcgaccatcgcggcctgccgctggcccttatcagcaaggaagggacaacagaatggtgcgcagaatacgatgaatggggcaacctgctgaatgaagagaacccgcatcagctgcagcagcttatccgcctgccggggcagcagtatgatgaggagtccggcctgtattacaaccgccaccgctattatgacccgctgcaggggcggtatatcactcaggatccgattgggctgaaggggggatggaatttttatcagtatccgttgaatccagttacgaatacagatcctctggggttagaagtttttcctagaccattccccttgccaattccatggcccaaaagccctgcacagcagcaagcagatgataatgctgcaaaagcattgacaaaatggtggaacgatacagcatcacaaagaatatttgactctctaatattgaataatccgggactagcattagatataacaatgatagcttctcgtggaaatgttgcagacacagggataactgatcgtgtcaatgacataataaatgacagattctggagtgatgggaaaaaacccgacagatgtgacgtacttcaggaactaattgattgtggtgatattagtgctaaagatgcaaaaagcacacagaaagcctggaattgtcgtcactccagacagtcaaacgataaaaaaagatagcccttgtggaggttcctgcaatgtcaaatacataccagaaaagaaaggcaagtaaagagtatggtttatataatcaatgtaagaaactaaatgatgatgaattatttcgcttacttgatgatcacaattccttgaaaaggatttcatctgccagagtattacagttaagaggtgggcaagacgctgttagattggcaattgagttctgctctgataaaaattatatccgtagagatatcggagcatttatactcgggcaaataaaaatttgcaaaaaatgcgaagataatgtttttaatattttgaacaatatggcattgaatgataagagcgcttgcgttcgagctacggcaatcgagtcaacggctcagcgatgcaagaaaaacccaatttattcacctaaaatagtagaacaatctcaaattactgcttttgataaatcgactaatgtcagacgtgctacagcatttgctatttctgttatcaatgataaagcaacaattccactattgattaatctgttaaaagatccaaatggagatgtcagaaactgggccgcatttgcaataaatatcaataaatatgataatagtgatattagggattgttttgtggagatgcttcaggataaaaatgaggaagtccgtattgaagcaataatcggactttcctacagaaaagataaaagggttttatctgttttatgcgatgagttaaaaaaaaatactgtttatgatgatatcattgaagctgcgggtgaattaggtgataaaacgctacttcctgttttagatactatgttgtacaagtttgatgacaatgaaattataacttccgctattgataagctgaagcgttcatagcgtgagttgcctatgcacagtgggggattcccgccggcacggtgcagatgctcgaccggctggaaagtgaaatcctggctgaccgggtgagtgaggaaagccgccgctggctggcatcgtgcggcctgaccgtggagcagatgaaaaaccagatggacccggtgtacacgccggcgcgaaaaatccacctgtaccactgcgaccatcgcggcctgccgctggcgctcatcagcacggaaggggcaacagcgtggtgcgcagaatatgatgaatggggcaacctgctgagtgatgagaacccgcatcatctgcagcagctcattcgcctgccgggtcagcagtatgatgaggagtccggcctgtattacaaccgccaccgctattatgacccgctgctggggcggtatatcactcaggatccgattggactgaaggggggatggaatttttatcagtatccgttgaatccggtcataaatgtagatccgcaaggtttggttgatataaatttataccccgaaagtgatcttatccattctgtagctgatgagattaatatcccaggcgttttcacaatcggggggcatggtacccccacatctattgaatccgcaacgcgcagtatcatgacagctaaagatctagcatatctaattaaatttgatgggaattataaagatgggatgacagtttggttattttcttgtaatacaggtaaaggacaaaattcatttgctagctaattagctaaagagttacatacaaatgtaataggacctgacacgctatggacgtggtgggggcgaggaactaatggtaagttaaaaatggatacagtgctaacagcaccaacgaaccttaattcaaataaggatctaatggctataacaacaaaagaccttggtaattggataacatatgggccatctgggcaccccatttctaatatgcaaggtacgccagaaaaacccagtgatataagataggttgtagatgtatgaaagcatgcttgttactatttttttatttctcttttatttgtcaattgcatggtgctgatgtgaaaataaaacaaaacgaaagtatgatggggtctacagcaatgacctatgatttaagtgaagaaaagttgatgaaactgaagtataaatcacaacatggtgattcagaggcatcatttcgactatatcaatattactgctttactaaaaataacatttacaaacaattgcgattcttggaaagatcagcatctcaggggaatgttacagcgcagtttaattatggggtctttttatcagatacaaatccaacattatcagaatattataatttgaatagagctatttattggatggaattcgctgtaaataacggtaatattgatgcaaagagcaaacttcaagagctcaaaaagctaaagcgaatggatagaaggaagaataaggagaatccgtaaaagcaatagttcatcagactgccgcagcagtagtatgatgatgaatcagggctgtactataactattatcggtaacattaaccgcagcaggggcggtataacactcaggctccgattgggctggaaggtaggtggaatttttatcagtatccgttgaacccgatttctggaatcgatccccttgggattagccacctgtttatacagcataactttaggtatgctttcgtgtgtttcagatataccatgtgatgataatttttatgatgtgcttagtattccagtcgcttctggtaataatatgcaatgtaaaaataatccccgttgtacacatttataaatagatggccaatacctcaaggcctatggagttggaatgttaatgacccgggagcaagcaatagaaaacctgacggcatacgattagtaccgtcagttaatacaggaacttataatcgcaatggattttcaatacatagttgtttaaacgcttttggtccgtctttaggacctcgattctgttccgagggttgtataactggtttatctaatgacatgcaaaaattaaatgagttaatattttcagagccagatagcacattaacagttacggactaaaaaatatggcaaggttattaacaattgtatttttttctctatttctgcgagtgcagttactgcaagacaatttcagagagagttagatttggcagacaaagcaatattatgggcactaatatcagccagtactaaagagggacgaaaagcgtgttcactaagctattttgcctgtaaggccgcagaggctgaactcggactggcatatatggctgcgaatgataacaaggaatttctcacatccttatctaatataatgaggtacaaaatagatgctggactttccgaatcctatacatgctatttattaagtaagggaaagatcataagaccatatctgaaaaatctaaatccactccaacttgccgctgattgcattgaaacagtaaataaaataaaagataagaataaaaaaaatcattgatataaattcagttaatatttgtagtgatgataaaaatataaaattgagagttaatagtactattatggccattgatgattctataaagtgcatcgatgaatgataacttaattttatttaaaaatatattaataactcactctccaggagtttttttaacttagttttataatgaatacgataattaaaagtgaagaagaaaatagttgtatacatatattccatgaccctacattgtgatctatagattaaatattttttaaatgtgactgtcatccttcagataataaagccatcatcgcaatagatggaaaagcactcctgctcttttttgattagagccgtcgcaggaggaacaactcatatcatcattgcgatctcgacgatgtatagtctcatcctgcggcagaacaagacggataaaaaatccaatgagagcacactcatccagaacttattaacataatgaatattaaagaaaaatcatcgaagctaatgaagtaatatgcaaaaataattagtccttacaaggagcaaagttccataatctcccccctccccctcaatgatccaaataaagataatgcatccagctggtcattcttagcagcactttccgcatcaccgaaacatggctgaaatggtcggagtaaaccgccacctgggcgtagatgccgtcgggtaaggcatcgatatcatcgttagggtccagttcaatggttcccagcacaccgtccgtgccgggcacgaccgttaatgattgcaataccccctgcgcctgataagaaccgcctggcacgacaggtaaaatactagtcagtttgccgtgaaacacctgcccaggtagcgcgttaaacaccacttccgcatcatcgccaggtttcagacgtaacagcgagttttgccgaaattgggcgacaatttgccgtttttgctcggggatgaagaccatcaccggacgcagcggcaaggcagctgcgtatgtacctgggcggatcagtacctgagtaacgtagccattgctcggcgcgcgaatgacagtctgctcaaggttatattttgcttcagtaagttgcgctcttaagctcacaatctgcgattgctcgccgttaaccatactgtcgagctggctctggatctgcgcctgctccgccaccgagcctttcaccagcgcatcctgcgcgaggaaattttgccgcgcatcgtcgatgtcacgttccgagaacggattcaccgccgcctggctgcctttcaagtaacgttgataatttttaaacagacggtcgcgctccgctgaaacctgggtggtgttggcctgcgcttcagtgagctgcgcacgcagcgtctttatattatgcgtcgccgtcatcaggtcagcctgaagtctgtcaactcgcgcctggtaacgaaccgggtcgagcttaaaaagcacctcgcccttttgaataagctgattattcttgtcagtgacttcagtaacaattcccgtcacctgtggcgtgatagggatcgctatcactgccttttgcgcggtaaaagtgtaagggtggttgtagttcatcaacaaaatcaaaccactcaccagaaacacgcctcccagcgccgccgtcgccagcgtccactgatttaccggaatgcggaagattttaaagaccgcccacgccagcgccacgtaagttaaaacaatcaatagatccataattagatctccgggaacgtggaatagtcagtctttttctcggcggcgagttgatgctccagccgggaaattcggtcagaaagtgcggcgatttccgggtcagtcgctttctcctgcgacgcaacatgtgactgcataccccagccacgctccggttgatagagcgtcgcccagatccacagaaacggccagataacatgcagagtaaacaggctcacccagcccgccgtatgaatagcgtcggcatggggatggttgcgctttttggcaatcagataagggatgtcatgtatcgcgatgattccataaaaaatcaccagaaagacgaagatcagcactcccaacgcgaaatagtttagaaacatatctgcctcggattcacgtttatcagtgttgtttttgggctggcagccagaagggagtcaggctgatattttgacaataatccgggttcgcgattctcgccataacaccaaagaataatttttagaggtgatgagttgcttagttacataacgattgtatgacgaaggcataacatgctgtagatcacatcaggtgaacgccgtaagaaaatatcttgtgattcagatcacaaagattcaacaaaccatcaaaacaaaaatgtgacactactcacatttaaatgccatttttagcgaaaatcgccgccttgttgcttttttacacaagcgttttgtgatgaacgtcacgtcaattacctctctaccccctatatttatgtgattgatatcacacaaaaggccgtcgactggacagttaaccgattcagtgccagatttcgcagtatctacaaggtccggctacctctgccgccacattaacaaaaaacctcgggcttccagcctgcgcgacagcaaacataagaaggggtgtttttatgtcatccgatattaagatcaaagtgcaaagctttggtcgtttcctcagcaacatggtgatgccaaatatcggcgcgtttatcgcgtggggtatcatcaccgcgttatttattccaacagggtggttaccgaacgagacgctggcgaagctggtcgggccgatgatcacttatctcctgccgctgctgatcggttataccggtggtaagctggtaggcggcgaacgtggcggcgtagtcggtgccatcaccaccatgggcgttatcgtcggcgcagacatgccgatgttcctcggttctatgattgcaggtccgctgggcggctggtgcattaagcacttcgaccgctgggtagacggtaagatcaaatccggttttgagatgctggtgaataacttctccgcaggcatcatcgggatgatcctcgctattctggcattcctcggcattggcccgattgttgaagccctgtccaaaatgctggctgcgggcgttaacttcatggttgtccatgacatgctgccgctggcgtctatctttgttgaaccggcgaaaatcctgttcctcaacaacgccattaaccacggtatcttctcgccgctgggtattcagcagtcccatgaactgggtaaatcaatcttcttcctgattgaagctaacccaggtccaggtatgggcgtgctgctggcgtacatgttctttggtcgtggtagcgctaaacagtctgcgggcggtgcggcaatcatccacttcctggggggtatccacgaaatctacttcccgtatgtgctgatgaatccgcgtctgatcctcgcagtcatcctcggcggtatgactggcgtgttcacgctgactatcctgggcggtggtctggtttctccggcatctccgggttctatccttgctgtactggcgatgacaccaaaaggtgcttacttcgctaacatcgcgggtgtgtgtgcggcgatggctgtctccttcgttgtctctgctattttgctgaaaaccagcaaagtgaaagaagaagatgatattgaagcagcaactcgtcgtatgcaggacatgaaagctgagtctaaaggcgcatctccgctgtctgctggcgatgtgactaacgacctgagccacgtacgtaaaatcatcgttgcctgtgacgccggtatgggttccagtgcgatgggcgcaggcgttctgcgtaagaaaattcaggatgcaggtctgtcgcagatttctgttactaacagcgcgatcaacaacctgccgccagatgtggacctcgtcatcactcaccgtgacctgaccgaacgcgctatgcgccaggttccgcaggcacagcatatttcgctgaccaacttcctcgacagcggcctgtacaccagcctgaccgaacgtctggttgctgcccaacgccacacggcaaacgaagagaaagtaaaagacagcctgaaagacagctttgacgattccagtgctaacctgttcaagctaggcgcggagaacatcttcctcggtcgcaaagcggcaaccaaagaagaagcgattcgttttgctggcgagcagctggtgaaaggcggttacgttgagccggaatacgttcaggcgatgctggatcgtgaaaaactgaccccgacttatctgggtgagtctatcgcggtgccacacggtacggttgaagcgaaagatcgcgtactgaaaacgggcgtcgtgttctgccagtacccggaaggcgtgcgcttcggtgaagaagaagatgacattgcccgtctggtgattggtattgctgcccgtaacaacgagcacattcaggttatcaccagcctgaccaatgcactggatgatgagtccgtcatcgagcgtctggcacacaccaccagcgtggatgaagtgctggaactgctggcaggtcgtaagtaatccaatcccaccctctccacatggagaaggtggggttaattgcctgatgcgctacgcttatcaggcctacaggatgcatcacaatttgttgaatttgcacgttcttgtaggccggataaggcgcttacgccgcatccggcgctgcccctctcctcacggagagggtttgggtgagggaaaagcctcaccccagccctctcgggtaaaaacattgatgaaggttaatactatgaaagcattacattttggcgcaggtaatatcggtcgtggctttatcggtaaactgctggcagacgcgggtatccaactgacgtttgccgatgtcaatcaggtggtacttgatgccctgaatgcccgtcatagctatcaggtacatgtggttggtgaaaccgagcaggtagataccgtttccggcgtcaatgctgtcagcagcattggtgatgatgtcgttgatctgattgctcaggttgatttagtcactaccgccgttggcccggttgtgctggaacgtattgctccggcaatcgccaaagggcaggtgaaacgtaaagaacaaggtaatgaatccccgctgaacatcatcgcctgtgaaaacatggtacgcggtaccacgcagctgaaaggccatgtgatgaacgccctgccggaagacgccaaagcgtgggtagaagaacacgttggctttgtcgattccgccgttgaccgcatcgtaccgccttcggcttcggcaactaacgatccgctggaagtgacggtagaaaccttcagcgaatggattgtcgataaaacgcagttcaaaggcgcactgccgaacatcccaggcatggagttaaccgacaacctgatggcatttgtcgaacgtaaactcttcaccctgaacacgggtcatgctataaccgcgtacctcggaaaactggccggtcatcagaccattcgtgacgcgattctcgacgagaaaatccgcgcggtggtaaaaggtgcgatggaagaaagtggtgcagtattgatcaagcgctacggctttgacgctgacaagcatgcggcgtacatccagaaaattctcggccgttttgagaacccgtatctgaaagatgatgtagagcgcgtaggccgtcagccactgcgtaaactgagtgctggcgaccgtctgatcaagccactgctcggtacgctggaatatggtctgccacataaaaacctgattgaaggtattgccgctgcaatgcacttccgcagtgaagatgatccgcaggctcaggaactggcagcactgatcgctgacaaaggtccgcaggcggcgctggcacagatttccggtcttgatgccaacagcgaggttgtatccgaggcggtaaccgcttataaagcaatgcaataatggtggaccaggcgcaggacaccctgcgcccgaataacagattgtcagatatgcaggcaacaatggaacaaacccaggcctttgaaaaccgtgtgcttgagcgtctgaatgctggcaaaaccgtgcgaagctttctgatcaccgccgtcgagctcctgaccgaggcggtaaatcttctggtgcttcaggtattccgcaaagacgattacgcggtgaagtatgctgtagaaccgttactcgacggcgatggtccgctgggcgatctttctgtgcgtttaaaactcatttacgggttgggcgtcattaaccgccaggaatacgaagatgcggaactgctgatggcattgcgtgaagagctaaatcacgacggcaacgagtacgcctttaccgacgacgaaatccttggaccctttggtgaactgcactgcgtggcggcgttaccaccgccgccacagtttgaaccagcagactccagtttgtatgcaatgcaaattcagcgctatcaacaggctgtgcgatcaacaatggtcctttcactgactgagctgatttccaaaatcagcttaaaaaaagcctttcaaaagtaagcaacgtctgcttactgcccctctacctgcttcggccgataaagccgacgataatactccagacgttgtagatataacggcacgctttcatcgggtattccggacggaatcgcgttacggggaggaagttttttcagatactcccggaacgcctggcttgatgccatgaaatctacggctttatcgataagaagcggaacgttttcacctaatttgcccatgatgatatctccgtattaccccgcgccgggaatgcgcggccgccaattttagtttaggttcccggtaaagatgacattaaggaaaacgtgctgaatcctcaataatcatccgctgctgtttattatcttttttctatagatttcttaattaatcaacgaattgcgcagtttttgagcatgttaatgattacgttacagaactattacaatgtcattagttgtgaacaaagcacctggtcgcgcatactaggggctataaatttatctttatcagaagccatcacatgaaagaagtcgaaaaaaacgaaatcaaacgcctcagcgatcgcctggacgccatccgccaccagcaggccgatctttcgctggttgaagccgcagacaaatatgccgagctggaaaaagagaaagccacgctggaagcagaaattgctcgcctgcgtgaagttcatagccaaaaactgagtaaagaagcacagaagctgatgaagatgccattccagcgcgcaattaccaaaaaagagcaggctgatatgggcaagctgaagaaaagtgttcgcggactggtcgttgtgcacccaatgaccgcactgggccgcgaaatgggcctgcaggagatgactgggttttcaaagaccgcgttttaagaacacagtatctacagggtgattctgcacattcctataggccgagtaaggtgttcacgccgcatccggcaagataaggcgctctggatcaacaacctaagggcaattctctgatgaggattgcccttttctttaccagacatctccccccacaagaattggccctaccaattcttcgcttatctgacctctggttcacaatttcccaattaaaactcacatcaatgttgccaatacataacatttagttaaccattcattgtcattatccctacacaacacaattggcagtgccacttttacacaacgtgtgacaaggagatgagcaacagactcattacacgatgtgcgtggactccaggagacctgcaatgaatctctggcaacaaaactacgatcccgccgggaatatctggctttccagtctgatagcatcgcttcccatcctgtttttcttctttgcgctgattaagctcaaactgaaaggatacgtcgccgcctcgtggacggtggcaatcgcccttgccgtggctttgctgttctataaaatgccggtcgctaacgcgctggcctcggtggtttatggtttcttctacgggttgtggcccatcgcgtggatcattattgcagcggtgttcgtctataagatctcggtgaaaaccgggcagtttgacatcattcgctcgtctattctttcgataacccctgaccagcgtctgcaaatgctgatcgtcggtttctgtttcggcgcgttccttgaaggagccgcaggctttggcgcaccggtagcaattaccgccgcattgctggtcggcctgggttttaaaccgctgtacgccgccgggctgtgcctgattgttaacaccgcgccagtggcatttggtgcgatgggcattccaatcctggttgccggacaggtaacaggtatcgacagctttgagattggtcagatggtggggcggcagctaccgtttatgaccattatcgtgctgttctggatcatggcgattatggacggctggcgcggtatcaaagagacgtggcctgcggtcgtggttgcgggcggctcgtttgccatcgctcagtaccttagctctaacttcattgggccggagctgccggacattatctcttcgctggtatcactgctctgcctgacgctgttcctcaaacgctggcagccagtgcgtgtattccgttttggtgatttgggggcgtcacaggttgatatgacgctggcccacaccggttacactgcgggtcaggtgttacgtgcctggacaccgttcctgttcctgacagctaccgtaacactgtggagtatcccgccgtttaaagccctgttcgcatcgggtggcgcgctgtatgagtgggtgatcaatattccggtgccgtacctcgataaactggttgcccgtatgccgccagtggtcagcgaggctacagcctatgccgccgtgtttaagtttgactggttctctgccaccggcaccgccattctgtttgctgcactgctctcgattgtctggctgaagatgaaaccgtctgacgctatcagcaccttcggcagcacgctgaaagaactggctctgcccatctactccatcggtatggtgctggcattcgcctttatttcgaactattccggactgtcatcaacactggcgctggcactggcgcacaccggtcatgcattcaccttcttctcgccgttcctcggctggctgggggtattcctgaccgggtcggatacctcatctaacgccctgttcgccgcgctgcaagccaccgcagcacaacaaattggcgtctctgatctgttgctggttgccgccaataccaccggtggcgtcaccggtaagatgatctccccgcaatctatcgctatcgcctgtgcggcggtaggcctggtgggcaaagagtctgatttgttccgctttactgtcaaacacagcctgatcttcacctgtatagtgggcgtgatcaccacgcttcaggcttatgtcttaacgtggatgattccttaatgattgttttacccagacgcctgtcagacgaggttgccgatcgtgtgcgggcgctgattgatgaaaaaaacctggaagcgggcatgaagttgcccgctgagcgccaactggcgatgcaactcggcgtatcacgtaattcactgcgcgaggcgctggcaaaactggtgagtgaaggcgtgctgctcagtcgacgcggcggcgggacgtttattcgctggcgtcatgacacatggtcggagcaaaacatcgtccagccgctaaaaacactgatggccgatgatccggattacagtttcgatattctggaagcccgctacgccattgaagccagcaccgcatggcatgcggcaatgcgcgccacacctggcgacaaagaaaagattcagctttgctttgaagcaacgctaagtgaagacccggatatcgcctcacaagcggacgttcgttttcatctggcgattgccgaagcctcacataacatcgtgctgctgcaaaccatgcgcggtttcttcgatgtcctgcaatcctcagtgaagcatagccgtcagcggatgtatctggtgccaccggttttttcacaactgaccgaacaacatcaggctgtcattgacgccatttttgccggtgatgctgacggggcgcgtaaagcaatgatggcgcaccttagttttgttcacaccaccatgaaacgattcgatgaagatcaggctcgccacgcacggattacccgcctgcccggtgagcataatgagcattcgagggagaaaaacgcatgattatttccgcagccagcgattatcgcgccgcagcgcaacgcattctgccgccgttcctgttccactatatggatggtggtgcatattctgaatacacgctgcgccgcaacgtggaagatttgtcagaagtggcgctgcgccagcgtattctgaaaaacatgtccgacttaagcctggaaacgacgctgtttaatgagaaattgtcgatgccggtggcactggctccggtgggtttgtgtggcatgtatgcgcgtcgtggcgaagttcaggcagccaaagcggcggacgcgcatggtattccgtttactctctcgacggtttccgtttgcccgattgaagaagtcgcgccagccatcaagcgcccaatgtggttccagctttatgtactgcgcgatcgcggctttatgcgtaacgcgctggagcgagcaaaagcagcgggttgttcgacgctggttttcaccgtggatatgccgacaccgggcgcacgctaccgtgatgcgcattcaggtatgagcggcccgaacgcggcaatgcgccgctacttgcaagcggtgacacatccgcaatgggcgtgggatgtgggcctgaacggtcgtccacatgatttaggtaatatctcagcttatctcggcaaaccgaccggactggaagattacatcggctggctggggaataacttcgatccgtccatctcatggaaagaccttgaatggatccgcgatttctgggatggcccgatggtgatcaaagggatcctcgatccggaagatgcgcgcgatgcagtacgttttggtgctgatggaattgtggtttctaaccacggtggccgccagctggacggtgtactctcttccgcccgtgcactgcctgctattgcagatgcggtgaaaggtgatatagccattctggcggatagcggaattcgtaacgggcttgatgtcgtgcgtatgattgcgctcggtgccgacaccgtactgctgggtcgtgctttcttgtatgcgctggcaacagcgggccaggcgggtgtagctaacctgctaaatctgatcgaaaaagagatgaaagtggcgatgacgctgactggcgcgaaatcgatcagcgaaattacgcaagattcgctggtgcaggggctgggtaaagagttgcctgcggcactggctcccatggcgaaagggaatgcggcatagtcgtttgcgccccctcaccctaaccctctccctcagggagaggggaccgttcggcgctgtatgtactccctcactctgaaacgacaccgcactctttttttctccctcgcccctccggggagagggccggggtgaggggaaaaggccgcactgctcaccaattttctgctatcctgcccccgcactaagggggcagtatgctaaacatcgtactttacgaaccagaaattccgccaaatactggcaacatcatccgtctttgcgctaataccggctttcgtctgcatatcatcgaaccgatgggatttgcctgggacgataagcgcctgcgccgcgcggggctggactatcacgagtttaccgccgttacgcgtcatcatgactatcgcgcgttcctcgaagcagaaaatccccagcgcctgttcgccctcaccacgaaaggtacacctgctcacagcgccgtaagctatcaggatggcgattatctgatgttcggcccggaaacacgcggcctgccagcgagcattcttgatgccctgcccgctgaacaaaaaattcgcattccgatggtgccggacagccgcagcatgaatctgtccaatgcggtgtcggtagtggtgtatgaagcctggcggcagttggggtatccgggagcggtattgagagattagttactgtaggccggatagatgattacatcgcatccggcacgatcacaggacattagatcccatccccatactcaaatgtatggttaataccgttgaaatgctggtccatatccattgatggcttatcgctgtctggtttaccgacaatacgagccggaacgccagcggcggtggtatgcggcggcaccggttgcagcaccacggaacctgcgccaatcttcgcgccgcgcccaacttcaatattgccgaggattttcgcgcccgcgccaatcatcacaccttcacgaattttcgggtgacggtcaccaccagatttacccgtaccgccaagcgtcacagattgcagaatcgatacgtcgttttcaatcaccgccgtttcaccaacgacgatgcctgtcgcgtggtcaagcatgataccgcgaccaatttttgctgccgggtgaatatcgacctggaacgtcacagaaacctggttttgcagaaagattgccagtgcgcgacgcccctgattccacaaccagtgaccgatgcgataggcctgcaaggcatgaaaacccttcaggtataacaacggggttgagtatttatcgactgccgggtcgcgggtacgcaccgcctgaatatcacaggccgcagaggcgatcatttccgggtcagcggcgtaggcttcttccaccacttcacggatagcaatagcaggcataattggcgatgacagcttgttcgccagcatgtagctcagtgcactgccaaggttttcgtgcttgagtagcgtcgcgtggtaaaaactggccagcattggctcacagtccgccagcgttctggcttcggctttaatattgttccagacaatttccagttcttcacacgacattgcttactccacacgatgagataatgaccggcccgttctgcgcgggccgggtcatagcggtaacaaaggttccctggggttagtggctgctgcgctcgtccttgcgtgcacgacctagtaaagtcaatgctgcctcgcgcgcgttttttccgcaatataatacttgataaatttcctcggttattggcatttcaacgccgaagcgatgcgccagttcgcggacttctttcgtattgcggtagccttccaccacctgaccaatcttctcctgcgcgctttgtacatccatgccctgaccgagcatcatgccaaaacggcggttacgcgactggttgtcggtacaggtaagcaccagatcgccaagccccgccatgcccataaaggtggcagggtcggcacccagcgccgcaccaagacgcgacatttcagccagcccacgggtgatcagcgccgtacgcgcattcgcaccaaaaccgataccgtcggacatccccgcaccaatggcaataacgtttttcaccgcgccgccaagctgcacgccaatgaaatccggattgctgtaaacgcggaaacttttgccgcagtgcagcagctgctggagatcatcggcaaaggtctgatcggtcgaggccagcgaaatagctgtcggtaaacctgccgccagttctttcgcaaacgttgggccagagataaccgccagcggaatttgatcgcctaaggcctcacgcgccacgtcctgtaacagacgtccggtttccgcttccagccctttggtcgcccacaccagacgcgcatcaggacgcatcagtggtttaatctggcgcagcacttcaccaaagacatggctgggtacgacgacgagaatattacggctggctgccagcgcagtggcgagatcgctttcaagatggagcgtatcgggaaaaggcacatcggggagaaacgcggcgttacagcggtcgcgttcaagcgttgcgatatgttcagggtcatggccccagaggacaacctcgtggccatttcttgccagggtgatggcaagagcggtgccgtacgagccggcaccgatcacagtcattgaagcattacgttggttcatcaggcatcctgatgttcttcagtaccttcgccagcctgctgctgcaaatagttcatgaacagcgcatcgaagttaaccggcgcaaggttcagttgcgggaatgtaccgcgggataccatgctggtgatgcactcacgagcatacgggaacagaatgttcgggcagtatgctcccaggcaatgcgccatctgggtgccttcgatacccgcgatggagaaaataccgccctgctgaacttcacacaggaacgcggtttcttcgcccaaagaggccgttacggtaacacgcagtaccacttcgtatacgtcatctgccagttgggaagatgccgtatccagatcaagtttaacttctggttgccaatctttctggaaaacgtgcggcgcgttcggcgcttcgaaagagatatccttggtataaatacgttggatctggaaagtcatttcagtgttgttttgttctgacatgtgtagaaaacccttaagtgttgtccttaaatactgcgcaatgtaatgccaacgttcacacgttatttcagcaggggatccagtccaccacgtgcatccaatgcatacaagtcatcacagccgccaatgtgctgtgcgtcaataaaaatctggggaaccgtggtgcgaccgctgcgtttgatcatctcttcacgcttggcggcgttgccatcgatcggcagctcctggaaactcacgcccttgctgctcagcagtgcttttgcacgatggcaatacgggcaggtttctttggtatagatttcaacattggccataaattagctcctgtttttttaccctgaaatttcatgttgcagggcggcagcaaaatggagtgtccccagaagcttataacaataagtcgctgggggcctaattgcagctaacggcctgcatcatgaaagacgacaggtaaattatttgccgcgcaccaaaggcaagttttcgccagcccagccagcgacgccttctttcagcacgaatacttgcgcaaaaccagctttcgtcagtgcgtttgcaggctcctggcactgcatgccagaaccgtctaccacgataaccggtttgtctttgtgcttctcaagctcaccaacattgttggctttgatttcgctcggcaacagattaatagaacctgcgatatggcctttacggaagtcatcacgctgacgtaaatccacaaccacagcgtcttctttgttgatcagacgcgtagcttcaccacgagtaatcaccttcactttcgaggtcaggctcttaaacgtagtcacaagaaccgccaccagtaacgcgatccaggcgatactcagtatgggatgacggccaacaaattgcataatttcttgcatggggggtaacaactcccgacgtagtgattaaaaaaaccaggaaaggagtatacctgcgcggtgcggcaaatacagccagcgcgttaactggaatgcaattttgcggggcgcgacgaaaaaaaagcgtaaatctggcatcggcttgccgcgagcggtcgtatattttgatcttcagaggctattttatcgattcagctgtagtaaaattacgcaaattttgactcttgagtatgaggttgtcgcaatgttggtttctaaaaaacctatggtactggtgattctggatggctatggctatcgcgaagaacagcaggataacgccatttttagtgctaaaaccccggtaatggatgcactgtgggccaatcgtccgcataccctaatcgacgcttccggtctggaagtcggtctgcctgaccgtcagatgggtaactccgaagtaggccacgttaacctgggtgccggccgcatcgtgtatcaggacctgactcgtctggacgttgaaatcaaagatcgcgctttctttgctaatccggtgctgactggcgcggtagataaagcgaaaaacgcaggcaaagcggtacacattatgggtctgctctccgcaggcggcgtacacagccacgaagatcacatcatggcgatggtagaactggcagctgaacgcggcgcagaaaaaatctacctgcacgcattccttgacggtcgcgacactccgccgcgcagtgctgaatcctcgctgaaaaaattcgaagaaaaatttgccgcgctgggcaaaggccgcgtagcgtccatcattggtcgttactacgcgatggaccgcgataaccgttgggatcgcgtagaaaaagcttatgacctgctgactctggcgcagggcgagttccaggccgataccgccgttgctggtttgcaggctgcttatgctcgcgacgaaaatgatgaattcgtgaaagcgaccgttatccgtgctgaaggtcagccagacgcggcaatggaagacggcgatgcactgattttcatgaacttccgtgctgaccgcgcgcgtgaaatcactcgtgctttcgtgaacgctgatttcgatggcttcgcgcgtaagaaagtggttaacgtcgatttcgtgatgctgaccgaatacgccgctgacatcaaaactgcggttgcttacccacccgcttccctggttaacaccttcggcgagtggatggcgaaaaacgacaaaactcagttgcgtatttccgaaaccgaaaaatatgcccacgttactttcttcttcaacggtggcgtagaagagtcgttcaaaggcgaagatcgcattctgatcaactcaccgaaagtggctacctacgatctgcaaccggaaatgagctccgcagagctgaccgaaaaactggttgcggccatcaagagcggcaaatacgacaccatcatctgtaactatccgaacggcgacatggtaggtcacaccggggtgatggaagcggcggttaaagcggttgaagcgctggatcactgcgtggaagaagtcgcgaaagcggttgagtccgtgggtggacaactgctgatcaccgctgaccacggtaacgctgagcagatgcgcgatccggcaacgggtcaggcacacacggcacacaccaacctgccagttccgctgatttacgttggtgataagaacgtgaaagcggttgaaggcggcaaactttctgacatcgcgccgaccatgttgtcgctgatgggtatggaaatcccgcaagagatgactggtaagccgctgttcatcgtggaataatccctccccatgaggggaaaggcgattaataccatgacacgggccgtgaaaccgcgcaggtttgcaatcaggcccatcatctacgccagcgttcttagcgctggcgtattgttgtgcgccttttccgcccacgcggatgagcgtgaccaactcaaatctattcaggctgacatcgccgcaaaagagcgcgcggtacgccaaaagcaacaacaacgcgcaagcctgctcgcacaattgaaaaagcaggaagaagcgatctctgaagccacccgtaagctgcgcgaaacgcaaaacacgctcaatcaactcaataaacagattgatgagatgaacgcgtcgattgccaaactggagcagcaaaaagccgcccaggagcgcagcctcgccgcacaactggatgccgcattccgtcagggcgagcataccggtattcagctgattctcagcggtgaagaaagccagcgtggacagcgtttacaggcttatttcggctatctcaaccaggcgcgacaagaaaccattgcccagttgaagcaaacgcgtgaagaagtcgccatgcagcgtgctgaactggaagagaaacagagcgagcaacaaacgctgttatatgagcagcgcgcccaacaggcgaaactgactcaggcgctgaacgagcgtaaaaagacgctggcagggctggagtcttccatccagcaaggtcagcaacagttgagcgagctgcgcgccaacgaatcccgtctgcgtaacagcattgcccgtgcggaagccgcggcgaaagcgcgtgcagaacgagaagcacgtgaggcccaggcggttcgcgaccgccagaaagaagcgacgcgcaaaggcaccacctacaaaccgaccgaaagcgaaaaatcgctgatgtcccgtaccggtggtctgggcgcgccgcgtggtcaggcattctggccggttcgcgggccgacgctgcatcgctatggcgaacagctacagggtgaattacgctggaaaggtatggttatcggtgcttctgaaggtactgaagttaaagcgattgccgacggtcgggtgattctggctgactggctgcaaggctacggtctggtggtggtggttgagcatggtaaaggcgacatgagtctttacggctataatcagagcgcactggtgagcgttggttcgcaggttcgcgcgggccagccgattgcactggtgggcagcagtggcggtcagggtcggccttcactctatttcgaaattcgccgccagggtcaggcggtcaatccacagccgtggttgggaagataagttttgtttccatttcgtcgtaacgttcttgcatttgccgctctgttggcgctctcctcccccgtacttgctggcaaacttgccatcgtcattgatgattttgggtatcgcccgcacaacgaaaaccaggtgctggcgatgccttccgctatctccgtcgctgtattacccgattcaccgcacgccagagagatggcgaccaaagcgcataacagcgggcacgaagtgttgattcatctcccgatggcaccgttgagtaaacagccgctggagaaaaatacgctacgcccggagatgagcagcgacgaaattgagcgcattattcgtagtgcggtcaataacgtgccctatgccgtggggatcaacaaccacatgggcagcaagatgacctctaacctgtttggtatgcagaaagtgatgcaggcgctggagcgttacaatctttacttcctcgacagcgtaaccatcggtaatacccaggcgatgcgcgccgcgcaaggcactggcgtgaaggtgatcaaacggaaggtattcctcgacgattcgcaaaatgaagcggacatccgtgtgcaatttaatcgcgcaattgacctggcgcgtcgcaacggttcgaccattgccattgggcatcctcaccctgcaacggtacgcgtgttgcaacagatggtttataacctgccgccagacattacgctggtgaaagccagcagcttgctgaatgaaccgcaggttgatacttctacaccgccgaaaaacgctgtgcctgatgcaccgcgtaatccgttccgtggcgtgaagctgtgcaaaccgaagaaaccgatagaacctgtttatgctaatcgcttctttgaagtattaagcgaaagcatcagccagagcacgctgatcgtttacttccagcatcagtggcaaggctggggcaaacagcccgaagcggcgaagtttaacgctagcgcaaattaaaggcgctacgcgtaatgcgatggtgcgaccgcgttttgtcgcgccattgccataagcggaaagaccacagtaacgcctggtaaccgaccttcacgctgcgcacattggtaatcaggcgcttatacataccggaagtaaatatctcggcaatcatccgttggcgggtaagaatatccggctctttgcgcaccgcatggcaaacacgcaatgcctcgtaagttatttgctgatgaaattccggataaatcataattttgtcggcataatttcgatttaatttctccagcaggcgggtaatcttaatatagtgacgttgataattaaggtttttattcccttgtctatgcaaccgactcactgacgtattatgcagataatatttatataatgattgctcggtatatcgcgcacgcagcgcgttaaacatgaattctgttgtccagacaatatcctgatgatgtaatccggcaataaatttaatgttatttttaacaataacatcacggcgataaacccccatccagacaacgtgagtccaacggcgcgaagaaagccccatccgcagccagtccgggccggttaatacgccggttgagcgaaggcgatcggtggggatggattgccaggtttctcccgtttcacgaaaacaccagtcagcgttgcactgcgccacgtcgaggtcgtcctctaacgccatggtcatcagcgtttcgtacatggtgggatagacttcatcgtcagcatcgacaaaagcgacatatttgcccgttgccacttcaatcccacgattacgcgccaccgatgcgccagcattcgcctgatgcaacaaacgaacgtgcggatagttttctgcgtaatactttgctatttcaacagaattatccgttgaaccatcgttaataataatgatttccagagcagtccaggtttgcgtaattaaagattccatacaagtgcggaaatcatcgcccgcattatataacggaataataacactaagtttattggtgctgttcatcataaattaccgacgacctctgaagttatcctgacgttttacaggctttgtattaagaaactattaagcctgtgagatattatttttacaggtgagagagtcacttcagggtagagagataatgagagcagctatataagagatcagcacaattacgaactctttattacactgacaggattttacatatttaacagattatcctcagataaaagggctggaataccagcccttgttcgtgttaatcccagctcagaataactttcccggactggcccgaacgcatagcgtcaaagcccttctggaaatcatcgatagagaaacgatgggtaatgatcggcgaaagatcgaggccagactgaatcagcgccgccatcttgtaccaggtttcaaacatctcacgaccgtaaatacctttaatgaacaagcctttaaagatcactttggtccagtcgatagacatatcagacggcggaatacccagcatcgcaatacggccgccgtgattcatggtgtcaagcatggtacgaaacgctggcggcgcaccggacatttccagaccgacatcaaaaccttcggtcatgcctaactccgccatcacgtcattgagattttctttggcgacgttaaccgcacgggtgatacccattttacgcgccagctcaaggcggtattcgttaacatcagtgatcaccacattgcgtgcaccaacgtgtttcgccaccgccgctgccataataccaatcgggcctgcaccagaaaccagcacatcttcgcccaccagatcaaacgacagcgcggtatgcacggcgttaccgaagggatcaaaaattgcggctaagtcatcggaaatattgtcggggattttgaaggcgttgaatgccgggatcaccagatattcggcaaagcagcccgggcgattaacaccaacgcctatcgtgttgcggcacaaatgggtacgaccaccacgacagttgcggcaatgaccacaggtgatatggccttcgccagaaacgcgatcgccgatcttgaagcctttcacttcctgaccaatacctaccacttcaccgacatattcatggcccacgaccatcggcaccgggatggttttttgcgaccactcatcccagttatagatgtgaacgtcagtcccgcagatggctgttttacggattttaatcagcagatcgttatgcccgagttccggtacaggaacgtcggtcatccagatgccctcttccgctttcagtttggataacgctttcatctcacatcctcaggcgataacgcccagttgtttaccaatacgcgtaaatgcttctactgcacgcgtaatttgctcaggggtatgcgccgcagacatctgggtacgaatacgcgcctgacctttcggaacgaccggatagaagaaaccggtaacgtaaatgccctctttttgcagctcacgggcaaatttctgcgccactaccgcatcaccaagcatgaccggaataatggcgtgatcggctcccgccagggtaaagcccgccgccgacatttgctcacggaactgacgcgcgttcgcccacagacggtcacgcagttcgctgcccgcttcgaccatctccagtactttgatggacgcggcaacaatggccggtgccagcgagttggagaacaggtacggacgagaacgctggcgcagccactcaaccacttctttgcgcgccgcggtataaccaccagaagccccgcccagcgctttaccaagcgtaccggtgataatatcgacccggcccatcacatcgcagtattcatgggaaccacgaccattttcaccgacaaaaccgaccgcgtgggagtcgtctaccatcaccagggcatcatatttatctgccagatcgcaaacgcccttcaggttggcaatcacgccgtccattgagaacacaccatcggtggcgatcagcacatgacgcgcaccggcttcacgcgcttctttcagacgtgcttccagctcctgcatatcgttgttggcatagcgatagcgtttagctttgcacagacgcacaccatcaataatagacgcgtggttcagtgcgtcggagataatggcgtcttccgcacccagaagcgtttcaaacaggccaccgttagcatcaaagcaggaagagtagagaatcgcatcttccatccccaggaaggccgccagtttttgttcaagctctttatggctgtcctgagtgccgcaaataaaacgcaccgaagccatgccgaaaccgtgagaatccattcccgcctttgccgccgcaatcagatcaggatgattcgccagcccgagatagttgttggcacaaaagttaatgacgtggcttccatcagccacagtgatatctgcttgctgcgcagacgtaataatgcgctcttctttaaacaacccttccgcccgtgcggtttccagatcgttggttaactgctgataaaattctccacgcattgcgattctccagacagggcaaattccagcacatattacccaaacttataggtcgcgacgagataacgcgttaacacttctgcaaaattcaggataaataacgtgtaacttgatgtctctcaacacctacagatagtagaaaaactgtacagttttggctgggcataatgatgattgattttactgcattgatataaaaagaaaaaatgatgccaaagcatcatttttcctatctcagttggtatcaaaacgctacccactaatggagggaaacctattttcttgaaaggaaaattctcagcgcctgcatttttgcccctaaagtgttactcctgaagcagcgaaacaaatcgaaccattttcctctccccagatagtttaggttgaagagatcggggcgtttgtaatagcacatgacaaaaatgccctggtcatcgtccacaatgttattatttagtgttattttttgactttccagaactaatttatagaattctttccatttatgctgtgaaccaacaattgcgcccccaataatatatacatgattgccaatcatgaaatcaaaaacctgttgttgagatgtgacagtaagccctttttttatagtgaaaagatgcatcttactttcatcaaatgggaaatcccaaattttcaatcctcgagttacatttggcttatggcaatagccaaaatctatccacgcaacaagaggcgttttcactaagcccatgttgatagctttatttacaaaataggccttaaggttacataccaaaacatactctggtgaccagtactctgggttttttaattgtcgaggctcaagtctatttgtaaacgactcatctttttgaattttttcgatacgacttctgatatatctaaatttcttttttatatcgataacgataaccgttgttggttttccgttgcgaatcgcttcaacccttggtttcaaatcgggagaagtgaaaataatcatctcattttcaagtgcggccagacgctcaaagtaactaaaataaacatcaactgaacgagctagtttttcacggaaccctttattagcagtccaatcccctctaccaatgtcaaaatatgcagtgataattgtggtggatgatttcattactaataagaccattaatataaaaaaagaattatatcataaatattaatagaatgtatactgtatattatccattcaaatgcttccgttatttatcatacatcggaatattgatactaaagcactattcacatgcaaaaccaacatccgccatgaaggactagctaaaacccaaactagtttgttgcaattagcatccttgcacctctatgtaaagggctgaagggattcggatgtgatggtatgattacagacattcgtgtctgagattgtctctgactccataattcgaaggttacagttatgatcatcgttaccggcggcgcgggctttatcggcagcaacatcgttaaagccctgaatgataaaggcatcaccgatattctggtggtggacaacctgaaagacggcaccaagtttgtgaacctggtggatctgaatatcgcagactatatggataaggaagacttcctgatccagattatggctggcgaagagttcggcgatgtcgaagcgattttccacgaaggcgcgtgctcttccaccaccgagtgggacggcaagtatatgatggataacaactatcaatactccaaggagctgctgcactactgcctggagcgtgaaatcccgttcctgtacgcttcttccgcagccacctacggcggacgcacctccgactttattgaatcccgcgagtacgaaaaaccgttgaacgtctacggttactcaaaattcctgtttgatgaatatgttcgtcaaatcctgcctgaagcgaactcgcagattgttggcttccgttatttcaacgtttatggaccgcgtgaaggccataaaggcagcatggcgagcgtcgctttccatctcaacacccagcttaacaacggtgaatcaccgaagctgtttgaaggtagcgagaacttcaaacgcgacttcgtctatgtgggcgacgtggctgatgtgaatctgtggttcctggaaaatggcgtttccggcatcttcaatctcggtactggtcgtgcggaatccttccaggcggtagctgatgctacgctggcttatcacaagaaaggccagatcgaatacattccgttcccggataaactgaaaggccgctatcaggcgttcactcaggcagatctgacaaatctgcgcgcggcgggttacgacaaaccgttcaaaaccgttgctgaaggtgtaacggaatacatggcctggctgaatcgcgacgcataagagctctgcatgaaaatactggtgatcggcccgtcttgggttggcgacatgatgatgtcgcaaagtctctatcgcacgctccaggcgcgctatccccaggcgataatcgatgtgatggcaccggcatggtgccgtccattattatcgcggatgccggaagttaacgaagctattcctatgcctctcggtcacggagcgctggaaatcggcgaacgccgcaaactgggtcatagcctgcgtgaaaagcgctacgaccgcgcctacgtcttacccaactccttcaaatctgcattagtgcctttcttcgcgggtattcctcatcgcaccggctggcgcggcgagatgcgctacggtttactcaacgatgtacgcgtgctcgataaagaagcctggccgctaatggtggaacgctatatagcgctggcctatgacaaaggcattatgcgcacagcacaagatctgccgcagccattgttatggccgcagttgcaggtgagcgaaggtgaaaaatcatatacctgtaatcaattttcgctttcatcagaacgtccgatgattggtttttgcccgggtgcggagtttggtccggcaaaacgctggccacactaccactatgcggagctggcaaagcagctgattgatgaaggttatcaggtggttctgtttggctcggcgaaagatcatgaagcgggcaatgagattcttgccgctttgaataccgagcagcaggcatggtgtcggaacctggcgggggaaacacagcttgatcaagcggttatcctgattgcagcctgtaaagccattgtcactaacgattctggcctgatgcatgttgcggcggcgctcaatcgtccgctggttgccctgtatggtccgagtagcccggacttcacaccgccgctatcccataaagcgcgcgtgatccgtttgattaccggctatcacaaagtgcgtaaaggtgacgctgcggagggttatcaccagagcttaatcgacattactccccagcgcgtactggaagaactcaacgcgctattgttacaagaggaagcctgacggatgcgggttttgatcgttaaaacatcgtcgatgggcgatgttctccatacgttgcccgcactcactgatgcccagcaggcaatcccagggattaagtttgactgggtggtggaagaagggttcgcacagattccttcctggcacgctgccgttgagcgagttattcctgtggcaatacgtcgctggcgtaaagcctggttctcggcccccataaaagcggaacgcaaagcgtttcgtgaagcgctacaagcagagaactatgacgcagttatcgacgctcaggggctggtaaaaagcgcggcgctggtgacgcgtctggcgcatggcgtaaagcatggcatggactggcaaaccgctcgcgaacctttagccagcctgttttacaatcgtaagcatcatattgcaaaacagcagcacgccgtagaacgcacccgcgaactgtttgccaaaagtttgggctatagcaaaccgcaaacccagggcgattatgctatcgcacagcattttctgacgaacctgcctacagatgctggcgaatatgccgtatttcttcatgcgacgacccgtgatgataaacactggccggaagaacactggcgagaattgattggtttactggctgattcaggaatacggattaaacttccgtggggcgcgccgcatgaggaagaacgggcgaaacgactggcggaaggatttgcttatgttgaagtattgccgaagatgagtctggaaggcgttgcccgcgtgctggccggggctaaatttgtagtgtcggtggatacggggttaagccatttaacggcggcactggatagacccaatatcacggtttatggaccaaccgatccgggattaattggtgggtatgggaagaatcagatggtatgtagggctccaagagaaaatttaattaacctcaacagtcaagcagttttggaaaagttatcatcattataaaggtaaaacatgctaacatcctttaaacttcattcattgaaaccttacactctgaaatcatcaatgattttagagataataacttatatattatgttttttttcaatgataattgcattcgtcgataatactttcagcataaaaatatataatatcactgctatagtttgcttattgtcactaattttacgtggcagacaagaaaattataatataaaaaaccttattcttcccctttctatatttttaataggcttgcttgatttaatttggtattctgcgtttaaagtagataattcgccatttcgtgctacttaccatagttatttaaatactgccaaaatatttatatttggttcttttattgttttcttgacactaactagccagctaaaatcaaaaaaagagagtgtattatacactttgtattctctgtcatttctaattgctggatatgcaatgtatattaatagcattcatgaaaatgaccgcatttcttttggtgtaggaacggcaacaggagcagcatattcaacaatgctaatagggatagttagtggcgttgcgattctttatactaagaaaaatcatccttttttatttttattaaatagttgcgcggtactttatgttctggcgctaacacaaaccagagcaaccctactcctgttccctataatttgtgttgctgcattaatagcttattataataaatcacccaagaaattcacttcctctattgttctactaattgctatattagctagcattgttattatatttaataaaccaatacagaatcgctataatgaagcattaaatgacttaaacagttataccaatgctaatagtgttacttccctaggtgcaagactggcaatgtacgaaattggtttaaatatattcataaagtcacctttttcatttagatcagcagagtcacgcgctgaaagtatgaatttgttagttgcagaacacaataggctaagaggggcattggagttttctaacgtacatctacataatgagataattgaagcagggtcactgaaaggtctgatgggaattttttccacacttttcctctatttttcactattttatatagcatataaaaaacgagctttgggtttgttgatattaacgcttggcattgtggggattggactcagtgatgtgatcatatgggcacgcagcattccaattatcattatatccgctatagtcctcttactcgtcattaataatcgtaacaatacaattaattaagaataaacaagtttaagaagtgagttaaaactcacttcttatctatacaacttaatctctttactgaattagttaaagtttcagtatcgatatcttttaccgtatatgttggggatactatttgtatagatttatgatgattcggggaccaaattaaatgcgagggatattccggagtacgtgaattagggtaaaatgcaagcgttggtttatgataagccgcagcgatatgaacaagagctgtatcaacagaaatgacaaaatcactatacttggtcaacgcaacggtataaataaactcatcaaatggtagtgtttcgatttcaagtattggtattgtcaataaatcttgcggtaacccggtaaatataatccgataattttcaaagtgtgttttcacttcttgatatataacttttatttgctcaaacgtaagacggcatattttttttgcacctaatggattaataatgactattcttgtatctccaataaattcttttattttatcttcaacatctactggtaaatgcaagtcgtagttggtggaaaatttaccctcaccataaatatgcttcagtatttctattgctcgtgtactcatatgttcttttaaacattcatcgtggggatggtaaaatgaatagtaacgcttataccaatgatcaaaacccagaatgtaagaatcttttaaacttgataatattaagctatgcttaaatgagggcatagtttcaaaggggtctaatacaatatcgaactgtaaatcccgcagatgcttacatagagtaagcatttcaagaaaaccggttgattctttaatacagaactcaaatatatttttattattagagagaaattccccaccctttctatttgtgagaagagttattttaacccctttactataaagttcacgataaatcgaacttaatacaattagatcaccaagtttattattatcatgaataataaggcatgatttaacttgtgctggatctgtaatttgattatttattttattacgaaataaaaaagaaaggaaattaatcttgattttgtttatataaaatcttttctttttgtgaaaagttcctaagcgcatttttataccatattattttagtttcaggatgattaattagcataagaatcggttgaagttctatattgcattttttttcttgtcatatcttttgattcttctgcactgatgtcttgaagtttaataaatggaattacatcgtaagaaatagctgtatcatctgataaattataaatattaatatcttttacattatcatgcataaaacgaaaaaatggcaatattttgaataaatccctacttaattccgagggcatgggatttttattctcatcatagaaacgagaacagctacccgttaaatcaagaccagaacaaataatccgcgcatacttaagtgaatatgcgatttgaattgcagcaaaggcaatagtatggcatgagcaataaccaagactaatgtccttgcaaaatccaaccagacgaccttttttagacaacggtacagagatcagcagttctttgtgaatctgtctcaaaatattaaatttaatcttctttataaaaccacctttttcccgacggtaaaaggaccgtaatacgaggcagttctggaggatataaagtttatcttctttggaagcgtgttcataaacgtcaacgtttactatggtataacgacttctctggctaaatttataaaaatcatcacgacgctgatgtaaaaatcggacatctgtaagtacatatataaaaggaacgatattattacttaacagatattgcgcagaaccattgacagcaataatatcctttgttcgtaatactgacaaaggtgttttttgcgatgtagggcccgaaagaaaaataataacatcatcagatattttattttcaatcaggttttcaacatcttttttgtcaatgtatctaatattcttcatgataaacctgtgaaataaataactccgcttaaaactgtcctggtgaagacatgtaattgtgggattttttttagcgcgctggtttccctttcaaacgccgcataaaattgcgcatttttttacgatatactaaaagataatagcctagatctctaatctcatttttaataccgtaatgacgctctaagtcaatacgatctttcgctttacgctgcgctgaagcacgctttccggagagatcgataattcgaacctcaccattttttataatgaagttaccacgatgggggtcgccagaaaccatgccatgttgatgtaaggcattaattgattgctgaattttattttttagcgcatcatcaatatcgggcatatcacacaactctatgccatcaatatactcgatgatcatgatataagtatggacaaaacgtaaggttttccgttcagccaataaataaaagtcattgagtgtatttaacccttcatttcgtactttttgggtttgctcaaaaaggcgttcgtaataatcaccttttaacagagacttaaagaaacgttcgttacgcttaactttcggagaaaaaaccttaagaatcaatttaccgtaatcggtatcaataagcataacttttgtatcatcaatagaacgaaaaaccttgatgatatttatattataagacaagaagtcatttaatacattgaggtactttgaattgttttcatcggtaaaaacaaccaagtctttgatcttgctcttctgaatcataataaaccagttaaatgttatttacggtaatattttcggcaaagataacagactcctgctataattcctgagatataatgatgttgcactaaaagatgtttatatctttttttaaattcaataattgatttcgcatctcgtggagagtcatctttccagggggaattttctaaagctattttatagtattttaccgatggataaattgcccatttgtgccacggtttagttgcacctgtataatgaataagaagagtactttctgtaatcagctttttatagttttgatgtgttttgtcttttaattcacttttaattgtataaattgtattgtactcacgaggcaaaaataatgtcatccctttcagtaagacattcataacatcctgatcagggtatttataaacattatctttactcataagaatagacaacgctttttctgttagttttgcgtcagcccatttttttaagtctaaataaacgacaccggaattaaagtactgcccaagtaattcaggatcagacaacctggataccgccttttcttgcattggctcaacatctttaacaacagcagcaaccgctccatttaaacccagatgtaatagttggctaatatcgcctttacaaacaacatctgcatcaagataaagcaaacgatcaagcgttaaacccaataattgaaatgcaaataaacggaagtacattgctcttgaccagacctgtgtacaaggcaagcactggagcttatcagtgttaattctatataacgtgattcttaattggttttgctctgcaagctttgcaattttttgaaaaaaaccatcattataaacatcagcaataatataaaaatcaagattaatatgtcgattatttaggacaattgatgtgatggaaacacctacaccatcaagataattagcatcgacaccataggcaacatttaaacattcagaagtatttatattagctagccgaaaatcccaggctttaactttatctatctctatggcaggaaatgagtccacaatgctacccttatatcattactttatagtttcccagttttaatgctttatcttttcaataaaataaaaaagatagttgctaaatccttttagatatctatgctttttaagcatatgttttgcgctatatcttaattgattgctattgttcggtttcagcaacgccgtattcttccatggcgaagcattttttgcctccataaaggcttgtgatacaggataatcccaggcccaatcatgccagggcttggttggcccgatataatggataaaaatagtatcgttggttactgggtttataaagctttctttgagttgataatttaagctgaactgggtgttatatttaatatcagcgaaaataagtttatccgccagcaacatatttaacacatcctgatcaggatgtgttatttttttgattatttctggctcatttagcattgcaatagctcgtgcagaaacctgctgagccgcccattgggcagtattaatcaataaaaaaccggagttaaagtaacctttagcaattcccgcaacacctaacgaatgggcgcgtttttcccaccagtcagcttgcccttctgtaacaaccattgcgactttatcgtcaggaaatgagaaattaattagtggctcaatagtcccctgacaaatgatatctgcatccagataaaggactttaggcgccttattaataaagtaatctgcaataacaaaacgaaaatatattgcatgagtccaattcttagtgctaggcaatgagcgcagtcgatcaccattaatcagatatattttaattctggttttatactgcaacgccagggcatcaaaatacttacgatcatcatcaccaaaataatcagtaaaaatatggaaacacaatcgacttccttcattatattttaatattgaagcaatcgaaattccgcaaccaaatagaaagtttttgtcagttccataagcgatgtccagacaaagattttctgtttctactttatgatcataatcaataactgaattaagaaactcagtttcctggaaaaacacctgctgcattatttcctccgggaaatagcagaaataattaccttatgtaatctatcgtaatacttcgattggtaaaattcatcgatcgacgcaggaattttttcatgttcgatatgaatttcacctgctatatatttatttagaagagttacaaaaccagcaatatctcccggttgatacagatggccattgacatcaggttgaataatgtcagcaggcccggagacacaatcggcactgatacaaggaatcccccacgacaaggcttcaagtagggtcattgggaaaccttcaaaagatgacgtgagcaataacgcactcactttttcaatatcttgctggaccaattcccagggatattgttgccaaccataccagacaattcgatcatcaatatttaattctctaccataagcctggcatttttcgaaatcggagccatcacccaatacatggagtttccagttacctttcgcttgtgataagccatcaagcaggtctttaactcttttctggccttcaaatttcatacgcccaacataaataaacgttgccgtttcaccttcctcgggcgcgggaatgactgagtctttagtttcgacgggattaaaaataacatttatcgtcgattctgctacacctcgattaatcatttgctgtttaatgccagagctgattgctaaatgatagtcggcacaggtgatatattcagcatgttttttgtgatctaaagaaaaatgtggccatgaaaatactggcatatcaattcctgattttttacgtgcttttgcggcaaacaggcaggagatcacatcaatacaaataacgatatctggttggtactcctgaagccatttacttagagcatgaatatgtttcgcccgacgcaaaaaacctaaacgaatattggaaaatgaacatgagtatttaataccttccagccatcccttatccattttgtcattacgacaaaagaaaaacatttcactttggatatgttgttgcctgaaggtagtaataacatcacggatgacagtttccatgccgccaaatccagaaacagcttcgccgataaacgctattttcatagaaactctcattaattgagtaaaactcactgttttaacggttttatttgtctataaaatcagaaacaatcgttgacatcattttatctggactgaatttatataaactatcataatccattggtttaacagatgagttaataaaatactctaacttatcccaatcatcatgacctattataaaaaagcgagattcactatagatttctgaaccaaatacatttatattattagtaattaattttttattgaaaaatagtgcctcaagtatacgaagagtccagccagattggttttctttggttatatcaacaattatattagcatttaatgttcttctaatattctcttcataagatatttgtttttcaatcaaatactttgaagtcgtagatgatgtcttatctttgacaacattaaaatctagcttacatcctagtgttgttaatctctcggctaactcattaattatttgaagacgccctttatcacgaccaaggaaaaaacatattggctggctgttatttttgtcagataaactataatttctaatttcatccattcctataggaaaaaattgttctattgccttgatcttttcattccctataaatctatgctcaaaatcatatataatatcgaaataattcgcgttatcaagaataaaatcttcgccaacagtatttcttagaagcaaaactttatgacagttaatattttttaatatttgtttattgatacctttattaacaacactgtcattaatgataattatgtcatcttttttaatatcattgaggtaatgcttgatgaataatcgccccagccatgcattatccatccctatttttgatatttttttattaatccagttatatttttttggtgttgttatattttttatcttgtacttttttttcaggtactgaatcatttttaattcataatctgcaacccaatttataaaataaatagtcataataaagttagttccagtacatactaataaatatttttataatcctttgcgttgtgttcgctctttaatacgctcggccttaacgcttgccatgttcaataaattctgttcaagagacaatattttgcgtaaaggcatcccaaaataaaccttcataaatcgccagatatctctttgcgtcaggccaatattcattgatgagaaatataaaccaatcaggtctttatcgcgccagcggcgcggtacttttgcacgtatctgtgcccgatgcagatcgataactgaaatttttaattcatcttcccggccagtaaatggcaaatgaagcaaaaagtggcaaatgtaacagtcgcggtgatttatccctgcagtatgcattttacgcaccatagttgctacacgtgcgatcagcatacgcttaacacgtatatcaggcgggttgactgcccaatcggcacaataatcttcaaggctaattgtgggagtgagatcttcggtaataataaatgatgcgcgagttaatggatttaaccctttttcgccaaacccaatgcccttcattgtatcaacgccaacatcactcaggcgatgaatagcgtgccactctctgtctgcgcccaaaacgggcatccgcaatgagagtagattttttataatctcttttaatgtcgtccccttgtgccatttaagaaaatagcttttcccggacagttcaaagcgtaatgtacgacgagtctccagttcacgaaagacctcgccgttcagttttttgacctctgcaaaagcatctttaccacgccaaagtgtggcaagcggctcttttaattcaaccatctaaaccacctgtaatgatatccgcggctttttctggcaagctatacaaatcctgagtatcggcataatggcgagcattctccgcccaggccattcgcaatggcgactgagttaacgctttacgtaaaacttcatttaattgttcctgagagaaaggttcagcgatgaccgttccacaattggcatccgcaatataatgcgcgtacccacataccgctgttgttaaaacaggtaacccagcagtgatcgcttctagaagaacgatacccgcggcttcctgataagcgggatgcagtaataaatcagcggctgccattaattctgacacatcattgcgaccggagaagaaatgcacattgctccgcacgccgagtttttctgccagcgcttcaaattttcgcggcttatcctgaccaacaacaaataaaagcgtattgtgacgtaatgattccggtaacgatgccaaagcttcaattgagcgatctacacctttacggccaaaatctgatccaacctgcagtaataagttttgttgctcttttatgccatttttctggcgataaatttcacggctgtttgggatttgctcactgtattttctgtccggataaataccgggaggaagaatttgaaaacgttcaggttcagtttgataatgcttctggaaatcggcgatttgcttatcggtcagcatcataagtttcgtcgatttaccctgctcgaaagtcgctcgctcaaatgcggcataatggcgatatcgtgatgttaaacgatataaaaaacctttttcttgcgcaactttctcggcgtaacaaacatcagcggcaaaataaacatccaggccaggcatcttattaaacccaacaacgcgatctgcgggatgctctttgagatgattttgtacccaggcataatattctgcattgcgtccatggttggtatgggacttaactggcacctgaataagctcaaatgctttcgggcaatcgccttcccacgactgtgtatatacccgaacatggtggccccgtgcggcaactgttgatgcaatgcgcataaagtcacgttgaagcccaccaaatggaaaatatttatataaacaaaacgccacgatcataattgtgcattcctgtcagctgaaggggcatcttctggcaacagcttttccgtagcggcgatcacatcctccgctgggataacagaaagatattttttgttgcggtcaagttcatgccgggtcggcattttctgataattccccgcccagaattgaataatattctcggtccagggacgccagaatacgtgatccgttgcaccaaatagactaatgactggcgttttcactgccgctgcaatatgtcccggcgcagaatccacaccaataaaaagcactgcatgatcaattaatgcacccagttcaggaaaacgtgttttacctgcaaggccagtaatgggttttgtttcgcaacctcgtgcaatctcatctacacaagcgagatcatctgccgagggcccacaggttagcacaacctgatagcctcgctgttgcagcgcatcgataaccttagaaaatttatcgttatcccaacacttaaatatctgacgcgctgtcggttggatgacaacataatgatcttttacgcccagggcatctaattcccggcgcatcttcttccagcaatcttcggcgtaactcattgttgtgtcggtgtagaaatcggtaatacctaatggctcaaggaccgataaattacgctcaacaatatgtgtaccgtgtattggcgctaagtgtgtgaagctttttttccaaataccatgctgccgatgaccataaagttgcgatattttcatccgtgcaggtaaacaacgtaccagcagcgccaccatccactgatccgtaagattaatgaccaggtcataattattcgcacgcagagtttttatcaacgaaagcacatttttaattttatcgaaagttcccgcacctttattgcttatcccatagagcgcattaatttccgggttttcagacaaaatagggatggtgtcctgataaagcagcatatcgatttttgcatcaggataattctgcttgagcgtactgatgacaggagtagttaataacatatccccatgatatcgcatctttatgaccaggatttttcgaaatggcttttccactagcgactcttttgtgtgattgtctggttaagttaagcagaaaaaagcacgctaccgccccaggctcaacagctacctgaatactgataacgcacttactttgacgtgctagtgtatcatttctttcgcagcaatccgacccgaatgatttttatacacaaaatatactttaatcataaaaatcaaatagataaaaaatagcatttcgataatgtcagtacggcctatgtagatttgaaaatggggccgagtttcaatgaatcgcataaaaatacaaaaaaaatgaagatgtagcggcagatcagaccaaactgaagctatttaagtcaaaaacgggaaaagtaatggtaaagccacagctaaatacatagaatccccagcacatccataagtcagctatttactatgctcgaattgctttacaccgcccttctctaccttattcagccgctgatctggatacggctctgggtgcgcggacgtaaggctccggcctatcgaaaacgctggggtgaacgttacggtttttaccgccatccgctaaaaccaggcggcattatgctgcactccgtctccgtcggtgaaactctggcggcaatcccgttggtgcgcgcgctgcgtcatcgttatcctgatttaccgattaccgtaacaaccatgacgccaaccggttcggagcgcgtacaatcggctttcgggaaggatgttcagcacgtttatctgccgtatgatctgcccgatgcactcaaccgtttcctgaataaagtcgaccctaaactggtgttgattatggaaaccgaactatggcctaacctgattgcggcgctacataaacgtaaaattccgctggtgatcgctaacgcgcgactctctgcccgctcggccgcaggttatgccaaactgggtaaattcgtccgtcgcttgctgcgtcgtattacgctgattgctgcgcaaaatgaagaagatggtgcacgttttgtggcgctgggcgcaaaaaataatcaggtgaccgttaccggtagcctgaaattcgatatttctgtaacgccgcagttggctgctaaagccgtgacgctgcgccgccagtgggcaccacaccgcccggtatggattgccaccagcactcacgaaggcgaagagagtgtggtgatcgccgcacatcaggcattgttacagcaattcccgaatttattgctcatcctggtaccccgtcatccggaacgcttcccggatgcgattaaccttgtccgccaggctggactaagctatatcacacgctcttcaggggaagtcccctccaccagcacgcaggttgtggttggcgatacgatgggcgagttgatgttactgtatggcattgccgatctcgcctttgttggcggttcactggttgaacgtggtgggcataatccgctggaagctgccgcacacgctattccggtattgatggggccgcatacttttaactttaaagacatttgcgcgcggctggagcaggcaagcgggctgattaccgttaccgatgccactacgcttgcaaaagaggtttcctctttactcaccgacgccgattaccgtagtttctatggccgtcatgccgttgaagtactgtatcaaaaccagggcgcgctacagcgtctgcttcaactgctggaaccttacctgccaccgaaaacgcattgaggttgttatgcaaaaacgggcgatttatccgggtactttcgatcccattaccaatggtcatatcgatatcgtgacgcgcgccacgcagatgttcgatcacgttattctggcgattgccgccagccccagtaaaaaaccgatgtttaccctggaagagcgtgtggcactggcacagcaggcaaccgcgcatctggggaacgtggaagtggtcgggtttagtgatttaatggcgaacttcgcccgtaatcaacacgctacggtgctgattcgtggcctgcgtgcggtggcagattttgaatatgaaatgcagctggcgcatatgaatcgccacttaatgccggaactggaaagtgtgtttctgatgccgtcgaaagagtggtcgtttatctcttcatcgttggtgaaagaggtggcgcgccatcagggcgatgtcacccatttcctgccggagaatgtccatcaggcgctgatggcgaagttagcgtagcgtttatgccggatggtatgccatccggcgcgcatgaattacttctggcactgccgacaataaaacgttgcccgctgcgcatgtttagtcgccacaatcggcgtaccgcacacccgacacggctcaccttttcgcccgtaaacctgcaattcctgagcgaaatagcccggtttaccatcactttgcagaaaatctttcagcgttgtaccaccctgctcaatcgaacgcagcaacaccgctttaatcacccgagctaacaattcacactctgccagcgacagtgatgacgccagccgatccggatggatccccgccgcaaacagtgattcgctggcatagatattccctacccctaccaccagcttgttatccatcagccacggtttaatcgccgtttttttcttcgcgcacttctgatgcagatactcaccattgaaatcgtcgctaagcggctccggtccaagatgggtcagcacattatgcccttccagctctttggtccacagccaggcaccaaagcggcgcggatcggtgtagcgcagcactttgccgttgctcatcaccaaatccacatggtcatgcttttcagggggaagttcttctggaaggatgcgcaggctgccagacatccctaaatgaatgataatccagccctcaggcagctccagcagcagatatttagcccgccgctgcacgctaagcactggttggtcgcttaaacggtagatctcttctgaaaccggccagcgcaagcgtccgttgcgcaccactgcatgaagaatggttgcaccaacgagatgcggttctatgccgcggcggctggtttcaacttcgggtaattcaggcatagcatctccaggaatgaacagatgcagtcaatatgggggcaagcagataacaaaaaaccccgccggagcgaggttttttgttacatcaaagcgagaattatttgattttcgcttctttgtagatcacgtgctggcgaacaactggatcgaattttttcagttccagtttttccggcttagtacgtttgttcttcgtagtggtatagaagtgaccagtaccagcagaagaaaccagcttgattttctcacgaatacctttagccatgatttatttcctctaagtacttagtacttttcgccacgggcacgcagttcagccagaactgtatcgatgccttttttatcgattacacgcatacctttagcagatacgcgcagggtgacaaaacgcttctcgctctcaacccagaaacggtgagagtgcaggttcggcaggaaacggcgtttagtcgcgttcagtgcgtgggaacggttgttaccggtcaccggacgcttgccagtaacttggcagactcgggacatgtctattctccaaaaatcaaattagctcgagcttcgtatggggtattggcgcctcgtcaggctttacagcccggtcatcgcagttctatgtgaactctcgattgccaggcccaaatgccaaacccgagattctcaaaggtggcgtagtatacgctgactcagcgatgtgctcaagtcccgaacagacaaagatcccgaaggatcgcgcatagcgggttaaatccagccgcgttcggcaaaagaaacatactctccacgcccaatcacgatatggtcgagcacgcgtaaatccatgaactgacaactctttattatccgttcagtaatgagtttatccgctttactgggttcagcacaacccgaagggtgattatgtgcaaggatcagcgccgaggcgtttatttttatcgcttcgcggataatttcccgaggatggacttcaacatggtttagcgtgccggaaaaaagacgcctatgcgttataacccggtgttgggagtcgagaaagatcaccataaagatctcccgctcctcacccgtgagctggctttgtaaaaattccctcgtcatctccgggctgagtaaagggctttcttcacgcatccgcacgttgtagtaacgccgcgccagttcagcaatcccctttaactgggcaaatttcgccacgccaattccatgaacgccactaaattgttcatattcagaggttaacaagccataaagagagccgaaattctccagcatctcttttgccagggttaatacatctttaccgcgcgttccggtacgcagaaatagcgccagcagctcgacatccgttaaggcgctaataccaaacttcagcattttttcgcgcggcatcaacagctgtgaattgtttttcaccttcacctcctttgtggtgctcgcatcctgtcatagccgtttcgttaaatcgacggccagttttcaatcctggaaagcgcctcgcaaagtgaatctcaggtgaaggcacgacaacaaaagtattgtgataaaatcgccaacttctggtgtcaccctacaggaaaaatcatcatgagcctggccggtaaaaaaatcgttctcggcgttagcggcggtattgctgcctataaaacccctgaactggtgcgtcgtttgcgcgatcgcggggccgacgtccgcgtagccatgaccgaagcggcaaaagcctttatcaccccacttagcttgcaggcggtttctggttatcccgtttccgacagtctgctggacccggcagccgaagccgctatgggccatattgagctgggtaaatgggctgatttagtgattctcgcccctgccacggcagatttgattgcccgtgttgctgccggaatggcgaatgacctggtatcgacgatttgtctggctacacctgcgcctgtagccgtgctccccgccatgaaccagcagatgtaccgtgccgctgccacgcagcataatttagaggtgcttgcttcccgtggtttgctcatctgggggccagacagtggcagtcaggcttgtggtgatatcggtcctgggcgaatgctcgatccgttaaccattgtggatatggcggtagcgcatttttcgcccgtcaacgacctgaaacatctgaacattatgattaccgccggcccgacgcgtgaaccgctcgatccggtgcgttatatctctaatcacagctccggcaagatgggttttgctatcgccgccgccgctgcccgtcgtggcgcgaacgtcacgctggtatcaggtccggtttcactaccgacgccaccgtttgttaaacgtgttgatgtgatgaccgcgctggaaatggaagccgccgtgaatgcttctgtacagcagcaaaatatttttatcggctgcgccgccgtggcggattatcgcgcagctaccgtggccccagagaaaatcaaaaagcaggccacgcagggtgatgaattaacaataaaaatggttaaaaaccccgatatcgtcgcaggcgttgccgcactaaaagaccatcgaccctacgtcgttggatttgccgccgaaacaaataatgtggaagaatacgcccggcaaaaacgtatccgtaaaaaccttgatctgatctgcgcgaacgatgtttcccagccaactcaaggatttaacagcgacaacaacgcattacaccttttctggcaggacggagataaagtcttaccgcttgagcgcaaagagctccttggccaattattactcgacgagatcgtgacccgttatgatgaaaaaaatcgacgttaagattctggacccgcgcgttgggaaggaatttccgctcccgacttatgccacctctggctctgccggacttgacctgcgtgcctgtctcaacgacgccgtagaactggctccgggtgacactacgctggttccgaccgggctggcgattcatattgccgatccttcactggcggcaatgatgctgccgcgctccggattgggacataagcacggtatcgtgcttggtaacctggtaggattgatcgattctgactatcagggccagttgatgatttccgtgtggaaccgtggtcaggacagcttcaccattcaacctggcgaacgcatcgcccagatgatttttgttccggtagtacaggctgaatttaatctggtggaagatttcgacgccaccgaccgcggtgaaggcggctttggtcactctggtcgtcagtaacacatacgcatccgaataacgtcataacatagccgcaaacatttcgtttgcggtcatagcgtgggtgccgcctggcaagtgcttattttcaggggtattttgtaacatggcagaaaaacaaactgcgaaaaggaaccgtcgcgaggaaatacttcagtctctggcgctgatgctggaatccagcgatggaagccaacgtatcacgacggcaaaactggccgcctctgtcggcgtttccgaagcggcactgtatcgccacttccccagtaagacccgcatgttcgatagcctgattgagtttatcgaagatagcctgattactcgcatcaacctgattctgaaagatgagaaagacaccacagcgcgcctgcgtctgattgtgttgctgcttctcggttttggtgagcgtaatcctggcctgacccgcatcctcactggtcatgcgctaatgtttgaacaggatcgcctgcaagggcgcatcaaccagctgttcgagcgtattgaagcgcagctgcgccaggtattgcgtgaaaagagaatgcgtgagggtgaaggttacaccaccgatgaaaccctgctggcaagccagatcctggccttctgtgaaggtatgctgtcacgttttgtccgcagcgaatttaaataccgcccgacggatgattttgacgcccgctggccgctaattgcggcacagttgcagtaatatgacgccggatgacttttcatccggcgagtttctttaaacgccaaactcttcgcgataggccttaaccgccgccagatgttccgccatttccggcttctcttccaggtaagcaatcaggtctttcagggtgatgatagagatcactttgcagttgtaatcacgctcaacttcctgaatcgccgaaatctcgccgcgcccgcgttcctgacgatcgagcgaaatcaacacgccagcaagcgtcgcgccattggcctgaataatctccatcgactcgcgaatcgccgttccggcggtgatcacatcatctaccagcattacgcgtccttgtaacgcgctaccaaccagattgccgccttcaccgtggtcttttgcttctttgcggttaaagcagtacggcaggtccaggtcgtgatgctccgccagtgccacagcggttgtggtggcaatcgggatccctttgtaagcagggccaaacagcagatcgaactcaatgccggaatccaccaacgcttcagcgtaaaaacggcctaacagtgccagatcgcgcccggtattaaacagcccggcgttgaagaaataggggcttttgcgcccggatttcagcgtaaactcgccaaactttaacacctgcttgctaagcgcaaattcaataaactggcgctgatatggtttcatgccttcgctcctcatcttacttttctacagacaaaaaaaaggcgactcatcagtcgccttaaaaatcagtttgccagcgccgccttctgcgtcgctacaatggattcgattcccctcgggccagagccaacaagatgagtagctcttcatgggtgaacggctcgccttctgccgtcccctgcacttcaatgatgcgcccgtcttcggtcatcactacgttcatgtcggtctctgcggcagagtcttcaacgtattccagatcgcaaaccgcttcgccgttcacaattccgacagaaactgcggctaccatccctttcatcggattggttttcagcttgccgttttccaccagcttctgtagcgcatctaccagcgccacgcaggcacccgtaatcgacgcggtacgcgtgccaccatcagcctgaagcacgtcgcagtccagcgtaatggtgaactcacccagcgctttcaaatctactgccgcgcgaagagcacgggcgatcagacgctggatttccattgtgcgtccaccctgcttacctttcgccgcttcacgagcgttacgggtgtgggtagaacgtggcagcatgccgtactctgcggtgatccagccctggccctgacctttcaggaagcgcggcacgccttcttcaatagaggcggtacacaacactttggtatcgccaaattcgaccagcaccgagccttctgcatgttttgtatagttacgagtcagggtaacgggacgcacctgattattgctacggcctgctggacgcatattgaaatctccggcttgaaacaaatgtggctgcgcattatacggacttccggcggttattcctatcctgacaaggcatcgatggctataatccttccacctctccttttataaacaggaacgtctatgatccgcagtatgaccgcctacgcccggcgtgaaatcaagggtgaatgggggagcgcaacctgggaaatgcgctcggtaaaccagcgttatctggaaacttactttcgtctgccggagcagttccgtagccttgaacctgtcgttcgcgagcgtattcgttctcgcctgacgcgcggtaaagtggaatgtaccctgcgctatgagccagatgttagcgcgcaaggtgagctgatcctcaacgaaaaactggctaaacagctggtaactgccgcgaactgggtaaaaatgcagagtgacgaaggggaaatcaacccggttgatattctacgctggccgggcgtgatggcagcccaggagcaggatcttgacgccattgccgctgaaattctcgcggcgctggatggtacgctggacgactttattgtcgcgcgcgaaaccgaaggtcaggcactgaaagcattgatcgagcagcgtctggaaggcgtcaccgccgaagtggtcaaagtccgctcccatatgccggaaatcctgcaatggcagcgtgagcgtctggtcgcgaagctggaagatgctcaggtgcaactggaaaacaaccgtctggagcaggaactggttctgctggcacaacgaattgacgttgccgaagaactggatcgcctcgaagcgcatgtcaaagagacctacaacattctgaagaaaaaagaagcggttggtcgtcgtctggattttatgatgcaggagttcaaccgcgagtcgaacactcttgcgtcgaagtctatcaatgccgaagtgacaaactccgccatcgagctgaaagtgttgattgagcagatgcgcgagcagattcagaacatcgaataactcgtaacgccaattcttacttttccgccttcacaaatgccgccactcaaacagagcggcatttttcttccccgcaacattcaattctgttttgcgtgcctgctccagattttgcgatgtttttttgcccagcacactgagaacgtgagatactcacaactgtatataaatacagttacagatttactttctttgcaattgatatcacatggagtgggcaatgaacgaacatcatcaaccttttgaagagataaaactgattaatgcaaacggagcagaacaatggtcagcaagacaacttgggaaactactgggttattcagagtatcgtcactttatacctgtattaacgcgcgccaaagaagcctgtgagaacagtggtcacacaattgatgaccatttcgaggagatcctcgatatggtcaaaattggctcaaatgccaaaagagcattaaaagacatcgtactctcccgctatgcctgttacctggtagtacaaaacggcgaccctgcgaaaccggtcattgcggcagggcagacttattttgctatccagacccgacggcaggagcttgctgacgatgaagcatttaagcaacttcgtgaagacgaaaagcgtctgtttctgagaaatgagttgaaagaacataacaaacaattggttgaggcagcacagcaagctggggtagcgacagctactgatttcgccatatttcagaatcatggttaccaggggctgtatggtggattagatcagaaagctattcatcagcggaaggggctgaaaaagaatcagaagatcctggatcatatgggttcaacagaactggcggctaatctctttcgagctacccaaacagaagaaaaactcaagcgggatggcgtgaattcaaaacagcaagcaaacaccacacactttgacgtgggtcgcaaggtgaggcaaaccattcaggaacttggcggaaccatgcctgaggagttgccgaccccgcaggtcagcatcaagcagttggaaaacagtgtaaaaattacagagaagaaatagcagaaactaaaaactctttttgttgattgagacacccgatgcgtaagccaaggtccaggtgcagtgaacacaatggctaaatattgcacctttcttttccccctcagttttaacctattttttcttatgcattttctcagacaagaagtcagaagaatgcatctctgctacagaaaatagcgatttcacataactacaagttatcaatttcccctccccttaaaaaatctcaatcgtgacaatgcgcacaaatcgctaccctgccagacagatttttagggagagaaccatgctgttacacattttgtatttggttggcattactgccgaagccatgacgggggcgctggcggccggacgacggcgcatggatacatttggcgtaattattattgcgaccgccaccgcaattggcggagggtcagtgcgcgatattctgctgggccactatccgctcggctgggtcaaacacccggaatatgtgattatcgtcgctaccgccgcagtactcaccactatcgttgctcctgtaatgccttacctgcgcaaagtgtttctggtgctcgatgcgctcggactggtggtcttttctatcatcggggcacaggttgcactggatatggggcacggcccaattattgccgttgtcgcggcggtaaccaccggcgtgtttggcggcgttttgcgcgatatgttctgtaaacgtatcccactggtattccagaaagagttgtatgccggtgtctcatttgcctccgccgtgctgtacatcgcgctgcaacactatgtttctaaccatgatgtggtaattatctccaccctggtattcggcttttttgcccgcttactggcgctacgccttaagctgggattaccggtcttttactacagccacgaaggacactaaggttcaaaacctgtgatctgctgggcagccagccaactgcccagcttcttgatttgcgcattttccttccattcaataacctgtctggcgcgtcccgatccagtccccggcagctgctgccagaactgctccgtgctaaataaaagttgcgaccaggaccgttcatcactggcattaagcgccgcccgggttagcggtattcccattgccatcacccagcgagtaaaaggctgcttacgagccagattaaactgatgccatagctgcgcacttttacttttcgcgatccccggcgtgttctgtaattgctctggcgttaataaaagccaggaaaagatatgttcaaagcgatgagtctgatgcagcgcgcgccaaccggcctcaccaatgccatccagcccaagaacctgttttgcccccagccagactaagcgtgaaatgaactgttcctgacaaacatcagaagcaaagtagcaggtcaacgagttaaagcggttttctggcggtgtcggttttgtacgttctgcaccgcgccacaccacatcatcaatgcgaggaataccctgaccggcaaggctgacgagaatctgatcaccaggcgcaatatcccactcctgccagcgcctgacggaaccaatattcacccgctggacttttttatcatccagcatgacaggtgcgagtgacgcaaccaccgatattttaccgctcttacccaccgcaaactgaattgccttcacttcggcaacctgagctacaggttgatatttccaggccaccagccactctgcctggcccggtagccaatggcgggattctggctctttcgccgctcgtacaactacgccatcggtgacgaagggtaattccgctttccaccactcattgcgtacgcgcgcaacttcatcagcatttttcaccgcacgggtatacgtctgcgttagagtaaaacctgcggtagccagctcttttaaacgatcagacattaactgcggtccatccggccatgcccagacaaaaacgcccagagaattcagcgtgtcgctatcgtcctggcgcatcatcaagccagcaacttttgcgcgggcatttattccccccatttgttgttggatatgcccctcgcgctggagaaatatttccccctgaagcgtactgttggctaaaggcccgctaacggtttgcggcacagcggaaattaagctaactttctgcgtccagtcctcgcctttcaggccattaccgcgactgattgctttgttcagtttcccgtcccgataaaccagggttaccgcaacgccatcaacttttggctgcacccaaagatcgctacgttctcgcatccacagacttaatgcgtttttatccaccattttgcgtacacccgtatgggcaaccggatgcataaccgcaccatttaaaggcggcatcatcacgtcgcggggctcgctcccaaagcagcgttgccactgcgtaagacgggcgcttaactgatcgtaaacaccgtcttccacctcactttttccttccttccagtagtcatcgtcccactgttttatttgctgttgcaggcgggaaatttcttcctgtgctctggctggcgaccaggccggacagaccgcccacacagatgattgccagcacaagatacctattaatatcgccatccatactttcatcatcacctccgctgtagatagtcaggcagatatacaacgtgatgaaagcaaagccgagtggcaaaaacggagtctgcgaggacgcttcctgaaaatcgtctttattgcagtgaatgacaggcaaatgcggaagcagctacgcaaaacgcaacaactttgcgcaaaaagtgtgagcaagggctacgtcacatggccgcgccgtgtataataagctcgtatgtaggctttatttcgctaatcacatacgaaagatactcatggctcaaggcacgctttatattgtttctgcccccagtggcgcgggtaaatccagcctgattcaggctttattaaaaacccaaccgttgtatgacacccaggtttctgtttcacacaccacacgccaaccgcgtcctggtgaagtccacggtgaacattatttctttgttaatcatgatgaatttaaagaaatgattagcagagatgcgttcctcgaacacgcagaagtttttggtaattactatggcacttcgcgtgaggccattgagcaagtactggcgaccggtgtcgatgtttttctcgatatcgactggcagggcgcgcagcaaattcgccagaagatgccgcacgcgcggagtatctttattttaccgccgtccaaaattgaactggaccgccgtctacgcggtcgcggtcaggacagcgaagaggtcattgcaaagcgtatggcgcaagctgttgcagaaatgagccattacgccgaatatgattatctgattgtgaatgatgacttcgataccgcgttgaccgatttgaagaccattattcgcgccgaacgtctgcgcatgagccgccaaaagcagcgtcatgacgctttaatcagcaaattgttggcagactgaacctgatttcagtatcatgcccagtcatttcttcacctgtggagctttttaagtatggcacgcgtaactgttcaggacgctgtagagaaaattggtaaccgttttgacctggtactggtcgccgcgcgtcgcgctcgtcagatgcaggtaggcggaaaggatccgctggtaccggaagaaaacgataaaaccactgtaatcgcgctgcgcgaaatcgaagaaggtctgatcaacaaccagatcctcgacgttcgcgaacgccaggaacagcaagagcaggaagccgctgaattacaagccgttaccgctattgctgaaggtcgtcgttaatcacaaagcgggtcgcccttgtatctgtttgaaagcctgaatcaactgattcaaacctacctgccggaagaccaaatcaagcgtctgcggcaggcgtatctcgttgcacgtgatgctcacgaggggcaaacacgttcaagcggtgaaccctatatcacgcacccggtagcggttgcctgcattctggccgagatgaaactcgactatgaaacgctgatggcggcgctgctgcatgacgtgattgaagatactcccgccacctaccaggatatggaacagctttttggtaaaagcgtcgccgagctggtagagggggtgtcgaaacttgataaactcaagttccgcgataagaaagaggcgcaggccgaaaactttcgcaagatgattatggcgatggtgcaggatatccgcgtcatcctcatcaaacttgccgaccgtacccacaacatgcgcacgctgggctcacttcgcccggacaaacgtcgccgcatcgcccgtgaaactctcgaaatttatagcccgctggcgcaccgtttaggtatccaccacattaaaaccgaactcgaagagctgggttttgaggcgctgtatcccaaccgttatcgcgtaatcaaagaagtggtgaaagccgcgcgcggcaaccgtaaagagatgatccagaagattctttctgaaatcgaagggcgtttgcaggaagcgggaataccgtgccgcgtcagtggtcgcgagaagcatctttattcgatttactgcaaaatggtgctcaaagagcagcgttttcactcgatcatggacatctacgctttccgcgtgatcgtcaatgattctgacacctgttatcgcgtgctgggccagatgcacagcctgtacaagccgcgtccgggccgcgtgaaagactatatcgccattccaaaagcgaacggctatcagtctttgcacacctcgatgatcggcccgcacggtgtgccggttgaggtccagatccgtaccgaagatatggaccagatggcggagatgggtgttgccgcgcactgggcttataaagagcacggcgaaaccagtactaccgcacaaatccgcgcccagcgctggatgcaaagcctgctggagctgcaacagagcgccggtagttcgtttgaatttatcgagagcgttaaatccgatctcttcccggatgagatttacgttttcacaccggaagggcgcattgtcgagctgcctgccggtgcaacgcccgtcgacttcgcttatgcagtgcataccgatatcggtcatgcctgcgtgggcgcacgcgttgaccgccagccttacccgctgtcgcagccgcttaccagcggtcaaaccgttgaaatcattaccgctccgggcgctcgcccgaatgccgcttggctgaactttgtcgttagctcgaaagcgcgcgccaaaattcgtcagttgctgaaaaacctcaagcgtgatgattctgtaagcctgggccgtcgtctgctcaaccatgctttgggtggtagccgtaagctgaatgaaatcccgcaggaaaatattcagcgcgagctggatcgcatgaagctggcaacgcttgacgatctgctggcagaaatcggacttggtaacgcaatgagcgtggtggtcgcgaaaaatctgcaacatggggacgcctccattccaccggcaacccaaagccacggacatctgcccattaaaggtgccgatggcgtgctgatcacctttgcgaaatgctgccgccctattcctggcgacccgattatcgcccacgtcagccccggtaaaggtctggtgatccaccatgaatcctgccgtaatatccgtggctaccagaaagagccagagaagtttatggctgtggaatgggataaagagacggcgcaggagttcatcaccgaaatcaaggtggagatgttcaatcatcagggtgcgctggcaaacctgacggcggcaattaacaccacgacttcgaatattcaaagtttgaatacggaagagaaagatggtcgcgtctacagcgcctttattcgtctgaccgctcgtgaccgtgtgcatctggcgaatatcatgcgcaaaatccgcgtgatgccagacgtgattaaagtcacccgaaaccgaaattaatgttttatgaacccaacacgttatgcacgcatctgcgaaatgctcgccaggcggcagcctgatctgaccgtctgcatggagcaggtccacaaacctcataacgtttctgcgattattcgtaccgcagatgccgttggcgtacatgaagttcacgccgtctggcctggtagccgcatgcgcaccatggcttcggcagcggcgggtagtaacagctgggtacaggtgaaaacacaccgcaccattggcgatgccgtcgctcatctcaaaggccagggcatgcagattctggcaacccatctttctgataacgctgtcgatttccgcgaaattgattacactcgcccgacctgcattttgatgggacaggagaaaacgggcatcacgcaggaagcattggccctggcggatcaggacatcatcattccgatgatcggcatggtgcagtcgctgaatgtttccgttgcctcagccctcattctttacgaagcccagcgtcagcggcaaaatgcaggcatgtacctgcgtgaaaacagcatgttgccggaagcagagcaacaacgcctgttgtttgaaggcggctatccggtgctggcgaaagtcgcaaaacgcaaaggcctgccttatccccacgtcaatcagcaaggcgagatcgaagctgatgccgactggtgggctactatgcaggctgcagggtaagtgccatgaaaggtcgcctgttagatgctgtcccactcagttccctaacgggcgttggcgcagcacttagtaacaaactggcgaaaatcaacctgcataccgtgcaggatctactcttacaccttcccctgcgctacgaagatcgcacccatctctaccccatcggagaactactgccgggcgtttatgccacggtggaaggcgaagtgctgaactgcaatatctccttcggcggtcggcggatgatgacctgccagatcagcgacggttccggcatcctcaccatgcgctttttcaatttcagcgcggcaatgaaaaatagcctggcggcgggccgccgtgtactggcttatggcgaagcaaagcgcggtaaatatggtgcggagatgatccacccggaataccgcgtgcagggcgatctcagcacgccagaattacaggaaacgctcacgccggtttatccaacaacggaaggcgtaaagcaggccacgctgcgtaaattaaccgaccaggcgctggatctgctcgacacctgcgccattgaagaactcctgccgccggaactgtcacaaggaatgatgacgctaccggaagcgttgcgcactttgcaccgcccgccaccgacgctacagcttagcgatctggaaaccgggcagcatccggcgcaacgtcgtctgattctggaagaactgctggcgcacaacctcagcatgttagccttacgtgccggagcacagcgttttcatgcccagccgctgagcgccaatgacacgctgaaaaataaactcctcgccgccttaccgttcaagccaacgggcgcacaggcacgcgtagtggcggagatcgagcgcgatatggcgctggatgtgccgatgatgcgtctggtgcagggcgatgtaggttccggtaaaacgctggtcgccgccctcgccgcgttgcgtgcgattgcccacggcaaacaggtagcattgatggcaccaaccgaattactcgccgagcagcacgccaataacttccgcaactggtttgcaccgctcggtatcgaagtgggctggctcgccggtaagcagaaaggtaaagcacggctggcacagcaggaagccatcgccagcggtcaggtgcagatgattgtcggtacacacgccatcttccaggaacaggtgcagtttaacggcctggcgctggtgattatcgacgaacagcatcgttttggcgtgcatcagcgtctggcattgtgggagaaaggccagcagcagggcttccatccgcatcagttgatcatgaccgccacgccgatcccccgcacgctggcaatgactgcgtatgccgatctcgatacctcggtgatagatgagctgccgccaggccgcacgccagtgactacggtcgctattcctgatacccgccgtaccgacatcattgaccgcgtgcaccacgcctgcataactgaaggtcgtcaggcatactgggtttgtacgttgattgaagagtcggaattgctggaagcgcaggcggcggaagctacctgggaagagttgaaactggcgctaccagagttgaacgttggcctggtacacgggcggatgaaacctgccgagaaacaggcggtgatggcgtcgtttaaacaaggtgagctacacctgctggttgccacaaccgttattgaagtcggcgttgatgtgcctaacgccagtctgatgattatcgaaaacccggagcgtctgggtctggcgcagttacaccagctgcgcgggcgcgtaggtcgtggcgcggtggcttctcactgcgtgctgctctacaaaacgccgctttctaaaacggcgcaaattcgcctgcaagtgctgcgcgacagtaacgacggttttgtgattgcgcaaaaagatctggagattcgcggccctggcgaattgttaggcacgcgtcagacgggtaatgctgaatttaaagtggcggatttactgcgcgatcaggcgatgatcccggaagttcagcgcctggcacgccatattcacgaacgttacccacaacaggcaaaagccctgatagaacgctggatgccggagacggaacgttactcgaatgcgtaaaaggcggcagtgagaagaccgccatttcaggttaccctaccttcctgccggatgcgattcatcaccctacaaattcaataaattatgaatcaatacgcaggcttgataagcgaagcgtatcaggcatttgtctttgttgcggcggcacttctaccgccgcttcatcggttaaccggcaaaaatcggcaacatcaaatacaacttaattaccagcgcattgacgatatcgataaagaacgcaccgaccatcggcaccaccaaaaacgccatgtgcgacgggccaaagcgttcagtgatcgcctgcatgttggcgattgccgttggcgttgcaccgaggccaaaaccacagtgacccgcagccagcactgccgcatcgtagtttttgcccatcatgcgccaggtaacgaagatggcatacaacgccatgaagatggtctgtaccaccagaatcgccagcatcggcagcgccagcgaagccagctcccacagtttcagccccatcaacgccatcgccaggaacaacgacaagcttacgttacccagcacggataccgcacgctcaaagacgcggtaaaagcccattattgacagaccgttgctcagaatcacgccaacaaacagtacacagacgaaggtcggcagttcaaaagcagtgccagccaaaagttgcgcaacaattttccccaccgtcaggcagatagcaatcagcgcgatagtttcaatcagcaccaacgaggtgatcatgcgtcccacatccggcttttcaaacgccgtcgggacttcctggtcatccggaataccgttcggcgtggtggagtgtttcaccagatagcgcgccaccggaccgccaatcaagccgcccagcaccagaccgaacgttgcacaggccatcgccacttccgtcgcattggtgaagccataacgttcaatgaacaatttactccacgcagcgcccgtaccgtgaccgccggaaagagtaatagaaccggccaacagccccatcagcggatcaagccctaacaagctagccataccaatgccaatggcattttgcatcaccaacagaccaacaaccacaatcaagaagatgccaaccacacgcccaccggcacgcaaactggcaatgttggcgttcaggccaatggtggcgaagaaagccagcattaacggatcgcgcagggacatatcaaagttgacttcccagcccatgctttttttcagtactagtagcgccagcgccaccaacaaaccacccgcaacaggttccggtatggtgtatttcttcaaaaaggagacggaatggaccaacttacgcccgagcagcaacgtcagcgttgcggcaacaagcgttgctaaagtatcgagatgaaacatagttactcctttgtatccgcatcactctttcatactcgtcatacttcatcgcgcagtggcaacttcatgaactatgacgggtatcgagttatgctttcctgggtcaaattctcagctgttaatgaacaaatggcatggattttaagcagaaaaataccaaaagttatataaaaaagtgcatttatctcatttaaatatttagatgaggatgtggcaaacgtttgcttttctctttcggtcagctaaaatgcccgctttgctaccacgggattgttttcgatgtctgtttccaccctcgagtcagaaaatgcgcaaccggttgcgcagactcaaaacagcgaactgatttaccgtcttgaagatcgtccgccgcttcctcaaaccctgtttgccgcctgtcagcatctgctggcgatgttcgttgcggtgatcacgccagcgctattaatctgccaggcgctgggtttaccggcacaagacacgcaacacattattagtatgtcgctgtttgcctccggtgtggcatcgattattcaaattaaggcctggggtccggttggctccgggctgttgtctattcagggcaccagcttcaactttgttgccccgctgattatgggcggtaccgcgctgaaaaccggtggtgctgatgttcctaccatgatggcggctttgttcggcacgttgatgctggcaagttgcaccgagatggtgatctcccgcgttctgcatctggcgcgccgcattattacgccgctggtttctggcgttgtggtgatgattatcggcctgtcgctaattcaggttgggttaacgtccattggcggcggttacgcagccatgagcgataacaccttcggcgcaccgaaaaatctgctgctggcaggcgtggtcttagccttaattatcctgcttaaccgtcaacgtaacccttacttacgcgtggcctcactggtaattgcgatggcggccggatatgcgctggcgtggtttatgggcatgttgccagaaagcaacgaacctatgacgcaagaactgattatggtgccaacgccgctctattacggtcttggcattgaatggagtctgctgctgccgctgatgctggtctttatgatcacttcgctggaaaccattggcgatatcacggcgacctctgacgtttccgaacagccagtgtccggtccgctgtacatgaaacgcctgaaaggcggcgtgctggcaaacggcctgaactcgtttgtttcggcggtgtttaacaccttcccgaactcctgcttcgggcaaaacaacggagtgatccagttgactggtgttgccagccgctatgtcggttttgtcgtcgcgctgatgttgatcgtgctgggtctgttcccggcagtgagcggttttgtacaacacattccagaaccggttctgggcggcgcaacgcttgtaatgtttggcaccatcgccgcctccggtgtgcgtatcgtttctcgtgagccgctgaaccgtcgggcgattctgattatcgcgctgtcgctggcggttggtctgggcgtgtctcagcagccgctgattttgcagtttgcccctgaatggctgaaaaacctgctctcctccgggatcgccgcgggcggtattactgccatcgtgctgaatctgattttcccaccagaaaaacagtaattcactggcggcggtaagataattaccgccgcagtctcacctctttaaccattcccgccttgaggattgcgcgtaaatcgtgcataactcccttatgtgcatttcacgggatggaagaccatgaaatttattgggaagctgcttctctacattctcatcgctctgttagtggcgatcgctggcctctattttcttctgcaaacccgctggggagcagaacatatcagcgcatgggtttccgagaatagcgactatcatctggccttcggggcgatggatcaccgtttttccgcgccatctcatatcgtgctggagaacgtcacgtttggtcgtgatggccagcccgcgaccctggtggccaaaagtgtcgacattgcgctaagcagtcggcaactgaccgaaccacgccatgtcgataccatcctgctggaaaacgggacgctgaatctcaccgaccagaccgcgccgctaccgttcaaagccgatcgtctgcaactgcgtgatatggcgtttaatagcccgaatagcgaatggaaactgagcgcgcagcgggtaaatggcggcgtagttccgtggtcaccaaaagccggtaaagtgctgggtacgaaggcgcagattcagtttagtgccggatcgctttcgctcaatgatgttcctgccaccaatgtactgattgaaggcagtattgataacgatcgcgttacgctgactaacctgggtgccgacatcgcccgcgggacattaaccggaaacgcgcagcgtaacgccgacggcagctggcaagtggaaaacctgcgcatggcggatatacgtctacaaagcgaaaaatcgctaaccgacttctttgcgccattacgctctgtcccgtcgttgcagattggtcgcctggaagtgatcgatgctcgtttgcaaggtccggactgggcggtgaccgacctcgatctcagcttgcgcaacatgaccttcagtaaagatgactggcagacacaggaaggcaaactgtcgatgaacgctagcgagttcatttatggttcgctgcatttatttgacccgattataaacacggaattttccccgcagggcgtagcgctgcgccagttcaccagccgctgggaagggggtatggtcagaacgtcagggaactggctgcgtgacgggaaaacgttgatccttgatgatgcggcaattgccgggctggaatataccttgccgaaaaactggcaacagttgtggatggaaacgacacccggttggttaaacagcctgcaactgaagagatttagcgccagccgcaatctgatcattgatatcgaccctgacttcccgtggcagctcaccgcgctcgatggttacggtgccaacctgacgctggttaccgatcataaatggggcgtctggagtggctcggcgaatctgaatgccgccgccgcgacattcaatcgtgttgatgttcgtcgcccgtcgctggcgctgaccgccaacagcagcacggtgaatatcagcgaactgagtgcatttactgaaaaaggcattctggaagccaccgccagtgtttcacaaacgccacaacgtcagacacatatcagcctgaatggacgcggtgtgccggtgaatattttgcaacagtggggatggcctgaattaccgttgactggcgacggcaatattcagcttaccgccagtggcgatattcaggccaatgtcccgttgaaacctacggttagcgggcaattgcatgccgtgaacgccgcaaagcagcaagtgactcaaaccatgaatgctggcatcgtttccagcggtgaagttacatcgacggagccggtgcggtaaacatcaatctcgccgggtacgactcagacgtacccggcattccatcaatagattacaacgtaattgtcagcgcattcccttgaggcttcaccaccagcccctgctcactttcagcctgcgaaccgtcttgcagaccatttactttcacaacattgcgcaggcacagtgtccagttcttcgcctcgcccgcaccagtcacagtaatcgtgttgccagtacgtgctgcttttaaagtaaagatcaccgatccgtcagcagcgggcacttcacagacggcttcatgcccgtcttgcagattgaagaggtggaatgccgtgccttcgtgccacacgtaatcgggacgttgatcgttgttgcccagcgccagtagagtgttatcacgcacataaacgggcagactcaggaagccgtgctgctgtttatgccagcgactaccgtcgagttcatcgttgtgccacaggtgtgtccagcgaccttccggcaggtagaactgcacatcgcccgcttcagtgaacaccggcgcaaccatcacgttgtcgcctaacatgtattgacggtcaaggtaatcacaagccggatcgtccgggaactccatcatcatggcccgcatcatcggcgtaccccgcgcgttcgcacgcgcagcttcacgatacagatacggcatcatgcggcatttcagttgcgtgaagaagcgcaccacatcacaggactcatcatcgtaggcccacggcacacgataagatttgctaccgtgtaaacggctatggctggagagcaaaccaaacgcgcaccagcgtttgtaaacgtgcgccggagcggtattttcaaagccgccgatatcgtggctccagaagccaaaacctgaaaggccaatagacaaaccaccgcgcaggctttccgccattgattcgtagttagcgtaacaatcgccaccccagtgtaccgggaatttctgcgcaccgacggaggccgagcgggcaaacaagacagcttcttcctcaccaacggtgtccttgagcacgttccacaccagttcgttgtagatgtacgcataatggttatgcattttctgcggatcggaaccgtcaaaccactgaacatcagttgggatacgttcgccaaagtcggtcttaaagcaatcaacgcccatcgcgaccagacctttcagtttgtcggcgtaccatttgcaggcatccggattggtaaagtcataaatcgccagacctggctgccatttatcccactgccatagcgaaccgtccgggcgtttgagtaaatagcctttctcttgtaactctttaaagacgggggatttttgaccgatataggggttaatccagacgcagattttcagtcctttcgctttcaggcggcggatcatcccttccgggtcagggaaagtcagcgggtcccactcaaaatcgcaccactggaaggctttcatccagaaacagtcaaagtggaaaacatgcagcggcagattgcgttccgccataccatcgataaagctgtttaccgtcgcttcgtcgtagttggtggtaaatgaagtggttagccacaggccgaaggaccacgcgggcggcagcgccggacgaccagtaaagcgggtataacgatcaagtaccgctttcggcgtcgggccgtcgataacaaagtattcgagatattcactctcaacgctgaactgcactttggagactttctccgatcccacttcaaaagagacacactggggatgattgaccagtaccccataaccacggttagtcatgtagaacgggatatttttatacgcctgttcagtacttgtgccgccgtcccggttccaggtctctaccgtctggccattgcgcaccagggcagtaaagcgctctcccagaccgtaaactgtttcgccaacgccaagatcaagccgctcaaacatataattgcgttgattattcgtgtcctgcacgtagccattatttttcacctgactaccggtaatacgttcgccgttgcgcagaaaatccagtgaccagaactcacctttgctgacacgcgcgcttaagttgccacttttaaactcagcataacgttctgtgttttcgattgtgaccttcacgtcctgcaaaatattgagcggataatgaggaccgttattcagcgccccctgaaaatgctcaatccgcacaccgacaataccttcctgtggggagaaaaagcgcaacgtaaataaaggcgtatcaagctgccaggtacgttcacgcacatcacggggggcagcatagaccaccatttcattatcctgctgttcaacctcgaacacctgaagcgggtgaatcaaattgaggccaggttgaatcaaccagtttccatcgctaattttcattgccgttccttagttctgcacttcttgagaggtgaattgttgctggcaacggcgtttaccctgagccagctgttccataacggttttcagattgtgcgtcgtgagtgagtagtagcgtttagcgataatcgcgctcagcaaataacagatcgccggaacaatcgtgaatagcgcaataatgatgctaatcgtggcgctgttctgcgctttttctgccgcatcatatccgccataagccagcatccagccgataagagcgccgccgaaggccaaccccagtttgagcacaaacagcgtgccagcaaaactgatcccggtcaggcgtttaccattgcaccactcgccgtagtcgacggtatcggacatcattacccactggataggtgtcaccagttgatgcaacacaccaatcacgaagatgaagacaaacatagtgatgctggcctgcatgggaacaaagaacatcgcgaggctaatcactgccagcagggcgttcgtccaccagaagatagtgactttacatttccagtcggtcagaggttttgccagtgcggaaccaatcaggttacccacgcaataagtggtgagaaaagcgacaaacacttccggcgtgcccaaaatccatgtgacgtaatacatcatcgccccaccgcgtacgcacaccgccaggatattgaaaatggttagtaaaccgacaatccgccactggtcgttttgccagatatcacgtaaatcttcccgcatagacgttgttgtaggtggtgcttcaacgcgttctttagtggtgaagaaacaaaatgccagcatcatgaatgccaccacggaaaggaccgcgataccgccctggaaaccgagtggtttattatcaccgccaattaaattaaccagtggcatcatcagaacagtagaaagcatgcctcccgcggtcgccagcacaaaacgccaggattgcagcgagatacgctgagtcgggtcattggtgattacaccacccaatgcgcagtaagggatattgacgacggtataaagtaaggtaagtagggtgtaagtaattgctgcatagatcattttgccgttcatactgagatctggcgtgctataggccagtacacagacgatcccgaatggcagtgcgccaaacagtacccacggacgaaatttaccccagcgagagcgcgttcgatcggccaacaaccccatgcaaggatcggaaatcgcatccagtgcacgagcgaccaaaaacatggttccgacaaaaccggcaggaatgccaaaaatatcggtataaaagaacatcatatataacattacgttatcgaaaataatgtggctggcggcgtctcccatgccataaccaattttctctttaacggacaacacttcactcttcatctgcttttccttgatgctataggggtgctgagaccgataacgcattttgtaaaccatccctgtgagagcgaatattccgatatctggttattaatttatgattcttgttttatgtgatcgtggtagcgttaattccgctcatatatcattgtaaaatatgggttttatatgaactataatgctttcgtgataatacgctgcgtgtattaggcggaaaaaactgatctgggggatgtagaaactcaaggaagtagctataatgcgccccgcctccatgtagcaatcgaggcgcggaagatcgtcgtctccggtgaggcggctggacttcaaatccagttggggccgccagcggtcccgggcaggttcgactcctgtgatcttccgccaaaatgcctctcctgacgttctccaaccccttgtaatactgtcaatccagatattttctactgctcaatattcaatcggcttcaggaatacctggtctaaggttttgtgatggacgatgagcggctgaagaatccgcctgtcggttcttctgtcctcgaacgcatccgcgatattcacgccagtatgcgccgtgtttatttgcaggtgatttgcccccctgctgactctcagccaactgtatcgccattaaggtgaagatgttgttttactcgccccagaacacccttttttatacgactattctatttctttaaccgctggcgaaaaaaactgactataaacttcaccaataatcagactgccatcaagattaatttgttcatttaatatatcaaatcaacttgttttatttttactatcaaaaatagctcattgccttactataattaatatataaattcggtaattaattcttaacatgcttttactaataatctcaattgctggccctataatattgcgctagcattgctttctggttgtatcagcgatactcaaaaattcttaatacaatactcattcgactggtacttatttgtaactcagttatattttttcgcccggtgattcagaagaatgcaaaaaacggctaccactccatcaaaaatacttgatctcactgccgcggcatttttacttgtcgcctttctgacgggtattgcgggcgctcttcagactcctaccctaagtatattcctcgcagatgaactgaaagcccgtcctataatggtaggttttttcttcaccggtagcgctattatgggaattctggtcagtcaatttctggcaaggcactccgataaacaaggcgaccgtaaattactgattctgctatgttgcttatttggagtgctggcctgcacgctttttgcgtggaatcgcaactacttcattctcctctcaacgggcgtacttctgagtagttttgcttccaccgcaaacccgcaaatgttcgccctcgcccgtgaacacgccgacagaacaggccgtgagacggtcatgttcagtacatttttacgtgctcagatctcgcttgcctgggttatcgggccaccgctcgcttatgaactggcaatgggatttagttttaaagtgatgtatctcaccgctgccatcgcatttgttgtttgcggactgatagtctggttgtttttgccatcaatacaaagaaatattcctgtcgttacccaacccgtagaaattttaccctccacccacaggaagcgggatacgcggctactttttgtggtctgttcaatgatgtgggcggcgaataatctctacatgataaatatgccgctatttattattgatgaactgcatctaaccgataaactgactggagaaatgattggtatcgctgccggtctggaaattccgatgatgttaatcgcaggctattacatgaaacgtattggcaagcgactattaatgctcattgctatcgtgagtggaatgtgtttttacgccagcgtactcatggcgacgactccggcggttgagctggaattgcaaattcttaatgccatcttccttggtattctctgtggtatcggcatgctttattttcaggacttgatgcctgaaaaaataggctctgcgacaacgttatatgcaaatacttcacgcgtcggctggattatcgccggctctgttgacggaattatggttgaaatctggagctaccatgcgttgttctggctggcgatagggatgttgggtattgcgatgatttgcctgctgtttattaaagatatttagctcaccagtctgggctaagaaaaatcggcgtggcgcaaacagagccatcctcgccatttttgctatcatgcctgcatacataaacgacaaaacagtatgcagagggaaaaatgggttccaccagaaaggggatgctgaacgttctgattgccgccgtgttgtggggaagttcaggggtctgcgcgcaatacatcatggagcaaagccagatgtcgtcgcagtttttgactatgacgcgtttgatattcgccggtttgattctactgacgctgtcatttgttcatggcgataaaatcttttctattattaacaatcataaagatgccattagcctgctgattttttccgtggttggcgcgctaactgtacagctcacttttttgctaaccatcgaaaaatcgaacgcagccacggcaacggtgctgcaattcctctcaccgacgattatcgtcgcctggttctcactggtgcgtaaatcgcgcccgggcattctggttttctgcgctattttgacatcgctggtcgggacttttttattggtgacacacggtaatccgacgtcattatcgatctctcctgccgcgttgttctggggcattgcctcggcatttgctgctgcattctataccacctatccctcaacgctaattgcccgctatggcacgttaccagtcgtcggctggagtatgctgattggcggtctgattctgttgcctttttatgccagacaaggaacaaactttgtcgttaacggcagtttgattctggcgtttttttatttggtggtcattggtacgtccctgacatttagtctgtacctgaaaggagcacaattaattggcggtccaaaagccagcattttgagctgtgcagaaccattaagtagcgcgctactctctttgctgttgctggggatcacgttcacattaccggactggctgggaacgctgctgattctgtcatcggtgattttgatttcaatggattcccgtcgccgcgccagaaaaataaatcgtccggcgcggcataagtgagaattaccagccaggcaccgcgccaccgttaaaaatggtttctgccgctttagcgacttcgggtgattgataagattgcagaaattccttcacgttttctgcattcttattatcttcccgtgccaccaaaatattcacatacggcgaattcttatcttcaataaatacgctgtcgtgcaccggagaaagcccggtctgctgaatgtaagtggtgctgataatcgctacatcaactttgggatcatccagtacgcgcgggagctgcgccccctcgagttccataatctgcaaatgacgaggattatcggttatatccagcgcggtaggtaataacccttttccctctttcagagtaattagcttctctttttgcaacagtaaaagtgcgcgaccaaggttggtcgggtcgttggggatcgccactgtcgcgccttcttttatttgcgccacggttttgatttttttggaataacccgccatagggaagacaaacgtatttcccaccgctaccagtttataaccatgcgcctgattatcttgttcaagaaagggtcgatgctggaagacattcgcatcaagttcgccatgatttgtcgcatcgttcggtagcaacgaaccgctaaatcctaccagttcaacatcgaggccatatttctcttttgccacctttttagcgacttccgcgacatcttgttctgcgccatttataacgccaactttaatgtgttttgcatcgctgctactctggtcgcaacctgccagcagaattccggccagcaataatgcggcccctgtccgtagatgatgtgttgtcagtttcatttttttatccttttattaatgattacctgactatagcggtaaggtcgctgcggtttaaaaaacgaaacgctatcgataagaataaaaaggaataaaagtggaatataaagtctggcacttcttactgaccacgcaagcgcgtttcgtacagcatgatgagagcgatgaaagcaaactacacttatgcttcattcgatacacatttgtaaaaggttgaatccatgaaaccaacgacactactgcttattttcacttttttcgctatgccaggcatcgtatacgccgagtcgccttttagctcactgcagtccgcaaaagagaaaaccacggtattacaagatttacgtaaaatttgcacgccacaggcgtcattatcagatgaagcgtgggaaaagttaatgttgtcagatgaaaacaataaacaacatatacgcgaggccatcgtggcgatggaacgtaataatcagagcaattattgggaagcgttgggtaaggtagaatgcccggatatgtaagaacagcaacaactactgaccaacgcttctttacctgatatcaggatttcttcattttcacctttgcagtaaccaacaatgcagtcagcaacatcaatgtgccggacaacatcaacggcgaagtcagaccaatattatccagcgcataaccgccgattgccgcgccacaggtattagcaagctgaataaccgccacctgaatagacccggctttttctgcctgatcggccagcgagcgggtgatccacgttgaccagccgacgggaaccaatgcaaaagttagcccccagataatcgccacgccggtagcaacgattttatcgcttccccacaacgtcagtaccaacgcactcacagccagtattaacggcgcgcctgctaaggccagttttaccgaacgtttaagaatgaacgacgaaagcgacgtaccaataaagctggcgataccaaaactcaacagcaccagcgttaagccatccacgccgaatcccgccaggttcatatacaccgggcgaatatacgtgaagaaagcaaactgcccggcgaaagacatgaagatggcgatcatccctgccatcacacccggacgttgtaataagcggaaagtattttgtttctgatgcgagggttcgcctggcagtgaaggcaatgatttgataatccagaaaatacacagcacgcccatcaccgccgccgcattaaagacattgcgccaaccgataagctcgcctaaaaaactgcccaacggcgcggcaatcaccagcgcaatagaaaccgcgccgaagatcaccgacagcgccttcggcaccgtacgcggcggcaccagacgcatggtcagcgacgccgacatcgcccagaacccgcccagcgccagccccagacaggcacgaccgattaaaagcaaactgaatgagttagcaaaggaaaccagcaagcaggagagcgtcagcaaaacggcaaacaaaataacaacgtagcggcggtcagtagcctgaattgtctgggtaataaacaaactggcaaacattgccacaaaggcggtcacggtcaccgattgcccggcaaccccttccgaaatgcctaaatcctgggccattggcgtcaacaaactgacgggcaaaaactcaacgataatcagacaggcgacacaaaacgccaccgagaaaacggctgaccagttcggtcgggtgatggcatccgcgccgcggttttcggcaataaattcactcatggtgttacccgtggcatgtttcaggggaaaagccgaccactttaacattgaaatgtgtgacgcatttaacgtttttgcaacttttacggtgttgcttgagctggagttaagatcgaaacggaacagggcaaagattaccggatgcggcgtgaacgtcttatccacccgacaggtcaggcgcggtctgtaggctgataagacgaaacggtttcaatgcaaccagtgaacgccctcggcaggctgaaagaacgcgttatagcgcatctgaaaagcattaatatcctgcatttcaggttcggtttcgcgcagaaaacctagcgccagcctgacctgagcgtcggtaatcggcgcggcgaggcgagctttttgtaaaatccgatgccattgcagcaggttctgttcgctaccatcgacaatgacaatttgccagatgagcaacacctgcgcggcgttttgcaggtgcgactcatccggacgatgcaaataacgtaaaaattcgtcaccagctgactttcccatttgatcgaccatcgactccacgggtacgacatcgatgttcagccgatcgctgagacggcgaatcgcttttctggccccggatgtcagcacccgaaaaccaaccacaaacactaccgccagcgtggcgagcattatccagatcatgagttctcctgcgtaatcagaactcatgatatctggaaaccctcgccagttactaatccaccagaataatcttcagtgcaaacagagctgcgaccaccaccacacacaggttcagatcgcgccagcgcccggtgcatactttcatgatgcagtacgacataaagccgagtgcaatcccttcggtgatcgagaaagtaaagggcatcatcaccgtggtaataaacgcaggcaccgattcggtaaaatcatcccagttaacgcgcgccaggctcgaagtcatcagcacgccaacaaagattaacgctccggcggttgcgtaaggaggaactatcgccaccagcggtgagaagaacataaccaacaggaacataacgccaaccacaaccgcagtcagccccgtgcggccaccgactgccacaccagaagtactttcaatataggcagtaacagacgaggtgccgataaacgcacccgccaccgaactgacgctatcaacatacagcgccttattcatattggggaatttaccgttaccatctattaagcccgctttatcagttacaccaattaatgttcctgatgaatcaaataggttgatcagcataaaggagaaaatgataccggcgagttcaagtgttaacgcgccgctcaaatctacttcaccaatgacgccgctaatatcaggcggaatggaatagacgccgctaaaatgaacatcaccgaaaaataatccacagcaagacgtcaccacaatagaaaccagcaccgcggcatgaaaatgacgtgatgacaacacggttataataaaaaaccctaaaatacctaacaacacgccgtgagaacttaaatcgccaatcatcaccagcgtgtctttattggcgacaataacgccagtattttttaatcccattaaggcgataaataatccaattccgctggtgataccaatacgtaaacttaagggaatgttggagatcatccagtaccggatacgaaacagcgtgagcaaaaatagtccaactgcgccccagaatattgcgcccatcccggtctgccaggagatgcccatcgcccccacgaccacgaaggcaaagaaggcgttcagccccattgccggagccagcgccacgggtaagttagcaaatatccccatcgcaatactgccgataccggcaatcaaacaggtggtaacaaacaccactttcgggtccatttgtgccgcgccgaggatttgcgggttcacaaaaacgatgtacaccatggttaaaaaagtggtcatccccgcaatcaattctgtgcggacggtggtcccatgctgaggtagtttaaataatcgcgaaagcgtccctgattcattactcacgtaatcggtattgtcattattcatttttttgtccattggaggagatttaatcccttgcttttgtaaaacaaatgacaacaacggttcagtgataattatcacatttcaattgcacattaatggatattctttaataatctcgcgacgtttctttatgataaataataatcaaattgataaaatcaaaatgagaaaaatatgaataattctattaaccataaatttcatcacattagccgggctgaataccaggaattgttagccgtttcccgtggcgacgctgttgccgattatattattgataatgtctctattctcgacctgatcaatggcggagaaatttccggcccaattgtgattaaaggacgttacattgccggtgttggcgcagaatacactgatgctccggctttgcagcggattgatgctcgcggcgcaacggcggtgccagggtttattgatgctcacctgcatattgaatccagcatgatgacgccggtcacttttgaaaccgctaccctgccgcgcggcctgacgaccgttatttgcgaccctcatgaaatcgtcaacgtgatgggcgaagccggattcgcctggtttgcccgctgtgccgaacaggcaaggcaaaaccagtacttacaggtcagctcttgcgtacccgccctggaaggctgcgatgttaacggtgccagttttacccttgaacagatgctcgcctggcgggaccatccgcaggttaccggccttgcagaaatgatggactaccctggcgtaattagcgggcagaatgcgctgctcgataaactggatgcatttcgccacctgacgctggacggtcactgcccgggtttgggtggtaaagaacttaacgcctatattactgcgggtattgaaaactgccacgaaagttatcagctggaagaaggacgccggaaattacaactcggcatgtcgttgatgatccgcgaagggtccgctgcccgcaatctcaacgcgctggcaccgttgatcaacgaatttaacagcccgcaatgcatgctctgtaccgatgaccgtaacccgtgggagatcgcccatgaaggacacatcgatgccttaattcgccgcctgatcgaacaacacaatgtgccgctgcatgtggcatatcgcgtcgccagctggtcgacggcgcgccactttggtctgaatcacctcggcttactggcacccggcaagcaggccgatatcgtcctgttgagcgatgcgcgtaaggtcacggtgcagcaggtactggtgaaaggcgagccgattgatgcgcaaaccttacaggcggaagagtcggcgagactggcacaatccgctccgccatatggcaacaccattgcccgccagccagtttccgccagcgactttgccctgcaatttacgcccggaaaacgctatcgggtcattgacgtcatccataacgaattgattacgcactcccactccagcgtctacagcgaaaatggttttgatcgcgatgatgtgagctttattgccgtacttgagcgttacgggcaacggctggctccggcttgtggtttgcttggcggctttggactgaatgaaggtgcgctggctgcgacggtcagccatgacagccataatattgtggtgatcggtcgcagtgccgaagagatggcgctggcggtcaatcaggtgattcaggatggcggcgggctgtgcgtggtacgtaacggccaggtacaaagtcatctgccgttacccattgccgggctgatgagcaccgacacggcgcagtcgctggcggaacaaattgacgccttgaaagccgccgcccgtgaatgcggtccgttacccgatgagccgtttattcagatggcgtttctttctctgccagtgatccccgcgctaaaactaaccagtcaggggctatttgatggcgagaagtttgccttcactacgctggaagtcacggaataataaaaaaagcccggcgtcatgccgggcaaaagtcaccagttacgtttatgccactgtcaactgctgaatttttttctcgcggcggattttgcgttcttccattaccgccactatcgccatcaggcagatacaaccaatcgcggcgatatccagcgcggcgaaggtgcctgcccagccggtaaggccgaataccggcgtcccatcggcaatcattcccagacctaacttggcaaagctgtcaccaatcaggtaagcaaaggtgcctttaataccatcggcagcgccaatcgcttttttaggtacaaagccaacagcagccacaccaatcaacaattgcgggccaaagaccaggaaacccaacgcaaagagagaagccagatagatatattcgttactggcatgttgatacacaccgagcgtggcgataatcagcgccagcgcgatgcaggccaccaggccacggcgaccgttcgccaggtcagagagccagccccacagcagcgtaccgaccagcgcaccagcttcaaacagcgtaaagccctgaatcgccaccgctttagagagtttcagttcctggaacgcgtatacggttgaccactggtcgataccaatacgtaccacatagaggaaaatgttggcgaagcacagcagccagatcactttgtttttcagcacatactcaacaaagatctgccacttggtcatatcggtagattctgtctctttgtcctcttcgctgatctcctcgccgaacagttcttcagctttgccgaggccataagattccggggagtcgctgccgtaacgcaggccgataaaaccgacaatcagcgcgataatcgacgggaagataaacatgccgatgacatggccatcgaacaggtaatttgccccgaacagcgccacacctgctgcgcctgcaccgccaaggttgtgagaaatattccagaaaccgaggaatgtcccgcgtttacgacgcggcgtccatttggtgatggtggagtaactgcacgaaccgccggtactctggaaaaagccgcttaaggcgtagaaggcaatcatcaggaacaggctaaccgagccgctgcccatactggcactgaagcccagcatacaaatagcagagaggatcagcatgaacggcaggaattgtttggtgtttttgccgtcggcgtagtaggaaaccagcgttttacccacgccataagtgatggagaaacccaggccgatcatccccagctgcgtcatgctcaacccgtaggtcgaaatcatatcgttctgcgcgatgttaaagttcttgcgaatcaggtacatcgtcaggtagccgataaagaccaccaggtaggattgcatgaacggtttgaaccacattttgcgccgcacttcgagcggaaggtccagggtcggcttgcgaacctggtttaagaaagccagcatgggttactcctgaaatgaatacctgcgtgaggcatgcattgtaaaaatcagcagcaaatcaggcctgagatagcgtccaggcaaaacctggaaaatttcttagttttgccggatatgaagtgaaaaggtgagatgcatcacgcttcgcgcggtgtctgggcgttcaaaaagggcagtaacagcagtgcggaaatcccggcggcgatagagataaccacaaaaaatccgctccagtgccaggtatcgagtactttcgccagcggccaaccagcaagcgacgcccccagataagcaaacaagccgacaaaccccgtcgccgcccctgccgcctctttgtgggaacactctgccgccgccataccgattaacatctgtgggccaaagacaaaaaaaccaatggtgaagaagcaggttgcctgcatcacgtagctggcaaatggcatcagccacagggagccgactgaaagcaaaattccggcggcgaaaatcaaattcatcggccctcggttgccgttaaacaatttgtccgagccccaaccggctaccagcgcaccgataaatccgcccagttcaaacatcgtcactgccgtattcgccgtgaccagatcgacgcccagtgtctcggacatatacaaattgccccagtcgttgatcgccgcccggaccacatagaccagcacatagcaaaacgaaagcagccagatatacggattcagcaacacatatttggtgaggatctctttacgcgtcaaccctgccccttcttgttgttgagcaatttccagcgcgtcgtgtcgccattcaccgaccgccggtaaacctaacgcctgcgggcgatcgcgtagccgccagcagagaaaaatccccacgactatcgccatacaaccagcaatcatcatcccggcacgccagccgtaatgcagcgcagccgctgccatcacaatgggaatgagtgcgccgccgacgttatgcgccgtgttccataatgcccaccaaccgccgcgctcggtacgtgaataccaggccgttaacagacgcgcacacaccggtgaaccccagccctggaaaaaggcgttcagcacccagagcacggcaaacgcccatagcgacgtcgagaagccaaacagaatgttgataatgcccgtggcgataagccctatccccataaaataacgggcatttgagcgatcgctgacaatgccggagacaaacttcgacacgccataggtaatgtaaaacagggtcgctaacaggccgatatcgctacggctgagcacgccgttagcaaggatttctggtacggcggcgttaaaacttttccgcgtgaagtaaaacagcgcgtaacccagccagatggtcagcagaatatgccgacgccagtagcgatagcgggcatcaatttcatatttatcagtcattaatggcgcatcggcaggcgctttcagaaacggcaacatcatcaaaccttagacatagcgttgaggtagagaaacgctgacacgcgtgccgtgcagacaggaaatgtgtaatgtgccacccagcgccgttacgcgctcgcgcattccggtgaggccaaaaccttgttgcccggaacccggcggcaaaccgctgccatcgtcttcaataaccagcatcaaccgttcatcctgctgccagccttgcagggtgaccgcgctggcatcagcatgtttcacaatgttgttcagcccttcctggcagacacgaaacagcgtcacgcgctggttttcgcttaacgctgattcatcgattcgccattcgagatggctgacaataccgcgcccttccagctccatttcccgcatcagtgagcggatggcctgctccagggtgagatcatccaactggcgcggacgtaaccgacccaacaaacggcgcaccgcgtcgtaaacgcccagcgatagttgttcgatgagctgcccgctctgcttcacgctggcgttatctgccgccagccgctgaacaatgcccgcctgagtacgaatagcagtgatggtctgaccgatatcatcatgcagctcacgcgccacatcacggcgcacgctctcttcggtttccagcaaccgttcagccagatgctgattgcgcgccagttccttttgcagcgactggttaagttcacgcaaccgctggatgccagcgccaagcaacaaccctgtcagactttgcaccagcagcgagagcaataaatccaccggatgatcgcgccaggtttgactggcgatcagcgcgatggcgttcatcaacgtcgcaatcagcgccccttgccaaccatagtgccaggccagcgcgataatcggcagcgccagacagaatggcgtaaagcgcgacagttcgtccggcaatcccaactggagccagagactgataacaaacagcagcaagtaccagaccagatgtcgcccgcgccagttgattggctgagaaaccagtgacggaccgagcggcagccaggtgttattggcgagatagtgccagaacaccagacatatcggggccagcgtcaggccgccagttaaagtcagcaacagcgcattccacgactctttgccgtgccaaagccagggcagcgactgcaacaacgccgccgccgttaacgccgccccctgtaacagcaaggtgcgccagtcacgctgatggcgatagcgcgagatcagcgctacgggcagtaacgtcagtaaactaccgatcatcaataacggaaaatgggttaaaccgaccgcctgcgttagccagtaaatcagcagccactccgcgcccagcaatacgggccagtatccgcgcgggcattgcagcattagccccagacgcagaccaaacggaaataacagcaccgccatatcagggcgctcaaccagatgcaggctgatactccacaggcaaaaccatgcggcagagaagataaaaaagcaggcaataacggtaattaagcgggagaacaacgtcttcatcaccagccatcaaacatgcggcgcgccagctctacgtcgttactgacgcccagtttttccatcagattggcgcgatggacgtgtaccgttttcggtgacaagcccagttcggcggcaatctctttcaccgccattccttgcgccagtttttccgccacctggcgttcacgtttggttagcgggtcctgacgaccggatgccagtttaatggcaatatccggcgtcagataacagccgcccgtggcaaccgtatgcaccgcagcaatgagttcatccgggctacagcgtttggaaagaaagccgcgtgcccccgcgttaagcgcctgctcaaccagcgcaggactgtcgtgaacggagagcataatcgtcgccatacctttcggcagctggcttagcagctccagaccggagatatcgggcatggagatatcgcaaatacacacctgcacaccgcgccccggcagccccgccagcgcctcgcgccccgaaccaaactcggcaactacctgcaaatcaggttccagccccagcagctgcgcaaagccggagcggacgatgaggtgatcgtctataagggcaacggtgatcatggtcttgtcctggcgggtaaaaaaaatacgcgcttaccttaacgataagcgcgatgttgttcaagccttgagcggttactgaaaaaacaccgcgatcttgttaaacatcgtcggatcggactgattacgctgcactttcacgacatcttccagcttatcgatttggcttatcatctgctccagacgctggtcgtcattgaccagtagccagatatggcttttgtcgctgtcctgaatcggcagacaaagaatgccttcaacgttaaaagcgcggcgggcaaaaaggccacaaacgtgggtcattacgcccggatggttgcgaacggtgagctccagaattacgttgtcatgagttgtgttttgcatggcttattcccccaccatttcagtattcgccgcacctggcggcaccatcgggtaaactttttcttcggcatcaatgcgcacatggatcagcgccgggccagggcgattgatgatttcctgcaatgaagcctgcggatcggcttcgttattcaaatcacaggtttcgaggccgaatccggcggcaatctgcataaagttgattttgcccggataggtggcggcaaaaacgccttgctcgtagaacagactctgttgctgatgcaccagccccagcgcttcgttgttcatcagaatgattttgacatccagctgattttcactggcggtcgccatctcctgaatattcatcatcaggctgccgtcgccggagaaacacaacactttgcgatccgggttcgccagcgcagcgccaatcgccgcaggcaggccaaaacccatcgtgcccagcccaccggaggtcagccactggcgtgggcgattgagcggataagcttgcgcggtccacatctgatgctgaccaacgtcggtggtgataattgcattgtcatcgacacaggcggcaacggcgttgatcaggccgtaatggcttaacggatcgcacgctttcgggattggacacggaaactcacgctgcaaatccgctaccaactggtgccactctgcacgcggttgcgcttccaccagcgggatcaactgcgccagcacgtcatcaacatccgcctgaatcgccacgtgcggctgcttgattttacccagctctgcacggtcgatatcgacatgaatgattttggcattcggacagaactgctcggttttgccaatcgcccggtcatcaaaacgcgcaccgagcactatcaacaaatccgcctcctgcaaaatatagttggtgctgcgcacgccgtgcatccccagcatacccagcgacaacggatgcgcttttggcaacatgcccagcgccattaaagtcatggtggtaggcagttgcgctttctccgccagttcacgcacccgtgcgggcgcattgatcacaccgccgcccagataaagcaccgggcgtttggcagcgttaatcatcgccgctgcgtcacgaatgctttcttcgctaaaggcgggggcggcggctttttctgccatagcgggctgtgtttcaatctcaaaaactgccgtttgcacatccttaggaatgtctatccacaccgggcctgggcggcctgattgcgcaatgcggaaggcatcgctcatgacctgcgggagttcttcgatatgtctgaccagatagttgtgtttggtgatggggatagagatgccgtaggtgtccacttcctggaaggcgtcggtgccgatcatcgaggcgggaacctgaccagtgatgcaaatcagcgggatggagtccagccgcgcatcggcaatggcggtcaccaggttagtcgcacccggtccgctacaggccatacagaccgccggtttaccgtcggtgcgcgccattccctgagcgataaagcccgcgccctgttcatgacgggccagaatatggcggatttgcgtgctttggcttaaggcatcgtaaacaggcaggatagaaccgcccggaatgcctgtcacaatcttaatgccctgctgttccaggaaatgaacgataaattctgcgccggtaaagcgcttacgcgtcgatgttgtgcccgaacttgccatgctccagtccttttcttctgggccgactttccgggaggtgcttaaacgaaaaaccccgcccggtttgcgccggcggggttttggaatcgtgtgttgttccagtccctacggcgcattgccgacgaccaccaccacacgcacgacgaccactgcggcggatggcgcagttggtagtagttttgcgttgagcatggaagtagtcattggggaccttgttggttttgtgtttaacaatatttatacaagcacagctttacaggggagacaatggaaaatttttcagcaagggaaaattgaggggttgatcacgttttgtactgaattgcagataacaaaaaaccccgccggagcgaggtttcgtcagtcgcctgcggctggtaaccgcaaagcacactgtattatgtcaacactgaaagtatacgtgttccgcgcagaacgcgcaatttcggcacgaattttgacgtatttagtgcatagttgagtatcgatcacagtttgcgttttgtccaaatattactgtttatttatacagtaaacttctataatatcactgtacgcaatgtgttatgcgggggccgcatcgttacccggcgcactaagtcctggctgaaacgggtggtgccgtcagcgccttaaccccgcgtgagcacactgtgttatgtcaacaagcacaacgtttctccttgagataccgcgtgcacaacagctggcaacaggcagcggaaaggtacgtcagctggcagtgctcctgaaccacaggagacgcgtatgaacctggtggatatcgccattcttatcctcaaactcattgttgcagcactgcaactgcttgatgctgttctgaaatacctgaagtaattcagattcaagtcgcaccaaaggggagcgggaaaccgctccccttttatatttagcgtgcgggttggtgtcggatgcgatgctgacgcatcttatccgccctaccatctctcccggcaacatttattgccgcttttgtttacatattctgccgctaaacaattccccattcctggcgtatatctggctaacattcatcaatgtgatagattcctctcccgcatttatgggaatgcgtagtgacttattctaattatttttataaaagcatccgtgataatgaaaaggcaaagaaacgtcaatttgttattgatgttggtattactcgtggccgtcggtcagatggcgcaaaccatttatattccagctattgccgatatggcgcgcgatctcaacgtccgtgaaggggcggtgcagagcgtaatgggcgcttatctgctgacttacggtgtctcacagctgttttatggcccgatttccgaccgcgtgggccgccgaccggtgatcctcgtcggaatgtccatttttatgctggcaacgctggtcgcggtcacgacctccagtttgacggtgttgattgccgccagcgcgatgcaggggatgggcaccggcgttggcggcgtaatggcgcgtactttaccgcgagatttatatgaacggacacagttgcgccatgctaacagcctgttaaacatggggattctcgtcagtccgttgctcgcaccgctaatcggcggtctgctggatacgatgtggaactggcgcgcctgttatctctttttgttggttctttgtgctggtgtgaccttcagtatggcccgctggatgccggaaacgcgtccggtcgatgcaccgcgcacgcgcctgcttaccagttataaaacgcttttcggtaacagcggttttaactgttatttgctgatgctgattggcggtctggccgggattgccgcctttgaagcctgctccggcgtgctgatgggcgcggtgttagggctgagcagtatgacggtcagtattttgtttattctgccgattccggcagcgttttttggcgcatggtttgccggacgtcccaataaacgcttctccacgttaatgtggcagtcggttatctgctgcctgctggctggcttgctgatgtggatccccgactggtttggcgtgatgaatgtctggacgctgctcgttcccgccgcgctgttctttttcggtgccgggatgctgtttccgctggcgaccagcggcgcgatggagccgttccccttcctggcgggcacggctggcgcgctggtcggcggtctgcaaaacattggttccggcgtgctggcgtcgctctctgcgatgttgccgcaaaccggtcagggcagcctggggttgttgatgaccttaatgggattgttgatcgtgctgtgctggctgccgctggcgacgcggatgtcgcatcaggggcagcccgtttaagcgcacgtcaccgcagcatcgtcatcagctccatgggagaacgatgctgctttatcagatcacgcatcacccgcatatgcggtgcggagtaagaataaaacgcctgatagcccgcacaaagcacgctgtctggcgtctcctgccgagcgtgcgggcacaggcgatgccagtcgcacgcctggcagtcacagcgcggttgcgggttttcgctgccacaccatttttgtaaggtggcgtcaaaaagctcaatcgagatacgactgatatctgcccgcacccaacactcgaacagggcaattaaaaatttcccccacagctctgctgtcaccgaagcggccgtcagatcgccccggtcatcaaattcaagatagggaatgagctgtacggagcggatgccccgctgtttgaaattgtgataaaaatcggcaggttgcagagcatccttgtactctacaaccagtttatgcctgtcctcttcagcatcaatgacctgacttcctgtcatgcgactctctcaataaatacgataagttgatgtatatgcgttacagcaaacagtattgcgagagataacaccgcgagggagatcaaaaatttgtcacggactacgtgaaattgggaaaaatcgctattcgtgacatccattaaattgcgattacgggtgtagtgccagaggatcagcgccacgatggcgagaatgccaatcgaaatccagaataacatgcccgcctggtgccagttgtgtttgatagccaacgccatcaacgcgccgtagcccagcatggtacgaaaccacgccagtgatgtgcgctccggctgcagtcctgggtcggcaatgcgtctggctttgcggctatccggcatacaacaccagtcccataacgatcaccgccacgaccatcaatattaagctaatgattaataagctgttggtgtagggcaggtcctctttcagacgcatcgctttttcattgcgtaaccagcgcaagtagccatacatcgctaacccgccggaaaacagacacaacaacaacgccagcagttcgcgaatgacgggcgtggcgaaatctggcgcaagttgatcaagcccaacccccgccgccagaaatcctagtgcagtacggatccacgccagaaaagtacgctcattagccagcgagaagcggtaatcaggcgcttctccgaggcgggaaattttcattgttgctcctttgcaatttcactaacgctctacctttagcggtttttttaagaatttcgtccgcccgtttcctgatatgcttttgccatccgctacaaggaggtcagatgggtatcatagctcaaaataaaatcagttcattgggcatgctgttcggtgccatcgctttaatgatggggattatccacttttcattcggccctttctccgcaccaccgccaacgtttgaaagcatcgtggcggacaaaacggctgaaattaaaagaggtcttctcgccggaataaaaggcgaaaaaattaccaccgtggagaaaaaagaggacgtagatgtcgataaaatcctcaatcaaagcggtatcgcactggccattgctgcgctactttgcgcatttattggcggtatgcgtaaggaaaatcgctggggcattcgcggcgcgctggtttttggcggcgggacgctggctttccataccttgctttttggtatcggcatcgtgtgcagcattttgctgatattccttatcttttccttcctgaccggcggttcactggtttaagcagcctgaataatgcccgccgggtgatcatcagcgggcattatcgtcagaacttctgttttttctcctccaccttcaccccttgtgtcggtaggccggtgtcatagtcgcgtacaactggcgaatagccatcttgtggacgtggacgaaacgcccccatccagcgcggccgtgcatctttacgccacggacgcagactccattggtaactgcggaacggatcgcgaattttgtccatgtaatccaataaggcgtcatgcattttgctgcgaacgtctgcaaaacggatatcatcgatcaggttatgcatttcatttgggtcattacggcgatcgtaaagttcatcactggtgaagaggttgagtaccagtttaaagtcatccgtcacccagcaacgcaccggaataaaaccgccaaagctgtcatgctcaatctcgtagcggttaaattccaccatcacgccgcgtggctctttcacggcaaggatattttcccccggcagaatctctggtttttcaatatctgccagcgccatcattgtcggcagtaaatcgatatgactgactggcgtatcgacctgtcgccgctccccttgcggcgaacggatgatcagcggaatgcgggtgatgtcgtcatacatcgccgcccctttactgatcagcttatgtgcgcccatcatttcgccgtgatcggaggtataaataacccacgtattttcacgttgctctggcgttaaggcattgatgacccgtccgatttggtcatcaacaaagtcattacaggcaaaatagagcggatggtgataaagcccgtcatcaccgactggcgatggcatcgcctgcgcccataagcggtgatgttccggtttgttagccaggtcatcctgtgctttctcgcccagctcgtagtaaaaatcagcgtatttctctaaatactccaccggacaggtgaacgggtgatgcggctcatcatacgaaaccaccatcaggaaaggctcgtctgcgcgcgcaggctgttgcagaaaatccaccgcccgattgctgatacgatgcgcccaggtgaaggtttcgtcgatatggttcgcctgtaaatcttcgacgctgtttaggccattgcgccacaggctaatctctttttccgtcagttcgctaagatagttcgccccatcgaaccagtaatcagcgtcccactccggcggacactcgccagtgccgaaatagtcatgaccgtcgagatgccatttgccgatgtaacaggtgtgatagccggcatccttaaagtagcgccccatagtggagatgtttttgcctggcgcgacgttgttggtccacgggccggactggttagcgtagataccggtaaatagtccggcccgtgcaggcgtacaaaccggtgaacaggtgtaggcggaattaaagcgaataccttccgccgccagactatcaatattttgcgtattcagcggtttaccgctatagcaaccgaccatattggtggcctgggtatcggtcatgacgaacagaaaattggggcgtttcataggctatccttcccgtcgggagtaaaggttacggctgggtcgtgacgatgccgccagctgtcaaaaatcaggtagacaatcactacggcggcaatgaaataactgatcatcgctaaccagcgcgtaccgtagccgccgaattcagccagcccggcatagacgccaatcatcgcgaacaggatgccaattgacgcgatcttgacgtttttccacggtttcatgtccaccgcaaacgcatctttgaaggtgaacggcgtggcgcgcggtttgataaaaccgatcaccagcatcacgaccacgttgatgcagaacgtacaggccagcacatagaggaaatggaagtcgaacttcaccagatagttgatggtgatgtagctgattatgccaatccccatcgctacttttgccgccagcgccgggatgcgcgggaagaaaaagcccataatgatgatggtaaccagcggcacgttgtaaatgccgttgagctgtttcatccagctatacagcccctgcggcgcgttggcgatccacggcgcgaccagcaccgaaacgatagcgataaagaaaccaaatttgcgcccgacggtgaccagctgctgcggctcggcattctggttaatgatgcgacggtaaatacccatactgaataacgtactggcgctattcagaaagccgttgaaggtactgatcaccgcaccaaataacaccgcgccgaagaaacccaccattggcactggcagaacgttattgaccagcgtcgggtaggccatgtcggctttcggtaaatcctgatacagatgaaacgcaatcaaccctggcagcaccagtaccagcgggtcgagcattttcagcaccgccgttaacagcgcccccttttgcccttccgccaggctttttgacgccagcgtgcgttgcacgatgccctgatttgtacaccagtaaaaggtgttcaccagaatcaaaccggtaaatgccgcgccaatcggcaagggatcggtcgggccaccgattgagtttaatttctcggcgtgaacggtggtgagttgctcaatgccctgcataaagctgcccttgcccatcgcgattaggccaaataccggcaccatcaacccgccgataaccagcccaataccgttgatggagtccgccactgccattgcgcgcagtccgccgatcaccgcatacaaaattcccgccagaccaagcaaaattaccagtagccagatagccgcaccgtgagaaatctgtagcgattccccgacgtgaaacaggctgttgagcgccaacgcgccggagtagagaacaatcggcagaaagcagacgccggtggcaattaggaagcagaagtcgatgataatacgcgtcgttttatcataacgttcctccagaaaatcggggatggtggcaatgccgcgcttcagatagcgcggtaaaaagattagcgcgaggaagatcagcgtcaccgctgaagtcacttcccagcccatcaccgacatgccgcttttgtaggcctgcccggaaaggccgaccagttgttccgtggaaaggttggttagcattaacgaagcggcaataaccggcgcttttagtgaacgtccggcaagaaaatagccttgttgcgatccggtatctgttttgcggaccttccaccaggtgatcaccgccaccagcagcgtaaaaccgacaaaactcaagatttgtaacgaattcatctcatagcccttatttatgtttatgtcccggacgcatgaatatagggagaggtaaaatgcgtcgggtcaggcagtcagattcttaaaatacaaacgtcgtatccctgaacggattgttttctgttaagttcaggttgtgagcataattcgccggagggatattaaaatgaatggaaaattgcaaagttcagatgtaaaaaacgaaactccgtacaatattcccttattgattaacgaaaatgtgatctccagcggaatttctctgatctcgctctggcatacctacgccgacgagcattaccgggtgatctggccgcgggacaagaagaaaccgcttatcgccaactcatgggttgcggtgtataccgtacaaggatgtgggaaaattcttttaaagaatggcgaacaaataacactgcatggcaactgtattatattcttaaagccaatggatattcactcttatcactgtgaaggtttagtctgggaacagtactggatggaatttacccccaccagtatgatggatattcccgttggtcagcaaagcgttatttataatggcgaaatttataatcaggaactcaccgaagttgctgagttaataacttcaccagaagcaataaaaaataatctggcagtcgcttttctgacgaaaattatttatcagtggatttgtcttatgtacgcagatggtaaaaaagatccacaacggcggcaaattgaaaaattaattgccactttacatgccagtctgcaacaacgctggagcgtagctgatatggctgccacgatcccctgtagcgaagcctggttgcgtcgtctgtttttacgctataccggcaagacgccgaaagaatattacctcgatgcgcgtctggatctggcgctatcgctattaaagcaacaaggaaactcggttggcgaagtcgctgatacgctcaacttcttcgactcctttcatttcagcaaagcctttaaacataaatttggttatgcgccgtcagccgtgctaaagaatacggaccagcacccaacggatgccagtccacacaattaacgtaactctggccagtacgctttgttggcctccagcaactcatccagaatagctttggcgaccgaggcgctcggtaccgttttcgacaacgtaatcgcctgccacaggtgctgatatgaacgctgttcccaggcgtccacgaccagtttttccaccgccacttgctgactcattaaccctttctgaaactgcgggatatcgccgaccaccagtggttcaggccgtagtagcgcacgcgcatctgtttgcgatcttgcagcccaacaatttgcgccatccggctttcaataccgattggcatgtcacagatgttgaggattttcgcattcgggcgcagacgacgcgtggcttctgcgacaatggctgccgggttggagtagttgagcatccaggcatttggtgaatatttttccatataatccaccagttccaggacgccgccaatggaacgcatgccgtacgctattccgccgggtccgcaagtttcctgaccaacaacgccgtggcgcagcgggattttttcatccagttcgcgcatcgggtatttgccgacgcggatgtgcgccatgacaaaatcaacgtcgctgaatgccacttcaggatcggtggtgtaactaaacgcaatgtccggcgctttttctttaaggatgactttacaggcttcggcaatcacttcctgccgcgcaccatcgttatcataaaatttcagtgcacgaagcgggaaacggtcctgattcgccaggagcatcaacacgatgcctggcgtaaaggtgcttccaccgcctgcgacaaccactgagaatttggtcattatactgcctccgtaatggcaacattttctgctgattgatgagaattaattaagctatcgagctgttcacgcagctgagatacatgcagaccaatgatcacctgaatggcatcgccactacggaagacgccgtgcgctcccagctttttaaagacttcgtcatccagcgtttgtgacatgtcatgcagtgcaatacgtaaacgcgtcgcgcaattgttaatgctggagatattgccgaccccgcccagggcttgcaggataccggcagcctgatccagctctttttttggctctgccgcggtggtttggcctcgcgaggctttgtattcggcttttgagtagagtttcacttccgcatcttcacgtcccggcgtgcacatgttgaactgcagaatcagtgtgcggaaaaccacgaagtacagcagggtaaagcacaacccaatggcgatttgggtcagcatcatatccgcgtggttgctgaacatcgggatccagttttgcggtaaaacctagtcaatcagacctccgcccatgttgcccaccacaccaaagagatacattacggtcgacattgaggccgccagcacggcgtgtaccgcaaacagcaacggtgaaatgaacaggaaggtaaattccagcggttcggtaattcccaccagcatggcggttaaggttgcgggaatcagcaagcccgccacttttacccgattttccggtgcggcagtgaagtacatcgctaaagaaatgcccacggcaccaaagatttttgagttaccgtgcagggcaaaaccgccttccgggaacaacgatttcagcggctcggcgctcaaactgaactcttgcagatgctgcgcccagtacatctgaatgccgccttcaacagctgccggaccaaagataaactgtccgtagatgaagtggtgtaaaccggttgggatcagaatacgttcgaggaaggtgtaaacccagaccccaagtgcacccgccgaacgcaggaacgcttgcagagattcaatccccatttgtacttttggccagccgagcaacgtcagccaggcacaggggatcatcaccaggaaggcgataatcaccacataagacgtcccctggaaaatgccgagaaaaaccggcagttttttatcgaacagacggttatgcagcgccgtcacaatgccggaaatgataattgcgccgataatgctggtatcgagggttttaatcccggccatcattgtcagaccgctacctgccaccgcgtcctgagtgaaatcgacgccgaagtagcttccccaggtcattcccatcgcgttgatgaaatagttccaggtcaggaaactcaccatcaccgccagacaagcacgcccctgcgcttgcttagcaaggccaatgggtaaaccgacagcaaaaatcagcggcatattacggaataccgtccaaccgccctcttcaataatgtgtacgatttgcgcgaataaactgttcggatcggtcagtgattccccgacaaacatcgggttttgcagcaagatggcaagacccaccacaatcccggcgaagggaaacagcagcactggcgtgaacatcgcgccgccaaagcgttgaatttgactgagcatttccacatcctcttttctcaattctgtaagtaggaagcctgattggttatgcggcaggcctggagcgaggataggaagatgcgatcggcagaacatgacgacccaatgggattcgtgatcgctttcatgcttttcgttgggcggtagagatctacgttttcgcgaaaaagtagacctctgtgagcacaggtacacagcatcgaacacatctttaaaaaaaagatgttttttcaatcgattaagcagaacttgtgtgcgcattacccgggcttgcaggcaaaaaagagatctagagatgatctacaaaagcattgcggagcggttaagaattcgacttaactccgcagatttcacgctaaacagccttcttcccggtgaaaaaaagctggcggaagagtttgcggtatcgcggatgaccatccgtaaagccattgacctgctggtagcgtgggggctggtggtccgccgccacggtagtggcacttacctggtgcgcaaagatgtactgcatcaaaccgccagtctgaccgggctggtggaggtgttaaaacggcagggaaaaacggtcaccagccaggtgctgatttttgaaatcatgcctgcgcctccggccattgccagccagttacggattcaaatcaacgagcagatctacttctcccgtcgcgttcgttttgtggaagggaaaccgctgatgctggaagacagctatatgccggtaaaactgttccgtaatctttcgctgcaacatctggaagggtcgaagtttgaatatattgaacaagagtgcgggattttgattggcggtaattatgaaagcctgacgccagtgctcgccgatagactgctggcgcggcaaatgaaggtagcggaacacacgccactgctgcggatcacctcgttgtcatatagcgagagcggggagtttttgaattattcagtgatgttcagaaatgccagcgaataccaggtggagtaccatttacggcgactccacccggaaaagagttaaccgatactccagaagagcaccgccagtaattggggggtgataatgcgcaggaacattaccaacggatagacagtggcgtaagagagcgccgccgcaccgctggttggatgaagattattagcaaacgccagcgccggaggatcggtcatggaacctgccagcatcccgcacatggtcaggtaattcattttggctaacatccgcgccagaatgccaacagtaatcagcggaacggcggtgatcagggcaccataaccaatccagcttagcccttcgccattgaccagggtattcacaaaatccccaccagatttcagaccaacgaccgagaggaacagcacgatccccagctcccgcagcgcgaggttggcgcttggcggcataaaccagtacagcttgccgatactgccgatacgcccgaggatcaacgccataatcagcggtccgcccgccagccccagtttcaacgcggccgggaatcctggcacaaagacgggaatagaacctaacaatacgcctagcccgatgccaataaacactggcagcatctgaacctgttgcagtttttgctgcgcattccccagcacattggcaacggcatcaattgcggacggacgccccaccagattgaggatatcgccgaactgcaggctgatatcgccactggcgaccagttcgaccccggcacggttcaggcgcgagataacaacgtcatagcgttctttaaagtgcaggtcgcgaatacgttttccgagcacgttttcattggtgaccaccacacgctcgacgcgcaaatcagtgcctttcgtggacagcgaagtatcgacctcctgaccaatcaccagttgcgcattatgtaaatccgctggctgacccaccagatgcagcaaatcgcccagttggataatggtatctggcgaaggaacttttagggtttcttcgcgtttcagacgcgagcagataattttgtcgccgttgagaatcggtacatctttaatggctaaatcatgcaggttagggttctcaacgcgaatattgatagtcttgatcagcgcgccgccattggtgcgtgaagactcgtgctgctgagcttctgtctcgacattgacgcggaaaataacccgcaacatccacatggtgaacaaaatcccgcaaatgccgaatggatacgccatcgcgtaactcatccccatctgatcgaccatttccattggtgtacccaggtcgcgcaaaatctgctgccctgcccccagcgctggcgtattggtaaccgcaccggagaaaatccccagcactaccggcagtggaatatcaaacagtttatgcaggatggcggtaaccagaccaccgatgatgacgatcagaacagcaaacaggttgaggcgtaatccggagacgcgcaatgaggcaaagaagcccggccctacctgaatcccgatagtataaacgaacaggatcaggccaaattcctgaataacatgcagcatatcgctacttaatgtcatccccgcctgagaaacaaaatggccgacgatgatcccaccaaacagcacgccgccaatacctaatcctatgccgcgaaatttgacgttgccgataaacaaaccgacgactgccaccaaagccagaatactgaccgttaatgctatatcactcatcgtccatttctcttgagataacattttaattgctacggattatggctgaatcggtgaagcagatttgccttatagcgcacattatcacgggaaagaacgtgccgaaatatcttaaacagtcgaaatttaacgcattgttgagtaagtaagacaaaaaaagccccaccagaatggcggggcaaagagaatagctagttagctatttaacgcgggacgttcgctgatagcgatacgctgcgctgcgatgggttcaggctcattacgaattaaatcaatatgcagtaaaccgtttacgaaggttgcgccagagacttccatattttcagccagcgtaaagctcaggctaaatggctgattcataagcccttgatgcagccattttttctcttcttttggctgctccggcgtgccttttacgctcaggcgcgtaccttccagttgaatctctaaatcttcctgacggaaacctgccagcgcaagggtaatgcggtagtggttatcgtcgcttttctcaatgttgtacggcgggaagctctggctttcaccggcgttttgcagtgcgttggccagtttgtcaaaaccgatccattgacgcatcagtggggataaatcgaagttacgcatagtcatttctccttctaagaagcgagtaagtacctgcaaatccgaagattcgcatatgctccctgacggcgagcatggagatgtcaggccgcgccaggcggccttagggaattagttgatttcgatacggcgcggttttttcgcttccggaatcacgcgttcgagatcgatatacagcaaaccatttaccaggttagcaccacgaacatgaatgttctcagctaactggaatttgcgttcaaagttgcgttcagcgatgccctggtacagataggtgcgctctttttgttcgtcggcgtgagcacctttcaccaccagcagattatcctgggcggtaatttccagttcgctctcagcaaaaccagccacagcgatagcaatgcggtaatggttttcgtctaccagttcaacgttatacggagggtagccgccattactctggctctggttgttttctaagtggttaaacaaacggtcaaatccaatagcagaacggtaaagcggggataaatcaaagttacgcataatcaatagctcctgaaatcagcgagaatgtaagaccttccacaatggacaggtcaggtagccagaacacccatcaggcgcgtcctcatcggctacgatgtaaaaatgggtctggaaatgaacttttcaagccttatcagcggacttttttttgcagtttatggtctattgcatagactgagggggcagcacgaaacgttaaagtgcgatagccgccacagtgcgacgtaatgatgatgttattttcagcaagggatcgctataactcatcaggccaacacccacgatcaacagatgaatttattatgataagaaatgtgttgttagcgttcatgatatgcagcggaatgacattactcggaggatgctccagcgtgatgtcccataccggagggaaagaaggaacgtatcccggcacccgcgccagcgcaaccatgattggcgacgatgaaaccaactggggcactaagtcgctggcgattctcgatatgccgtttaccgctgtgatggacacgcttttactgccgtgggatgtgttccgcaaagacagctcggtgcgctcgcgcgttgaaaaaagcgaagccaacgcgcaagccaccaatgcggttattccaccggccagaatgcctgataactgatttagcgatcagtttcggtgatccacagctggccgccttccatccacgccagccactgaccatccggcgagaagaccacggcgtccgcagaaggtgaattggcgtggtgttcggttaaatactcaacctcgccgctttgcgcatgggcacaagcaattcgattatccagcacaaagcccaaccattctcctgacggatgccagttaaatgcagactgaatatccgttttgttatgggttaactggcgcggctcgccgccctgtggcgagataagccacagttgcacaatgccgttatcatctcgcattaaaaacgcgatttgtgtaccctgcggattacagcgcacccagtggcgcgggacgttgactaaccccggataagcccgatggtgggtaaaggttaaacgtcgctgcacgacgccacgcggtggcgcgggcagggttgtttccgttccgcttaacggcgcatcacctgccgctttccagccagcttcatcttgcggtaactcaacgataaacagctccggcactttctcgccctttggcgaaagtgtgtcgccaataaatgccagcgcgtgatttcctacccatccttcttcataagcacgattgatttcatcactgccaggctgtggcgtgggcgtggttttgctcaccagcacgcaccagtggctaccgctgtattcacgcggatgctgcttttgtacgttgaccgggccaaacggcgcagcaacaccgacgtttcgcaaatccagcgccggatcgagttcatgcattacatggtcgttataggtaaagctcaccctttcaccgttcgggctaaagacatgcacatggctgccgccgcgcagcactcctggcgtatacggcgcggtaatatccatcgcatcaaggttactcatcttgccgccttcaacaatcactccgcgccgatgatggaagtcgtaatgccatgtttcatcaggattttccgggccgtggatgaaaacatatttctctgacttcggatgaacggtcaccacgccgacgtgtgcgccctgtgacgcgcgatagataacctcgacctcgccggtatggatattcacacgctcaatggtctcgccggtaaacgacgcgccagaaggacgcacgtcaaataccagccactggctgtcgggcgtccaggtattggtattggtgagcaggtgattacggggagcaaaggttatctgtttcatggcgcggtcctgatacaaaacgggtcccgccatcatacttcacaaggacttcactttcagacaatagtcttttgccatcgtgatgaatgtgagtgaaaagatggaacatttcgacgtggcgattattggcctcggcccggcaggatcggcgttggcacgaaagttagcaggcaaaatgcaggtgatcgcgctggataaaaagcaccagtgtggtactgaaggtttcagcaaaccctgcggcggtctgctggcaccggacgcgcagcgatcttttattcgcgatgggctgacgcttcctgtcgatgtgatcgctaatccgcagattttcagcgtcaaaaccgtcgacgtcgccgcatcgctcacgcgtaactaccagcgaagctatatcaatattaatcgccatgctttcgacttgtggatgaaatcgctgatccccgccagcgttgaggtttatcacgacagcctgtgccgaaaaatctggcgtgaggatgataaatggcatgtcatttttcgtgcagacggctgggagcaacatattaccgcccgctatctggtcggtgccgatggcgcaaactcgatggtgcggcgacatctctacccggatcatcaaatccgtaaatatgtcgctatccagcagtggttcgcggagaaacatccggtgccgttctactcctgcatctttgataattcgataactaactgttattcatggagtatcagcaaagacggttattttatctttggcggtgcctatccaatgaaagacggtcagacgcgtttcacgacgctgaaagagaaaatgagcgcctttcagttccagtttggtaagacggtgaaaagcgaaaaatgcacggtgctgtttccctcgcgctggcaggattttgtctgcggtaaggacaacgcctttctgattggtgaagcggcgggatttatcagcgccagctcgctggaggggattagctatgcgctggatagcacagacattctgcgttcggtgttactgaagcagccagagaagctcaataccgcttactggcgcgccacccgcaaactgcgtttaaaactcttcggcaagatagtaaaaagccgatgcctgaccgcaccggctttaagaaagtggattatgcgcagtggtgtggcacatattccacagttgaaggattagccaacgcgcttcacatcgcccaccagcaggatataagagagcgcgccaatcaacgcgacggcggagatataaaccagtgcaggtgcgaaaccgtaaccctgcgccaggtaccccaccaccagcggaacggtgatgccgcccagaccaccggcgaagttaaacacgccgccggttaaaccaatcaggcgcatcggtgccagagaagaaaccagcgaccaggtaatcgaagcaaaaccgttaccgaagaatgccagcgccatcaggcacataatcatcatcggatcgttagtgtagttagcgcccataatgcaggtggagatcagcaagccgcagataatcggcgttttacgcgcaaagcccagtgaaaagcccttacgtaccagcagatccgctacccagccagagagcaggacgccgacaaacgccgcgaggaatggcaccgtggtcataaagcctgctttcagcgccgtgattcctttttcctgggttaaatagttcgggaaccaggttaagaaaaaccacagtgtagaagccaccgcaaattgcccaagataaacgccgatcagtttacgatggaacaccagtttccagtctttggctgttaacggctgacgcgcctctttcttcaccggcgcatcaccatccaccagaccgccgccatcacgaatgtaatccagttcagctttgctgatacctttggtcaggcgcggcggctgataaaccttaaaccaaatcagcgaccagataatgccgataccaccagtgacaatgaacacccagtgccagctcaacatctcctgaatccagatcagcagcggcgtcagaaacgccagaccgacaaactgaccagacgtataaaaaccaacggcagaagcgcgttcatgttccgggaaccagctggtcaccatccggttattggtcgggaaagcaggcgcttcgaaaataccggttatcgcgcgcagaccaattaatgacattaagcccgtggcaaagccctggaataaagtcgccactgaccagccaaatatcgcaataaaataagtcacgcgagaacctacgcgatctaaaaaccaaccgccggggatctgacatagcgtataaagccaggcgaaggccgaaaatacatagcccatttccgctttggtaatgccgaactcttcctgaatatgggcggaagccacggccaggttggcgcggtcgacataacaaatgactaccgtaataaagatcatcaccagcgtcagataacgccgacgccccggctttgctgcattaacgggaatatccatagcgagctttctccagattttgggcatagcgaagccgctcaccatgccctgtaatttacagagggttatatttttgtattgctgttttagtgcccgatgaggggcttacgtggcaggaattaccactctgctacgctgttatcttcatgacgccagagcggattacgccagtccggggcatttttactgaactcaatcactttagcttcgtcgatttccacgcctaagcccggtttcgttaacggtttaaagaagccgccgaccatgctgaagtcttctttgtttttcacaaagtcgagtaactccgcgcctttgttgtaatgaattcccatactttgttcctgaagtacggcgttataggaaacaaagtcgatatgcaggcaagccgccagtgcaatcggtccgagcggacagtgcggcgcaagggtcacgtcataggcttctgccattccggcgattttgtagcattcggtaataccgcccgcgtgggagagatccggttgcagaatcgaaataccacctgcctccagcacgcgtttaaaatcgaagcgtgagaacatgcgttcacccgccgccagtggaatatgcgtttgtgccgccagtttcgggtagtattcggcttgttccgccagcaccggctcctcaataaacagcgggcgatacggctccagttctttaatcagcactttcgccatcggcgcgctgacgcgaccgtggaaatcaagaccaaactcaatctgattgccaaaagcttcacgaatttgtgccacggtgttaaccgccgcatctaccgcgcgggagttatcaattagccccagttcttcacaaccgttcagtttgaaggtatcgaagccgatttcgcgtagcgttttaatgccgtcgataacatccgccggacgatcgccgccaacccaactgtaggctttaattttgtcgcgaaccaggccgcccatcagttgccagaccggcgcattcagcactttacctttgatatcccataacgcctggtcaatcccggcgatggcgctcatcaggatcggaccgccgcgatagaatccggcgcgatacatcacttgccataagtcattgatgcgcgatggatcctgaccaatcaaatagtcacccagctcgtgaactgccgcttccaccgtacgggcgcggccttcgatcacgggctcgccccaaccgaccacgccttcatcggtttcaattttcaggaacatccagcggggaggtaaacgatacgtggtaattttggtgattttcattgcactgcctctcgatacgccttaacaaatgctgctgcctgctgcgcggtgcgctctacggattgcccggcgcgatagagatcgctgcctaagcccgcccctgcacaacctgcgtctatccactgcgccaggttttctggcgtcacgccgccaacggcaaagactgcgatgtccgatggcaataccgcttttaacgctttgatgtattgcggaccaaaagccgatgacggaaatattttcagcgcctgcgcgcccgcttcgagcgcggtaaaggcttcggtcgccgtcgcgcagccggggcagacggtcatgccgtagcccaccgcacggcggatcacttcactatggatattgggcgtaacgatgagctgacagcccatcctggcgagcgcatcgacctgttcaggtttcagtaccgtacctgcgccaatcaacgccttgtcgccgtacgcatcaacgatggcgggaatgctttgctcccattgtggggaattcagcgggatttcaaccgcgtcgaacccggcgtcaatcaccgcgccaacatgcgccagcgcctcgtcgggcgtaataccgcgcaaaatggcgatcagcgggagtttagtttgccactgcatgagcgatgctccttataccagcctgaaatgccgtgtcgcccgccaccgccgtcacgtcgcaacccatcgcctgaaaggcttgctggtagcgcgcggtcagcgatgttccggcgacaagggtgatggcgtgttgatgggccacatagtcgcgcatactggcgacctctgcgccaatcaacaaaccagagagaaattcgctgacctgttcgcggggaagtgttcccagcacatgcgaggcgcgaacttcaaaaagctgcggcaatatggcgggcgtattaagaccacgctcaaggccagctgtgaaggcatcggcagagttttcctgcggcggcaaacctgcgccaatcaatgagtgatttaacagtaaatgatgtaattcaccggtcatcacggtgcgaaaatcgttgatttgctggctatcggcctgcacccatttgcaatgggttccgggcatgacataaagagaggaaggagccagagctcgcgcgccgatcaattgtgtttcttcgccgcgcatcacattgtggttatcgtcatgagagacacataatccgggaataatccagatattgtcgccaactgacgttaattgttcgccaatagacgaaaaacaggcaggaacagataaatacggtgcaactttccagccgacgttgctgccaaccattcctgccattaccactggcgttttctcttcacgccagtcggtcgtgacttctgctaacaccgcagccggagattttccgttcaggcgcgtgacgcctgcttctgattgcctgctctccaggcagtggtcgccctgataaagccaggcgcgcagattggtcgatccccagtcaattgcgatgtagcgagctgtcatgtgatttcctttaaccttcgtgtcgagctggcgatcatggtaagcgccgcctgctctgccgcatcgccgtcctgatgtcgtatcgcatcgaacagcgccttatgttcctggagcgtttgcggcatgttggcctcatcgcccatccaggttcgttcaaaaaccgcccgctgcagcgaactgatcgcaatgctaagttgctgtaacaccgggttatgcaccgactgcagcaccgcctcgtggtagcgaatatccgcttcgttaaacgcttcgcggtcctgattgttggcaatcatctcgttcagcgccgattcaatctgcgccagatcgctggaagtcgcgcgctctgctgcccaacgggcaatcgccggttccaccagatttcgcacttcgctcatggcactgataagccgtgggtcgtagtcattttccagcacccattgcagtacgtcagtgtcgaggtaattccactggttacgcggtgccacaaacgccccgcgataacgtttcatttcaatcagccgcttcgccatcagcgaacggaacacctcacggatgatgttgcgcgaggttgcaaactcctcacagagttccgcctcagccggaagcggcgagcctggcacgtatttgccgtgaacgatctgtttacccagcgtaatgacaatgcgatcggttttattgagagtcatggagagtccttgtgctctgtatgttcttctctactttaccccgatcgatgcataacgcggcaactttgtagtaccagcgtgatgacgttcgcgtttgccgtgcgtgtaatgtagtacaaacttatattgttgtactacaatttagatcacaaaaagaacaatgcataaaaaaatgacatgcgtcgggcagaaatctgaaaagggatatcaggcgctaaacaggagggaaagaagagtatgctttcaacggcttagctactcgtttaaaggattaatcatgaagttgaattttaagggattttttaaggctgccggtttattcccactggcgctgatgctttcaggctgtatctcgtatgctctggtttcccataccgcaaagggtagttcaggaaagtatcaatcgcagtcagacaccatcactgggctatcgcaggcaaaagatagtaatggaacaaaaggctatgtttttgtaggggaatcgctggattaccttatcactgatggtgccgatgacatcgttaagatgctcaatgatccagcacttaaccggcacaatattcaggttgccgatgacgcaagatttgttttaaatgcggggaaaaagaaatttaccggcacaatatcgctttactactactggaataacgaagaagaaaaggcactggcaacgcattatggttttgcctgtggtgttcaacactgtaccaggtcactggaaaacctaaaaggcacaatccatgagaaaaataaaaacatggattactcaaaggtgatggcgttctaccatccatttaaagtgcgattttatgaatactattcacccagaggcattccggatggtgtttccgcagcattactgccagtgactgttacgctggacatcattactgcaccgctgcaatttctggttgtatatgcagtaaaccaataatcagtaagcgggcaaacgcgtttatgctgtttgcccgcccacagattaattcagcacatacttctcaatagcaaacgccacgccatcttcaaggttagatttggtgacaaagttcgccacttctttcactgaaggaatagcgttatccatcgccacaccgacgcctgcatattcaatcattgcgatatcgttttcctgatcgccaatcgccatgatttcttccggtttaatacctaacacgtcggccagtgatttcacccccgtacctttgttaacgcgtttatcgaggatttcgaggaagtacggcgcacttttcagcacggtatatttctctttcacttcctgcggaatacgcgcgatagcctggtcgaggatggcgggttcatcaatcatcatcactttcaggaactgggtattggggtccattttctccgcttcgcagaacaccagcggaatggtggcaacgaaggattcatgcaccgtgtagtagctgatatcacggttggcggtgtacagcgtggtgcggtccagggcgtggaaatgagaaccgacttcgcgagagagtttttccaggaaacgatagtcgtcatagctgagagcagtttgcgccacggtgctaccatcagcggccttctgtaccagcgcgccgttataagtaatgcagtagtcgcccggctgttccatatgcagctctttcaggtagttgtgcacacctgcatacgggcgacccgtcgttagcacgacattcacgccacgggcgcgagctgcggcaatcgcatttttaacggcgggtgaaatggtgtgatcgggcagcagaagggtgccatccatatcgatagcaatgagtttaatagccatgagttccccaggtagattggttcctgacccatgctaacgcgattccgctcaaaaatcagtacaacacccgagggaaaagggggatgcaacgcgcgttgcgtgctccctttttgcttagcggaagagtttccctttcagcagttccatgcctgcggaaagcagatcgttattggcttgtggtgacacttcaccttgcggtgagagcgcatcaataatcttcggcaattgttctgccagtaaactggaagctgtactggtatccacgccaagtttttgcccgagatcggacaccgcatttgtgccgagcgccgattccagttgctcgccactaaccgattgattgccctgttgattactcagccaggttgagagaatggcccctaagccgccactttgcagtttttccagcagcacctgaatgccgccctgctcctcaacccaacttaaaatagcctgatatttccccgcatcgcctttcagaaaggcaccgacaacttcatcaaaaagccccatgataatcacctgtaaagcgttacgtgttgacccaaaaagtatagatttgcgggatgataattgcggattgcagaaataaaaagggcggagatgatctccgcccttttcttatagcttcttgccggatgcggcgtgaacgccttatccggcctacaaaatcatgaaaattcaatacattgcaagattttcgtaggcctgataagcgtagcgcatcaggcacgctcgcatggttagcgccattaaatatcgatattcgccgctttcagggcgttctcttcaataaacgcacggcgcggttcaacggcgtcgcccatcagcgtggtgaacaactggtcggcagcaatcgcatctttaacggtaacgcgcagcatacgacgactttccgggtccatagtggtttcccacagctgttccgggttcatctcgcccagacctttataacgctggatggagaggccgcgacgggactctttcaccagccagtccagcgcctgctcgaagctggctaccggctgacgacgctcgccacgttcgataaacgcatcttcttccagcaagccacgcagtttctcacccagcgtgcagatacgacgatattcgccaccggtgataaactcgtgatccagcggatagtcagtatccacaccgtgggtacgcacgcgaacaatcggctcgaacaggttttgctcagcattggtgtgaacatcaaacttccactggctgccgtgctgttctttgtcgttcagttcgctgaccagcgcgttcacccagcgggtaacggtctgctcatcagaaaggtcagcttccgtcaacgtcggctgatagataagctctttcagcattgctttcggataacgacgctccatacgattgatcattttctgcgtcgcgttgtactcagataccagtttctctaacgcttcgccagccaatgccggtgcactggcgttggtgtgcagcgttgcgccgtccagcgcgatagagatctggtactgatccatcgcttcgtcgtctttaatgtactgttcctgcttgcctttcttcactttgtacagcggcggctgagcgatgtagacgtgaccgcgttcaacgatttccggcatctgacgatagaagaaggtcaacagcagcgtacgaatgtgcgagccgtcgacgtccgcatcggtcatgatgatgatgctgtgataacgcagtttgtccgggttgtactcgtcacgaccgataccacagccaagcgcggtgataagcgtcgccacttcctgagaagagagcatcttatcgaagcgcgctttctcgacgttgaggattttacccttcagcggcagaatcgcctggttcttgcggttacgcccctgcttcgcagagccgcccgcggagtccccttccaccaggtacagttcggaaagcgccggatcgcgttcctggcagtctgccagtttgcccggcaggcccgctaagtcgagcgcacctttacggcgggtcatttcacgcgcgcgacgcgccgcttcacgggcacgggcagcatcgataattttgccaaccacgattttcgcgtcggttgggttttccagcaggtattctgccagcagttcgttcatctgctgttcaaccgccgatttcacctcagaagaaaccagtttgtctttggtctgggaggagaatttcgggtccggcactttcacggaaacgaccgcaatcaggccttcacgcgcatcgtcaccggtggcgctgactttggcttttttgctgtagccttctttgtccatgtaggcgttcagggtacgggtcatcgccgcacggaagcctgccaggtgagtaccgccgtcacgctgcggaatgttgttggtaaagcagtagatgttttcctggaagccatcgttccactgcaacgccacttcgacgccaataccgtctttttcagtggagaagtagaagatattcgggtggatcggcgttttgttcttgttcagatattcaacgaacgccttgatgccgccttcatagtggaagtggtcttctttgccgtcgcgcttgtcgcgcagacgaatggaaacgccggagttgaggaacgacaactcacgcagacgtttcgccagaatttcatattcgaactcggtcacattggtgaaggtttcgaggctgggccagaaacgcaccatggtgccggttttttcagtctcgccggtaaccgccagcggggcctgcggtacaccgtgttcgtagatctgacggtgaattttaccctcgcgctggataaccagctccagtttttgcgacagggcgtttactaccgaaacaccaacgccgtgcagaccgccggacactttataggagttatcgtcaaatttaccgcctgcgtgcagaacggtcatgatcacttccgccgccgatacgccctcttccgggtgaataccggtcggaatgccgcgcccgtcatcctgtacagagacagagttatcggcgtgaatggtgacgataatttctttacagtgacccgcgagcgcttcgtcgatagcgttatctaccacctcgaataccatgtggtgcagaccggtgccgtcatccgtgtcgccgatatacatacccgggcgcttacgcaccgcatccagccctttcaggactttgatactggaggagtcataagaattcgacatcaacgtttctcgctcatttatacttgggttaatccgttattttacccttttccacggtaaacatcttcgaattttcgtccgacatgtctataacgtgttcagcactgatcgcgctgacaaagacctgtgattgcgtcgcttttaagcggctggcaagcagcccgcgacgctcatcatcaagctcagaggcaaaatcatctatcaggtagagacaccgccgcccgctttcacgggtgaggaactctccttgcgccagacgtaaggcgcacatcaacagcttaagctgcccacgcgataaggtatcttccaccggcgcaccgtcggcgcgaatgcgtaagtccgctttgtgcgggccgtgcgcggtgtaggttagctggcgatcgcgttcaaaattacgttccagcacctcagcatattctgtctctttctcccagccgcgctggaaagagaaagtcagagaaaactcagggagaaattgcttacaggtatcagccatatcggccgcgataccggcgctatactccgcgcgccaggtgctgatttgctccgccagcgggatcagctctttatcccacgggcgtagctgttcgtaacgtgtcacctggcgcagcgccgcattgcgctgcttgagcaatcgcttgagattgctccaggcggtgaaaaatccgggttcgttgtgaaagcatccccagtcgaggaatgctcttctgtatttggggccgccgttgagtaaagtaaacccttctggcgttatcaactgcattggcatcaggtgcgccagttccgcgaccttatgcccgtctgtaccgtcgatgcggactttgctgtcgccctgtttgtctttggttaagccaatcgctgtctcgcgctcttcgccctgtaatcgcccgtggagaacaaacgcctcctgctcatggcgaatgacgcgaccaatctgcaaactgcgaaacgcccgaccatggccgagcgtatagatggcttccagcacgctggttttgccactgccgttggcacctaccagaaagttaaagccgggagataaggcgagatccgcggtttcaatgttgcggaaatcgcggatcaacaagcgggtgagggacattacagtctcattggcatgacaacataagccgcgctctggctggccgcatcttcaatctgcacgctggaaaccgaatcggtcagcatcatgcggacgttttcgcatttcagcgcgttcagaacatccagcacataactgacgttgaagccgatttccatctccgcaccgctataggtaacgtcgaggatctcttccgcttcttcctgttccgggttgttggcggtgattttcagctggttttcgctgacataaagacgtacgccgcggaatttctcgttagagagaatcgccgcgcgagcaaacgcctgcttgagcagatcgcagccagcttccagatgtttgtccgggttcttcggcagaacgcggcgataatccgggaagcgaccatccaccagtttggaggtgaagataaagtcgccaacgtgggcgcgaatgttgttgctgccaatctgtacgcgcagcggattgtcgccgccgtcgagcatacgcatcagttcaatcacgcctttacgcggtacgatcaccgaatggcttggcaaagattgaccaattggcattgaacagaccgccagacggtggccgtcggttgccacggtgcgcagttcttcaccttcggtttcaaacagcataccatttaagtaatagcgaacgtcctgatgcgccatagaaaactgggtcgcttcaatcagacgcttcatcgttgcctgcggcagggtaaattcgacttcactctgccagtcatcgaggttcgggaaatccgccgctggcagggtagacagcgaaaaacggctacgcccggagcgtaccagcatccgttcaccttccagctgcacggcaatttccgcgccttcaggcagaccacggcagatatcaaagaatttgcgcgccggaacggtcgtcgctcctggctcgtgtggctgaaccagcgcaacacgtgccaccatttccatctcgagatcagtaccggtcagcgacaacgtaccgtcagcaacctgtaacagcagattaccgagaatcggtagcgtaggacgaccacctaacggaccgctcacctgttgtagcggttttaataaatgctcacgttctacggtaaatttcataggtttacgatgacaatgttctgattaaatttgaaaaatcttctttgatatcgtggctctcttcacgcaactgctcgatcttacggcaggcatgaagcaccgtcgtgtggtcacggccaccaaacgcatcgccaatctccggcagactgtggttagtcagctctttcgccagcgccatcgccatctggcgcggacgcgccaccgagcgggatcgacgcttggaaaggagatccgcgactttgatcttgtagtactccgccaccgtcttctgaatattgtcgatggtgaccagtttttcctgcaatgccagcaagtcgcgcagcgcctcacgcacgaagtcgatggtgatcgcccgtccggtaaagttggcattggcaatgacgcggttcagcgccccttccagctcacgtacgttagatcgtagacgcttggcgataaagaacgccacttcgcccggcaaacgaatgtcgttttcgtcggcctttttcatcaggatcgccacacgggtttccagctctggcggttcgatcgccacagtcagtccccaaccgaagcgggatttcaaacgatcctcaacgccgttgatctctttcggatagcgatccgaggtgagaatgatctgttgattaccttccagcagggcgttgaaggtgtggaaaaactcttcctgagatcgttctttattagcaaaaaactgaatatcgtcgatcagcagtgcatctacggaacggtagtagcgtttaaactcttcgatcgcgttgttttgcagggctttaaccatgtcctgaacaaagcgctcggagtgcatataaaccactttggcattcggcttgcgcgccataatgccgttacccaccgcatgcagcaggtgagttttacccagacccgtgccgccataaaggaacaacgggttataggcaccgccagggttatccgccacctggcgagccgccgcgcgcgccagttggttagatttaccttcaacgaagttatcaaacgtgtgtttgacgtttacgttagaacgataggtcggttctgccggggccgggacgttatcccaacctgagcgcgtagaaggcgcagcacgttgcggctgcgtttgcgccacctgtgcaggggccgcgacgttgctcgtcactgccgcttgtggcgtttgcgtcaccggtttggtgccgacttcaaaacgcagctgtggggcatccgctccgcagaaactggttagcagtccattgatattattaaggtacttgtcccgtacccaatcgaggacaaaacggtttggcgcgtacagggccagcgtgttatcgctcagttccgcctgcaatgggcgtatccacatactgaattctgtggctggtaactcatcctgcaatcgggcaagacactgctgccaaagcgaaagtgacacggcggactccactcgaacaaaagtcgataatgactaaggctgaaacattcatgattgttgacgtacgtcgaaaagaccctgcttgagggtgacgcacgaaccgctgtctgcggttatatgcccgatcaagatcctgcaaaacgatcgggaccgcggatcatagcctaaactgcgcaagagatcttctgtttctcacagattttcccgatttatccacaggactttccagaactcgctaagtgtaaacgatcctgccgcgaggcgggcacgatttacgccgcatattggaaaatttaatgaccatagacaaaaattggcttaatcgatctaataaagatccaggacgatccttgcgctttacccatcagcccgtataatcctccacccggcgcgccatgctggtttccactggtgtgaggtcgtacattttccctgcgaaaaggtgcggaaaagcgcggtaaataaggaaagagaattgactccggagtgtacaattattacaatccggcctctttaatcacccatggcttcggtgtccatcgtttcatttttcggcggatatccaataaagccattgaatttattcaagtttaggtagaaatcgccatgaaacgcacttttcaaccgtctgtactgaagcgcaaccgttctcacggcttccgtgctcgtatggctactaaaaatggtcgtcaggttctggcacgtcgtcgtgctaaaggccgcgctcgtctgaccgtttctaagtaataaagctaacccctgagtggttaagctcgcatttcccagggagttacgcttgttaactcccagtcaattcacattcgtcttccagcagccacaacgggctggcacgccgcaaattaccattctcggccgcctgaattcgctggggcatccccgtatcggtcttacagtcgccaagaaaaacgttcgacgcgcccatgaacgcaatcggattaaacgtctgacgcgtgaaagcttccgtctgcgccaacatgaactcccggctatggatttcgtggtggtggcgaaaaaaggggttgccgacctcgataaccgtgctctctcggaagcgttggaaaaattatggcgccgccactgtcgcctggctcgcgggtcctgatagccctcattcgggtctatcaacgcctgattagtccgctactcgggccgcattgtcgtttcactccaacctgttcaagctacggaattgaggcattgcgcaggtttggagtgataaaaggcagttggttgacggtgaaacgcgtattaaaatgccaccctttacaccctggtggtgacgatcccgtcccgcccggaccatttgataccagagaacactaacgatggattcgcaacgcaatcttttagtcatcgctttgctgttcgtgtctttcatgatctggcaagcctgggagcaggataaaaacccgcaacctcaggcccaacagaccacgcagacaacgaccaccgcagcgggtagcgccgccgaccagggcgtaccggccagtggccaggggaaactgatctcggttaagaccgacgtgcttgatctgaccatcaacacccgtggtggtgatgttgagcaagctctgctgcctgcttacccgaaagagctgaactctacccagccgttccagctgttggaaacttcaccgcagtttatttatcaggcacagagcggtctgaccggtcgtgatggcccggataacccggctaacggcccgcgtccgctgtataacgttgaaaaagacgcttatgtgctggctgaaggtcaaaacgaactgcaggtgccgatgacgtataccgacgcggcaggcaacacgtttaccaaaacgtttgtcctgaaacgtggtgattacgctgtcaacgtcaactacaacgtgcagaacgctggcgagaaaccgctggaaatctcctcgtttggtcagttgaagcaatccatcactctgccaccgcatctcgataccggaagcagcaacttcgcactgcacaccttccgtggcgcggcgtactccacgcctgacgagaagtatgagaaatacaagttcgataccattgccgataacgaaaacctgaacatctcttcgaaaggtggttgggtggcgatgctgcaacagtatttcgcgacggcgtggatcccgcataacgacggtaccaacaacttctataccgctaatctgggtaacggcatcgccgctatcggctataaatctcagccggtactggttcagcctggtcagactggcgcgatgaacagcaccctgtgggttggcccggaaatccaggacaaaatggcagctgttgctccgcacctggatctgaccgttgattacggttggttgtggttcatctctcagccgctgttcaaactgctgaaatggatccatagctttgtgggtaactggggcttctccattatcatcatcacctttatcgttcgtggcatcatgtacccgctgaccaaagcgcagtacacctccatggcgaagatgcgtatgttgcagccgaagattcaggcaatgcgtgagcgtctgggcgatgacaaacagcgtatcagccaggaaatgatggcgctgtacaaagctgagaaggttaacccgctgggcggctgcttcccgctgctgatccagatgccaatcttcctggcgttgtactacatgctgatgggttccgttgaactgcgtcaggcaccgtttgcactgtggatccacgacctgtcggcacaggacccgtactacatcctgccgatcctgatgggcgtaacgatgttcttcattcagaagatgtcgccgaccacagtgaccgacccgatgcagcagaagatcatgacctttatgccggtcatcttcaccgtgttcttcctgtggttcccgtcaggtctggtgctgtactatatcgtcagcaacctggtaaccattattcagcagcagctgatttaccgtggtctggaaaaacgtggcctgcatagccgcgagaagaaaaaatcctgattcggtgagttttcgctaaaataagggcggtcagttgaccgccttttttcttttcgtagggcggataagcaccgcgcatccgccacacaaagcaacaggaacatcatgagcgataatgacactatcgtagcccaggccacgcctccgggacgtggcggcgttggcatcctgcgcatctccggcttcaaagcccgtgaagttgccgaaaccgtgctgggtaaactgcctaagccgcgctacgccgattatcttccgtttaaagacgccgacggcagcgtgctcgatcaggggattgcgctatggttccctggcccgaactcgttcaccggcgaagatgtgctggaactgcaaggtcatggcggtccggtgatcctcgacctgctgttaaaacgcattctgaccattcccggcctgcggattgctcgccctggtgagttttccgaacgcgcgtttcttaacgataaacttgacttagcccaggccgaggcgattgccgatcttatcgacgccagttcggaacaggcggcccgttcggcacttaactcgctgcaaggcgcattctccgcacgggttaatcatctggtagaagccctcacccacttgcgcatttacgtcgaagcggcaattgatttccccgatgaagagatcgatttcctctccgacggaaaaattgaagcccagctcaatgacgttattgccgatcttgatgcagtgcgtgctgaagcacgtcagggtagtttgttgcgcgaagggatgaaagtggtgattgccggacgtcctaacgccggtaaatcgagcctgttaaacgcgctggcggggcgtgaagcggcaatcgtaaccgatatcgccggaactacgcgtgacgtgctgcgtgagcatatccacattgacggaatgccgctgcatatcatcgataccgccgggctacgtgaagccagtgacgaagtagaacgtattggtatcgagcgcgcgtggcaggaaattgaacaggccgaccgcgtgctgtttatggtcgatggcaccacaacagacgccgtggatccggcagagatctggccggaatttattgcccgtctgccagcgaaactgccgatcaccgtggtgcgcaataaagccgatatcaccggcgaaacgctgggaatgagtgaagtgaacggtcacgcgttaattcgtctctcggcaaggactggtgaaggcgtggacgtgctgcgtaaccatctcaaacagagcatgggctttgacaccaacatggaaggcggcttcctggcgcgtcgtcgccacctacaggcgctggaacaggcagcggaacatctacaacagggcaaagcgcaactgttgggagcctgggcaggtgaactgctggcggaagagttgcgtctggcacagcagaacttaagcgaaatcaccggggaatttacttcagacgacctgctggggcggattttctccagcttctgtattggtaagtaaccgcgcttacgaagccgcattctgactgtcagatgcggcttcgcttcattgttaccactcctgttattcctcaaccctttttttaaacattaaaattcttacgtaatttataatctttaaaaaaagcatttaatattgctccccgaacgattgtgattcgattcacatttaaacaatttcagaatagacaaaaactctgagtgtaataatgtagcctcgtgtcttgcgaggataagtgcattatgaatatcttacatatatgtgtgacctcaaaatggttcaatattgacaacaaaattgtcgatcaccgcccttgatttgcccttctgtagccatcaccagagccaaaccgattagattcaatgtgatctatttgtttgctatatcttaattttgccttttgcaaaggtcatctctcgtttatttacttgttttagtaaatgatggtgcttgcatatatatctggcgaattaatcggtatagcagatgtaatattcacagggatcactgtaattaaaataaatgaaggattatgtaatggaaaactttaaacatctccctgaaccgttccgcattcgtgttattgagccagtaaaacgtaccactcgcgcttatcgtgaagaggcaattattaaatccggtatgaacccgttcctgctggatagcgaagatgtttttatcgatttactgaccgacagcggcaccggggcggtgacgcagagcatgcaggctgcgatgatgcgcggcgacgaagcctacagcggcagtcgtagctactatgcgttagccgagtcagtgaaaaatatctttggttatcaatacaccattccgactcaccagggccgtggcgcagagcaaatctatattccggtactgattaaaaaacgcgagcaggaaaaaggcctggatcgcagcaaaatggtggcgttctctaactatttctttgataccacgcagggccatagccagatcaacggctgtaccgtgcgtaacgtctatatcaaagaagccttcgatacgggcgtgcgttacgactttaaaggcaactttgaccttgagggattagaacgcggtattgaagaagttggtccgaataacgtgccgtatatcgttgcaaccatcaccagtaactctgcaggtggtcagccggtttcactggcaaacttaaaagcgatgtacagcatcgcgaagaaatacgatattccggtggtaatggactccgcgcgctttgctgaaaacgcctatttcatcaagcagcgtgaagcagaatacaaagactggaccatcgagcagatcacccgcgaaacctacaaatatgccgatatgctggcgatgtccgccaagaaagatgcgatggtgccgatgggcggcctgctgtgcatgaaagacgacagcttctttgatgtgtacaccgagtgcagaaccctttgcgtggtgcaggaaggcttcccgacatatggcggcctggaaggcggcgcgatggagcgtctggcggtaggtctgtatgacggcatgaatctcgactggctggcttatcgtatcgcgcaggtacagtatctggtcgatggtctggaagagattggcgttgtctgccagcaggcgggcggtcacgcggcattcgttgatgccggtaaactgttgccgcatatcccggcagaccagttcccggcacaggcgctggcctgcgagctgtataaagtcgccggtatccgtgcggtagaaattggctctttcctgttaggccgcgatccgaaaaccggtaaacaactgccatgcccggctgaactgctgcgtttaaccattccgcgcgcaacatatactcaaacacatatggacttcattattgaagcctttaaacatgtgaaagagaacgcggcgaatattaaaggattaacctttacgtacgaaccgaaagtattgcgtcacttcaccgcaaaacttaaagaagtttaattaatactacagagtggctataaggatgttagccactctcttaccctacatcctcaataacaaaaatagccttcctctaaaggtggcatcatgactgatcaagctgaaaaaaagcactctgcattttggggtgttatggttatagcaggtacagtaattggtggaggtatgtttgctttacctgttgatcttgccggtgcctggtttttctggggtgcctttatccttatcattgcctggttttcaatgcttcattccgggttattgttattagaagcaaatttaaattatcccgtcggctccagttttaacaccatcaccaaagatttaatcggtaacacctggaacattatcagcggtattaccgttgccttcgttctctatatcctcacttatgcctatatctctgctaatggtgcgatcattagtgaaacgatatcaatgaatttgggttatcacgctaatccacgtattgtcgggatctgcacagccattttcgttgccagcgtattgtggttaagttcgttagccgccagtcgtattacctcattgttcctcgggctgaagattatctcctttgtgatcgtgtttggttcttttttcttccaggtcgattactccattctgcgcgacgccaccagctccactgcgggaacgtcttacttcccgtatatctttatggctttgccggtgtgtctggcgtcatttggtttccacggcaatattcccagcctgattatttgctatggaaaacgcaaagataagttaatcaaaagcgtggtatttggttcgctgctggcgctggtgatttatctcttctggctctattgcaccatggggaatattccgcgagaaagctttaaggcgattatctcctcaggcggcaacgttgattcgctggtgaaatcgttcctcggcaccaaacagcacggcattatcgagttttgcctgctggtgttctctaacttagctgttgccagttcgttctttggtgtcacgctggggttgttcgattatctggcggacctgtttaagattgataactcccacggcgggcgtttcaaaaccgtgctgttaaccttcctgccacctgcgttgttgtatctgatcttcccgaacggctttatttacgggatcggcggtgccgggctgtgcgccaccatctgggcggtcattattcccgcagtgcttgcaatcaaagctcgcaagaagtttcccaatcagatgttcacggtctggggcggcaatcttattccggcgattgtcattctctttggtataaccgtgattttgtgctggttcggcaacgtctttaacgtgttacctaaatttggctaaatccttcaagaagccagccattcgctggcttcttgcctctcaggaaatcacttatgtccaaatggcaactcgcctgatcctccttcaccacgtatgctttgcgtcaccttactatcaggacgctttagcccatgtcccgctttttgatttgtagttttgccctggttttactttatcccgccgggattgatatgtacctcgttggtttaccgcgcatcgccgccgatctcaatgccagcgaagcgcagttgcatattgcgttctccgtatatctggcggggatggcagctgcgatgttatttgccggtaaagtggccgatcgttcagggagaaagccggtcgccatacccggcgcggcgctatttattattgcctcggtgttctgttcactggctgaaaccagcacgttatttcttgcaggccgatttctacaggggttgggcgcaggctgttgttacgtagtggcgttcgctattttgcgcgacacgctggatgatcgacgtcgggctaaagtgctgtcattactcaacggtattacctgcatcattccggtgttagcgccagtgctcggacatctgattatgcttaaattcccgtggcagagtctgttctgggcgatggcaatgatgggcatcgcggtactgatgttgtctttgtttattttaaaagaaacgcgcccagcggcccccgcagcttcggataaaccacgagaaaatagcgagtcgctgcttaaccgttttttcctcagccgtgttgttatcaccaccctcagcgtttcggtgatcctcactttcgtcaacacgtcaccggtattgctgatggaaatcatggggtttgagcgcggtgaatacgccaccattatggcgctgaccgctggcgtcagcatgaccgtttcattctccacgccatttgcgctgggaatttttaagccacgtacgttgatgatcacctcgcaggtgttattcctggcggcggggatcactcttgccgtttcaccttcccatgcggtttctctgtttggtatcacgctgatttgcgccggtttctcggtaggttttggtgtggcgatgagtcaggcgttagggccgttttcattacgcgcgggcgtagccagctcgaccttaggtattgcgcaggtttgcggttcgtcactgtggatttggctggcagcggtggttggtatcggcgcatggaatatgctgatcgggattctgattgcctgtagcatagtgagcctgttgctgattatgttcgtcgcgcctggacgccccgttgccgctcatgaagaaatccatcaccacgcttgatctcaatctgctgctttgtctgcaactgctgatgcaggagcgcagcgtaaccaaagcggcgaagcggataaacgtgacaccttcggcggtgagtaagtcgctggcaaagttaagagcgtggtttgacgacccgctctttgtgaactcaccgctgggtctgtcgcccacaccgctgatggtcagcatggagcaaaatctggcggagtggatgcaaatgagcaacctgctgctggataaaccgcaccaccagacaccgcgcggcctgaagtttgagctggcggcggaatcaccgctgatgatgatcatgcttaatgcgctgtcgaaacagatctaccaacgttacccgcaggcgaccatcaaattacgtaactgggattacgattccttagatgccattactcgtggtgaagtggatatcggtttttccggtcgcgaaagccatcctcgctcgcgggagctgttaagctcgctaccgttagccattgattatgaagtgctgtttagtgatgtgccctgcgtctggttacgcaaagatcatccggcactgcatcaaacgtggaatctggacaccttcttacgttatccgcatatcagcatttgctgggaacagagcgatacctgggcgctggacaatgtgttacaggagctgggacgcgaacgcacgattgctatgagcctgccggaattcgagcagtcactgtttatggcagcgcaacccgacaatctgctactggcgaccgcgccgcgctactgtcagtactacaatcaactccatcaactgccgttggttgctcttcctctcccgtttgacgaaagccagcaaaaaaagctggaagttccttttaccctgctgtggcataaacggaacagccataatccgaagatcgtctggttacgggaaaccattaaaaacctttacgcgtcgatggcataaccgaatcgtatgaaacgcgacccaatttcacaataaaatgtaaaaaagttgtaataagcttgtctgaatcgaacttttagccgctttagtctgtccatcattccagtaaatgattactcttgtattcataatggaccattaagcatggagcgaaaaatggcgactcactttgcccgagggattttaacggaaggacatctgatttctgttcgtctcccctcccagtgtcatcaagaagcccgaaacattccccctcatcgtcaaagccgttttctggcgtccagaggtttactcgcagaactgatgttcatgctgtatggcattggcgaattgccggaaatcgtcaccctgccgaaaggtaaaccggttttcagtgataaaaatttgccttcgttttccatttcctatgccgggaatatggttggcgtggcgttaacaaccgaaggtgaatgtggcctcgatatggaactacagcgtgcgacgcgcgggtttcatagcccacacgcgcccgataaccacaccttttccagcaatgaatcgctatggatcagtaaacaaaacgatcctaacgaagcgcgggcgcagctcatcacgctgcgccgaagcgtgctaaaactaaccggtgatgttttgaatgacgatccgcgcgatctgcagctgctgcccattgccggacgcctgaaatgtgctcatgtaaatcatgtagaagcgttatgcgacgcggaagacgtgctggtgtggtccgtggcggtcacgcccacgattgaaaagctcagtgtctgggagttagatggcaaacacggctggaaaagcctgccggatattcacagccgcgccaacaatcctaccagccggatgatgcgttttgcccaactctctaccgtgaaggctttttcgccaaattgatagacaaccacaggagtcatcatgtctgaaaaattgcaggtggttacgttactggggagcctgcgcaaaggctcatttaatggcatggttgcacgtaccctgccgaaaattgctccggcgagcatggaagtcaatgcgttaccatccattgccgacattcccttgtatgacgctgacgtacagcaggaagaaggttttccagcaacggttgaagctctggcggaacagatccgtcaggctgacggtgtggtgatcgtcacgccggaatataactactcggtaccgggtgggctgaaaaatgccatcgactggctttcccgcctgccggatcaaccgctggccggtaaaccggtattgattcagaccagctcaatgggcgtgattggcggcgcgcgctgtcagtatcacctgcgccagattctggttttcctcgatgcaatggtgatgaacaagccggaatttatgggcggcgtgattcagaacaaagttgatccgcaaaccggagaagtgattgatcagggtacgctggaccacctgaccgggcaattgaccgcatttggtgagtttattcagcgagttaagatctaaataaaaaacccgccagcaatcatgcatggcgggtttttaacgcgctatcgattttagtgagcgtcgataaagacaatcttcaggataaacagcagcgcaacgatgattacgcacgggcttagatcacgcagacgtccggtaccgattttcatcacgcagtaggagataaagcccagcgcgataccttcggtaatcgagaagctgaacggcatcatcacggcggtaataaacgccggaacagattcagtaagatcctgccagttcacgcgtgccagactggaagtcatcagcacgccaacgtaaatcagcgcaccagctgcagcgtagcctggcaccatccccgccagcggcgacagaaagataaccagcaggaacagcagaccaacaaccactgccgtcagaccggtacgaccgccaaccgatacgccggaagaggactcaatataagccgtaacggaagaagtaccgataaacgaaccggtcacggaagagatactgtcgacatacagcgcctgcttcatgcgcgggaatttccccttctcatccgccagacctgctttatcggtcacgccaatcagcgtaccggaggagtcaaacaagttgaccaacatgaaagagaaaatcacccctgccagcccgaggttaaacgacccggctaaatctacatgacccacaactgtcattacgctcggcggcgcagaaacgatgccattgtagtgcacatcacccagcatccagcccagcagcgtcgtcaccacgatagaaaccagcaccgctgcgtgaatgttgcgcgaggccagaatagcaatgatgaagaagccgaggatacccagaagtacgctgtgagaagtcagattaccgatgctcaccagcgtttccgggttagcgacaatcacacctgcgtttttcagccccatcatgccaatgaacagaccgataccgctggtaatacccacacgcagactcaccggaatgttggctatcatccagtagcgaacgcggaaaatcgtcagtaacagcagacctatcgcgccccagaagattgcgcccatcccgacctgccacggcaagcccatcgcctgtacaacgacaaaagcgaagaacgcattcaggcccatagcgggtgccagtgcaactggcaggttagcaaacagtcccatcataatactgccgaatgcagcgatcagacaggtagtgacgaagacggcgctggtatccatgccagcaacgccaagaatttgcgggttaacaaaaacgatgtaaaccatcgtcaggaaggtggtaaaaccggcgatcacttcggtccgtgccgtcgtgccatgttcgcgcagtttaaacacgcgttccagcatcccctgaccagaagtctgggtggtatgttgatgactcattatctatttccgaacaaggagggaaaatccgtcgctatcgtataccaaaatgcgacaataggcgcgtttgtgagagacttttttattggatttacttatacggcaacgattgcgttgcgcaaatcggctctacgaaaacgttaaactgattaaaaaggaaaggcatgtcccggatagaagcggtatttttcgactgcgacggtacgctggtcgacagtgaagtcatttgctctcgcgcatatgtaacgatgtttcaggaatttggtattacgctcgatcctgaagaggtattcaaacgtttcaaaggtgtaaaactgtacgaaattatcgatattgtttcccttgaacatggtgttacgttagcgaaaacagaagctgaacacgtttaccgtgcagaagtcgctcggctgttcgattcagaactggaagccatcgaaggggctggagcgctcctgtcagcgatcactgcgccaatgtgtgtggtatctaacggcccaaataacaaaatgcagcattctatgggcaagctgaatatgttgcactacttcccggataaactgttcagcggctacgatattcagcgctggaagccagacccggcgttaatgttccatgcggcaaaagcgatgaatgtaaatgtagaaaactgcattctggttgatgactcagttgccggtgcacaatctggtatcgacgcaggtatggaagtgttctacttctgcgccgacccgcacaataagccgatcgttcacccgaaagtcaccacctttacccatctttcgcagttacctgaactgtggaaagcgcgtggttgggatattacggcatagttcttcacactcccttcacttaccccgcttaaattggcgctcaaaggtaagtaaagggagtttgatatgtctgtttcacgtcgggtaatacatcacggactttattttgcagttttaggaccgttaattggtgttctgtttcttgtcctctacatattcttcgcaaaagaaccgctggttctttgggtgataatacatccaatttttctcttattgtcgataactacgggagctattcctgcgttgttaaccggtgtaatggttgcctgtctgccggaaaagatcgggtcacagaaacgttatcgttgtctggctggtggcataggtggcgtcgttatcaccgagatctattgtgcagttattgtacatattaagggcatggcttcctcggagttgtttgaaaacattctttctggtgacagtctcgttgtccgcatcattcctgcattgctggcaggtgtggtgatgagcagaatcattacccgtctacccggattggatatttcatgtcctgaaacagactctttaagttaagcgggatactttatctttgggctactcaaaagcagacaggatgtttctatgactcaaaatatcaggccgttaccccaattcaaatatcatcccaagccactggaaacaggcgcatttgaacaggataaaaccgtagagtgcgattgctgtgaacaacagacgtcagtttattactcgggtcccttttattgcgttgatgaagttgaacatctctgtccgtggtgtattgcggacggttctgctgctgaaaagtttgcaggtagttttcaggatgatgccagcatagaaggtgttgaatttgagtatgatgaagaggacgaatttgccggtattaagaacacatatcctgatgaaatgctgaaagagttggttgaacgcacgccaggttatcatggatggcagcaggaattctggctcgcgcattgtggcgatttctgtgtttttatcggctatgtgggctggaatgatataaaagatcgcctcgatgaatttgccaaccttgaagaagattgtgagaatttcggtattagaaattctgatctagctaaatgcctgcaaaagggtggtcattgtcagggttatctcttccgctgtctccactgcggcaagctgagactgtggggtgatttttcgtagttatttaaataatgagaacaggccggagcgtaattcacacatccggccttatttcttaagcttaaccgagtgctaattctgcggcagcggctttatcagcgattaccatcagcgaaggatgcagctgcaacacggaagctggaacatcttcggtaaccggaccttgcagaacatttttcagtgcctgcgctttacccgcgccgctgacaattatcagcaagtttttcgccgccatgatgcttttcggccccatcgtcacgtagctgtcaggcactaacgaaaagtcgccgcccaactcgccatgcgccacaatatcaaccatctctccctggatcgggaactccacggtttgctcatggaaatgggtcgtattcggcaaattgccacaaaaatgaccatctgcacctaatcccagcaccaccaaatccagtccgccttcacgcgccagtttctgatcatgctcgcggtagttatcaatagtgagcttctggatattctcttctttgatccccgcaggggtgaaaaacagattacgcagattggtaatcgttacgccttctccctctttgccgcgaaatggaatttcatcaaaattatagaaatagcagttatcgtaccagggcttacctttaaccagggtggtgaggtattcatacatgcctttgggcgtgctaccggcggtaattgccaggttaacacgacgcgtcttcgacatataaccaagcagatggtgtgccgcgacacggctcatttcctggtaatcttcggtaatgattaatttcatcttaatgccttattttatttaaataatttctgtacaaaggctgcataggctggtcgccagacatccatttcatggttcagacccggatattcctggtaatcaaagttaatttttttctgctcaagctcagttttcagcccggcgatatccttgccggttacgacatctttatcccccacaaccacagtaaaattacgtagttgctggttgatagctgccggatcgttcagtcgggccgcgacaccttcatccggtacggttgtcgtggtaacaccactgaatgtggccagccagccaaagctttccagatgattcattccggaaaccagcgcctggtacccgccttgtgaaagccctgccagcgcgcggccatcggcatctttacggacattaaaacgcttgctaatcagcgggataatatcgttcatcagttcgcgatctgccgctttagcattcagcggataaaagactttacgtctttcctgaggcacgaaatcttcgggaataatgcccttcgcatcggtttctgtatccgggatcaccaccagcatcggtttaattttcccttcagcaagcaggttatccatgatttgcgggatacgcccctgatcgatagcggaacgtccggtatcaccaaagccgtgatagaaatagagcactggcaaaggctcgcccatgccggtgtatcctggcggggtccagacatacatctgacgttcagattgcaatgcgttggagtggtaagttatggcgatcaaatcaccatgcgcaacagaacgcgtatccagataactgcctggcaccagaatcatactggagttaacctggcgctgaggattagtcattgcggtgcctgtatcaatgctgcgtacaccatcaacattgaaaaaatactcgtacaggttgcctttcaggataggtgtgcgccacgaccagactcctgcttcgtctttggtcatcgggtgaatattgtccggaaccggaacacccaccactacagagacattttttgccccaggggcaaagtagcgaaaggtcacgctgttatcggcattgacctgagtcacatactgtttcaccgggatagtgggtgccgggctggctggcatatccgctgctatggcccactgagcagaaataccgctggcaatagccagcgttaaagcagcaatttttatattcatcgtaatattcctttcattaagttccattaccaccagatttcagcctgggcaccgacagcaaactggtcgtctttattgtcttcaaaggtgaagccatccagttcgttttccagggctttgatatacgtggcgtagaaacgaatttccggacgcgaggtcaacatactggtattgactttaaaggtatggaagagcgtggttttataaccagactcattaaatttattactattcgcatctttgttttgctgggtgaaatagcccagttcaacacctgtctggttatattggtcccaaatataggccgggcgaacaaccgcacgaatagattcgaaatcagagtgggcgcctgtttcgtagctatatatatcgttaccgaaggagtaaacaatcgcgttagctacaatgaaatgatcgccaatataggcttcgccctgcgaagtcagacgtaccgctgttccgccggtgtgatcaccataataacgaccattaaaggtggtaaatggacttgcgccagcataacggccaaagttactggcgatagagttattcgcgaccaggaaggagaattcgttgaagccacctttatcaaatttctgcgttaaagatgtgccaaacatccaggtatctttccagtcataatacccgttattatcctgattatctttttccgatgcgctttcgtttgccgtgacataacgaccacttaccattaaggtggctttatcccataacgggatatctttatagcgtaaatcaatggtattggtattaatctgctgtttgttttgcaggctgcgatcgtaatcatcgacatcttcgcgaaccagcgcgatatcaattttacccggaccgactttccagttttccagacctacacccgctgcggcatcagtacgctgcgttttccagtcaagcatctggatttcaattttcggcgcaccgtgtttacccacccagaaatcagcctctggcgcaaagggcaggaaacctttggtggtaacgtacatatcggagaactgcatatagttctcgccaccggcgttatcgccaaaccagccggtagagtactgctgaccaacgttaccatccatcatcacaacggcatcaacccgtttgccgttttcgttgtagacacgttgttttaactgcaaatcaaaccagccggagtattcgttaccaaagcggcccagagaaccaatcgcccatgatttaggtgaaccatgagaggcggtcccccaaccagaacggtaatagccgttgtaactaaagccaatttcatctttcacaaatttactgaaatctttcagagtcatggaagaataaatcgagcctgtctcactggcatttttctcttcatttttgaccagtacagcatcaggttttgcggcactactggtcgggaacggattggcggcatacccttgatcattcgtacttacgctacgattcaccgtcgctggcgtatactttttcttctcttcatctttatactttttgagttcgctttgcgtttctcttaacgccttttctaataactcaaggcgttgttccaccgttaatgattcagccaatgattgtgcagaaaaggctaacggtgccattaataagatggcagaggtaataagatttcgtctaaacataatatccctttatggtgcaaagaaagaattaacgcatcgcatccagactgttctgaatgcgacgataattaaggtgctttaatggttattttttttaatgacagcccccgcgtcttgatcacctctgcataccatccgaagcttttcttgcgtgttcttgtgaggcttccttcgccattatcatcacgatccacataaataaagccgtagcgcttagacatttgtgaatgagatgcactgactaaatcaattggcccccaactggtgtaccccataatatccacaccatcggcaatcgcttcatttacctgtaccaggtgatcgtttaaataggcaattcgataatcgtcctgtatcgaaccatccgcttcaacgctgtcttttgcgcctaatccgttctcgacaataaataacggtttttgataacgatcccaaagcgtatttaacagaacccgtaatccaaccggatcaatttgccacccccactctgaacttttcagatgcggattggggatcatattcagtatgttgccctgcgcatttttattaatgctttcgtcgtgggaaacacaaccagtcatgtaataactaaaagagatgaaatcgacggtatgttttaaatcttctgcgtcactttcagtcatctcaatggtgatattgtggtcgcggaagaaacgctgcatatagccgggatactggccacgcgcctgaacatcaccaaagaacatccagcgccggttctcttccatggcctgcaacatatcctgtggctggcaggtgagggggtaaaccagcccaccgagaagcatattgccgattttcgcttcggggagcaggctatgacaggctttaactgcccgcgcactggcaaccagttgatggtggatagcctgataaacttccgcctcgccactctcttctgccagccccacgcccgtgaatggcgcgtgtaacgacatgttgatttcattaaacgtcagccataacgccactttatgttggtagcgagtaaagaccgtgcgggcgtaatgctcgaagtgatcgatgaccgctcgattagcccaaccgccgtagtttttcaccagcccatatggcatttcgtaatgggataacgttaccagcggcttgatccccgcctgcgccatttcatcaaacagccgatcgtaaaacgctaaccccgcttcattcggttcgacttcgtcgccctgagggaaaattcgcgcccaggcaatggaaatacgcagacaggtgaagcccatctcggcaaataacgcgatatcttccgggtaacggtgataaaaatcgatggcgacatctttgatattctctttccccaggatgcgcggttccatttttcccattacgccatgaggctgtaaatctgaggtcgagatccctttgccatcttcctgccaggcaccttccacctgattggcagctgttgcgccaccccaaagaaatgtttctggaaatgctttcataattaactccttttatcgttagcgaatgatggataacagcggttcacctgcgcttatctgcgccgtgccgtggggtaatacgtccgtaaaatcatcgctattactgattaataccggcgtcgtcagatcaaatccggcctcgcgaatagcagggatatcaaaagaaatcagccgatcgcctgtattgaccttgtcacccacgttgacgtgagcggaaaagaatttgccgtccagttttacggtgtcgataccgacatgaatcaggatctccacaccatcatctgactcaatgccaatggcgtgtaatgtggcgaacaacgaagcaattcgacccgcaaccggagaacgcacttcaccaaccgagggcagaatggcaatacctttacccaacaggccactggcaaacgtggtatcagcgacgtgaatgagcggcacaatctctcccgtcatcggtgaacagataccgccctgctcaggtggtgtaataacctctggtgttttctcttgcggggcaccctgcgctggctgacgtttagcggtgatgaaatgaagcatcaccgtaccgacaaatgcgcaaccgatggcaatgacaccgccaataacgctggcccagacggtgaaatcaattcccgttgacgggatggtttgcatgaaggtgaaaatacttggcaaaccaaaggagtagactttcgtttgcgcgtagccaataatggtggcccccaaagccccactgatacaggcgataacaaaggggtacttacgcggcaggttgacgccatataccgctggttcggtgataccaaacagactcgtcaacgccgctgatcccgccaccacttttttctgcgcatcgcgttcgcagaggaagacgccgagcgccgccccgacctgcgccataatggcgggcattaacagcgggatcatggtgtcgtagcccagcacggtgaagttattgatacacagcggcaccaggccccagtgcagtccgaacatgacgaagatttgccagaagccgcccattaccgcgcccgcaaatgcaggaaccgcctgataaagccagagataaccggcggcaatcagttcgcttatccaggttgatagcggccccaccagcagaaaggtgacgggtgtgataaccatcagacatagcaatggtgtgaagaaatttttgattgccgacggtaaccacgcattaagtcggcgttccagaatgctgcacaaccaggcagaaaaaataatgggaataaccgatgacgagtaattcaacaatgtgaccggaatacccaggaaatccagccccagcgcatccgctttttgcccgttctcgaaagcagtcagaattaatggatgcactaacgctccaccaatcaccatggcagtaaatggattaccgccgaagcgtttccccgcggtgtatcccaggattatcgggaagaaccaaaacaaggcatcactggcgctgaataaaattaaataagtaccactttgttcggtcgtccactgaaaagtgagcgccagagccagcatacctttcaagatcccggttgccgccatcaaaccgatcagaggcgtaaaaatacctgaaataacataaacaaagcggtttagcagattacctttatcatcattttccggtgcctgttgcgctttttcgtcaaggcctgccacactgttaaccgccaggaagacatcggccacatggttacctatgaccacctgaaactggccaccgctttccaccaccataataataccgggggtctttttcagtacctctgcttgcgctttgctttcatcctttaatttaaaacgtaatcgcgttgcgcaatgcatcagactcacaatgttatctgcgcccccgactcctgcgactatttttctggctaactccgtcataacttgccctctaccgctttgcggcaaaactccaaaaaaaaacctgaaaaaaacggcctgacgtgaatcaagcaatttttttcaggttttgcccgcttagtgcggtaacaatcctttactcagtaataatatttcagtgttctttgcgcacgcgctctatatttatggctaaaaacataatctctgcgggtgaaattttacgttgatactgcaaaccaataaaaatggcgatccgttccgcacattgccatgcttgcgggtaattttgttttactgcttgttgtaatgattcatcactatcgttaattgaagcatgttcaagaatacgccaggataaaaacttcagatgtgtaaccagtcgctgataactcaagctttcttcctggtaattaaggctgaactgaaattttattaattgcagcatttcgcgcattaactgcgtgacacctgcaacatcctccatatttccgctcatttgggcactgaccagatgcatggcaataaagcccacttcatctttcggtaactgcacgcccaaccgtttatcaataatggttaacgcttcttcccctagctggaactctttcgggtaaagccgctggatatcccacagcaacgggttgggcagcaacacgttttgctgaaagcgtttaatcgcaaactggcaatggtcagttagcgagatataaatactgtcctgtaattttcccaagcgctcctgcgctaaagagataatacgatcacaggttgccatcacctcaagaggaatatgacttaagagttcgcttaatcgcccgttcagttcatgactgctcaaggcatactctttttctattccacttgagttaattctttcgccagcgcgtttttgaaagccaattccgcgccccatgacgactttttcccgctgttgatcatcaataaccaccacaacattattgttgagaattttggtgatttgcatgttcatagcaaggaccttttttataaacaaaaaaacccgacttcaccagtattctctggttatgtcaggttttgcctgcgaatgcagtaacaatccagtcatttattaatggtttttataacgaacatccaggttcggaaattaatttaattgcgtgcagagaaaatagcaatgcgctattgataaaaatatgaccatgctcgcagttattaactttgtgtaattttaggaatttataaagttatatataacaaatcccaataattaagttattgggatttgtctggtgaattatttgtcgctatctttccccgccagcagtttatccagctcatcgccaccgacgtgacggaaatcctgccccttcacgtagtagaagataaactcacaaatattctggcagcggtcgccaatacgttcgatagaacgcgcgcagaacagcgcagtaagtacgctcggaatggtacgcgaatcttccatcatgtaggtcatcagttgacgaacaataccttcgtattcctgatcgacttttttatcttcacgataaatacgtaccgcttcgtcaatgtccatccgcgcgaacgcgtccagcacgtcgtgcagcatctggatggtatgacggcccagcgactccagacttaccagcaacggctgatgctgctgggagaatttctccagcgcagtacggcagattttgtccgccacgtcgccaatacgctccagctcggcaatggttttactgatcaccataaccagtcgcaggtcgctcgccgtcggctgacgtttggcgataatgcgcacgcaggcttcatcgatcgccacttccatcatgttgacgttcttgtcgccttcgatgacgcgcttcgccagatcgctgtcctggttatgcatcgcggtgattgcatcagaaagctgctgctccaccatgccgcccatggtcatcacctgcgtgcggatactttccagttcggcgttgaactggccggaaatatgtttattaagattgagactgtccataacgcactcctgaatcaaccgtaacgaccggtgatgtagtcttctgtttgtttcttcgctggcttggtgaacagatcgtccgtgttgctgaactcaatcaattcgcccaggtacataaacgccgtgtggtcggaacaacgcgcagcctgctgcatgttgtgggtgacgatcaccacggtgtaatcctgcttcagttcggtgatcagctcttcaatacgcccggtagagatagggtcgagcgccgaacacggttcgtcgagcagcagcacttccgggcgaatggcgataccacgcgcaatacacagacgctgttgctgaccaccagagagagagtaaccgctctggtgcaatttatctttggtttcgttccacaatgcggctttggtcaatgcccactgcacgcgctcgtccatgtcggcacgggagagcttctcaaacagacgaacgccaaaagcgatgttgtcgtagatggacatcggaaacggcgtcggtttctggaacaccatgcccactttcgcacgcagcagtgcgatatcctgagagttggtcaggatgttgtcgccatcaagcagaatttcaccttccgcacgctgctccgggtacagttcaaacattttgttgaaggtacgcagcagcgtcgatttaccgcagccggacggcccgataaacgccgttacctggtttttagcgatatccaggttgatgtttttcagggcatggaatttgccgtagtagaagttcaaattacgaacctgaattttactcggggcagtttcaaccatactcattgcaatcttttcctcatcgtgcctgatgcacttcgctaatcaggcttaccgtaggccggatcaggcgttcacgccgcatccggcaaagtgttaaccgtgtacagagtcaaaaaggcgctcggtcggtcccctcgcccctctggggagagggttagggtgaggggaaaaccgtgtcagcaatatcaaccgtgtttattcttcgcaaaaacaacgcgcgccagaatgttcagcagcagtacgcacagggtaatgatcaataccccggcccaggccaattgctgccattccgcaaacgggctcatcgcaaacttaaagatcgtcaccggcaggttggcgatcggctgcatcatgtccgtgctccagaactggttggagagcgcggtaaacagcagcggcgcggtttcaccagcaatacgggcaatcgccagcaggataccggtcataatcccggacaccgacgctttcagcgtaatcgcagagatcatcttccacttcggtgtacccagcgcataagccgcttcacgcaggctgtacggcaccagtttcagcatgttctcggtggtgcggataacaatcggcacctgcaacaacgccagggcaatcacgcccgcccagccggagaagtgctccatctgcgccaccacaatggtgtaaacaaacagaccaaccacaatcgacggcgcagagagcagaatgtcgttaatgaagcgaatcacttctgccagccaggatttacgaccatattccgccagataaatccccgccataatgcccagcggcgtaccgaataccgtggcccacaaaattaacagcccgctacccgccagagcgttcgccagaccaccaccttccgtattgggcggcggcgtcatttcagtgaacagcgccagcgacataccgtcgataccgcgagtgatggtggacattaaaatccagatcagccagaacaggccgaaggccatcgtcgccatcgagagcgtcagcgcaatacggtttttgaggcggcgacgcgcctgcattttgcggcgagattcagccagcgccgcagtggtttgcatttcaaccatagccattagcgtgccccctcattcttagccaggcgcataatcataaacttcgatgcggcgaggacgatgaaggtaatcacaaacaggatcaggcccagttccatcagtgcggcaacgtgcagaccggattccgcttccgcaaattcgttcgccagcgcagaggtgatactgttgcccggcatatacagcgaggcgctgtcgagctggtaggtgttaccgatgataaaggtcaccgccatggtttcaccgagcgcgcggcccagccccagcatgatgccgccgataacaccatttttggtgaacggaagaacgatacgccagataacttcccaggtggtgcagccaataccgtaggccgactctttcatcatcaccggggtttgttcgaacacatcacgcattaccgccgcaatgtacggaataatcatgatggcgaggatcacgcctgccgcgaggataccgataccaaatgcggggccagagaacagcgcgccaacaatcgggatattcgacatgatattgccgaccggctcctgaaagtaaacggcgaacagcggcgcaaagataaacaggccccacatgccgtaaacgatacttggaatggctgccagcagctcaatggcgatacccagcgggcgtttcagccagccaggcgcaagctcagtcaggaacagggcgataccgaaactcaccgggacggcgatcagcagcgcgataaacgaagtcaccaacgtaccgtagatcggcaccagcgccccgtagatatcgttcggtgcatcccactctttggtccataggaaagccagaccaaatttctgaatgctcggccaggaggagatgatcagagagacaataatgccacccaacatcaatagcacaatcagcgccgccagttttaccagcacgctgaaaattatgtcgccctttttacccggtgggttaaaagcaggcttggttgcagccataagttactcttcagttaaacgcgtttacaaagtcattttgtaatgccggatgcggcgtaaaacaccgtacccggcctggagttttattagtacagcggcttaccgctactgtctttaatattggtcttccacgcagcgcgaacctgttcaactacactatccggcaggctggcgtaatccaggtcgttcgcctgtttagccccggttttgtacgcccagtcgaagaatttcagcacttctgtgccttgttctggtttcttctgatctttgtggatcagaatgaacgtggtagaggtaataggccatgcatcttcgcctttctggttggtcagatcctgagcgaaggttttgctccagtctgcaccttttgctgcattagcgaagttttcttcggtcggactaaccggtttaccatcagcggagatcagtttggtgtacgccaggttgttctgcttcgcgtaagcatattcaacataaccaattgcacccggcagacgctgaacgaacgcggcgataccgtcgttacctttaccgcccagaccgatcggccattttacggtagagccagtaccaacgttgtttttccactcttcgttcactttcgccaggtagctggtgaagacgaaggaagtcccggagccatctgcgcggcgtactacagcaatgttttgtgaaggcagtttcagacccggattcagtttggcgatggcttcatcatcccacttcttgattttgcccaggtagatgtcgccgagggttttaccatccagcaccagttcgccagacttcagccctggaatgttaaccgccagcaccacgccgccaatcacggtcgggaactggaacagaccttcctgagccagtttttcgtcagacagcggcgcgtcagaggcaccaaaatcaacggtattagcgataatctgttttacgccaccggaagaaccgataccctggtagttaactttattaccggtttctttctggtaagtgtcagcccatttggcatacaccggcgcagggaaggttgcacctgcacctgtcaggcttgcttctgcaaacacagagaaagcactcatcgataaggtcgcggcgacaacagttgcgacggtggtacgcataactttcataatgtctcctgggaggattcataaagcattgtttgttggctacgagaagcaaaataggacaaacaggtgacagttatatgtaaggaatatgacagttttatgacagagagataaagtcttcagtctgatttaaataagcgttgatattcagtcaattacaaacattaataacgaagagatgacagaaaaattttcattctgtgacagagaaaaagtagccgaagatgacggtttgtcacatggagttggcaggatgtttgattaaaaacataacaggaagaaaaatgccccgcttacgcagggcatccatttattactcaaccgtaaccgattttgccaggttacgcggctggtcaacgtcggtgcctttgatcagcgcgacatggtaagccagcagctgcagcggaacggtgtagaagatcggtgcaatcacctcttccacatgcggcatctcgatgatgtgcatgttatcgctacttacaaaacccgcatcctgatcggcgaagacatacaactgaccgccacgcgcgcgaacttcttcaatgttggatttcagtttttccagcaattcgttgttcggtgcaacaacaataaccggcatatcggcatcaattagcgccagcggaccgtgtttcagttcgccagcagcgtaggcttcagcgtgaatgtaagagatctctttcaacttcaatgcgccttccagcgcgattgggtactgatcgccacggcccaggaacagcgcgtgatgtttgtcagagaaatcttctgccagcgcttcaatgcgtttgtcctgagacagcatctgctcaatacggctcggcagcgcctgcagaccatgcacgatgtcatgttcaatggaggcatccagacctttcaggcgagacagcttcgccaccagcatcaacagcacagttaactgagtggtgaatgctttagtggatgccacgccgatttctgtacccgcgttggtcattagcgccagatcggattcgcgcaccagagaagaacccggaacgttacagattgccagtgaaccaaggtaacccagctctttcgacagacgcaggccagccagggtatccgcggtttcgccagactgtgacaaggtgatcatcaggctgttacgacgcacggcagatttgcgatagcggaattcagaggcgatttcgacgtcgcacggaatacctgctagcgattcaaaccagtagcgggaaaccataccggagttataagaagtaccacaggcgaggatctgaatatgctcaaccttcgacagcagttcgtcggcgttcggtcccagctcgcttaaatcaacctgaccgtggctgatgcgtccggtaagggtgtttttgatcgcgttcggctgttcgtagatctctttctgcatgtagtgacggtaaatgcctttatcgcccgcgtcatattgcagattggattcgatatcctgacgttttacttccgcgccagttttatcgaagatgtttaccgaacggcgagtgatttccgcaatatcgccctcttcaaggaagataaagcgacgggtcaccggcaacagcgccagctggtcagaagcgataaagttttcgcccatccccaggccaatcaccagcggactaccagaacgtgccgccagcagggtatccgggtgacgggagtccatgatcactgtaccgtacgcaccacgcagctgcgggatagcacgcagaacggcctcacgcagagtcccgccttgtttcagctcccagttcaccagatgggcaatcacttcggtgtcggtttcagaaacgaaggtatagccacgcgcttttagctcttcacgcagcggttcatggttttcgatgatgccgttatgcaccaccacaatgtgttcagaaacatgcggatgcgcattcacttctgaaggttcaccgtgggtcgcccagcgagtgtgagcaataccagtgccgccatgcagaggatgttcttccgctgcctgtgccagcatctggactttaccgaggcgacgcaggcgggtcatatgaccttctgcatcaacaacggccagaccggcagagtcatatccgcggtattccagacgacgtaaaccttcaagaaggatttctgctacatcacgttgcgcgatcgcgccaacaattccacacatagtttttgattccgatttatatcgttgtcggtcaacctgtatgcccgttttttcgggcgccccgagccttgtagagagtggggttatttttatagttactgcttgtgggagggagattatgttatctcctcatcccatgtgaccgggttagccggccagaatcactttttctttaccggacgacgccagccttctttctgagtctgcggcacacggctgatagctaatgcattttcgccgacattacgcgtcacagttgtacccgcagcaatggtcgcgcctttgcctactgttaccggggccaccagctgagtgtcggaaccaacaaacacatcgtcgccgataatggtcttaaatttattcgcaccatcgtagttgcaggtaatggttcccgcgccgatgttaacgttatcgccaatttccgcatcgcccaggtaagtcagatgaccagctttcgagcctttacccagacgcgcttttttcatctcaacgaagttaccgacgtgagcaccttccagcaactcagcaccaggacgcaaacgggcaaacgggccaatggtacaggccgctgccagattcgcatcttccacaacggtatacggactgatttcgcaatcatcgccaatcacgctgtttttaatcacgcaaccggtgccaattttcacgcgatgaccgagagtcacgttgccctcgatgataacgttagtatcaatttcaacatcgcgcccgtgagttagcgtaccacgcagatcaaaacgcgctggatcgcgcagcataacgcctgctaacagcagtttttcagcctgttcggactgataaacacgctccagacgggagagttgcaggcggttattcacgccttctacttcgcttaaacgttgcggatgaacggcgacgatttcacgcccttcctgatacgccagcgcaataatgtcggtgatgtagtattcgccctgagcattattgttggtcagcttcgccagccagcgtttcatatctgcgccgttggcaatcagaatgccggtgttgatctcctgaatctgacgctgctcgtcggtggcatctttgtgctcaacaatgccggtaactttgccgttttcacgggtgatacgtccataaccggtcggatcatccagtttcaccgtcagcagaccaatgccaccctgcggtttagcatcacgcagacgctggagtgtttcgacagagatcagcggcacgtcgccgtagagcattaaaatgtcttcatcatcggcaaagaaaggtgcggcctgctgcattgcatgacccgtacccagctgctctgcctgaagcacccagttaaggttgtcgtctttcagcgcctgttttagcagatcgccgccgtgaccgtacaccaggtgaacgtgcgctgcgcctaattcattcgcagcatcaatgacatgctgaaccatcgctttcccggcaagggtatgcagcactttcggaagatcggaatacatgcgcgtgcctttgcctgcggcaaggatcactacgctcatagcattattcaacatacgcgtcctgactgtaatttgagaacgaatttaaaccgcttcaccttgaaaaaactacatttttttcatcgtgaaatggacagaggataaattgttcaataacggattatccccgctgacgaaagcgccattttcgaccatcgtcacgccttttgtctgcagaaaattaaggcagtaccttaatttaagcgtcaggtggatgtttttgctcttatttcgatcaatgaataaacaggaaaacaggggggttttatatcagcaggatctatgtgaacgctattcaggacgggtcacacgcgcaaaaaaaagccagcctgtttccagactggcttttgtgcttttcaagccggtgttacatcgcttttttggtcaactcgataacgcgcagctgcgcgatcgctttggccagttccgcagacgcctgagcgtaatctacgtcgccgtgagagctgctaatgtgctcttcagccttacgtttcgcttccatggctcgcgcttcgtcgagatcctggccgcgaattgcggtgtcggccagaacggtcacgttgccaggctgcacttcaagaatgccgccagacagatagataaactcttcgtgaccgtgctgtttcacgatgcgaatcataccaggcttaatggcggtgagcagcggtgcgtggccagggtagatccccagttcaccttcgctacccgttacctggattttctcgaccagaccagagaacatttgttgctctgcgctgacgacgtccaggtggtaagtcattgccatatcaccctccgattaaggcgttaaagttttttggctttttccacagcttcttcgatggaaccgaccatgtagaacgcctgctccggcaggtgatcgtattcgccttccatgatgcctttaaagccacggatggtgtctttcagggagacgtatttacccggagaaccggtgaatacttctgccacgaagaacggctgggacaggaagcgctggatcttacgagcacgcgctaccaccagtttgtcttcttcagacagttcatccatacccaggatggcgatgatgtctttcagttcctgataacgttgcaggatggactgaacgccacgcgcggtgtcgtagtgttcctgaccaaccaccagcgggtccagctgacggctggtggagtccagcgggtcaacggccgggtagatacccagagacgcgatctgacggctcagtaccacggttgcgtcaaggtgcgcaaaggtggttgccggagacgggtcagtcaagtcatccgcaggtacgtatactgcctgtacggaggtgatagaaccagttttggtggaggtgatacgttcctgcagaacgcccatctcttccgccagggtcggctgataacctaccgctgaaggcatacggcccagcagtgcggatacttccgtaccggccagggtgtaacgatagatgttgtcaacgaacagcagaacgtcacgaccttcgtcacggaatttctcagccatggtcagaccggtcagagcaacgcgcagacggtttcccggcggctcgttcatctggccatacaccagggatactttgtcgataacgttggagtcggtcatttcgtggtagaagtcgttaccctcacgagtacgttcacctacgcccgcaaacacagagtaaccggagtgctcgatcgcgatgttacgaatgagctccatcatgtttacggttttacctacacccgcaccaccgaacagaccaactttaccgcccttagcgaacggacacatcaggtcgataactttgataccggtttccagcagttcctgagagtttgacagctcttcgtaggaaggtgctgcgcggtgaatcgcccaacgctcttcttcaccgatctcgcctttcatgtcgaccggttcacccagtacgttcatgatacggcccagagtcgctttacctaccgggacttcaatcgggtgttcgaggtcttttacatccagaccgcgacgcagaccgtcggaggaacccattgcgatggtacgtacgataccgccgccgagctgctgctgaacttccagcaccagacgctcattaccattttgcacctcaagagcatcgtacacgcgcggtacggcatcctgagggaattcgacgtcaactacggcgccgattacctggacaatctttccagtagccatcttaaatcctctacgaaataacctgtttaaaccgcggcggcccccgagacgatctcggtgagttcctgagtaatgctggcctgacgagctttgttgtataccaactgcagctctttaatcaggctgccgccattgtcggtcgcggctttcatcgccaccatacgggcggcctgctcgctggccaggttttcaaccacgccctgataaacctgagattcgacataacgacgcagcagggtatccagcaacgccttcggatcgggttcgtacaggtaatcccaggatttatgtttcagatcatcatcatctgatgccggtaacggcagcagctggctgatggtcggaacctgagacatggtgttaataaatttgttgctgacaatgtaaagcttgtccagacggccttcgtcgtaggcctgcaacatcacttttaccggaccgatcagttcggacagggaagggttatcccccatgccggtgacctgggcaacaacattgccgcccacggagttgaagaacgacacgcctttcgagccgatcattgcgaggtcgcattgaacgcctttgtcggtccaggtcttcatttccgccagcagttttttgaacaggttaatgttcaaaccaccgcacaaaccacggtcggtcgacaccaccaggtagcccacgcgtttaacgtcgcggtcttccaggtaagggtgcttatattccagattaccgtgtgcaaggtgaccaatcactttgcgcatggtttctgcataaggacggctggccgccatgcgatcctgcgatttacgcattttggaagcggcgaccatctccatcgctttagtgatcttttgcgtgttctggacgcttgcgatcttactacgtatctcttttgcgccggccatgagcttctcctcaatgccttgcggcctgccctaaggcaagccgccagacgttaccaggattgggttgctttgaaggaatcgaggatgcctttcagcttgccttcgatttcgtcgttgtagccaccggtctggttgatctcttgcatcaacggagcgtgatcacggtcgacgtaagccagcagagcggcttcgaagctgccaattttcgacagttcaacatccgccaggtaaccacgttctgctgcgaacagaaccagagactgctgcgcaacggacatcggcgcatactgtttctgtttcagcagttcggtcactttctgaccgtggtcaagctgcttacgtgttgcatcgtcaaggtcggatgcaaactgagagaacgctgccagttcacgatactgtgccagagcggtacggataccaccggacagttttttcatgatcttggtctgtgctgcaccaccaacacgggatacggaaatacccgggttaaccgcaggacgaataccggcgttgaacaggttggtttccaggaagatctgaccatcggtaatggagattacgttggtcggaacgaacgcagaaacgtcacccgcctgagtttcgataatcggcagtgcggtcagagaaccggttttccctttcacttcacctttggtgaaggcttcaacgtattcggcgttaacacgtgcagcacgctccagcagacgagagtggaggtagaaaacgtcgcccgggaatgcttcacgtcctggcggacgacggagcagcagggagatctgacggtaagcaacagcctgtttagacaggtcatcgtaaatgatcagcgcatcttcaccgcggtcacggaagtattcgcccattgcgcaaccggcatacggtgccaggtattgcagtgcagcggattcagacgcggttgctaccacaacgatggtgttagccagtgcgccgtgctcttccagtttacgtaccacgttagaaatggtggacgctttctggccgatagcgacatagatacatttgataccggaatcgcgctggttgatgatggcatcgatagccagtgcggttttacctgtctgacggtcaccgatgatcaattcacgctgaccacgaccgattgggatcatggagtcaacggctttataaccggtctgtaccggctgatctacggactgacgttcgataacgcccggagcgattgcttctacagcagagaagccgtcgtgatccagcggacctttaccgtcgattggtgcacccagagtgttaaccacacggcccagcaggccacggccaaccggaacttccaggatacggccagtacacttaactttcatgccttcggcaaggtcagcgtacggacccataacaaccgcacctacagagtcgcgctcgaggttcagtgcgatagcgtaacggttacccggcagggagatcatttcaccctgcatacaatcggccaggccgtgaatgcggataacaccgtcacttacagaaacaatagtaccttcgttgtgagcttcactcacaacattgaactgagcaatgcgctgcttgatcagttcgctgatttcggtggaattcagttgcatgctccagtccccttaagactgcaagacgtctgcaaggcgctcaagacgaccgcgtacgctgccatcaatgaccatatcacccgctcggatgataacgcctgccattacagacttatcgattttgcaattcagcttaactttgcgtgacagacgtttttccatcgcagcagaaattttcgcgagctgttgttcactcagtgcggcagcggaaatgacgtctacctcagcggtagcctcactcacggcacgcaggtgaataaactgctccagaacatccgggagcgcgttaagacgaccattttcagccataacccgaatcaggttctgaccgttttcgtccagttgctcaccacaaactgcgataaacgactcggcgagcgtttctggcgcaagcgcgccagagagaagctctgccatttgttcgtttttggttacctcggcggcaaacgccagcatgtcctgccagcgttctacactttggtgttcgacggcaaagtcaaaagctgctttggcgtaggggcgagctaccgtaataaattcagacatcagcccctccctccttacagttcagcgacaagtttatccacgatgtcgctgttagcagcttcatccacggaacgttcgatgatcttctcggcgccagcaacagccaggatagcaacttgcttacgcagctcttcacgggcacgtttacgctcggcttcaatttccgcctgcgcctgggccacgattttagtacgttcctgttctgcctcagctttcgcttcgtccagaatctgcgagcggcgtttgttcgcctgctcgatgattacctgggcttccgctttcgcttttttcagctggtcggtcgcgctggcctttgcaaggtcaaggtccttatgtgctcgttctgcggaagcaaggccgtcagcaatttctttttgacgtttttcgatggctgccattaatggcggccatacgtacttcatgcagaacagaacgaacaggacaaacgcgatggcctggccgaggattgttgcgttaagattcacagcacaatgcctctatttagttaacgttctgatattgctctttaaataaaagcaacgcttactacgcgacagcgaacatcacgtacagacccagacctacagcgatcatcgggatagcatccaccagacccataacgataaagaactgagtacgcagcagaggaatcagatcaggttgacgcgctgcgccttccaggaatttacccccgaggatgccgataccgatcgcagcaccgattgccgccagacccatcatcacagcggcagccatgtacagcagatccatattcaggttttccatgacagtctccagtttgtttcagttaaaacgtagtagtgttggtaaattaatgttcttcagacgccatcgacagatagacgatcgtcagaaccatgaagatgaaggcttgcagcgtaatgatcaggatgtggaaaatggcccacggcacattcaggatccactgtgaccaccacggcaacagaccagcaatcagaatgaaaatcagctcaccggcatacatgttaccgaacagtcgcaaaccgagtgaaactggtttggacagcaggcttaccccttcaaggattaagttgacaggaatgaacgcccagtgattgaacggctgcagcgtcaactctttcgtgaagccgccgatgcctttcattttgatgctgtagaacagaatcaggataaatacgcccagtgccatagacagcgttacgttcacgtccgcagacggaaccacacgcagtgcaggcagacccagtacatgttcagcaatgtacggcagcaggtcgataggcagtaaatccatcaggttcatcaggaatacccagacgaagatcgtcagggccagcggagcaatcagcttgcttttgccatggtacatgtctttcacgctaccattaacaaagccgatcaccagctcaatcgcggtctgaaacttacctggcacaccgctggtcgcctttttggctacgctacggaataaaaccaggaacaacagacccagcaccaccgagaagaacatggagtcaatattgattgtccagaaggtggctggggggttttgtggatccaccagcgagaatgtacgcaggtccagctgaaggttattcaggtggtgtcctatgtaatcctgcggcgtcatattttctgaagccatgatgccttttaccctttgttgttaattacagccggtgccagtatctgaaccaccagcaccaaaacccacgtaacgatcagcggcaagaataccgcctttaaaaccgccaacgccaccaccagtaacaccaacatcgccagaactttgaaagcttcgccaaatgcgaatgtccaggccacccggcctttcgctggtgtatgcgcctggtgacgccaggcaaatatcataaacaaaacgttaggcagaaagactgccaggcccccgcttattgcagagacgccccagaaggggtctttgaggctgaacagcaatccacttgctatcaccaccagtaactgaacgagcagaagcttccgagcaacgtttcgactcacgagcgacacagacatcacgtttttcactcctgctcccttcgaggtatgccgcgtgtcgtataaaactttctttaaggcttagagtcaagcatcaaaaagcggtcaaattatacggtgcgcccccgtgatttcaaacaataagtagccaaaaggtgaataaatgtttaaatatttttccagtgcatacaattgcgacttttctgctaaccctgttcgatcatgaaaaactgtaaataacgcgtaaacactggtgataaagcgtgcttcagatcacatattgcgcatgttcgcgcacagcatatttatttacttggcaaatgatgcctttgcaagtttatgatatttcagtctaaaaacagatactgttttaataaatgacatttacacaacaaaaaccacccattgacatttttaataatgttttaacagccaatgatggttcttagcgccgatttttagcagactgatattttcactaatgacttattttctgcttaccaaaaaaagccacgttatcttgttgatgcaaaagagtgaacgtggcgttaaatgtaaccagttatatcagtagaaaacctggttgttgttaacagtctaaccggtcaattttttatgatttttttgataaaaattaaattttatttgctttaatcaccaccagatgacgttcgccatccagggctggaacctgaagtttaaccactgattcgacctgatattcttcgggcaacaaagcgatttcatcttccggcatttgccctttcagcgcgtagaaacggccttgctcaccaggaagatggtggcaccagctcaccatatcgttcagagaggcaaaagcgcggctaattacgccatcaaatggcggctctgaaggaaactcttctaccctgctctgtactggttcaatattctccagtttaagctcatgttgcacctgacgaaggaaacgcacgcgtttaccaaggctatccaacagagtgaaatgggcttcaggacgcacgatagagagtggaatgcctggcagtcctggtccggtgccgacatcgataaaccgttcaccttgcagatacggtgccaccacaatgctatcgagaatatggcgtaccagcatctcattaggatcgcggaccgaagtcaggttgtacgctttgttccatttatgcagcatattcacgtaggcaataagctggtttttctggtgatcggtaagcgaaatacctgcgtctttcagcagtaaggagagtttgttgagcacggtgattacctgttcttgatgcgttgcctggtaagcgggtgcttaccaggcatttttaatgcgttatgcgctacgacgcagcataccctgttttttcagccacaccagcagaatggagatggccgcaggcgtgacgccagaaatacgcgaagcttggccgatagaggctggtttgtgatcgttaagtttggcgatcacttcgttagaaagaccggatacctggcggtaatccagtgtcgcgggtagcagggtgttctcgttacgcagctgcttttcgatctcatcttgctggcgcgcgatataaccttcgtatttaacctgaatctcaacctgttccgccgcctgttcgtctgtcaacgcaggggcaaacggcgtcagcgtggttaatttttcataagtcatttccggacgacgcagcagatcttcaccactggcttcacgggaaagcggcgcagtcaggtgagcattcacttcggctgcagcttccgccgacggggttacccaggtcgatttcagacgctgacgctcacgctcgatattctcaagtttctcgttaaagcgcgcccaacgttcgtcatccaccaggcccagttcacgaccgatttcagtcaaacgcagatccgcattatcttcgcgtagcatcagacgatattctgcgcgcgaagtaaacatacgatacggttctttggttcctaaagtgcacaggtcatcaactagtacgccgagatacgcctgagaacgtgccggagcccaaccttctttgtcagcagacagacgggcagcgttaagaccggccagcaaaccttgcgcagcggcttcttcgtaaccggtagtgccgttaatctgaccagcaaagaacagcccctggataaacttgctctccagcgtcggtttcaggtcgcgaggatcgaagaagtcatactcaatggcataacccggacgcacgatcttcgcgttttccatcccctgcatagagcggacgatttgcatctgcacatcgaacggcaggctggtggagataccgttcggataaatttcattagaggtcagtccttccggttcaaggaagatctgatgctgatttctgtcggcgaagcgcatgactttgtcttcgatcgacgggcagtagcgtgggccgacaccttcgatcacccctgcgtacattgggctacgatcgaggttactgcggatcacatcatgggttttctcgttggtatgagtgatataacacggcacctgctggggatgctgggacgcattgcccataaacgagaataccggcattgggttatcgccatgctgttgcgccagtacgctaaagtcgatggttcgagcatcaatacgcggtggtgtcccggttttcagacgaccaacgcgcagcggcagttcacgcaaacggcgagaaagcggaatggacggcggatcaccagcacggccaccgctgtaattatccagaccgatatgaattttaccgtcgaggaacgtcccaacggtgagcacgacggctttggcacggaacttcagtcccatttgggtaacagcaccgaccacgcgatcgttttcgacaataagatcttcaaccgcctgctggaagatcatcaggttcggttggttctccagcgccgtacgtaccgcctgacggtagagcacacgatccgcctgagctcgggtagcgcgaaccgccggtcctttgcttgcgtttagtatcctaaactggatacccgcctgatcgatcgctttcgccatcagaccgccgagtgcatccacttcttttaccagatgtcccttcccaataccgccgatcgccgggttgcagctcatctgccccagagtgtcgatattgtgtgtcaaaagcagagtctgttgacccatacgcgccgcggccatcgcggcctcggtgcctgcatgacccccgccaatgatgatgacgtcaaaaggatccggataaaacatggtgattgcctcgcataacgcggtatgaaaatggattgaagcccgggccgtggattctactcaactttgtcggcttgagaaagacctgggatcctgggtattaaaaagaagatctatttatttagagatctgttctattgtgatctcttattaggatcgcactgccctgtggataacaaggatccggcttttaagatcaacaacctggaaaggatcattaactgtgaatgatcggtgatcctggaccgtataagctgggatcagaatgaggggttatacacaactcaaaaactgaacaacagttgttctttggataactaccggttgatccaagcttcctgacagagttatccacagtagatcgcacgatctgtatacttatttgagtaaattaacccacgatcccagccattcttctgccggatcttccggaatgtcgtgatcaagaatgttgatcttcagtgtttcgcctgtctgttttgcaccggaatttttgagttctgcctcgagtttatcgatagccccacaaaaggtgtcatattcacgactgccaataccgattgcgccaaagcggactgcagaaagatcgggcttctgttcctgcaatgcttcatagaaaggagaaaggttgtccggaatatctccggcaccgtgggtggagctgataaccagccagatccctgaggcaggtaaatcttctaacagcggaccgtgcagcgtttcggtggtaaaacccgcctcttccagcttttcagccaggtgttctgctacatattcggcaccgccgagggtgctgccgctgataagagtgatatctgccataaaccgccacctttattaagagtggcgtattgtacgctgtgaacgcgttgggatctacctgtggaaaagtatgggattaaaaaagccgatcagggcttgatggtacgcatgatcgggttttgcaggacgatcaatgtctcggtggactgaatttcatcaattgtttggatcttgttgataagtacatgctggagagcgtcgatcgaacggcacatcacttttataaagatgctgtagtggccggttgtgtaataggcttcagtgacttcatcaaggctttccagctttgccagcgcggaagggtagtctttggcgctctttaatataatgccgataaagcagcctacgtcataaccgagctgcttcgggctgacatcaatacgcgccccggtaatgatccccgcctgcttcattttctctactcgaacgtgaatcgtccccggactgacgccaaattgtttcgccagttcggcgtaagcggtgcgcgcattgcccattaatgcttccaggatgccacggtccagattgtcgatcagataattttccataggattttcttatgcggattgatgattcattctattttagccttcttttttaatgaatcaaaagtgagttaggctttttattgaatgattattgcatgtgtgtcggtttttgttgcttaatcataagcaacaggacgcaggagtataaaaaatgaaaaccgcttacattgccaaacaacgtcaaattagcttcgtgaaatctcacttttctcgtcaactggaagaacgtctggggctgatcgaagtccaggcgccgattcttagccgtgtgggggatggcacgcaggataacttgtcgggctgtgaaaaagcggtgcaggtaaaagtgaaagctctgcctgatgcccagttcgaagtggttcattcactggcgaagtggaaacgtcagaccttagggcaacacgacttcagcgcgggcgaagggctgtacacgcacatgaaagcccttcgccccgatgaagaccgtctttctccgttgcactcggtctatgttgaccagtgggactgggaacgcgtaatgggcgacggtgagcgtcaattctcgactctgaaaagcacggtagaggcgatctgggcgggaattaaagcaaccgaagctgcggttagcgaagagtttggcctggcaccgttcctgccggatcagatccacttcgtacacagccaggagttactgtctcgttatccggatcttgatgccaaagggcgtgagcgggcgatagcgaaagatcttggcgcggtattccttgtcgggattggcggcaagctgagcgatggtcatcgccacgacgtgcgcgcaccggattatgatgactggagcaccccgtcagagctgggccatgcgggtctgaacggcgatattctggtgtggaacccggtactggaagatgcgtttgagctttcctccatggggatccgtgtagatgccgacacgctgaagcatcaactggcgctgaccggtgacgaagatcgcctggagctggagtggcatcaggcgctgctgcgcggtgaaatgccgcagaccatcggcggcggtatcggccagtctcgtttgactatgctgctgctgcaactgccgcatatcggccaggttcagtgtggagtatggccagctgctgttcgcgagagcgtcccttctctgctgtaataatttatcgccgccagcgtctgagcaggcggcttcgcatcccggtatcaaagcgccagatatgatcgaaaatgcgcatgatgccgggtttgccgtgtgccgacatcgccacggcatgaaagcgatgctgatgtacccgctgcagctctttcactttactcgtcacgtcgtcaggcaaccgctgagcgataaaatcagaaatcaccaccgcatcggcatcaaaccattccctgctttgcaagcgttccataatggcgcgaaaacaactggcaagatcggtgccgccacgaaactgctggcttaaaaaacggattgcttgttcgatgccttgtgggcctgaaagctcataacggacgatctcggtggaaaatagcataatatagcagcgccggttttctgcgagagcaatgcgcatcaaggccaggcagaacgctttcgcacactgttcattaaagccgcccattgagccggaagtatccacacagacaataaacggcccgcgcggctgttcatcgtaatctttatgtaccaccggacgttcgatcactttttcacgccacgactcaccgtgcaggcgataggtgagcaactgtttttccaccagccgacggtaaaactcatactccagttccgttatccctagtgtcgccagttctggcggcaggagacgtaaaatatcatcgctttgttgcagaccatcaacctgctcaggaaccgtcgccggttcgcgcaccatggtgcggaaggtttccatctgcgcatcgttgcgcggtattgatttggcttcccgagaacgccccagctgctctgccaggcgtttcagttccggctgttcgttaagaaattcaccgtatttcacaatcaactgatagtcgccacgtttaagctgaccggcgctcatatcccacagacgaccagctgcagtattgttatctgcgagaatcggttcaagttgtccgctcagcgtcatgcgttcctgaacttcactcaacagttgttcgcgttcttcttctaatagctgttgatttaacgtcgttgcttgcacgatcagacttaaacgccaacgctggagaaaaagcgtgtgtaacgctgaagtgatcgtgctgttagcatcaaccaactgtcgggcttgttctgcccatggagaattcagacgatgcagtaagtccaggatctgtggtagctgcacaataaactgtggcgtggagaggagctggctttgctgatagcacatcacctcttcggtgagttccggcgggactcgggcatctttcagccgactgcgcagcgcttcacgccagcggggaacatcatcagtgattgccgccttcaggcgtgggaatttttcaaagaagaccgccagctgcggtgaggccagcagtgcgatgatcatctcttcgatcaatccctcttcgctgacggccagcatcacattaagcgtatccagcgttagcattgttgtgcctggcgaatctgtgcaccgacatcctgtaggctggcttcaatgcgacctaaccagtcgccagggataaacagacatttttgctgttcgctgaataaagcgtgttgcttgcgccagtcgctttcaagctcttccagttgttgttttatttcaccaggcagaccttcagccgatgaaccgggaagtgccagcgtactgccttgtaaacttacatcgcgaacgacaagatgttgggcgctatcaacttccagattcagtttctgggcaaagccgataccgttcagtttaccgcgaatttcaccacctttgctcagccactgttccagcgcgctacgctcaaaggagatatgaaccacttccatatcatgcagttttaacggtttttgcagcagtagagtcagagtggaagcagtaacgttaacaggaagttgatactgctgacgacggctgaaaatgccgcccagacgaattaccgttaaggctgttttatcgctttgttgctgctggagttgcaggtgacgttgcacaatcgcgccaaggcgagtcaacatcccttgctgttgccaggcgtgaccggtcatcaatacatcaatttgttgttgtatcaaattcaggctttgcgcgtcataccacaggcaatctttcagcaaaatgagatctaccggggcaacagcactgcgaccgctaaaaaaggcgctggcctgcaataatcggatcgcttttttccagcgacgatccgagacataaggcgcatccggtaatttatccagttgctggcgcagcataaaaatcagctcaaatacatgatcgggcagcgtaatttcaccaatctctttctgccagcgttcatattcttcatctgtgacctgcaaggcatcaggaaccggattgtcgttttcatcctgttgactggtcagcatggagcggaaattcgctttatcctgcactttatctaaccacagacgaatcagcatgcggtcatataacgcttccagactgctgtctgcttccggcagctcgttggaggccgccaccagcagacgcatcgggattttttctacgtgtgcaccgttgcggaactggcgctcgttaatggcggtgagcaaggtattaagaattgccgggcccgctttccagatctcatccagaaagacaatttctgcttccggcaggtaaccgctggttaaacgttcatagcgcccttcatcttttagcgcctgaatagaaaggggaccaaaaacttcttccggcgtggagaagcgggtcatcagatattcaaacgcgcgggcattctgaaaggcgaattttaagcgccgggcgatcaaacttttggcaatacctggcgggccaaggaggaacacactttcaccacttaatgccgctaataaacacaagcggatggcgtggctacgttcataaagccccttttccaacgaactgctcaggcgggaaattctttccgctaataaatgagggtgagccataatgaagtggcgtcctttcgtcaaaagttctgcgtaaattgcgagtatagacgtttcttgctggtggctaaaatagtctcaaagggggggtatttttctttgagccaggttaatgtggccgcatttaggagtacgattttgccgttaatcgtgcatactgtgcgcttttttgtgggccaagggactaagcacacatttcatatttcaacgaaagactagtctatgagcactgataataagcaatcattgcccgcgattaccctcgcggcgattggagttgtctacggcgatattggtaccagcccgttatatacacttcgtgaatgtttgtccggccagtttggttttggcgttgaacgcgatgccgtgtttggctttttatcgctgatcttctggctgctaatctttgtggtttccattaaatatctcaccttcgtgatgcgggcagataacgccggtgagggggggatcctgacgttgatgtcgcttgccgggcgtaatacgtcggcgcgaaccacatcaatgctggtgattatggggctaatcggcggcagctttttctatggtgaagtcgtcataacacccgctatttcggtgatgtcagccattgaaggtctggaaatcgtcgccccgcagctggatacctggatagttcccctctcaattatcgttctcactttattatttatgattcaaaaacatggcacggctatggtcggtaagctgtttgcgccgatcatgctgacctggtttttgattctggcaggactggggttacgtagcattattgctaacccggaagtgctgcatgcgctgaatccaatgtgggcggtgcatttcttccttgaatacaaaacggtttcttttattgcattaggggcagtggtgttgtcgattacgggggtcgaggcgctgtatgctgatatggggcactttggtaagttccctattcgcctggcgtggttcaccgtcgtattaccttccttgacccttaattacttcggtcagggagcgctgttgttaaagaacccggaagcgattaagaacccgttcttcctgttggcaccggactgggcgctgatcccgctgctgatcatcgccgcactggcgacggtaattgcctcgcaggcggttatctctggcgtcttctcattgacgcgtcaggcggtacgtctgggatatttgtcgccgatgcgcattattcacacctccgaaatggagtcagggcaaatctatattccgtttgtgaactggatgctctatgtcgcggtcgtgattgtgattgtcagctttgagcactccagcaacctggcggcggcgtacgggattgcggtgaccggaaccatggtgctgacgtctattctctcgactaccgtggcacgtcagaactggcactggaataagtattttgttgcgctgatcctgattgctttcctttgtgtcgatattccattgttcaccgctaacctcgataaactgctctccggcggctggttgccattgagcctcggtactgtgatgtttatcgtgatgaccacctggaagagcgagcgtttccgcttgctgcggcggatgcatgaacatggtaactctctggaagcgatgattgcttcgctggagaaatcaccgcctgttcgcgtgcccgggaccgcggtgtatatgtcgcgtgcaatcaacgtcattccctttgcgctgatgcataaccttaaacataacaaggtattgcatgagcgggtgattctgttaactctgcgcaccgaagacgctccatatgtccataacgtccgtcgggtacagattgaacaactgtcgcccactttctggcgcgtggtggcaagttatggttggcgagaaacgccaaacgtagaagaagttttccaccgctgcggtctggaaggattaagttgccggatgatggaaacctccttctttatgtcgcatgagtcgttgatcctcggcaaacgcccgtggtatttgcgtctgcgcggcaagctgtacttgctgctgcaacgtaatgcgctgcgtgcaccagatcaatttgaaatcccgccaaacagggttatcgaactgggtactcaggtcgaaatctaacgccagacgcctcctttcttcataagggggcgtttttgttttcatggttaatcaccatgtaaaacgtttcgaggttgatcacatttccgtaacgtcacgatggttttcccaactcagtcaggattaaactgtgggtcagcgaaacgtttcgctgatggagaaaaaaatgaaaaaaggcaccgttcttaattctgatatttcatcggtgatctcccgtctgggacataccgatacgctggtggtgtgtgatgctggtttacccatccccaaaagtacaacgcgtatcgatatggcattaacccagggtgtaccttcttttatgcaggtgctgggcgtcgtcacaaatgaaatgcaggtcgaggcggccattatcgcggaagagatcaaacaccataatccgcaactccacgaaacgttgctcactcaccttgagcagctgcaaaaacaccagggaaataccattgaaattcgttacaccacgcatgaacaattcaaacaacaaaccgcagaaagtcaggcggtaattcgcagcggagaatgttctccgtatgcgaatatcattctctgtgctggcgtgacgttctgaggccgtcatggaagcattacttcagcttaaaggcatcgataaagccttcccgggcgtaaaagccctctcgggcgcagcgttaaatgtctatccgggccgcgtgatggcgctggtgggcgaaaacggcgcgggtaaatccaccatgatgaaagtgcttactggcatctatactcgcgatgccggtacgcttttatggctggggaaagaaacgacatttaccgggccaaaatcttcccaggaagccgggattgggattatccatcaggaactgaacctgatcccgcagttgaccattgccgaaaacattttcctcggtcgtgagtttgttaatcgctttggcaaaattgactggaaaaccatgtatgccgaagcggataaattgctggctaaacttaacctgcgctttaaaagcgacaagctggtgggcgatctttccatcggtgaccagcaaatggttgaaatcgccaaagtgctgagctttgagtcgaaagtcatcattatggatgaaccgaccgatgcgctgaccgataccgaaaccgaatccctgttccgcgtcatccgcgagctgaaatcgcaaggccgcggtattgtctatatctcccaccgcatgaaagaaatcttcgagatttgcgatgacgttaccgtttttcgtgatgggcaatttattgctgagcgcgaagtggcatcactgaccgaagattcgctgattgagatgatggtgggtcgcaagctggaagatcaatatccgcacctggacaaagcgccgggagatatccgcctgaaagtcgataatctctgcggacctggcgttaacgatgtctcttttactttacgcaaaggcgaaattcttggcgtctctggtttgatgggcgcaggtcgtaccgaactgatgaaagtgctctacggcgcactaccgcgcaccagcggttacgtcaccctggatgggcatgaagtcgttacccgttcaccgcaggatggcctggcaaacggcattgtgtatatctccgaagaccgtaaacgtgacggtttagtgttgggcatgtcagtaaaagagaacatgtcgctgacagcgctgcgctacttcagccgcgctggcggcagtttgaagcatgccgatgaacagcaggctgtgagtgatttcattcgtctgtttaatgtgaaaactccgtcgatggaacaggcaattggtctgctttccggtggcaatcagcaaaaagtggcgattgcccgcggtctgatgacacgccccaaagtgttgatccttgatgaacctacccgtggcgtagatgtcggcgcgaaaaaagagatctatcaactgattaaccagttcaaagccgatggcttgagcatcattctggtgtcatcggagatgccagaagtattaggcatgagcgatcgcatcatcgtcatgcatgaagggcatctcagcggggaatttactcgtgagcaggccacccaggaagtgttaatggctgccgctgtgggcaagcttaatcgcgtgaatcaggagtaaaaaaatgacaacccagactgtctctggtcgccgttatttcacgaaagcgtggctgatggagcagaaatcgcttatcgctctgctggtgctgatcgcgattgtctcgacgttaagcccgaactttttcaccatcaataacttattcaatattctccagcaaacctcagtgaacgccattatggcggtcgggatgacgctggtgatcctgacgtcgggcatcgacttatcggtaggttctctgttggcgctgaccggcgcagttgctgcatctatcgtcggcattgaagtcaatgcgctggtggctgtcgctgctgctctcgcgttaggtgccgcaattggtgcggtaaccggggtgattgtagcgaaaggtcgcgtccaggcgtttatcgctacgctggttatgatgcttttactgcgcggcgtgaccatggtttataccaacggtagcccagtgaataccggctttactgagaacgccgatctgtttggctggtttggtattggtcgtccgctgggcgtaccgacgccagtctggatcatggggattgtcttcctcgcggcctggtacatgctgcatcacacgcgtctggggcgttacatctacgcgctgggcggcaacgaagcggcaacgcgtctttctggtatcaacgtcaataaaatcaaaatcatcgtctattctctttgtggtctgctggcatcgctggccgggatcattgaagtggcgcgtctctcctccgcacaacccacggcggggactggctatgagctggatgctattgctgcggtggttctgggcggtacgagtctggcgggcggaaaaggtcgcattgttgggacgttgatcggcgcattaattcttggcttccttaataatggattgaatttgttaggtgtttcctcctattaccagatgatcgtcaaagcggtggtgattttgctggcggtgctggtagacaacaaaaagcagtaataacgactacaggacatcttgaatatgaacatgaaaaaactggctaccctggtttccgctgttgcgctaagcgccaccgtcagtgcgaatgcgatggcaaaagacaccatcgcgctggtggtctccacgcttaacaacccgttctttgtatcgctgaaagatggcgcgcagaaagaggcggataaacttggctataacctggtggtgctggactcccagaacaacccggcgaaagagctggcgaacgtgcaggacttaaccgttcgcggcacaaaaattctgctgattaacccgaccgactccgacgcagtgggtaatgctgtgaagatggctaaccaggcgaacatcccggttatcactcttgaccgccaggcaacgaaaggtgaagtggtgagccacattgcttctgataacgtactgggcggcaaaatcgctggtgattacatcgcgaagaaagcgggtgaaggtgccaaagttatcgagctgcaaggcattgctggtacatccgcagcccgtgaacgtggcgaaggcttccagcaggccgttgctgctcacaagtttaatgttcttgccagccagccagcagattttgatcgcattaaaggtttgaacgtaatgcagaacctgttgaccgctcatccggatgttcaggctgtattcgcgcagaatgatgaaatggcgctgggcgcgctgcgcgcactgcaaactgccggtaaatcggatgtgatggtcgtcggatttgacggtacaccggatggcgaaaaagcggtgaatgatggcaaactagcagcgactatcgctcagctacccgatcagattggcgcgaaaggcgtcgaaaccgcagataaagtgctgaaaggcgagaaagttcaggctaagtatccggttgatctgaaactggttgttaagcagtagttttaatcaggttgtatgacctgatggtgacataaatacgtcatcgacagatgaacgtgtaatataaagaaaagcagggcacgcgccaccctaacacggtggcgcattttatggacatcccgaatatgcaaaacgcaggcagcctcgttgttcttggcagcattaatgctgaccacattcttaatcttcaatcttttcctactccaggcgaaaccgtaaccggtaaccactatcaggttgcatttggcggcaaaggcgcgaatcaggctgtggctgctgggcgtagcggtgcgaatatcgcgtttattgcctgtacgggtgatgacagcattggtgagagcgttcgccagcagctcgccactgataacattgatattactccggtcagcgtgatcaaaggcgaatcaacaggtgtggcgctgatttttgttaatggcgaaggtgagaatgtcatcggtattcatgccggcgctaatgctgccctttccccggcgctggtggaagcgcaacgtgagcgtattgccaacgcgtcagcattattaatgcagctggaatcaccactcgaaagtgtgatggcagcggcgaaaatcgcccatcaaaataagactatcgttgcgcttaacccggctccggctcgcgaacttcctgacgaactgctggcgctggtggacattattacgccaaacgaaacggaagcagaaaagctcaccggtattcgtgttgaaaatgatgaagatgcagcgaaggcggcgcaggtactgcatgaaaaaggtatccgtactgtactgattactttaggaagtcgtggtgtatgggctagcgtgaatggtgaaggtcagcgcgttcctggattccgggtgcaggctgtcgataccattgctgccggagatacctttaacggtgcgttaatcacggcattgctggaagaaaaaccattgccagaggcgattcgttttgcccatgctgccgctgcgattgccgtaacacgtaaaggcgcacaaccttccgtaccgtggcgtgaagagatcgacgcatttttagacaggcagaggtgacgcttggctacaatgaaagatgttgcccgcctggcgggcgtttctacctcaacagtttctcacgttatcaataaagatcgcttcgtcagtgaagcgattaccgccaaagttgaagcggcgattaaagaactcaattacgcgccatcagctctggcgcgtagcctcaaactcaatcaaacacataccattggcatgttgatcactgccagtaccaatcctttctattcagaactggtgcgtggcgttgaacgcagctgcttcgaacgcggttatagtctcgtcctttgcaataccgaaggcgatgaacagcggatgaatcgcaatctggaaacgctgatgcaaaaacgcgttgatggcttgctgttactgtgcaccgaaacgcatcaaccttcgcgtgaaatcatgcaacgttatccgacagtgcctactgtgatgatggactgggctccgttcgatggcgacagcgatcttattcaggataactcgttgctgggcggagacttagcaacgcaatatctgatcgataaaggtcatacccgtatcgcctgtattaccggcccgctggataaaactccggcgcgcctgcggttggaaggttatcgggcggcgatgaaacgtgcgggtctcaacattcctgatggctatgaagtcactggtgattttgaatttaacggcgggtttgacgctatgcgccaactgctatcacatccgctgcgtcctcaggccgtctttaccggaaatgacgctatggctgttggcgtttaccaggcgttatatcaggcagagttacaggttccgcaggatatcgcggtgattggctatgacgatatcgaactggcaagctttatgacgccaccattaaccactatccaccaaccgaaagatgaactgggggagctggcgattgatgtactcatccatcggataacccagccgacccttcagcaacaacgattacaacttactccgattctgatggaacgcggttcggcttagatttacgctgtcttttgatcaaattattaccatcggttgttttcagaagcatgaacattgctgctgaagcaacagtaataatgcccattgtgataaacgtatagtggaattgttcgacagtcgttgtgccttccattccttcataaacgcgaaggacggccgcacttacagcaacgcctaaactaatcgacagttgctgcgtgaccgccagaacactgttaccgctgctggcattgtcatcggtcagatcggcaagtgtgatggtattcatcgcggtaaactgcgtcgacatagccatccctaatataaacaacggcaagatcagcatccatatagccattgctggtgattgcaaagagaactgagcgatcattagcccaataatcaccgtgatccccactaacgtatggcgatagcccagacgacgtaagacttgggtaaccatcgattttgcaataatggaacctaacgctgtcggtgccatcatacagccagcaataaacgcctgataaccaaatcctacctgtaacatcaatggcataaggaacggtacacagccggtccccagacgggttgcaatattgcctacgataccgatcgagaaagtgcgggttttaaataaatctaatgaaattaatgggtttggcgtgcgtcgtgcatggagaatatagagaagcagtaacccgatgctggtgacaattaccgtcaaggcaatccagctggcgacaatcttttccccgaatagctctattccgcttgagaagagaacaaggctgaggccaaacagcaaaaagccagtgatatcgaatctgcgtcgtgcggtggtgaaattgggcatatgtttgcgcgcgtaaagaaggcccgcaatacctatggggatattgattaaaaatatccagtgccaggttgcccaggtgaccagcacgccgccaagaacggggcctaaaattggccccaccagacccggcatggcgacaaaattcaatactggaagaagttcattacgaggataagcgcgcagtaaggccagccgagcaacaggcatcatcattgcgccgcctatcccctgaataacccggaagacaaccagctgtggtagcgaattagaaagtgcgcaggccagagaacccaatgtgaacagactcacggcaagggtaaaaatgcgacgcgtaccgaagcgatcggctagccatccgcttaccggaataagcatcgccaccgtcagcgtataactgatgatggctgattgcatcgcgagaggagaacgattaaggctatgagcgattgcgggtaaggcggtattaagaatagtggcatcaagtgcctgcatgaagaaggccatcgccgcgatccacggcaaacccgccatactgcgcttctttttatcgctcattcaatgtcctgttatcgggttatcacttatcaggtgagcgtagcagcgcctgacaagctttaaatgccgcgtcgccatcgctttggataatcgcatcgacaatcgcctgatgcagatccagctttatcactgtgtcgctggtaattgacgtgaagtaagtgtgataaaccgaatggaatagcgaggcgaatgaggtcaaaaacggattggcgctcatttcatagatatgctcatgccaggccatatcgacttcgatccagcgttcacggcgaaagttctcttttaatgccgccatttcggccattaacgtattgagatgcgctttctgttccgcggtgccaaccgttgctgccagtaggcaggcttgcggctccagacagatacgcataaccagaaagtgatcgatgacctgatgaaagttctcttctgtcatccaccaggtaagcaattcctgatcaagaaaattccagttcgattgtggcatgacccgagtaccaattcgcggtcgcggtaaaaccatcccttttgccgttaacgttttgaccgcttcgcgtaccgctgtacgactcactccaaattgctcgcccagctcaatctcaccgggcaaaatggtgccgggttcatattcaccttttaagatccgttgcgccagcttctcagccagaacatacgaaaggtttttctgtgcagctaactgttgtgcgcttaaaggcattacttatcttcctttttctttttattcctccttagtatgccaccaggaagtgtgattacggttgcaaaaacggcaaattgcttgttttatggcacattaacggggcttttgctgaaaaaatgcgcggtcagaaaattattttaaatttcctcttgtcaggccggaataactccctataatgcgccaccactgacacggaacaacggcaaacacgccgccgggtcagcggggttctcctgagaactccggcagagaaagcaaaaataaatgcttgactctgtagcgggaaagcgtattatgcacaccccgcgccgctgagaaaaagcaaagcggcactgctctttaacaatttatcagacaatctgtgtgggcactcgaagatacggattcttaacgtcgcaagacgaaaaatgaataccaagtctcaagagtgaacacgtaattcattacgaagtttaattctttgagcatcaaacttttaaattgaagagtttgatcatggctcagattgaacgctggcggcaggcctaacacatgcaagtcgaacggtaacaggaaacagcttgctgtttcgctgacgagtggcggacgggtgagtaatgtctgggaaactgcctgatggagggggataactactggaaacggtagctaataccgcataacgtcgcaagaccaaagagggggaccttcgggcctcttgccatcagatgtgcccagatgggattagctagtaggtggggtaacggctcacctaggcgacgatccctagctggtctgagaggatgaccagccacactggaactgagacacggtccagactcctacgggaggcagcagtggggaatattgcacaatgggcgcaagcctgatgcagccatgccgcgtgtatgaagaaggccttcgggttgtaaagtactttcagcggggaggaagggagtaaagttaatacctttgctcattgacgttacccgcagaagaagcaccggctaactccgtgccagcagccgcggtaatacggagggtgcaagcgttaatcggaattactgggcgtaaagcgcacgcaggcggtttgttaagtcagatgtgaaatccccgggctcaacctgggaactgcatctgatactggcaagcttgagtctcgtagaggggggtagaattccaggtgtagcggtgaaatgcgtagagatctggaggaataccggtggcgaaggcggccccctggacgaagactgacgctcaggtgcgaaagcgtggggagcaaacaggattagataccctggtagtccacgccgtaaacgatgtcgacttggaggttgtgcccttgaggcgtggcttccggagctaacgcgttaagtcgaccgcctggggagtacggccgcaaggttaaaactcaaatgaattgacgggggcccgcacaagcggtggagcatgtggtttaattcgatgcaacgcgaagaaccttacctggtcttgacatccacggaagttttcagagatgagaatgtgccttcgggaaccgtgagacaggtgctgcatggctgtcgtcagctcgtgttgtgaaatgttgggttaagtcccgcaacgagcgcaacccttatcctttgttgccagcggtccggccgggaactcaaaggagactgccagtgataaactggaggaaggtggggatgacgtcaagtcatcatggcccttacgaccagggctacacacgtgctacaatggcgcatacaaagagaagcgacctcgcgagagcaagcggacctcataaagtgcgtcgtagtccggattggagtctgcaactcgactccatgaagtcggaatcgctagtaatcgtggatcagaatgccacggtgaatacgttcccgggccttgtacacaccgcccgtcacaccatgggagtgggttgcaaaagaagtaggtagcttaaccttcgggagggcgcttaccactttgtgattcatgactggggtgaagtcgtaacaaggtaaccgtaggggaacctgcggttggatcacctccttaccttaaagaagcgttctttgcagtgctcacacagattgtctgataggaagtgaaaagcaaggcgtcttgcgaagcagactgatacgtccccttcgtctagaggcccaggacaccgccctttcacggcggtaacaggggttcgaatcccctaggggacgccacttgctggtttgtgagtgaaagtcacctgccttaatatctcaaaactcatcttcgggtgatgtttgagatatttgctctttaaaaatctggatcaagctgaaaattgaaacactgaacaacgaaagttgttcgtgagtctctcaaattttcgcaacacgatgatgaatcgaaagaaacatcttcgggttgtgaggttaagcgactaagcgtacacggtggatgccctggcagtcagaggcgatgaaggacgtgctaatctgcgataagcgtcggtaaggtgatatgaaccgttataaccggcgatttccgaatggggaaacccagtgtgtttcgacacactatcattaactgaatccataggttaatgaggcgaaccgggggaactgaaacatctaagtaccccgaggaaaagaaatcaaccgagattcccccagtagcggcgagcgaacggggagcagcccagagcctgaatcagtatgtgtgttagtggaagcgtctggaaaggcgcgcgatacagggtgacagccccgtacacaaaaatgcacatattgtgagctcgatgagtagggcgggacacgtggtatcctgtctgaatatggggggaccatcctccaaggctaaatactcctgactgaccgatagtgaaccagtaccgtgagggaaaggcgaaaagaaccccggcgaggggagtgaaaaagaacctgaaaccgtgtacgtacaagcagtgggagcacgcttaggcgtgtgactgcgtaccttttgtataatgggtcagcgacttatattctgtagcaaggttaaccgaataggggagccgaagggaaaccgagtcttaactgggcgttaagttgcagggtatagacccgaaacccggtgatctagccatgggcaggttgaaggttgggtaacactaactggaggaccgaaccgactaatgttgaaaaattagcggatgacttgtggctgggggtgaaaggccaatcaaaccgggagatagctggttctccccgaaagctatttaggtagcgcctcgtgaattcatctccgggggtagagcactgtttcggcaagggggtcatcccgacttaccaacccgatgcaaactgcgaataccggagaatgttatcacgggagacacacggcgggtgctaacgtccgtcgtgaagagggaaacaacccagaccgccagctaaggtcccaaagtcatggttaagtgggaaacgatgtgggaaggcccagacagccaggatgttggcttagaagcagccatcatttaaagaaagcgtaatagctcactggtcgagtcggcctgcgcggaagatgtaacggggctaaaccatgcaccgaagctgcggcagcgacgcttatgcgttgttgggtaggggagcgttctgtaagcctgcgaaggtgtgctgtgaggcatgctggaggtatcagaagtgcgaatgctgacataagtaacgataaagcgggtgaaaagcccgctcgccggaagaccaagggttcctgtccaacgttaatcggggcagggtgagtcgacccctaaggcgaggccgaaaggcgtagtcgatgggaaacaggttaatattcctgtacttggtgttactgcgaaggggggacggagaaggctatgttggccgggcgacggttgtcccggtttaagcgtgtaggctggttttccaggcaaatccggaaaatcaaggctgaggcgtgatgacgaggcactacggtgctgaagcaacaaatgccctgcttccaggaaaagcctctaagcatcaggtaacatcaaatcgtaccccaaaccgacacaggtggtcaggtagagaataccaaggcgcttgagagaactcgggtgaaggaactaggcaaaatggtgccgtaacttcgggagaaggcacgctgatatgtaggtgaagcgacttgctcgtggagctgaaatcagtcgaagataccagctggctgcaactgtttattaaaaacacagcactgtgcaaacacgaaagtggacgtatacggtgtgacgcctgcccggtgccggaaggttaattgatggggtcagcgcaagcgaagctcttgatcgaagccccggtaaacggcggccgtaactataacggtcctaaggtagcgaaattccttgtcgggtaagttccgacctgcacgaatggcgtaatgatggccaggctgtctccacccgagactcagtgaaattgaactcgctgtgaagatgcagtgtacccgcggcaagacggaaagaccccgtgaacctttactatagcttgacactgaacattgagccttgatgtgtaggataggtgggaggctttgaagtgtggacgccagtctgcatggagccgaccttgaaataccaccctttaatgtttgatgttctaacgtggacccgtgatccgggttgcggacagtgtctggtgggtagtttgactggggcggtctcctcctaaagagtaacggaggagcacgaaggttggctaatcctggtcggacatcaggaggttagtgcaatggcataagccagcttgactgcgagcgtgacggcgcgagcaggtgcgaaagcaggtcatagtgatccggtggttctgaatggaagggccatcgctcaacggataaaaggtactccggggataacaggctgataccgcccaagagttcatatcgacggcggtgtttggcacctcgatgtcggctcatcacatcctggagctgaagtaggtcccaagggtatggctgttcgccatttaaagtggtacgcgagctgggtttagaacgtcgtgagacagttcggtccctatctgccgtgggcgctggagaactgaggggggctgctcctagtacgagaggaccggagtggacgcatcactggtgttcgggttgtcatgccaatggcactgcccggtagctaaatgcggaagagataagtgctgaaagcatctaagcacgaaacttgccccgagatgagttctccctgactccttgagagtcctgaaggaacgttgaagacgacgacgttgataggccgggtgtgtaagcgcagcgatgcgttgagctaaccggtactaatgaaccgtgaggcttaaccttacaacgccgaagatgttttggcggatgagagaagattttcagcctgatacagattaaatcagaacgcagaagcggtctgatgaaacagaatttgcctggcggccgtagcgcggtggtcccacctgaccccatgccgaactcagaagtgaaacgccgtagcgccgatggtagtgtggggtctccccatgcgagagtagggaactgccaggcatcaaattaagcagtaagccggtcataaaaccggtggttgtaaaagaattcggtggagcggtagttcagtcggttagaatacctgcctgtcacgcagggggtcgcgggttcgagtcccgtccgttccgccaccctaattaggggcgtagttcaattggtagagcaccggtctccaaaaccgggtgttgggagttcgagtctctccgcccctgccagaaatcatccttagcgaaagctaaggattttttttatctgaaataaccctctccgaagtaaatccttctaccggcatccttgccagccattcatattaatacacttcatccagcacgttaattttcaaaagatcgcgaatcaacgcatttttatcgctattttgcagccatatggcataaagcggccgtgaaagtgttgtgctatcgacaacggtatgcaggccgccttttttacgcgcccagctgacgggtagccaggtgcaaccattaagcatcgcaatctgttgctgtgccagttcagcagaactggttgtcagaatgggcacttcgtcagcaccgatcaaacctgcctcatgctgttgaaaatctggcccccactcaagtcgcagataattaagatctccctttagttttgaaggggcactggtataaagcgctaaagtgaaatatcccagcaactgactactaaattcgtccattttgggcgcttcagtggtaataagaagatcaagctggcgttcatgcagctgttttaccagagactgccgttgggcaattcgcgcttcgaactgtaagcctgtatgggcatcctgattttgatacaagcgtcccagccactgattaagcatacattcccacaacgaggcgctggcaccgatagaaaactcgttatgtcgtgaggtatgcgccacctccttacgggcggcctgccaggtgctcatgagcgtttctgcataaggcagtagtttttcaccggcagcggttaaacggatattgtttctgtggcgggtgaaaaggttcacacccagttgattttccagttgtctgattcgaaagctcactgctgactgggtcagatagagcgattcagccgctcgaccaaagtgacgcgttcggctaacttccaggaaagtttttaacaattccgtatccacagtgctctccgcaaaattatttgtcgttatgatttaaatgttttgttttacactctgtcaagcgtaactaatactccgcgccataactagctcggtcaaagaattaggagcgtgcaggatggcggaaagctttacgacgactaatcgatatttcgacaataaacattatccacgtggattctctcgtcatggtgatttcaccatcaaagaggcacaactgcttgagcgtcatggttatgccttcaatgagttggatcttggcaaacgcgagccggttaccgaggaagagaaactcttcgtagcagtatgccgtggcgaacgtgagccagtgacagaagcagaacgcgtgtggtccaagtatatgacgcgtattaagcgtccaaaacgttttcacaccctttccggcggtaaaccgcaggttgaaggtgctgaagactacaccgattctgacgattaataaaaagggcgaaatgccctttttttatgtcagtagtttctgcagatggatgagcaaacggtcaatcgctcgatagctaactgcctcctgcaaatgctgacgtgtgataatgtcagactgatcaatatcagcaatggttcgtgcaactttcaataaccgctgccaggcacgaatcgataaccccagatggatcagtgttccttccaaccacatcgcatcttcgctctcaagtttgcagaattggcgtatttccggactatccagccaggcattcagtttattctgccgcttaaattggcgctctctggcggccattacgcgttgtttaacggtggcgctgctttctcccggcactaccgttttactcaaaatgccggggggtggtaatgggatctccagtgagagatcgaagcggtcgagaaagggccccgagagccggttgagataacgtaatgtctgttctggcgtgcagcggttatggtttccctgataatgtccggtagggctgggattcatcgccgcaacaagctggaaacgggctggataggttatttttgctcgtgtgcgtgaaagatggatctgcccggattcaatcggctctcgcaaggcatccagtgtacgccgttcaaattcaggtagctcatcaagaaaaagcacgccgttatgcgccagcgaaatttcaccgggccctggaattgcgccaccgcctaccatcgcagttaacgatgcactgtgatgaggtgagcggaacgggcgctgccgccattgtttttgtactgattcagcatttaccagacttaatatcgcagcactctccagtgcctcttcattgcttaaatctggcaacaggccattaatacggctggcgagcattgttttacctgttcccggcggcccaatcagtaaaaggttgtgcccgccagcagcggtaatttccagtcctcgctttccttgttcctgaccgataacatcactgagatcatgttgtagcgcccgggatactgcatcagttggtttcgggcgttcgagagcgtgcttaccttccagaaacgcacagacagcttgcagatgatcggctatcaggcatccttcaccgttaattagccccacttcatcttcgttatctttcgcgacgataatttttctgcccgacttaatagcttcagttgcactggagattgcgccgggaacgccacgcagagcgcctgtaagcgccagttctccgactaattcatattcatctaacttattggctgtaagctgttctgaggccgccagcaacgcaatggcgataggtaaatcatatcgtcccccttcttttggcagatcagctggagccaggttgatggtgatttttttcgccggatattcatatccgctattgataatggcgctgcgcacgcgatcgcgagcttcttttaccgttgtttctggtaagcccaccatcgttaagccgggtagacctttactgatatgtacctcaacagtgatcgggggcgcatttactcccagggctgcgcgggtatgaacaattgacagtgacataagccctccttgagtcaccattatgtgcataagatatcgctgctgtagcccgctaattcgtgaattttagtggctgattcctgtttatttgtgcaagtgaagttgagttgttctggcggtggaatgatgctcgcaaaaatgcagcggacaaaggatgaactacgaggaagggaacaacattcatactgaaattgaatttttttcactcactattttatttttaaaaaacaacaatttatattgaaattattaaacgcatcataaaaatcggccaaaaaatatcttgtactatttacaaaacctatggtaactctttaggcattccttcgaacaagatgcaagaaaagacaaaatgacagcccttctacgagtgattagcctggtcgtgattagcgtggtggtgattattatcccaccgtgcggggctgcacttggacgaggaaaggcttagagatcaagccttaacgaactaagacccccgcaccgaaaggtccgggggttttttttgaccttaaaaacataaccgaggagcagacaatgaataacagcacaaaattctgtttctcaagattcaggacggggaactaactatgaatggcgcacagtgggtggtacatgcgttgcgggcacagggtgtgaacaccgttttcggttatccgggtggcgcaattatgccggtttacgatgcattgtatgacggcggcgtggagcacttgctatgccgacatgagcagggtgcggcaatggcggctatcggttatgctcgtgctaccggcaaaactggcgtatgtatcgccacgtctggtccgggcgcaaccaacctgataaccgggcttgcggacgcactgttagattccatccctgttgttgccatcaccggtcaagtgtccgcaccgtttatcggcactgacgcatttcaggaagtggatgtcctgggattgtcgttagcctgtaccaagcacagctttctggtgcagtcgctggaagagttgccgcgcatcatggctgaagcattcgacgttgcctgctcaggtcgtcctggtccggttctggtcgatatcccaaaagatatccagttagccagcggtgacctggaaccgtggttcaccaccgttgaaaacgaagtgactttcccacatgccgaagttgagcaagcgcgccagatgctggcaaaagcgcaaaaaccgatgctgtacgttggcggtggcgtgggtatggcgcaggcagttccggctttgcgtgaatttctcgctgccacaaaaatgcctgccacctgtacgctgaaagggctgggcgcagtagaagcagattatccgtactatctgggcatgctggggatgcacggcaccaaagcggcaaacttcgcggtgcaggagtgtgacctgctgatcgccgtgggcgcacgttttgatgaccgggtgaccggcaaactgaacaccttcgcgccacacgccagtgttatccatatggatatcgacccggcagaaatgaacaagctgcgtcaggcacatgtggcattacaaggtgatttaaatgctctgttaccagcattacagcagccgttaaatcaatgactggcagcaacactgcgcgcagctgcgtgatgaacattcctggcgttacgaccatcccggtgacgctatctacgcgccgttgttgttaaaacaactgtcggatcgtaaacctgcggattgcgtcgtgaccacagatgtggggcagcaccagatgtgggctgcgcagcacatcgcccacactcgcccggaaaatttcatcacctccagcggtttaggtaccatgggttttggtttaccggcggcggttggcgcacaagtcgcgcgaccgaacgataccgttgtctgtatctccggtgacggctctttcatgatgaatgtgcaagagctgggcaccgtaaaacgcaagcagttaccgttgaaaatcgtcttactcgataaccaacggttagggatggttcgacaatggcagcaactgttttttcaggaacgatacagcgaaaccacccttactgataaccccgatttcctcatgttagccagcgccttcggcatccatggccaacacatcacccggaaagaccaggttgaagcggcactcgacaccatgctgaacagtgatgggccatacctgcttcatgtctcaatcgacgaacttgagaacgtctggccgctggtgccgcctggcgccagtaattcagaaatgttggagaaattatcatgatgcaacatcaggtcaatgtatcggctcgcttcaatccagaaaccttagaacgtgttttacgcgtggtgcgtcatcgtggtttccacgtctgctcaatgaatatggccgccgccagcgatgcacaaaatataaatatcgaattgaccgttgccagcccacggtcggtcgacttactgtttagtcagttaaataaactggtggacgtcgcacacgttgccatctgccagagcacaaccacatcacaacaaatccgcgcctgagcgcaaaaggaatataaaaatgaccacgaagaaagctgattacatttggttcaatggggagatggttcgctgggaagacgcgaaggtgcatgtgatgtcgcacgcgctgcactatggcacttcggtttttgaaggcatccgttgctacgactcgcacaaaggaccggttgtattccgccatcgtgagcatatgcagcgtctgcatgactccgccaaaatctatcgcttcccggtttcgcagagcattgatgagctgatggaagcttgtcgtgacgtgatccgcaaaaacaatctcaccagcgcctatatccgtccgctgatcttcgtcggtgatgttggcatgggagtaaacccgccagcgggatactcaaccgacgtgattatcgctgctttcccgtggggagcgtatctgggcgcagaagcgctggagcaggggatcgatgcgatggtttcctcctggaaccgcgcagcaccaaacaccatcccgacggcggcaaaagccggtggtaactacctctcttccctgctggtgggtagcgaagcgcgccgccacggttatcaggaaggtatcgcgctggatgtgaacggttatatctctgaaggcgcaggcgaaaacctgtttgaagtgaaagatggtgtgctgttcaccccaccgttcacctcctccgcgctgccgggtattacccgtgatgccatcatcaaactggcgaaagagctgggaattgaagtacgtgagcaggtgctgtcgcgcgaatccctgtacctggcggatgaagtgtttatgtccggtacggcggcagaaatcacgccagtgcgcagcgtagacggtattcaggttggcgaaggccgttgtggcccggttaccaaacgcattcagcaagccttcttcggcctcttcactggcgaaaccgaagataaatggggctggttagatcaagttaatcaataaatacaaaaaatgggacggcacgcaccgtcccatttacgagacagacactgggagtaaataaagtatgcctaagtaccgttccgccaccaccactcatggtcgtaatatggcgggtgctcgtgcgctgtggcgcgccaccggaatgaccgacgccgatttcggtaagccgattatcgcggttgtgaactcgttcacccaatttgtaccgggtcacgtccatctgcgcgatctcggtaaactggtcgccgaacaaattgaagcggctggcggcgttgccaaagagttcaacaccattgcggtggatgatgggattgccatgggccacggggggatgctttattcactgccatctcgcgaactgatcgctgattccgttgagtatatggtcaacgcccactgcgccgacgccatggtctgcatctctaactgcgacaaaatcaccccggggatgctgatggcttccctgcgcctgaatattccggtgatctttgtttccggcggcccgatggaggccgggaaaaccaaactttccgatcagatcatcaagctcgatctggttgatgcgatgatccagggcgcagacccgaaagtatctgactcccagagcgatcaggttgaacgttccgcgtgtccgacctgcggttcctgctccgggatgtttaccgctaactcaatgaactgcctgaccgaagcgctgggcctgtcgcagccgggcaacggctcgctgctggcaacccacgccgaccgtaagcagctgttccttaatgctggtaaacgcattgttgaattgaccaaacgttattacgagcaaaacgacgaaagtgcactgccgcgtaatatcgccagtaaggcggcgtttgaaaacgccatgacgctggatatcgcgatgggtggatcgactaacaccgtacttcacctgctggcggcggcgcaggaagcggaaatcgacttcaccatgagtgatatcgataagctttcccgcaaggttccacagctgtgtaaagttgcgccgagcacccagaaataccatatggaagatgttcaccgtgctggtggtgttatcggtattctcggcgaactggatcgcgcggggttactgaaccgtgatgtgaaaaacgtacttggcctgacgttgccgcaaacgctggaacaatacgacgttatgctgacccaggatgacgcggtaaaaaatatgttccgcgcaggtcctgcaggcattcgtaccacacaggcattctcgcaagattgccgttgggatacgctggacgacgatcgcgccaatggctgtatccgctcgctggaacacgcctacagcaaagacggcggcctggcggtgctctacggtaactttgcggaaaacggctgcatcgtgaaaacggcaggcgtcgatgacagcatcctcaaattcaccggcccggcgaaagtgtacgaaagccaggacgatgcggtagaagcgattctcggcggtaaagttgtcgccggagatgtggtagtaattcgctatgaaggcccgaaaggcggtccggggatgcaggaaatgctctacccaaccagcttcctgaaatcaatgggtctcggcaaagcctgtgcgctgatcaccgacggtcgtttctctggtggcacctctggtctttccatcggccacgtctcaccggaagcggcaagcggcggcagcattggcctgattgaagatggtgacctgatcgctatcgacatcccgaaccgtggcattcagttacaggtaagcgatgccgaactggcggcgcgtcgtgaagcgcaggacgctcgaggtgacaaagcctggacgccgaaaaatcgtgaacgtcaggtctcctttgccctgcgtgcttatgccagcctggcaaccagcgccgacaaaggcgcggtgcgcgataaatcgaaactggggggttaataatggctgactcgcaacccctgtccggtgctccggaaggtgccgaatatttaagagcagtgctgcgcgcgccggtttacgaggcggcgcaggttacgccgctacaaaaaatggaaaaactgtcgtcgcgtcttgataacgtcattctggtgaagcgcgaagatcgccagccagtgcacagctttaagctgcgcggcgcatacgccatgatggcgggcctgacggaagaacagaaagcgcacggcgtgatcactgcttctgcgggtaaccacgcgcagggcgtcgcgttttcttctgcgcggttaggcgtgaaggccctgatcgttatgccaaccgccaccgccgacatcaaagtcgacgcggtgcgcggcttcggcggcgaagtgctgctccacggcgcgaactttgatgaagcgaaagccaaagcgatcgaactgtcacagcagcaggggttcacctgggtgccgccgttcgaccatccgatggtgattgccgggcaaggcacgctggcgctggaactgctccagcaggacgcccatctcgaccgcgtatttgtgccagtcggcggcggcggtctggctgctggcgtggcggtgctgatcaaacaactgatgccgcaaatcaaagtgatcgccgtagaagcggaagactccgcctgcctgaaagcagcgctggatgcgggtcatccggttgatctgccgcgcgtagggctatttgctgaaggcgtagcggtaaaacgcatcggtgacgaaaccttccgtttatgccaggagtatctcgacgacatcatcaccgtcgatagcgatgcgatctgtgcggcgatgaaggatttattcgaagatgtgcgcgcggtggcggaaccctctggcgcgctggcgctggcgggaatgaaaaaatatatcgccctgcacaacattcgcggcgaacggctggcgcatattctttccggtgccaacgtgaacttccacggcctgcgctacgtctcagaacgctgcgaactgggcgaacagcgtgaagcgttgttggcggtgaccattccggaagaaaaaggcagcttcctcaaattctgccaactgcttggcgggcgttcggtcaccgagttcaactaccgttttgccgatgccaaaaacgcctgcatctttgtcggtgtgcgcctgagccgcggcctcgaagagcgcaaagaaattttgcagatgctcaacgacggcggctacagcgtggttgatctctccgacgacgaaatggcgaagctacacgtgcgctatatggtcggcggacgtccatcgcatccgttgcaggaacgcctctacagcttcgaattcccggaatcaccgggcgcgctgctgcgcttcctcaacacgctgggtacgtactggaacatttctttgttccactatcgcagccatggcaccgactacgggcgcgtactggcggcgttcgaacttggcgaccatgaaccggatttcgaaacccggctgaatgagctgggctacgattgccacgacgaaaccaataacccggcgttcaggttctttttggcgggttagggaaaaatgcctgatagcgcttcgcttatcaggcctacccgcgcgacaacgtcatttgtggttcggcaaaatcttccagaatgcctcaattagcggctcatgtagccgctttttctgcgcacacacgcccagctcaaacggcgttttctcatcgctgcgctctaaaatcatcacgcggttacgcaccggttcggggctgttttccagcaccacttccggcaacaatgccacgccacagccgagtgccaccatcgataccatcgcttcatgcccgccaaccgtggcgtaaatcatcgggttactgattttattgcgtcgaaaccacagttcaatgcggcggcgtaccggcccctgatcggccataataaacggcaccgttgaccagtccggcttctctaccgacacctgattacgcaccgggcagggcagcgcgggggcaatcagcactactgccagattctccagcatcgaaaacgccactgcgccgggcaaggtttccggtttacccgcaatcgccagatccgcttcaccagtgaccaccttttccatcgcatctgccgcatcaccagtagtaagtttaatctccaccgacgggtgttccgcgcggaagcgatccagaatcggcggcagatggctgtaggcagcggtcaccgagcagaagatatgtaattcgccagagagcgacggcccttgctgatcgatggtgtggcgcaactgctgatactgcaacagcgtttgctgggcgaaaacgcgcagctcttcgcccgcttcagtcagcgtcaccgtgcggttatcgcgcacaaacagcggctgaccgagatcttcttccaggcgctgaatctgccgtgagagcgtggatgggctaacgtgcatcgcccgcgcgctgcggccaaaatggcggctttccgccagatgcaggaaggttttcagatcgcgtaaatccacagggacagccctcgatgttgacgttgcaaaaattgcaatgtgacgttgtgaatatatcaatttccgcaataaatttcctgtcatatagtgaattcaatctcgcaaacgcgaaccgaacaataagaagcacaacatcacgaggaatcaccatggctaactacttcaatacactgaatctgcgccagcagctggcacagctgggcaaatgtcgctttatgggccgcgatgaattcgccgatggcgcgagctaccttcagggtaaaaaagtagtcatcgtcggctgtggcgcacagggtctgaaccagggcctgaacatgcgtgattctggtctcgatatctcctacgctctgcgtaaagaagcgattgccgagaagcgcgcgtcctggcgtaaagcgaccgaaaatggttttaaagtgggtacttacgaagaactgatcccacaggcggatctggtgattaacctgacgccggacaagcagcactctgatgtagtgcgcaccgtacagccactgatgaaagacggcgcggcgctgggctactcgcacggtttcaacatcgtcgaagtgggcgagcagatccgtaaagatatcaccgtagtgatggttgcgccgaaatgcccaggcaccgaagtgcgtgaagagtacaaacgtgggttcggcgtaccgacgctgattgccgttcacccggaaaacgatccgaaaggcgaaggcatggcgattgccaaagcctgggcggctgcaaccggtggtcaccgtgcgggtgtgctggaatcgtccttcgttgcggaagtgaaatctgacctgatgggcgagcaaaccatcctgtgcggtatgttgcaggctggctctctgctgtgcttcgacaagctggtggaagaaggtaccgatccagcatacgcagaaaaactgattcagttcggttgggaaaccatcaccgaagcactgaaacagggcggcatcaccctgatgatggaccgtctctctaacccggcgaaactgcgtgcttatgcgctttctgaacagctgaaagagatcatggcacccctgttccagaaacatatggacgacatcatctccggcgaattctcttccggtatgatggcggactgggccaacgatgataagaaactgctgacctggcgtgaagagaccggcaaaaccgcgtttgaaaccgcgccgcagtatgaaggcaaaatcggcgagcaggagtacttcgataaaggcgtactgatgattgcgatggtgaaagcgggcgttgaactggcgttcgaaaccatggtcgattccggcatcattgaagagtctgcatattatgaatcactgcacgagctgccgctgattgccaacaccatcgcccgtaagcgtctgtacgaaatgaacgtggttatctctgataccgctgagtacggtaactatctgttctcttacgcttgtgtgccgttgctgaaaccgtttatggcagagctgcaaccgggcgacctgggtaaagctattccggaaggcgcggtagataacgggcaactgcgtgatgtgaacgaagcgattcgcagccatgcgattgagcaggtaggtaagaaactgcgcggctatatgacagatatgaaacgtattgctgttgcgggttaagtgcgcgctgatgccctcaccccgaccctctcccacagggagagggagaaaacactcaaggccttctcctggagaaggccttgctattagttgcggtacagcaccttaatgatgtgatatccgaactgggtgtgcagcgggccggtcggctccagtaccggacaagagaaaaccactttatcgaacgccggaaccatctgaccctggcggaattcacctaaatcaccgccgcgtttgcctgatgggcaaatggagtgtttcttcgccagcttgccgaaatcggccccgttcttaatctgctcgagaagatccagagccagtttctcttcttttacaaggatatgcagtgctgctgctgtttttgccatgatcgtgccttgagtgaataattgtcaggcggcgattttagcatgatccgcagatgctaacgtaattgtcagtcagggagtggctggtacatatatggcaaaagcccggaaaatccgggcttcgcaggtccctcaaggggagaaaacttagggcctctatgggctacaaagtcattatcggggatggttattttattgtcaatttatgagcgatatggcattgattgacttgatgaccgccctctgtatgtctgcaaccaactcatgtggcaaacattgattaagataccctctgtaagtccttgctctgtttaatctgtttcgactgacttgttgtaccaggtcggctttggcccaacgaatctgctgatcaaagaattgcaggtcattgataacattactggctatttcaacatgcattccacgttttaacttgtctggtcgcgagtggttgataatggaacgacgatgcatgcgttgccattaatttttccgttgagcacgacaactaacctgttttttatcatttcaggaggaatgcggccatcgtaatacgtcgtgctgaacggtccattttggctaacaggatagttaccaaagttgcattccagtatttcaccaaccttagggctgaaattaatcgccacgagtaaacctctccttagtaaactctgaaaaagtaataacacaacgttacgacccgatattttctaagtctaatggattcacgatgaactccgatttcggtcttctctctctgatttaaacatccgcagccaaccggttagcggcttacacgcggtcacattcaaatgcgattctgctacaatcctccccccgttcgaagattgagcaatacacctatgcgtctaaaccccggccaacaacaagctgtcgaattcgttaccggcccctgcctggtgctggcgggcgcgggttccggtaaaactcgtgttatcaccaataaaatcgcccatctgatccgcggttgcggttatcaggcgcggcacattgcggcggtgacctttactaataaagcagcgcgcgagatgaaagagcgtgtagggcagacgctggggcgcaaagaggcgcgtgggctgatgatctccactttccatacgttggggctggatatcatcaaacgcgagtatgcggcgcttgggatgaaagcgaacttctcgttgtttgacgataccgatcagcttgctttgcttaaagagttgaccgaggggctgattgaagatgacaaagttctcctgcaacaactgatttcgaccatctctaactggaagaatgatctcaaaacaccgtcccaggcggcagcaagtgcgattggcgagcgggaccgtatttttgcccattgttatgggctgtatgatgcacacctgaaagcctgtaacgttctcgacttcgatgatctgattttattgccgacgttgctgctgcaacgcaatgaagaagtccgcaagcgctggcagaacaaaattcgctatctgctggtggatgagtatcaggacaccaacaccagccagtatgagctggtgaaactgctggtgggcagccgcgcgcgctttaccgtggtgggtgacgatgaccagtcgatctactcctggcgcggtgcacgtccgcaaaacctggtgctgctgagtcaggattttccggcgctgaaggtgattaagcttgagcagaactatcgctcttccgggcgtattctgaaagcggcgaacatcctgatcgccaataacccgcacgtctttgaaaagcgtctgttctccgaactgggttatggcgcggagctaaaagtattaagcgcgaataacgaagaacatgaggctgagcgcgttactggcgagctgatcgcccatcacttcgtcaataaaacgcagtacaaagattacgccattctttatcgcggtaaccatcagtcgcgggtgtttgaaaaattcctgatgcaaaaccgcatcccgtacaaaatatctggtggtacgtcgtttttctctcgtcctgaaatcaaggacttgctggcttatctgcgcgtgctgactaacccggacgatgacagcgcatttctgcgtatcgttaacacgccgaagcgagagattggcccggctacgctgaaaaagctgggtgagtgggcgatgacgcgcaataaaagcatgtttaccgccagctttgatatgggcctgagtcagacgcttagcggacgtggttatgaagcattgacccgcttcactcactggttggcagaaatccagcgtctggcggagcgggagccgattgccgcggtgcgtgatctgatccatggcatggattatgaatcctggctgtacgaaacatcgcccagcccgaaagccgccgaaatgcgcatgaagaacgtcaaccaactgtttagctggatgacggagatgctggaaggcagtgaactggatgagccgatgacgctcacccaggtggtgacgcgctttactttgcgcgacatgatggagcgtggtgagagtgaagaagagctggatcaggtgcaactgatgactctccacgcgtcgaaagggctggagtttccttatgtctacatggtcggtatggaagaagggtttttgccgcaccagagcagcatcgatgaagataatatcgatgaggagcggcggctggcctatgtcggcattacccgcgcccagaaggaattgacctttacgctgtgtaaagaacgccgtcagtacggcgaactggtgcgcccggagccgagccgctttttgctggagctgccgcaggatgatctgatttgggaacaggagcgcaaagtggtcagcgccgaagaacggatgcagaaagggcaaagccatctggcgaatctgaaagcgatgatggcggcaaaacgagggaaataatcaaggccggaaaagatgcgtcagcatcgcatccggcacttactcattaatgcacttccagcggccagtggacatagctctgccactggctttcctgagcaataatctctttacccagcggatgttgggttagccaaccttgcggaagcgtcaaggtcaacagttcatggttagcctgtaatgtcatctctggcacgagatcgtcacggcgacggctggcaaaaatgatggccaggcgtagtaaacggcagagttgttctgcgacgcgcggcggtacggcattttgctgatgcagcgatgagagatcgaccggattagtctggttgagcagtagcgtcgccagcaattttttctgtgcgggggtaaaaccgggaagatccagattacgcaccagataagcagcgtgttgcggcgcttgtttgaagtcaacgctcaggccgatttcatgaagctgacaggcgctgatgagcaaatcgcggcttattgcttcaagatgccattcgttttccacctgatcgaagaagttagccgcaactttggctacgcgctgtgcctgatcaatatcgatcataaagcggcgttgaatattacgcagcgtacggctgcgaatatcctgctcgacggccagatgcaacatgccgtagaccaggccttcacgcagcgcaccgcccgccagggtcatacactgaatattcagttcggtaaaaatggcgatcaggatcgccagaccactcgggaacactaacgcacgttccagcgtcagcccgtcaatctccagttcctccagccgaccgcaatgaatggctcgctgtttcaattgctgcaacttttccagggtaatgcgttcatccatcccctgtgccatcatgatttcctgtaacgcctgcacggtgccggaagcaccaacgcacactttccagccgtgataccgtaattcatcggcaaccggacgtaacacttcgcgtgccgctttttctgcagcatcaaaattttcctgccccagattacgatcggcaaaatagcgttccagccaggtgacgcagcccatcgacaggctgaacaacgaggtggtttgtgcacccgtgccggttaccagttcagtactggctccgcctatatccaccaccaggcgctgatcggcaccaccagtggtgtgagcaacgccctgataaatcagacgtgcttcctcttcaccgctgatcacctgtaccggacaaccgagaatttcctgcgctttggcaataaaatcacccgcattgacggcaaggcgtaacgtcgccgtagcgacaacgcgaatttgcgagggaggaatatcttgcagacgttcagcaaacaggcgcaaacattgccaaccgcgctccattgcttcattggagagggcattttcgctattcaggccagcagccagacgcactttgcgttttattcgcgtcagcgtctggatgcttccagccacctcgcgcacaaccagcatatgaaaactattcgaaccgagatcaatggctgcatacagcgacgaggtggaacccatactcttcatccttcaatctgtctctgtgttggctgcattctttcacctgaatcacttactacagtaagctcatcgggattcattctcttgccatcttgatacagtttgaatgattttgagtatgacattttttatttaacctgaacgacgacgattacgcggagcgccagtacgacgcggaccattgcctgtgcgcgggcgcgtgaggcgcagcggttttggcagatcggtcatcaatgcgtccggattgtatttgcttaccggaattgagtgaccaatataggtctcaatagcaggcaaattcaatgcatactcttcacacgccaggctgatagagtgaccgcttgcgcctgcgcgacctgtacgaccaatacggtgaacgtaatcttcacagtcatcgggtaaatcgtagttaaagacgtgcgtcactgccggaatatgcaaaccacgcgcggcaacgtcggtggcaaccagaatatccagatcgccacgggtaaattcatcaagaatacgcagacgttttttctgcgcgacatcgcctgtcaataaaccgacacgatgaccatctgctgccaggtggccccagatctcttcacaacggtgtttggtgttggcgaaaataatcgctctgtctggccactcttcttcgatcagcgtttgcagcaaacgcattttttcttcgttagaagggtagaaaagctcttctttaatacggtggcccgttttctgttccggttccacttcaatatattcggcattgttcatctgctcgaacgccagttcacgtacccggtacgaaagcgtggcggagaacagcatgttgaggcgctggtttgcaggcggcatacggcggaacagccagcggatatctttaataaagcccagatcgtacatgcgatcggcttcgtccagtaccaccacctgaatggcaccgaggttaatgtggttctgcttggcgtagtcaattaaacgccccgtggtgccaatcagaatgtcaacgccgctttccagcactttcagctgtttgtcgtagccatcaccaccgtaagccagacccagcttcaggccagtagcttccgccagcggttctgcgtcggcatggatctgcacggcaagttcacgcgtcggtgccataattaaggcacgcggctgattcaccttgcgatcggcaatcgcaggatgagagagaagataatgaaacgttgacgtaagaaacgccatcgttttcccggtaccggtttgcgcctgcccggctacgtcacgacccgccagcgtcagcggaagggccagtgcctgaatgggcgtacagttatgaaacccttttttttcaagggcttctacaaccttcggatgcagggcgaagtcggaaaacttctgttctgttaaatgtgttttgctcatagtgtggtagaatatcagcttactattgctttacgaaagcgtatccggtgaaataaagtcaacctttagttggttaatgttacaccaacaacgaaaccaacacgccaggcttattcctgtggagttatatatgagcgataaaattattcacctgactgacgacagttttgacacggatgtactcaaagcggacggggcgatcctcgtcgatttctgggcagagtggtgcggtccgtgcaaaatgatcgccccgattctggatgaaatcgctgacgaatatcagggcaaactgaccgttgcaaaactgaacatcgatcaaaaccctggcactgcgccgaaatatggcatccgtggtatcccgactctgctgctgttcaaaaacggtgaagtggcggcaaccaaagtgggtgcactgtctaaaggtcagttgaaagagttcctcgacgctaacctggcgtaagggaatttcatgttcgggtgccccgtcgctaaaaactggacgcccggcgtgagtcatgctaacttagtgttgacttcgtattaaacataccttattaagtttgaatcttgtaatttccaacgcttcccgttttatcttaaatgcgaagtgaacagatttctggctcgtcactcaatccgtcttgtcgtttcagttctgcgtactctcctgtgaccaggcagcgaaaagacatgagtcgatgaccgtaaacaggcatggatgatcctgccataccattcacaacattaagttcgagatttaccccaagtttaagaactcacaccactatgaatcttaccgaattaaagaatacgccggtttctgagctgatcactctcggcgaaaatatggggctggaaaacctggctcgtatgcgtaagcaggacattatttttgccatcctgaagcagcacgcaaagagtggcgaagatatctttggtgatggcgtactggagatattgcaggatggatttggtttcctccgttccgcagacagctcctacctcgccggtcctgatgacatctacgtttcccctagccaaatccgccgtttcaacctccgcactggtgataccatctctggtaagattcgcccgccgaaagaaggtgaacgctattttgcgctgctgaaagttaacgaagttaacttcgacaaacctgaaaacgcccgcaacaaaatcctctttgagaacttaaccccgctgcacgcaaactctcgtctgcgtatggaacgtggtaacggttctactgaagatttaactgctcgcgtactggatctggcatcacctatcggtcgtggtcagcgtggtctgattgtggcaccgccgaaagccggtaaaaccatgctgctgcagaacattgctcagagcattgcttacaaccacccggattgtgtgctgatggttctgctgatcgacgaacgtccggaagaagtaaccgagatgcagcgtctggtaaaaggtgaagttgttgcttctacctttgacgaacccgcatctcgccacgttcaggttgcggaaatggtgatcgagaaggccaaacgcctggttgagcacaagaaagacgttatcattctgctcgactccatcactcgtctggcgcgcgcttacaacaccgttgttccggcgtcaggtaaagtgttgaccggtggtgtggatgccaacgccctgcatcgtccgaaacgcttctttggtgcggcgcgtaacgtggaagagggcggcagcctgaccattatcgcgacggcgcttatcgataccggttctaaaatggacgaagttatctacgaagagtttaaaggtacaggcaacatggaactgcacctctctcgtaagatcgctgaaaaacgcgtcttcccggctatcgactacaaccgttctggtacccgtaaagaagagctgctcacgactcaggaagaactgcagaaaatgtggatcctgcgcaaaatcattcacccgatgggcgaaatcgatgcaatggaattcctcattaataaactggcaatgaccaagaccaatgacgatttcttcgaaatgatgaaacgctcataaatttgtcttatgccaaaaacgccacgtgtttacgtggcgttttgcttttatatctgtaatcttaatgccgcgctggcgatgttaggaaaattcctggaatttgctggcatgttatgcaatttgcatatcaaatggttaatttttgcacaggactggtgggtttggaacggactttcccttctgaataaaggtcttcgtggttatacttctgctaataattttctctgagagcatgcattgtgaatttactgacagtgagtactgatctcatcagtatttttttattcacgacactgtttctgttttttgcccgtaaggtggcaaaaaaagtcggtttagtggataaaccaaacttccgcaaacgtcaccagggattgatacctctcgttggggggatttcggtttacgcagggatttgcttcacgttcggaattgtcgattactatattccgcatgcatctctctatctcgcttgtgccggtgtgcttgttttcattggcgcgctggatgaccgttttgatatcagcgtaaaaatccgtgccaccatacaggccgctgttggcattgttatgatggtgttcggcaagctttatctcagtagcctgggttatatctttggctcctgggagatggtgctcggaccgtttggttacttcctgacgctatttgccgtctgggcggccattaatgcgttcaacatggttgatggcattgatggcttgctgggcgggttgtcctgcgtctcgtttgcagcaatcggtatgattttgtggttcgacgggcaaaccagcctcgcaatctggtgctttgcgatgatcgccgccatcctgccatacatcatgcttaaccttggtatcctgggtcgccgctacaaagtctttatgggtgatgcgggcagtacgctgattggttttaccgttatctggatcctgctcgaaacgacccagggcaaaacccatcccatcagcccggttaccgctttgtggataatcgccattccgctaatggatatggtggcgattatgtaccgtcgcctgcgtaaaggcatgagcccattctctcctgaccgtcagcatattcaccatttgatcatgcgtgccgggtttacttcccgtcaggcgtttgtgctgattacccttgccgcagcactgctcgcttccattggcgtgctggcagaatattctcattttgtcccggagtgggtcatgctggtgctctttttgctagcattcttcctctatggatattgcattaagcgtgcctggaaagttgctcgctttattaagcgcgtaaaacgcagactgcgtagaaatcgtggtggcagccccaatttaaccaaataaatgaggatgtgatgacacaaccaatgcctgggaaaccggccgaagacgctgaaaatgaactggatattcgtgggttgtttcgtaccttgtgggctgggaagctatggattattggcatggggctggcgtttgcgttaatcgcgctggcgtatacgttttttgctcgtcaggagtggagctcgacggcgattaccgatcgtccaacggtgaatatgctggggggatattactcgcagcagcaatttttgcgtaacctggatgtccgttcaaacatggcttctgccgaccaaccatcggtcatggacgaagcctataaagagtttgttatgcaactggcctcgtgggatacccgcagagagttctggctgcaaaccgactattacaaacagcggatggtgggcaacagcaaagccgatgcggcgttgctggatgaaatgattaacaacatccagtttatccccggagactttacccgcgcggtcaatgacagcgtgaagcttattgccgaaaccgcgcctgacgctaataacctgttacgtcagtatgttgcttttgccagccagcgtgcagccagccatctgaatgatgagctgaaaggcgcatgggcggcgcgtaccatccagatgaaagctcaggtgaagcgtcaggaagaggtggcgaaagccatctacgaccgccggatgaacagcattgagcaggcgctgaaaattgctgagcagcataatatttcgcgcagtgcgacagatgtacctgccgaggaattacctgattcagaaatgttcctgcttgggcgtccaatgcttcaggctcgactggaaaatttacaggccgtcggtccggcctttgatctcgactatgatcagaatcgggccatgttaaacaccctgaatgttggtccaaccctggatccgcgttttcagacctatcgctatttgcgtacgccggaagaaccggtaaaacgcgatagcccacgtcgtgccttcctgatgattatgtggggcattgtcggggggctgatcggggctggtgtcgcattaacccgccgttgctcgaaatagcaacactgctgcggtgagcgcaaaggcgctcgccgcttattcgaagagaatcgatgtgaaagtactgactgtatttggtacgcgcccggaagccatcaagatggcgccgttggtgcatgcgttggcaaaagatcctttttttgaggctaaagtttgcgtcactgcgcagcatcgggagatgctcgatcaggtgctgaaactcttttccattgtacctgactacgatctcaacataatgcagccaggacagggcctgacagagataacctgtcggattctggaagggctaaaacctattcttgccgagttcaaaccagacgtcgtgctggttcacggcgatacgacgacgacgctggcaaccagcctggcggcgttttatcagcgtattcctgttggtcacgttgaggctggtctgcgcacgggcgatctctattcgccgtggccggaagaggctaaccgtacattgaccgggcatctggcgatgtatcacttctctccaaccgaaacttcccggcaaaacttgctgcgtgaaaacgttgcggatagccgaatcttcattaccggtaatacagtcattgatgcactgttatgggtgcgtgaccaggtgatgagcagcgacaagctgcgttcagaactggcggcaaattacccgtttatcgaccccgataaaaagatgattctggtgaccggtcacaggcgtgagagtttcggtcgtggctttgaagaaatctgccacgcgctggcagacatcgccaccacgcaccaggacatccagattgtctatccggtgcatctcaacccgaacgtcagagaaccggtcaatcgcattctggggcatgtgaaaaatgtcattctgatcgatccccaggagtatttaccgtttgtctggctgatgaaccacgcctggctgattttgaccgactcaggcggcattcaggaagaagcgccttcgctggggaaacctgtgctggtgatgcgcgataccactgagcgtccggaagcggtgacggcgggtacggtgcgtctggtaggcacggataagcagcgaattgtcgaggaagtgacgcgtcttttaaaagacgaaaacgaatatcaagctatgagccgcgcccataacccgtatggtgatggtcaggcatgctctcgcattctggaagcgttaaaaaataatcggatatcactatgagttttgcgaccatttctgttatcggactgggttatatcgggctgccaacggcagcagcgtttgcctcacggcaaaaacaggtaattggtgtcgatatcaaccaacatgcggttgataccatcaatcgtggcgaaatccatatcgtcgaacctgatttggcgagtgtagtaaaaactgccgtagaaggcggttttttacgagcgagcacgacgccagttgaagcggatgcctggctgattgctgtacccacgccgtttaagggcgatcatgagccagatatgacctacgttgaatcggctgctcgctccattgcgccagtgctgaaaaaaggcgcgctggtgatccttgaatccacctcgccggtggggtcaaccgagaagatggcagaatggttagcagagatgcgtccggatctcactttcccgcagcaggtgggcgagcaggcggacgtcaacattgcttactgcccggaacgcgtgttaccaggacaggtaatggtcgagctgattaaaaacgatcgcgtgattggtggtatgacgccggtttgttcggcccgcgccagcgaactgtacaaaattttcctcgaaggtgagtgtgtcgtcactaactcgcggacggcggaaatgtgtaagctcaccgaaaacagcttccgcgatgtgaatatcgcttttgctaatgaattgtcgctgatttgtgccgatcaggggattaacgtctgggaactgattcgcctggcgaatcgtcaccctcgcgttaatattcttcagcctggccctggcgtgggcggtcactgcattgctgttgatccgtggtttatcgtggcacagaacccccagcaggcgcggcttatccgtaccgcgcgcgaagtgaacgatcacaaaccgttctgggttatcgatcaggtgaaagcggcggtggctgattgcctggcggctaccgataaacgcgccagtgaactgaaaatcgcctgctttggtctggcgtttaaaccgaatattgatgacctgcgcgaaagcccggcgatggaaatcgctgaactgatcgcccagtggcatagcggcgaaactctggttgttgagcctaacatccaccagttgccgaaaaaactgaccgggctttgtactctggcgcagcttgacgaggcgctggcaacggcagacgtgctggtgatgctggtcgatcatagtcagttcaaagttatcaatggcgacaatgtccatcagcagtatgtcgtcgatgccaaaggagtctggcgctgatgagaaaaattctgataacaggtggtgccgggtttattggctcggcgctggtgcgttatatcatcaacgaaacgagcgacgcggtggtagtggtcgataagctgacctacgccggaaacctgatgtcgctggcaccggtcgcgcaaagcgagcgctttgcctttgagaaagttgatatctgcgatcgggcagaactggcacgcgtattcactgagcatcagccagactgtgtcatgcatctggcagccgaaagccatgttgaccgttctattgacggcccggcagcgtttattgaaaccaacattgtcgggacttatacattgcttgaagcggcgcgggcttactggaatgcgctgacggaagataaaaaatcagcgttccgttttcatcatatctccactgacgaagtatatggtgacctgcactcgacggatgatttcttcaccgaaaccacgccgtatgcgccgagcagcccttattccgcgtcaaaagccagcagcgaccatctggtgcgcgcctggctgcggacctatggtctgccgacgcttatcaccaactgctcgaataactacggcccttaccactttccggaaaaactgatcccgctgatgatcctcaacgcgctggcgggtaaatcgctgccggtatatggcaacgggcagcaaatccgtgactggctgtatgtggaagatcacgcccgcgcgctgtattgcgtggcgaccaccgggaaagtcggtgaaacctataatattggtggtcacaacgagcgtaagaatctcgatgttgtggaaaccatttgcgagctgctggaagaactggctccgaacaagccgcacggcgtggcgcactatcgtgacctgatcacctttgtcgctgaccgtccggggcatgatctgcgttatgccattgatgcttcgaaaattgcccgtgaacttggctggctgccgcaggaaacctttgaaagtggaatgcgtaaaacggttcagtggtatctggctaatgaaagctggtggaagcaggtgcaggacggcagctatcagggcgagcgtttaggtctgaaaggctaattttcagcggaggcaaacatgaaaggtattatcctggcgggcggttccggcacccgattgcatccgattacgcgcggcgtatcgaagcaactgttgccgatttacgataagccaatgatttactatccgctgtcggtgctgatgctggccggtatccgcgaaattctcatcatcactacgccggaagataaaggttatttccagcgcctgctgggcgatggtagtgagttcggtatccagctggaatatgccgaacagcccagcccggacggtctggcgcaggcctttatcatcggtgaaaccttccttaatggtgaaccttcttgtctggtgctgggcgataacatcttcttcggtcagggcttcagtccgaagctgcgtcatgttgcggcgcgcaccgaaggggcgacggtttttggctatcaggtgatggacccggaacgctttggcgtggtggagtttgacgacaatttccgcgctatctcgctggaagaaaagccaaaacagccgaagtcaaactgggcggtgaccgggctttatttctacgacagtaaagtcgtggagtacgcaaagcaggtgaagccgtcggagcgtggtgaactggagattacctccatcaaccagatgtacctcgaggcgggcaacctgaccgttgaactgctcgggcgcggatttgcctggctggataccggcactcacgacagcctgattgaagccagcacctttgtacagacggtggaaaaacgccagggctttaagattgcctgcctggaagagattgcctggcgtaacggctggctcgatgacgagggtgtgaagcgtgctgccagttcattagcgaaaactggctacggccaatatctgctggagttacttcgtgcccgtccgcgccagtattgagccactaacctgggaaaacgccttctttggtgttaacagcgccatcgtgcgcattacgtctgaagcaccgctcctgacgccagacgcgttagcgccgtggtcacgggtgcaggccaaaattgcggcatcaaatacgggtgaactggatgccctgcaacagctgggattctccctggtagaaggtgaagttgatttggcgctacccgtgaacaatgccagtgatagcggtgctgtagtggcacaagagaccgatattcccgcattacgtcagttagccagcgccgcatttgcgcaaagccgttttcgtgcgccgtggtatgcgcctgacgccagcagtcgcttttatgcacagtggattgaaaatgccgtgcgcggcacctttgatcatcaatgtctgattttacgtgcggcgtccggcgatattcgcggctatgtctctttacgggaactcaatgcgacagatgcgcgaattggcctgctggctggacgcggtgcaggtgctgagctgatgcaaacggcgctaaactgggcgtatgctcgcggtaaaacaactttgcgggtggcgacccaaatgggcaacaccgccgcgcttaaacgatacatacaaagtggtgcgaatgtagaaagcaccgcgtactggttatacaggtgatcacatgattccatttaacgcaccgccggtggtgggaaccgaactcgactatatgcagtcggcaatgggtagcggcaaactgtgtggcgatggcggttttacccgtcgctgccagcagtggctggagcaacgttttggcagcgccaaagtgttactgacgccgtcctgcaccgcttcgctggagatggcggcgctgctgctcgatatccagcctggcgatgaagtgatcatgccgagctacacctttgtctccaccgccaatgcctttgtgctgcgtggcgcaaaaatcgtttttgtggatgttcgcccggacaccatgaacatcgacgaaacgctgattgaagcggcgatcaccgacaaaacgcgcgttatcgtgccggtccattacgcgggtgtggcctgcgaaatggacaccattatggcgttggcgaaaaagcataatttgtttgtggtagaagatgccgctcagggcgtgatgtccacttacaaagggcgtgcactgggaaccattggtcatattggctgctttagcttccatgaaaccaaaaactacacggcgggcggtgaaggcggcgcgacgctgattaacgataaagcgttaatcgaacgagccgagatcatccgtgaaaagggcactaaccgcagccagttcttccgtggtcaggtcgataaatatacctggcgcgatattggctccagctatttgatgtccgatctgcaagctgcatacctgtgggcgcaactggaagcagcggatcgtatcaaccagcaacgtctggcgctgtggcaaaactactacgatgcgttagcgcctctggcgaaagccgggcgtatcgagctgccgtcgattcccgatggctgcgtgcagaacgcgcatatgttctacattaaactgcgggatattgatgaccggagcgcgttgattaactttctgaaagaagcggaaatcatggcggtgtttcattacattccgctgcacggttgccctgcgggggaacactttggtgagttccacggtgaagatcgctacaccaccaaagagagcgagcgcctgctgcgcctgccgctgttctacaacctgtcgcccgtcaatcagcgtacggtaattgcgactttgttgaactacttttcctgatatgtcgttggcaaaagcgtccttgtggacggcggccagtacactggtcaagattggtgccgggttactggtcggtaagttgctggcggtgtcatttggtccggcggggcttgggctggcggcaaatttccgccagttgattaccgtgctcggcgtgcttgccggggctggcatctttaacggtgtaaccaaatacgttgcccagtaccatgataatccgcaacagctgcgccgcgtggtcggcacttcatcagcgatggtacttggtttctctacgctgatggcgctggtttttgtgctggcagctgcgccaatcagccagggattgtttggtaataccgactatcaggggctggtgcgtttagtggcgctggtgcaaatggggatcgcctggggcaacctgttactggcgctgatgaaaggctttcgcgatgccgcaggtaatgcgttatcgctgattgtcggcagcttgattggcgttctcgcgtactacgtcagttaccgtttgggcggttatgaaggggcgttgctgggtctggcgctgattcccgcgctggtggtaattcctgccgccatcatgttgatcaaacgtggtgtcatcccgttaagctatctgaaacccagctgggataacggtctggcagggcagttgagcaaatttacgctcatggcgttgattacgtcggtgaccttgcctgttgcttacatcatgatgcgtaaactgctggcggcgcagtatagctgggatgaggtggggatctggcaaggggtgagcagtatttccgatgcctacctgcaatttattacggcatcgttcagcgtatatttgctgcccacgttgtcgcggctaacggaaaagcgcgatatcacccgggaagtggttaaatcgctgaaattcgtcttaccggcagtggcggcggcgagttttaccgtctggctgctgcgtgattttgctatctggctgctgttgtcgaataaatttaccgctatgcgcgatctctttgcctggcagttagtgggtgatgtgttaaaagtgggcgcttatgtctttggttatctggtgatcgccaaagcgtcactgcggttttatattctggcggaagtcagccagttcactttattgatggtatttgcccactggctaatccctgcgcatggtgcactgggcgcggcgcaggcatatatggcaacttatatcgtctatttttctctttgttgtggcgtgtttttactctggcgtaggcgggcatgactgtactgattcacgtactgggatcggatatccctcaccataaccgaaccgttttgcggtttttcaatgacgcgctggccgcgacgagcgagcacgcgcgcgagtttatggttgttggcaaggacgacggcttaagtgatagctgtccggcgctttctgtgcaatttttccctgggaaaaaatcgctggcggaagcggtcatcgcgaaagcaaaagctaaccgtcagcagcgttttttcttccacggtcagttcaatcccacactgtggctggctctgctgagtggtggcattaagcccagccagtttttctggcatatctggggggcagacctgtatgagctttccagtggcttgagatataagcttttttacccactacgtcgcctggcgcaaaagcgagtcggctgtgtatttgccacccgcggcgatttgagcttttttgccaaaacgcacccaaaggtgcggggcgaactgctgttcttcccgacgcggatggacccttcgctcaatacgatggcgaacgatcggcaacgtgaagggaaaatgaccattctggtggggaactccggcgaccgcagcaatgagcatattgctgccttgcgcgccgttcatcagcaatttggcgatacggtaaaagtggtggtgccgatgggatatccgcctaataacgaagcgtacattgaggaagttcgtcaggcggggctggagttattcagcgaagaaaatctacaaattctgagcgaaaaactggaatttgacgcctatctggcgctacttcgtcagtgcgatcttggttactttatttttgcccgccagcagggcattggtacgctgtgcttactgattcaggcgggcattccttgtgtgcttaaccgggaaaatccgttctggcaggatatgacggaacaacatttgccggtgctgtttactaccgacgatctcaacgaggatattgtgcgtgaagcgcagcgccagttggcgtcggtggataaaaacaccattgccttctttagccctaactatctacaaggctggcagcgggcgttggcgattgccgccagggaggtcgcatgagtctgctgcaattcagtggcctgtttgttgtctggctgctctgcacgctgtttattgccacgctgacctggtttgagtttcgccgtgtgcgctttaacttcaatgtcttcttttcattgctgtttttgctcacctttttcttcggcttcccgctgaccagcgtgctggtatttcgctttgatgttggtgtcgcgccgccagaaatcttgttgcaggcgttgctttctgcgggctgcttctacgcggtttactatgtcacctacaaaacccgcctacgcaaacgcgttgctgatgtaccgcgccgtccgctgtttaccatgaaccgcgtggagaccaatcttacgtgggtgatcctgatgggtatcgcgctggtaagcgtcggcatcttcttcatgcacaacggctttttgctgttccggcttaactcctacagtcagatcttttccagtgaagtctccggcgtggcgttaaaacgcttcttttactttttcatcccggcgatgctggtggtctactttctgcgccaggacagcaaagcgtggctgtttttcctcgtcagcacggtcgcctttggcttgctgacttatatgattgtcggcggcactcgcgccaatatcatcatcgcattcgctatcttcctgtttattggcattattcgcggctggatttcgttgtggatgctggcggcggcgggcgtgctggggattgttggcatgttctggctggcactaaaacgctatggaatgaatgtgagcggcgatgaagcgttctatacgtttctctatctcactcgcgacaccttctcgccgtgggagaatctggcgttgctgttgcagaactacgacaacatcgacttccagggcctggctccaattgtccgcgatttctatgtctttatcccttcctggctgtggccgggtcgcccgagtatggtgctgaactcagccaactactttacctgggaagtgctgaataaccactccggactggcgatctcgcctacgcttataggctcactggtggtgatgggcggcgcgttgttcatcccgctcggggcgatcgtggttggtctgatcatcaaatggttcgactggctgtatgagctgggcaaccgcgagcctaatcgctataaagctgcgatattgcacagtttctgctttggggcgatcttcaatatgatcgtgctggcgcgtgaagggctggattcgtttgtctcacgcgtggtcttttttatcgtggtcttcggcgcatgtctgatgatcgcaaaactgttgtactggctttttgaaagcgccggactcattcataaacgtacaaaatcatcgctccggacgcaggttgaaggataacaatgaataacaacaccacggcaccaacctatacgctgcgtggcttacagttgattggttggcgtgatatgcagcacgccctcgattatctgtttgctgacgggcagcttaagcagggaacgctggttgccattaatgctgaaaaaatgctgactattgaagataacgccgaggtcagggagttaattaacgctgccgaatttaaatatgcggatggcatcagcgttgtacgttcagtacgtaaaaagtacccgcaggcgcaggtttcccgcgttgccggtgccgatctctgggaagagctgatggcgcgcgcaggcaaagaagggacgccggtatttcttgtgggcggtaaacctgaagtgctggcgcaaactgaagctaaactgcgcaaccagtggaatgtgaatatcgttggcagtcaggatggttattttaaacccgagcagcgtcaggcgctgtttgaacgcattcatgccagcggtgcgcaaatcgtcaccgttgcgatgggatcgccaaagcaggagatcatcatgcgcgactgccgtctggtacatccagatgcgctgtatatgggcgttggcgggacttacgatgttttcaccggtcacgtaaaacgcgcaccgaaaatctggcaaacgctggggctggagtggctctaccgcctgctttcgcagccgagccgcattaagcgtcagcttcgtttgctgcgttatttacgctggcactacaccggcaacctatgattttcctctctttgtaaagcgacggagtggtcactccgtcgcctgtctgcttttttattacacaaagcattcaaatttttaatgctttatttgccatttctcctgaattacgaaaacatttgcaacactcgatgtacccataacgataaccggtaacaccggaaagcatgcaaacacaacacgaggatttatggcagataacaaaccagagctacagcgtgggctggaagctcgacatatcgaactcatcgccctggggggcaccattggcgtcggcctgtttatgggggccgccagtaccctgaaatgggccgggccatccgtattgttggcctatatcatcgccgggctgttcgtctttttcatcatgcgttcaatgggcgaaatgttgttcctcgaaccggttaccggttcgttcgccgtttatgcgcatcgttatatgagcccgttctttggctatctcaccgcctggtcttactggtttatgtggatggcggtggggatctctgaaatcaccgccattggcgtttatgtccagttctggttcccggagatggcgcagtggatacccgcattgatcgcagtggcgctggtggcgttggcgaatctggcggcggtgcggttgtacggcgaaatcgagttctggttcgcgatgatcaaagtcaccacgattatcgtgatgattgtcattggcctgggcgtgattttctttggctttggcaatggcgggcagtcgattggttttagcaatctcacagagcatggcggtttctttgcgggtggctggaaagggttcctgaccgctctgtgtattgtggtggcgtcctaccagggcgtggagctgattggcattactgccggtgaagcgaagaatccgcaggtgacgctgcgcagtgccgtaggcaaggtgctgtggcggatcctgattttctacgtaggcgcgattttcgttatcgtcaccatcttcccgtggaatgaaataggcagcaacggcagcccgttcgtactgacttttgccaaaatcggtattaccgcagcggcgggcattatcaactttgtggtgctgacggctgcgctctctggctgtaacagcggcatgtacagttgcggacgtatgctctacgcactggcgaaaaaccgtcagttaccggcggcaatggcgaaagtttcccgtcacggcgtaccggttgcgggtgtggcagtatctattgctattctgctaattggctcatgcctgaactacatcattcccaatccgcagcgtgtgtttgtctacgtctacagtgccagcgtgcttccggggatggtgccatggtttgtgatattgataagccagctgcgttttcggcgtgcacataaagcggcgattgccagccatccgttccgctcaatcctgttcccgtgggccaattacgtaacaatggcattcctgatttgcgttttgatcggcatgtactttaatgaagatacgcgtatgtcgctgtttgttggcatcatctttatgctggcggtgacggcgatttataaagtttttggccttaatcgccacgggaaagcgcataaactggaggaataagcagcaaaacgcacaaaccgtaaccaaacgcgcaatttatttaaaaagggactagacagaggggtgggaagtccgtattatccacccccgcaacggcgctaagcgcccgtagctcagctggatagagcgctgccctccggaggcagaggtctcaggttcgaatcctgtcgggcgcgccatttagtcccggcgcttgagctgcggtggtagtaataccgcgtaacaagatttgtagtggtggctatagctcagttggtagagccctggattgtgattccagttgtcgtgggttcgaatcccattagccaccccattattagaagttgtgacaatgcgaaggtggcggaattggtagacgcgctagcttcaggtgttagtgtccttacggacgtgggggttcaagtcccccccctcgcaccacgactttaaagaattgaactaaaaattcaaaaagcagtatttcggcgagtagcgcagcttggtagcgcaactggtttgggaccagtgggtcggaggttcgaatcctctctcgccgaccaattttgaaccccgcttcggcggggttttttgttttctgtgcatttcgtcaccctcccttcgcaataaacgcccgtaataactcattgccccacggtatgatttcgcccttaacgtattgaaggatgacttcaggcaaggagcgaccatgctgcaacaggttccaacgcgtgcttttcatgtgatggcgaaaccgagcggttccgattgtaatctgaactgtgactactgtttttatctcgaaaaacaatccctttaccgcgaaaagccagtcacgcatatggacgatgacacgctggaagcgtatgtccgtcactatatcgctgccagcgaaccgcaaaacgaagtggcttttacctggcagggcggcgaaccaacgctactcgggctggcgttttaccgccgtgccgtagcgctacaggcgaaatatggtgctggcaggaagataagtaacagcttccagactaacggcgtgctgctggatgacgaatggtgcgcgtttctcgcggagcatcattttcttgttggtttatcgctggatggcccgcctgagatccacaatcaatatcgcgtgactaaaggtggcagacccacgcataagctggtgatgcgtgccctgacgctcctgcaaaaacatcatgtcgactataacgtgctggtctgcgttaatcgcaccagcgcgcagcaaccgttgcaggtatatgattttttgtgcgatgcgggagtcgaattcatccagtttattccggtggtcgagcgcctggctgatgaaacaactgcccgcgatggacttaagttacatgcgcctggtgatattcagggtgagctaacggaatggtcggtgcgccccgaggagttcggtgagtttctggtggcgatattcgaccactggatcaaacgcgacgtcggcaagattttcgtgatgaatatcgaatgggcgtttgccaattttgtcggtgcgccgggtgcggtttgccatcatcagccaacctgtgggcgctcggtgattgttgagcacaacggcgacgtttacgcctgtgatcactatgtttatccgcaatatcggctggggaatatgcaccagcaaacaattgcagaaatgatcgattccccgcaacagcaggcgtttggtgaagataaatttaagcagttaccggcgcagtgtcgcagttgtaacgtgttaaaagcgtgctggggaggctgcccgaaacaccgcttcatgctcgatgccagcggcaaaccgggactgaattatttgtgtgccgggtatcagcgttatttccgccatctaccgccatatcttaaagcaatggctgatttgctggcgcacggtcgcccggccagcgacattatgcatgcgcatttgctggtggtgagtaagtagaaatcggcggccgcctgcggttgattgccggatgcggcgtaaacgccttatccggcctacatgatcgtgcaaattcaataaattgcagcgttctgtaggctggataagatgcgtcagcatcgcatccggcaaaggcagatctcagcgatagcgccggcttagtcagatttaatctgcgcgcgtggtggatattttttcaggatctccatatacgcgtgcatttcggtctgtagcggtacacccatcggaatatggcgcacgccgatggagtcgctttcctgcggatcggtgtagaggttaaacaccgacgatcccgccgtttgcattactgtgccggtgaatccaccctgatatccgctctgggtataagcgtaaggttgctgaatcaggacgtgatacttgaactcatccatacgcacagcagcgagtttaccgttgaggaagtagtgctcggccttacggttagactgaccatttgttcccaggaagaaggatgtctggtccacaccatcgataaaggtggttttcggcactaaattcgccactttcgctccaggatgccctgccagatccagcgcggtagggaagagatctgccagatcgacaataccgtcagatttacgcggttggatcatccctttccagtaaacgaaagtcggtacgcgaacgccgccttcccaggtcgaacctttcgcaccacggaacggggtgcgtccgtgcggcggtacttcggcttccggtccgttatcggaggtaaagacgatcagcgtgttatcaagctgaccgtttttctccagtgttttatacagattagcgaacacatcgttcatctccaccatgcagtcgccatacgaggtgcgtgccggagagctacccgcatatttcgcatttgggtagttatcgaagtggcagccacgagtgccgtagtagaggaagaatggtttatcgctcttcgccatcttgtcgaggaacttaacgccatagtccatccagcgttgatccagatcttccatatatttcggcgtaatgtcggcaatggcctgttgttcgccgccgcgcaccgcatgaacgtcatctttgctgaacggtaattgcttgatgtattcagaacggtccggactcagggccacttccggattgacgtgaacgtcgcgccattcggtgtacatatcagacaccgagttaaagccacggaaatcatcaaagccaacgttctgcggctgcgactctttgttttcccccatatgccattttccgatggcctgagtgacgtagccctgatcgtgcagcaactgcggcagcgtggttaacccttgcagcccgcccggttgcccgtacattggcggcatcagaatgccgtggtggatggagtattgtccggtgagaatggtggcgcgggttggggaagagcttggttgagaatacgccgaagttaaaatcagcccctggctggcaacggcgtcgatatctggtgtagggttacccaccgccacgccgccaccgttaaaaccgacgtccatccagcccacatcgtccagcaagaaaacaaccacattcggtttcttaccggtttttttctcaagttctgccagcttctgctgggtttctttatcctgcgccggatgctgcattactggcatcatattgtcggcaatagtggtcgccggtttaaccagatactggtttgggtgatcgtatccggcaaagcctttgcgtgcggtggcagttgacggggtatctgctgcgctggccatgagaggaagagcggcggcgacagcaacaacaagacgtttgggtgaaaacgaaaattccatgcaaaatgctccggtttcatgtcatcaaaatgatgacgtaattaagcattgataattgagatccctctccctgacaggatgattacataaataatagtgacaaaaataaattatttatttatccagaaaatgaattggaaaatcaggagagcgttttcaatcctacctctggcgcagttgatatgtaaggcaggtttattatatcgcgttgattattgatgctgtttttagttttaacggcaattaatatatgtgttattaattgaatgaattttatcattcataataagtatgtgtaggatcaagctcaggttaaatattcactcaggaagttattactcaggaagcaaagaggattacagaattatctcataacaagtgttaagggatgttatttcccgattctctgtggcataataaacgagtagatgctcattccatctcttatgttcgccttagtgcctcataaactccggaatgacgcagagccgtttacggtgcttatcgtccactgacagatgtcgcttatgcctcatcagacaccatggacacaacgttgagtgaagcacccacttgttgtcatacagacctgttttaacgcctgctccgtaataagagcaggcgtttttttatgtatcaggaaggccccggaggtgcttgcctccgggtgagaaggaactactgtggcgggttattctgcaacgttaacatcaaaccgtcgcgacgcatagctgcagcttcttccggcttgtgcagtctgtccagcgcgtcggcaagccatgcgtaatcgtaggcgtccggacgttgtttcagcgctgcgcggaaggcgagcgatgcttcctgccattctccgtgcttcatcagtgactggcccagtgtgctccacaacagcgggcgatcgccgacgtttttgatttgctggcgcagcactttttccagctgttccggattgtttgttttcagtcgaggaatcggcagcagtaggcgatcgtcgtactggcgtttcaggccatcgatgataatttgctgggcagtatcatgatcgtcacattcaataagatgttccgccattgccacctgcaacgctacctgatgacgcgttttccggctttggtttttccaccagttacgcaaaccttcgctaccgttatcggcacgcgcctgatccatcaggccaatccatgcctgttgttccagcattgcacgatgttcttcatcaccaacatgggctttcgccattgatgggataatatccagcagcgaactccatgcacctgtgcggatatacgcctgttccgccagacgtaatacttccggatggcgtggcgtaacttccagcagcttatccacgccgtggcgtgcagcatggttttcattacgggccagttgcagacgtacgcgggtgatttctaccggaatggtgtcgttgccggccagctccgctgcgcgttccagatgttggttggcgcgtgcttcatcaccacgttgttgcgcggcttcggcagccagtagatagttcaccaccggttgttccgcgtgatcggcatttttcgccatcagcttttcaacttgctgataatcgccttccgccagtttcagcagcgcctgttcggtctgcttacgtgcacggcgacgcttacgtccgacaaaccacccacgggtgtgcgcgccagtgcggaagatccgccgcagtagccactcaatggcaaacagcactaccatcgccagaatcaatatgatcgccaggcccgtgacgctggtttcgatattgtagttgtcggtctggatcagcacataaccctgatggccggcaatcatcgggccaaccacgatccccgcaatcagcaacacaaagagcaataacacttttagcatggttattctccttgcggcgcggctgccggagtatcagcttgcggtgcaggtgcaggtttagcttccgttgtccccgctgccggttgtgccagcaggttacgcacgcgagtctgcatcagtttttccagcatcgcctggctttgcagggtttccggaagatccatcgagatattttgctggcttaactggtccacctcgtcgaggaacgctttggtggtggcatcatcagtatcgtagtaagcacgtacccaggtggagacgttctccagcgcctggcgataagtctcttcctggtgacgcggtacagcttgtgctgcgaccagcaggcgagagcgaatattttcgcgcagatagatatcctgatttggcgctaacagcggtacggcggtgtcatcacgacggcgaatcgtaatgaagttgtccataaagttctgccagcttttttgcagattgatacgccattcgctgatggaactggaaagctcttcaccgtctgaatccatcggcgaaccatcgctgtcattatcggccagacgcaggttatctacctgatttgaaagctgattaagcttaaggatgatgccgtcataatccacctgcgatactgcagaaaggctggcgatatcatcggtaattgcccgacgaacggtaatcagactcgggtcattcatatccgccaggctggcgtctgcacttttcagcaacgctgcagcggtcgtgacgtcctgatcgctccacagcttccgtccggcgagtttcaccagaaaatcggcctgagccagcagccaggttttagcatcgctgccggaaatggtggcgaccttttgttggacttcatccaactgttttgccagcgtttcttgctgacgattcgcctgcttaagttgtgcagcttgttgcttaataatgccttccagctcggctttttggctctcctgggctttttgcaatgccgtcagttggttagccagggcatcgctggtggcggtctgattgacggcctgttgtttaccccagccatacaaaccgatgcccgccgccagagcaatagcgatagccaccgcgctgagaatcaatgcggtattgttcttactctttttttctgttgcgacaggttgtgacgtggtgtccacggcctccctggtctcttcaaccacggcggaggttttttcttgttccgtcattatggcttcctgttatgagagttattgtaatgcccgtaaaagcgcatcgttgtcagcgttatcggcgaccttaatgtcttgccagcccagttcccgggcgagtttcgccaaacgctcactgacgaccaatagtcgacagtgtagtaaccagtgctcacgataccattgtgggatcagcgaccagagttgctgcaacatttcaccgctggtaacaacgaccatcgtcacctcgcgggcttgccagcgcatcgcttcttctgcaccatcgtaatggattgcgcatcgttgataacattcacaaaaagtgacctcagcaccgcgcgccgtcagggtatccccaattagctcacgaccaccattgccacgtaatatcagcgcacgtttgcccgcaatattttgtaattcaggtaattgtagcaagacttcgctgatttcccgatcctgcgggtagagaatcttctgtccacttacggtatgtagtgccagtgcggtggtgcgtccaatggcgaaataatcaggtagtcggggccatttacgatcttgctgatgcagctgtgattgggcaaaagcaaccgcgtgttgcgagagggcaaacaacagatcgctctcccccagcgctgccagttgatcagcaagttgcggtaattgttgacccggagaaaactcaatcagcggaaaatgccaggccacctgccccagtgtgcgcagacggctcactaactcttctccagcgggagacgggcgggtgacaaggatactcatgccggggcgtctccgttatagacttcagcgaggatctcgcgcgcgccgttattcagtagctcttctgccagcgaaatccccatttgttcggcatcttgcggcgcaccgcggcgttcaccgcgaataatctgcgaaccgtccggcgcgccgaccagcgcacgcagccagatttcgccatcaataagctcggcgtagctaccaattggcacctgacatccgccttcgagacgggtattcatggcgcgttctgcggtaacgcgcagtgcagtttcgtggtgattcagcgcggcaagcagctcgcgagtgcgtgaatcatcaaggcggcattcaatacccaccgcaccttgtcctaccgccggaagagaaatctcgggtggcaacgcggcgcgaatacgtgactccagacctaaacgttttagtccggctacggcaagaatgatggcatcgtattcgccgttatccagtttgctcaggcgagtgccgacgttgccgcgcagggagcggataatcagatccggacggcgttcagccagttggcactggcgacgtaaactggacgtcccgacgatactgcctgccggtaacgcatccagactgtcatagttattggacacaaaggcatcgcgaggatcttcacgctcacaaatagtgaccagtcccagaccttgcgggaattcaaccggcacatctttcattgagtgtacggcgatatcggcgcgattttcgaggagcgcgacttccagctcttttacaaataagccttttccgcctactttcgccagcggcgtatcaagaatcacatcgccgcgcgtcaccatcggtaccagttcaacgaccaggcccggatggctcgccatcaacttgtctttgacatagtgtgcctgccagagtgcaagtgggctttggcgtgtggcaattcttaaaacattgtctaacatgcttgttaccgtcattatcatccgtggtccatcctaacatccttgccagagtgatgtcagtgttgtggtgaaacgtagacgcctgcgcaaaccgtaaaatgaggtctggcagtggatcctgacaggcgtttcacgccgttgtaataaggaatttacagagaataaacggtgctacacttgtatgtagcgcatctttctttacggtcaatcagcaaggtgttaaattgatcacgttttagaccattttttcgtcgtgaaactaaaaaaaccaggcgcgaaaagtggtaacggttacctttgacatacgaaatatcccgaatgccgcgtgttaccgttgatgttggcggaatcacagtcatgacgggtagcaaatcaggcgatacgtcttgtacctctatattgagactctgaaacagagactggatgccataaatcaattgcgtgtggatcgcgcgcttgctgctatggggcctgcattccaacaggtctacagtctactgccgacattgttgcactatcaccatccgctaatgccgggttaccttgatggtaacgttcccaaaggcatttgcctttacacgcctgatgaaactcaacgccactacctgaacgagcttgaactgtatcgtggaatgtcagtacaggatccgccgaaaggtgagcttccaattactggtgtatacaccatgggcagcacctcgtccgtagggcaaagttgttcctctgacctggatatctgggtctgtcatcaatcctggctcgatagcgaagagcgccaattgctacaacgtaaatgtagcctgctggaaaactgggccgcctcgctgggtgtggaagtcagcttcttcctgattgatgaaaaccgcttccgtcataatgaaagcggcagcctggggggcgaagattgtggctccacccagcatatactgctgcttgacgaattttatcgtaccgccgtgcgtctcgccggtaagcgtattctgtggaatatggtgccgtgcgacgaagaagagcattacgacgactatgtgatgacgctttacgcgcagggcgtgctgacgccaaatgaatggctggatctcggtggcttaagctcgctttctgctgaagagtactttggtgccagcctttggcagctctacaagagtatcgattccccatacaaagcggtactgaaaacactgctgctggaagcctattcctgggaatacccgaacccacgtctgctggcgaaagatatcaaacagcgtttgcacgacggcgagattgtatcgtttggtctcgatccatactgcatgatgctggagcgtgttactgaatacctgacggcgattgaagattttacccgtctggatttagtacgtcgctgcttctatttaaaagtgtgcgaaaagctcagccgtgaacgcgcctgcgtaggctggcgtcgcgcagtgttgagccagttagtgagcgagtggggttgggacgaagctcgtctggcaatgctcgataaccgcgctaactggaagattgatcaggtgcgtgaggcgcacaacgagttgctcgacgcgatgatgcagagctaccgtaatctgatccgctttgcgcgtcgcaataaccttagcgtctccgccagtccgcaggatatcggcgtgctgacgcgtaagctgtatgccgcgtttgaagcattaccaggtaaagtgacgctggtaaacccgcagatttcacccgatctctcggaaccgaatctgacctttatttatgtgccgccgggccgggctaaccgttcaggttggtatctgtataaccgcgcgccaaatattgagtcgatcatcagccatcagccgctggaatataaccgttacctgaataaactggtggcgtgggcatggtttaacggcctgctgacctcgcgcacccgtttgtatattaaaggtaacggcattgtcgatttgcctaagttgcaggagatggtcgccgacgtgtcgcaccatttcccgctgcgcttacctgcaccgacaccgaaggcgctctacagcccgtgtgagatccgccatctggcgattatcgttaacctggaatatgacccgacagcggcgttccgcaatcaggtggtgcatttcgatttccgtaagctggatgtcttcagctttggcgagaatcaaaattgcctggtaggtagcgttgacctgctgtaccgcaactcgtggaacgaagtgcgtacgctgcacttcaacggcgagcaatcgatgatcgaagccctgaaaactattctcggcaaaatgcatcaggacgccgcaccgccagatagcgtggaagtcttctgttatagccagcatctgcgcggcttaattcgtactcgcgtgcagcaactggtttctgagtgtattgaattgcgtctttccagcacccgccaggaaaccgggcgtttcaaggcgctgcgcgtttctggtcaaacctgggggttgttcttcgaacgcctgaatgtatcggtacagaaactggaaaacgccatcgagttttatggcgcgatttcgcataacaaactgcacggcctgtcagtgcaggttgaaaccaatcacgtcaaattaccggcggtggtggacggctttgccagcgaagggatcatccagttctttttcgaagaaacgcaagacgagaatggctttaatatctacattctcgacgaaagcaaccgggttgaggtatatcaccactgcgaaggcagcaaagaggagctggtacgtgacgtcagtcgcttctactcgtcatcgcatgaccgttttacctacggctcaagcttcatcaacttcaacctgccgcagttctatcagattgtgaaggttgatggtcgtgaacaggtgattccgttccgcacaaaatctatcggtaacatgccgcctgccaatcaggatcacgatacgccgctattacagcaatatttttcgtgatgaacgtgccggaaagcgaggcttatccggcatgcaatcttagcggaaactgactgtttcacccgcctgctgcgtcgccgcctgttccagcaaatcccagaaggtttcgccgctgcgatcacaaatccactcatcgcctttcaggtcaaaatggtagccgccctgtttggttgccagccatacctggtgcagcggctcctggcggttgataatgattttgctgccattctcaaaggtaatggtcagtacgccgccgttgatttcgcagtcgatatcgctgtcgccatcccagtcgtccaggcgttcttcaatggtcagccagagttgatcagccaggcgatgaaattcactgtcgttcattgttgtatcctgtttttaagtgatggcggcagtatagcggcatggggtcagggcttcaaagtttgcacctctgcggctgcgttccggcacgattcatccgtcaccggaataatgatgtctctgtgtagcgaaagatttgtctcttcattagggcgcagttacaccacgtctttccctgtttctggtaaacattatgatcaggtttaccgagcgagcatcctcacgctgacggaactaaaaaagacaacaaacaaaccacattgcgatagtgcataaagccatcctggcgcgaggtgccgatcacgaaactaccagcaaaacataaatccccacgagtaagcgttatactcgcagcatttcctcacttttcagacttcataaagagtcgctaaacgcttgcttttacgtcttctcctgcgatgatagaaagcagaaagcgatgaactttacaggcaatccataatgaaaaacgtgtttaaggcactcactgtattacttactctcttcagcctgacgggctgcggtctgaaaggtccgctctatttcccgcctgcagataaaaacgcaccgccgccgaccaaaccggtagagacgcaaacgcaatccacggtgccggataaaaacgatcgcgccactggcgatggtccatcccaggtgaattactaaaagtcagtttctgtacccgcgtgattggagtaaatgatgcagttctcgaaaatgcatggccttggcaacgattttatggtcgtcgacgcggtaacgcagaatgtctttttttcaccggagctgattcgtcgcctggctgatcggcacctgggggtagggtttgaccaactgctggtggttgagccgccgtatgatcctgaactggattttcactatcgcattttcaatgctgatggcagtgaagtggcgcagtgcggcaacggtgcgcgctgctttgcccgttttgtgcgtctgaaaggactgaccaataagcgtgatatccgcgtcagcaccgccaacgggcggatggttctgaccgtcaccgatgatgatctggtccgcgtaaatatgggcgaacccaacttcgaaccttccgccgtgccgtttcgcgctaacaaagcggaaaagacctatattatgcgcgccgccgagcagacaatcttatgcggcgtggtgtcgatgggaaatccgcattgcgtgattcaggtcgatgatgtcgataccgcggcggtagaaacgcttggtcctgttctggaaagccacgagcgttttccggagcgcgccaatatcggttttatgcaagtggttaagcgcgagcatattcgtttacgcgtttatgagcgtggggcaggagaaacccaggcctgcggcagcggcgcgtgtgcggcggttgcagtagggattcagcaaggtttgctggccgaagaagtacgcgtggaactccccggcggtcgtcttgatatcgcctggaaaggtccgggtcacccgttatatatgactggcccggcggtacatgtctacgacggatttattcatctatgaagcaaccaggggaagaactgcaggaaacactcacggagcttgatgaccgggcggttgtcgattatctgattaaaaatcctgagttttttatccgtaatgcgcgcgcagtagaagcgatacgtgtgccgcatccggtacgcggcaccgtttcgttggtcgagtggcacatggcccgcgcacgtaatcatattcatgttctggaagagaacatggcgctgttgatggaacaggctatcgccaacgaaggcctgttttatcgcctactctacctgcagcgcagtctcaccgccgccagcagtctcgacgatatgctgatgcgctttcaccgctgggcgcgcgatctcggcctggcaggtgcgagtctgcgcctgtttccggatcgctggcgcttaggtgcgccgtcgaaccacactcatctggcattaagccgtcagtctttcgaaccgctgcgtattcagcgtttggggcaggaacagcactatcttgggccgcttaacggaccagagctgctggtggtgctaccggaagcgaaagcggtgggatcggtggcgatgtcgatgctgggaagcgatgctgatttgggtgtcgtgctgtttaccagtcgcgatgccagtcactatcaacaagggcaaggaacgcagttacttcatgaaattgcgctgatgttgccggagcttctggagcgttggattgaacgcgtatgaccgatttacacaccgatgtagaacgctacctacgttatctgagcgtggagcgccagcttagcccgataaccctgcttaactaccagcgtcagcttgaggcgatcatcaattttgccagcgaaaacggcctgcaaagctggcagcaatgtgatgtgacgatggtgcgcaattttgctgtacgcagtcgccgtaaagggctgggagcagcaagtctggcgttacggctttctgcgctacgtagcttttttgactggctggtcagccagaacgaactcaaagctaacccggcgaaaggtgtttcggcaccgaaagcgccgcgtcatctgccgaaaaacatcgacgtcgacgatatgaatcggctgctggatattgatatcaatgatcccctcgctgtacgcgaccgtgcaatgctggaagtgatgtacggcgcgggtctgcgtctttctgagctggtggggctggatattaaacacctcgacctggagtctggtgaagtgtgggttatggggaaaggcagcaaagagcgccgcctgccgattggtcgcaacgctgtggcgtggattgagcactggcttgatttgcgcgacctgtttggtagcgaagacgacgcgctttttctgtcgaaactgggcaagcgtatctccgcgcgtaatgtgcagaaacgctttgccgaatggggcataaaacaagggctgaataatcacgttcatccgcataaattacgtcactcgttcgccacgcatatgctggagtcgagcggcgatcttcgtggtgtgcaggagctgctgggtcatgccaacctctccaccacgcaaatctatactcatcttgattttcaacaccttgcctcggtgtacgatgcggcgcatccacgcgccaaacgggggaaataatgcgtttttaccggcctttggggcgcatctcggcgctcacctttgacctggatgataccctttacgataaccgtccggtgattttgcgcaccgagcgagaggcgcttacctttgtgcaaaattatcatccggcgctgcgcagcttccagaatgaagatctgcaacgcctgcgccaggcggtacgggaagcggaacccgagatttatcacgacgtgacgcgctggcgttttcgttcgattgaacaagcgatgctcgacgccgggctgagtgccgaagaagccagtgcaggcgcacacgcagcaatgatcaactttgccaaatggcgcagccgaatcgacgtcccgcagcaaactcacgacaccttaaaacagctggcgaagaaatggccgctggtggcgatcaccaacggtaacgcccagccggagctgtttggtttgggggattattttgagtttgtgctgcgcgctggcccgcacgggcgctcaaaaccgttcagcgatatgtactttttggctgcggaaaaactcaacgtgccgatcggcgagatcttacatgttggggacgatctcaccactgacgtgggtggggcaattcgcagcggaatgcaggcttgttggatcagaccggaaaatggcgatctgatgcaaacctgggacagccgtttactgccgcatctggaaatttcccggttggcatctctgacctcgctgatataatcagcaaatctgtatatatacccagctttttggcggagggcgttgcgcttctccgcccaacctatttttacgcggcggtgccaatggacgtttcttacctgctcgacagccttaatgacaaacagcgcgaagcggtggccgcgccacgcagcaaccttctggtgctggcgggcgcgggcagtggtaagacgcgcgtactggtgcatcgtatcgcctggttgatgagcgtggaaaactgctcgccatactcgattatggcggtgacgtttaccaacaaagcggcggcggagatgcgtcatcgtatcgggcaactgatgggcacgagccagggcggtatgtgggtcggcaccttccacgggctggcgcaccgtttgctgcgtgcgcaccatatggacgccaatctgccgcaggatttccagatcctcgacagtgaagaccagctacgcctgcttaagcgtctgatcaaagccatgaacctcgacgagaagcagtggccgccgcggcaggcaatgtggtacatcaacagccagaaagatgaaggcctgcgtccgcatcatattcaaagctacggtaatccggtggagcagacctggcagaaggtgtatcaggcgtatcaggaagcgtgtgaccgcgcgggcctggtggacttcgccgagctgctgctgcgcgctcacgagttgtggcttaacaagccgcatatcctgcaacactaccgcgaacgttttaccaatatcctggtggacgaattccaggataccaacaacattcagtacgcgtggatccgcctgctggcgggcgacaccggcaaagtgatgatcgtcggtgatgacgaccagtcaatctacggctggcgcggggcgcaggtggagaatattcagcgtttccttaatgatttccccggtgccgaaactattcgtctggagcaaaactaccgctctaccagcaatattctgagcgccgctaacgccctgattgaaaacaataacgggcgtctgggtaaaaaactgtggaccgatggcgcggacggtgagcctatttccctctattgcgcttttaacgaactcgatgaagcgcgttttgtggttaaccgcatcaaaacctggcaggacaacggcggagcgcttgccgagtgcgccattctctaccgcagcaacgcccagtcgcgggtgctcgaagaggcgttattgcaggccagtatgccgtaccgtatttacggcgggatgcgcttcttcgaacgccaggaaatcaaagatgcgctctcgtatctgcgcctgattgccaaccgcaacgacgacgcggcctttgagcgtgtggtgaatacgccaacgcggggtattggtgaccggacgctggacgtggtacgtcagacatcgcgcgatcgccagttaacactctggcaggcatgtcgtgagctgttgcaggaaaaagccctcgccgggcgagctgccagcgccttgcagcgatttatggaattaatcgacgccttagcgcaggaaactgccgatatgccgctgcatgtacagactgaccgggtaattaaagactccggcctgcgtaccatgtatgagcaggagaagggcgaaaaaggtcagacgcgtatcgaaaacttagaggaactggtgacggcaacgcgccagttcagctacaacgaagaagacgaagatttaatgccgctgcaggcgttcctctcccatgcggcactggaagcaggtgaagggcaggcggatacctggcaggatgcggtgcagttgatgacgctacactcggcgaaaggcctggagttcccgcaggtgtttatcgttggtatggaagagggcatgttcccaagccagatgtcgctggatgaaggcgggcgtctggaagaagaacgccgtctggcctacgttggcgtaacccgcgcgatgcagaaactgacgctgacctacgcggaaacccgccgtctgtatggtaaagaggtttaccatcgcccgtcgcgctttatcggcgagctgccggaagagtgtgtggaagaggtgcgcctgcgcgccacggtaagccgcccggtcagccatcagcggatgggtacgccgatggtcgagaacgacagcggctacaagctcggccagcgcgtacgccacgctaagtttggtgaaggcaccattgtcaatatggaaggcagcggtgagcatagccgtttgcaggtggcatttcagggccagggtattaaatggctggtggcggcatacgcccggctggagtcggtgtaacgttgccggatgcggtgctgcgcaccttatttggcctaaaaaatcattcagattcaataaattgcaacgtcatgtaggccggatagggcgtttacgccgcatccggcatctgcgccatcttcagtatctgacacaaaactatcgttttaacctttccgctcgacggaaatcatggtgacaaaaggatagcgttgccacgggattgccccgcctttcatatacatatgtgaaatcgtgccatcaagataaagcagctgctcaacgttcagtttcgctttggcataacaggcaaaatcataaaaatttgttgcctgctggctcaacaaaaacacggcgttcccatgtttattaatcccaacaccgttacgaattttgcttgaggcgacgttgggatgaatacgcggattaattacaccgttttccatcaacattggccctgactgcaccgcaaactgaatctctttactggttttgaaggcatccagacgaacgatgccgactttatctcccgcgacataaaacacgccgccaggacggataaagaaattcccttcacctgaagcgagatttaacgccaccttctgctgaccgttttcgatgtacaaaccgagcggcgcatagctttcatcatagatgccgccgttcatcgccatctgcacctgaccctgactattaatatccgccagcagagcatgtaacgttccccacgcttcgccattggctttttgccagtacattttcacccgctctgtttgaggattaacggtatacgcctgtacggtcagcgtcggatctgagagtgcgcaatcatcagcggcaacagcaaacaagggaagtaaggtgagggcgagaaaaatccgtttgagattcaaggtgatcattcctttaccaatgagtagctgatgcgccattataggtcctggatgtgggatttttttatcctgttagcgaccttgacgagtaccaaaaagcgcgaagttcaactattgttctgtggtgttctgttgcgtgttgacggcaaaattttgctggcgtaacatgcgcgcacgatcactctaagaggacattcgccttggacacacccagtagatactggctcactatcctgtcatccaggatcaactcctaaggctatccctttttgctgatagccttagcggttgtcagcgacctcaatttttcccgtcgcgctgagtcaggctgtttaatggtctgaaacccaatttgtttctgtgtgcccaccgaactgtccgatattttaagcattgggagtcccggtcatgctgagcgcatttcaactggaaaataaccgactgacccggctggaagtcgaagagtcacaaccccttgtaaatgcagtatggattgatcttgtcgaaccggacgacgacgagcgactgcgcgtacaatctgaacttggccagagcctggcaacccgcccggaactggaagacatcgaagcatcggcacgtttctttgaagacgacgacggcctgcatattcactccttcttcttctttgaagatgcggaagatcacgccggtaactccactgtggcatttaccatccgtgatggtcgtctgtttactctgcgtgagcgtgaactgcccgcttttcgtctgtatcgtatgcgtgcccgtagccagtcgatggtagacggtaacgcctacgagttgctgctggatctgttcgaaaccaaaatcgaacagttggcagatgaaattgaaaatatctatagcgacctggagcagttgagccgggtgattatggaagggcatcagggcgatgagtacgacgaggcgctctccactctggcggaactggaagatatcggctggaaagttcgcctgtgtctgatggatacccagcgcgcgctcaacttcctggtgcgtaaagcgcgtttaccgggtgggcaactggagcaggcgcgtgaaatcctgcgagatatcgaatccctgctgccgcataacgaatccctgttccagaaggtgaacttcctgatgcaggcggcaatgggttttatcaacatcgagcagaaccgcatcatcaaaatcttctcggtggtatccgtggtattcctgccgccgacgctcgttgcttccagctatggcatgaactttgagtttatgccagaactgaagtggagcttcggctaccctggcgcgattatctttatgatcctcgcgggcctggcaccgtatctgtactttaagcggaagaactggttgtaaaaaacgagagcggtggcttagtctggctaagccacctgttattcaaaggctccaggtatttaacccttttacctctttctcatagaaccatttgttcgtgttaacagcaacataggctgctacggcaattcccagaatgttaacgccaattagtgcaccaacaaatagagatagaataccaagtaatagaactataattgcttttttccataaccccaggacaaataaatatatccaggaacagaagaaagcaatgaaattcatttgaatagttaagcgttgtcttacttttaatgctttaaatgctgctttatattctggtgttgccccccagaatccaggaaaaccatgttgatcataaaaattaaatcggtatttccatttttcacttaatgaaccatcgttcatatattccttactcataaatactccataactattgttttgatgaatcagtaggtgcaagcattagcatactgaaagtggaaaaataacaaatcaaaaaaatcatcgaaccattgcctgaacaggcaaaatcttcggctatcattgtgatgatagagatgatatatactgctaatgtaccaaaaacataagtttttatatagatgaaaccactatcacggagtcgctggcaattcatgttgatgacgagataatggagtacgatggtagagactataacaagaaagcctgcttctccatcgttaaaaaagataataagaaaggcaaaaatgaaatttattaaaataaatgaaaatatataacgacgtctggaaatcttaccgttagatgttgggataaatatacgtaacataaattttacatccttgtatgagtctccggtcagcatggcaatatgcccactctcatgcaagagtcggcatattttttcagaatatatttattttttatttggacgttctacgctgcgtataaatcgcatccatcacaaaaattgccagcgccacccaaataaaggcgaaagtcaccatcttatcggcacccggtttttcaccataaaacgtcacagccagcaggaacatcagcgtcgggccaatgtactggaaaaagcctaacgttgagagacgcaagcgcgtggcagcggcggtaaaacacaacagcggtacggtagtgacaataccggcggcgatcagcagtaaattcagcgacatcgggttttgccccatatggctggttgagctgtcggcaatagcaaacaggtaaattgccgccacgggcagcagccacatggtttcgattaacatgccggtttgcgcttcaacggcaatcttcttgcgtaccagaccgtagaaggcaaaactaaatgccagtcccagcgcgataataggtagcgaaccaaaagtccacagctggactaacacgccacatatcgccagaatcaccgccagccattgcatccggcggaatcgctcgccgaggaaaatcatccccagcacaatgttcaccagcgggttaataaagtaaccaaggctcgcttccagcatatggtgattgttcaccgcccagataaacagtagccagttgccaccaatcagcacggcagagactgccagcataaaaattttctgtggcgtctgaatcagcgtttttaaataggaccactggcggcaaatgctcatcagcaccaccataaagaaaaacgaccagatcacgcgatgcgtcaggatttcatcggcgggcacgtagtaaatcaacttgaagtacgctggcgctataccccaaataaaataagcggcaagagcgagtaatacgccctgccgcgtttgttttgcatccatcgggaatactcatttttaattggtaacagcagtttacctgcttttatgtcttcaacctaccatataggtggcggtggcactggcaatataaagctgttcttcattgtgtaattcaacgcgggcgacggcgactttattgcctgcacgcaacaggctactagtagcagtaaaacgctcgcccctgcctgggcgcagataatcaacgcgaagatcaatggtccccatccgcgatagccgctggcgtagttcatcttcactgatggtttcgtggcgggttaaggtacttcccacgcacaccagaccggcggcgacatccagcgccgacgcaatgaccccgccgtgcaaaatgctttgcgcccagttgcccaccatcattggctgatttttaaaggccagctgtgcgaactctttttcgtaacgctccagttccatccccaatgcgcggttaaatggcatgtgataaacaaacatctcacccactaatttcagggcttgttcagcggtcagtacggcagacatatcatccttacacttcattggttaatgaaatgttgattttatgcttctttgttgttggtttctactttaggaagggataactaacggctatggagttaagtatgtaaaatagcccgcagaaaaatattcaccttatcaataattcgttacggagaacacgaccgatgcggactctgcagggctggttgttgccggtgtttatgttgcctatggcagtatatgcacaagaggcaacggtgaaagaggtgcatgacgcgccagcggtgcgtggcagtattatcgccaatatgctgcaggagcatgacaatccgttcacgctctatccttatgacaccaactacctcatttacacccaaaccagcgatctgaataaagaagcgattgccagttacgactgggcggaaaatgcgcgtaaggatgaagtaaagtttcagttgagcctggcatttccgctgtggcgtgggattttaggcccgaactcggtgttgggtgcgtcttatacgcaaaaatcctggtggcaactgtccaatagcgaagagtcttcaccgtttcgtgaaaccaactacgaaccgcaattgttcctcggttttgccaccgattaccgttttgcaggttggacgctgcgcgatgtggagatggggtataaccacgactctaacgggcgttccgacccgacctcccgcagctggaaccgcctttatactcgcctgatggcagaaaacggtaactggctggtagaagtgaagccgtggtatgtggtgggtaatactgacgataacccggatatcaccaaatatatgggttactaccagcttaaaatcggctatcacctcggtgatgcggtgctcagtgcgaaaggacagtacaactggaacaccggctacggcggcgcggagttaggcttaagttacccgatcaccaaacatgtgcgcctttatactcaggtttacagcggctatggcgaatcgctcatcgactataacttcaaccagacccgtgtcggtgtgggggttatgctaaacgatttgttttgatgaacggttgagtggttggcaaatctggaatccagcatccaggattaccctctcagagactaaaagcattgcagtttctcgcgcaggcgctgaaaatagcgcctgtttttatttcaggcaatcggggtgaatgtggcgcaggcggaagtgttgaatctggagtccggagctaaacaggttttacaagaaacctttggctaccaacagtttcgccccggccaggaagaaattatcgacactgtgctttccggccgcgattgcctcgtcgtcatgcccactggtggcggaaaatccctttgctatcaaatccctgccttattgctaaacggccttaccgtggttgtttcaccgctgatttcgttgatgaaagatcaggtggatcaactgcaagccaacggcgtggcggcggcgtgccttaactcgacgcaaacccgcgaacagcaacttgaagtgatgacaggctgccgcaccgggcaaattcgtctgctttatatcgccccggaacgcctgatgctggataactttcttgagcatctggcgcactggaatccggtgttattagccgttgatgaagcgcactgtatctcccaatggggccacgatttccgcccggaatatgccgcgctcggtcagttgcgccagcggttcccgacgctgccgtttatggcgctgaccgccacagccgacgacaccacgcgccaggatatcgtgcgcctgctggggctgaacgatccgctgattcaaatcagcagttttgaccgtccgaatattcgctacatgctgatggagaagttcaaaccgctcgatcagttgatgcgctacgtgcaggaacagcgcggtaagtcaggcattatctactgcaacagccgcgcgaaagtagaagacaccgctgcgcgcctgcaaagcaagggaattagcgcggcggcctatcatgccgggctggaaaataatgttcgcgccgatgtgcaggaaaaattccagcgcgatgacctgcaaattgtggtggcgacggtggcgttcggcatgggcatcaataaaccaaacgttcgcttcgtggtccactttgatattccgcgcaatatcgaatcctattatcaggaaaccggacgcgccgggcgtgatggcctgcccgcggaagcgatgctgttttacgatccggctgatatggcgtggctgcgccgttgtctggaagagaagccgcaggggcagttgcaggatatcgagcgccacaaactcaatgcgatgggcgcgtttgccgaagcgcaaacttgccgtcgtctggtattgctgaactattttggcgaagggcgtcaggagccgtgcgggaactgcgatatctgcctcgatccgccgaaacagtacgacggttcaaccgatgctcagattgccctttccaccattggtcgtgtgaatcagcggtttgggatgggttatgtggtggaagtgattcgtggtgctaataaccagcgtatccgcgactatggtcatgacaaactgaaagtctatggcatgggccgtgataaaagccatgaacattgggtgagcgtgatccgccagctgattcacctcggcctggtgacgcaaaatattgcccagcattctgccctacaactgacagaggccgcgcgcccggtgctgcgcggcgaatcctctttgcaacttgccgtgccgcgtatcgtggcgctcaaaccgaaagcgatgcagaaatcgttcggcggcaactatgatcgcaaactgttcgccaaattacgcaaactgcgtaaatcgatagccgatgaaagtaatgtcccgccgtacgtggtgtttaacgacgcaaccttgattgagatggctgaacagatgccgatcaccgccagcgaaatgctcagcgttaacggcgttgggatgcgcaagctggaacgctttggcaaaccgtttatggcgctgattcgtgcgcatgttgatggcgatgacgaagagtagtcagcagcataaaaaagtgccagtatgaagactccgtaaacgtttcccccgcgagtcaaatgtatgttgatgttatttctcaccgtcgccatggtgcacattgtggcgcttatgagccccggtcccgatttcttttttgtctctcagaccgctgtcagtcgttcccgtaaagaagcgatgatgggcgtgctgggcattacctgcggcgtaatggtttgggctgggattgcgctgcttggcctgcatttgattatcgaaaaaatggcctggctgcatacgctgattatggtgggcggtggcctgtatctctgctggatgggttaccagatgctacgtggtgcactgaaaaaagaggcggtttctgcacctgcgccacaggtcgagctggcgaaaagtgggcgcagtttcctgaaaggtttactgaccaatctcgctaatccgaaagcgattatctactttggctcggtgttctcattgtttgtcggtgataacgttggcactaccgcgcgctggggcatttttgcgctgatcattgtcgaaacgctggcgtggtttaccgtcgttgccagcctgtttgccctgccgcaaatgcgccgtggttatcaacgtctggcgaagtggattgatggttttgccggggcgttatttgccggatttggcattcatttgattatttcgcggtgatgccagacgcgtcttcagagtaagtcggataaggcgtttacgccgcatccgacattatttttcacgcatgcctcgccgatgctaacagcgctcccaccagcataaacaacgagccgaaaatcttattcagcgccttcatctgctttggtcctttaatccatagagcaatccgttgagcaagggtggcgtaaccgatcatcacaataatatcgaccacaatagtggtgacgccgagcacgatatactgcatcagttgcggctgttgcggcatgatgaattgcggaaatagcgccgccagaaacacaatacttttgggattggtgagattcacaaaaactgcgcgctggaacaaatgtcgacgcgattgagtagaggccagcgatttaaggtcaattgcaccagcggcgcgccactgctggattcccagccaaatcaagtaagccgcgcctgcccacttcaacacttcaaacgcaatcactgagcgggaaaatagcgtccccaaccccacgccaaccagcacaatatgaatcgccagtccggtctgaagcccagcaatagacgccaccgcgccgcgataaccgtggttgagcgaggtggtcatagtgttgattgcaccagagcctggcgacaggcttaaaatgatcgatgtcagcaggtaggcaaaccaccattctaaggtcatgatgaactcccggtgtgtctatttttgtgccacaatacgctactgtcgcagcgttgtgtcaggcacgctaaaaaaaacgattttacgtggtttaagaggcagattacccgatgtttcagcagcaaaaagactgggaaacaagagaaaacgcgtttgctgcttttaccatgggaccgctgactgatttctggcgtcagcgtgatgaagcagagtttactggtgtggatgacattccggtgcgctttgtccgttttcgcgcacagcaccatgaccgggtggtagtcatctgcccggggcgtattgagagctacgtaaaatatgcggaactggcctatgacctgttccatttggggtttgatgtcttaatcatcgaccatcgcgggcagggacgttccggtcgcctgttagccgatccgcatctcgggcatgttaatcgctttaatgattatgttgatgatctggcggcattctggcagcaggaggttcagcccggtccgtggcgtaaacgctatatactggcacattcgatgggcggtgcgatctccacattatttctgcaacgccatccaggtgtatgtgacgccattgcgctaactgcgccaatgtttgggatcgtgattcgtatgccgtcatttatggcacggcagatcctcaactgggccgaagcgcatccacgtttccgtgatggctatgcaataggcaccgggcgctggcgcgcgttgccgtttgctatcaacgtactgacccacagcagacagcgatatcgacgtaacttacgcttctatgctgatgacccaacgattcgcgtcggtgggccgacctaccattgggtacgcgaaagtattctggctggcgaacaggtgttagccggtgcgggtgatgacgccacgccaacgcttctcttgcaggctgaagaggaacgcgtggtggataaccgcatgcatgaccgtttttgtgaactccgcaccgccgcgggccatcctgtcgaaggaggacggccgttggtaattaaaggtgcttaccatgagatcctttttgaaaaggacgcaatgcgctcagtcgcgctccacgccatcgttgattttttcaacaggcataactcacccagcggaaaccgctctacagaggtttaaatttcttatgtaccaggttgttgcgtctgatttagatggcacgttactttctcccgaccatacgttatccccttacgccaaagaaactctgaagctgctcaccgcgcgcggcatcaactttgtgtttgcgaccggtcgtcaccacgttgatgtggggcaaattcgcgataatctggagattaagtcttacatgattacctccaatggtgcgcgcgttcacgatctggatggtaatctgatttttgctcataacctggatcgcgacattgccagcgatctgtttggcgtagtcaacgacaatccggacatcattactaacgtttatcgcgacgacgaatggtttatgaatcgccatcgcccggaagagatgcgcttttttaaagaagcggtgttccaatatgcgctgtatgagcctggattactggagccggaaggcgtcagcaaagtgttcttcacctgcgattcccatgaacaactgctgccgctggagcaggcgattaacgctcgttggggcgatcgcgtcaacgtcagtttctctaccttaacctgtctggaagtgatggcgggcggcgtttcaaaaggccatgcgctggaagcggtggcgaagaaactgggctacagcctgaaggattgtattgcgtttggtgacgggatgaacgacgccgaaatgctgtcgatggcggggaaaggctgcattatgggcagtgcgcaccagcgtctgaaagaccttcatcccgagctggaagtgattggtactaatgccgacgacgcggtgccgcattatctgcgtaaactctatttatcgtaatcgttctttatttggtcagttgtcaacctgatacttcgctacaatggatacccgttaatcaaagagttttccattgtggcgctacttatcatcaccacgattctgtgggccttctcctttagcttttatggcgagtaccttgcggggcacgtcgatagctattttgcggtgctggtgcgcgttggcctggcggcactcgtttttctgccgtttctgcgtacccgtggcaatagcctgaaaacggtcggcctgtatatgctggtgggcgcgatgcagcttggcgtgatgtatatgctgagtttccgcgcttatctctacctgacggtttccgagctgctgctgttcaccgtgctgacgccgctctacatcacgctgatttatgacatcatgagtaagcgccgtctgcgctggggctatgcctttagcgccttgctggcggtgattggtgccgggattattcgctatgatcaggtcaccgaccatttctggactggcttgctgctggtgcaactctccaatatcacttttgccattggcatggtgggttacaaacgcctgatggaaactcgcccgatgccacagcataacgcctttgcgtggttctatcttggcgcgtttctggtggcagtgattgcatggttcttgctgggaaatgcgcagaaaatgccgcaaaccacgctgcaatggggcattctggtgtttcttggcgtggtggcttccgggattggctactttatgtggaactacggcgcgacgcaggtggacgccggaacgctgggcattatgaataatatgcacgttccggcagggctgctggtaaacctggctatctggcaccaacagccgcactggccaacgtttattacaggcgcgctggtgatcctggcctcactgtgggtgcatcgtaagtgggtcgctccgcgctcttcacaaacggcagatgatcgcaggcgtgattgcgcgctgagcgaataaacgcttccgtaactggctgacgctgctcgccatcgcgcacggcggcgtacagtcggctccacaagccttcgcccagggttttggtcaccaccagaccctggcgctcaaaactctctactacccaatgcggtagcgcggcaatacccatccgcgcggcaaccatctgaatcaacaataaggtgttatcgacgcttttcagtgacgggctgacgcctgccggctgaagaaaatgccgccagacatccagtcgactacgctgcaccggataaattaatagcgtctcgctggcgagatcttccggtgtaattcgcgttttcgccgccagtggatggtcaggtgctaacaccagacgcacttcatagtcgaacatcggcgaataatgcaggccactgcgcggcagaatatcggacgtcattaccagatccagctctccctgttgcaaggcgggctgcgggtcaaatgtcacgcccgatttaaaatccatctctacctgcggccagttcttatggaaattttctaacgcgggtgtcagccactgaatacagctatggcactcaatggcaatgcgcagacgcgtctgctgcggttcattgcaggcttgcagggcctggctaatttgcggcagtacctggtttgccagttgcaacaggatttctccctgcggtgtaaagcgtagcggctggctcttacgcacaaatagccggaagccaaggcgttgttccagatcgctaaactggtgagacagggcggattgcgtctgatgcaacgtcgccgcagcggctgcgagcgagccgcagttccgcaacgcttgtagcgttttcaggtgttttacttcgatcatgaaagtccttcacttcggcatgaataatttgcgcttgaggaatatacagtaaccgccaattatggatgtgtaaacatctggacggctaaaatccttcgtcttttaaatttatggtgcgttggctgcgtttctccaccccggtcacttacttcagtaagctcccggggatgaataaacttgccgccttccctaaattcaaaatccataggatttacatataattagaggaagaaaaaatgacaatattgaatcacaccctcggtttccctcgcgttggcctgcgtcgcgagctgaaaaaagcgcaagaaagttattgggcggggaactccacgcgtgaagaactgctggcggtagggcgtgaattgcgtgctcgtcactgggatcaacaaaagcaagcgggtatcgacctgctgccggtgggcgattttgcctggtacgatcatgtactgaccaccagtctgctgctgggtaacgttccggcgcgtcatcagaacaaagatggttcggtagatatcgacaccctgttccgtattggtcgtggacgtgcgccgactggcgaacctgcggcggcagcggaaatgaccaaatggtttaacaccaactatcactacatggtgccggagttcgttaaaggccaacagttcaaactgacctggacgcagctgctggacgaagtggacgaggcgctggcgctgggccacaaggtgaaacctgtgctgctggggccggttacctggctgtggctggggaaagtgaaaggtgaacaatttgaccgcctgagcctgctgaacgacattctgccggtttatcagcaagtgctggcagaactggcgaaacgcggcatcgagtgggtacagattgatgaacccgcgctggtactggaactaccacaggcgtggctggacgcatacaaacccgcttacgacgcgctccagggacaggtgaaactgctgctgaccacctattttgaaggcgtaacgccaaatctcgacacgattactgcgctgcctgttcagggtctgcatgttgacctcgtacatggtaaagatgacgttgctgaactgcacaagcgcctgccttctgactggttgctgtctgcgggtctgatcaatggtcgtaacgtctggcgcgccgatcttaccgagaaatatgcgcaaattaaggacattgtcggcaaacgtgatttgtgggtggcatcttcctgctcgttgctgcacagccccatcgacctgagcgtggaaacgcgtcttgatgcagaagtgaaaagctggtttgccttcgccctacaaaaatgccatgaactggcactgctgcgcgatgcgctgaacagtggtgacacggcagctctggcagagtggagcgccccgattcaggcacgtcgtcactctacccgcgtacataatccggcggtagaaaagcgtctggcggcgatcaccgcccaggacagccagcgtgcgaatgtctatgaagtgcgtgctgaagcccagcgtgcgcgttttaaactgccagcgtggccgaccaccacgattggttccttcccgcaaaccacggaaattcgtaccctgcgtctggatttcaaaaagggcaatctcgacgccaacaactaccgcacgggcattgcggaacatatcaagcaggccattgttgagcaggaacgtttgggactggatgtgctggtacatggcgaggccgagcgtaatgacatggtggaatactttggcgagcacctcgacggatttgtctttacgcaaaacggttgggtacagagctacggttcccgctgcgtgaagccaccgattgtcattggtgacattagccgcccggcaccgattaccgtggagtgggcgaagtatgcgcaatcgctgaccgacaaaccggtgaaagggatgctgacggggccggtgaccatactctgctggtcgttcccgcgtgaagatgtcagccgtgaaaccatcgccaaacagattgcgctggcgctgcgtgatgaagtggccgatctggaagccgctggaattggcatcatccagattgacgaaccggcgctgcgcgaaggtttaccgctgcgtcgtagcgactgggatgcgtatctccagtggggcgtagaggccttccgtatcaacgccgccgtggcgaaagatgacacacaaatccacactcacatgtgttattgcgagttcaacgacatcatggattcgattgcggcgctggacgcagacgtcatcaccatcgaaacctcgcgttccgacatggagttgctggagtcgtttgaagagtttgattatccaaatgaaatcggtcctggcgtctatgacattcactcgccaaacgtaccgagcgtggaatggattgaagccttgctgaagaaagcggcaaaacgcattccggcagagcgcctgtgggtcaacccggactgtggcctgaaaacgcgcggctggccagaaacccgcgcggcactggcgaacatggtgcaggcggcgcagaacttgcgtcgggggtaaaatccaaaccgggtggtaataccacccggtcttttctcattacagcgacttcttcccaccatactgcttaaaccattccagcatacgctgccagccatcttctgcagatgcggcatgatagctcgggcgataatcagcgttgaatgcatgcccggcgtccgggtacacgataatctctgctttcgcattagcagcccgcagcgcctggcgcatggtttcaacgctctcctgcggaatgctgttatcctgaccaccatataagccgagaatcggcgcgttaagatcggttgcgatatcaacaggttgtttcggtgaattcagcgacttgtcgcccgtcagtttgccgtaccacgccactgcggcttttagctgtggattatgcgcggcatacagccaggtgatacgtccaccccagcagaatccggtgatcattaaacgatgaacatcgccgccgttgcgggaagcccaactggcgacatgatcgagatcggccagcacctgcgagtcaggcacttttgctaccagaccgctaagcaacgtggggatatcggcaaaatcattcggatcgccttcgcggaagtaaagttcaggtgcgatagccagatacccctccagcgccagacggcgacaaatgtcgcggatatgttcatgcacgccaaaaatttcctgcactacaatgaccactggcagtgggccatcgctttgctttggtctggcatggtaagcaggcatgttatccccttgtgaagggatagaggtgaagcccgccacaatcgcgtcgtccggggtctgaacgatggtcgaagcgagaggcgatgcagcaggtgcaaatccagattgttgtgttgttgccatggtattctccgtacccttataaaaatgttgcgcaatgttaactatagtcagcatgcaacaaatcacattgcctgaatcggctcatcttttatgcagtcctgcagaatgaagggtgatttatgtgatttgcatcacttttggtgggtaaatttatgcaacgcatttgcgtcatggtgatgagtatcacgaaaaaatgttaaacccttcggtaaagtgtctttttgcttcttctgactaaaccgattcacagaggagttgtatatgtccaagtctgatgtttttcatctcggcctcactaaaaacgatttacaaggggctacgcttgccatcgtccctggcgacccggatcgtgtggaaaagatcgccgcgctgatggataagccggttaagctggcatctcaccgcgaattcactacctggcgtgcagagctggatggtaaacctgttatcgtctgctctaccggtatcggcggcccgtctacctctattgctgttgaagagctggcacagctgggcattcgcaccttcctgcgtatcggtacaacgggcgctattcagccgcatattaatgtgggtgatgtcctggttaccacggcgtctgtccgtctggatggcgcgagcctgcacttcgcaccgctggaattcccggctgtcgctgatttcgaatgtacgactgcgctggttgaagctgcgaaatccattggcgcgacaactcacgttggcgtgacagcttcttctgataccttctacccaggtcaggaacgttacgatacttactctggtcgcgtagttcgtcactttaaaggttctatggaagagtggcaggcgatgggcgtaatgaactatgaaatggaatctgcaaccctgctgaccatgtgtgcaagtcagggcctgcgtgccggtatggtagcgggtgttatcgttaaccgcacccagcaagagatcccgaatgctgagacgatgaaacaaaccgaaagccatgcggtgaaaatcgtggtggaagcggcgcgtcgtctgctgtaattctcttctcctgtctgaaggccgacgcgttcggccttttgtatttttgcgtagcgcctcgcaggaaatgcctttccaactggacgtttgtacagcacaattctattttgtgcgggtaagttgttgcgtcaggaggcgttgtggatttctcaatcatggtttacgcagttattgcgttggtgggtgtggcaattggctggctgtttgccagttatcaacatgcgcagcaaaaagccgagcaattagctgaacgtgaagagatggtcgcggagttaagcgcggcaaaacaacaaattacccaaagcgagcactggcgtgcagagtgcgagttactcaataacgaagtgcgcagcctgcaaagtattaacacctctctggaggccgatctgcgtgaagtaaccacgcggatggaagccgcacagcaacatgctgacgataaaattcgccagatgattaacagcgagcagcgcctcagtgagcagtttgaaaacctcgccaaccgtatttttgagcacagcaatcgccgggttgatgagcaaaaccgtcagagtctgaacagcctgttgtcgccgctacgtgaacaactggacggtttccgccgtcaggttcaggacagcttcggtaaagaagcacaagaacgccataccctgacccacgaaattcgcaatctccagcaactcaacgcgcaaatggcccaggaagcgatcaacctgacgcgcgcgctgaaaggcgacaataaaacccagggcaactggggcgaggtagtattgacgcgggtgctggaggcttccggtctgcgtgaagggtatgaatatgaaacccaggtcagcatcgaaaatgacgcccgctcgcggatgcagccggatgtcatcgtgcgcctgccgcagggaaaagatgtggtgatcgacgccaaaatgacgctggtcgcctatgaacgctattttaacgccgaagacgactacacccgcgaaagcgcgctacaggaacatatcgcgtcggtgcgtaaccatatccgtttgctgggacgcaaagattatcaacagctgccggggctgcgaactctggattacgtgctgatgtttattcccgttgaacccgcttttttactggcgcttgaccgccagccggagctgatcaccgaagcgttgaaaaacaacatcatgctggttagcccgactacgctgctggtggcgctgcgcactatcgccaacctgtggcgttatgagcatcaaagccgcaacgcccagcaaatcgccgatcgtgccagcaagctgtacgacaagatgcgtttgttcatcgatgacatgtccgcgattggtcaaagtctcgacaaagcgcaggataattatcggcaggcaatgaaaaaactctcttcagggcgcggaaatgtgctggcgcaggcagaagcgtttcgcggtttaggagtagaaattaaacgcgagattaatccggatttggctgaacaggcggtgagccaggatgaagagtatcgacttcggtcggttccggagcagccgaatgatgaagcttatcaacgcgatgatgaatataatcagcagtcgcgctagcccattgggagtagttaagccgggtagaaatctagggcatcgacgcccaatctgttacacttctggaacaattttttgatgagcaggcattgagatggtggataagtcacaagaaacgacgcactttggttttcagaccgtcgcgaaggaacaaaaagcggatatggtcgcccacgttttccattccgtggcatcaaaatacgatgtcatgaatgatttgatgtcatttggtattcatcgtttgtggaagcgattcacgattgattgcagcggcgtacgccgtgggcagaccgtgctggatctggctggtggcaccggcgacctgacagcgaaattctcccgcctggtcggagaaactggcaaagtggtccttgctgatatcaatgaatccatgctcaaaatgggccgcgagaagctgcgtaatatcggtgtgattggcaacgttgagtatgttcaggcgaacgctgaggcgctgccgttcccggataacacctttgattgcatcaccatttcgtttggtctgcgtaacgtcaccgacaaagataaagcactgcgttcaatgtatcgcgtgctgaaacccggcggccgcctgctggtgcttgagttctcgaagccaattatcgagccgctgagcaaagcctatgatgcatactccttccatgtgctgccgcgtattggctcactggtcgcgaacgacgccgacagctaccgttatctggcagaatccatccgtatgcatcccgatcaggataccctgaaagccatgatgcaggatgccggattcgaaagtgtcgactactacaatctgacggcaggggttgtggcgctgcatcgtggttataagttctgacaggagaccggaaatgccttttaaacctttagtgacggcaggaattgaaagtctgctcaacaccttcctgtatcgctcacccgcgctgaaaacggcccgctcgcgtctgctgggtaaagtattgcgcgtggaggtaaaaggcttttcgacgtcattgattctggtgttcagcgaacgccaggttgatgtactgggcgaatgggcaggcgatgctgactgcaccgttatcgcctacgccagtgtgttgccgaaacttcgcgatcgccagcagcttaccgcactgattcgcagtggtgagctggaagtgcagggcgatattcaggtggtgcaaaacttcgttgcgctggcagatctggcagagttcgaccctgcggaactgctggccccttataccggtgatatcgccgctgaaggaatcagcaaagccatgcgcggaggcgcaaagttcctgcatcacggcattaagcgccagcaacgttatgtggcggaagccattactgaagagtggcgtatggcacccggtccgcttgaagtggcctggtttgcggaagagacggctgccgtcgagcgtgctgttgatgccctgaccaaacggctggaaaaactggaggctaaatgacgccaggtgaagtacggcgcctatatttcatcattcgcacttttttaagctacggacttgatgaactgatccccaaaatgcgtatcaccctgccgctacggctatggcgatactcattattctggatgccaaatcggcataaagacaaacttttaggtgagcgactacgactggccctgcaagaactggggccggtttggatcaagttcgggcaaatgttatcaacccgccgcgatctttttccaccgcatattgccgatcagctggcgttattgcaggacaaagttgctccgtttgatggcaagctggcgaagcagcagattgaagctgcaatgggcggcttgccggtagaagcgtggtttgacgattttgaaatcaagccgctggcttctgcttctatcgcccaggttcataccgcgcgattgaaatcgaatggtaaagaggtggtgattaaagtcatccgcccggatattttgccggttattaaagcggatctgaaacttatctaccgtctggctcgctgggtgccgcgtttgctgccggatggtcgccgtctgcgcccaaccgaagtggtgcgcgagtacgaaaagacattgattgatgaactgaatttgctgcgggaatctgccaacgccattcagcttcggcgcaattttgaagacagcccgatgctctacatcccggaagtttaccctgactattgtagtgaagggatgatggtgatggagcgcatttacggcattccggtgtctgatgttgcggcgctggagaaaaacggcactaacatgaaattgctggcggaacgcggcgtgcaggtgttcttcactcaggtctttcgcgacagctttttccatgccgatatgcaccctggcaacatcttcgtaagctatgaacacccggaaaacccgaaatatatcggcattgattgcgggattgttggctcgctaaacaaagaagataaacgctatctggcagaaaactttatcgccttctttaatcgcgactatcgcaaagtggcagagctacacgtcgattctggctgggtgccaccagataccaacgttgaagagttcgaatttgccattcgtacggtctgtgaacctatctttgagaaaccgctggccgaaatttcgtttggacatgtactgttaaatctgtttaatacggcgcgtcgcttcaatatggaagtgcagccgcaactggtgttactccagaaaaccctgctctacgtcgaaggggtaggacgccagctttatccgcaactcgatttatggaaaacggcgaagcctttcctggagtcgtggattaaagatcaggtcggtattcctgcgctggtgagagcatttaaagaaaaagcgccgttctgggtcgaaaaaatgccagaactgcctgaattggtttacgacagtttgcgccagggcaagtatttacagcacagtgttgataagattgcccgcgagcttcagtcaaatcatgtacgtcagggacaatcgcgttattttctcggaattggcgctacgttagtattaagtggcacattcttgttggtcagccgacctgaatgggggctgatgcccggctggttaatggcaggtggtctgatcgcctggtttgtcggttggcgcaaaacacgctgattttttcatcgctcaaggcgggccgtgtaacgtataatgcggctttgtttaatcatcatctaccacagaggaacatgtatgggtggtatcagtatttggcagttattgattattgccgtcatcgttgtactgctttttggcaccaaaaagctcggctccatcggttccgatcttggtgcgtcgatcaaaggctttaaaaaagcaatgagcgatgatgaaccaaagcaggataaaaccagtcaggatgctgattttactgcgaaaactatcgccgataagcaggcggatacgaatcaggaacaggctaaaacagaagacgcgaagcgccacgataaagagcaggtgtaatccgtgtttgatatcggttttagcgaactgctattggtgttcatcatcggcctcgtcgttctggggccgcaacgactgcctgtggcggtaaaaacggtagcgggctggattcgcgcgttgcgttcactggcgacaacggtgcagaacgaactgacccaggagttaaaactccaggagtttcaggacagtctgaaaaaggttgaaaaggcgagcctcactaacctgacgcccgaactgaaagcgtcgatggatgaactacgccaggccgcggagtcgatgaagcgttcctacgttgcaaacgatcctgaaaaggcgagcgatgaagcgcacaccatccataacccggtggtgaaagataatgaagctgcgcatgagggcgtaacgcctgccgctgcacaaacgcaggccagttcgccggaacagaagccagaaaccacgccagagccggtggtaaaacctgctgcggacgctgaaccgaaaaccgctgcaccttccccttcgtcgagtgataaaccgtaaacatgtctgtagaagatactcaaccgcttatcacgcatctgattgagctgcgtaagcgtctgctgaactgcattatcgcggtgatcgtgatattcctgtgtctggtctatttcgccaatgacatctatcacctggtatccgcgccattgatcaagcagttgccgcaaggttcaacgatgatcgccaccgacgtggcctcgccgttctttacgccgatcaagctgacctttatggtgtcgctgattctgtcagcgccggtgattctctatcaggtgtgggcatttatcgccccagcgctgtataagcatgaacgtcgcctggtggtgccgctgctggtttccagctctctgctgttttatatcggcatggcattcgcctactttgtggtctttccgctggcatttggcttccttgccaataccgcgccggaaggggtgcaggtatccaccgacatcgccagctatttaagcttcgttatggcgctgtttatggcgtttggtgtctcctttgaagtgccggtagcaattgtgctgctgtgctggatggggattacctcgccagaagacttacgcaaaaaacgcccgtatgtgctggttggtgcattcgttgtcgggatgttgctgacgccgccggatgtcttctcgcaaacgctgttggcgatcccgatgtactgtctgtttgaaatcggtgtcttcttctcacgcttttacgttggtaaagggcgaaatcgggaagaggaaaacgacgctgaagcagaaagcgaaaaaactgaagaataaattcaaccgcccgtcagggcggttgtcatatggagtacaggatgtttgatatcggcgttaatttgaccagttcgcaatttgcgaaagaccgtgatgatgttgtagcgtgcgcttttgacgcgggagttaatgggctactcatcaccggcactaacctgcgtgaaagccagcaggcgcaaaagctggcgcgtcagtattcgtcctgttggtcaacggcgggcgtacatcctcacgacagcagccagtggcaagctgcgactgaagaagcgattattgagctggccgcgcagccagaagtggtggcgattggtgaatgtggtctcgactttaaccgcaacttttcgacgccggaagagcaggaacgcgcttttgttgcccagctacgcattgccgcagatttaaacatgccggtatttatgcactgtcgcgatgcccacgagcggtttatgacattgctggagccgtggctggataaactgcctggtgcggttcttcattgctttaccggcacacgcgaagagatgcaggcgtgcgtggcgcatggaatttatatcggcattaccggttgggtttgcgatgaacgacgcggactggagctgcgggaacttttgccgttgattccggcggaaaaattactgatcgaaactgatgcgccgtatctgctccctcgcgatctcacgccaaagccatcatcccggcgcaacgagccagcccatctgccccatattttgcaacgtattgcgcactggcgtggagaagatgccgcatggctggctgccaccacggatgctaatgtcaaaacactgtttgggattgcgttttagagtttgcggaactcggtattcttcacactgtgcttaatctctttattaataagattaagcaatagcatggagcgagcctcaccatcgggttcggtgaaaatggcctgaaagccttcgaacgcgccttcggtaataatcaccttatcacccggataaggggttgccggatcgacaatgtctttcggtttatataccgatagctgatgaataaccgccgatgggactatcgctggcgacgcgccaaagcgcacgaagtggctgacaccgcgggtcgcgttgatagtcgtggtatgaatcacttctgggtcaaattccacaaacaggtagttggggaacaatggctcactgactgcagtacgttttccacgcacgattttttccagggtgatcatcggtgccaggcaattcacagcctgtctttcgaggtgttcctgggcacgttgaagttgcccgcgcttgcagtacagtaaataccaggattgcataatgactcttatccgtttaatcggggcgcaaggatagcaaaagctttacgctaagttaattatattccccggtttgcgttataccgtcagagttcacgctaatttaacaaatttacagcatcgcaaagatgaacgccgtataatgggcgcagattaagaggctacaatggacgccatgaaatataacgatttacgcgacttcttgacgctgcttgaacagcagggtgagctaaaacgtatcacgctcccggtggatccgcatctggaaatcactgaaattgctgaccgcactttgcgtgccggtgggcctgcgctgttgttcgaaaaccctaaaggctactcaatgccggtgctgtgcaacctgttcggtacgccaaagcgcgtggcgatgggcatggggcaggaagatgtttcggcgctgcgtgaagttggtaaattattggcgtttctgaaagagccggagccgccaaaaggtttccgcgacctgtttgataaactgccgcagtttaagcaagtattgaacatgccgacaaagcggctgcgtggtgcgccctgccaacaaaaaatcgtctctggcgatgacgtcgatctcaatcgcattcccattatgacctgctggccggaagatgccgcgccgctgattacctgggggctgacagtgacgcgcggcccacataaagagcggcagaatctgggcatttatcgccagcagctgattggtaaaaacaaactgattatgcgctggctgtcgcatcgcggcggcgcgctggattatcaggagtggtgtgcggcgcatccgggcgaacgtttcccggtttctgtggcgctgggtgccgatcccgccacgattctcggtgcagtcactcccgttccggatacgctttcagagtatgcgtttgccggattgctacgtggcaccaagaccgaagtggtgaagtgtatctccaatgatcttgaagtgcccgccagtgcggagattgtgctggaagggtatatcgaacaaggcgaaactgcgccggaagggccgtatggcgaccacaccggttactataatgaagtcgatagtttcccggtatttaccgtgacgcatattacccagcgtgaagatgcgatttaccattccacctataccgggcgtccgccagatgagcccgcggtgctgggtgtcgcactgaacgaagtgtttgtgccgattctgcaaaaacagttcccggaaattgtcgatttttacctgccgccggaaggctgctcttatcgcctggcggtagtgacaatcaaaaaacagtacgccggacacgcgaagcgcgtcatgatgggcgtctggtcgttcttacgccagtttatgtacactaaatttgtgatcgtttgcgatgatgacgttaacgcacgcgactggaacgatgtgatttgggcgattaccacccgtatggacccggcgcgggatactgttctggtagaaaatacgcctattgattatctggattttgcctcgcctgtctccgggctgggttcaaaaatggggctggatgccacgaataaatggccgggggaaacccagcgtgaatggggacgtcccatcaaaaaagatccagatgttgtcgcgcatattgacgccatctgggatgaactggctatttttaacaacggtaaaagcgcctgatgcgcgtttgttttgccctatttatcgatccgacagagaaagcgcatgacaaccttaagctgtaaagtgacctcggtagaagctatcacggataccgtatatcgtgtccgcatcgtgccagacgcggccttttcttttcgtgctggtcagtatttgatggtagtgatggatgagcgcgacaaacgtccgttctcaatggcttcgacgccggatgaaaaagggtttatcgagctgcatattggcgcttctgaaatcaacctttacgcgaaagcagtcatggaccgcatcctcaaagatcatcaaatcgtggtcgacattccccacggagaagcgtggctgcgcgatgatgaagagcgtccgatgattttgattgcgggcggcaccgggttctcttatgcccgctcgattttgctgacagcgttggcgcgtaacccaaaccgtgatatcaccatttactggggcgggcgtgaagagcagcatctgtatgatctctgcgagcttgaggcgctttcgttgaagcatcctggtctgcaagtggtgccggtggttgaacaaccggaagcgggctggcgtgggcgtactggcaccgtgttaacggcggtattgcaggatcacggtacgctggcagagcatgatatctatattgccggacgttttgagatggcgaaaattgcccgcgatctgttttgcagtgagcgtaatgcgcgggaagatcgcctgtttggcgatgcgtttgcatttatctgagatataaaaaaacccgcccctgacaggcgggaagaacggcaactaaactgttattcagtggcatttagatctatgacgtatctggcaaaccatgcccgatgcgacgctgtcgcgtcttatcgtgcctacaaatagtccgaaccgtaggccggataaggcgtttacgccgcatccggcaattggtgcatgatgcctgatgcgacgctgtcgcgtcttatcgtgcctacaaatagtccgaaccgtaggccggataaggcgtttacgccgcatccggcaattggtgcatgatgcctgatgcgacgctggcgcgtcttatcaggcctacattggtgccggatcggtagaccggataaggcgttcacgccgcatccggcaagtggttaaacccgctcaaacaccgtcgcaataccctgacccagaccgatacacatcgtcgccagaccaaactgaacgtctttgcgttccatcagattcagcagcgtggtgctgatacgcgcaccggaacaacccagcggatgacccagcgcgatcgcgccaccgttgaggttgatcttctcgtcaatctgctcaattagtcccagatctttaatacatggcaggatctgcgcggcaaaggcttcgttcatttcaaacacgccgatatcgctggcagaaagccccgcttttttcagcgccagtttcgaggccggaaccgggccgtaacccataatcgatgggtcacaaccaacgaccgccatcgaacgcacacgagcgcgcggcttaagacctaattcatgggcgcggctttcactcatcaccagcatggcagctgcgccatcggaaagtgcagaagatgtgcccgccgttaccataccgtttactggatcaaacgccggacgcagcgtggcgagggcttccacggtggtttccgggcgaatcacttcgtcgtaattaaactgcttcaggacgccgtcggcatcgtgaccaccggtcgggatgatttcatttttaaatgcggccgactgcgtggcggcccaggcgcgggcgtgtgaccgcgcggcaaaggcatcctgcatttcacggctgataccgtgcatacgcgccagcatttctgccgttaagcccatcatgcccgccgctttggcgacattgcggctcaggccggggtgaaaatcgacgccgtgactcatcggcacatggcccatatgctccacgccgccaaccagacatgcctgcgcatcgccagtcatgatcattcgtgctgcgtcatgcagtgcctgcatggatgaaccacacaagcgattaacggtaaccgccgggacagagtgtggtacttctgccagcagcgccgcgttacgggcgatattaaaaccctgctccagcgtctgctgcacacaaccccagtaaatatcgtcgagggccgccgcttccagcgccgggttacgcgccagcaggctacgcattaaatgagcggagagatcttctgcacgcacgttacgaaaagcaccgcccttcgaacggcccatcggggtgcgaattgcatcgacaatgacaacctgttccattgtgactccttaagccgttttcaggtcgccaaccggacgggctggctcaaccggaggatagtacggttcgttatgacgcgctttattacgcagaccttccggcacttcatacagcgggccgaggtgctgatattgctgtgccatatcgaggtattttgcgctaccgagggtgtccagccagcggaacgcgccgccgtggaacggagggaagcccaggccgtagaccagcgccatatccgcttccgccggagtggcgataatgccttcctccagacagcgcaccacttcgttgaccatcgggatcatcatgcgggcgataatctcttcttcgctgaaatcgcgcttcggctggctcacttctgccagcaggtcttcaacggcggcgtcttcttctttcttcggcttacctttgctgtcttctttataacgccagaaaccgaggccgttcttctgaccaaagcggttggcatcaaacagcgcgtcgatggcatcgcggtaatctttctgcatccgctgcgggaagcctgctgccatgacagcctgagcgtgatgcgcggtatcaatgcccacaacgtccagcagatatgccgggcccatcggccagccaaactgtttttccatcactttgtcgatcttgcggaaatccgcgccgtcgcgcagcagctggctgaaaccggcgaaatacgggaacagcacgcggttaacaaagaagccggggcagtcgttaaccacaatcggcgtcttgcccatcttgctcgcccaggcgacaactttcgcgatggtttcgtcggagcttttctcgccgcgaataatttctaccaacggcattcggtggaccgggttaaagaagtgcatcccgcagaagttttccgggcgttccagcgcgttggccagttcgctgataggaatggttgaagtgttagacgccagcacggtatcctggcgtactttttgttcggtttctgccagtacggcttttttcactttcgggttttcaacaaccgcttctaccacaatatccacgcggtcaaatccggcgtagtcgagcgttgggtggattgtggagatcacgccagccagtttcagaccatcgatcttgccgcgctcaagctgcttgttcagcagtttcgcggcttcggtcatgccgagggttaacgacttgtcgttgatatctttcatgacaaccggcacgcctttccacgcagactggtaagcgatgccgccgcccataatgcctgcacccagcaccgcggcctgtttcggggtttcaacgtctttggtgagtttcttcgctttgccttttacatattgatcgttaaggaaaatgccgaccagtgcgcgggcttcgttggtatgcgccagcgggacaaaacttttgttttccaggtttaaggcttcttcacgaccaaaacgggccgcagcttcaatggtttttactgcggtgatgggggccggataatgtttccccgctgtttgtgcgaccatccctttagcgatggtgaagctcatggtggcttcaatcttgctcagttttagtggttccagcttcggctgacgttttgctttccagtcgaggtcgccgttaatggcctggcgtaaaaccgcctttgcgccttcaaccagtttttctgctttgactacgccatccaccagaccgattttcagcgcctgatccgcgccgacatctttaccggcggcaatgatttccagcgcactgtcagcgcccagcatacgtggcatacgtacagaaccgccaaagccaggcatgatgcccagtttggtttccggcagaccgatgcgcagatccggcgtcgccagacgataatcggtcgccagcacgcattcgcagccaccgcccagcgcatagccattgacggcagcaatggtcggcaccggcagatcttccaggcgattaaacacgctattggcaaagtgcagccactgacttaactgttcttcaggaacgaggaacagggacaaaaattcggtgatatcagcaccgacgataaaggctgctttgttcgaacgcagcagcagcccttttagatctgattgctgttccagcacgccgatggcctcgccgaggctggcgacggtcgcagtgtcgagtttattaactgaacctggggcatcaaataccagttcggcaatgccatcttccagccagtcaaggtacagggtgtcgcctttgtaaagcatgtcagtctcctgaatccgcaaggtgatctggtcgtaccagatgagtcgaagtgtgtattttgtgttaaaaatatgcaaacaaaagattaaagaaatgccgatctgatcacgctcggcagaaatcacgctctggatgaacgatgtgctaagatgcggagacttaaggtcaaaaaaacagaagggtaaaaaatggaatcactggcctcgctctataaaaatcatatagctaccttacaagaacggactcgcgatgcgctggcgcgcttcaagctggatgcgttacttattcactccggcgagctgttcaatgtttttctcgacgatcatccctatccgtttaaagtgaacccgcaattcaaagcgtgggtgccggtaactcaggtgccaaactgctggttgctggtggatggcgtgaacaagccgaaactgtggttctatctgccggttgattactggcacaacgtcgaaccgctgccgacctctttctggactgaagatgtggaagtgatcgcgctgccgaaagccgatggcattggtagcctgctgcctgctgcgcgcggcaatatcggttatatcggtccggtgccggaacgtgcgctgcaactgggtattgaggccagcaacatcaacccgaaaggggttatcgactacctgcattactatcgctccttcaaaactgagtacgaactggcctgtatgcgtgaagcgcagaaaatggcggtcaacggtcaccgcgcggcagaagaagcgttccgttctggcatgagcgagttcgatatcaacattgcctatctgaccgcgaccggtcatcgtgataccgacgtaccttacagcaacattgtggcgcttaacgaacacgctgcggtactgcattacaccaaactggaccatcaggcaccggaagagatgcgcagcttcctgctggatgccggggcagaatataacggctatgcggctgacctgacccgtacctggtcggcaaaaagtgacaacgactacgcgcagctggtgaaggacgttaatgatgaacaactggcgctgatcgccaccatgaaagcaggcgtcagctatgtggattaccacatccagttccatcagcgcatcgccaaactgctgcgtaaacatcaaatcatcaccgatatgagtgaagaagcgatggtcgaaaacgatcttaccgggccgtttatgccgcatggtatcggccatccgctgggcctgcaggtgcatgacgtcgctggttttatgcaggatgatagcggtacgcacctcgcggcaccggcaaaatatccgtacctgcgctgcacccgtattctccagccgggcatggtgttaaccatcgaaccgggtatctacttcatcgaatcgctactggcaccgtggcgtgaagggcagttcagcaagcacttcaactggcagaaaattgaagcactgaaaccgttcggcggcattcgtatcgaagacaacgtggtgatccacgaaaacaacgtggaaaacatgacccgggatctgaaactggcgtgatggaaagctggttaattcctgcggcaccggtcacggtcgttgaagagatcaaaaagagccgcttcataacgatgttggcgcataccgatggcgttgaggcggcgaaagcgtttgttgaatcggtgcgggcagaacaccccgatgcccggcaccattgcgtggcgtgggtcgcgggtgcgccggatgattctcaacagctgggtttctctgacgacggggagccggcgggaacggcaggtaaaccgatgctcgcccagctaatgggcagcggcgtcggggaaattaccgctgtggtagtgcgctactacggcggcatattgcttggcaccggtgggttagtgaaagcgtatggcggcggcgtgaatcaggcgctgcgccagctaacgacccaacgcaagacgccattaaccgaatatactttgcaatgtgaatatcatcagttaaccggcattgaagcgttgctggggcagtgtgacggcaaaattatcaacagtgattatcaggcattcgttctgctgcgggtggcgcttccggcggcgaaagtggctgaattttccgcaaagctggcggattttagccgtggttcattgcaattgttagcgattgaagaataatccccacttcgttttgcagaactaaggaagcggcagagatgcattttcgcgccattacccgaatcgttggactactggtcatcttattttcagggaccatgattatccctgggctggtagcactcatctaccgggatggagcgggccgcgcttttacccagaccttttttgtcgccctcgccattggctctatgctgtggtggccgaaccgcaaagagaaaggcgaacttaaatcccgtgaggggtttctgatagtggtgctgttctggaccgtgctgggtagcgtcggtgcgctcccttttatcttctcggaaagcccgaacctcacgattaccgatgcgttttttgaatctttctctggcctgaccactacgggagccactacgctggtggggctggattcgctccctcacgccatcctcttttatcgccagatgctgcaatggtttggcgggatggggatcatcgtgttggcggttgcgatactgcctatcctcggcgtgggtgggatgcagctctatcgcgcagaaatgcccggcccgctgaaagataacaaaatgcgcccgcgaattgcggaaacggcgaaaaccctgtggttgatttatgtcttgctgaccgtcgcctgtgcgctggcgttgtggtttgccggaatggatgcctttgatgccatcggccatagctttgcgactatcgctattggcggcttctcgacacatgatgccagtatcggttatttcgatagcccgactattaacactatcattgctatcttcctgctgatctccggctgtaactacggtctgcacttttcactgttaagtgggcgtagtctgaaggtttattggcgcgatccggaatttcgcatgtttatcggcgtacagtttacgctggtggttatttgtaccctcgtactgtggtttcataatgtctacagttcggcgctgatgacaattaaccaggcgtttttccaggtggtgtcgatggcgacaaccgccgggtttacaactgacagcattgcccgctggccgctctttttgccggtactgcttttatgttcagcctttatcggcggttgcgccgggtcaacgggcggtggcctgaaggtgatccgcatcctgctgctgtttaagcaggggaaccgtgagctgaaacgactggtgcatccgaacgccgtctatagcattaagctggggaatcgcgcactgccggaacgtatcctcgaagccgtttggggatttttctccgcctatgcattggtgtttattgtcagtatgctggcgattatcgccacgggcgtggatgacttttctgcctttgcgtcggttgttgcgacattgaataacctggggccagggcttggcgtggttgctgataactttaccagtatgaacccggtggctaaatggatcctgattgccaacatgctgtttggtcgtctcgaggtctttacattgctggtgctctttaccccgactttctggcgtgaatgatggagtaatacgtgaaaacattaattcttttctcaacaagggacggacaaacgcgcgagattgcctcctacctggcttcggaactgaaagaactggggatccaggcggatgtcgccaatgtgcaccgcattgaagaaccacagtgggaaaactatgaccgtgtggtcattggtgcttctattcgctatggtcactaccattcagcgttccaggaatttgtcaaaaaacatgcgacgcggctgaattcgatgccgagcgccttttactccgtgaatctggtggcgcgcaaaccggagaagcgtactccacagaccaacagctacgcgcgcaagtttctgatgaactcgcaatggcgtcccgatcgctgcgcggtcattgccggggcgctgcgttacccacgttatcgctggtacgaccgttttatgatcaagctgattatgaagatgtcaggcggtgaaacggatacgcgcaaagaagttgtctataccgattgggagcaggtggcgaatttcgcccgagaaatcgcccatttaaccgacaaaccgacgctgaaataagcataaagaataaaaaatgcgcggtcagaaaattattttaaatttcctcttgtcaggccggaataactccctataatgcgccaccactgacacggaacaacggcaaacacgccgccgggtcagcggggttctcctgagaactccggcagagaaagcaaaaataaatgcttgactctgtagcgggaaggcgtattatgcacaccccgcgccgctgagaaaaagcgaagcggcactgctctttaacaatttatcagacaatctgtgtgggcactcgaagatacggattcttaacgtcgcaagacgaaaaatgaataccaagtctcaagagtgaacacgtaattcattacgaagtttaattctttgagcgtcaaacttttaaattgaagagtttgatcatggctcagattgaacgctggcggcaggcctaacacatgcaagtcgaacggtaacaggaagaagcttgcttctttgctgacgagtggcggacgggtgagtaatgtctgggaaactgcctgatggagggggataactactggaaacggtagctaataccgcataacgtcgcaagaccaaagaggggtaccttcgggcctcttgccatcggatgtgcccagatgggattagctagtaggtggggtaacggctcacctaggcgacgatccctagctggtctgagaggatgaccagccacactggaactgagacacggtccagactcctacgggaggcagcagtggggaatattgcacaatgggcgcaagcctgatgcagccatgccgcgtgtatgaagaaggccttcgggttgtaaagtactttcagcggggaggaagggagtaaagttaatacctttgctcattgacgttacccgcagaagaagcaccggctaactccgtgccagcagccgcggtaatacggagggtgcaagcgttaatcggaattactgggcgtaaagcgcacgcaggcggtttgttaagtcagatgtgaaatccccgggctcaacctgggaactgcatctgatactggcaagcttgagtctcgtagaggggggtagaattccaggtgtagcggtgaaatgcgtagagatctggaggaataccggtggcgaaggcggccccctggacgaagactgacgctcaggtgcgaaagcgtggggagcaaacaggattagataccctggtagtccacgccgtaaacgatgtcgacttggaggttgtgcccttgaggcgtggcttccggagctaacgcgttaagtcgaccgcctggggagtacggccgcaaggttaaaactcaaatgaattgacgggggcccgcacaagcggtggagcatgtggtttaattcgatgcaacgcgaagaaccttacctggtcttgacatccacggaagttttcagagatgagaatgtgccttcgggaaccgtgagacaggtgctgcatggctgtcgtcagctcgtgttgtgaaatgttgggttaagtcccgcaacgagcgcaacccttatcctttgttgccagcggtccggccgggaactcaaaggagactgccagtgataaactggaggaaggtggggatgacgtcaagtcatcatggcccttacgaccagggctacacacgtgctacaatggcgcatacaaagagaagcgacctcgcgagagcaagcggacctcataaagtgcgtcgtagtccggattggagtctgcaactcgactccatgaagtcggaatcgctagtaatcgtggatcagaatgccacggtgaatacgttcccgggccttgtacacaccgcccgtcacaccatgggagtgggttgcaaaagaagtaggtagcttaaccttcgggagggcgcttaccactttgtgattcatgactggggtgaagtcgtaacaaggtaaccgtaggggaacctgcggttggatcacctccttaccttaaagaagcgttctttgaagtgctcacacagattgtctgatgaaaatgagcagtaaaacctctacaggcttgtagctcaggtggttagagcgcacccctgataagggtgaggtcggtggttcaagtccactcaggcctaccaaatttgcacggcaaatttgaagaggttttaactacatgttatggggctatagctcagctgggagagcgcctgctttgcacgcaggaggtctgcggttcgatcccgcatagctccaccatctctgtagtgattaaataaaaaatacttcagagtgtacctgcaaaggttcactgcgaagttttgctctttaaaaatctggatcaagctgaaaattgaaacactgaacaacgaaagttgttcgtgagtctctcaaattttcgcaacacgatgatgaatcgaaagaaacatcttcgggttgtgaggttaagcgactaagcgtacacggtggatgccctggcagtcagaggcgatgaaggacgtgctaatctgcgataagcgtcggtaaggtgatatgaaccgttataaccggcgatttccgaatggggaaacccagtgtgtttcgacacactatcattaactgaatccataggttaatgaggcgaaccgggggaactgaaacatctaagtaccccgaggaaaagaaatcaaccgagattcccccagtagcggcgagcgaacggggagcagcccagagcctgaatcagtgtgtgtgttagtggaagcgtctggaaaggcgtgcgatacagggtgacagccccgtacacaaaaatgcacatgctgtgagctcgatgagtagggcgggacacgtggtatcctgtctgaatatggggggaccatcctccaaggctaaatactcctgactgaccgatagtgaaccagtaccgtgagggaaaggcgaaaagaaccccggcgaggggagtgaaaaagaacctgaaaccgtgtacgtacaagcagtgggagcacgcttaggcgtgtgactgcgtaccttttgtataatgggtcagcgacttatattctgtagcaaggttaaccgaataggggagccgaagggaaaccgagtcttaactgggcgttaagttgcagggtatagacccgaaacccggtgatctagccatgggcaggttgaaggttgggtaacactaactggaggaccgaaccgactaatgttgaaaaattagcggatgacttgtggctgggggtgaaaggccaatcaaaccgggagatagctggttctccccgaaagctatttaggtagcgcctcgtgaattcatctccgggggtagagcactgtttcggcaagggggtcatcccgacttaccaacccgatgcaaactgcgaataccggagaatgttatcacgggagacacacggcgggtgctaacgtccgtcgtgaagagggaaacaacccagaccgccagctaaggtcccaaagtcatggttaagtgggaaacgatgtgggaaggcccagacagccaggatgttggcttagaagcagccatcatttaaagaaagcgtaatagctcactggtcgagtcggcctgcgcggaagatgtaacggggctaaaccatgcaccgaagctgcggcagcgacactatgtgttgttgggtaggggagcgttctgtaagcctgtgaaggtgtgctgtgaggcatgctggaggtatcagaagtgcgaatgctgacataagtaacgataaagcgggtgaaaagcccgctcgccggaagaccaagggttcctgtccaacgttaatcggggcagggtgagtcgacccctaaggcgaggccgaaaggcgtagtcgatgggaaacaggttaatattcctgtacttggtgttactgcgaaggggggacggagaaggctatgttggccgggcgacggttgtcccggtttaagcgtgtaggctggttttccaggcaaatccggaaaatcaaggctgaggcgtgatgacgaggcactacggtgctgaagcaacaaatgccctgcttccaggaaaagcctctaagcatcaggtaacatcaaatcgtaccccaaaccgacacaggtggtcaggtagagaataccaaggcgcttgagagaactcgggtgaaggaactaggcaaaatggtgccgtaacttcgggagaaggcacgctgatatgtaggtgaagcgacttgctcgtggagctgaaatcagtcgaagataccagctggctgcaactgtttattaaaaacacagcactgtgcaaacacgaaagtggacgtatacggtgtgacgcctgcccggtgccggaaggttaattgatggggttagccgcaaggcgaagctcttgatcgaagccccggtaaacggcggccgtaactataacggtcctaaggtagcgaaattccttgtcgggtaagttccgacctgcacgaatggcgtaatgatggccaggctgtctccacccgagactcagtgaaattgaactcgctgtgaagatgcagtgtacccgcggcaagacggaaagaccccgtgaacctttactatagcttgacactgaacattgagccttgatgtgtaggataggtgggaggctttgaagtgtggacgccagtctgcatggagccgaccttgaaataccaccctttaatgtttgatgttctaacgttgacccgtaatccgggttgcggacagtgtctggtgggtagtttgactggggcggtctcctcctaaagagtaacggaggagcacgaaggttggctaatcctggtcggacatcaggaggttagtgcaatggcataagccagcttgactgcgagcgtgacggcgcgagcaggtgcgaaagcaggtcatagtgatccggtggttctgaatggaagggccatcgctcaacggataaaaggtactccggggataacaggctgataccgcccaagagttcatatcgacggcggtgtttggcacctcgatgtcggctcatcacatcctggggctgaagtaggtcccaagggtatggctgttcgccatttaaagtggtacgcgagctgggtttagaacgtcgtgagacagttcggtccctatctgccgtgggcgctggagaactgaggggggctgctcctagtacgagaggaccggagtggacgcatcactggtgttcgggttgtcatgccaatggcactgcccggtagctaaatgcggaagagataagtgctgaaagcatctaagcacgaaacttgccccgagatgagttctccctgactccttgagagtcctgaaggaacgttgaagacgacgacgttgataggccgggtgtgtaagcgcagcgatgcgttgagctaaccggtactaatgaaccgtgaggcttaaccttacaacgccgaaggtgttttggcggattgagagaagattttcagcctgatacagattaaatcagaacgcagaagcggtctgataaaacagaatttgcctggcggcagtagcgcggtggtcccacctgaccccatgccgaactcagaagtgaaacgccgtagcgccgatggtagtgtggggtctcctcatgcgagagtagggaactgccaggcatcaaataaaacgaaaggctcagtcggaagactgggcctttcgttttatctgttgtttgtcggtgaacgctctcctgagtaggacaaatccgccgggagcggatttgaacgttgcgaagcaacggcccggagggtggcgggcaggacgcccgccataaactgccaggcatcaaattaagcagaaggccatcctgacggatggcctttttgcattggcgcagaaaaaaatgccggatgcgacgctggcgcgtcttatccagcctactcttgcttatccgttctgcttttgcatccactccaccacaaaatcagccagcccctcaacatcattaatatccagtaatgcgacatcaagattaagcggcacatcactggctacagcaataacatgcctgtctatcactaattcttcaggtcgatgtccggctccatcgcgaaacagcacaatctttgcgatctcttcatgcttaaacccttcgaccagaatcaaatccagctttgaggtatccattcgacttgcgagaaactgtagatccagctcttcttcgtctggtgtttccgtcatcaaggcccatcgttgctggctggcaacgatggtttgtgccgcgccagccttgcgcagctcatagctatctttgcctggcttatcaacatccatatcatggtgcgtatgcttaatcagccctggacggatccctctggcgcataatgccgggatcagttttttcaaaagcgtagtttttccggtaccactccacgcggcaaaggcgagtaacggtatcatcgtttttcctgccatcgggcaagctcctctggcgtattcacgttaacaaatgcatctttatgatcgctgaaatcaaccgcatgaccgccagccagacgcataaataccattacccggcgttctcctgcttgcagatattccagtaataaaggctcaatagcgcggtttaccagagcaatagtcgggtgatcgcgttcaccgtcatggacccacacgacaggcgcatctttgcgctgatgattaagcctggctgctaaatcagggggaatgtaaggcgtatcgcacgggcaaaacaaaaaccactcaccagcttcctgctgcattactgaaagcattcctgccagagggcctgggtaatccgccagtgaatcttcaatcactttcagaccgcttgcctgatagatttcctgatgacgattagcattaaccacgacgtgagagagctgcgtcataagcgcgtcagcgacatgttgccataatggtttgccgtttaattcaagcaatcctttatctacgccgcccattcgtctggctttaccgcctgccagcacaacgcctgttatcgtcgtcatcagattcaccgatatcgcctcttttattgtgggattgaccctgctaacgtgtctgtctcaagagtaaggagcatcactatgaaatgtaaacgtctgaatgaagttattgaactcctccagccagcctggcaaaaagagccagaccttaacctgctgcaatttttgcagaaactggcgaaagagtcaggttttgacggcgaactggcggatttgacggatgacattctgatctatcacctgaaaatgcgtgattccgcgaaagatgcggtgatcccgggtttgcagaaagattatgaagaagacttcaaaacggcgctgttacgcgctcgcggcgtaattaaagagtaaaagcttgtaagcggcgccaccaaaatcatcgtgaaatgatatccttcgtcattcgtaatgttttccggatgatgggatgaataacagcgcttttactttccagacactacacccggataccatcatggacgctctgtttgagcatgggatccgggtggattccggtcttaccccgcttaacagctatgaaaaccgtgtctatcaatttcaggacgaagatcgtcgacgttttgtcgtcaaattttatcgccctgaacgttggacagccgatcaaatcctcgaagaacatcaatttgcgttgcagctggtaaatgatgaagttccggtcgcagcacctgtggcctttaacggtcagactttattgaatcatcagggattttatttcgctgtttttccaagcgtcggtggtcgccagttcgaagctgataatatcgatcagatggaagcggttgggcgttatttagggcgtatgcaccagacggggcgcaaacagctttttatccatcgcccgaccatcggtttgaacgaatatctcattgagccacgcaagctgtttgaggacgctacactgataccttccgggttgaaagcggcattcctgaaagcgacagatgagctgattgccgccgttacagcacactggcgggaagatttcaccgttctgcggctacatggagactgccacgccgggaatattctctggcgcgatggtccaatgtttgttgatctggatgatgcacgtaatggtccagccgttcaggatttgtggatgttgctcaatggcgataaagccgagcagcggatgcaactggaaactattattgaagcttatgaagaatttagcgagttcgacaccgctgaaatcggactgattgaacctttacgcgccatgcgtttggtttattatcttgcctggctaatgcggcgttgggctgatcccgcgttcccgaaaaatttcccgtggttaaccggggaagattactggctgcgacagacggcgacttttatagaacaggcaaaagttctacaagaaccccctttgcaattaacacctatgtattaatcggagagagtagatcatgaaaaagatttggctggcgctggctggtttagttttagcgtttagcgcatcggcggcgcagtatgaagatggtaaacagtacactaccctggaaaaaccggtagctggcgcgccgcaagtgctggagtttttctctttcttctgcccgcactgctatcagtttgaagaagttctgcatatttctgataatgtgaagaaaaaactgccggaaggcgtgaagatgactaaataccacgtcaacttcatgggtggtgacctgggcaaagatctgactcaggcatgggctgtggcgatggcgctgggcgtggaagacaaagtgactgttccgctgtttgaaggcgtacagaaaacccagaccattcgttctgcttctgatatccgcgatgtatttatcaacgcaggtattaaaggtgaagagtacgacgcggcgtggaacagcttcgtggtgaaatctctggtcgctcagcaggaaaaagctgcagctgacgtgcaattgcgtggcgttccggcgatgtttgttaacggtaaatatcagctgaatccgcagggtatggataccagcaatatggatgtttttgttcagcagtatgctgatacagtgaaatatctgtccgagaaaaaataattcaatgtaaattacataaagcccgtgaatattcacgggctttttttattatttaataaatataaatacattctgataatgcatcctgccgctggacattatttcagcataagtggatattcaaagttttgctgttttatcagggaatatttatatgatacgtaagtcagctacaggtgttattgttgcgttagccgtaatctggggtggtggcacatggtacacaggtacgcaaattcagcctggtgtcgaaaaatttattaaagattttaacgatgctaaaaagaaaggtgaacatgcctacgatatgacgttaagttatcaaaattttgacaaaggcttttttaattcccgttttcaaatgcaaatgacattcgataacggtgcacccgatctcaatatcaagccaggccagaaagttgtatttgatgtggatgttgagcacggtccgttgcccatcacaatgttaatgcatggtaatgtcatcccagcactggcagcggcaaaagtgaacttagtgaataatgaactgacacaaccgctatttatcgccgcgaaaaataaatcgcccgtggaagcgacattgcgattcgcgtttggtggctcattctctacgacattagatgttgcccctgcagagtatggaaagttttcttttggtgagggccagtttacttttaatggtgatggtagttcattgtctaacctggatattgaaggcaaagtcgaagatattgttctgcaattatcaccaatgaacaaagtaacggcaaaaagttttaccattgattctctggcgcgattagaagaaaagaaatttccggttggtgaaagcgagtcgaaatttaatcagattaacattatcaatcacggggaagacgttgcccaaatcgatgctttcgttgcaaaaaccaggctggatcgcgttaaagacaaagattatatcaatgtcaatctcacctacgaacttgataagttaacaaaagggaatcagcaactcggtagtggtgagtggtcattgattgctgaatctattgatccctcagcagtgcgccaatttatcatccagtataacattgcgatgcagaagcagcttgctgcacaccctgagttagcaaacgatgaagttgctctgcaagaagtgaatgctgcattgttcaaagagtatttaccgttattacaaaaaagtgagccgaccattaaacaaccggtaagatggaagaacgcactcggcgaactaaatgccaatctggatatcagtattgccgacccagccaaatcttcatcatccacaaacaaagatatcaaatcgctcaattttgatgtgaagttaccgcttaatgtcgtcacagaaaccgcaaaacagcttaatttatctgaaggaatggatgcggaaaaagcgcaaaagcaggctgataaacaaatcagcgggatgatgacattaggtcagatgtttcagttaatcacgattgacaacaataccgcctcgctgcagctgcgttatacaccgggtaaagttgtttttaacggacaggagatgagcgaagaagaatttatgtctcgtgccggacgttttgttcattaaaatactcactcgcctctgctcattcagaggcgagtaaaacttacttattctgacgctgtgatgacatgagagacgtcagaagccggtctttttcctgccacaatgagttcagccattgctgaaaatggcgcttaaagcttttgtcattgatgtagtcgccatgtaactcatcggcaataggctgtaaatccacatgtacgacaatccgcgtcagtttaccgcttaacatatcgaagaacggctgacggttattgtccggataacacagcgtaacattaagcagtttatcgaattgtttacccagtacatttagcgccatcgcaatgcctgccgcctttggtggcaacaagttttgaaaagtggagtgggtttgctgatgtttttcttgcgtgaaacgggagccttcaacgaaattgacaatggtggtgggatgcaggcgaaacttttcacaagaacgccgagtggtttcaacatctttaccacgtcgctccggatgacgtaataaataagcgcgggaataacgcttcataaacggcatatccagcgaccagcacgccaggccaagaaatggcacccaggccagctgttgcttgaggaaatatttattcatcggaatgtgcttacgaaacagcacgcacagtacgacaatatctgcccaactacggtggttacaaataagcagataccagttcttcttacttaacccttccagcccgtgaacttcccattgaaggtgtgggttcagatgcagtaataccgccagaccttcacaccagcaatacatcataaaatcacaaaaacgcgaaacctttcgccaaatgactggcacaggtagcaatagttttacaatcccggcaatgatgatcgggacggaacaaaaaatagtgaccaaaatggtcaatacgatactcagcaaaagggttatcgcagcgagtattctcgtcataatgaatttattcaaaaggttagccatagacagtgcgctaaagaagcgcaaggcgcagattttagcagaaaacgacccaaataacggatgatccttaaggagaaaaataattcatatctatccacattagaaaaaatcccattatctcaattattagggatggatttatttttaactgcatgaaaaacaaagacaaacatcatgctgtaaaaagcatgataataaattaaaagcgatgtaaataatttatgcacaaagttatccacatgacgatttgcgagcgatccagaagatctacaaaagattttcacgaaaagcggtgaaaaactcatgttttcatcctgtctgtggcatcctttacccataatctgataaacaggcacggacattatggttcagatcccccaaaatccacttatccttgtagatggttcatcttatctttatcgcgcatatcacgcgtttcccccgctgactaacagcgcaggcgagccgaccggtgcgatgtatggtgtcctcaacatgctgcgcagtctgatcatgcaatataaaccgacgcatgcagcggtggtctttgacgccaagggaaaaacctttcgtgatgaactgtttgaacattacaaatcacatcgcccgccaatgccggacgatctgcgtgcacaaatcgaacccttgcacgcgatggttaaagcgatgggactgccgctgctggcggtttctggcgtagaagcggacgacgttatcggtactctggcgcgcgaagccgaaaaagccgggcgtccggtgctgatcagcactggcgataaagatatggcgcagctggtgacgccaaatattacgcttatcaataccatgacgaataccatcctcggaccggaagaggtggtgaataagtacggcgtgccgccagaactgatcatcgatttcctggcgctgatgggtgactcctctgataacattcctggcgtaccgggcgtcggtgaaaaaaccgcgcaggcattgctgcaaggtcttggcggactggatacgctgtatgccgagccagaaaaaattgctgggttgagcttccgtggcgcgaaaacaatggcagcgaagctcgagcaaaacaaagaagttgcttatctctcataccagctggcgacgattaaaaccgacgttgaactggagctgacctgtgaacaactggaagtgcagcaaccggcagcggaagagttgttggggctgttcaaaaagtatgagttcaaacgctggactgctgatgtcgaagcgggcaaatggttacaggccaaaggggcaaaaccagccgcgaagccacaggaaaccagtgttgcagacgaagcaccagaagtgacggcaacggtgatttcttatgacaactacgtcaccatccttgatgaagaaacactgaaagcgtggattgcgaagctggaaaaagcgccggtatttgcatttgataccgaaaccgacagccttgataacatctctgctaacctggtcgggctttcttttgctatcgagccaggcgtagcggcatatattccggttgctcatgattatcttgatgcgcccgatcaaatctctcgcgagcgtgcactcgagttgctaaaaccgctgctggaagatgaaaaggcgctgaaggtcgggcaaaacctgaaatacgatcgcggtattctggcgaactacggcattgaactgcgtgggattgcgtttgataccatgctggagtcctacattctcaatagcgttgccgggcgtcacgatatggacagcctcgcggaacgttggttgaagcacaaaaccatcacttttgaagagattgctggtaaaggcaaaaatcaactgacctttaaccagattgccctcgaagaagccggacgttacgccgccgaagatgcagatgtcaccttgcagttgcatctgaaaatgtggccggatctgcaaaaacacaaagggccgttgaacgtcttcgagaatatcgaaatgccgctggtgccggtgctttcacgcattgaacgtaacggtgtgaagatcgatccgaaagtgctgcacaatcattctgaagagctcacccttcgtctggctgagctggaaaagaaagcgcatgaaattgcaggtgaggaatttaacctttcttccaccaagcagttacaaaccattctctttgaaaaacagggcattaaaccgctgaagaaaacgccgggtggcgcgccgtcaacgtcggaagaggtactggaagaactggcgctggactatccgttgccaaaagtgattctggagtatcgtggtctggcgaagctgaaatcgacctacaccgacaagctgccgctgatgatcaacccgaaaaccgggcgtgtgcatacctcttatcaccaggcagtaactgcaacgggacgtttatcgtcaaccgatcctaacctgcaaaacattccggtgcgtaacgaagaaggtcgtcgtatccgccaggcgtttattgcgccagaggattatgtgattgtctcagcggactactcgcagattgaactgcgcattatggcgcatctttcgcgtgacaaaggcttgctgaccgcattcgcggaaggaaaagatatccaccgggcaacggcggcagaagtgtttggtttgccactggaaaccgtcaccagcgagcaacgccgtagcgcgaaagcgatcaactttggtctgatttatggcatgagtgctttcggtctggcgcggcaattgaacattccacgtaaagaagcgcagaagtacatggacctttacttcgaacgctaccctggcgtgctggagtatatggaacgcacccgtgctcaggcgaaagagcagggctacgttgaaacgctggacggacgccgtctgtatctgccggatatcaaatccagcaatggtgctcgtcgtgcagcggctgaacgtgcagccattaacgcgccaatgcagggaaccgccgccgacattatcaaacgggcgatgattgccgttgatgcgtggttacaggctgagcaaccgcgtgtacgtatgatcatgcaggtacacgatgaactggtatttgaagttcataaagatgatgttgatgccgtcgcgaagcagattcatcaactgatggaaaactgtacccgtctggatgtgccgttgctggtggaagtggggagtggcgaaaactgggatcaggcgcactaagattcgcctgaacatgccttttttcgtaagtaagcaacataagctgtcacgttttgtgatggctattagaaattcctatgcaacaactgaaaaaaaattacaaaaagtgctttctgaactgaacaaaaaagagtaaagttagtcgcgtagggtacagaggtaagatgttctatctttcagaccttttacttcacgtaatcggatttggctgaatattttagccgccccagtcagtaatgactggggcgttttttattgggcgaaagaaaagatccgtaatgcctgatgcgctatgtttatcaggccaacggtagaattgtaatctattgaatttacgggccggatacgccacatccggcacaagcattaaggcaagaaaattattcgccgtcctgcgtttcttctacaggctgcatctcgctaaaccaggtatccagtttctgccgcagcttgtccacgccttgtttcttcaacgaagaaaacgtttcaacctgcacatcaccgttaaacgccagtacagcttcacgcaccatattcaattgcgctttacgtgcgccgcttgccagtttgtccgctttggtcagcagcaccagaacggcgatattgctgtctaccgcccactcaatcatctgctgatccaaatctttcagcggatggcgaatatccattagcaccaccagaccttgcaggctctgacgtttttcgaggtattcgccgagcgcacgctgccatttgcgcttcatctcttccgggacttccgcataaccgtacccaggcaagtcaaccagacgcttgccgtcagccacttcaaacaggttgataagctgggtgcgccctggggtttttgaggtacgagccaggcttttctggttagtcagcgtgttcagcgcgctggatttacctgcgttggaacggcctgcaaaagccacttcaattccggtatcggaaggtaggtggcgaatatcaggcgcactcatcacaaaatgcgtctgttgataattcaaattagtcaaagcggtcgtctccgtcagtcaaagctttgtggcgattatacctgaaccataataaaaggcggatttttcggcgtgagcgttgtaagtaaaagccatacgctttgtgagacattgccgatagtctttatgcgaaatagcagagaaaattctgcgatgcatgtcaaataagctatataaatcagtgaattgcttttatataaaactctgaaaatgtgcaaatactgatggcggttgattgtttgtttaaagcaaaggcgtaaagtagcacccatagagcgaggacgctaacaggaacaatgactcaggatgagggtcaggagcgccaggaggcgaagacagaggattgtcaggaagacaaacgtccggagacgtaattaaacggaaatggaatcaacacggattgttccggctaaaggaaaaacagggtgtgttggcggcctgcaaggattgtaagacccgttaagggttatgagtcaggaaaaaaggcgacagagtaatctgtcgccttttttctttgcttgctttctgttagattccgccgcaaatctatactgaataaaacggctaaaagacgaaccattatgaaaccatcatcttcaaactcacgcagcaaaggtcatgcaaaagcgcgtcgaaaaacacgcgaggagctggatcaggaagctcgtgatcgcaagcgtcagaaaaaacgtcgtggtcatgcgccgggcagccgcgcagcgggcggaaacaccacgtcaggcagcaaaggccagaacgcaccaaaagatccacgtattggcagtaaaacccctattccattgggcgtgactgaaaaagtcaccaaacagcacaaaccgaagagtgagaaacctatgctttcaccgcaggcggagttggaattactggaaacggatgagcgtctggatgcgctgctggaacgtctggaagcaggcgaaaccctgagtgccgaagagcaatcctgggtggatgctaaactggatcgtattgatgagttgatgcagaaactcggcctctcttatgacgatgacgaagaagaggaagaagacgagaagcaagaagacatgatgcgtctgctgcggggcaactaacggattgccgccgtgggccttcccgttctgctgataacccttccggttatatgttatctggtgtggttattcgttaaactacagcggttgtcgcggcgacaaaagtggctgcgcaaccggctgatgacccgaaacgggcatccgccggtacgccgtagccgccagagacgccatcggaaggagtgagcatgtctgtacagcaaatcgactgggatctggccctgatccagaaatataactattccgggccacgatacacctcgtacccgaccgcgctggagttttcagaagacttcggcgaacaggcgtttttacaagccgtggcgcgctatcctgagcgtccattatctctctacgtacatatcccgttctgccataagctttgttacttctgcggttgcaataagattgttactcgccagcagcacaaggccgatcagtatctggacgcgctggagcaagaaatcgtccatcgtgcaccgctgttcgccgggcgtcacgtcagccaattgcactggggcggcggaacgccgacgtatctgaataaagcgcaaatcagccgcctgatgaagctgctgcgcgaaaacttccagttcaatgccgatgcggagatttcgatcgaagtcgatccgcgggaaatcgaactggatgtactcgatcatttacgcgccgaaggctttaatcgcctgagcatgggcgtgcaggacttcaacaaagaagtgcaacgtctggttaaccgcgagcaggatgaagagttcatctttgcactgcttaaccatgcgcgtgagattggttttacctccaccaacatcgacctgatttacggcctgccgaaacagacgccggagagtttcgcctttaccctgaaacgtgtggcggagctgaaccccgatcgtctgagtgtctttaactacgcgcatctgccgaccatttttgctgctcagcgcaaaatcaaagatgctgacctgccgagtccgcagcaaaaactcgatatcctgcaggaaaccatcgccttcctgacgcaatcgggctatcagtttatcggtatggatcactttgcccgtccggatgacgagctggcggtggcccagcgtgaaggcgtgctgcatcgtaacttccagggctacaccactcagggcgataccgatctgctggggatgggcgtttccgccatcagcatgattggcgactgctacgcgcagaaccagaaagagttgaagcagtactatcagcaagtggatgaacaaggcaatgcgctgtggcgtggtattgcgctaacgcgtgatgactgtattcgccgcgatgtgattaagtcgctcatctgcaacttccgtctggattacgcccctattgagaaacagtgggatttgcacttcgctgattactttgcggaagatctcaagctgctcgccccgttagcaaaagatgggctggtggatgtggatgagaagggaatacaggtgacggcgaaaggtcgcttgctgatccgcaacatttgcatgtgctttgatacctatctgcgccagaaagcgcggatgcagcagttctctcgggtgatttaaatagtgaatggcgcttcgtttacaaagtagaaaacgaaagcgccatcaatgtgctgagaacaagattgcctgatgcgctgggcaacaaaacctgttgaaattattgcttttgtaggccggataaggcgtttacgccgcatcaggcatctgagcatgatgcctgatgcggcgctggtcgcgtcttatcaggcctacgactttctccgcatccggcataaacaacgagcttcagctaaacagcccaatcattgcggcacacagcacggcagcaacggcagtttgcggtgtgtggctgtcaactgcgccactcgataccagattaattattgattccagcataatgactctccccgttttccgggcaagatcatactgaacttatcggaacagtaaagcgtaaaataccagcaatttgcgctcaataatcaatctttacacacaagctgtgaatcactccatccccagctcttttaacttacgcgtcagggtgttgcggccccagccgagtagccgcgccgcttcctgtttatgcccctgcgtatgtcgcaacgcggtcgtcagtaacgtccgctccagctctggctgcgcttcggaaagcagattttgatgaccggaacgcagcgctctgtctgcccactgcgcaagaagcgtcgcccagctgtccggttgcatttgcgaagtactctccgcaaccgttgattcaaacagttcgccgggcaaatcctgaatcaacacttcctgcccggcggccatcaccgttagccagcggcaggtgttttccagctggcgcacgttgcctggccacgccagacgcgtcagagcagcttcggtttccggatgcagtaacttcgcttctacgcccagttcgcgcgcggcaacctgtaaaaaatggcgcgccagacggggaatatcttcccgacgttcgcgcagcggcggcagatgaacgcggataacgttcaggcggtggaacagatcctcacggaacttaccttcctgcactcgctgttcgagattctggtgagtggcagcgataatccgcacatccactttcaccggcgcatagccgccaacgcggtaaaactgaccgtctgccagcacgcgcagcaaacgcgtctgcacatccagcggcatatcaccaatttcgtcgaggaataatgtaccgccatcggcctgttcaaaacgcccctgacgaatggtattcgcgccagtaaacgcgcctttctcgtggccaaacagttctgattcgatcaaatcttttgggatagctgccatattcagcgcgataaacggcgctttggcgcgcggactgtggcgatgcagggcatgagcgaccagttctttaccggtgccggattcgccgttaatcagcacgctaatagaagaacgcgaaagccgaccgataatacggaacacgtcctgcatggctggcgcttcgccgatgatatcggtcgttgggccgttaagctgaacattacgcggctgctgctgttcctggtaatgactgatagcgcgctcaaccagcgccactgcttcgtcgatatcaaacggtttgggcagataatcaaacgccccttgttgataggcgctgacggcagcatccagatcggaatgtgcggtcataatgatgaccggaagcattggatggcgctgtttaatctgcttgagcagcgccagcccgtccattcccggcatacggatatctgaaagcagcacatccggcgttttgctcgccagcgcctccagcacttctgcgccgttctcaaacgtcgtacaggttaaacctgccccagcgagcgcacgttcaagcacccaacggatggaactatcgtcatcgactacccagactatccctcgttgcataaacgtcacctttatttcctgataggcaggtaaaccgagaactcggtatgccctggccaactggtaaattcaattttgcctgaatgctgatcaatcaaattacgagcgatggataagccaagcccggtgccaccttcgcggccgctgaccatcgggtaaaacagcgtatcctgcaaatgaggcggaatgcccggcccgttatcttccacatcaatccgcgccgccagccggtagcgctcgccgtgtaaggtcagttgaaacgcggtgcgggtacgcagaatgatttcaccgccttccggccccagcgcctgtagcgcattgcgcacaatattcagcaagacctgttcaatttgatccgggtcgtgcgccagttccggtaggctgggatcgtaatcacgaatcaaccgcacgttgtccggcagttccatcgacaccagcgttaccacgcgttcagccactttgtgaatactttcggtaacgcgcgtaccgggcagctgcggccccaacagacggtcgaccagatttcgcagccggtccgcctgttcgataatcactttggtatattcgagtagtgatgggtcaggtaacgctttgctgagcagctgcgccgcgccacgtaaaccgccaagcggatttttaatctcatgtgccaggccgcgcactaaatcacgggcagcaacctgctgggcgtgctgtagctgttcctgacttaagcggcgctggttatccatcggagccatctccagcaggatcatgccgtccggcatacgctgggccgtcacagaaaggatatgcgagcgcccgtcgatgaccagcgtcacttcgttatcggtaaaaccttgccccgcctccagactttcttgcatcagctcgatatttaatgagaagtagctcaacagttccggtaacggtgtaccaaacaatttgcgggagctttgggcgagcagttgttgcgcggcagggttggcgtaatggatcgccaggttgtcatcgattaacaaaatactgttaatcagcgagttgaggatctgcccagcatcgggctgcgtgcctgttgccataaagcagtctcctgaacaggttgcaccattttagtgcattatagctttttacggataaaaagcgcgaagcatcagagaattgacggagaaaaaagcccatgcagagatgggctacagatagctgacaaacttcacgttggagagcgactcacctgctccggcctaccacatcatcaccgtgtaggccggataagacgcatttgcgtcgcatccggcgtgatgtgcttgccaccgatcccaggcctgccagagacaggcgaaaagtttccacggcaactaaaacacttagacgctgtagtacagctcaaactctaccggatgcggagtcatacgcacgcggtcatcttcttcgcgacgcagagcgatgtacgcatcaattgcttcgtcagtgaacacgccaccggctttcaggaactcgcggtccagatccagttcgttcagtgcttcttccagagagcctgcaacctgtgggatctctttcgcttcttctggcggcaggtcatacaggtttttgtccatggcttcgcccggatggatcttgttcttgataccatcaagaccggccatcagcagggcagcaaagcacaggtacgggttagctgccggatccgggaaacgtacttcgatacgacgtgctttcggagaagaaaccaccggaatacggatagacgcagaacggttacgcgcagagtaagccagcattaccggtgcttcatagcccgggaccagacgcttataagagttggtggtcgggtttgccagggcgttaatcgctttagcgtgtttgattacgccgccaatgtagtacagcgcctgctcagacagacctgcgtatttgtcgcctgcgaacaggttaacgccgtttttagacagagacatgtggcagtgcataccggagccgttatcaccgaacatcggttttggcataaaggtcgcggttttaccgaagcggtgcgctacgttgtgcacaacatatttgtagatctgaatttcgtcagcttttttggtcatggtattgaagcgggtagccacttcgttctgaccagcagtcgctacttcgtggtgatgggcttcaaccaccagacccatctgttccatcaccagacacatttcagaacgaatatcctgagccgagtctaccggtggaaccgggaagtaaccgcctttcactgccggacggtgacctttgttaccaccttcgtattgggtggaggagttccatgcgccttcgatatcgtcgatagcaacgtgggaaccggagatagatgatccgaaacggatgtcatcgaacaggaagaattcaggttctggcccgaacagtacggtgtcggcaatgccagtggaacgcaggtaatcttcggcgcgcttcgcaatggagcgcgggtcacggtcatagccttgcagggtgccaggttcaaggatgtcgcaacggataatcagggtggagtcggcgaagaacgggtcaatcactgcggtggatgcgtctggcatcagcaccatgtcggactcgttaatgcctttccagccgccaatcgaggagccgtcaaacattttgccttcttcgaagaattcagcattcacctgatgagcagggatagtgacgtgctgttctttacctttagtatcggtgaagcgcaaatcaacaaacttcacttcgtgctcgttcagcatcgtcagtacgtgttcagcggacatactttaactctcctggattggtcatggtcgtcgtggtaacgaaatctgcaattattttggccgtgtcgccgtaaaaaagataaagcgaaatctgtgccaacttttaaattgcccctaaaaggcgttatcatgcgcaccatcgtgcaaaagggctgcaccacgatgtgaatgttgcaccaatatagtgcttcaatggaaacattaagcaccatgttggtgcaatgacctttggataaccctttttatgctccgtgaaagcgatcacaaagggactctgcaatacttgtttgcggaggatgtttgtgatcctgttttgtagtgcgattaatccgtgtacaataacgcgctatttctaatgcctgaggcaaagttgtgatcgaaaaattgcgtaatatcgccatcatcgcgcacgtagaccatggtaaaaccaccctggtagacaagctgctccaacaatccggtacgttcgactctcgtgccgaaacccaagagcgcgtgatggactccaacgatttggagaaagagcgtgggattaccatcctcgcgaaaaacaccgctatcaaatggaatgattaccgtatcaacatcgttgataccccggggcacgccgacttcggtggtgaagttgaacgtgtaatgtccatggtagactcagtgctgctggtggttgacgcatttgacggcccgatgccgcaaacgcgcttcgtaaccaaaaaagcgtttgcttacggcctgaagccgattgttgttatcaacaaagttgaccgccctggcgcgcgtcctgattgggttgtggatcaggtattcgatctgttcgttaacctcgacgcgaccgacgagcagctggacttcccgatcgtttacgcttctgcgctgaacggtatcgcgggtctggaccacgaagatatggcggaagacatgaccccgctgtaccaggcgattgttgaccacgttcctgcgccggacgttgaccttgacggtccgttccagatgcagatttctcagctcgattacaacagctatgttggcgttatcggcattggccgcatcaagcgcggtaaagtgaagccgaaccagcaggtcactatcatcgatagcgaaggcaaaacccgcaacgcgaaagtcggtaaagtgctgggccacctcggtctggaacgtatcgaaaccgatctggcggaagctggcgatatcgttgcgatcacgggccttggcgaactgaacatttctgacaccgtttgcgacacgcaaaacgttgaagcgctgccggcactctccgttgatgagccgaccgtttctatgttcttctgcgttaacacctcgccgttctgcggtaaagaaggtaagttcgtaacgtctcgtcagatcctggatcgtctgaacaaagaactggtacacaacgttgcgctgcgcgtagaagaaaccgaagacgccgatgcgttccgcgtttctggtcgtggcgaactgcacctgtctgttctgatcgaaaacatgcgtcgtgaaggtttcgaactggcggtatcccgtccgaaagttatcttccgtgaaatcgacggtcgtaaacaagagccgtatgaaaacgtgactctggacgttgaagaacagcatcagggttctgtaatgcaggcgctgggcgaacgtaaaggcgacctgaaaaacatgaatccagacggtaaaggccgcgtacgtctcgactacgtgatcccaagccgtggtctgattggcttccgttctgagttcatgaccatgacttccggtactggtctgctgtactccaccttcagccactacgacgacgtacgtccgggtgaagtgggtcagcgtcagaacggcgtactgatctctaacggtcagggtaaagcggtcgcgttcgcgctgttcggtctgcaggatcgcggtaagctgttcctcggtcacggtgcagaagtttacgaaggtcagattatcggtattcatagccgctctaacgacctgactgtaaactgcctgaccggtaagaaactgaccaacatgcgtgcttccggtactgacgaagccgttgttctggttccgcctatccgcatgactctggaacaagctctggagttcatcgatgatgacgaactggtagaagtgactccgacctctatccgtattcgtaaacgtcacctgacggaaaacgatcgtcgccgcgccaaccgcgcaccgaaagacgattaatttcgttttttagtcataaaaaacctgccagcgatggcaggtttttttttgcctgtcgtgagcgcacaccaatgcgagtatctcccttataagtctgtggttacgtcaatagagagctttgtcacaattatctgcaaagtcatacgccgttaattgctttcttttttggcgtaagcgtaagatgcttcatctggtttaaaccaaaaggattaaacaatggcggagaatcaatccaccgtagaaaatgcaaaagagaaactggatcggtggttgaaagatggcatcaccacgccgggtggaaaactcccttcagaaagagagctgggagaactgctgggcattaaacgtatgacgctgcgccaggcgttgttgaacctcgaggcagaatccaaaatcttccgtaaggatcgtaaggggtggttcgtgacccagccgcgatttaattacagtccggagctgtcggcgagctttcagcgggccgcaattgagcaagggcgagagccttcctgggggtttaccgagaaaaaccgtaccagcgatattcccgagacgctcgcgccactgattgcagtgacgccatcaactgaactctatcgcatcaccggctggggggcgctggaaggacataaagttttctatcacgaaacatatattaatcctgaagttgctccgggctttattgaacaacttgaaaaccactcattttctgcagtctgggaaaagtgctaccaaaaagagacggtagtaaaaaaattgattttcaaacccgtcagaatgccgggcgatatcagcaagtatcttggcggttctgcgggtatgccagcgatcttaattgaaaagcatcgcgccgaccagcaaggcaatattgtccaaatagatattgaatattggcgatttgaggccgtagacctcatcattaatctgtaggtgttttatggtgacaataaataacgcaagaaagattctacaacgtgtcgacactcttcctctttatttacatgcttatgcctttcatttaaatatgcggctggaaagagtgttgcctgctgatttacttgatatcgcaagtgaaaataatctacgtggcgtcaaaatccatgttctcgatggcgagcgtttttctcttggtaatatggacgataaagaactctctgcctttggggataaagcccgccgtctgaaccttgatattcatattgaaaccagcgcctcagataaggcatctattgacgaagccgtcgccatcgcgttgaaaactggggcatcgtccgtacgtttttatccacgttatgaaggtaatttgcgcgacgtattatcgattatcgctaacgacattgcctatgtacgggaaacgtatcaggacagcggcctgacttttacgatcgagcagcatgaagatttaaaaagtcatgagctggtgtcgctggtcaaagaaagtgagatggaatctctttccttactgtttgattttgcgaacatgatcaatgcaaatgagcatcccatcgacgctttaaaaacgatggcaccgcatattacccaggtccatatcaaagatgccttgatcgttaaagaaccgggtggcctgggtcataaagcctgtatttcaggtcagggtgatatgccgttcaaagcgttattaacgcaccttatctgcctgggtgatgatgagccgcaggtgacggcatatggcctggaagaagaggttgattactatgcgccggcgttccgctttgaagacgaagatgataatccgtggatcccttatcgccagatgagtgaaacaccattgccagaaaatcatttactggatgcgcggttacgtaaagaaaaagaagatgcaattaatcagataaatcatgtgcgtaacgtactacaacaaatcaaacaagaggcaaaccatcttctgaaccactaataagttttaactcatacgcagttaataaaaccattccatatgaatggtcggtatcttattgcctttaaaacagtgattttaaaaatcgcttaggggatgttatgctcacgaaaaagaaatgggcgttatttagtctattaacactgtgtggcggtacaatttataaattaccgtcgctgaaagatgcgttttatatcccgatgcaggaatatttccatttgaccaatggtcaaattggtaatgctatgtcggtaaactcatttgtcaccacagtgggcttttttctgtctatttattttgccgataaactaccgcgcagatacaccatgtcattctcactcattgcgacaggattactgggtgtttatttgacgacaatgccggggtattggggcatcctctttgtctgggcgctatttggcgttacttgcgacatgatgaactggccggtcttgctcaagtcggtaagtcgattgggcaatagcgaacaacaaggtcggttgtttggcttcttcgaaacagggcgtggcattgtcgataccgtggtggcattttctgcgttggcagtatttacctggtttggcagtggcttattaggttttaaagcaggcatctggttctattcccttattgtgattgccgtaggcattattattttctttgtcctgaatgacaaagaagaggcaccgtccgttgaggtgaaaaaagaagacggagcatcgaaaaacaccagtatgacctcggtgctgaaagacaaaactatctggcttatcgcttttaacgtcttcttcgtttacgcggtttactgtggcctgacattcttcattccattcctgaaaaacatctatctattgcccgttgcgctggtgggggcttacggcatcattaaccaatactgtctgaaaatgattggtggaccgattggtggcatgatttcagataagatcctgaaatcgccaagtaaatatctatgctacacctttatcattagtaccgctgcgctcgtactgttgattatgctgccgcacgaaagtatgccggtctatttagggatggcatgtacgctgggctttggcgcgatagtctttacacagcgagccgtattttttgcacctatcggcgaagcaaaaattgctgaaaataaaacaggtgcggcgatggcgttgggtagctttattggttacgctccggcgatgttctgcttcagtctgtatggctacattctggatttaaatccggggattattggctacaaaatcgtgtttggcattatggcctgcttcgcattcagtggtgcggtggtttccgtaatgctggttaagcgtattagccaacgtaagaaagagatgctggcggctgaagcttaattaatggccggatgtgcttaatccggccaacgaaaaccgtatcaaccgtaggccggataaggcgtttacgccgcatccggcagtttcacatcagaagaaatacttcgtcccgatacggatctggttttgctcgcggtggtacggttcgacgttgcggtctaaccagcgcaattcgaaataagggagccagtgttcattaatacggtaacggaaggtgttagtgatttcccaatgatgatctttcccgttgctactattaaagtcattcactcgcatgaagtaatgtggctcaaatgtataggaaaatttatcggtgattttaaaattccagtaggtgccaatttcataggtgtcattattatccagttccccgctcaaatctgttgaactatagttattatggttatagcgatttcgtactgtcagattaaaccatggtacaaatttatagttgacgtccagatacactgcaccacccgaaccgatactcttatcattaattaagccaccgggctggatggttaatttatcggttggtttaaataacggataccagccttcaatttcgttatatccatgttttagttcatcttctcgctgaaagttgtaggtattggttaacataatacccgcgcccatatcgaagttataacccacacgtagcataacctcgccctgatcggaggcaagattatatgcctccctgttttcgacgtatgcgccagcaaataccgaggcagaggtcagagaagataataaaattattgcattaatctttttcataataagtccattttttaaacgtagggaggccgccacccaccaggatggaaatagcggctattgacatttataacgttacggaagccgttttttcttctgtcgccatctctttatttttgcgttggttgatttcctcaataatcaatgcaaaccgtttttcattgagtgtgtaaaagaatcccatcgtcaatgcagcaataattgccagtgcacaaggccagataaaaatgagctgacgcaaaccctgtaatgtcgcatcgctttgcgcgatgttgggaacataaccaatttgcgtcagcataatgcctggcaagaagccagcaagtgcggcagaaattttacgaaagaaggtataaccggtataaacagaaccttcggcacgaataccggttttccattcaccgtaatctacggtatctggtaccagtgcccagttcaggctgtttacaaaggccgtgccaaaaaaggcgacacaagagaacatgacgaaagtgaaagagttacttccccagaaataattcagtatatcacccaccgcccacagcaccatgccagccagataaacctgttttttaccaaaacattttacagttaatggcaccagtaatacgccgatgaggatgcatcccatactgaagaatcccatccacgacaataaattaatatcattcagcacatactgggtgtaatagacctgaatcgccagtttgatattaaatgccgccagggtacacaagttagcaatgcataaaaccagcaatggcggattccgaaatatcgcgcaaaatgatttgagaatactggctttatgtccggttggcgttgtgtccacataatgctctttgacgcctctgtagcacagcatcataaaaataaagccgccaatggagaacataagtgccgcacaggcataaccgacggttgagtcagaaaaaagcgactgcaacggaataaacgccacggtacaaatcaatagccctatggttgcaccaccctggcggtaagccgcgagctgcgcgcgctcattcgggtttttggtaattgccgggatcatcgcaccatacgagcagttcatcagactgtatgaaagtccaaacatcataaacagcgcggtggcaatcgtcgttttaaccggcaaacaaaaggtggtggcgataaactggagcgttgcaattaacgccgccggaaccgctgcatataaaataaagggacgaaatttgcctttaggcccaatatttttccgcgagtcgagtaaaaatccggtgagcatatcggtaaacgcggtaaaaaacttcgccaccagaaagataatcccgccatagtaagcaggcatccctaattcatcggtataaaatttgaggagatacagagtaccgatgcagagcattaaattcgaaccgacgtcgcccataccataggcgattttttcccgcagattcagttttaatgtcagtggattatggtcagacataatcactccttataacgccccgcagggcgtcgtttattattattacgccgtgcgtttacgggcttctatctcttccacaatgcggacatacatcttctcgttcaggctgtagaagcaacccatcgccacaatggtgactaccgccagtgcgcttgggtagatgaagatcaactggcgtaacccttcaatggtgtggtcagcctgtgcgacgttcggcacatagccaatttgcgtcagcatccagccggggaagaaaccagccagcgcctgagacactttgcgaaagaaggtaaaaccggtgtagaccgttccttccgaacgcacgccggtgcgccactcgccgtactcgacggtgtcggaaaccagcgcccagttcaggctgttaacaaacgctgagccaaagaacgccaggcaggagaacgccacgaagctgaccgaaccgccgccgaagaaatagttgagcagatcgcccagcacccaaatcagcaggccgccgatataaactttcttcttgccaaaacgtctgactgaggcaggcatcaggaatacgccgatgaaaatacagcccatgctgaaaaatcccatatacgacaacaggatgggatcgttaagcacgtactgggtgtaatagacctggatggcgagcttgacgttaaacgcccctaaagtgcagaggttggcaatgcacagaatgaacagcgggcggttacccgcaattgcgcggaaagattgcagcaggcccggcttttgcgccggattagcaggctgggtttcgacataacgctctttcacgcccgagtagcagatccacataaacagcaggccaaacagtgaaaacagcgtggcggcgaagatatagccaagttgctgattaccttcgataagattcataactggcacgaatcccaccgtgcacagcagcaggcccagcgtagcgccgccctgacgccatgccgccagtgaggcgcgttcgttggggtttttggtgatagcgggaaccattgcgccgtaggagcagttcatcatgctgaaaaacagtccgtaaagcataaacagaatagtggccatcaccgttttaccggtgacatcaaacggtgtgccgacaaagttggcgatcgccagtaaggtgaccgggaatgacgcatacagaataaaaggacggaacttaccttttggaccgatcttgcgtcgggaatccaacataatgccggtacccatatcggtaaacgcagtaaagaattttgaaatcaaaaagataatgccgccataggtgcctggcagccccagaacgtcggtataaaacttcaaaagataaagcgtaccgatatccagcaggatgttagaggccaggtcgccaataccgtaagagagtttctctttaaagggcaggcgtaaagttgctggatcttccgttgtgatgtgactcatcgatgttctccctttgcccatgagtttccccacgggcggatgtgattagatgctttttaacgacgcgaacagtgccgcccattcgctatcggcgcgataaaagaccggcggcttgccgatgggcgcattaacggtaacttccccgccccggaacgcttcacccgtccaggcgtggacccagttatcctccggcagatagagcgtccagtcgctacggccttcttcatgcaccggagcgaccagaatgtcgcgacctaacaggtactgatatttcagggtgtaagtgtgcgcatcgtcttcgtaatgcaggaacagcgggcgcataaccggcaggccggacttcgcattcagcgcgacggcctctttcaggtaaggtttcagggtggtgaagacggtggtcatacgggcgaaatgggcgatggtttctgcgtcgccgtcaaactgccagttgtcgccaggacggttaccttcgtgggtgcgcatcatcggcgtgaaggcgctgaaatcgcaccagcgcagcagcagctctttgctgcgcttcatctcaaacagggtggtgtaaccgccaatgtcgctgtggtgcaggccatgtccggtcattgccagcgacagcgccgccgggacaaccgacgccaggccatcgtcgagactccagtcgacgttctggtcgcccgcccacatcatggtggagtatttctggctaccggtagaaccggcgcgcataaagaaaaggatctcgccgagcttgcccgtttcttcaagggcttcgtagttacacttcgcccacagcgcaggccaggcgttatgcataatttcggcactgacgccgttatgcaagtacgtgtcggtgggcagatactcgccgaagtcagccatccagccgccgcagccgagttcaatcatgttctttttgatcacttccttgaaccaggcgtaggcttctggattagtgagatcgacaacgccgccgtaaaactcgccaaactccaccagatagtcaccgccagaggcatcttttgccagatagccgtgttgtgccgcttcttcgcagagatctttatcgctggcaacatacgggttgatataggccaggaactgcacgccctcctgattccactgcttaatgcgtgaatccagttgcgggtagttttcgctgttccacttccagttccacatcacgcgtttgccaaaagaggtcatacgaataccggaccagtcctgcgcccagatgccgttgaccttcacgcccgcgttacgcatggtgtccagtttcttctggcacacttccgtcccgccctgaatgccgagcgttactccgtcataaatccagtcgggcagttctggctggcgtcccagcagggcggttaatttttccagcagggaaatgtatgtgtcagcacattcaaaacgcagcgttgctttgtcttcccacagcgccagttcatggtattccggggcactaaagtcgaagttcatatagcaactgttatcaacatggcagtaatacttctgcgtgctgacaaacgtaggctgtgggaagaaagtccagtaatagtcgccgcccgcattttctttgcagtcggcctgccaggtgacataggtttgtttgttgcgaccaacgccttgttcactggtccatagcgggaacggtttgccacgcagatcgaagtaggaaaactgttcgccgcagccgtagatatggtcctctggttgagcggcaaggcgcagccagatacggttgtggttaaggttgtcgttttgtagttccagcaataaacgcccctgatcgtcggcagagatattcagcgtggcgctaatgtcagaaccacggctgaaatgaattaaccaaccatccggtgactggctgacgatggcgtcggtaagcgcaattttctcctgtagtttatctttaatgctgaaattaccgcggaacatatcgatatccgctatacctgagccaatccataaacaaggattatctttgctatgggttaaaataagacgttgttgaaaatgtagggtaaaactgtcgttattctgatgaaattgaaaatctaataactgtggacgtggcgtatccataactaatctccatagagttgagaacgagattgttgccttcctgttattacaggcttatgtaaaatgattctcataaaactgatatataaaaactttacagaagctgagctgtttttaacttaataaattgaagatacataatgttgcctttagcgagtgaaatgttcttcaatgattttgactgctaatcaatacaagttattttctctgtccgtaaatattaaaaaacaggcggtgcggttttcctgattccagtaataataagtcgatacctgaattaaaggcgttaggcgggcaactcataggttcaactgccagtccctgacgctgtaatttttcaccgctataaacctgcacccagagttgatcggaacaaaggcttaccgaaagcgcctgctgtggatgggtaatggtcatttcccacaaatcattagcggttttaaaggtgtggtcgatttttgtcgcggctatttttttcgcctgcgtgaaatttaaatccagctcatcaacgtggtgaagcgttgtcggattcgcgtgctcatcgacggcataaacctggtttgccggaagctggaacagatattcatcaacagatgttaagttgcaggttaaataaggatgaatacccacgccataaggcgctgcgacagtgccgatattctggcttgcgatctcaacggaaagacccgtgtgtgcgttgagcgaataaacaacttgtgaagccagcataaacggatagccgtaactgggcggcagaaaagctgtcagggtaacgctggtggcggttaattcactaatttgccagtctcgccaggcaagcagcccgtgaatagcggcttttgaactatgttcattaatgggtaactgatattcctgcccctgatagcggtaacagccgttggcgatccggttcggccacggaataagcactttacccagatgcgccagcggcatctcttcgggtttgtgcgggatgactaaatgacaaccctgaaaggttaattcagccagaccagcaccgacggtcacaatggtcgcgtgataatcccccgcggcaagtgaaacggtctgtccactgcaatgcatattggtgatttgcatacaaggcaccttaattaacgacatacagcctcccgtgaggctgatgtcaaacccaaaaactgcaccggacggtcccctcgcccctttggggagagggttagggagaggggaaaacccgcaccctattttcagatcagttatttcgcattaatatccagcagacccgctgcaaccgctggagccatgccgggcgctaacgggatacgcgggatcaccaggcaatgcagcaggtgataaatatcctgtttgccgtcccagactttggtggtgaccttattgtccgcatccagctcctgccaccaggaaccattttcatagtccatcaggtacttaatgcagtactcccaccatgtttgataccaggtttcatactggcgatcgccagtgacggtgtagagcgcgtaggccgtacccattgcttcgacgataggccaacgtacacgttcgcggaccaccggttttccttcccagtcaacggtataaacaatcccgtccgcgccatcgggtgcccaggcatcgcgcacggtggcgttaaacagacctttggcatcttctagcagccatgctggtggttgttcgcaacgggcttccagggcagcatggatgtgcagcattaaacggccccattcgatccagtggcctggtgtacctccgaacgcgcggaagcgatgcgccgggttatctttgttgtaatccggcagcggattccactgggtatcgaagtgttcgttaacgcgataatgattatttctggcgacgtcgtggataatcacggaagccacgcgaatcgcgcgatccagccattttttgtcgtgagtgacgtcataaacaatcaagaaagcttccaccgcgtgcatattggcattgccgccgcggtactcttcggttttgctgaaggcttcgtcccaggattccaggcacatctgctcttcttcgctccagaaatatttctcgataatttcaatggtgtaatcgagcagcttgcgcgcttccgggtgacccgttgtgacggcgctggcggcacccagcagagcaaagaagtgttgatagccctgtttggaggcatccaccacgccctcgtcattcacgcaggcataccagccgccatattttttatcacgcagtgcgccgttcatggctttgataccgtgatcaaccaacgagtaagcgccaggtcgacccatcgccgcagcaacggaataaacgtgcaacatacgagcggtgatccacagatgggtgcccatctcttctttgatttgccctttattgcctaaccagccaaaaccagtcggcactacggaatttttaccaaaatcaaagatgcggtcggtttcctgttccagccaacggttgtggcttagggtgttaaaccatttcattccttttatcctcatcttagcggcgtttagccatcatttcgtcgacgatatcgccaagttgttgtaatttcggtgcgcaaacgtcacgcagcatcagctcgttgtctggtaaaccgacgaccgatgcccagactgcacggcctgccaggaatcccgatgcgcccgccgtcattgccacgcgtacggcacgcgggaacagtttttcgtcgacaccggaagagaggatcacccatggcatattgatatggtcattcagacgttgtgaagcacagagaagctcttgttgcggacctttgccataaagcggcatttcaactttgtagaggtcagcgccactgtcgcccagctctttggcggcatcgatgatcgcttgttcgcgatcgaatttatcgccacgacgcggtgggcggacgactggctcaatgatgcttaccagaccgtgtgagtggcacagttcgttgaactctttcaccatatccagacgttgctgcgcatcttcatcactacgccacagcaccagcagttttaaggctttgccaccgtcttgtttgatctgtagcggattgattttgcggtcaataaccacgctatcgaccggaataccgttgccaggaatgaactcatcggcggcgacaatcatggcgcaacttttggcaatcgcgttttgctcaaccacctggcggtagcagaattgttgatctaccagaatcgccgaggcataaggcgagagggcctttgcagcgttaactttgaaatcagttaaaacgctatcggctaccggagcgggtgccccagccgcggcaaacatcatgcgcatggcttcgcgctgatcgaccgccagcatggcaaaaccgcccgatgcgcgcgtaatgtcgttgatggtgtacttattcattcatttattcctttatccagtcgttacatttttactttggcagtcatcccggcactgacacggacctgttccagaatggcggaccagtcctggcgaccgcgacccgctgcgcgcgcctggctataaacctcccgtgaggcggcccccagcggcattggcacatgcagctggttggcgacatcaagggcgatgccaagatccttatgggcaagatcgatcatgaaggcgggagaaagatctccgctgaggactttgtttggccaggaagtggtgaagtgacctttaccggcggcggtaccgctcatcactttgacggcaacatcgaagggaagattcagggcttcgcacaaaacggcggcttctgccgaaagcgcattgagcgcgatgctcatgtagttgttgatgagcttaacgcggatccccatgcccggaccgccagcgttgatcaactcactgcccatcgccatcaggatcggtgtggcacgttcaacttgttcagcggtgccgccagccagcagtaacagagtaccggtaatggcatttgcagaagtacggcctaccggaacatccatcatgctgaagcctttggcttgcatatcggcaatcaatttatcggtttgcagcggatggatggtggacatatcaatgaccagcgcatcggtagataagccttcgcaaacgccgttttcaccgaacaacacgttgcgcaccagatcgccattcggcaacatggtaatgataaattcggcatctttagcggcctgcgccgggttggcggcgggagtcgcacctttgtctaccagatgccgcacagcttcggcgttcacatcaaagacgcgaagttgatgcccttgctgcaataaattgctcgccattggcgaacccatttgtcctaaaccgataaacgcgattgctgccataaccctctcctgaatacagttatgtcactttttgtcatttatgacatgctttgcttgtctgtttttgatcgtatttgtaatttatcgtcaaaaaattgacagccgtcactttttaaacaattggtgaaattaaaatgaacgcatcccaaaatgtttaaggaatgaccatgattcgtgttgcttgtgtaggtataaccgtgatggatcgcatctattacgtggaagggttaccgacggagagcggtaaatacgtggcgagaaattatacggaagttggtggcgggccagcggcgacggcagcggttgcggcggcaaggctgggggcgcaggtcgattttattggtcgcgtaggtgatgacgacacgggcaacagcctgctggcagagctggaatcctggggcgttaacacccgttacaccaaacggtataaccaggcgaaatcttcgcaatccgccatcatggtggataccaaaggcgagcggataatcattaactaccccagcccggatctgctgcctgacgcagagtggttggaggaaattgatttctctcagtgggatgttgtgctggcagatgtacgctggcacgacggcgctaaaaaagccttcaccctggcccgtcaggcgggtgtgatgaccgttctggacggggacattacgccgcaggatatcagtgagctggtggcattaagcgatcacgcggccttttcagaaccgggtctggcgcgcttaacgggcgtgaaagagatggccagtgcgctaaaacaggcacaaacgctcacaaatggtcatgtctatgtgacccagggtagcgcaggctgcgactggctggaaaatggtgggcgtcagcatcaaccggccttcaaagttgatgtggtagataccacaggtgcgggtgatgtttttcacggcgctttggcggtggcgctggcaacaagtggggatttagcggagtcagtccgcttcgccagcggtgtagcggcgttaaaatgcacacgtcccggtggacgagccgggatccctgactgtgatcaaacccgatcttttttgtcactttttgtataaaatgccagggtgatggtttttcgaggaattttcatgagccttaccgaactaaccggtaacccgcggcacgaccaactcctcatgctgatcgccgagcgtgggtatatgaatattgatgagctggcaaatctgctggatgtctccacgcagacggtccgccgggatattcgtaaattaagcgagcaaggcctgattacgcgccatcacggtggcgcgggtcgggcttccagcgtcgttaatacggcgttcgagcagcgtgaggtttcgcaaaccgaggaaaaaaaagcgattgccgaagcggtggcagactatattcctgatggttcaacaatatttatcaccattggtacgactgttgagcatgttgcccgggcgttacttaaccataatcatttgcggataatcaccaacagcctgcgtgtggcgcatattctttaccacaacccgcgctttgaagtgatggtgcccggcggtacgttgcgctctcataatagcgggatcattggcccttcagcggcgtcctttgtggctgattttcgtgctgattatctggtaacaagcgttggggcgattgagagcgatggcgcgttgatggagtttgatgtaaacgaagctaacgtggtgaaaacgatgatggcgcacgcgagaaatattctgctggtcgccgatcacactaagtatcatgcttcggcggcggttgaaattggtaacgtggcacaggtcactgcgctctttaccgacgagctgccgcccgctgcgctaaaatcacgcttacaagacagccaaattgaaatcattcttccccaggaagacgcgtagatttttgtgaccgttaacctggcttcataccttgccacatagccaaacccatcctttcccgctacagttaatttcttgtggcgcgaaaggaggcaaaaatgctctatatctttgatttaggtaatgtgattgtcgatatcgactttaaccgtgtgctgggagcctggagcgatttaacgcgtattccgctggcatcgcttaagaagagttttcatatgggggaggcgtttcatcagcatgagcgtggggaaattagcgacgaagcgttcgcagaggcgctgtgtcatgagatggctctaccgctaagctacgagcagttctctcacggctggcaggcggtgtttgttgcgctgcgcccggaagtgatcgccatcatgcataaactgcgtgagcaggggcatcgcgtggtggtgctttccaataccaaccgcctgcataccaccttctggccggaagaatacccggaaattcgtgatgctgctgaccatatctatctgtcgcaagatctggggatgcgcaaacctgaagcacgaatttaccagcatgttttgcaggcggaaggtttttcacccagcgatacggtctttttcgacgataacgccgataatatagaaggagccaatcagctgggcattaccagtattctggtgaaagataaaaccaccatcccggactatttcgcgaaggtgttatgctaaaaaccattcaggacaaagccaggcaccgtacccgtccactatgggcctggctaaaactactctggcaacgcattgatgaggacaacatgacaaccctggcaggtaaccttgcctatgtgtcgttgctctcattagtgccgctggttgccgttgtttttgcgcttttcgccgcttttcccatgttttccgacgtcagcattcagttacgtcactttatttttgccaactttctgcctgctactggcgatgttattcagcggtatatcgaacaatttgttgccaattccaacaagatgaccgccgttggggcgtgcgggctgatcgtcaccgcgttattgttgatgtactccatcgatagcgcgttgaataccatctggcgcagtaaacgagcgcgaccaaaaatttactcgttcgccgtgtactggatgattttaacgctggggccgctgctggcaggggccagtctggcgatcagttcctatttgctctccctgcgctgggcgagcgatctcaatactgtcatcgacaacgtgctgcgtatttttccgttgctgttgtcgtggatctccttctggttgctgtacagcattgttcctaccatccgcgtacctaaccgcgacgcgattgtcggcgcgtttgtcgccgcactcctgttcgaagcaggaaagaaaggtttcgcgctttatatcaccatgttcccgtcatatcagctcatttatggtgtgctggcggtgatccccattctctttgtttgggtctactggacatggtgtatcgtcttgcttggcgcggaaattactgtcactctcggggaataccgcaaactaaaacaagcagctgaacaagaagaagacgacgaaccatgattgcattaattcaacgcgtaacccgtgccagcgtcaccgtggagggagaagtgacgggcgaaattggcgcgggacttttggtgttattgggtgtcgaaaaggatgacgacgaacagaaagcaaaccgtctgtgcgagcgtgtgctcggctaccgcatctttagcgatgccgaaggcaagatgaatctcaacgtgcaacaggcgggcggcagtgtgctggtggtttcccagtttaccctcgccgcagataccgaacgggggatgcgcccaagtttctccaaaggtgcatcaccggatcgcgcagaggcgttatatgactatttcgtcgaacgctgccgtcagcaagagatgaacacgcaaacaggacgcttcgctgcggatatgcaggtatcgctggtcaatgatggccccgtgacattctggttgcaggtatgagccagcttccagggttgtcacgggaaacaagagagagtatcgctatgtatcaccttcgggttccacaaacagaagaagaattagagcgttactatcagtttcgctgggaaatgttgcgtaagcccctgcatcaaccaaaaggttcggaacgcgacgcgtgggatgcgatggcgcatcaccagatggtcgtcgacgagcagggtaatctggtggcggtaggccgactgtatattaatgccgacaatgaagcgtccattcgctttatggccgttcatcccgacgtgcaggacaaagggttaggcacgctgatggcgatgaccctggagtcggtggcgcgtcaggaaggcgttaagcgcgtgacctgtagcgcccgtgaagacgcggtggagtttttcgccaagctggggtttgttaatcagggagaaatcaccacgccaaccaccacgccgattcgccattttttgatgattaagcccgtcgccactctggatgacattctgcatcgcggcgactggtgcgcgcagctgcaacaggcgtggtacgaacatatcccgcttagtgaaaaaatgggcgtgcgcattcagcaatataccgggcaaaaatttatcactaccatgccagaaaccggcaatcagaatccgcaccatacgctgtttgccgggagtttattctcactggcgacgctcactggttggggacttatctggctgatgctgcgtgaacgccacctcggcggaacgattattcttgcggatgcgcatatccgctacagcaagccgattagcggtaaacctcatgcggtagccgacctcggtgccttaagcggcgatctcgaccgtctggcgcgcggacgaaaagcacgggtgcagatgcaggtcgaaatctttggcgacgagacgccgggtgcagtgtttgaaggcacgtatatcgttctgcccgcgaagccatttggcccgtatgaagagggcgggaacgaagaagagtagctgatggagaggggcggtgctgcctctctcattcaggtcatttatattagtccttggctatttcggttatattaaataagaactctataaatttttattcttcgttggctccatacgtgtcttgctacatcactgttcaggagcatttaaatattatttgtagaactgagtggcaattatcgcagataatgcttaattcatcatcttagttcatgtttgagcgatttttgatagtcaaaaccccctctggtgccatacttttctcataaatatttttaaaatctatagctaacaaatattatgcaaagataatggactagcatcattgtcagtatcattcatttactgctctgtatgttatgaataattatgttgtatgtttgctcttaaaccgtgggaaggaggctataatggttgccaatattaatctcattaaacaagaaagttattctgttgttaatttagaaaaacaactttcccgaactgttaccaacaaaattataacgatgagcaagtaaagaccggttggtggcagtactgaccggtctgtgatgaaagattaatttcaccttaaatcctggtgctgttaggatgctgacgtttttcggctacaccattcagattatgcaaataaatatctctgaatataatatattcatagcacccataattcatcctgggcgataactaaaccatttttgagtaataaatgaaacaactgcaacactcttattatttctggaaaacgcctcgcaaaaacaaaacaacatgcaaaaatccgctttttttaaatgattttccggcgtaattttcgcacatacattaatgagtaatatatgtaaggtattggtaatggcgatgaatacggtttttcttcatttatcagaagaggcaattaaacggctgaacaagcttcggggctggcgtaaggtttcacgatctgcaattttacgcgaagcggtagagcaatatctggaacgtcagcaattcccggtgcgtaaagcaaagggaggcaggcaaaagggggaggtagttggtgttgatgatcagtgtaaggagcataaggaatgacaaaaatttttcattcttgaatataaaaaacagatgcccttattctggtattaatacaaggctgttttacttgaacttataataactgcaactgttacatcatatctggaaaacgcctcgcaaaaataaaaaatgatgcgtaaatgagctttctttaaagattcggcaagggtacttttctctccatagattcaaaaatgatattggcgagatatttatgaactctctggcaggtatagatatgggcagaattttactcgatttatcgaatgaggtgattaagcaacttgatgatctcgaggtgcagcgtaatcttcctcgtgcggacctattaagggaagcggtagatcaatacctgataaatcaatcgcaaacagcaagaaccagtgttcctggcatctggcaagggtgtgaggaagatggtgtcgaatatcagcgtaagctgcgcgaggaatggtaatgggaaaaaatgatgtcaatcagattgctgacaacgtgcgcgttgttcatgccggatgcggcgtgaacgccttatccggcctacaaagtcgtataaattcaatgtattgcagtttattggtaggcctgataagcgcagcgcatcaggcaatcttacgcttgtcatcagtctcatgcccataaccttattgatgtggtggtgggtaaattgaggccaaaccggcactggcggcatagcttgaggtggtaacgcggaatacgagagatggtgtcgtcacaccctatgagctgtaatccgggcgacctgcgccacccggaaaacgtcagagattactctccttcacccggaaacaggaacgggttgatggaactgcgggcatagccttcttgctccattcgtgcgtccagtaccagagaggcgaggtcatctgctacggcttcgatttttggatctttttcctgatagagaattttcaggtaagtgtcgcagtcatcgcagctttcggctttaatcgcggcctgttcgtcatccagcgaccagtaatgcagtttgccgctctgctcgcagttgctgcattttacgcgcactacgtgccattcagtttcacacaggttgcagtgcaggtaacgtagcccctgagtggtgccaatttgcaccatgctggacaccggcatagaaccacaaaccgggcaatattgacgttgctcgccgtattcagcgcgggctttgccggggatcagattggccatctgcgcccagtagagcgacagtgcagcccagataaacggcgctttatcgctgctgacggacgagaaatcagaggcaaacagcgcgctggccatatcttccagctcctgagtcgatgccttctccagattctcaatcactgccagcgccgggccgctcatttcaggtttcagctcagcaatcagcgccatcagcagcttttgccagtgcttatcacgcggcagaacgtgaatatccagcgggggcttgccttgtgcgctggcttctttaatgcgcgcagtcagatccatctccagcggatggtcgtacagcaccacttcctgggcgtgggcgataagcgcagcaaagcgcaggtaatcacccagaggattattttctgccagctcgcgcagacgctcggcgcggcggttgtataaattcttgagccgagggaacaataacggcggaatcatatccgccgtacgtttctcgcttgaacccagctcatcttgcgggattatgcgaatactcattcagctttcttttccgttgtcttgcggacctcacggtaccagcgcgggtgatgtttcttcgcccaggcgctggtaacccatccttccaccatggcggtaatcgtgcctttcacccaaagggcggcgtagatatgcaccatgataaccacaattaacgccactgcggcaaatgaatgcagcattaacgcgaatcggatcaccgggattgagaaagcaggcgcaaaataaggacgccagataatcacgccgctcaccagcagcagaaccaggaaaataatcgccgcccagaaaacgcatttctgaccgaagttataacgcccggtgtcacctacttcctcgttgacgacgatcttacgaatattcttcgcccaaaagatatcatcccgattgattaggttgtgatgccagtaacggaaaaacatgatgatgaacgaggcaaacataaccacgccgacaaacgggtgcagaattcgcgccagctgcggtgtgcccatgatttgcatcaaccagttgaaggacgggaacaaaaagcccagcccgctcaccgccgccaggatgaagcagaaggcggtgatccagtggttgatacgttccggcgcggtgtagcgcacgatggtgtcacgtcgtttcatttgcgctcctcgtctttctcttcgtgcagattattctcttcctcatccgcacggttcggaccgacacccacgtagtggaagatactggccgcaaaggtagccgcaaagccaacagccgcgagcggtttccagatgcctttccagaatttcacggtttcgctgatttccgggttctccggcaagccatgatacagatttggcttgtcagcatggtgcagcacgtacatgacgtgtgtaccaccgacgcctgccggatcgtacagacccgcattgtcgtaaccgcgggttttcagctcagcaacgcgctcgctcgccagcgttttcatcgactctttcgtaccgaagtgaatcgcgcccgttgggcaggtcttcacgcaggctggttcttgcccaaccaccacgcggtcaacgcacagcgtacatttgtagacgcggttgtcttccgggttgaggcgcggaatgtcgaacggacagcccgcaatgcaataaccgcagccaatgcactgctcggactggaagtcgacgataccgttggcatactgaataattgcaccttccgccgggcacgctttcaggcagcctggatcggaacagtgcatacagccgtctttgcggatcagccattccagtttgtcgttctgctccacttccgagaagcgcattaccgtccacgatttggcgcttaaatcattggggttgtcgtacaccccaatgttattgccgacggtatcgcgaatgtcgttccactctgaacacgccacctgacaggctttacagccgatacaggtggtaacgtcgatgagtttcgccacttcttcctggaagtcccgcgcctgaggcgcgggggtcagaccgttagtcgcggaacgacgaatgatatcttgagattgataagccatatgtcgtctccgttacaccttttccacattcacaaggaaggacttaaactccggcgtctgcgtgttcgcatcaccaacgaatggcgttaaagtattggcaataaagccttttttagctacgccttcatagccccagtgaatcggaataccgatggtatcgatatctttgccgttcgctttcagcgtgcgaatacgtttggtcaccaccgctttggctttgatatagccacggttggaggagactttcacggtatcgccctgggcaatgccaagtttattcgccagcgactccccgatttccacaaactgctctggctgcaaaatcgcgttcaacagcgcgtgtttggtccagtagtggaagtgctcggtcagacgataggtggttccgacatacgggaacttatcggctttacccaatgcttcggcgtcgtctttaaagatacgtgcagccgggttcgagataacgtttggatgcagcgggttagttcccagcggcgtttcaaacggctcgtagtgttccgggaacggaccttccgccatcttatcgagggcaaacagacgccccatgccttcctgctgcatgataaacggcccgacgccgctacccggaggcgctgcgctgtagtccggaatatcccagccggtccacttagtgccgtcccatttcagcaactgacgcttcggatcccacgggttaccctgcggatctgcggaggcgcggttatacagaatgcggcggttaagcggccatgcccatgcccagcccagcgtgttaccgaggccagacggatcggcgttatcacggcgtgccatctggttgccttccggcgtccagctaccggcgaaaatccagcagccacaggaggttgtaccgtcatcgcgcaattgggcgaacgaactaagttgttggcctttcttgacgataaccgcaccggttgccggatcggtaatatcggccagcgccttaccgttgctctccatcgccacttcttctgaagatggctcatgcggaatggcgtagttccatgtcatgttcagcacctggtccgggttcgcgccaccctgttcggcatacatcttgcgcaagcgcaggaagataccggagaggatctcgccgtcagtcagcgcaatccccggggcgtccgcacctttccagtgccactgtaaccagcgacctgagttaacgatagaaccgttctcttccgcgaagcaggtcgatggcagacggaacacttcggtctggatcttcgacgagtcaacttcgttcagctcaccgtggttctgccagaagttagaggtttcagtgttcagtgggtcgatggtgacgaggaacttcagtttcgacagacaaccgatcactttgtttttgttcgggaatgaggcaacagggttaaagccctggcagatatagccattgaccttgccctctttcatcatctcgaagtattgcaggacgtcgtagcctttatcccacttcggcaaccagtcaaagccccagctattttccgccgtcgctttatcaccaaagaaggccttcatcatagagacgaagaatttcgggtagttgccccagtagtttacctggccttccagcagcggttttggcgtgttggcggtaaggtaggtttgcagatcggtctgcttctcgcttggcagcgtcatgtaacctggcaggctctgcgacagcagccccaggtccgtcagcccctgaatattggagtgaccgcgcagggcgttaacgccgccgcctgccatccccatattgccgagcagcagctggatcatcgccatcgtacgaatgttttgcgcaccaacggagtgttgcgtccagccgagggcatacaggaacgaggcagttttatcgtgagcactggtttctgcgatgtattcgcagactttcaggaacgcgtcttttggcgtaccacagatgttttcaaccacatctggcgtgtagcgggaaacgtgctgtttcagcaagttccacacgcagcgcggatgttgcagcgtggtatcgcgtttggcgaagccgttttcgtccagttcataagtccaggaggatttatcgtacttgcgtttttccgcgtcgtagccggtgaacaggccatcttcaaagccgtaatcctcacgcacgatcaggctggcgttggtataggcttcggtgtattcgcggttgaatttttcattgttcagcaggtacagcaatacgcctgacaggaaagcaatgtcagtaccggaacgaataggggcatagtagtcagctaccgccgccgtacgcgtaaagcgaggatcgatcacaatcagcttcgcgccgttgtgaattttggcttccatcgcccagcggaacccgaccgggtgagcttcagcggcgttaccgcccatcaccacgacgaggttggcgttcttgatgtcgacccagtggttggtcatcgcaccgcgaccaaatgttggagcaagacttgctaccgttggtccgtgtcagacacgcgcctggttgtcgaccgcgagcatacccagcgcgcgggagaatttttgcgttaaatagccggtttcgttactcgacgcggaagcacacagcatcccggtggagagccagcggttaacagtcacgccttcggcgttttgcgcaatgtagttagcatcgcggtcttctttcatcagtttggcgatgcgatcaaacgcctcttcccaactgatttgctgccatttatcagaacctggcgcacggtattccggaaacttcagacggctttcggagtggatgaaatccaccaggccagcgcctttcggacaaagtgcaccgcggttgaccgggtgatccggatcgccttcgatatggaagatagatgctttggcgttttttgctccgtcaccgaggctgtacatcaacagcccacagcctacggaacaataggtgcaggtattacgggtttcgcgggtgcgcagcagtttatactgccgggtttccgcgagtgctacgctgggtgcaaaacccagtgccgctgccgtggtgcctgccataccgccagcgcagatcttaaagaactgccttctgctgacctgcatggattgctccttgtttcgacattgtcacgtcccatttacattcgcttgctgcgtgtgcagggagtgggagttatttttctttgcggaaggggccgcaaaggtccagaattggctcaatttccctccatccaggaagggtttgtaacagaataccataatgttggtgtgtgtgttcttatctggttaagagaaagtgaaaaaaacacagcgaaaagaaatcgaaaatgtgacaaatatcacaggtgttcgtcaaattgagttatggcggcgtgatgatttacaacacccacggttagatgaggtcgcggaagaagttcccgttgcgctggtctacaacggcatttcgcatgtggtgatgatggcgtcgcccaaagaccttgagtactttgcgctcggtttttcgctttccgaggggattatcgaaagtccgcgcgatatcttcggcatggatgtcgttccttcctgtaatggtcttgaagtacaaattgagctttccagccgccgctttatggggttgaaggagcgccgccgggcgctggcgggacgtacgggctgtggcgtatgcggcgtggagcaacttaatgacatcggaaaaccggtgcagccgctaccgttcacccagacgtttgatctcaacaaactggatgatgcattacgtcatctcaacgattttcagccagtggggcaactgactggttgtactcacgccgctgcctggatgttgccatctggcgaactggtcggcgggcatgaagacgtgggtcgccatgtggcgctggacaaactgttaggccgccggtcacaagaaggggaaagctggcagcaaggtgcggtactggtttccagtcgtgccagttatgaaatggtgcaaaagtcggcgatgtgcggcgtagagattttgtttgcggtgtctgccgcgaccacgcttgctgtagaagtggctgagcgctgtaatctgacactggtaggtttttgtaaaccgggtcgggcaacggtttatacccatccgcagcgtttgagcaattaattaaaataagtcctgcgaaatatattaaattgcaggacttattcatttcgtgaattttattattttatttataaacaaaatgcgtgtagtggcgttttcttttttcatttattatgttcactctcttatctatatatttataaggcaattaaatgaaaaggaatttattatcttccgctattatagtcgccatcatgtccctcggtctgacgggttgtgatgataaaaaagccgaaacagaaacgctcccgcctgccaatagtcaacctgccgcaccagctcctgaagcgaaacctactgaagctcccgttgcaaaagcagaagctaaacctgaaacacctgcgcaaccggtggtcgatgaacaagcggttttcgacgaaaaaatggatgtctatatcaagtgctacaacaagttacagatcccggtacagcgcagtctggcgcgttatgctgactggctgaaagattttaaacaggggcctaccggtgaagagcgtactgtttatggcatctacggcattagtgaatccaacctcgctgagtgtgaaaaaggcgtaaaaagtgctgtggcgttaacgcctgcgctgcaaccaattgatggcgtggcggtgagttatatcgatgctgccgtggcgttgggtaataccattaacgaaatggataaatattacacccaggaaaattataaagacgatgcgtttgcgaaagggaaaacgctgcaccagacattcttaaaaaatctggaagcctttgaacctgtagccgaatcttatcatgcggcgattcaggaaattaatgataagcgtcagcttgcggaactgaaaaatattgaagaaagagaagggaaaacattccactactactctctggcagtcatgatttcagcgaaacaaattaataacctgatatcgcaagataagtttgatgcagaagcggcaatgaagaaagtgtctgaactggaaacgctagtggcgcaggccaaagaagcggataaaggcggcatgaatttctcgtttattaattcggcaggccagtatcaactcgaggctaaaaaatacgttcgccgcatcagagataaagtcccgtactctgactgggataaagagcaacttcaggacgcaaactcaagctggatggtcgaagactctttcccgagagcattacgcgagtacaacgaaatggttgatgactataatagcctgcgttaaacgtttttgatgataaatgcagtgtcggatgcggcgcatccgacacagttcaccccttgtgaagtaactccataaatgcctcatatcctgttaacccggcaataatctccgccggatgctgacacaatatgcttgccagatagctaaatatttttagctcatgacgcgcatcggcggcggcgcaggcgatcaagacatggttaatgacttcgttattcacctcaactggttgggcgagggtaataaaaaatccacgaaaacgtcgctcctgttcgctccagcaatgtgggatggcgaggcgattaacaatcaggttttcaccttcgccttcgcgggcgatgatgcgttgtgcttcatcggcggtaatatggtgttgtgcgactaattgcgcacaaatttgccgggtaatatgttgccagctttcaccgcgtacattcgaataatgaaaacttccgggggcagagaaaaaacgctccggctgttggcgaataaatgccgtcgccagaaaatgttttatttgttcgataccggcagccgtaatgatattttttacggtgatgtaattatttaccgcgtcatccagtaaataatggctgttgttaatgatcaataacggctcaatctcttcgcgaatggcaacaagttcgcttaagctacgggcaataattacccgacaatttaaaacatcgcgctcaatggcgagctgattaatagtggcaatcgcgttctggtccgagagcaaaatgatcggctggcgttcgttttgatgccgctccagcgcacaggcaaaatacaaaccgatcagatcgctgtcgaaaaggggaatatcgagctgttcacgcagtagcgtaataaagtgcagactcatatcaaaggccgcaggccaggcggctttcaggttattcatgctgctctggcggtgctcagcaatccacactggtgcggcaaggcaacgtaataaatgcccggtaatattctcaaccagctgcgcatcaataatattcaatgacgcgatgcccggcaccctttgcagcaacccctgcacattatcggctgaaattacctgcgcttgctgatgctgtttctctatcaaacccgtcagggttcttacagcgttatcaccaagaaacagaccgctatgttcaacgatttgttttatctcgtcaccgggatattgcggccactcatcggtcagttgattacgcagggcgtaaatcgccagaatcaggctggagagataatcaccctgcatgagcggccagcggtgttggttgtcgcaggccgtggataaatgctgaaggttgtctcgtgttatgcccgccagcggaattaaaaacggatctttgcgcagcaagttcgccagcaagataacgcgtttctcttctgtctcatcaatgaaatggcccaaaccagggcggctggccaggcaacaagtgcgttcataacgctgttttaaccggggcagacgctctgctacccacgtttctggcaaattaagcgccgaggcgagttgcgcacggggagtgaaagtattcagtaataacagcgccagcagccgatcgtcgttatcgtgcttttgcagcaactgaaaaaagctgcggcgctcgaagatttccagctgatagcccgcactgccactggcgaaaatgcgggctttgccgttaagggtgaagttgagatagtcaatatcacgcaggatggtcctgcctgaaacgccagtctgttgcgccagctcgccaggcgtgcgcggctgttgctccagcagatcgacaatctttaactggcgttcgtttagcattaatccacctgacggaactggctaaacgcgttgactttctccgcagttaaggtcgtcagaaaaccccgtatcagcgtgagcagagcttcgtaatcggcttttgaaatcataccgctgttggcgtgcagataacgagttggcagacacagcgcgacaaccggacgcccgccgcccatcacgttgtagcgcccgccatccgtcgcaccggttttcatggtggaaaattgcagcggtaaatcgttatgtgcggcacagctttttaacgctgctaccagtttctggttggggaagtagcgcttgtcaaacagcatcagccccggcccctggcccagtttcagcgggtatttaatgttatcaatgcccggaacatcgcccgctacggcggtatccaacacgatcacgacgtccggtttaatgtgttccgccgaggtttgcgccccgcgtagcccaacttcttcttccacactgccaacgccatacagcgtaatttcgggattattcaccgtctgcaatagttcagccatcattgcgcagccgatgcggttatccaacgccttgccgaccactttatcttcgccccagcaggcaaaattggcttccgggctaataaaattaccaatttccacgccgcgcttttccacctcttcgcgactgttcgcgccaatatcaatgaacatctcatcaaatgacagcggttgttgcttttgcttttccgttaacgcatgaggcgcgacggaaccaatcacaccagggattttcactcccttgtgtgtgcgtatggttacccggtggttgagcatcgactgattccaccagccgccaatggtggtaaaacgcagaaaaccgctctcgtcgatgtgggtgaccataaagccgacttcatccatatgtccgacaacggcaacttttggacctttattccccttacgggcaacaaagctgcccagaccatcgaaggtgatttcattcacgcaaggttccagcgtgtttatcagaatgtcgcgaacttcctgttcatcgccgctgacggcgctggcttcgcacaactgttgcagtaactcaatgttcatggacaagctcctgttgcgcggctttcgctttgcggcgtaaccacaatcctttcaggacgataatgaatgaaatgttcagcgcgaggccaatcgccagcaccagataaaacgaacccaccggcgacatcaggccgatcagcgggtcaaagatacccaaaccaggtgccagacgtttgattccgaaagcgatcaccagcacgccggtaatgccgcccgccagcgtattggcggtaatcatcggcaacggagctgccagagcgtaaggaatagccggttcggttgcgactgtggcaccgaccacaatggcactactggcagcctctttttcctgtcgggtaaacagtttgggcgcaatgaacgtcgcaagacccgccgcgacgggcggcatcagcgcgacaacgccgacgatggcgtaccagtcataaatgtgtttttccagcagtgagaagcagaagaaccaggcggttttattgatggggccgcccatatcgaacgccagcatcgcaccgaccagaaacgctgccgcaaacttcattgatggaggaatggtattcaggaagtggagcagcccgcccatgaggtcggacatcaccggcccgataacgtagtaagtgagcacgccgaaaaccagcagagtaacgaacgggatcagcattgaaccgagcagcggttgtaatgctttgccaaggcgcactttgcggaaccagaagacgaaatagccaatcgccagccccagcaccaccgcgccgaggaatcccgcacccgactgggtgccgagcagcgctttgtcgttcgccagatagcaaaccagaaacgccggagcgaaagccggtttatcggcaatcgacgaggcaatataagcgcccatgatggggatcataaaggtgaagccaaggtaaccgatggattcaactacccaggtaaacgacggcgcgcctttcgacatatcggtatacggcaaaccgaactgcaccagcatgttggcaagcgccaccaggataccaccgccgatgacaaacggcagcgccgcagagacgcccgccatcaggtggctcatcacgctaccgctttgcacttcctgtttgccaagcttcacgccgctatctgcggcaaaaagctgcgagtttgtcggtaattcgctgaaaatctggtcgatatttttcaacgcctgggagatggcaatctcataaactttcttcccggcaaaccgcgcgcgatcatcaccgctcaggccacgcccggtagcgagaatgacgtaatcggcagcggcaatctcttcgctggataagcggttttcaacgccactggacccttgagtttccacttttatggtatgaccgagagaacgggctttctgttccagggcttccgccaccatgtaggtgtgagcgatcccggcggggcagttggtgatcgcgacaatacgtaaggatgactccatcgccacttccttatgagctgagggtttgatttaacaaggcaagcacctggtcggtatcgccctgttgcagttgatgaataaattccttgtgaataattttgcgacacagtgtgccgatgattttgacctgatcctcttcgccgctttgcggcacgccgaggcagatccagcaattgacgtcttcgccatcgctggctttccagtcaatagcctgcgctttgcgggcgaataatacgaacggttgtttaacgcaggcgcttttaccgtgcggcacggcgacaccggaaccaaatccagtagagtgcattttttcgcgcagcagcagggtttgcaggaactggtgtgagtcggtgataaaaccgttttgtaacgctattgtcgccaactgcttcagaacggaataagcgccattgccctgaatattcaggtcaatacagcttgcagtaagagctgccattaatcggactccataaaatatattttaatcaattgtaatggtggagcgattaagtgatgagaggcgatatgtcggtaaacaatgacaatttgagacagagtgaaaggtcagatttgcggagtaatgcacataatggttatttaaataaaccacatgaatcattaatgggttattcattatttttgtgatttactcacaatgtatcagggaaatataacttaccgggagatgtaatatgtttaatttttcaaatcgaaatttaaaatattgtgccggaggcatctctggcacattgggcaattacggcaggtaaaacacttcttgcagctcgctactcaccgggctgttatccgggttagcgggcataacatcggtcatatatttccaccaacgttggcaaacatcagtgctggcaaccgcattccagcgttcttcagattcaatctctaccatggcaaacagcagattacgcgctttgtcgagatagatggcgtagttatgcgcaccgtgagatttcagcactgcttccagttctggccagatgggattatgccgacgctgatactcttcgtgggcgtcggggtttacctgcatgacaaaggctttgcggatcatgtttgctccttacagcgccagcgcactggcgagtggcgtaacgccgaaacgcttgccgagcgctatcaactcttcacggctgatggtctgtttcatgccgcccatcgaataaaccttcactaatacttgtgctgatttttctgcggtgtcgattaaaccgaaggtttcatccagcgtcggtccgctgccgaagacgccgtggaagggccacaacaccagcgaatgtttttgcatctcttgtgcggtcgcctggccgatttcgtccgtgccgggcaccatccacggcaaaatgccaacgccatccgggaataccaccagacactcggtgctgccttcccacagttggcgagtgaagaccgcggtgtcgttttcaagtacataggtgagggcgatcaggttggtggcgtggcagtgcatgatcacccgatctttgccgttggtggctttaatgcgctcgcagtgggaaaggaagtgagccggaagttcggaagtggggacggcttcgttggttaacccccaaagaatgtggtagcccgcgccgtcgctgtcgacttttacgatgcctaagttagccgcaggatcaagctggacgttacggaagaatttgcccgagccggtgacaataaacggtgtatttgccagtaaaggcatgggctggctgagcgggatatagcgcggttgttggtggaaattgtcgtgatatggtgcgatatcggcgtcatccaggcgtagcgtcaggttgccgccgttgcgctcatcccagcctttcagccaggcgtcggtggtggctttgatcattccctggacaaaccaggactgagtaatgttttgcatgttctgtgttcctgtaaattcggtgttgtcggatgcacgacccgtaggccggataaggcgctcgcgccgcatccggcaatcaatgcctgatgcgacgctgtcgcgtcttatcaggcctacaactattgccgacctgtaggcctgataaggcacttgtgccgcatccggcaatcaatgcctgatgcgacgctgtcgcgtcttatcaggcctacaactgttgccgacctgtaggccggataaggcacttgtgccgcatccggcaatcaatgcctgatgcgacgctgtcgcgtcttatcaggcctacaactattgccgacctgtaggccggataaggcacttgtgccgcatccggcaatcaatgcctgatgcgacgctgtcgcgtcttatcaggcctacaactgttgccgacccgtaggccggataaggcgctcgcgccgcatccggcagtgtttacccgcggcgactcaaaatttctttctcataagcccgcacgctctccagccattcgctacctgctggcgtatcgtgacgttggcaatacatttcccagaccgcctgccacggcaacgatttctgctcttccagcagtgccagacgcgcagtgtaatcgcccgccgcttccagcttgcgcagctcagcggtaggttccagcaacgcacgcagcagggcttttttcatattgcgtgtaccaatgacccacgcggcaatgcggttgatagaggcatcgaagaagtcaaggccgatatgcacccggtcaaacagatcgtgacgcacaatctcactggcaattgcctgggtttcatcatccagcagcactacgtgatcgctgtcccagcgaaccggacggctgacgtgcagcagcaactgcggcacatacagcatggcggcggaaatcttgtcggaaatcacttcagtcgggtggaagtgcccggcgtccaggcacagcgcagtctggcggctggtggcataccccatgtaaaactcattggagccaaccgtgtagctctctgcgccaatgccaaacaatttgctctcaacggcgtcgatatggtgcgcagggtttagcttctcgctgatcacctcatccagtgctgccagcagacgctgacgcggggcgagacggtcaacggtgatatctttcataccatccgggatccagatgttcatcaccgatggtgtgccgagttgctcgccaaaataggccgaaacgcgacggctggctttgcagtgatcaatccagaactggcgaatgctgtcgtcggcatgggaaagcgtaaagccatcggcgcttagcggatgcgaaaagcaggaggggttaaaatccagaccgagctgattggctttcgcccattcaacccagtttttgaagtgctctggtttgatctggtcgcgcgagactggcgtatctgattccagatagatggcatgtaaattaagccgtttcggccccggaatcagccgcatagcctgttccagatcggcacgtagctcactggcattacgcgctttgcccggataattgcctgtggcctgaatccccccggtcagcgaaccttccgggttttcaaaaccggaaacatcatcgccctgccagcagtgcattgaaacgggtaaacgatcaagttggcgcagcgcctcctcgacatcaatccccaccgccgcgaaacgctgtttcgctagctcccaggcctgttccagttgagtggtcatgcgcaaagctcctttgtctgtcgtgtagagtgaatctgcgccacatagtgggcaatttcactgtcaggattaggggtaaaggtggtcagattcgcggtggtgctgacgacctgacggaaatcatccacattgttgagttcatccagcgtcattaactggatgccgatattgccgagcgtcgaggcttcaacaggcccggcgatcacccgaataccgcaggcatcggcgcatagctggttgagcagcgtgttctggcagcctccgccgacaatatgcagttgcgagaaatcttcaccgcgcagctgcgccagctcatgcaacacatcggcatacagcagcgccagactgtcgaaaatgcagcgcgccagttcagcatcactttccgggatcggttgcgccgtttcccgacacgcagcctgaatttcgctgcacatcgtctcaggattaataaagcgatcgtcattgggattgataatgaagcggcaagccggaagtgcctgtgtcgcggagataagcgccggaagatcgttgatttgctgctcctgaagcactcgctgaagcagccataagcccataatatttttcagcacccgatagcgaccttccgccccgccttcattggtgatgttggctgccagtgccgtgtcattggtaaatggcgtctggctttcgaagcccatcaatgaccaggtgccagaagagagataagcagcacgtgagccgtttaacggcgaggcgataaccgcgctggcggtatcatggctggcaacggcgaccactggaatctcattaccctgcgggcaaatccagtgacctatgacattacccggatgcgtcgggcgaccaaaccaggctttgttggccccgctccacgccagtagcgactcgtcccagtcgtcgctattgatattgaccagttgcgtggtcgtggcgttggtatattcccagttcatcttgccggtcaggcgataactgaagtaatccggcatcagcagagcgtgagcaatgtgtggaataagttcaggttgttgctccgtcagcgcacgcaactgataaagcgtattgaagggcagaaactggatgccgctacgttgataaatatcgcgtttgccgagttgttgttgtgcctgcgccattaggccattggtgcggctatcgcgataagcaacgggcaggcccacacgctgaccctgttggtcgagcagcacaaagtccacgccccaggtatcaatcccaatgctatcgatacgaatcccttcctcgcacaccttgtttaatccaaggcgaatggcactttcaaggctatccacatcccaggtgacatagccgttctgactatgcagcccattgttaaaacgatggatttcgcgcagcgtcaggctgcggcattcacgctcgtaacgcgccagcatcacgcgcccactggatgcgccgagatcgacggcgacacaattgcgaaaggtcataatgtgatcctgctgaatttcattacgaccagtctaaaaagcgcctgaattcgcgaccttctcgttactgacaggaaaatgggccattggcaaccagggaaagatgaacgtgatgatgttcacaatttgctgaattgtggtgatgtgatgctcaccgcatttcctgaaaattcacgctgtatcttgaaaaatcgacgttttttacgtggttttccgtcgaaaatttaaggtaagaacctgacctcgtgattactatttcgccgtgttgacgacatcaggaggccagtatgaccgtattacatagtgtggatttttttccgtctggtaacgcgtccgtggcgatagaaccccggctcccgcaggcggattttcctgaacatcatcatgattttcatgaaattgtgattgtcgaacatggcacgggtattcatgtgtttaatgggcagccctataccatcaccggtggcacggtctgtttcgtacgcgatcatgatcggcatctgtatgaacataccgataatctgtgtctgaccaatgtgctgtatcgctcgccggatcgatttcagtttctcgccgggctgaatcagttgctgccacaagagctggatgggcagtatccgtctcactggcgcgttaaccacagcgtattgcagcaggtgcgacagctggttgcacagatggaacagcaggaaggggaaaatgatttaccctcgaccgccagtcgcgagatcttgtttatgcaattactgctcttgctgcgtaaaagcagtttgcaggagaacctggaaaacagcgcatcacgtctcaacttgcttctggcctggctggaggaccattttgccgatgaggtgaattgggatgccgtggcggatcaattttctctttcactgcgtacgctacatcggcagcttaagcagcaaacgggactgacgcctcagcgatacctgaaccgcctgcgactgatgaaagcccgacatctgctacgccacagcgaggccagcgttactgacatcgcctatcgctgtggattcagcgacagtaaccacttttcgacgctttttcgccgagagtttaactggtcaccgcgtgatattcgccagggacgggatggctttctgcaataacgcgaatcttctcaacgtatttgtacgccatattgcgaataatcaacttcgttctctggccgaggtagccacggtggcgcatcagttaaaacttctcaaagatgatttttttgccagcgaccagcaggcagtcgctgtggctgaccgttatccgcaagatgtctttgctgaacatacacatgatttttgtgagctggtgattgtctggcgcggtaatggcctgcatgtactcaacgatcgcccttatcgcattacccgtggcgatctcttttacattcatgctgacgataaacactcctacgcttccgttaacgatctggttttgcagaatattatttattgcccggagcgtctgaagctgaatcttgactggcagggggcgattccgggatttaacgccagcgcagggcaaccacactggcgcttaggtagcatggggatggcgcaggcgcggcaggttatcggtcagcttgagcatgaaagtagtcagcatgtgccgtttgctaacgaaatggctgagttgctgttcgggcagttggtgatgttgctgaatcgccatcgttacaccagtgattcgttgccgccaacatccagcgaaacgttgctggataagctgattacccggctggcggctagcctgaaaagtccctttgcgctggataaattttgtgatgaggcatcgtgcagtgagcgcgttttgcgtcagcaatttcgccagcagactggaatgaccatcaatcaatatctgcgacaggtcagagtgtgtcatgcgcaatatcttctccagcatagccgcctgttaatcagtgatatttcgaccgaatgtggctttgaagatagtaactatttttcggtggtgtttacccgggaaaccgggatgacgcccagccagtggcgtcatctcaattcgcagaaagattaattcgccatgccgatgccgacgatgttagcggcgacaataatcaccacacaaccgaggctcaacaccgttaccggacggcgtcctgcattgttccactctttcagcaccagcccgacgataccgccgcacaatacatagaaactcatatgcagcatccaactgatgtagtcatactgcgccggaatgcgggcgtggccccaggcatagaaaaagaattgcagataccacatcaacccgcccagtgtcgagagtaacacattgtgaatgatcagcgattttgccagcgagaagtcggcttttagcgacaaatccttcacttttgccagacgaataaaacagaaaccgaggttaatgatcgcgccgccgcccatgatgacaacatagcttggcagagcgacatacagtggatcgacgccaagtgcggcagcggcttcatgcatcggttttgcggcgttcatcgcaaaggacatcccggcagagaaaatgccgcacatcaccgccagcaccagcccttttttcagattgaactcttcggctttaatgcccatcttgcgctctttcaactgcccggcgcgagttacaatccctacgccaatcagcgccaccagaacgccgagcaacgtcatgcgtccgccttcggtgctaatcaacacatcgaaattgccgttgataattggcgtcatcagcgtaccgacaatcaacgtaatgccaatggcgatgccaattcccatcgacatgccgagataacgcatggtcaggccgtagttgatattaccgatcccccacatagcgccgaacagaaaaacaggcagtcgcgtagagagactaaacgagctgtaatacgcccagaaattcggtagtaacagggcgctgatggcccacggcagaataatccacgaaacaatcccaccgactgaccacatggtttcccatgaccatttttttacttttttgaacggagcgtaaaaacaggctgcactggccgcgccgatcaaatgccaaaatatccccatcgtaatcgcgttactcatcttcttatcctcatcatttttcgtcgcgtcacatctccgacgagatgagtgtaaaaatcgtgctgtcgattaacctttcgcctgttgccgccgttgtcgatttactggcaatcacggcattaagtgggtgatttgcttcacatctcgggcattttcctgcaaaaccatacccttacgaaaagtacggcattgataatcattttcaatatcatttaattaactataatgaaccaactgcttacgcggcattaacaatcggccgcccgacaatactggagatgaatatgagctataccctgccatccctgccgtatgcttacgatgccctggaaccgcacttcgataagcagaccatggaaatccaccacaccaaacaccatcagacctacgtaaacaacgccaacgcggcgctggaaagcctgccagaatttgccaacctgccggttgaagagctgatcaccaaactggaccagctgccagcagacaagaaaaccgtactgcgcaacaacgctggcggtcacgctaaccacagcctgttctggaaaggtctgaaaaaaggcaccaccctgcagggtgacctgaaagcggctatcgaacgtgacttcggctccgttgataacttcaaagcagaatttgaaaaagcggcagcttcccgctttggttccggctgggcatggctggtgctgaaaggcgataaactggcggtggtttctactgctaaccaggattctccgctgatgggtgaagctatttctggcgcttccggcttcccgattatgggcctggatgtgtgggaacatgcttactacctgaaattccagaaccgccgtccggactacattaaagagttctggaacgtggtgaactgggacgaagcagcggcacgttttgcggcgaaaaaataatcatttgccgcctgctgcaatgaggcgtataggccgcatatcagcttaaaaaatgaaccatcgccaacggcggtggtttttttgtgatcaatttcaaaataaaaacaatgatccgataaaaataaaacagcgtttcaattgatgtggttttgatcacttttattgattaaatgaatgtctatcttcgtttccatcaacactgatgctccattgaggaattacgcatcagcccttaaaaatatgccgacaggtgatggaaatgcagataaaacgctcgattgagaaaatcccgggggggatgatgctcgtcccgctattccttggcgcactgtgccacaccttctcgccgggggcggggaaatattttggatcattcaccaacgggatgattaccggtacggtgcccattctggcggtgtggtttttttgcatgggggcgtcaataaaattaagcgcgacgggaacggtactgcgtaaatccggtacgctggtggtaactaaaattgccgtcgcgtgggtggttgcggcaattgcctcgcgtattattccggaacatggtgttgaagttggattctttgccggactttcaacgctggcgctggtggcggcgatggatatgaccaatggcggactttacgcttccatcatgcagcagtacggcacaaaagaagaagctggggcatttgtgttgatgtcgttggagtccgggccgctcatgacgatgattattctgggcactgccgggattgcctcgtttgaaccgcatgttttcgtcggcgcagtattaccgttcctggtgggctttgccctggggaaccttgaccctgaattgcgagaatttttcagcaaagcggtgcaaacgctgattccattctttgccttcgcgctgggcaataccattgatttgactgtgattgcccagactggtttgctggggatcctgttgggtgtggcagtaattatcgtgaccggtattccgttgattatcgccgataaattgattggcggtggcgatggcactgccggaattgccgcttccagttccgcaggggccgcggtagcgacacctgtgctgattgcagaaatggtgcctgcgtttaaaccgatggctccggcagcaacttcgctggtagcgacggcggtcattgtgacttcgattctggtgccaattcttacctctatctggtcacgtaaagtcaaagccagagcagcgaaaatcgaaattttaggtacggtgaaataaacctgcttccttaatccccacagccggatgaactaacgttcgtccggtttgctattgagttcctgcctggatacttaccgcgaaaacagcacgcctgacataaaataaatatggtctaatggggaaatttctcgtggagagggaacagatgcgatatccggttgatgtatacacaggcaagattcaggcttatcccgaaggcaaacccagcgcaattgctaaaatccaggttgatggtgagttgatgctgacggagctggggctggaaggtgacgagcaggcggagaaaaaggttcacggcgggccagacagagcgctgtgtcattatcctcgtgagcattatctctactgggcgcgggaatttccggaacaggcggagttgtttgttgcgcctgcgtttggtgaaaacctctcaaccgacggcctgacggaaagtaatgtttatatgggcgatattttccgctggggagaggcattaattcaggtcagccagccgcgctcgccttgctataaactcaattaccattttgatatcagcgatatagcgcagttgatgcaaaacacaggtaaggtggggtggttgtatagcgtgatagcgccagggaaagtgtctgcggacgcgccgctggagttggtttcccgtgtcagcgatgtgaccgtgcaggaggctgccgccatcgcatggcatatgccgtttgatgacgatcaatatcaccgtttactctccgctgccgggttatcgaaaagctggacgcggacgatgcaaaagcgccgactgagcggcaagatcgaagatttttcccgccggttgtggggaaaataacccccggagtgtaggcctgataagacgctatcagcgtcgcatcaggcatcctgctcaaatgccggatgcggcgtaaacgccttatcctgcctgcaaatgcgaagtttaactccgcttatacagcggcaaccaaatcaccagccgtaaaccgcccagcgggctgtcttctgccttcacccagccacgatgctgctgaatggcggtttcaacaatcgccagccccaaacctgtaccgccagattcacgatcgcgtgcttcatcggtacgatagaacggacggaaaatctgttcgcgatcttccgggctaacgccaggaccatcgtcgtccaccgtaatggtgataccgtctttatctaccgcaaagcccacttcaatcttcgtatgggaataacgcagagcattacgaacaatgttttccagcgcactttccagggcgttcggattgccgtacagcggccacggcccaggcgggaagttaactgtcaacgacttgcccatttgctcggcttcgaacgccgcgttatccagcacttcactccacaactggttggctttgatggtttcgctaaccagcgcgtttttttgctgattacgtgacatcaccaacagatcgttgatcatgctgtccagacgttgcgcttcggtttcaatacgctccagttccttgctttcaccgctacgacggcgcagtaacgccgtacccagttgcagacgcgtcagcggggtgcgcagctcgtgagagatatcagaaagcagacgctgctgagaggtcatcatgcgctccagcgcggtgaccatctggttaaaactggcacctgcggcaaggaattcctgtggccccgcttccagttccgggtgctggcgtaagtttccctgggcaacttcatcggcagcgtttttcagcttacgcgccggttttgccagactccaggccaaccacaacagcagcggcgtactgaccaacatggtgacaatcagcagtaatagcgggcggtcaaacagtaagttaatgaaatcggattgagaactgctggccggacgaatcagataaagttggtaattatcttcgccatcacgcacggagaacggaccgaccagttccacgcggccatactttttcttctgcggatgatcggcgttatcggcctgaccaataaagttacgaatgatctgcatttcgctgcgttcagcgccgatcacgcggccttcggtggtcaccaataacaaacgctgtcctggcggtgcccacttatcaatcgcccggaacagacgccgccaccacattaaatcgttgggcggatcgttcgccagctccgcttcgacatgctgctcaatcatcagcccctgacgctgttcgctatccagaagctcggtcatctggcgtgaatcgagcttgggtaacatcaaaaccaacatcaacaccagcgccagcgtcagccagaagatggcgaagatgcgcgcggttaagctgcctatcatgaagcagaaaccatcagatagccgcgaccacgcaaggttttaaaccacgggtgaccatctttacgatccggcagtttacgacgcaggttggaaatgtgcatatcaatagcgcggtcgaaaggcgtcaggcgtttgcccaacacttcctggcttaaatgttcacgggaaaccacctgacccagatgctgtgccagcaaatagagcagggtaaactcagtaccggttaactccagcgtttgcccgtcgaagctggcttcctgacggcctggattcagcactaaggcatcaacttccagtgtcggtgaaccgttgtcgttgttttgctgttgctcgctccagtgcgaacggcgcaggatcgcgcgaatacgtgccaccagctcacgatcattaaacggtttcgggagatagtcatctgcgcccagctcaaggccgagaacgcgatcaagttcactgccgcgcgccgtcaacataatgacaggcgtctggtgtgtctggcgaagtgcttttaatgtgtcgataccatttttcttcggcatcattacgtcaagcaaaagtaaatcaatgctgtcgtccagaagatcaagcgcctgttccccatcgtgggcaacaatcacgttgaagccttccatctcgagcagctcctttaatagggaagtcagctctcggtcatcatcaactaacaggattttattcattgtttaaatacctccgaggcagaaattacgtcatcagacgtcgctaatccatgactttacgttgttttacaccccctgacgcatgtttgcagcctgaatcgtaaactctctatcgttgaatcgcgacagaaagattttgggagcaaatgatgcgcatagttaccgctgccgtcatggcctcaacgctggcagtcagttcattaagccacgctgctgaagtcggttcaggcgataactggcatccgggtgaagaacttacgcagcgcagtacgcagagccatatgttcgacggcataagtttaaccgaacatcagcgtcagcagatgcgagatcttatgcaacaggcccggcacgaacagcctcctgttaatgttagcgaactggagacaatgcatcgccttgtcaccgcagaaaattttgatgaaaacgctgtgcgcgcacaggcagaaaaaatggcgaatgagcaaattgctcgtcaggttgagatggcaaaagtccgcaaccaaatgtatcgcctgttaacgccggagcagcaagcggttttaaacgagaaacatcaacaacgaatggagcagttgcgtgacgtgacgcaatggcaaaaaagttcatcgttgaagctattgagtagtagcaactcacgttcccagtagtaaaccctgttttccttgccatagacaccatccctgtcttcccccacatgctgtgggggttttttttatcctcaatttgcctgctgcttaatgcattgcagatgatttgcttccgttatactagcgtcagttgatagcgggagtatttatgaatcaatcttatggacggctggtcagtcgggcggcgattgctgcgacggcgatggcttcgctgctattgctgattaaaatttttgcatggtggtataccgggtcggtgagtattctcgccgcgctggtggattcgctggtggatatcggcgcgtcgttgacgaatttattggtggtgcgatattccctgcaacctgccgacgataatcactcgtttggtcacggtaaagctgagtccctcgcggcgctggcgcaaagtatgtttatctccggttcggcactattcctgtttttgacgggtattcaacatctgatatctccaacaccgatgacagatccaggcgtcggggttatcgtgacaattgtggcgctaatttgtacgattatccttgtctcgtttcagcgttgggtggtgcggcggacgcaaagccaggcggtgcgggctgatatgctacattaccagtctgatgttatgatgaacggcgcaattctgctggcgctggggttgtcctggtacggctggcatcgcgccgatgctctgtttgcattgggaatcggcatctatattttatatagcgcgttacgcatgggatatgaggcggtacagtcattactggatcgcgcattgcctgatgaggaacggcaagaaattattgatatcgtgacttcctggccgggtgttagcggcgctcacgatcttcgcacgcggcagtcagggccgacccgctttattcagattcatttggaaatggaagactctctgcctttggttcaggcacatatggtggcggatcaggtagagcaggctattttacggcgttttccgggatcggatgtaattatccatcaggacccctgttccgtcgtacccagggagggtaaacggtctatgctttcataatcagtataaaagagagccagacccgcattttgtgtataaaataccgccatttggcctgacctgaatcaattcagcaggaagtgattgttatactatttgcacattcgttggatcacttcgatgtgcaagaagacttccggcaacagatttcattttgcattccaaagttcagaggtagtcatgattaagaaaatcggtgtgttgacaagcggcggtgatgcgccaggcatgaacgccgcaattcgcggggttgttcgttctgcgctgacagaaggtctggaagtaatgggtatttatgacggctatctgggtctgtatgaagaccgtatggtacagctagaccgttacagcgtgtctgacatgatcaaccgtggcggtacgttcctcggttctgcgcgtttcccggaattccgcgacgagaacatccgcgccgtggctatcgaaaacctgaaaaaacgtggtatcgacgcgctggtggttatcggcggtgacggttcctacatgggtgcaatgcgtctgaccgaaatgggcttcccgtgcatcggtctgccgggcactatcgacaacgacatcaaaggcactgactacactatcggtttcttcactgcgctgagcaccgttgtagaagcgatcgaccgtctgcgtgacacctcttcttctcaccagcgtatttccgtggtggaagtgatgggccgttattgtggagatctgacgttggctgcggccattgccggtggctgtgaattcgttgtggttccggaagttgaattcagccgtgaagacctggtaaacgaaatcaaagcgggtatcgcgaaaggtaaaaaacacgcgatcgtggcgattaccgaacatatgtgtgatgttgacgaactggcgcatttcatcgagaaagaaaccggtcgtgaaacccgcgcaactgtgctgggccacatccagcgcggtggttctccggtgccttacgaccgtattctggcttcccgtatgggcgcttacgctatcgatctgctgctggcaggttacggcggtcgttgtgtaggtatccagaacgaacagctggttcaccacgacatcatcgacgctatcgaaaacatgaagcgtccgttcaaaggtgactggctggactgcgcgaaaaaactgtattaatgatttcggaaaaaggcagattcctttaccctgaaaccgatgacagaagcaaaaatgcctgatgcgcttcgcttatcaggcctacatgaattctgcaatttattgaatttgcaaacttttgtaggccggataaggcgttcgcgccgcatccggcatggacaaagcgcactttgtcagcaatatgaggcggatttcttccgcctttttaatccctcaacatatacccgcaagttatagccaatctttttttattctttaatgtttggttaaccttctggcacgctttgctcatcacaacacaacataagagagtcgggcgatgaacaagtggggcgtagggttaacatttttgctggcggcaaccagcgttatggcaaaggatattcagcttcttaacgtttcatatgatccaacgcgcgaattgtacgaacagtacaacaaggcattcagcgcccactggaaacagcaaactggtgataacgtggtgattcgtcagtcacacggtggctcaggtaaacaagcgacgtcggtaatcaacggtattgaagctgatgttgtcacgctggctctggcctatgacgtggacgcaattgcggaacgcgggcggattgataaagagtggatcaaacgtctgccggataactccgcaccgtacacttccaccattgttttcctggtacgtaagggaaatccgaagcagatccatgactggaacgatctgattaaaccgggtgtttcggtgatcacgcctaatccgaaaagctctggtggcgcgcgctggaactacctggcagcctggggctacgcgctgcatcacaacaacaacgatcaggcaaaagcacaggattttgttcgggcactgtataaaaacgtcgaagttctggattctggcgcgcgtggctccactaacacttttgtcgagcgcggaattggcgatgtactgattgcctgggaaaacgaagctctgctggcagcgaatgaactggggaaagataaattcgaaatcgtcacgccgagtgagtctatcctcgcagagccaaccgtgtcggtggtcgataaagtggtcgagaaaaaaggtactaaagaggtggcggaagcctacctgaaatatctctactcgccagaaggtcaggaaattgccgcgaaaaactactaccgtccgcgcgacgctgaggtggcgaaaaagtacgaaaatgcgtttccaaagctgaagttattcaccattgatgaagagttcggcggctggacgaaagcgcaaaaagagcattttgctaacggcggtacgttcgatcagatcagcaaacgctgatttccccaggataattatcaaacccggtggtttctcgcgaccgggttttttatttgtcacgattttgcgttacccttgcatctctttgaggtacagggaaaaaaagatgaaaaaagcgggtcttctttttttggtgatgatagttatcgccgttgtggctgccggtattggttactggaaattaaccggtgaagagtcggatacattacgtaagattgtccttgaggaatgtttgcccaatcagcagcaaaatcaaaatccttcgccatgtgcggaagtcaaacccaatgccggatacgtggttttaaaagatcttaatggcccactgcaatatctgttgatgccaacgtatcgtattaacggtactgaaagtcctttgttgaccgatccttcaacgccgaacttcttttggttggcttggcaggcgcgtgattttatgagcaaaaaatacggccagccggttcccgatcgcgcggtttctttggcgatcaactcccgcaccgggcgtacgcaaaaccattttcatattcatatctcttgtattcgtcctgatgtgcgcaaacagctggataacaatctggcgaacatcagcagccgctggttgccactgccaggtggtttgcgcgggcatgaatacctggcgcgtcgggtaacggaaagcgaactggtacaacgcagcccatttatgatgctggcagaagaagtacctgaggcgcgggaacatatgggacgctacgggctggcgatggtacggcagagtgataactcatttgtattgctggcgacacaacgaaatctactgacgcttaaccgtgcttcagccgaggaaattcaggatcatcagtgtgagattttgcgttaaggcgaagagttaaggaaagtaagtgccggatatgaaatccggcacctgtcagacttaagcctgtttagccgcttctgcagctttaacgattactgcgaaggcgtcagctttcagagaagcaccaccaaccagcgcgccgtcgatatccggctgagcaaacagttctgcagcgttagacgcgtttacagagccgccgtactgaatgatcacttgttcagcgatgttagcgtcaactttagcgatgtggtcacggatgaatttgtgaacagcctgtgcctgagccggagttgcagatttgccagtaccgattgcccatacaggttcgtaagcgataaccgcaccttcgaatgccgcagcaccctgagttttcagtaccgcgtcgatctgacgtgcgcaaacttcttcagttttgcccgcttcattttcagcttcggtttcaccgatgcacagaaccggagtcaggccctgctctttcagcaccgcgaattttttcgcgatcagttcgtcagattctttgtggtaagtacgacgttcagagtgaccgatgatgatgtactgtgcgccgatgtctttcagcatagcagcagaggtttcaccggtgaatgcgccggacaggttcaggtccacgttttgcgcacccagcatgatgtggctgccttcagcttcgcgcttcgccatatcgatatacatttccggtggtgcgattgcaaccgcacagccagcaacacctgccagctctttacgcaggttagaaaccagctcgtgaaccatgtggcggctgccgttcagtttccagttacccatcactaaaggatgtcgcattttaattctccacgcttataagcgaataaaggaagatggccgccccgcagggcagcaggtctgtgaaacagtatagagattcatcggcacaaaggctttgctttttgtcatttattcaaaccttcaagcgattcagatagcgccagcttaatcggttcaacagcgaaggtcagccccttttcgccgttgtccgcgacaacataacgcagtgcaccttctgtctcggtgtaataacgtttgtttttccccgccgttagtagcgactgcagttttttctggctttgtgttttggtcattaatggggtgagtgtgcggatcaccgctgccatgtattcctgagctttcgctttcgcggctttttgctctggcccctggatgggtagccaggtcatttgaatgcttttgatttttaaggtaccgcgctccagcgctgtagaagcatacaagttctcattaattttacttgcagcacgagtgagattggctttgtcgggactgctgtcgatggcacgaaattcgttcagtggcaggctgggattctggctgttaaagtcttctcgaaactggctgatggagagatcgaaagtaggggctccagccagcagataaggcgcggtcgttgccgtatctggtgtttgtgcatgcgcctctgttgtaacggttaatgcagaacataagagaaaaaacagcgtacaccctggcttcattgacagtaccttttgttatgactggctccgattaaaacgatatctgtcgcccttgtcaaaagggtagaatcctggaaaagacaaccatcaaggaacttacatgaccatacagcaatggttattctcatttaaagggcgtattggacgccgtgatttctggatttggataggcctgtggttcgcaggcatgctggtgcttttctcactggcgggtaagaatctactcgatattcagaccgcggcgttttgccttgtgtgcttgctctggccaacagcggcagtaactgttaagcgcttgcatgatcgcgggcgttccggcgcatgggcatttctgatgattgtggcgtggatgctgctggcgggtaactgggcgattttaccgggtgtctggcaatgggcggtggggcgttttgtcccgacgttgattctggtgatgatgcttatcgatcttggtgcgtttgttggcacacaaggcgaaaataaatatggtaaagatactcaggatgtgaagtataaagccgacaataaatcaagtaattaacctttaatatatctcttactgctatttttttccgggattgttatttccacgatgcaaatgacaatacccggaaaatccttctgaactcttcaccttaagcaatatcaaaaaaaatggtaatccataagatcattacttgtttgttcttcccttaacggcgcattattcttaagtcgtaatcgacagagaggcgaatatacagaggtgccctatgaaagatgtcgtagataaatgcagtactaaaggatgtgcgattgatatcggtacggtgattgataacgacaactgtaccagtaagttttcgcgcttttttgccacccgcgaagaagcagagtcttttatgaccaaactgaaagagcttgccgccgctacatcctctgcagatgaaggggccagcgtggcctataagattaaggatctggaggggcaagttgagcttgatgcggccttcactttctcatgccaggccgagatgattatttttgagttatcactgcgttcgttagcttgatggagttgctttagaaggagttaaacatggcttataaacacattggcgtggcaatttccgggaatgaagaagatgccttactggtgaataaagccctggagctcgccagacataatgacgctcacctgacgttaattcatattgatgatggcttaagcgagttgtatccgggtatctacttccctgcaacagaagatattcttcaattgttgaagaataagtcggataacaagctgtataaactgacgaaaaatattcaatggccgaagacaaaactgcgtattgaacgcggagaaatgccggaaacactgctggaaattatgcaaaaagagcagtgcgacctccttgtctgtggtcatcatcactcatttatcaaccgtttgatgccggcatatcgcgggatgatcaataagatgagtgcggatttgctcatcgtgccgtttatcgataagtaaccgcttaccagtaatgctccgctgtcatatggcccggtcggcgacgtaaatgtttcgtcatctgccgggtctctttcagcaactgttgtgtatcgcgcaccatctgtggattgccgcacagcatcacatggctggtttctttattcatcggcaggccaatcgtgctttccagttccccactttcaattaatgccggtatccgtccggtgagcgaccccgctgccgtttcccgactgaccaccgtctgaatgcgcagttttccttcgtagcgtttttccagttcctgcatcagtggcaaatagcttaagtcggcggcataacgtgcggcgtgcaccaggaccagatttttgaagcgatctaaatctttacctagttgcagaatcgataaataagggccaatcgctgtaccggttgccagcatccatagcgtttcgcagtgcggcacttcatcgagcacaaagaatcctgccgcttcgctaaccacctgcacttcatcgcctggtttcagtgccgccagtcgtgggcttaatttgccatcggggacggtgaccaggtaaaactccagatcgggattatcgggcgagtttacataggagtaggcgcgctggacgcgttcgccgtcgatttcaaggccaagcttggtaaattgcccggcggtaaacggaagcacgggggcgtgaacggtgagactaaacagggcgtcggtccagttctgcactttagtgactttgcctgttacccaatcagccatgtttttctcctgttttgattgacttgccttatcttcgttctccgaacaaaaaaattccagtcccgaaggactggaaggctcaatcgatcaaatcaatcagaggatgtgcacctgcatttccgggtctttgcgatccagatagtggatggactgaatgcggcgaatggtgcgtgacttgccgcggatcagcagcgtttcggtagtcgcgatattgcctttgcggctaatgccttccagcagatcgcctttggtaataccggtggcagagaagatgacgttatcgctgcgcgccatatcgcccaggcgcaatactttaccggcttcgatgcccatcgctttgcagcgtgccagctcctgctcgccaatgcgacgattctcttcgttgtcgcctttgacgtcatgacgcgccagcagacgaccgttcatgtcgccatctaatgcgcggatcaccgccgcagaaactacgccttccggcgcgccaccaataccgtacagcacgtcaacttcgctgtctggcatacaggtgagaattgaggccgcaacgtcgccgtccggaatagcaaatacgcgtacgccgagttgctgcatttcagcgataacggcatcgtggcgtggtttagccagaatcgttaccgtcagttcgctcaacggtttgccgagcgccgccgctacattgcgcaggttatccgccagcggcaggttcagatcaatggtgcctttggctcccggcccgacaatcagcttctccatatacatatccggcgcattgaggaagcagcctttatcgcctactgccagcaccgccagcgcgttagcctggcccatcgccgtcatgcgcgtgccttcaatcggatcaacagcaatatctaccgcgtcgccgcgaccagtaccgactttttcaccaatgtagagcatcggtgcttcgtcgatttcaccttcaccaatgacgatggtgccgtcaatgttgacctggttgagcataatacgcatggcgtttaccgccgcgccgtccgcggtgtttttatcgccgcgtcctaaccatttgtagccagccagcgccgctgattcggtgacgcgggaaaattcgatggcaagttctcgtctcatagcaaactctaagcagtaaggaatggcgcgaagtgtagcacaggggaagggagggattattgatgtgtgcggggttgcccccgcacgtttcgggactaccggatgcggcataaacgcttcattcggcatttacattattcgtcgtgttcttcccacgccatcgcgcgtttaaccgcttttttccagcctgcgtaacggtaattacgctcagtggtttcgatgcctggacggaactcgcgctcaatcaccgctttctcttgcagctcgtcgaggttctgccagaagccaaccgccaggcctgcgagataggccgcacccaatgcggtgacttcgcgcacttccgggcgctcaacgcgggtgccgagaatatcggactggaactgcatcaggaaattgtttgctactgcgccaccatccacgcgcagggcgtgcagacggataccagagtcggcctgcatcgcttccagcacgtcacgcgtctgataagcaatagactccagcgtcgcgcgtataatgtggttagcgttcaccccacgagtcagaccgaaaatcgccccgcgcgcatacgggtcccagtacggcgcacccagcccggtaaatgccggaaccacatacacaccattggtgttttgcactttggtggcgaaatattcggaatcgtaggcgtcgttaatcaacttcatttcatcgcgcagccactgaatggatgcgcctgccataaacaccgcaccttccaacgcatagttcacttcgccagtcgggccgcaggcgatggtggtcagcaggccgttttctgatttcaccgctttctcgccagtgttcatcagcataaagcagccagtgccataggtgttcttcgccatcccttctttcacgcacaactgaccaaacagcgcggcctgctggtcaccggcgatcccggagattggaatacgcgtgccgcctttgccgccaatgttagtctgaccgtatacttcggaagaacgacgcacttctggcagcatctcgcgcggaatatccagcacttccagcattttgtcgtcccagtccagggtatggatgttgaacaacatggtacgagaggcgttggtgtaatcggtcacatggacacggccctgagtcattttccagataagccacgtatcaaccgtaccaaacagcaattcaccacgacgtgcacgctcgcgagagccttccacatggtcgaggatccacttcactttggtgccagaaaagtacgggtcaatcaccagaccggtattgctgcggatataatcttctaaaccgtcacgttttaaatgctcgcagatttctgcggtacgacggcactgccagacaatggcgttatagataggcttgccggtttctttttcccagacaatagtggtttcacgctggttcgtaataccgatagctgcaatttgatcggaactgatatcggctttcgccagcacttctaccagcgtggagctttgggtggcccagatttccattgggtcgtgttctacccaacctggttttgggtagatttgctcaaattcgcgctgcgacacgctaatgatattggcatcgtgatccattacgaccgcgcgggagctggtggtgccctggtcgagcgcaacgatatattttttttcagtcatgtttaattgtcccgtagtcatattacagcgaagctttttgttctgaaggagttgtggtttccttttcttccacaacacagatatcgcaaggcaaatggcgaccaatcagtttgcggtaggcaaatgcacctacaatcgcgccaacgatagggccgaaaagcggcaccaggaagtaaggaatgtctctgccgccggtaaaggcgacattgccccagcccgccagccaggcaaagactttcggaccgaagtcacgcgctgggttcatggcaaaacctgtcaatgggcccatagatgcgccaatgaccgcaatcagtagaccaatcagcaagggagccaaagggccgcgtggtacaccgttgccatcgtccgttaacgccaggatcagccccatcagaatagcggtaatcaccatctcaactgcgaaagcctgcacaaaattgatatgaggattagggtaagtagagaaagtgccagccagatcaacactttcaacgctgccgcgaacaatgtgatgagtctgctcgaagtcgaaaaataaattgtagtaaagcccgtaaactaaagccgcagcacagaaagcgccggcaacttgtgaaacgataaaaggaataactttgcgcttgtcgaaacaggcaaacagccacaatgcaatggtaacagcgggattaagatgcgcgccggaaacccctgcggtcaggtagatggccattgccacccccagtccccaaatgacactgatttcccactgaccaaaagacgcaccagcgacttttagtgctgcaacgcaacccacaccgaagaaaatcaacaacccggtaccgaggaattcagcaatgcactggcctttcaaggttgatgtttgactcataatcggatcctgaagagttaatgtttgttgtatgcgtgaaagtcacggacctccacgatgcttgtaggcatgctgtaaacttatcgttaacgagcaaaaacgagaaatatcgaacttaaaatgtgtgtgcctcgtcataaaatgagcgttatcgcgccatttattccatctgattgtacatgatgcatgtttgttagatcattcgcgcaacaaatttattaacattttcgattgatgtggattatgtcaccaggagaaggatgaaaagtgtggcaaaccgtaatctgcaaggcgtgccgctggacagcgatggcgcggcttcatacaatcggagctaactaaagtgcgctcgtatttattaaggcgtcaccggtaatcgggacgaggatttttatccatcaacgccttgcaattcaggagaggtatgacaatgtcattagaagtgtttgagaaactggaagcaaaagtacagcaggcgattgataccatcactctgttgcagatggaaatcgaagagctgaaagaaaaaaacaactcactgtcgcaggaagttcaaaatgcccagcatcagcgcgaagagctggagcgtgagaacaaccatctgaaagaacagcagaacggctggcaggaacgtctgcaggccctgctgggtcgcatggaagaggtctgattacgcttcatcttccgcgtaatttctttactgtgtaggccaacaggtaacgcagaaaaaaggcaccttgcggtgcctttcttatcattcaatatccagcggatcttctgaaagaataatcccggtattgtcggcataaagatggtcgccggagaagaaggtgacaccgccaaaattgacgcggacatcgctttcgccaatgccttcgccagcggcaccaaccggaattgccgccatcgcctggatgccgatatccaactcttccaggtcatctacctgacgcaccgcgccgtaaatgaccagaccttcccattcattttgtactgccagacgcgccagttcagcatcgaccagtgcgcgacgaacagaaccaccgccatcgacgacaagaacacgaccacggccattctgttcgagcagatcgtacagcaacccgttgtcctcgaaacattttaccgtgattatttgtccgccaaacgacgcccgtccgccaaagttggagaacagcggttccacgacgttaacatcttcttgatagatgtcacaaagctcggaagtatcgtatttcataggcttaacattcagttgctgcgagaattttcagtatatcgcgctatgtgggctgttggcaaaatcatcaattgttaattgatatttgtcagttatgctgcccactggcttaggaatatccctaaaacaaacagcaggttagtcagtaacgctcccttgacagtacgttccagcattggtcgcatcgccaccgggtccatttcccgcatcacataacgggcttgcttcaccagtaatggtgccgccagcaggaacagccagccccacaggctatgcagcgaaaagagattaaacagcgccagacacaccagcgagcccatcagcaggcaggcatgataacgacgcgcgttcacttcacctaagcgcaccaccagcgtgtttttgccattttcgcggtcgctattgatatcacgcaggttattaatattcagtactgccgttgccagcaggccgcatgcggtcgccggaaggatcagtgccggaatcaatgtatgagcctgtaaataccagctccccatgacactcaaccagccaaagaaaaccagtacggaaatatcacccagaccgatataaccataaggacgattgcccacggtgtaggtgatagcggcaatgatcgacaacccgccaagaatcaggaaaccgacaaaatcggccagcgtatggcatgccactgcaaccagtgccagcccggagagacagatgagcacgacggtaataatgagcgcccgtttcatctcttgctgggtaatgacccctttttgcatgccgcgtagcggcccaatgcggtcaggtttatcgctgccttttaccgcatcgccgtaatcattggcgaggttagaaaggatctgtaatagcccggcggtaattagtgccagcagggcgaccagcggatcgaagtgaccttgccaccatgccagcgctgtcccgacgataattgcagcaaaggcgagggggagggttttaggtcgtaaactttccagccacgcctgagttcggctaatttgttgttcagtcataatacgcgccaataaaaatggggcctttcagccccatcaaacaatgatgaaaatgattgaacgcgattataggataaaacggctcagatcttcatctgccaccaacgcatccagatgtttgctcacataatctgcgtcaatagtgatattttgaccgcttaaatcgctggcgtcgtaggaaatctcttccattaaacgctccagaacagtgtgtaaacgacgagcaccgatgttttcggtagattcgttcacctgccatgccgcttccgcgatgcgtttaataccggagtcggtaaactcgatatttacgccttcagtcgccatcagtgctttgtactgcacggtgatagaggcattcggctcggtcagaatacgctcgaagtcgctggtggtcagcgcctgcagttcaacgcggattggcagacgaccttgcagttccgggatcaggtcagacggtttcgcaatctggaacgcgccagaagcgataaacagaatgtggtcagttttgaccatcccgtgtttggtggaaacggtgcaaccttctaccagcggcagcaggtcacgctgaacgccttcacgagaaacatccggaccggaagactcgccgcgcttacagattttgtcgatttcgtcgataaacacgatcccgtgctgctcaacagcgtcgatagcgtcttgcttcagctcttccgggttcaccagtttcgccgcttcttcttcaatcagcagcttcatggcgtctttgattttcagcttacgcgctttttgcttctggccgcccaggttctggaacatggactgcagctggctggtcatctcttccatgcccggaggagccataatttcaacgcccatcggtgctgcggcaagatcgatctcgatttctttgtcatcaagctggccttcacgcagttttttgcggaatgcctgacgagcagcggacggttcctgctgctgttcggtctgtccccagttgtttttagcaggtgggatcagcacgtcgagaatacgttcttctgccagttcttcagcgcgataacggtttttctcgatagcctggacgcgtaccattttcacggcggcatcggtcagatcgcgaataatagaatccacttccttaccgacgtagcccacttcggtgaatttggtcgcttcaactttgatgaacggcgcattcgccagcttagccagacgacgggcgatttcagttttaccgacaccggtcgggccgatcatcaggatatttttcggggtcacttcatggcgcagctcttcgttgagctgcatgcgacgccagcggttacgcagagcaatcgccacagaacgcttggcgttgtcctggccgatgatgtgcttatccagttcgctgacgatttcgcgtggggtcatttcagacatgggagatccttacgctttgtagcttaattcttcgatggtgtggaaatggttggtatagatgcaaatgtcgcctgcaatatccaacgccttttcagcaatttcacgggcgctaagttcagtgttttctaacagcgcgcgcgccgcagcctgggcgtaagggccgccggagccgatagcaataagatcgttttctggctgcaccacgtcaccgttaccggtgatgataagcgatgcagtttcatccgcgactgccagcagtgcttcaagtttgcgcagcatgcgatcggtacgccagtcttttgccagctcaacggcggctttgaccagatggccctgatgcatttccagtttacgttcaaacagttcgaacagcgtaaaagcatccgcagtaccgcccgcaaagcccgcgatgactttgtcgttgtacagacggcggacctttttcacgttgcctttcattacggtattgcccaacgtggcctgaccatcaccagcgatgaccacatggccgttacggcgtacgcttactatagttgtcacgagctgaccccttggttacgaatacagagtacaaaccccgtacaaaagtacggggcataatgcaattatagatgggggggattttgagggtttcaacccccggcggcgagccgaatgcagtttgtatgacccgccatcttcaaccgattgagggtgctgtctgcgttctctttgcctttcaccgggccaatgaccacacgattccagccattgttggtggtgattttcgagtcaaagccttcgaacgccagctgagcacgtaccgtctctgcctgttccgcgcctctgaacgaaccgcactgcaccatccagcggcgttcgtcttttttctccgccgtcggttttggcgcgtcagcggcacgagcaactggcgcagcttgctgcggcttcgactgcgcagtcgtgtgcgcaggagtttgcagcagatcctggtacggctgctgagaagaagccggtttagactggcgcggttgcgcctgtaccggtgcggcttgcgacgtacgcgtctgctgctgccagctttgttcagtcgtacgcgactgctgagccaggcgttgctgttccgctaattgctgcgcctgacgttggcgctgtagcgtttgctgacgctgttccggcgtctgttcattccacggaacttcaaccagctgcgttggctgctggcgcatatcagcctgcatttgttcaagaagctgacgttgttctggtgtcagttgctccggcgttttcacttcaccaccggcagaaggttctgtgggcgcacgcactcccggctggcgactttccagctctttaatgtagcgccagcgttcttctggttttggtggtagtccgtttccggtcactttctggctttgcagcgtctcggactcttctttcttgtgatgcgtaatgaagtacagaccaccgataaaggtcacaagaacggcggcagcaatagcgaccatagcgggagaaaccgcaggcagatttcgttgctttttccgtgaggtgctcttttttcgccgcgaaggtgccggttggctgcggcgtacataatctcgttgtgccactatcgtttcgctgtatttattcgttcgtcagcccgccatgttacttaagcggcgggcctttgaccagtcacggcagtcttaaaggtttactttaaggtaacgcgcgtgttgatccccggatgataagttcgcagtccattaaacgagagccactgccaacgtgttgcccctgcatttgatcaagcaataacagcatagcttcccgaccgatttcgtaacgcggctgcgcgatggttgtcagcggcggatcacaaaattgcgtcaggtcgatgttatcaaaaccgattatggaaaggtcttccgggactttcagcccctggcgttttgcctgagaaagtgcgccgagcgccatcacatcgctatggcagaagacagcagtaggcggttgtggaagatcaagcagctgctgcatcgctttgcttccggcttcgaaggtgaagtcgccacgggcgatgtattgcggatcaaccataatgccgcagcgacgcagcgcctgaacatagccttgcaggcggtagtgacacagcggcatctcttcgggaccggctatacagccaatccgtttatgcccttgctcatataaataatttactgcatcaaatgcggcggtcagattgtcgatatgaactgtaggcagctccagctccggtgcaaattcgttcgccatcaccatcggcggcagattacgctgttcctcaatgctggcatcaaacggcagccttgaacccagcaacaacatgccatcaatttgcttggtgatgatcaaatcgataaaggttttttcctgctgattttgatgcgcacagtcgccaatcagcaccagatatccgtgatttgccgccgtaacttcgataccgcgaataatttcgctaaagaagggatcgcagatatccgggacaatcaccagaatggtgcgggattcattacgcttgacgttgcgccccataggctgcggtaaataacccacttcccgggccgctttttcaacccgattacgggtggcctgggagactttatcgggattcattaatgctcgggagacggtcgctgtagagacttttgccttgagggcaacgtctttcatggtcgcggcagtttcctgcttcttcgctttcacactcactcctcgcctggcacgtcaggcgtactacatccatgtttacttcacatcggcaacatttttagcagatagcgcgtgaaaacggttacagaattttcatgaaaagtgtgatgaatattgaatttttcgatccgcctcgcatcgtgagcggtttaaccctcaatcggatcaacatccagcacccatttcaccttacgggaatccggtattgtattgatgagcgccagcgtaccgttaatgatgtgttgcaagcgcacgcgggaagggtgctgcaacaatatctgccagcgccagcgaccgccacgtttaggtgccagagccggaaccggaccgagaacccacagtttctcgtctgccagtgggctggagaggatcagattacgcagttgttgcaggaacaatggcgcgtgctgattgttatgatcttccgcacgcacaatcacatggctggtccacggcggtagctgcatcattcgccgctcagccagcgcctgttcggcaaaggcgtcgtagcctttatagagcaacgtttgcaacagaggatgttccggatggtgcgtttgcagcaccacttcgccctgtttacccgcacgcccggcacgaccggcgacctgggtgtaaagctgagcgaaacgctctgccgagcgaaaatcggcagaaaacagcgcgccgtccacgtccagtaatgcaaccagcgtcacatccgggaaatggtgacctttcgccagcatttgtgtaccaatcaaaatccgcgcgccgccgcgatgtacttctgccagttgctgttccagcgcccctttgcggctggtggtatcgcggtcgatacgagaaatgggcacgccggggaacaacggcgcgagcgtctgttcaagctgttcggtgcccagccccacggggaccaggtgcgtggaaccgcaggaagggcactggcgcggcaccggacgctgactgtcacagtggtggcagcgcagatggtgctgcgcctgatgcagcgtgtagtagtgatcgcaacgtgggcattcggcaatccagccacagtcgtggcacagcagtgcaggcgcaaagccacggcggttaagaaagagaatgacctggttatcagcctgtaaatgctggcgcatacgagtgattaacgccggagccagacctgcctgcaccttctgaccttttaaatccagcacatgttgaattgccggacgcgcattccctgcccgacgggtcaggcgcagcaggcggtattttttctgctggacgttgcataacgtttccagcgcgggcgttgcggagccaagaataatcgggatttgctcgctgtgcgcacgatacaccgccaggtcgcgggcatgatagcgccagccttcctgctgcttgtaggagctgtcgtgctcttcatcaatgacaatcacgccgagatttttaaacggcgtaaacagcgcggagcgggtgccgatcacaatcgccgcctcaccatttttcgctttcagccacgccgaaagacgctcgctgtcgttcaggccggaatgcagaacttccacgggggcattaaaacgttcacgaaaacgggcgatagtttgcggtgtcaggccgatttccggcaccatcaccagcgcctgtttgccctgagcgagcacgttttccagtacgctgagataaacctccgttttaccggaaccggtaacgcccgccagcagccaggcagaaaaagtatctgccgcgctatgaattgcgccaacggcggtggcctgttcggtattcaatcgcaaccgctcaccagaaacggcatagttcgttcgccagtcgctaaactctggtgtttcacttgctaaatcacacagaccttttttgcgtagcgcctgcaacgcggcatcattaaattcgagcgtggcgacctggtcgcgccagattttgccttgccgtaacgccgccagcgcctgttgttgcttgggggagcgtttcaggctgttcagatccaccgcctggccttgttcagtggcaaaccagtaccacatcggcgcgttcgccgcaggccgcccctggcgtagtaaaatcggcaaggcatgaaacagcacatcgccaatcggatgatgatagtaatctgccgcccatagcagcaatcgccagacggagtgagtaaacaccggctcactatccagcacttcgactaccgcttttagctcattgagcggcagttcgctggcatcgctaactgataccacaatcccgatgcgctcctgctgtttgccaaacggcacgcgcacgcgacacccagctttaaccgtcatgccttctggcagcagatagtcaaaggtacgaggaagcggaacgggcaaggcaacgtgggcaacgggcatagcatcatcctgacttgaaattcggtgggttagtatacacattgccgtagaagagtgcggatcagtttgcatacgctggttaatttctgtatgatttcgcgccttcgtacgaaatgatcgtattgaagctatacttttaacatcgcgtggtgtctggcgttagggctggaagagcgacgcggccttaaaccgaggttttcccatgaaaaaagatattcacccgaaatacgaagaaattactgctagctgctcttgcggtaacgtaatgaaaatccgctccaccgttggtcatgacctgaacctcgacgtgtgcagcaagtgccacccgttcttcactggcaaacagcgtgatgttgctaccggtggccgtgttgaccgcttcaacaagcgtttcaacatcccgggcagcaaataagaccggatttccgaaaaaagcgccgcacggcgctttttttgtgcctgaattttggtcgtattaccacgaaaacagcggccattctttggcgaccgtggtgagttgtggcgcatcgaaaacggcttgtggcgagaccaccgtttcctcaagcggaatattcttgccgtaacgttctttgagctttgcctgaacttgtgggctgctcaggtcgaactctttcaacttctgctgctcgcccacgcgcattcccagcgcgttctggtaaaccttccacaccacttccgaacagtactggcgatcgtcgctccatgagaagctgaaatcatacggtttaccgagataacgttttgccgtttgcgccagtttttgctgttgttcaacactcagtccgccttcaacgcggcgaacaacgtatttgcccttttcaccatgggcgatccactgcttgagcggggtgtatttcaccgggccgactgcttcaaaaacgtagggctttttgttgcgtatcaccagcataccggtgtggctataatcggtatgggtcgccagttggatcgctttactttgcgatgagcgagagatctgaaagatgatgtcgccggtttgtggctgccaggcaaaggcaggtacagaaaccagcaggctgaggatcagcagcctgtttttcatagttaaacgtccatgtataaaaagcggtgggtcgcagacaacgtgctcgttgtttatgccggatgcggcgtgaacgccttatccggcctacaagttcgtgcaaattcaataaattgcaatatgacgtaggcctgataagcgtagcgcatcaggcgattccactccgcgccgctcttttttgctttagtattcccacgtctccgggttaatccccatctcacgcatgatctcttttgccgcttccgggatttcgtcgctgcgctctttacgcagatcggcatcatccggcaaaggttgcccggtaaaggcatgcagaaacgcttcgcacagcagctcgctgttggtagcgtgacgcaggttgttcacctgacgacgcgtgcgttcatcggtgaggatttttaacaccttaagaggaatggaaaccgtaatctttttgacttgttcactcttcttgccgtgctcagcgtatgggctgatatattcgccgctccattcagccatgagatacttaatcctcttcgtcaataaattgagaccagaccacacagttgatgtgggtactgaccgtaaacccgcatagtttaccgtacaggcgttaccgtgacatcgtgtaatgcacctgtcggcgtgataatgcatataattttaacggctatttgggatttgctcaatctatacgcaaagaagtttagatgtccagatgtattgacgtccattaacacaatgtttactctggtgcctgacatttcaccgacaaagcccagggaacttcatcacatgacgcgtaaacaggccaccatcgcagtgcgtagcgggttaaatgacgacgaacagtatggttgcgttgtcccaccgatccatctttccagcacctataactttaccggatttaatgaaccgcgcgcgcatgattactcgcgtcgcggcaacccaacgcgcgatgtggttcagcgtgcgctggcagaactggaaggtggtgctggtgcagtacttactaataccggcatgtccgcgattcacctggtaacgaccgtctttttgaaacctggcgatctgctggttgcgccgcacgactgctacggcggtagctatcgcctgttcgacagtctggcgaaacgcggttgctatcgcgtgttgtttgttgatcaaggcgatgaacaggcattacgggcagcgctggcagaaaaacccaaactggtactggtagaaagcccaagtaatccattgttacgcgtcgtggatattgcgaaaatctgccatctggcaagggaagtcggggcggtgagcgtggtggataacaccttcttaagcccggcattacaaaatccgctggcattaggtgccgatctggtgttgcattcatgcacgaaatatctgaacggtcactcagacgtagtggccggcgtggtgattgctaaagacccggacgttgtcactgaactggcctggtgggcaaacaatattggcgtgacgggcggcgcgtttgacagctatctgctgctacgtgggttgcgaacgctggtgccgcgtatggagctggcgcagcgcaacgcgcaggcgattgtgaaatacctgcaaacccagccgttggtgaaaaaactgtatcacccgtcgttgccggaaaatcaggggcatgaaattgccgcgcgccagcaaaaaggctttggcgcaatgttgagttttgaactggatggcgatgagcagacgctgcgtcgtttcctgggcgggctgtcgttgtttacgctggcggaatcattagggggagtggaaagtttaatctctcacgccgcaaccatgacacatgcaggcatggcaccagaagcgcgtgctgccgccgggatctccgagacgctgctgcgtatctccaccggtattgaagatggcgaagatttaattgccgacctggaaaatggcttccgggctgcaaacaaggggtaaaaatgagtgtgattgcgcaggcaggggcgaaaggtcgtcagctgcataaatttggtggcagtagtctggctgatgtgaagtgttatttgcgtgtcgcgggcattatggcggagtactctcagcctgacgatatgatggtggtttccgccgccggtagcaccactaaccagttgattaactggttgaaactaagccagaccgatcgtctctctgcgcatcaggttcaacaaacgctgcgtcgctatcagtgcgatctgattagcggtctgctacccgctgaagaagccgatagcctcattagcgcttttgtcagcgaccttgagcgcctggcggcgctgctcgacagcggtattaacgacgcagtgtatgcggaagtggtgggccacggggaagtatggtcggcacgtctgatgtctgcggtacttaatcaacaagggctgccagcggcctggcttgatgcccgcgagtttttacgcgctgaacgcgccgcacaaccgcaggttgatgaagggctttcttacccgttgctgcaacagctgctggtgcaacatccgggcaaacgtctggtggtgaccggatttatcagccgcaacaacgccggtgaaacggtgctgctggggcgtaacggttccgactattccgcgacacaaatcggtgcgctggcgggtgtttctcgcgtaaccatctggagcgacgtcgccggggtatacagtgccgacccgcgtaaagtgaaagatgcctgcctgctgccgttgctgcgtctggatgaggccagcgaactggcgcgcctggcggctcccgttcttcacgcccgtactttacagccggtttctggcagcgaaatcgacctgcaactgcgctgtagctacacgccggatcaaggttccacgcgcattgaacgcgtgctggcctccggtactggtgcgcgtattgtcaccagccacgatgatgtctgtttgattgagtttcaggtgcccgccagtcaggatttcaaactggcgcataaagagatcgaccaaatcctgaaacgcgcgcaggtacgcccgctggcggttggcgtacataacgatcgccagttgctgcaattttgctacacctcagaagtggccgacagtgcgctgaaaatcctcgacgaagcgggattacctggcgaactgcgcctgcgtcaggggctggcgctggtggcgatggtcggtgcaggcgtcacccgtaacccgctgcattgccaccgcttctggcagcaactgaaaggccagccggtcgaatttacctggcagtccgatgacggcatcagcctggtggcagtactgcgcaccggcccgaccgaaagcctgattcaggggctgcatcagtccgtcttccgcgcagaaaaacgcatcggcctggtattgttcggtaagggcaatatcggttcccgttggctggaactgttcgcccgtgagcagagcacgctttcggcacgtaccggctttgagtttgtgctggcaggtgtggtggacagccgccgcagcctgttgagctatgacgggctggacgccagccgcgcgttagccttcttcaacgatgaagcggttgagcaggatgaagagtcgttgttcctgtggatgcgcgcccatccgtatgatgatttagtggtgctggacgttaccgccagccagcagcttgctgatcagtatcttgatttcgccagccacggtttccacgttatcagcgccaacaaactggcgggagccagcgacagcaataaatatcgccagatccacgacgccttcgaaaaaaccgggcgtcactggctgtacaatgccaccgtcggtgcgggcttgccgatcaaccacaccgtgcgcgatctgatcgacagcggcgatactattttgtcgatcagcgggatcttctccggcacgctctcctggctgttcctgcaattcgacggtagcgtgccgtttaccgagctggtggatcaggcgtggcagcagggcttaaccgaacctgacccgcgtgacgatctctctggcaaagacgtgatgcgcaagctggtgattctggcgcgtgaagcaggttacaacatcgaaccggatcaggtacgtgtggaatcgctggtgcctgctcattgcgaaggcggcagcatcgaccatttctttgaaaatggcgatgaactgaacgagcagatggtgcaacggctggaagcggcccgcgaaatggggctggtgctgcgctacgtggcgcgtttcgatgccaacggtaaagcgcgtgtaggcgtggaagcggtgcgtgaagatcatccgttggcatcactgctgccgtgcgataacgtctttgccatcgaaagccgctggtatcgcgataaccctctggtgatccgcggacctggcgctgggcgcgacgtcaccgccggggcgattcagtcggatatcaaccggctggcacagttgttgtaatttcagaaatttaataatgcccggtactcatgttttcgggtttatggtttctaatgaaatatattgaattatcataggattaggccggattaagcgtttacgacgaatccggcaagaagcaataagtacatggttagtttatatttgcagtccggtttgctttgcataccggattttctttttcttaccatcctgaagttttttcatcttccctgatttttcctcaccatcattggtcatttttcggttgacgcccttcggcttttccttcatctttacatctggacgtctaaacggatagatgtgcacaacacaacatataactacaagcgattgatgaggtaaggtatgagcttttttcacgccagccagcgggatgccctgaatcagagcctggcagaagtccaggggcagattaacgtttcgttcgagtttttcccgccgcgtaccagtgaaatggagcagaccctgtggaactccatcgatcgccttagcagcctgaaaccgaagtttgtatcggtgacctatggcgcgaactccggcgagcgcgaccgtacgcacagcattattaaaggcattaaagatcgcactggtctggaagcggcaccgcatcttacttgcattgatgcgacgcccgacgagctgcgcaccattgcacgcgactactggaataacggtattcgtcatatcgtggcgctgcgtggcgatctgccgccgggaagtggtaagccagaaatgtatgcttctgacctggtgacgctgttaaaagaagtggcagatttcgatatctccgtggcggcgtatccggaagttcacccggaagcaaaaagcgctcaggcggatttgcttaatctgaaacgcaaagtggatgccggagccaaccgcgcgattactcagttcttcttcgatgtcgaaagctacctgcgttttcgtgaccgctgtgtatcggcgggcattgatgtggaaattattccgggaattttgccggtatctaactttaaacaggcgaagaaatttgccgatatgaccaacgtgcgtattccggcgtggatggcgcaaatgttcgacggtctggatgatgatgccgaaacccgcaaactggttggcgcgaatattgccatggatatggtgaagattttaagccgtgaaggagtgaaagatttccacttctatacgcttaaccgtgctgaaatgagttacgcgatttgccatacgctgggggttcgacctggtttataaatagtgtggcttttgtgaaaatcacacagtgatcacaaattttaaacagagcacaaaatgctgcctcgaaatgagggcgggaaaataaggttatcagccttgttttctccctcattacttgaaggatatgaagctaaaacccttttttataaagcatttgtccgaattcggacataatcaaaaaagcttaattaagatcaatttgatctacatctctttaaccaacaatatgtaagatctcaactatcgcatccgtggattaattcaattataacttctctctaacgctgtgtatcgtaacggtaacactgtagaggggagcacattgatgagcacgtcagacgatatccataacaccacagccactggcaaatgcccgttccatcagggcggtcacgaccagagtgcgggggcgggcacaaccactcgcgactggtggccaaatcaacttcgtgttgacctgttaaaccaacattctaatcgttctaacccactgggtgaggactttgactaccgcaaagaattcagcaaattagattactacggcctgaaaaaagatctgaaagccctgttgacagaatctcaaccgtggtggccagccgactggggcagttacgccggtctgtttattcgtatggcctggcacggcgcggggacttaccgttcaatcgatggacgcggtggcgcgggtcgtggtcagcaacgttttgcaccgctgaactcctggccggataacgtaagcctcgataaagcgcgtcgcctgttgtggccaatcaaacagaaatatggtcagaaaatctcctgggccgacctgtttatcctcgcgggtaacgtggcgctagaaaactccggcttccgtaccttcggttttggtgccggtcgtgaagacgtctgggaaccggatctggatgttaactggggtgatgaaaaagcctggctgactcaccgtcatccggaagcgctggcgaaagcaccgctgggtgcaaccgagatgggtctgatttacgttaacccggaaggcccggatcacagcggcgaaccgctttctgcggcagcagctatccgcgcgaccttcggcaacatgggcatgaacgacgaagaaaccgtggcgctgattgcgggtggtcatacgctgggtaaaacccacggtgccggtccgacatcaaatgtaggtcctgatccagaagctgcaccgattgaagaacaaggtttaggttgggcgagcacttacggcagcggcgttggcgcagatgccattacctctggtctggaagtagtctggacccagacgccgacccagtggagcaactatttcttcgagaacctgttcaagtatgagtgggtacagacccgcagcccggctggcgcaatccagttcgaagcggtagacgcaccggaaattatcccggatccgtttgatccgtcgaagaaacgtaaaccgacaatgctggtgaccgacctgacgctgcgttttgatcctgagttcgagaagatctctcgtcgtttcctcaacgatccgcaggcgttcaacgaagcctttgcccgtgcctggttcaaactgacgcacagggatatggggccgaaatctcgctacatcgggccggaagtgccgaaagaagatctgatctggcaagatccgctgccgcagccgatctacaacccgaccgagcaggacattatcgatctgaaattcgcgattgcggattctggtctgtctgttagtgagctggtatcggtggcctgggcatctgcttctaccttccgtggtggcgacaaacgcggtggtgccaacggtgcgcgtctggcattaatgccgcagcgcgactgggatgtgaacgccgcagccgttcgtgctctgcctgttctggagaaaatccagaaagagtctggtaaagcctcgctggcggatatcatagtgctggctggtgtggttggtgttgagaaagccgcaagcgccgcaggtttgagcattcatgtaccgtttgcgccgggtcgcgttgatgcgcgtcaggatcagactgacattgagatgtttgagctgctggagccaattgctgacggtttccgtaactatcgcgctcgtctggacgtttccaccaccgagtcactgctgatcgacaaagcacagcaactgacgctgaccgcgccggaaatgactgcgctggtgggcggcatgcgtgtactgggtgccaacttcgatggcagcaaaaacggcgtcttcactgaccgcgttggcgtattgagcaatgacttcttcgtgaacttgctggatatgcgttacgagtggaaagcgaccgacgaatcgaaagagctgttcgaaggccgtgaccgtgaaaccggcgaagtgaaatttacggccagccgtgcggatctggtgtttggttctaactccgtcctgcgtgcggtggcggaagtttacgccagtagcgatgcccacgagaagtttgttaaagacttcgtggcggcatgggtgaaagtgatgaacctcgaccgtttcgacctgctgtaatctgaccccgttcagcggctgcttgctggcagtcgctgaacgttctttaccagcgtatagtgggcgaacgaaaactacacactggatctctcatgtctgccgcaggaaagagcaacccactggcaatcagtggcctggttgtgctcacacttatctggagttatagctggattttcatgaagcaagtcaccagttacatcggtgccttcgactttaccgccttacgctgcattttcggcgctctcgttttattcatcgtccttttattacgtggtcgcggaatgcgcccgacaccgtttaaatacaccttagccattgccctgttacaaacctgcgggatggttggtctggcgcagtgggcgttggtcagcggaggtgcggggaaggtggcgatcctgagctataccatgccgttctgggtggtgattttcgccgcgttgtttctcggtgaacgcctgcgacgtgggcaatatttcgcgattctgattgccgctttcggcttatttttggtgttgcagccgtggcaactcgatttctcttcgatgaaaagtgccatgctggcaatcctctccggcgtcagttggggggcgagcgcgattgttgctaaacgtctgtatgcccgtcatccgcgcgtggatttattgtcgttaacatcctggcagatgctgtatgcggcgctggtgatgagtgtggtcgctttactggtgccgcaacgtgaaattgactggcagcccaccgtgttctgggcgctggcctacagtgcgattctggcgacggcactggcgtggagcttatggttgtttgtattgaaaaacttgcctgccagtattgccagcttaagcacactggccgttcccgtttgcggcgtactcttttcctggtggctgctcggcgagaatccgggggccgttgaaggtagcggtattgtgctgattgtgctggcactggcgctggtgagccgtaagaaaaaagaagccgtcagtgtaaaaaggatctgaattttttcttcatgtggggcgatctcttatttaacaaaataacgataatgccccaccatccgccagttaaacagcacatcttcttcctgcgcgcctgcgccaatgttatgtatcaccagcggcgtaccgtcgcgggcgaagccatctgaaaccaccccaatatgtgccagcccgttatccagtcgccaggagacaatatcgcccgcttgatagtcactggggttcttgctggtggggcgtgttttatcatggcggctaaaccaggtttccagattaggcacccgacggtgatcgatgttgctgtccgggcgctttaacttccatttttgcgggtactcagcaaaattcttcgccatatcttcgtgaaccagtttctgcaaatcgaccttctggctgcgcaatgcgcggatcaccacatcggaacatacaccgcgttcttgcggaacatcaccgccaggataagtaagctgcacatacgccggatcgtaaaatagcgtgctgccaatttgctgtctggcaccgtctgcgatggcaaggttggtattggcctggatttgtaccacggttggtggaacggcgggagattttaaggagtggctggtaaatgccgttagcaggctgagcagcgccagtgaagctttcatctggttcgtccgtgaaaataagagtcacagattcgaccttccgggctaacgattgttctgtagagaaaatgtccagaagcggataaaaaattcctgaacaacgtgggagtttcagattactggcacagagtgccggatgcggagtgaacgccttatccggcctacaaaagcacgcaaattcaatatattgcagagattgcgtaggcctgataagcgtagcgcatcaggcaattttgcgttcaaactcccggacaagccgggagtttggagtaggttattcccactcttgcaggaaacgctgaccgtactggtcggctaccagcagagcggcgtaaacctgatctggcgtcgcgccgccaggcatgttgtgaatggtttcaccttctgcacatgccgcttctgccacaattcgcattttcgccgggacatcttctttaatatccagttgagcgagagttattggcaaacctaccgcatggctaagggcagctacggtttcgatttcctccaccggcgcattttccagaaccagctgcgtcagcgtaccgaatgccactttttcaccgtgataatagtgatgcgcgtccgggatagcggtcaggccgttatgcactgcgtgcgccgcagccagaccaccactttcaaaaccaacaccgctcaaataggtgttcgcttcaatcacgcgctccagcgccggagtcactacatgctgttcggcagcaagcatcgctttttcgccttcttccagcagggtgttgtagcacagttcagccagtgccagcgcagcctgggtgcacttgccgcccgccatggtggtcgcgccgctacgagagcaggcacgcgcttcaaaccaggttgccagcgcatcgccgatacccgccgctaacagacgtgcaggtgcgccagcgacgattttggtgtcgacaatgaccatattcgggttatttggcaacagcagatagcggtcaaactcaccctcatcggtgtagataacagacaatgcgctgcacggtgcatcggtagaggcgatagtcggtgcgatcgctaccggaacacccatgaaatgtgccagtgctttggcagtatcgagggtttttccgccaccgataccgagaattgcgccacactgcgcagtctccgcgatgccacgcagacggtcgatctcattttgcgaacattcaccgccaaacggcgcaatttctactaccagtccagcatctttaaagcttttctcgacagtggattgagcaaaacctaaaacaaatttgtcacccaccactaaccagcgttctgccagcggcttcaggtattcgcccagacgattaatcacatcagcgccctggatgtatttacccggtgattgaataatgcggtccataattgctcctttagagatgagtagtgccaaatgcggcattccagtcgtgttcgaacttctctatagctgactctaccgcaggggtgttgagcatttgttgcgctacatctaagggcagggtgatggattcacatcctgccagtaaacagtccagcgcctgacgcggcgttttaaagctggctgccagcaccatgctttctggcgcgtgcatttctaacagcgtttgcagctcctgaaccgtacgaatgccgtctccgccctgggcatctacgcggttaacatacggagcaacgtattttgcccctgccagtgcggctaataacccttgtgcggcgctatatacagcagtgccaagtgtagtaataccctcttttttcagtattttaattgctgccagaccttcggaagtcaccgggattttcaccacaatacccggaatagcgtcgcgcaggcgcttcgcttcttccaccatcccctgcgcgtcgcggctcatggtctgagcaaacagaatgccctcatcaccaatcgctttttgcagacgcggcagcacttcccatatggactccttgctggcagcgataatgctcgggttagttgtcaccccggcaatggggaatatgcgtgccagacgttcgacttctgcgacgttagcggtgtccagatacagttccatgatgtttccttttacagttccagttcatgttgcagcaggctggcgatagcgtcggcagaggcggcgttaaccagcgcgttacggaattcttcgtgcatgatgcggcgagcgaggcgcgagaaaatgcgcatatgctgatcgcccgcagcgtgtttgttcagggttaacataatgatgaattgcgcttcatcatcgccccagcgcaccggcgcttgcagacgcgccacgctgatggtggattgctcaatgtgttctgatttgctgtgtggaatggcaaaactaaagcccagaccggtagagaaaacggcctcgcgcgcccacaagtcggcttccagtttacgcggatagcggcagcggcccgccagcagcaggttatcggtcatgcctttgagcacttcttctttgctgcgccagtcgctttccagtgtgatgcactcggcggtgaccagcggtgcgtcttgttgggtcatgcggaattgcgccagcaggtgttctacttccagcgaagtacggcaggccattgcctggttgagcaacttgcggcactcacggctatcaagttgcgccatccgagctttcgccgccggaattgatggtgcgctcatgctgagttcatccagccctaagccgaccagcaacggcagcacggaacctttcgctcccagctcaccgcacagaccaatccatttgccctggcgatgcaccgcttgcacggcgtaatcgagcgcccgcaagaatgccggattcaggctgttgtagtgacgagtaaccttagcgttatcgcgatccaccgccagcagatactgcgtcaggtcattactaccaatactaaagaaatcaatctcttcgcagcattgatcgatgatgaacatcaccgacggcacttccagcatgatgccgagctggattttctcatcaaacggaatgtgttcgttacgtagttgctgtttggcttccgccagtttttctttcacccataagatctcttccattgaggagatcatcgggatcatgattttcaggctgccgtgagcggaggcgcggaggatcgaccgtagctgcgtggtaaacaacgacgcgtactcttcataaatacgcacggcgcgataaccgaggaacgggtttgcctctgcgggaatgttcagataatcaacgggtttgtcgccgccaatgtccatagtgcgcacaataatgctgcgtccgttggcggattccagcgcctgacaaaaaatgttgtacaactcgctttcgcccggtgcgctggtgcgatccatatagagcatttcagtgcggaacaaaccaacgccttccgcaccattgccgaatgcggcctgcgcttccacggagtgagcgatgttagcggcaatttcaatgcggataccgtcagcggtacgggcttgttgggtcagccagacacgctgttgctcacgcagggcgtcctgtacgcgggcttcttgctgataataacgagctacggcttcccctggctcaaccacaatcgccccggcgttgccgtcgatataaatcgtttgttgctgccacggagtaagggcatcaatatccacaccaaccagcgttggaatgttgaacgaacgggcaaggatcaccgtatgtgaggtggtgccgccgcttttgagcaacaatcctttgaggtgatttttatccagttcgaggaactggctgggggtcagttcatcagccatacaaatggcgggctgcgtcagtttgcccggtgccgggaagcgttgctcaccgtagatttgctggagtaactggaagcagacgtcgcgtacgtccagggcacgttcttgcaggtagctgctgctggaacgggaaaactcttcgcaaaagtgattcgcgctggcaacaattgcttcggcgcagcttaatccggcgctgacgcctgccagtaaatgttcgcgcagggaagtatcgccagccagggatcggtgagcttccagaatcgcgctggtagcaccgtcgctatccagcagacgaaactcaatgtttttcagtaccagcgtcaggccgttttccagtgcggattgctcggcgtcaacgcctttggctgcgggaagattacccagcgcattgagatctaaagaagagatcggcgtcagaatgccgcctgcactaccgctgcacacggtgcgggcgcggataatttgcggattcagattggtcagtgaaaccggcagtggttccagttcgtcagatttaacttccgccagcggcgcatcgcagtgggggaattcatcgcgcagccattggcttaaacgctggtgcgcttcctgttcgtcggccccggaaatcagtaactggcagttatcgcccgccagcgtatcggtgccaatcagcgcaagggcgcttttggcgttgcccttgcggtcagtgcgcaggttatgccactcaatttgtgatgaaaaagtattacacagcgtttcaacgtggcttgccggacgcgcatgtacgccgttaggtagctcacaaataaattccacaatcagggccattgcctctctcccggtacggttttctgtttacaggataagagcgcacggcaacggcctgccatgtgacaaatctgccaaaagctggacaaatgtaatgtaaccgtcaatttgcgacgcgtctcacaagacgctgttttgcggcatgcttccggtttatcgcaagttatgaggcggatcgcatttttgtactgatattacaaaagtccagtaaatggcctttttatccactgtttgctccgcctgcgattgcctattgtttcctccatcaaaaatatggacatgggctttcgcaagcccgggagcagcttatgaatgagttggtgcagatcctgaaaaatacccgtcagcatttaatgacgggcgtttcacacatgattcccttcgtggtatcgggcggtattttgctggcggtttccgtcatgttgtatggcaaaggcgcagtgccggatgccgtagccgatccaaatctgaaaaaactgtttgatatcggcgttgcgggcttgacgctgatggtgcctttcctcgcagcgtacatcggttattccattgcagagcgttctgcgctggctccgtgcgctatcggtgcctgggttggtaacagctttggtgcgggcttctttggtgcactgatcgccgggattatcggcggcatcgtggtgcattacctgaagaaaattccggtgcataaagttctgcgctcggtgatgcctatcttcattattcctatcgtcggcacactgattaccgcaggcatcatgatgtggggcttgggcgagcctgtaggggcgttgaccaacagcctgactcagtggcttcaggggatgcagcagggcagcattgttatgctggcggtgatcatgggtctgatgctggcgttcgatatgggcggtccggttaacaaagtggcctatgccttcatgctgatttgcgttgctcagggtgtttataccgtggtggccatcgctgccgtgggtatttgtatcccgccgctggggatggggctggcgacgctgattggtcgtaaaaatttctccgcagaagagcgcgaaaccggcaaagcggcactggtgatgggctgtgttggcgttactgaaggggcgattcctttcgccgctgccgatccgctgcgtgtcattccttccatcatggtcggttcagtttgtggtgcagtaactgcggcgctggtcggtgcgcagtgctatgcaggctggggtggtctgattgtgctgccggtggttgaaggcaagctgggttatatcgcagcagtggctgtcggagcagtggtgacggctgtttgtgtgaacgtgctgaaaagtctggcgcgtaaaaatgggtcttcgactgatgaaaaagaagacgacctggatttggattttgaaattaattaattgaggaacgagccatgacgaaaattattgcagtaaccgcatgtccttcaggtgttgcccatacctatatggcagcagaggcgctggaaagtgccgcgaaagcgaaaggctgggaagtgaaagtagaaacccaggggtcaattggtctggaaaatgaactgactgcggaagatgtggcgagcgctgatatggtgattctgaccaaagatatcggcatcaagtttgaagagcgttttgctggcaagaccatcgtgcgcgtcaacatcagcgatgcagtaaaacgtgctgacgccattatgagcaaaattgaagctcacctggcgcaaaccgcttaagttcttctcccgctcgcaagggcgggttcgctttcccacaggagttcctcatgacgaatcgtatctctcgcctcaaaactgcactgtttgccaatacccgtgaaatctcgctggagcgggcgctgctttataccgccagccatcggcaaaccgaaggcgaaccggtgatattgcgccgggcgaaagcaacagcgtatatccttgaacatgttgaaatttcgattcgtgatgaagaactgattgccggtaaccgcaccgtaaaaccgcgcgccgggattatgtcgccggaaatggacccttactggctgctgaaagagctggatcaattcccgacgcgtccgcaggaccgctttgctatcagcgaagaagataaacgtatctaccgtgaagagttgttcccgtactgggaaaaacgttcgatgaaagatttcatcaacgggcagatgacagatgaagtaaaagccgcgaccaacacgcagattttcagcatcaaccagacggataaaggccaggggcacattattattgattacccacgcctgttgaatcacgggctgggtgagctggtggcacagatgcagcaacattgtcagcaacagccggagaatcacttttatcaggccgcgttgttactgctggaagcctcgcagaaacacattttgcgttacgccgaactggcggaaacgatggcggcaaactgcacagatgcccagcgtcgcgaagagctgctgactattgcagagatctcccgccataacgcgcaacataagccgcagacgttctggcaggcgtgccagttattctggtacatgaacatcattctgcaatacgaatccaacgccagttcgctatcgttggggcgcttcgaccagtatatgttgccgttctatcagacatcattaacccagggcgaagatgcggcgttcctgaaagaactgctcgaatctttatgggtgaaatgcaacgacatcgtgctgttgcgctccaccagtagcgcgcgttatttcgccggtttcccgaccggctataccgcactgctcggcgggttaaccgagaacggacgtagcgcggtgaacgtgctttcgttcctttgccttgacgcctatcaaagcgtgcaattaccgcaaccgaacctcggcgtgcgcactaacgccttgatcgacacgccgttcctgatgaaaaccgccgaaaccattcgcttcggtaccggtattccgcaaatctttaacgatgaagtggtggtgccagcgttcctcaaccgtggcgtttcgctggaagatgcgcgcgactattccgtagtgggctgtgtggaattatctattcccggcagaacctacggcttgcatgacatcgcgatgtttaatctgctgaaagtgatggaaatctgcctgcatgaaaatgaaggcaatgctgcgctgacttatgaaggtttactggagcagatccgcgccaagatcagccactacatcaccctgatggttgagggcagcaatatttgtgatatcggccatcgcgactgggcacctgtaccgctgctctcatcgtttatcagcgattgtctggaaaaaggccgcgatattaccgatggcggcgcgcgttataacttctccggcgtacaggggatcggtatcgccaacctgagcgattctctccatgcgttgaaagggatggtttttgagcaacagcgtttaagttttgacgaattgctgtcggtattaaaagccaacttcgcaacgccagaaggcgaaaaagtccgcgctcgcttaattaaccgcttcgagaaatacggtaacgatatcgacgaggtggataacatcagcgccgaactgttgcgccactactgcaaagaagtggaaaaataccagaacccgcgcggcggctacttcacgccgggatcgtataccgtttctgctcacgtcccgttgggatcggtggttggcgcgacgccagacggtcgttttgccggagaacagctggcagacggcggcttgtcacccatgctgggccaggacgcacaagggccaacagcggtactgaagtcagtcagtaagctcgataacacgctgctgtctaacggtacgttgctgaacgtgaaattcactccggcgaccctggaaggtgaagcaggattacgcaaactggccgacttcttacgggcgtttacccagcttaagttacaacatattcagtttaacgtggtgaacgccgacacgttgcgggaagcgcaacagcgcccacaagattatgccgggctggtggtgcgcgttgccggatacagcgccttctttgtcgaactgtcgaaggagatccaggatgacatcatccgccggacagcgcatcagctgtaacgttgtggaaacgcgccgcgatgatgtggcgcgcattttcaacattcagcgttattcactgaatgacggcgagggcattcgtacggtggtcttttttaaaggctgtccgcatctttgcccgtggtgtgctaatccggagtcgatctccggcaaaatccagacggtacgcagagaggcgaaatgtctgcactgtgcgaaatgtttgcgtgatgcggatgaatgcccctccggggcgtttgaacggattggtcgcgatatcagccttgacgctctggaacgggaagtgatgaaagatgacattttctttcgcacgtccggcggcggcgtcacgctttctggcggcgaagtgttaatgcaggcggagtttgctacccgttttttacagcgactgcggctgtggggtgtgtcatgcgccattgaaactgccggagacgcaccagccagcaagctattaccgctggcgaaattgtgcgatgaagtgttgttcgatttaaaaattatggacgcgactcaggcgcgggatgtggtgaagatgaacctgccacgcgtgctggagaatctgcgtttgctggtgagtgagggcgtcaacgtgatcccgcgtttaccgctgatccctggtttcacgctcagccgggagaatatgcagcaggcgctggatgtactgatcccgctgaatatcaggcagatccatctgttaccgtttcatcagtacggcgaaccgaaataccgcctgctggggaaaacatggtcgatgaaagaggtgcctgcgccgtcgtcagctgatgtggcaacgatgcgcgaaatggcagaacgggccggacttcaggttaccgtgggaggttaaaatggcatacctggtggcagtaaccgcctgcgtaagcggcgtggcgcatacttatatggcggcggaacggctggaaaagttgtgcctgttagagaagtggggagtcagcattgaaactcagggcgcgctgggaacggagaatcgtttagcggatgaggatatccgccgggcggatgttgctctgttgattacggatatcgagcttgccggtgccgagcgatttgaacattgccgctatgtgcaatgcagcatctacgcattcctgcgtgagccgcagcgggtaatgagcgcggtgcgcaaagtgctttctgcgccgcagcaaacccatcttattctggagtagtcggtttttctgtcagttggctgtggtactgccggcgatattccgacggcgagcgttcggtgtttttacgaaacagacggcagaagtagttgctgtcgacaaagccgcaggcgtgcgccacttcttttaccttcaggtcatagcctttcaataacgtcttagcgtgctccagtcgcgtgtgattcaggtattcgttaaaaccaatggcccccgttttttgaaacaggtgcgagaggtaatttggcgaaatataaaacgcctgtgcaacagattcgcgggtaagcgcggaggcatagcgttcgtcgatataatcgcgaatagcttcaaatagtgcctggctgcgtgaggcggtctggatttggctgccaagcaaatcgcggcagtggctaagcaggctggcgacgataagccttgccgtttgctgctcctgcggctgcatttgcatttcattgagcgtttgtagcagaaaagaacctatgcgtgggccgcgtcgggcgacgtgttgcttcgccagattttgatattgtttgccatcccattgcacgacgctgaagccgagttgctgtttgccaaacagcacgctaaaggtagtagcgggggcttgccattgtggaaaattccagccaccagcaggaacgtacagcacatcgccgggaactaacgttgctccagcgccggtatcaacaaactcaccttccagcacaatttccagccgtggaaaatcgacctgatacgcaagatcgggcaccgggccgttactgctggcaaagtaaatctggcgcagggacagcgggccgttgatcaggcgggagagcagatagctgacgtcgtgatacatgttattcccttaggtatgtagacgggaaaacagtaactggcattattaaaaaaggccacctgaaaagtgtggcctgaggggagttcgatgtaaacattgcggcagttgtattgccggatgtggcgtaaacgccttatccagcctaccgccgcgatctgtaggccggataagacgcgtcaagcgtcgcatccggcaaatagcgcctggctgataattactgattacccacctgatcgccatagggcagtgtgtcgtaatcgatcagtgcgtttttcttatacgggttaccaatccagcgggtagtttctttgaactgcggattcaccactgaacgggttggatcgtaaccgtcgtaagataagcccgccaaatctgaccaggtgtggatcagttccgccaggctgtatttacgatcaacatcctgcgagaaatcacggggatgagtcgcttgccatttttctgacgtccacagcaggaacggaatggtgtacatatgacgcgtcgggttgtcctcattacgcccctgagttttgtgcggcggcgtgtcgtaaacctcttcaccgtggtcagagaaataaaccaggaaaccgttcgggtttgctgctttaaagtctttaatcaggctggcaaccacatgatcgttatacaggttagcgttgtcataatcgttatatgactccagctcttccgcgtttaatcccggcggaacatgatcggtattgccatcaaacttgccctgattttccgggtagcggtatttgtatttgatatgcgtacccagcagatgaacaatgatcagtttcttcggcgcagggtcattcagcacttcctggaacggcttcagcacgttggtgtcgtattcacgcgcactctgcgtacgttgctggttcatgtagtactgcttgtcggtctggcgcgaaaataccgtcagcatggtattgcgggcggtcatcgtctgctggttggtgatccagaaggttttataacccgcctgtttcatcatgttcatcagcgacggctgcgtcagatacagatccgggttcttttcattggcaaaggtcagcgcctgttgcaggatttcaatggtgtacggacgagacgtaactacgttattaaacacggtcagattcggatcggttttatgcagcgcatccagctccggcgtggtttcacgcggataaccgtacagactcatgcgtccgcgctgggtcgactcgccaatcaccagcactaaagtgcgcggttcgttacccgattcatctttgaaattagccagtggcggcaaggcattattttcattcagtaactttgttagcgagtttagttgctgacgatactgataatagccggtcaggaattgccacggtgcggcaggctccatacgcgaggccaggttatccaacgttttctcaaacggcttgtttttgataaacgtattcatggcgatcggatgcagaatcaagccataaagcagggcaaaagagacaacataacgccacggctttggaatatagaccgggcgcaggcgtgtccacagcagaactgccaccgccgtataggccagcgcgataagcacaattttcaggctgaaatactggcttaaatactcgctggcttcgttggtgttggtttcgaacatcacaaacagaacgctctgcgagaactcctgaccgtagatgacgtagtagcacagcgccgccagagaggccgcccatagcaccacgccgattactgcggcaataattttaatccgcttcggaaagaggaataccgggatcaaccacagcgaactgaataacagcgagtcgcgaatgccgttagtgccactataaccactgatgtaaataatggcctgtagcagagtagagaaaaaccaaaagtagagcagtgcccaacccagggctttccagctaaaaagaggtttagcctggacttctgtggaatgcatagtaagaacctgtcttgaaaaaatatcgccgaatgtaacgacaattccttaaggatatctgaaggtatattcagaatttgaataaaatgcagacagaaatatattgaaaacgagggtgttagaacagaagtatttcagaaaaccctcgcgcaaaagcacgagggtttgcagaagaggaagattagccggtattacgcatacctgccgcaatcccggcaatagtgaccattaacgcttgttcgacgcgaggatccggttcctggccttctttttctgcctggcgggagcggtgcagcaactcggcctgcaatacgttcagcgggtcggtgtaaatattccgtagctgaatagactctgcaatccacggcagatcggccatcagatgggaatcgttggcaatcgccagcaccactttgatgtcttcttcttgcaggttgcgtaactctttacctaacggccacagtgctttgtctaccaggcgttggtcatagtattccgccagccacaggtctgctttggcgaagaccatctccagcatgccgagacgcgtcgagaagaatggccaatcgcggcacatagcctccagctcgctctgtttgccgtcttcgaccactttttgcagcgccgtacctgcacccagccaggcggggagcatcagacggttttgcgtccaggcgaagatccacggaatggcgcgtagtgactcgacgccgccggttgggcgacgtttcgccggacgtgaacccaacggcagtttgcccagttcttgttccggcgtagcggagcggaagtaaggcacaaaatctttgttttcacgtacgtagccgcggtagacatcgcaggagatgactgacagttcatccataatgcgacgccagctctctttcggctccggcggtggcagcaggttggcttccagaatcgccccggtataaagcgacaggctgctgacggtgatttctggcagaccatatttaaagcggatcatctcgccctgttcggttacgcgcaggccgcctttcaggcttcctggcggttgtgacagcagcgccgcatgagcaggtgcgccgccgcgaccaatggaaccgccgcgaccgtggaacaacgtcagctcaatacccgctttttcgcaggttttgattaatgcatcctgtgcctgatattgcgcccaggaagctgccatcactcccgcatcttttgctgagtcggaatagccaatcatcaccatctgtttgccctgaatcaggccacgataccagtcaatattgagcagctgggtcatgacatcgttggcgttgttcagatcatcgagggtttcaaacagcggagcaaccggcatcgcaaacccgatacccgcttctttcagcagcaggtggacagccagtacgtcggacggcgttttcgccatcgagatcacgtaggcggcaatggagccttgcggtgcttcggcaatcacctggcaggtatcgagcacttcgcgcgtttcggcgcttggttgccagttgcgcggcagaagcggacgtttggagttcagttcgcggatcaggaacgcctgtttgtcggcctctgaccagctttcgtagtcgccgataccgaggtagcgggtcagctcgcccagcgcttcggtatgacgcgtgctctcctgacggatatcaatacggaccagcggtacgccgaaacatttcacgcggcgcagggtgtcgagcagatcgccgttggcgataatacccatgccacacgcctgaagtgactggtagcaagcgtagagcggttcccacagttcttcgttttgtgtcagcaggccttctggttttggcagttcttcgcctttcaggcgcgcttccagccatgcctgtgtcgccatcaggcgagaacgcaggtttttcatcagatagcgatacggttctgcggcaccttcttcgccaaccagcgccagcagttcaggggtcgcttcaaccatcgacagttcagaaaccagcacctgaatatctttcaggaacaaatcggtggctttccagcggctgagtagcaggacgtggcgggtgatatcggcagtgacgttcgggttgccgtcgcggtcgccgcccatccacgaagtaaaacggaccggaacaaattcgacgggcagtttgtagccgaggttctcttccagttgttcgttcagttcgcgcaggtaatttggtacgccttgccacaggctgttttccactacggcaaagccccatttggcttcatctaccgggcttggacgcagcttacggatttcatcggtatgccatgactgggcgatcaactggcgcaggcgacgcatcagctggttgtgttcgtagtcagcgatatctttgttatcgagctgttttaaacaggcgttcacttccaccattttgtggatcagtgtacgacgggtaatttcggttgggtgagccgtgaggaccagttccagcgacagcgattccactgcttttttgatggtgtcttcgctcagttccggctggtttttcagtttacgcagggtgcgggcgatcacttccgggttgctggcagcttcgcctttcggcgaaatgctgtggtattgctcggcggtgttggccaggttcaggaactgactaaacgcacgcgcaacgggcagcagctcgtcgttcgacaaattttgtaaggtggtgagcaactcctggcggttagcatcattgccagcgcgtgaagatttcgacaacttacggatagtttctacgcgttcaagaatgtgttctcccaacgcatccttgatggtttctcccagcactttgccgagcatactgacattactacgcaatgcggaatattgttcgttcatattaccccagacaccccatcttatcgtttgatagccctgtatccttcacgtcgcattggcgcgaatatgctcgggctttgcttttcgtcgtcttttataaagccacgtaaaagcggtgacgtcaaatgctgcgaaatcgcttcagcaaacgaataaatagcaggaatttacgtcattaaattcacgacgctttaaataagcgtaacttatggaaatgttaaaaaatcgccccaagtaacaccaaaggtgtaggtcggataagatgcgcaagtatcgcatccgacattattgcggcactggagtttggcaacagtgccggatgcggcgcgagcgccttatccggcctacagttgggcatcgtttgagtcactgtcggtcggataagatgcgcaagtatcgcatccgacattattgcggcactggagtttggcaacagtgccggatgcggcgcgagcgccttatccggcctacggttgggcatcgtttgagtcactgtaggtcggataagatgcgcaagcatcgcatccgacattattgcggcactggagtttggcaacagcgccggatgcggcgcgagcgccttatccggcctacgttttaatgccagcaaaaatggtgaattacctgggttatcagttcgcgggtgggcttgataaaccgtgtttccagatattcatcaggttgatgagcctgattaattgagccaggccccaacaccagcgtcgggcataacgtttgaataaacggcgcttcggtacagtagttcaccacttcggtttttgctccgagcaatttctcaaccacttcaaccagttgatgattcggtgggcattcatagccagggatcggcggatgcagctcgtcgaccgtcagacgacccggccagcgttcgctcaccggagccaatgcatcgttgagcaaaccattaagttcattgagtgtcatgccaggcagcggacgaatatccatatgcaactcacagcaagcgcaaatacggttagaagcgtcgccaccgtgaatatgcccgaggttgagcgtagggtatggcacggtaaacgcttcgtagtgataacgttctttcaggttatcgcgcaattgcaaaatatgcccgatggcgtcgtgcattagttcgatagcgttaactccgcgtgctggatcgctggagtgccccgactggccctgaatacggatggcgttagagatatgacctttatgtgcgcgtaccggttgtagtgacgtcggttcgccaatgatggcgcaatccgggcgcagggcggtagtttcggcaaaataacgcgctccggccatactggtttcttcatcagcagtcgccagaatgtagagcggttttttcagtttcgtgacgtcgacatcgcgtagcgcatcaaggataaacgcaaaaaagcctttcatgtcggcggtgcctaagccgtaaagcttgccgtcatgctccgtcagtgtaaacggatcgcgcgtccagcgaccgtcatcaaatggcaccgtatcggtatgccccgccagcaacaagccgccagccccctgtccgatacttgccagcatattgaatttgttgcgagttcctggaacaggctgcacttccacattgaagcccaaatctttaaaccagtccgccagcagagtgattaaatctgcattgctttgatcgagtgcctcttccgtggcgcttattgaaggtgtggcaatcagagcgcggtaaatctcgataaatggcggtaatttgtttttcattgttgacacacctctggtcatgatagtatcaatattcatgcagtatttatgaataaaaatacactaacgttgagcgtaataaaacccaccagccgtaaggtgaatgttttacgtttaacctggcaaccagacataagaaggtgaatagccccgatgttgaatacgctgattgtgggtgccagcggctacgctggcgcagagctagtgacctatgtaaatcgccatccgcatatgaacataaccgctttgactgtttcagcgcaaagcaatgatgcgggaaagttaatctccgatttgcatccgcagctaaaaggcatcgttgatctgccgttgcagccgatgtcggatatcagcgagtttagcccaggggtggacgtagtgtttctcgccaccgcccatgaagttagccacgatttagcgccgcagtttcttgaagcgggctgcgtggtgttcgacctttccggcgcgtttcgtgttaacgacgccaccttctatgaaaaatattacggctttacccatcaatacccggaactgttggaacaggcagcctacggtctggcggagtggtgcggtaataaattaaaagaagcgaatttgattgcggtgccgggctgttatccgacggcggcacagctggcgctgaaaccgttgattgatgccgatcttcttgacctcaatcagtggccggtgatcaacgccaccagcggcgtgagcggtgcagggcgtaaagcggccatttcaaacagcttttgtgaagttagcctgcaaccgtatggcgtctttactcatcgccatcaaccagagatcgccacacacctcggtgctgacgttatcttcaccccacatctgggcaatttcccgcgcggcattctcgaaaccattacctgccgcctgaaatcgggtgtgacccaggcgcaagtcgcgcaagtgttacagcaggcgtatgcccataaaccgctggtgcggctgtatgacaaaggcgttccggcgctgaaaaatgtcgttgggctgccattttgcgatatcgggtttgccgttcagggcgagcatctgattattgtggcgaccgaagacaacttactgaaaggcgcggcggcacaagcggtacagtgcgccaatattcgtttcggctatgcggaaacgcagtctcttatttaagggtgcaatgatgaatccattaattatcaaactgggcggcgtactgctggatagtgaagaggcgctggaacgtctgtttagcgcactggtgaattatcgtgagtcacatcagcgtccgctggtgattgtgcacggcggcggttgcgtggtggatgagctgatgaaagggctgaatctgccggtgaaaaagaaaaacggcctgcgggtgacgcctgctgatcagatagacattatcaccggagcactggcgggaacggcaaataaaaccctgttggcatgggcgaagaaacatcagattgcggccgtaggtttgtttctcggtgacggcgacagcgtcaaagtgacccagcttgatgaagagttaggtcatgttggactggcgcagccaggttcgcctaagcttatcaactccttgctggagaacggttatctgccggtggtcagctccattggcgtaacagacgaagggcaactgatgaacgtcaatgccgaccaggcggcaacggcgctggcggcaacgctgggcgcggatctgattttgctctccgacgtcagcggcattctcgacggcaaagggcaacgcattgccgaaatgaccgccgcgaaagcagaacaactgattgagcagggcattattactgacggcatgatagtgaaagtgaacgcggcgctggatgcggcccgcacgctgggccgtccggtagatatcgcctcctggcgtcatgcggagcagcttccggcactgtttaacggtatgccgatgggtacgcggattttagcttaagttttgttggccggaggcgcagctttccggcattgaatttcaaaataaggaaacagagttatggcactttggggcgggcgttttacccaggcagcagatcaacggttcaaacaattcaacgactcactgcgctttgattaccgtctggcggagcaggatattgttggctctgtggcctggtccaaagccctggtcacggtaggcgtgttaaccgcagaagagcaggcgcaactggaagaggcgctgaacgtgttgctggaagatgttcgcgccaggccacaacaaatccttgaaagcgacgccgaagatatccatagctgggtggaaggcaaactgatcgacaaagtgggccagttaggcaaaaagctgcataccgggcgtagccgtaatgatcaggtagcgactgacctgaaactgtggtgcaaagataccgttagcgagttactgacggctaaccggcagctgcaatcggcgctggtggaaaccgcacaaaacaatcaggacgcggtaatgccaggttacactcacctgcaacgcgcccagccggtgacgttcgcgcactggtgcctggcctatgttgagatgctggcgcgtgatgaaagccgtttgcaggatgcgcttaagcgtctggatgtcagcccgctaggctgtggcgcgctggcgggaacggcctatgaaatcgaccgtgaacagttagcaggctggctgggctttgcttcggcgacccgtaacagtctcgacagcgtttctgaccgtgaccatgtgttggaactgctttctgctgccgctatcggcatggtgcatctgtcgcgttttgctgaagatctgattttctttaacaccggcgaagcggggtttgtggagctttctgaccgcgtgacttccggttcatcattaatgccgcagaagaaaaacccggatgcgctggagctgattcgcggtaaatgcggccgggtgcagggggcgttaaccggcatgatgatgacgctgaaaggtttgccgctggcttacaacaaagatatgcaggaagacaaagaaggtctgttcgacgcgctcgatacctggctggactgcctgcatatggcggcgctggtgctggacggcattcaggtgaaacgtccacgttgccaggaagcggctcagcagggttacgccaacgccaccgaactggcggattatctggtggcgaaaggcgtaccgttccgcgaggcgcaccatattgttggtgaagcggtggtggaagccattcgtcagggcaaaccgctggaagatctgccgctcagtgagttgcagaaattcagtcaggtgattgacgaagatgtctatccgattctgtcgctgcaatcgtgcctcgacaagcgtgcggcaaaaggcggcgtctcaccgcagcaggtggcgcaggcgattgcttttgcgcaggctcggttagggtaagaacatttatatgtataaatttgagcctggcttatcgccgggcttttttatggcaaaaaaaagcggatcctggagatccgcaaaagttcacgttggctttagttattcgagttgagaaactctcgaaacgggcagtgacttcaagggttaaaagaggtgccgctccgtttctgtgagcaattatcagtcagaatgcttgatagggataatcgttcattgctattctacctatcgccatgaactatcgtggcgatggaggatggataatgaatattcgtgatcttgagtacctggtggcattggctgaacaccgccattttcggcgtgcggcagattcctgccacgttagccagccgacgcttagcgggcaaattcgtaagctggaagatgagctgggcgtgatgttgctggagcggaccagccgtaaagtgttgttcacccaggcgggaatgctgctggtggatcaggcgcgtaccgtgctgcgtgaggtgaaagtccttaaagagatggcaagccagcagggcgagacgatgtccggaccgctgcacattggtttgattcccacagttggaccgtacctgctaccgcatattatccctatgctgcaccagacctttccaaagctggaaatgtatctgcatgaagcacagacccaccagttactggcgcaactggacagcggcaaactcgattgcgtgatcctcgcgctggtgaaagagagcgaagcattcattgaagtgccgttgtttgatgagccaatgttgctggctatctatgaagatcacccgtgggcgaaccgcgaatgcgtaccgatggccgatctggcaggggaaaaactgctgatgctggaagatggtcactgtttgcgcgatcaggcaatgggtttctgttttgaagccggggcggatgaagatacacacttccgcgcgaccagcctggaaactctgcgcaacatggtggcggcaggtagcgggatcactttactgccagcgctggctgtgccgccggagcgcaaacgcgatggggttgtttatctgccgtgcattaagccggaaccacgccgcactattggcctggtttatcgtcctggctcaccgctgcgcagccgctatgagcagctggcagaggccatccgcgcaagaatggatggccatttcgataaagttttaaaacaggcggtttaaaccgtttaacgcagctacccgataggcttccgccatcgtcgggtagttaaaggtggtgttgacgaagtactcaatagtgttgccgccacctttctgttccataatcgcctgaccgatatgaataatttcggcagcgcgctcgccaaagcagtgaatacccagaatctcttttgtttcccgatggaacaaaattttcagcgtgcccacgttcatgccgacgatttgtgcgcgtgccagatgtttaaactgggcgcggcccacttcatatggcactttcattgcggtcagctgctgttcggttttgcccacagagctgatttccgggatggtgtaaataccggtagggatatcttcaatcagatgtgcggtggcttcgccttttaccagcgcctgcgcggcaatgcgcccctggtcataggccgccgacgccaggctcggataaccaatcacgtcgcccaccgcgtaaacgtgtggctgtgcggtctgatacatgctgttgaccttcagctgtccgcggctgtcagtttctagcccaatgttctgtaacgccagcgaatcggtattaccggtgcgaccgttggcatagagcaggcagtcagctttcagttttttacccgacttcagatgcatgatcacaccatcgtcacagccttcgatcttctcgtactcttcgttgtgacgaatcactacgccactgttccagaagtgataggagagagaatctgacatctcttgatcgagaaatgccagcaggcgatcgcgggtgttgatcagatccacttttacatccataccgcggaagatcgacgcatattcacagccgatcactccagcaccatagataagtacatggcgcggttcgtggtgcatgctgagaattgagtcgctgtcgtaaatgcgtggatgggtgaaatcaacatctgttggatgatatggacgagagccgcaggcaataacaaatttttcagcggttagtgtttcaacgctgccgtccgggcaatccagcgccaacgtatgctcgtcaacaaagcgagcgtttccctgcaatatttcacagtgattacgttcgtaaaatccctgacgcatgcgcgtttgttgattaatcacgttatcggcatggttaaggatatcggcaaaagaagagcggagcagtcgggaatggtcgctgtaaagtgggttttgattgaattctataatgcggctgacggcgtgacggagagctttcgacgggatggtgccccagtgggtgcaaccgccgccaacattttgataacgctcgataactgcgacgcgcgcaccttgcttaaccaggcccattgcagcgccttcgccgccggggccggaacctattactatggcatcgtaatcgtaggaatgtggcatggtagggcttacctgttcttatacataaaagcaacagaatggtaacattttatcgcgggtaagccaattgatccccgtcatttatctggctatatcctgagcggcctttgctttgtctgtttcttacttttgccctgacgttttattggatttttatcgacgatactctccgtttaagcggcaggtttccgctgtacgtaaaagaaccggccaaagaattgcagtaaatatgttttattgcgttaccgttcattcacaatactggagcaatccagtatgttcattctctggtatagtgccagcagtacttttggcaaggattcagacatcgtgatgggcgtaagagcgcaacaaaaagaaaaaacccgccgttcgctggtggaagccgcatttagccaattaagtgctgaacgcagcttcgccagcctgagtttgcgtgaagtggcgcgtgaagcgggcattgctcccacctctttttatcggcatttccgcgacgtagacgaactgggtctgaccatggttgatgagagcggtttaatgctacgccaactcatgcgccaggcgcgtcagcgtatcgccaaaggcgggagtgtgatccgcacctcggtctccacatttatggagttcatcggtaataatcctaacgccttccggttattattgcgggaacgctccggcacctccgctgcgtttcgtgccgccgttgcgcgtgaaattcagcacttcattgcggaacttgcggactatctggaactcgaaaaccatatgccgcgtgcgtttactgaagcgcaagccgaagcaatggtgacaattgtcttcagtgcgggtgccgaggcgttggacgtcggcgtcgaacaacgtcggcaattagaagagcgactggtactgcaactgcgaatgatttcgaaaggggcttattactggtatcgccgtgaacaagagaaaaccgcaattattccgggaaatgtgaaggacgagtaatgaaacaagcaaatcaagatagaggtacgctgctgctggcgttagttgctggcttatcgattaatggtactttcgcagcgctgtttagctccattgtgccattttctgtattcccgattatttccctggtgctgacggtttactgcctgcatcaacgttatcttaatcgcactatgccggtaggcttgccgggtctggcagctgcctgttttattctcggcgtactgctgtacagcacggtagttcgtgcggaatatccggatatcggctctaacttcttcccggcagtactctccgtcattatggtgttctggattggcgcgaagatgcgtaaccgtaagcaggaagttgctgagtaatcggtattatgccggatgctggcgcatccggcatgggttttacttcgcggtcagtaatacgccgcactccatatggtgcgtgtaggggaactgatcaaacagagccagacgttcgaccttgtgcgtctggcttaatgtttccagattcttgcataacgtttccgggttacaggagatgtacaaaatacgcggatacgcctgcaccattttctcggtttcactgtccagaccgctgcgcggagggtcgacaaaaatggtttcgcactgataactctttaagtcgatcccttgcaggcggttaaactcgcgcacaccattcatcgcctgagtaaattcttctgccgccatacgaataatttgtacgttatcaatatggttagctgcgatgttgtattgcgcagcagcaaccgacggcttagcgatttcggtggctaatacccgatcaaaattacgcgccagcgctaatgaaaagttaccgttgccgcagtacagctccagtaaatcgccttttgagcctttggttacgtccagcgcccattccagcatctgaatattcatcgccgcgttcggctgggtaaagctgttttctacctgacggtagatcatctctttccctgcgaccggcagacgttcatcgatgtaatcctgatccagctcgattttggttttcgttgcccgaccaatcagatgcacattcagattctgcgcgcgcagtgcatcgcgcagggcctccgcttcctgacgccactcatcatccagcttcttatggtatagcagggaaaccaccgcctgattactcagtgtagtgaggtaatcaatctggaacaacttgtggcgcagaacgggattattacgcacacccgcaatcatcgccgtcatcaactggttgataagttcactggcggcggggaagctatccacgcggatgcggcttttggtttgttgatcgaaaatgatgtgatacaggtcatcgccatcgtgccagatgcggaactccgcgcgcatccggtaatgactgaccggcgagcgaaacacttccggaaccaggtcagaaaacggtgccatcatactttgcaaacgtaccactttttcggctaactgcgcttcatactgttctgttggaaggtgttcgggggtcatgatgtatcctgaaaaattaaagtacgcggcgattgtagggattgctcatcagatgtccagatcttgatgaattcctatttgtgagctacgtctggacagtaacttgttacaacctgtagcatccacttgccggtcctgtgagttaatagggaatccagtgcgaatctggagctgacgcgcagcggtaaggaaaggtgcgatgattgcgttatgcggacactgccattcggtgggaagtcatcatctcttagtatcttagatacccctccaagcccgaagacctgccggccaacgtcgcatctggttctcatcatcgcgtaatattgatgaaacctgcggcatccttcttctattgtggatgctttacaatgattaaaaaagcttcgctgctgacggcgtgttccgtcacggcattttccgcttgggcacaggataccagcccggatactctcgtcgttactgctaaccgttttgaacagccgcgcagcactgtgcttgcaccaaccaccgttgtgacccgtcaggatatcgaccgctggcagtcgacctcggtcaatgatgtgctgcgccgtcttccgggcgtcgatatcacccaaaacggcggttcaggtcagctctcatctatttttattcgcggtacaaatgccagtcatgtgttggtgttaattgatggcgtacgcctgaatctggcgggggtgagtggttctgccgaccttagccagttccctattgcgcttgtccagcgtgttgaatatatccgtgggccgcgctccgctgtttatggttccgatgcaataggcggggtggtgaatatcatcacgacgcgcgatgaacccggaacggaaatttcagcagggtggggaagcaatagttatcagaactatgatgtctctacgcagcaacaactgggggataagacacgggtaacgctgttgggcgattatgcccatactcatggttatgatgttgttgcctatggtaataccggaacgcaagcgcagacagataacgatggttttttaagtaaaacgctttatggcgcgctggagcataactttactgatgcctggagcggctttgtgcgcggctatggctatgataaccgtaccaattatgacgcgtattattctcccggttcaccgttgctcgatacccgtaaactctatagccaaagttgggacgccgggctgcgctataacggcgaactgattaaatcacaactcattaccagctatagccatagcaaagattacaactacgatccccattatggtcgttatgattcgtcggcgacgctcgatgagatgaagcaatacaccgtccagtgggcaaacaatgtcatcgttggtcacggtagtattggtgcgggtgtcgactggcagaaacagactacgacgccgggtacaggttatgttgaggatggatatgatcaacgtaataccggcatctatctgaccgggctgcaacaagtcggcgattttacctttgaaggcgcagcacgcagtgacgataactcacagtttggtcgtcatggaacctggcaaaccagcgccggttgggaattcatcgaaggttatcgcttcattgcttcctacgggacatcttataaggcaccaaatctggggcaactgtatggcttctacggaaatccgaatctggacccggagaaaagcaaacagtgggaaggcgcgtttgaaggcttaaccgctggggtgaactggcgtatttccggatatcgtaacgatgtcagtgacttgatcgattatgatgatcacaccctgaaatattacaacgaagggaaagcgcggattaagggcgtcgaggcgaccgccaattttgataccggaccactgacgcatactgtgagttatgattatgtcgatgcgcgcaatgcgattaccgacacgccgttgttacgccgtgctaaacagcaggtgaaataccagctcgactggcagttgtatgacttcgactggggtattacttatcagtatttaggcactcgctatgataaggattactcatcttatccttatcaaaccgttaaaatgggcggtgtgagcttgtgggatcttgcggttgcgtatccggtcacctctcacctgacagttcgtggtaaaatagccaacctgttcgacaaagattatgagacagtctatggctaccaaactgcaggacgggaatacaccttgtctggcagctacaccttctgaaccacgtcccaccgtgctggtgtttgactccggcgtcggtgggttgtcggtctatgacgagatccggcatctcttaccggatctccattacatttatgctttcgataacgtcgctttcccgtatggcgaaaaaagcgaagcgtttattgttgagcgagtggtggcaattgtcaccgcggtgcaagaacgttatccccttgcgctggctgtggtcgcttgcaacactgccagtaccgtttcacttcctgcattacgcgaaaagttcgacttcccggttgttggtgtcgtgccggcgattaaacctgctgcacgtctgacggcaaatggcattgtcggattactggcaacccgcggaacagttaaacgttcttatactcatgagctgatcgcgcgtttcgctaatgaatgccagatagaaatgctgggctcggcagagatggttgagttggctgaagcgaagctacatggcgaagatgtttctctggatgcactaaaacgtatcctacgcccgtggttaagaatgaaagagccgccagataccgttgtattgggttgcacccatttccctctactacaagaagaactgttacaagtgctgccagagggaacccggctggtggattctggcgcagcgattgctcgccgaacggcctggttgttagaacatgaagccccggatgcaaaatctgccgatgcgaatattgccttttgtatggcaatgacgccaggagctgaacaattattgcccgttttacagcgttacggcttcgaaacgctcgaaaaactggcagttttaggctgatttggttgaatgttgcgcggtcagaaaattattttaaatttcctcttgtcaggccggaataactccctataatgcgccaccactgacacggaacaacggcaaacacgccgccgggtcagcggggttctcctgagaactccggcagagaaagcaaaaataaatgcttgactctgtagcgggaaggcgtattatgcacaccccgcgccgctgagaaaaagcgaagcggcactgctctttaacaatttatcagacaatctgtgtgggcactcgaagatacggattcttaacgtcgcaagacgaaaaatgaataccaagtctcaagagtgaacacgtaattcattacgaagtttaattctttgagcgtcaaacttttaaattgaagagtttgatcatggctcagattgaacgctggcggcaggcctaacacatgcaagtcgaacggtaacaggaagaagcttgcttctttgctgacgagtggcggacgggtgagtaatgtctgggaaactgcctgatggagggggataactactggaaacggtagctaataccgcataacgtcgcaagaccaaagagggggaccttcgggcctcttgccatcggatgtgcccagatgggattagctagtaggtggggtaacggctcacctaggcgacgatccctagctggtctgagaggatgaccagccacactggaactgagacacggtccagactcctacgggaggcagcagtggggaatattgcacaatgggcgcaagcctgatgcagccatgccgcgtgtatgaagaaggccttcgggttgtaaagtactttcagcggggaggaagggagtaaagttaatacctttgctcattgacgttacccgcagaagaagcaccggctaactccgtgccagcagccgcggtaatacggagggtgcaagcgttaatcggaattactgggcgtaaagcgcacgcaggcggtttgttaagtcagatgtgaaatccccgggctcaacctgggaactgcatctgatactggcaagcttgagtctcgtagaggggggtagaattccaggtgtagcggtgaaatgcgtagagatctggaggaataccggtggcgaaggcggccccctggacgaagactgacgctcaggtgcgaaagcgtggggagcaaacaggattagataccctggtagtccacgccgtaaacgatgtcgacttggaggttgtgcccttgaggcgtggcttccggagctaacgcgttaagtcgaccgcctggggagtacggccgcaaggttaaaactcaaatgaattgacgggggcccgcacaagcggtggagcatgtggtttaattcgatgcaacgcgaagaaccttacctggtcttgacatccacggaagttttcagagatgagaatgtgccttcgggaaccgtgagacaggtgctgcatggctgtcgtcagctcgtgttgtgaaatgttgggttaagtcccgcaacgagcgcaacccttatcctttgttgccagcggtccggccgggaactcaaaggagactgccagtgataaactggaggaaggtggggatgacgtcaagtcatcatggcccttacgaccagggctacacacgtgctacaatggcgcatacaaagagaagcgacctcgcgagagcaagcggacctcataaagtgcgtcgtagtccggattggagtctgcaactcgactccatgaagtcggaatcgctagtaatcgtggatcagaatgccacggtgaatacgttcccgggccttgtacacaccgcccgtcacaccatgggagtgggttgcaaaagaagtaggtagcttaaccttcgggagggcgcttaccactttgtgattcatgactggggtgaagtcgtaacaaggtaaccgtaggggaacctgcggttggatcacctccttaccttaaagaagcgtactttgtagtgctcacacagattgtctgatagaaagtgaaaagcaaggcgtttacgcgttgggagtgaggctgaagagaataaggccgttcgctttctattaatgaaagctcaccctacacgaaaatatcacgcaacgcgtgataagcaattttcgtgtccccttcgtctagaggcccaggacaccgccctttcacggcggtaacaggggttcgaatcccctaggggacgccacttgctggtttgtgagtgaaagtcgccgaccttaatatctcaaaactcatcttcgggtgatgtttgagatatttgctctttaaaaatctggatcaagctgaaaattgaaacactgaacaacgagagttgttcgtgagtctctcaaattttcgcaacacgatgatgaatcgaaagaaacatcttcgggttgtgaggttaagcgactaagcgtacacggtggatgccctggcagtcagaggcgatgaaggacgtgctaatctgcgataagcgtcggtaaggtgatatgaaccgttataaccggcgatttccgaatggggaaacccagtgtgtttcgacacactatcattaactgaatccataggttaatgaggcgaaccgggggaactgaaacatctaagtaccccgaggaaaagaaatcaaccgagattcccccagtagcggcgagcgaacggggagcagcccagagcctgaatcagtgtgtgtgttagtggaagcgtctggaaaggcgcgcgatacagggtgacagccccgtacacaaaaatgcacatgctgtgagctcgatgagtagggcgggacacgtggtatcctgtctgaatatggggggaccatcctccaaggctaaatactcctgactgaccgatagtgaaccagtaccgtgagggaaaggcgaaaagaaccccggcgaggggagtgaaaaagaacctgaaaccgtgtacgtacaagcagtgggagcacgcttaggcgtgtgactgcgtaccttttgtataatgggtcagcgacttatattctgtagcaaggttaaccgaataggggagccgaagggaaaccgagtcttaactgggcgttaagttgcagggtatagacccgaaacccggtgatctagccatgggcaggttgaaggttgggtaacactaactggaggaccgaaccgactaatgttgaaaaattagcggatgacttgtggctgggggtgaaaggccaatcaaaccgggagatagctggttctccccgaaagctatttaggtagcgcctcgtgaattcatctccgggggtagagcactgtttcggcaagggggtcatcccgacttaccaacccgatgcaaactgcgaataccggagaatgttatcacgggagacacacggcgggtgctaacgtccgtcgtgaagagggaaacaacccagaccgccagctaaggtcccaaagtcatggttaagtgggaaacgatgtgggaaggcccagacagccaggatgttggcttagaagcagccatcatttaaagaaagcgtaatagctcactggtcgagtcggcctgcgcggaagatgtaacggggctaaaccatgcaccgaagctgcggcagcgacgcttatgcgttgttgggtaggggagcgttctgtaagcctgcgaaggtgtgctgtgaggcatgctggaggtatcagaagtgcgaatgctgacataagtaacgataaagcgggtgaaaagcccgctcgccggaagaccaagggttcctgtccaacgttaatcggggcagggtgagtcgacccctaaggcgaggccgaaaggcgtagtcgatgggaaacaggttaatattcctgtacttggtgttactgcgaaggggggacggagaaggctatgttggccgggcgacggttgtcccggtttaagcgtgtaggctggttttccaggcaaatccggaaaatcaaggctgaggcgtgatgacgaggcactacggtgctgaagcaacaaatgccctgcttccaggaaaagcctctaagcatcaggtaacatcaaatcgtaccccaaaccgacacaggtggtcaggtagagaataccaaggcgcttgagagaactcgggtgaaggaactaggcaaaatggtgccgtaacttcgggagaaggcacgctgatatgtaggtgaggtccctcgcggatggagctgaaatcagtcgaagataccagctggctgcaactgtttattaaaaacacagcactgtgcaaacacgaaagtggacgtatacggtgtgacgcctgcccggtgccggaaggttaattgatggggttagcgcaagcgaagctcttgatcgaagccccggtaaacggcggccgtaactataacggtcctaaggtagcgaaattccttgtcgggtaagttccgacctgcacgaatggcgtaatgatggccaggctgtctccacccgagactcagtgaaattgaactcgctgtgaagatgcagtgtacccgcggcaagacggaaagaccccgtgaacctttactatagcttgacactgaacattgagccttgatgtgtaggataggtgggaggctttgaagtgtggacgccagtctgcatggagccgaccttgaaataccaccctttaatgtttgatgttctaacgttgacccgtaatccgggttgcggacagtgtctggtgggtagtttgactggggcggtctcctcctaaagagtaacggaggagcacgaaggttggctaatcctggtcggacatcaggaggttagtgcaatggcataagccagcttgactgcgagcgtgacggcgcgagcaggtgcgaaagcaggtcatagtgatccggtggttctgaatggaagggccatcgctcaacggataaaaggtactccggggataacaggctgataccgcccaagagttcatatcgacggcggtgtttggcacctcgatgtcggctcatcacatcctggggctgaagtaggtcccaagggtatggctgttcgccatttaaagtggtacgcgagctgggtttagaacgtcgtgagacagttcggtccctatctgccgtgggcgctggagaactgaggggggctgctcctagtacgagaggaccggagtggacgcatcactggtgttcgggttgtcatgccaatggcactgcccggtagctaaatgcggaagagataagtgctgaaagcatctaagcacgaaacttgccccgagatgagttctccctgaccctttaagggtcctgaaggaacgttgaagacgacgacgttgataggccgggtgtgtaagcgcagcgatgcgttgagctaaccggtactaatgaaccgtgaggcttaaccttacaacgccgaagctgttttggcggatgagagaagattttcagcctgatacagattaaatcagaacgcagaagcggtctgataaaacagaatttgcctggcggcagtagcgcggtggtcccacctgaccccatgccgaactcagaagtgaaacgccgtagcgccgatggtagtgtggggtctccccatgcgagagtagggaactgccaggcatcaaataaaacgaaaggctcagtcgaaagactgggcctttcgttttatctgttgtttgtcggtgaacgctctcctgagtaggacaaatccgccgggagcggatttgaacgttgcgaagcaacggcccggagggtggcgggcaggacgcccgccataaactgccaggcatcaaattaagcagaaggccatcctgacggatggcctttttgcgtttctacaaactcttcctgtcgtcatatctacaagccatccccccacagatacggtaaactagcctcgtttttgcatcaggaaagcagctatgaaccactccttaaaaccctggaacacatttggcattgatcataatgctcagcacattgtatgtgccgaagacgaacaacaattactcaatgcctggcagtatgcaaccgcagaaggacaacccgttcttattctgggtgaaggaagtaatgtactttttctggaggactatcgcggcacggtgatcatcaaccggatcaaaggtatcgaaattcatgatgaacctgatgcgtggtatttacatgtaggagccggagaaaactggcatcgtctggtaaaatacactttgcaggaaggtatgcctggtctggaaaatctggcattaattcctggttgtgtcggctcatcacctatccagaatattggtgcttatggcgtagaattacagcgagtttgcgcttatgttgattctgttgaactggcgacaggcaagcaagtgcgcttaactgccaaagagtgccgttttggctatcgcgacagtatttttaaacatgaataccaggaccgcttcgctattgtagccgtaggtctgcgtctgccaaaagagtggcaacctgtactaacgtatggtgacttaactcgtctggatcctacaacagtaacgccacagcaagtatttaatgcggtgtgtcatatgcgcaccaccaaactccctgatccaaaagtgaatggcaatgccggtagtttcttcaaaaaccctgttgtatctgccgaaacggctaaagcattactgtcacaatttccaacagcaccaaattacccccaggcggatggttcagtaaaactggcagcaggttggcttatcgatcagtgccagctaaaagggatgcaaataggtggggctgcggtgcaccgtcaacaggcgttagttctcattaatgaagacaatgcaaaaagcgaagatgttgtacagctggcgcatcatgtaagacagaaagttggtgaaaaatttaatgtctggcttgagcctgaagtccgctttattggtgcatcaggtgaagtgagcgcagtggagacaatttcatgaaggataacaccgtgccactgaaattgattgccctgttagcgaacggtgaatttcactctggcgagcagttgggtgaaacgctgggaatgagccgggcggctattaataaacacattcagacactgcgtgactggggcgttgatgtctttaccgttccgggtaaaggatacagcctgcctgagcctatccagttacttaatgctaaacagatattgggtcagctggatggcggtagtgtagccgtgctgccagtgattgactccacgaatcagtaccttcttgatcgtatcggagagcttaaatcgggcgatgcttgcattgcagaataccagcaggctggccgtggtcgccggggtcggaaatggttttcgccttttggcgcaaacttatatttgtcgatgttctggcgtctggaacaaggcccggcggcggcgattggtttaagtctggttatcggtatcgtgatggcggaagtattacgcaagctgggtgcagataaagttcgtgttaaatggcctaatgacctctatctgcaggatcgcaagctggcaggcattctggtggagctgactggcaaaactggcgatgcggcgcaaatagtcattggagccgggatcaacatggcaatgcgccgtgttgaagagagtgtcgttaatcaggggtggatcacgctgcaggaagcggggatcaatctcgatcgtaatacgttggcggccatgctaatacgtgaattacgtgctgcgttggaactcttcgaacaagaaggattggcaccttatctgtcgcgctgggaaaagctggataattttattaatcgcccagtgaaacttatcattggtgataaagaaatatttggcatttcacgcggaatagacaaacagggggctttattacttgagcaggatggaataataaaaccctggatgggcggtgaaatatccctgcgtagtgcagaaaaataagaaaggggagtattcgctcccctgcaaattatttgcgtagtctgacctcttctaccgcatgattagcacttttcgtcaggattaaactggcgcgctcacgagtaggtagaatattttgctttaagttcagccagttgatctctttccacaatgtcatggcagtcttaatcgcttcttctttagttaatttcgcgtagttatgaaaataggaatccgggtcggtaaaagccccttcgcggaatttcagaaaacggttgatataccatgtctgaagtaagtcttccggtgcatcaacatatatcgaaaaatcgacaaaatcagaaacaaatacatgatgtggatcgtgtggataatccatcccgctctgtaagacatttaacccttcaagaattaaaatatcaggctgaacaaccgttttatctccatccgggatcacatcataaataagatgtgagtaaacaggtgctgtaacgtttggcacgccggatttgagatcggaaacaaacttcaccaggcgatgcatatcatacgattccgggaagcctttcttcttcatcagaccacgttctttcagaacctgattagggtgaaggaagccatctgtagtgatcagttcaacacgacgatgttccggccaacggcttaatagcgcctgcaatacacgggcggttgtacttttccccaccgcgacactgccagcaatactgataatgtaaggaatgcgttgcccgttggtaccaagaaactgttccagaactgcctgacggcgcagattcgagcttatatagaagttcagcaaacgtgacaaaggtaaatagatctcggcaacttcttctaacgagagatcttcattaatacctttgagacgggcgatctcatcttccgataacgtcataggtacggaatcacgcagagctgcccactggttgcggtcaaactgtaggtaaggcgtcattaacgtttgctcttttatactcataagcatgtttctggcggtcatagctctatcggcaaagcgatatttgccatggcgcgtcacagttctgttgaatgggttaatgggcaggagggtaacaccagatggggaggaataataagaaaaaatctctgccaggaagctatcgttgaaaagcaatgtgacagatattccatctgataaaaagaattatggtttagcaggagcgcattgttgagcacaatgatgttgaaaaagtgtgctaatctgccctccgttcggctgtttcttcatcgtgtcgcataaaatgtgaccaataaaacaaattatgcaattttttagttgcatgaactcgcatgtctccatagaatgcgcgctacttgatgccgacttagctcagtaggtagagcaactgacttgtaatcagtaggtcaccagttcgattccggtagtcggcaccatcaagtccggtggggttcccgagcggccaaagggagcagactgtaaatctgccgtcacagacttcgaaggttcgaatccttcccccaccaccaatttcggccacgcgatggcgtagcccgagacgataagttcgcttaccggctcgaataaagagagcttctctcgatattcagtgcagaatgaaaatcaggtagccgagttccaggatgcgggcatcgtataatggctattacctcagccttccaagctgatgatgcgggttcgattcccgctgcccgctccaagatgtgctgatatagctcagttggtagagcgcacccttggtaagggtgaggtcggcagttcgaatctgcctatcagcaccacttcttttctcctccctgttttttccttctgtttattgcattcaacaagtcgggcatgttgcctggttgatgtggtgatatcaccgatttatccgtgtcttagagggacaatcgatgtctaaagaaaagtttgaacgtacaaaaccgcacgttaacgtcggtactatcggccacgttgaccatggtaaaacaacgctgaccgctgcaatcactaccgtactggctaaaacctacggcggtgctgctcgcgcattcgaccagatcgataacgcgccggaagaaaaagctcgtggtatcaccatcaacacttctcacgttgaatacgacaccccgacccgtcactacgcacacgtagactgcccggggcacgccgactatgttaaaaacatgatcaccggtgctgcgcagatggacggcgcgatcctggtagttgctgcgactgacggcccgatgccgcagactcgtgagcacatcctgctgggtcgtcaggtaggcgttccgtacatcatcgtgttcctgaacaaatgcgacatggttgatgacgaagagctgctggaactggttgaaatggaagttcgtgaacttctgtctcagtacgacttcccgggcgacgacactccgatcgttcgtggttctgctctgaaagcgctggaaggcgacgcagagtgggaagcgaaaatcctggaactggctggcttcctggattcttacattccggaaccagagcgtgcgattgacaagccgttcctgctgccgatcgaagacgtattctccatctccggtcgtggtaccgttgttaccggtcgtgtagaacgcggtatcatcaaagttggtgaagaagttgaaatcgttggtatcaaagagactcagaagtctacctgtactggcgttgaaatgttccgcaaactgctggacgaaggccgtgctggtgagaacgtaggtgttctgctgcgtggtatcaaacgtgaagaaatcgaacgtggtcaggtactggctaagccgggcaccatcaagccgcacaccaagttcgaatctgaagtgtacattctgtccaaagatgaaggcggccgtcatactccgttcttcaaaggctaccgtccgcagttctacttccgtactactgacgtgactggtaccatcgaactgccggaaggcgtagagatggtaatgccgggcgacaacatcaaaatggttgttaccctgatccacccgatcgcgatggacgacggtctgcgtttcgcaatccgtgaaggcggccgtaccgttggcgcgggcgttgtagcaaaagttctgagctaattgccgataacatttgacgcaatgcgcactaaaagggcatcatttgatgccctttttgcacgctttcgtaccagaacctggctcatcagtgattttctttgtcataatcattgctgagacaggctctgttgagggcgtataatccgaaaagctaatacgcgtttcgatttggtttgcctcgcgatcgcggggtgaaaatgtttgtagaaaacttctgacaggttggtttatgagtgcgaataccgaagctcaaggaagcgggcgcggcctggaagcgatgaagtgggtcgttgtggtggcattgctcctggtggcgattgtcggcaactatctttatcgcgacattatgctgccgctgcgtgcgctggccgtagtaattctgattgctgcagcgggtggtgtcgcgctgttaacgacaaaaggtaaagctaccgttgcttttgcccgtgaagcgcgtaccgaagtccgtaaggtcatttggccgactcgccaggaaacattgcacaccacgctgattgtggctgcggttaccgcagtaatgtcactgatcctgtggggactggatggtattctggttcgcctggtatcctttatcactggcctgaggttctgagatgtctgaagctcctaaaaagcgctggtacgtcgttcaggcgttttccggttttgaaggccgcgtagcaacgtcgctgcgtgagcatatcaaattacacaacatggaagatttgtttggtgaagtcatggtaccaaccgaagaagtggttgaaatccgtggcggtcagcgtcgcaaaagcgaacgtaaattcttccctggctacgtcctcgttcagatggtgatgaacgacgcgagctggcacctggtgcgcagcgtaccgcgtgtgatgggcttcatcggcggtacttccgatcgtcctgcgccaatcagcgataaagaagtcgatgcgattatgaaccgcctgcagcaggttggtgataagccgcgtccgaaaacgctgtttgaaccgggtgaaatggtccgtgttaatgatggtccgttcgctgacttcaacggtgttgttgaagaagtggattacgagaaatctcgtctgaaagtgtctgtttctatcttcggtcgtgcgaccccggtagagctggacttcagccaggttgaaaaagcctaacccagcgatcaaaaaagcggcgatttaatcgttgcacaaggcgtgagattggaatacaatttcgcgccttttgtttttatgggccttgcccgtaaaacgattttttatatcacggggagcctctcagaggcgttattacccaacttgaggaatttataatggctaagaaagtacaagcctatgtcaagctgcaggttgcagctggtatggctaacccgagtccgccagtaggtccggctctgggtcagcagggcgtaaacatcatggaattctgcaaagcgttcaacgcaaaaactgattccatcgaaaaaggtctgccgattccggtagtaatcaccgtttacgctgaccgttctttcactttcgttaccaagaccccgccggcagcagttctgctgaaaaaagcggctggtatcaagtctggttccggtaagccgaacaaagacaaagtgggtaaaatttcccgcgctcagctgcaggaaatcgcgcagaccaaagctgccgacatgactggtgccgacattgaagcgatgactcgctccatcgaaggtactgcacgttccatgggcctggtagtggaggactaagaaatggctaaactgaccaagcgcatgcgtgttatccgcgagaaagttgatgcaaccaaacagtacgacatcaacgaagctatcgcactgctgaaagagctggcgactgctaaattcgtagaaagcgtggacgtagctgttaacctcggcatcgacgctcgtaaatctgaccagaacgtacgtggtgcaactgtactgccgcacggtactggccgttccgttcgcgtagccgtatttacccaaggtgcaaacgctgaagctgctaaagctgcaggcgcagaactggtaggtatggaagatctggctgaccagatcaagaaaggcgaaatgaactttgacgttgttattgcttctccggatgcaatgcgcgttgttggccagctgggccaggttctgggtccgcgcggcctgatgccaaacccgaaagtgggtactgtaacaccgaacgttgctgaagcggttaaaaacgctaaagctggccaggttcgttaccgtaacgacaaaaacggcatcatccacaccaccatcggtaaagtggactttgacgctgacaaactgaaagaaaacctggaagctctgctggttgcgctgaaaaaagcaaaaccgactcaggcgaaaggcgtgtacatcaagaaagttagcatctccaccaccatgggtgcaggtgttgcagttgaccaggctggcctgagcgcttctgtaaactaatgcctttacgtgggcggtgattttgtctacaatcttacccccacgtataatgcttaatgcagacgtatatccgagatattcgggttgtggcaaggcggcaactgagtgagtcgccaggagcatagctaactatgtgactggtgcgaatgaaggaagccaacgccgtcacaagctgaatagcgacggatagaaaagatttgttcgttggagcctggcctatccaggcctccgtcgaagaccgcaggagtttcgcaagaaacttaatcccctgcgtagacggtgacagaacgctaagattattcttttatattctggcttgtttctgctcaccgtaattaagacgctctctccgtttggaggagtgaagtgagttccagagattttctctggcaaacatccaggagcaaagctaatggctttaaatcttcaagacaaacaagcgattgttgctgaagtcagcgaagtagccaaaggcgcgctgtctgcagtagttgcggattcccgtggcgtaactgtagataaaatgactgaactgcgtaaagcaggtcgcgaagctggcgtatacatgcgtgttgttcgtaacaccctgctgcgccgtgctgttgaaggtactccgttcgagtgcctgaaagacgcgtttgttggtccgaccctgattgcatactctatggaacacccgggcgctgctgctcgtctgttcaaagagttcgcgaaagcgaatgcaaaatttgaggtcaaagccgctgcctttgaaggtgagctgatcccggcgtctcagatcgaccgcctggcaactctgccgacctacgaagaagcaattgcacgcctgatggcaaccatgaaagaagcttcggctggcaaactggttcgtactctggctgctgtacgcgatgcgaaagaagctgcttaatcgcagttatctttttaacgcattcgcttacgtataaacttattctgatattcaggaacaatttaaatgtctatcactaaagatcaaatcattgaagcagttgcagctatgtctgtaatggacgttgtagaactgatctctgcaatggaagaaaaattcggtgtttccgctgctgctgctgtagctgtagctgctggcccggttgaagctgctgaagaaaaaactgaattcgacgtaattctgaaagctgctggcgctaacaaagttgctgttatcaaagcagtacgtggcgcaactggcctgggtctgaaagaagctaaagacctggtagaatctgcaccggctgctctgaaagaaggcgtgagcaaagacgacgcagaagcactgaaaaaagctctggaagaagctggcgctgaagttgaagttaaataagccaacccttccggttgcagcctgagaaatcaggctgatggctggtgactttttagtcaccagcctttttgcgctgtaaggcgccagtagcgtttcacactgtttgactactgctgtgcctttcaatgcttgtttctatcgacgacttaatatactgcgacaggacgtccgttctgtgtaaatcgcaatgaaatggtttaagcgtgatagcaacaggcattgcggaaagtgttccattttccggtcaacaaaatagtgttgcacaaactgtccgctcaatggacagatgggtcgacttgtcagcgagctgaggaaccctatggtttactcctataccgagaaaaaacgtattcgtaaggattttggtaaacgtccacaagttctggatgtaccttatctcctttctatccagcttgactcgtttcagaaatttatcgagcaagatcctgaagggcagtatggtctggaagctgctttccgttccgtattcccgattcagagctacagcggtaattccgagctgcaatacgtcagctaccgccttggcgaaccggtgtttgacgtccaggaatgtcaaatccgtggcgtgacctattccgcaccgctgcgcgttaaactgcgtctggtgatctatgagcgcgaagcgccggaaggcaccgtaaaagacattaaagaacaagaagtctacatgggcgaaattccgctcatgacagacaacggtacctttgttatcaacggtactgagcgtgttatcgtttcccagctgcaccgtagtccgggcgtcttctttgactccgacaaaggtaaaacccactcttcgggtaaagtgctgtataacgcgcgtatcatcccttaccgtggttcctggctggacttcgaattcgatccgaaggacaacctgttcgtacgtatcgaccgtcgccgtaaactgcctgcgaccatcattctgcgcgccctgaactacaccacagagcagatcctcgacctgttctttgaaaaagttatctttgaaatccgtgataacaagctgcagatggaactggtgccggaacgcctgcgtggtgaaaccgcatcttttgacatcgaagctaacggtaaagtgtacgtagaaaaaggccgccgtatcactgcgcgccacattcgccagctggaaaaagacgacgtcaaactgatcgaagtcccggttgagtacatcgcaggtaaagtggttgctaaagactatattgatgagtctaccggcgagctgatctgcgcagcgaacatggagctgagcctggatctgctggctaagctgagccagtctggtcacaagcgtatcgaaacgctgttcaccaacgatctggatcacggcccatatatctctgaaaccttacgtgtcgacccaactaacgaccgtctgagcgcactggtagaaatctaccgcatgatgcgccctggcgagccgccgactcgtgaagcagctgaaagcctgttcgagaacctgttcttctccgaagaccgttatgacttgtctgcggttggtcgtatgaagttcaaccgttctctgctgcgcgaagaaatcgaaggttccggtatcctgagcaaagacgacatcattgatgttatgaaaaagctcatcgatatccgtaacggtaaaggcgaagtcgatgatatcgaccacctcggcaaccgtcgtatccgttccgttggcgaaatggcggaaaaccagttccgcgttggcctggtacgtgtagagcgtgcggtgaaagagcgtctgtctctgggcgatctggataccctgatgccacaggatatgatcaacgccaagccgatttccgcagcagtgaaagagttcttcggttccagccagctgtctcagtttatggaccagaacaacccgctgtctgagattacgcacaaacgtcgtatctccgcactcggcccaggcggtctgacccgtgaacgtgcaggcttcgaagttcgagacgtacacccgactcactacggtcgcgtatgtccaatcgaaacccctgaaggtccgaacatcggtctgatcaactctctgtccgtgtacgcacagactaacgaatacggcttccttgagactccgtatcgtaaagtgaccgacggtgttgtaactgacgaaattcactacctgtctgctatcgaagaaggcaactacgttatcgcccaggcgaactccaacttggatgaagaaggccacttcgtagaagacctggtaacttgccgtagcaaaggcgaatccagcttgttcagccgcgaccaggttgactacatggacgtatccacccagcaggtggtatccgtcggtgcgtccctgatcccgttcctggaacacgatgacgccaaccgtgcattgatgggtgcgaacatgcaacgtcaggccgttccgactctgcgcgctgataagccgctggttggtactggtatggaacgtgctgttgccgttgactccggtgtaactgcggtagctaaacgtggtggtgtcgttcagtacgtggatgcttcccgtatcgttatcaaagttaacgaagacgagatgtatccgggtgaagcaggtatcgacatctacaacctgaccaaatacacccgttctaaccagaacacctgtatcaaccagatgccgtgtgtgtctctgggtgaaccggttgaacgtggcgacgtgctggcagacggtccgtccaccgacctcggtgaactggcgcttggtcagaacatgcgcgtagcgttcatgccgtggaatggttacaacttcgaagactccatcctcgtatccgagcgtgttgttcaggaagaccgtttcaccaccatccacattcaggaactggcgtgtgtgtcccgtgacaccaagctgggtccggaagagatcaccgctgacatcccgaacgtgggtgaagctgcgctctccaaactggatgaatccggtatcgtttacattggtgcggaagtgaccggtggcgacattctggttggtaaggtaacgccgaaaggtgaaactcagctgaccccagaagaaaaactgctgcgtgcgatcttcggtgagaaagcctctgacgttaaagactcttctctgcgcgtaccaaacggtgtatccggtacggttatcgacgttcaggtctttactcgcgatggcgtagaaaaagacaaacgtgcgctggaaatcgaagaaatgcagctcaaacaggcgaagaaagacctgtctgaagaactgcagatcctcgaagcgggtctgttcagccgtatccgtgctgtgctggtagccggtggcgttgaagctgagaagctcgacaaactgccgcgcgatcgctggctggagctgggcctgacagacgaagagaaacaaaatcagctggaacagctggctgagcagtatgacgaactgaaacacgagttcgagaagaaactcgaagcgaaacgccgcaaaatcacccagggcgacgatctggcaccgggcgtgctgaagattgttaaggtatatctggcggttaaacgccgtatccagcctggtgacaagatggcaggtcgtcacggtaacaagggtgtaatttctaagatcaacccgatcgaagatatgccttacgatgaaaacggtacgccggtagacatcgtactgaacccgctgggcgtaccgtctcgtatgaacatcggtcagatcctcgaaacccacctgggtatggctgcgaaaggtatcggcgacaagatcaacgccatgctgaaacagcagcaagaagtcgcgaaactgcgcgaattcatccagcgtgcgtacgatctgggcgctgacgttcgtcagaaagttgacctgagtaccttcagcgatgaagaagttatgcgtctggctgaaaacctgcgcaaaggtatgccaatcgcaacgccggtgttcgacggtgcgaaagaagcagaaattaaagagctgctgaaacttggcgacctgccgacttccggtcagatccgcctgtacgatggtcgcactggtgaacagttcgagcgtccggtaaccgttggttacatgtacatgctgaaactgaaccacctggtcgacgacaagatgcacgcgcgttccaccggttcttacagcctggttactcagcagccgctgggtggtaaggcacagttcggtggtcagcgtttcggggagatggaagtgtgggcgctggaagcatacggcgcagcatacaccctgcaggaaatgctcaccgttaagtctgatgacgtgaacggtcgtaccaagatgtataaaaacatcgtggacggcaaccatcagatggagccgggcatgccagaatccttcaacgtattgttgaaagagattcgttcgctgggtatcaacatcgaactggaagacgagtaattctcgctcaaacaggtcactgctgtcgggttaaaacccggcagcggattgtgctaactccgacgggagcaaatccgtgaaagatttattaaagtttctgaaagcgcagactaaaaccgaagagtttgatgcgatcaaaattgctctggcttcgccagacatgatccgttcatggtctttcggtgaagttaaaaagccggaaaccatcaactaccgtacgttcaaaccagaacgtgacggccttttctgcgcccgtatctttgggccggtaaaagattacgagtgcctgtgcggtaagtacaagcgcctgaaacaccgtggcgtcatctgtgagaagtgcggcgttgaagtgacccagactaaagtacgccgtgagcgtatgggccacatcgaactggcttccccgactgcgcacatctggttcctgaaatcgctgccgtcccgtatcggtctgctgctcgatatgccgctgcgcgatatcgaacgcgtactgtactttgaatcctatgtggttatcgaaggcggtatgaccaacctggaacgtcagcagatcctgactgaagagcagtatctggacgcgctggaagagttcggtgacgaattcgacgcgaagatgggggcggaagcaatccaggctctgctgaagagcatggatctggagcaagagtgcgaacagctgcgtgaagagctgaacgaaaccaactccgaaaccaagcgtaaaaagctgaccaagcgtatcaaactgctggaagcgttcgttcagtctggtaacaaaccagagtggatgatcctgaccgttctgccggtactgccgccagatctgcgtccgctggttccgctggatggtggtcgtttcgcgacttctgacctgaacgatctgtatcgtcgcgtcattaaccgtaacaaccgtctgaaacgtctgctggatctggctgcgccggacatcatcgtacgtaacgaaaaacgtatgctgcaggaagcggtagacgccctgctggataacggtcgtcgcggtcgtgcgatcaccggttctaacaagcgtcctctgaaatctttggccgacatgatcaaaggtaaacagggtcgtttccgtcagaacctgctcggtaagcgtgttgactactccggtcgttctgtaatcaccgtaggtccatacctgcgtctgcatcagtgcggtctgccgaagaaaatggcactggagctgttcaaaccgttcatctacggcaagctggaactgcgtggtcttgctaccaccattaaagctgcgaagaaaatggttgagcgcgaagaagctgtcgtttgggatatcctggacgaagttatccgcgaacacccggtactgctgaaccgtgcaccgactctgcaccgtctgggtatccaggcatttgaaccggtactgatcgaaggtaaagctatccagctgcacccgctggtttgtgcggcatataacgccgacttcgatggtgaccagatggctgttcacgtaccgctgacgctggaagcccagctggaagcgcgtgcgctgatgatgtctaccaacaacatcctgtccccggcgaacggcgaaccaatcatcgttccgtctcaggacgttgtactgggtctgtactacatgacccgtgactgtgttaacgccaaaggcgaaggcatggtgctgactggcccgaaagaagcagaacgtctgtatcgctctggtctggcttctctgcatgcgcgcgttaaagtgcgtatcaccgagtatgaaaaagatgctaacggtgaattagtagcgaaaaccagcctgaaagacacgactgttggccgtgccattctgtggatgattgtaccgaaaggtctgccttactccatcgtcaaccaggcgctgggtaaaaaagcaatctccaaaatgctgaacacctgctaccgcattctcggtctgaaaccgaccgttatttttgcggaccagatcatgtacaccggcttcgcctatgcagcgcgttctggtgcatctgttggtatcgatgacatggtcatcccggagaagaaacacgaaatcatctccgaggcagaagcagaagttgctgaaattcaggagcagttccagtctggtctggtaactgcgggcgaacgctacaacaaagttatcgatatctgggctgcggcgaacgatcgtgtatccaaagcgatgatggataacctgcaaactgaaaccgtgattaaccgtgacggtcaggaagagaagcaggtttccttcaacagcatctacatgatggccgactccggtgcgcgtggttctgcggcacagattcgtcagcttgctggtatgcgtggtctgatggcgaagccggatggctccatcatcgaaacgccaatcaccgcgaacttccgtgaaggtctgaacgtactccagtacttcatctccacccacggtgctcgtaaaggtctggcggataccgcactgaaaactgcgaactccggttacctgactcgtcgtctggttgacgtggcgcaggacctggtggttaccgaagacgattgtggtacccatgaaggtatcatgatgactccggttatcgagggtggtgacgttaaagagccgctgcgcgatcgcgtactgggtcgtgtaactgctgaagacgttctgaagccgggtactgctgatatcctcgttccgcgcaacacgctgctgcacgaacagtggtgtgacctgctggaagagaactctgtcgacgcggttaaagtacgttctgttgtatcttgtgacaccgactttggtgtatgtgcgcactgctacggtcgtgacctggcgcgtggccacatcatcaacaagggtgaagcaatcggtgttatcgcggcacagtccatcggtgaaccgggtacacagctgaccatgcgtacgttccacatcggtggtgcggcatctcgtgcggctgctgaatccagcatccaagtgaaaaacaaaggtagcatcaagctcagcaacgtgaagtcggttgtgaactccagcggtaaactggttatcacttcccgtaatactgaactgaaactgatcgacgaattcggtcgtactaaagaaagctacaaagtaccttacggtgcggtactggcgaaaggcgatggcgaacaggttgctggcggcgaaaccgttgcaaactgggacccgcacaccatgccggttatcaccgaagtaagcggttttgtacgctttactgacatgatcgacggccagaccattacgcgtcagaccgacgaactgaccggtctgtcttcgctggtggttctggattccgcagaacgtaccgcaggtggtaaagatctgcgtccggcactgaaaatcgttgatgctcagggtaacgacgttctgatcccaggtaccgatatgccagcgcagtacttcctgccgggtaaagcgattgttcagctggaagatggcgtacagatcagctctggtgacaccctggcgcgtattccgcaggaatccggcggtaccaaggacatcaccggtggtctgccgcgcgttgcggacctgttcgaagcacgtcgtccgaaagagccggcaatcctggctgaaatcagcggtatcgtttccttcggtaaagaaaccaaaggtaaacgtcgtctggttatcaccccggtagacggtagcgatccgtacgaagagatgattccgaaatggcgtcagctcaacgtgttcgaaggtgaacgtgtagaacgtggtgacgtaatttccgacggtccggaagcgccgcacgacattctgcgtctgcgtggtgttcatgctgttactcgttacatcgttaacgaagtacaggacgtataccgtctgcagggcgttaagattaacgataaacacatcgaagttatcgttcgtcagatgctgcgtaaagctaccatcgttaacgcgggtagctccgacttcctggaaggcgaacaggttgaatactctcgcgtcaagatcgcaaaccgcgaactggaagcgaacggcaaagtgggtgcaacttactcccgcgatctgctgggtatcaccaaagcgtctctggcaaccgagtccttcatctccgcggcatcgttccaggagaccactcgcgtgctgaccgaagcagccgttgcgggcaaacgcgacgaactgcgcggcctgaaagagaacgttatcgtgggtcgtctgatcccggcaggtaccggttacgcgtaccaccaggatcgtatgcgtcgccgtgctgcgggtgaagctccggctgcaccgcaggtgactgcagaagacgcatctgccagcctggcagaactgctgaacgcaggtctgggcggttctgataacgagtaatcgttaatccgcaaataacgtaaaaacccgcttcggcgggtttttttatggggggagtttagggaaagagcatttgtcagaatatttaaggaatttctgaatactcataatcaatgtagagatgactaatatcctgaaactgactgaactaattgagtcaaactcggcaaggattcgatactattcctgtgtaactttcttaaggaacgagaatgaaacaggaagtggaaaagtggcgaccttttggacatccggatggtgatattcgtgatttatcatttcttgatgctcatcaggctgtctacgttcagcatcatgagggcaaagagcctttagagtatcgcttttgggttacctactctcttcactgcttcacaaaagattatgaacatcagacgaacgaagaaaaacaatcgttaatgtaccacgcgcctaaagaatctcgtcccttctgccagcaccgttataacttagcgcgcacacacttaaaaagaactattttggcgctgccagaaagcaacgttattcatgccgggtatggtagctatgccgtgattgaggtggacttagacggaggagataaggcattttactttgttgcgttcagggctttcagggaaaagaaaaaactccgtttgcatgtaactagcgcttatcccatttctgaaaaacagaaaggtaaatcagtgaaatttttcaccattgcctacaacttattgagaaataagcagcttcctcagccctcaaaataacaaaacccaccttaaggtgggtttcgccagagaattatctctggtattcagaacgccattaccggactttgccttgaccttgcgataatcgcaggttgcgggatgtctgaatttcttcagtctgctgcatcctggaagatgagaacatgtgttcttattttcgtctctatcatagttgagtatttactctcttacaatcagatctctttcattgctcaacaggcgatggcttcagactttgcattacggaatttttaagaaaggcagggcgaaacgaggaagaagcttttcgccctggacaacattcctgctgacggcactaccataaaaaaacacaacgctttcaacaaccttgcgtttttcatcttccgtagcggctcggaataaatttacgttcttacattccgtctcatagtctttgcgaggcgcgtcccagatagctgtcccagtctttccataccggctgcaaaccctgagcggttaacgcggcagcaaccgcttccggtctgcgatcgtcgtgcggtgagaactgttccaactcggggtgattatcggcatagccacctggctgcgttttcgagaaggcgctgacgttattgatcgccagcggaataacgcgatcgcgaaaccacggtgattcccgcgtggagagtgacagttcaatctccggtgcaagcagtcggaaggcgcagatggtttgcactaactggcgttcatccataatcgacgcaggctcaatgccgccagtacacgggcgcaggcgcggaaaggagacagagtaacggctttgccagtaatgctgttgcagccatagcaaatgttcggcaaccatatagctgtcaacgcgccagttgtcggaaaggccaattagcgcgccgaggcctatcttatcaatccccgcacgccccagccgatccggcgtttccagccgccagaagaagtcctgttttttgcctttcagatgatggcgggcataagtcgcctcgtgatatgtctcctgataaaccatcacgccatccagaccaagttgctttaactcggcgtattccgtctccgccagcggttgcacttccatctgtagtgaagagaactgttcacgaagggcagggagatgacgacgaaagtaatccatccccactttcgcctgatgttcaccagtgactaacagcagatgttcaaagcccatctcccgtatagcggcactttccctggcaatatccgcttcatccagcgttttgcgcttgatgcgattactcatggaaaatccacagtacgtgcagtcgttagcgcaaagattggaaagataaagcgggacgtagaaactaactgtgttgccaaatcgctgacgggtcagacgctgcgcccgttgggccagttgttccagatagccactggcggcaggcgataacagcgccatcatgtcgtcgcgggtgagttgcgaggcatttagcgcccgctctacgtcagcagccgttttgccgttgatacgcaggcggatgtcgtcccagtccagttgtcgccagcgatcgctgaaggttttcatgccgatgcctccagaaatccggtcagcgggctggtggcatgagcaaaataactgcggctgcccggtccggactgacgtgccagtaggcctgcttctaccgccagacgaaatgccttcgccatgttgacgggatcgtccgcgacggcaatcgccgtattcactaacaccgcgtcggcccccatttccagcgcctgcgcggcatggctgggaacgccgatgccagcatcgacaaccaccggcactgtggcctgctggataataatctccagcatggcgcgggtttccagtccctgattcgagccaatcggcgcgccgagcggcatcaccgctgcacagccgacttcttccagacgtttacacaataccggatcggccccgcagtaaggcagcacgacaaatccctgttgtaccagcgtttcggcggctttcagggtttcgatgggatcgggcaacagccagcgggcgtcagggtgaatctctaattttaaccagtttgtgcctaacgcttcacgagccagatgggcggcgaaaatggcttcttccgctgttttcgccccggatgtatttggcagcagggtcacacccgccgcgataagcggttcgaggatagcgtcgttgtgctggcgcaagtcgacacgtttcatcgccagtgtcaccagctggctgccggaagcgcggatcgcctccaccatcagttgtgaagaagcgaatttccctgtgccggtaaacagatgtgaatcaaacgttttgtccgcaatacgtaacatttcaaccccctgcaataacctgaaaaagcaggatctggtcgccatcctgcacgatatgttgcgcccactgctcacgcgggacgatttgctgattaatcgccagagccgcgcccgcttgtcgttggtcgagttgctccagtagttcgtgaacagtttgcccggcggcgcactgcatcgcttgatcgttaaacaggatctgcattgcttcctccgcataccgggcaaccactggcgcggcgcaacgccaggctgcgccactggctcgatttaccgtcgaacagtcggagttctcccgcaggtgtctctataccgcttaataacttaatggcttccagtgcctgcaaagtgcccataaccccgaccaccgggccaaccacgcccgccgtgcggcagttgcgttctggctcctggttatctggccacaggcagcggtaacacccctgctcccagggcggcgtcagtaccatcaactgaccgccaaatccgaccgcgctggcggtgataagcggcgtgttgagtgccacgcaggcggcattaatctcctggcgagtcgccatattgtcggtacagtcgagcaccacatcggcccgtgcaaccgcatcttttaacgcctcacccgttaaccgttgttgtaatgctgtcagttgaatgtcgggattcaactgtgtcagtcgctgttggctgacctgcgatttcgggcgatcgatatcttcagtggtaaagaggatttgtcgttgcagattgcttaaatgcacatcgtcgtcatctgccagtaccagcgtcccgacgccagcgcccgccaggtacagcgcagcaggtgtacccagcccgcccagaccgataatcagcacctggctgtcgagcagtttttgctgcccgtccagagcgatatcgtcgagcaggatttggcggctataacgcataaagtcacggtcattcatcgccaactcctgcaatttccagcaactgtgccgttgccaaacgccagtctgcggcttgagtaatggcgctgacgacggcgatactgccgacacccgttgctatcaccgcaggcgcgcgtgccagactgataccgccaatcgccacggtgggataatccgccagtcgctcaacatgccgtgccagctgttccagcccctgcggtgcagaaggcatctgtttggtttgcgtcgggaacacatgtcccagcgcgatataagaggggcgtgctgccagcgcgacgtcgatttccatatcgtcatgtgtcgaaacgcccagccgcaggcctgccgcgcggatggcattgagatcggtggcttgcaaatcttcctgccccaaatggacgccatacgcctgatgcttgatcgccagccgccagtaatcgttgataaacaatcgcgcgttatagcggcggcccagcgcaattgccgccacgacatcggcttccacctcttcatcgcgccgatctttgatgcgtagctggagagtacgtacgcctgcatccaacagacgttcgatccactgtacgctgtccaccaccgggtacagtcctgaacgaaaaggtacaggaggaaaatcaggctgatacatcacgcttcctccttacgcaggtagatttctccgcctctggcacggaagttctccgacatatccgccattcccatttcaatagtttgcgtggcggcgtaatcacgcacttcctggctgattttcatcgagcagaatttcggcccacacatggagcaaaaatgggcgactttacctgactcttgcggcagggtttcatcgtgataagcgcgggcggtaaacgggtcgagggccagattaaactggtcttcccagcgaaattcgaagcgggctttcgacatggcgttatcgcgaatttgcgcgcccggatgccctttcgccaggtcagcggcgtgggcagcaatcttataggtgataagcccctgcttaacatcttctttattgggcagacccagatgctcttttggcgttacgtaacagagcatcgcgcagccaaaccagccaatcatcgccgcaccaatccccgacgtgaagtggtcatagcccggcgcaatatcggtagttagcggccccagagtgtaaaacggcgcttcgtggcagtgctctaactcctcggtcatattgcggcggatcatctgcatcggcacgtggcctgggccttcaatcatcacctgcacgtcatattcccaggcaattttggtcagttcgcccagcgtatgcagctcggcaaactgcgcttcatcgttggcgtcctgaatagaaccggggcgcagaccgtcgcccagcgacagcgaaacgtcataagcggcacagatttcacaaatttcgcggaagtgttgatagaggaaattttcctgatgatgggagaggcaccatttcgccataatcgaaccgccgcgagagacgataccggtcaggcgtttcgcggtcatcggcacatagcgcagcagtacgcccgcatggatagtgaagtaatccacaccttgctcggcctgttccagcagcgtgtcgcggaacgcttcccaggtaagatcttcggcgatcccgttaaccttctccagcgcctggtagatcggcactgtaccgatcggcaccgggctgttacgcaaaatccactcgcgggtttcgtgaatatagcgaccggtggagagatccatcaccgtatccgctccccagcgcgtggaccataccagcttttccacttcttcttcgatggaagaggtgaccgccgagttgccgatattggcgttaacttttaccaggaaattgcgaccaataatcatcggctccgattccggatgattaatgttggccgggataatcgcacgtccggcagcaacttcatcacggacaaattccgcagtgatattttccggcagatgtgcgccaaagctcattcccggatgctggtggcgtaaaacctcgctacggatgcgctcgcggcccatattctcgcggatggcgatgaattccatttccggcgtgatgatgccctggcgggcgtagtgcagttgggtgacacggcgtcctgctttggcgcgttttggtgttagtacgccgctaaaacgcagttcgtcgaggccatcatctgccagccgcgctttagtgtaatcggaactgcgcacggtaagttcttcggtatcgccgcgcgcatcgatccacggctggcgtagttttgccagcccttgctgcacgttaatggcaatctgcggatcaccatacgggccggaggtgtcgtagaccggaatcgcttcgttttcttcgtactgcggctgttctttgctaccgccaattagcgtcgggctaagctggatctcacgcatcggcacgcgcacgccggggtgtgtgccagtgatataaatgcgttttgagttgggaaaggcggtgccttccagggtgtcgataaaatgttgggcccgggcgcgttgttcgcggcgggtcagttttgttgcagacatagctcattccaaaaagttaaggacgtggcttgtcagacgacggatgaagcaagagacgatcgccgcaggggcgatgcgatagcagattaactcttgttcccttcgcaggtattagcctgatcaggttccgcggatcccgaataaacggtctcagccagttaaggcactccgacaagaaattagccccgcaaatggggcattgaatgtaaattacgcgttaacagcgcagaactcaagcaggatgtttgacgcgggcggcgtcaagcaccagcagaatcagcttatcttccagcacaaagcgcgcttccagcgcctcgccgatgtcagataaaacctgttgaaactcaaggtaattatcatgatcgatggcggtttccagactggaatcgtagtaatccataatctgttgagtattggcttcgagttgcggccaaatcttcgcggcgcgcgcgagttgcccgttgccttccagcttatgaagaatgcgctcataaatactgaaatgtccggcagacaagtaatcgaccaggctctgacaaaaatcatcaagggctttttcgtttagcctcatgtacgattctttgccaggcttaatgccaaccagattgtagtaagccacgagcagatgcttacgtacatgtagccagcgatcaaccagtttgttacttcctctgacgcgctccgtcaggttatcgagctggttaagcatgattgactccgcaagtttgtattcaaaaactgctcagtgagaaatgtaaaaaccatgttaaacatgccagtgatgcaaaggtagtgcaagagctatggatcgtataattgaaaaattagatcacggctggtgggtcgtcagccatgaacaaaaattatggttgccgaagggagaattgccatatggcgaagcggcaaatttcgatcttgtgggtcagcgcgcactacaaatcggcgaatggcagggggaacctgtttggttagtacaacagcagcggcgtcacgatatggggtcggtacgtcaggtcattgatctcgatgttgggctgtttcaactggccggacgaggcgtacaactggcggagttttaccgatcgcataaatactgtggttactgcgggcatgaaatgtatccgagcaaaaccgaatgggcgatgctgtgcagccattgccgtgagcgttactacccgcaaatcgccccctgcattattgttgccatccgtcgcgatgattcgatcctcctcgcccagcatacccgccatcgtaacggtgtccatacagtacttgccggattcgtcgaagtgggcgaaaccctcgagcaggcagtcgcgcgggaagtgatggaagagagcggaattaaagttaaaaacttgcgttacgtgacttctcagccgtggccgtttcctcagtctttaatgaccgcgtttatggcggaatatgacagcggcgacatcgtgatcgacccgaaagaattgctcgaggcgaactggtatcgctatgacgatttgccgttactcccgccgcccggcaccgtagcgcgccgtctgatagaagatacggtggcgatgtgtcgggcagagtatgagtgatgatacactgaccgcctgacgcactaaggaacagccaaaatgaccgaacttaaaaacgatcgttatctgcgggcgctgctgcgccagcccgttgatgtcactccagtatggatgatgcgccaggcgggtcgctatctaccggaatataaagccacgcgcgcccaggcaggcgattttatgtcgctgtgcaaaaacgccgagctggcgtgcgaagtgactttgcaaccgctgcgtcgctacccgctggatgcggcgatcctcttttccgatatcctcaccgtgccggacgcgatggggttagggctctattttgaagccggagaaggtccgcgttttacctcgccagtcacctgcaaagctgacgtcgataaactgccaattccggacccggaagatgaactgggttacgtgatgaacgcggtgcgtaccattcgtcgcgaactgaaaggcgaagtgccgctgattggtttttccggcagcccgtggacgctggcgacctacatggtggaaggcggcagcagcaaagccttcaccgtgatcaaaaaaatgatgtatgccgatccgcaggcgctgcacgctctgctcgataaactggcgaaaagcgtcactttgtatctgaatgcgcagattaaagccggtgctcaggcagtgatgattttcgacacctggggcggcgtgcttaccgggcgcgattatcaacagttctcgctctattacatgcataaaattgttgatggtttactgcgtgaaaacgacggtcgccgcgtaccggtcacgctgtttaccaaaggcggcggacagtggctggaagccatggcagaaaccggttgcgatgcgctgggcctcgactggacaacggacatcgccgatgcgcgccgccgtgtgggcaataaagtcgcgttgcagggtaatatggatccgtcgatgctgtacgcgccgcctgcccgcattgaagaagaagtagcgactatacttgcaggtttcggtcacggcgaaggtcatgtctttaaccttggtcacggcattcatcaggatgtgccgccagaacatgctggcgtgttcgtggaggcagtgcatcgactgtctgaacagtatcaccgctaaggagtgattatggatctcgcgtcattacgcgctcaacaaatcgaactggcttcttctgtgatccgcgaggatcgactcgataaagatccaccggatctgatcgccggagccgatgtcgggtttgagcagggcggagaagtgacgcgagcggcgatggtgctgctgaaatatccctcgcttgagctggtcgagtataaagttgcccgcatcgccaccaccatgccttacattccaggttttctttccttccgcgaatatcctgcgctgctggcagcgtgggagatgctgtcgcaaaagccggatttagtgtttgtcgatggtcatgggatctcgcatcctcgccgtcttggcgtcgccagccattttggcttattggtggatgtgccgaccattggcgtggcgaaaaaacggctctgcggtaaattcgaaccgctctccagcgaaccgggcgcgctggccccactgatggataaaggcgagcagctggcctgggtctggcgcagcaaagcgcgctgtaacccgttgtttatcgctaccggccatcgggtcagcgtggacagcgcgctggcgtgggtacaacgctgcatgaaaggctatcgtctgccggagccaacgcgctgggcggacgcggtggcctcggaacgtccggcgttcgtgcgctatacagcaaatcagccctaattcaggtaaactgcggataatttccgtatttgagaactcaacatgttacaaaacccaattcatctgcgtctggagcgcctggaaagctggcagcatgtcactttcatggcttgcttatgcgaacgcatgtaccccaattacgccatgttctgccagcaaaccggttttggtgatgggcaaatttaccgtcgcattctcgatctcatctgggaaacgctgaccgttaaagacgcaaaagtaaatttcgacagccaactggagaaatttgaagaagcgattccttcagccgacgatttcgatctgtacggcgtttatccggcaatcgatgcctgcgtggcgttaagtgaactggtccattcgcgtttgagtggtgaaacgctcgaacacgcggtggaagtgagtaagacctccatcacgaccgttgcgatgctggaaatgactcaggctggtcgcgaaatgagcgatgaagagcttaaagaaaacccagctgtagagcaagaatgggacattcagtgggaaatattccgacttttagctgagtgcgaagaacgcgatatcgagctgataaaaggccttagggcagacctgcgtgaggcgggtgagagcaatattggtataatttttcagcaataagaccagaaaacgtgatttaacgcctgatttgtcgtacctggagtcttccctttcgccccccgtctggtctacatttggggggcgaaaaaaagtggctatcggtgcgtgtatgcaggagagtgctattctggcatttccgtcgcactcgatgcttagcaagcgataaacacattgtaaggataacttatgaacaagactcaactgattgatgtaattgcagagaaagcagaactgtccaaaacccaggctaaagctgctctggagtccactctggctgcaattactgagtctctgaaagaaggcgatgctgtacaactggttggtttcggtaccttcaaagtgaaccaccgcgctgagcgtactggccgcaacccgcagaccggtaaagaaatcaaaattgccgcagctaacgtaccggcatttgtttctggcaaggcactgaaagacgcagttaagtaagattgcgtggcagtgaacagttttaacgaaggggtggtttcaccccttttgtctttctggcgtcgatcattgatgctggctggcgctctgcttctcactgcctgtagtcataactcttcacttcctccctttaccgccagtggatttgctgaagaccagggcgcggtacgcatctggcgaaaagacagcggcgataatgtgcatctgcttgccgtgtttagcccgtggcgcagtggcgataccacgacgcgagagtatcgctggcagggcgataacctcacgctcatcaatatcaatgtttacagcaaaccgccggtgaatattcgcgcgcgttttgacgatcgcggtgatctgagctttatgcaacgtgaatccgatggggaaaagcagcagctttctaacgaccaaatcgatttataccgttatcgtgctgatcagatccgccagattagcgatgccttacgtcaggggagagtcgtgctgcgccaggggcgctggcatgcgatggaacagaccgtgaccacctgcgaagggcaaaccattaaacctgatttagattcgcaggcgatagcgcatatcgagcgccgccagagccgctcttctgttgatgtcagcgtggcatggctggaagcgcccgaaggttcgcaattactgttagtggcaaactctgatttctgtcgctggcaacccaacgagaaaacgttctgatttaccagtggcccatacccatatgaccgccaccaccgcagccgccgtagcccatgcccattccggctccgcgcggaatacccgcttcagccatcgcgatatctcgtttcacccgtaactcatctaacgactgacgcaaattctccatctctttggcgaccgcgttaattttgctgctatccggtgggttcgcggctaacagggcattgtattcataacgcttcgtcaccagttgctgttgcagtgcgctgctttgagcgtaaaagtcattatggattttctgccacgctgtctgttgttcgctggtcaaaggcgcggcattttgctgccacataccgtgtccgccgtgagcaaatgcagatgtcgatcccatcgccattgctgaaagcgccatcattaccagggcaattttcgtgttccgtttcatggttaatcctccagtggttgtcttacttcgggtattgcatcttccgtgccaacgatgaaacgctgatatgacgggtaatctggcatgataaacgagtaaaaatgactcgcctgctgcgggtagcgagtcatttttactcattgaaacttaagcctttgtgttacagcgcagggtaagcgctgataaaagatggcatgatttctgctgtcagaaagggatgagcaggcaaagaagaagatgcgttttatgcaacgttctaaagactccttagctaaatggttaagcgcgatcctccccgtggtcattgttgggctggtgggattgtttgcggtaactgtgattcgtgattatgggcgggcaagcgaggcagaccgccaggcattactggaaaaaggtaatgtgcttatccgcgctctggagtcgggaagccgcgtagggatggggatgcgaatgcaccatgtacagcaacaggcgcttctggaagagatggcgggacagccgggagtgttgtggttcgcagtcaccgatgcgcagggcatcattattcttcatagcgaccccgataaggtcgggcgtgcgctctattcgccggatgaaatgcagaaattaaagccagaggaaaactcccgctggcggctgcttgggaaaacggaaactacgcctgcacttgaggtctatcgtttgttccagccaatgtcagcgccctggcggcatggaatgcacaatatgccgcgctgtaacggcaaagctgtgccacaagtagatgcacaacaggctatttttatcgccgttgatgccagtgatctggttgcaacccagagtggggaaaagcgcaataccctgattatcctcttcgccctggcgacggtcttgctggcaagcgtattgtcattcttctggtatcgccgctatctgcgctcgcgccagcttctacaagatgaaatgaagcgcaaagagaagctggtggcgctggggcatcttgcggcaggcgttgcccacgaaatccgtaacccactttcctcgattaaaggactggcgaaatactttgccgagcgcgcgcctgcagggggagaagcgcatcaactggcgcaggtgatggcgaaagaggccgaccgtttaaaccgcgtggtaagcgagttgctggaactggttaagccaacgcatctggctttgcaggcggtggatctcaacacgctgattaaccactcattacagctggtaagtcaggatgcaaacagccgggagatccagttacgctttaccgccaacgacacattaccggaaattcaggccgacccggacaggctgactcaggtcctgttgaatctctatctcaatgctattcaggcgattggtcagcatggcgtgattagcgtgacggccagcgaaagcggcgcgggcgtgaaaatcagcgttaccgacagcggtaagggaattgcggcagatcagcttgatgccatcttcactccgtacttcaccactaaagccgaaggcaccggattggggctggcggtcgtgcataatattgttgaacaacacggtggtacaattcaggtcgcaagccaggagggaaaaggctcaacgttcaccctctggcttccggtcaatattacgcgtaaggacccacaaggatgacgcacgataatatcgatattctggtggtggatgatgacattagccactgcactattttgcaggctttactgcgcggctggggctataacgtcgcgctggcgaacagcgggcgacaggcgttggagcaggtgcgggaacaggtttttgatcttgtgctttgcgatgtgcgaatggcggagatggacggcatcgccacgctgaaagagatcaaagcgttaaacccggcaattccggtgctgattatgactgcgtactccagcgtcgagacggcggtagaggcactgaaaactggggcgctggattatctcatcaagccgctggatttcgataacctacaggcgacgctggaaaaagcgctcgcgcatacgcacagtattgatgctgaaacacctgcggtgactgccagccagttcggtatggtcggtaaaagcccggcgatgcaacacctgctcagtgaaatcgccctcgtcgcgccatcggaagccacggtactgatccacggcgattccggcaccggtaaagagctggtcgccagggcgattcacgccagtagcgcacgtagcgaaaaaccgctggtaacgctcaactgtgcggcactcaacgaatccttgctggaatctgaattgttcggtcacgaaaaaggggcgtttactggagccgataaacgccgggaagggcgctttgttgaggcggacggcggcacgctgtttctcgatgaaattggcgatatctcgccgatgatgcaggtgcgtctgctgcgtgcgattcaggagcgcgaagttcagcgtgtcggtagcaaccagattatctcggttgatgtccggctgattgcggcgacccatcgcgatcttgccgcagaggtgaatgccgggcgttttcgccaggatctctactatcgcctgaatgtggtggcgattgaagtaccatcgctgcggcaacggcgggaagatatccctctgctggctggccattttctgcagcgctttgccgagcgtaatcgcaaggcggtaaaaggttttacgccccaggcgatggatctgttgattcattacgactggccgggaaatattcgtgagctggaaaacgcggtggaacgggcagtggtgctgctgaccggggaatatatttccgaacgcgagctgccgctggcgattgccagtacgccgatcccgctgggacaaagtcaggatattcagccgttggtggaagtggaaaaagaggtgattctggcggcgctggagaaaacgggcggcaacaaaaccgaagccgcccgtcagttagggatcacgcgcaaaacgctattggcaaaactgtcgcgttagttctgctcgcgttcgatagcgcgccagccgatatctttccggcagaagcagtcgtcccagtggatatcggtcattaaggcataggcgcgtttctgcgcttctgccacggtatgacccagcgcggtgacgcacagtacgcgcccgccgttggtcactacctgctcgtcatccgccagttttgtgcccgcgtggaacactttgccgcctgccacttcttccagcggcaggccgtggatcacgtcaccggtgcggtaatcacccggatatccacccgcagccatcaccacgccgagagaagcgcgttcatcccactcggacgttttctcgtccagtttgctttcacaggccgccaggcagagctcaaccagatcggacttcatgcgcagcataatcggctgggtttccggatcgccaaagcggcagttaaattcaataaccttcggattgccctgtttgtcgatcatcaggcccgcgtagagaaaaccggtgtaggtgttgccttccgccgccatgcctttcacggttggccagataatacgttccatggtgcgctgatgaacgtcatcggttactaccggcgcgggggagtaagcgcccatcccgccggtgtttggtccggtatctttatcgcctacgcgtttgtgatcctggctggtagccatcggcagcacatgctcgccgtccaccatcacgataaagctcgcttcttcgccatcgaggaactcttcgataacgatgcgatgacccgcgtcgccaaaagcgttgcccgccagcatatcgtgaacagccgcttccgcttcttccagcgtcatcgccacgataacgcctttcccggcagccagaccgtccgctttaatgacgattggcgcgcctttctcacgcagatacgccagcgcaggttctacctcggtgaagttctggtattccgccgtagggatcttatggcgggccaggaaatctttggtaaacgcttttgagccttccagttgggccgcacctgcggttgggccgaagattttcagcccggcggcgcggaaggtatcgaccacgcctttcaccagcggcgcttccgggccgacgatggtcagatcaatcttttcgttttgtgcgaaatccaacagcgccgggatatcggtcacgccaatagcaacgttttgcagcgcgggttccagtgcagtgcctgcattacccggagcaacaaaaacagtctcaaccagcggcgactgggccgctttccaggccagcgcgtgctcgcgcccgccgttaccaatcactaatactttcatctattgctccattaatggcggaagtggcgcatgtcggtgaagagcatcgcaataccgtgctcgtcggcggcggcaatcacttcgtcatcacggatagaaccgccaggctggattacgcaggtcacgcccgcagcggcggcggcatcaataccgtcgcggaacgggaagaacgcgtcagaagccatcgaggaacctttcacttccaggccttcatcggccgctttaataccggcgatttttgcggagtacacgcggctcatctggcccgcgccaatgccgatagtcatattgtttttggcatagacgatagcgttggatttcacaaacttcgccaccttccagcagaacagcgcatcacgcagttcctgttcgctcggctgacgtttggtcaccacgcgcagttcttccgcaccgaccatccccaggtcacgatcctgaaccagcagaccgccgttcacgcgtttgaaatcgaggcccggaacacgctcgccccactgaccgcaggtcagaacgcgtacgttctgtttggcggcggtgattttcagggcttcttcgctggcggacggcgcaataatcacttcgacaaactgacgagaaatgatggcctgtgcggtttccgcatccagctcgcggttaaaggcaatgatgccgccgaatgcggaggttgggtcggttttgtacgcgcgatcgtaagcatcaagaatggaattgccgatagccacgccgcaagggttggcgtgcttcacaatcacacatgccggctcggcgaactctttcacgcactccagcgccgcatcggtatcggcgatgttgttataagagagggctttaccctgaacctgggttgcggtagcaacggaggcttctttcacattctcttctatatagaaggcagcctgctggtggctgttctcgccgtaacgcatatccagcttcttaatgaagttcaggttcagcgtgcgtgggaagcgaccggcggcttctttgctttcaccgtggtaagccggaaccatgctgccgaagtagttggcaatcatgctgtcgtaggcggcagtgtgttcgaaggctttgatggcgaggtcgaaacgggttgcaagcgtcagcgatccttcgttgtcatccatctctttaataatggcgtcatagtcgctgctcttcaccacgattgcgacatctttatggttcttggcggcggagcgcaccatcgttgggccgccgatatcgatgttctcaaccgcatcttccagcgagcaaccttcacgggccacggtctgggcgaacggatacaggttaacaaccaccatatcgataggctggatctgatgttcttccataatggcatcgtcctggccgcgacggcccagaatgccaccatgtactttcggatgcagggtcttcacgcgtccatccatcatctccgggaaaccggtgtaatcggaaacttcggttaccggcagacctttttctgctaacagacgggcagtgccccctgtagacagcagctccacaccgcgtgcggaaagtgcctgggcgaattcgacgataccggctttgtcagaaacactgagcagagcgcggcggactggacgacgttgttgcatggtaaatcccctggatttgactattacagagagcgttagctgaatttttcgcgaaaaactcagctaacgcccctaacggggcatccttatttttcgcccgcattgtaacgaaaacgtttgcgcaacgctcgcgaatttttctctttcaatggtgatcacaattttgactgtggttaccgtgggcaaaatacagaaattacattgatgattgtggataactctgtgcgtaaaaaggtataaagcgggcttttgctggggaatgcagcagtcagtcatttttctgcaatttttctattgcggcctgcggagaactccctataatgcgcctccatcgacacggcggatgtgaatcacttcacacaaacagccggttcggttgaagagaaaaatcctgaaattcagggttgactctgaaagaggaaagcgtaatatacgccacctcgcgacagtgcgctaaagcgcgtcgcaactgctctttaacaatttatcagacaatctgtgtgggcactcgaagatacggattcttaacgtcgcaagacgaaaaatgaataccaagtctcaagagtgaacacgtaattcattacgaagtttaattctttgagcatcaaacttttaaattgaagagtttgatcatggctcagattgaacgctggcggcaggcctaacacatgcaagtcgaacggtaacaggaagaagcttgcttctttgctgacgagtggcggacgggtgagtaatgtctgggaaactgcctgatggagggggataactactggaaacggtagctaataccgcataacgtcgcaagaccaaagagggggaccttcgggcctcttgccatcggatgtgcccagatgggattagctagtaggtggggtaacggctcacctaggcgacgatccctagctggtctgagaggatgaccagccacactggaactgagacacggtccagactcctacgggaggcagcagtggggaatattgcacaatgggcgcaagcctgatgcagccatgccgcgtgtatgaagaaggccttcgggttgtaaagtactttcagcggggaggaagggagtaaagttaatacctttgctcattgacgttacccgcagaagaagcaccggctaactccgtgccagcagccgcggtaatacggagggtgcaagcgttaatcggaattactgggcgtaaagcgcacgcaggcggtttgttaagtcagatgtgaaatccccgggctcaacctgggaactgcatctgatactggcaagcttgagtctcgtagaggggggtagaattccaggtgtagcggtgaaatgcgtagagatctggaggaataccggtggcgaaggcggccccctggacgaagactgacgctcaggtgcgaaagcgtggggagcaaacaggattagataccctggtagtccacgccgtaaacgatgtcgacttggaggttgtgcccttgaggcgtggcttccggagctaacgcgttaagtcgaccgcctggggagtacggccgcaaggttaaaactcaaatgaattgacgggggcccgcacaagcggtggagcatgtggtttaattcgatgcaacgcgaagaaccttacctggtcttgacatccacggaagttttcagagatgagaatgtgccttcgggaaccgtgagacaggtgctgcatggctgtcgtcagctcgtgttgtgaaatgttgggttaagtcccgcaacgagcgcaacccttatcctttgttgccagcggtccggccgggaactcaaaggagactgccagtgataaactggaggaaggtggggatgacgtcaagtcatcatggcccttacgaccagggctacacacgtgctacaatggcgcatacaaagagaagcgacctcgcgagagcaagcggacctcataaagtgcgtcgtagtccggattggagtctgcaactcgactccatgaagtcggaatcgctagtaatcgtggatcagaatgccacggtgaatacgttcccgggccttgtacacaccgcccgtcacaccatgggagtgggttgcaaaagaagtaggtagcttaaccttcgggagggcgcttaccactttgtgattcatgactggggtgaagtcgtaacaaggtaaccgtaggggaacctgcggttggatcacctccttaccttaaagaagcgttctttgcagtgctcacacagattgtctgatagaaagtgaaaagcaaggcgtcttgcgaagcagactgatacgtccccttcgtctagaggcccaggacaccgccctttcacggcggtaacaggggttcgaatcccctaggggacgccacttgctggtttgtgagtgaaagtcacctgccttaatatctcaaaactcatcttcgggtgatgtttgagatatttgctctttaaaaatctggatcaagctgaaaattgaaacactgaacaacgaaagttgttcgtgagtctctcaaattttcgcaacacgatgatgaatcgtaagaaacatcttcgggttgtgaggttaagcgactaagcgtacacggtggatgccctggcagtcagaggcgatgaaggacgtgctaatctgcgataagcgtcggtaaggtgatatgaaccgttataaccggcgatttccgaatggggaaacccagtgtgtttcgacacactatcattaactgaatccataggttaatgaggcgaaccgggggaactgaaacatctaagtaccccgaggaaaagaaatcaaccgagattcccccagtagcggcgagcgaacggggagcagcccagagcctgaatcagtgtgtgtgttagtggaagcgtctggaaaggcgcgcgatacagggtgacagccccgtacacaaaaatgcacatgctgtgagctcgatgagtagggcgggacacgtggtatcctgtctgaatatggggggaccatcctccaaggctaaatactcctgactgaccgatagtgaaccagtaccgtgagggaaaggcgaaaagaaccccggcgaggggagtgaaaaagaacctgaaaccgtgtacgtacaagcagtgggagcacgcttaggcgtgtgactgcgtaccttttgtataatgggtcagcgacttatattctgtagcaaggttaaccgaataggggagccgaagggaaaccgagtcttaactgggcgttaagttgcagggtatagacccgaaacccggtgatctagccatgggcaggttgaaggttgggtaacactaactggaggaccgaaccgactaatgttgaaaaattagcggatgacttgtggctgggggtgaaaggccaatcaaaccgggagatagctggttctccccgaaagctatttaggtagcgcctcgtgaattcatctccgggggtagagcactgtttcggcaagggggtcatcccgacttaccaacccgatgcaaactgcgaataccggagaatgttatcacgggagacacacggcgggtgctaacgtccgtcgtgaagagggaaacaacccagaccgccagctaaggtcccaaagtcatggttaagtgggaaacgatgtgggaaggcccagacagccaggatgttggcttagaagcagccatcatttaaagaaagcgtaatagctcactggtcgagtcggcctgcgcggaagatgtaacggggctaaaccatgcaccgaagctgcggcagcgacgcttatgcgttgttgggtaggggagcgttctgtaagcctgcgaaggtgtgctgtgaggcatgctggaggtatcagaagtgcgaatgctgacataagtaacgataaagcgggtgaaaagcccgctcgccggaagaccaagggttcctgtccaacgttaatcggggcagggtgagtcgacccctaaggcgaggccgaaaggcgtagtcgatgggaaacaggttaatattcctgtacttggtgttactgcgaaggggggacggagaaggctatgttggccgggcgacggttgtcccggtttaagcgtgtaggctggttttccaggcaaatccggaaaatcaaggctgaggcgtgatgacgaggcactacggtgctgaagcaacaaatgccctgcttccaggaaaagcctctaagcatcaggtaacatcaaatcgtaccccaaaccgacacaggtggtcaggtagagaataccaaggcgcttgagagaactcgggtgaaggaactaggcaaaatggtgccgtaacttcgggagaaggcacgctgatatgtaggtgaggtccctcgcggatggagctgaaatcagtcgaagataccagctggctgcaactgtttattaaaaacacagcactgtgcaaacacgaaagtggacgtatacggtgtgacgcctgcccggtgccggaaggttaattgatggggttagcgcaagcgaagctcttgatcgaagccccggtaaacggcggccgtaactataacggtcctaaggtagcgaaattccttgtcgggtaagttccgacctgcacgaatggcgtaatgatggccaggctgtctccacccgagactcagtgaaattgaactcgctgtgaagatgcagtgtacccgcggcaagacggaaagaccccgtgaacctttactatagcttgacactgaacattgagccttgatgtgtaggataggtgggaggctttgaagtgtggacgccagtctgcatggagccgaccttgaaataccaccctttaatgtttgatgttctaacgttgacccgtaatccgggttgcggacagtgtctggtgggtagtttgactggggcggtctcctcctaaagagtaacggaggagcacgaaggttggctaatcctggtcggacatcaggaggttagtgcaatggcataagccagcttgactgcgagcgtgacggcgcgagcaggtgcgaaagcaggtcatagtgatccggtggttctgaatggaagggccatcgctcaacggataaaaggtactccggggataacaggctgataccgcccaagagttcatatcgacggcggtgtttggcacctcgatgtcggctcatcacatcctggggctgaagtaggtcccaagggtatggctgttcgccatttaaagtggtacgcgagctgggtttagaacgtcgtgagacagttcggtccctatctgccgtgggcgctggagaactgaggggggctgctcctagtacgagaggaccggagtggacgcatcactggtgttcgggttgtcatgccaatggcactgcccggtagctaaatgcggaagagataagtgctgaaagcatctaagcacgaaacttgccccgagatgagttctccctgactccttgagagtcctgaaggaacgttgaagacgacgacgttgataggccgggtgtgtaagcgcagcgatgcgttgagctaaccggtactaatgaaccgtgaggcttaaccttacaacgccgaaggtgttttggcggattgagagaagattttcagcctgatacagattaaatcagaacgcagaagcggtctgataaaacagaatttgcctggcggcagtagcgcggtggtcccacctgaccccatgccgaactcagaagtgaaacgccgtagcgccgatggtagtgtggggtctccccatgcgagagtagggaactgccaggcatcaaattagaaaaaccccggtccataaggccggggttttttgcatatcaattatttgcatgatgaagggaatctcatgtcagttctgtatatccaaattcgtcgtaatcaaattactgttcgcgatcttgaaagcaaacgtgaagtgtcaggagacgctgccttcagtaaccagcgcctgttaatcgccaatttctttgttgcagaaaaagttctgcaagatcttgttctgcaactccacccacgttcaacctggcattcttttttgccagcaaaacgtatggatattgttgtgagcgcactggaaatgaatgagggcggtttgtcacaggttgaggaacgcattctccatgaagtggtcgctggggcaacgttaatgaaatatcgccagttccacatccatgcgcaatcagcggtactcagtgatagtgcggtcatggcaatgcttaagcagaaataatcgtgtcaccattggtgggtactaaacctgaagttcagcccaccgggatgagaaaaaatcgcctacgcccccacatacgccagattcagcaacggatacggtttccccaaatcgtccacctcagagcgtcccgtaaccttaaaacccaccttcttatagaacccaaccgcctgctcattttgctcattaacgttggttgtcagttccggtgccatcgagagcgcatgctccaccagcacccgacctacgccgcagccgcgcacatcaggatcgataaacagcgcatccatatgctgcccacttagcaacataaatccaaccggctgatcccgctcattaaccgcgacccacaacggcgcttccggcaggaaggaacgaactaggtcctccagctcggtccgatactctgctgatagaaaatcgtgagtggcatcgacagaacgacaccaaatcgcaacgagttcctccccttcctcatgccgtgagcggcgaatactaataaccattttctctccttttagtcattcttatattctaacgtagtcttttccttgaaactttctcaccttcaacatgcaggctcgacattggcaaattttctggttatcttcagctatctggatgtctaaacgtataagcgtatgtagtgaggtaatcaggttatgccgattcgtgtgccggacgagctacccgccgtcaatttcttgcgtgaagaaaacgtctttgtgatgacaacttctcgtgcgtctggtcaggaaattcgtccacttaaggttctgatccttaacctgatgccgaagaagattgaaactgaaaatcagtttctgcgcctgctttcaaactcacctttgcaggtcgatattcagctgttgcgcatcgattcccgtgaatcgcgcaacacgcccgcagagcatctgaacaacttctactgtaactttgaagatattcaggatcagaactttgacggtttgattgtaactggtgcgccgctgggcctggtggagtttaatgatgtcgcttactggccgcagatcaaacaggtgctggagtggtcgaaagatcacgtcacctcgacgctgtttgtctgctgggcggtacaggccgcgctcaatatcctctacggcattcctaagcaaactcgcaccgaaaaactctctggcgtttacgagcatcatattctccatcctcatgcgcttctgacgcgtggctttgatgattcattcctggcaccgcattcgcgctatgctgactttccggcagcgttgattcgtgattacaccgatctggaaattctggcagagacggaagaaggggatgcatatctgtttgccagtaaagataagcgcattgcctttgtgacgggccatcccgaatatgatgcgcaaacgctggcgcaggaatttttccgcgatgtggaagccggactagacccggatgtaccgtataactatttcccgcacaatgatccgcaaaatacaccgcgagcgagctggcgtagtcacggtaatttactgtttaccaactggctcaactattacgtctaccagatcacgccatacgatctacggcacatgaatccaacgctggattaatcttctgtgatagtcgatcgttaagcgattcagcaccttacctcaggcaccttcgggtgccttttttatttccgaaacgtacctcagcaggtgaataaattttattcatattgttatcaacaagttatcaagtatttttaattaaaatggaaattgtttttgattttgcattttaaatgagtagtcttagttgtgctgaacgaaaagagcacaacgatccttcgttcacagtggggaagttttcggatccatgacgaggagctgcacgatgactgaacaggcaacaacaaccgatgaactggctttcacaaggccgtatggcgagcaggagaagcaaattcttactgccgaagcggtagaatttctgactgagctggtgacgcattttacgccacaacgcaataaacttctggcagcgcgcattcagcagcagcaagatattgataacggaacgttgcctgattttatttcggaaacagcttccattcgcgatgctgattggaaaattcgcgggattcctgcggacttagaagaccgccgcgtagagataactggcccggtagagcgcaagatggtgatcaacgcgctcaacgccaatgtgaaagtctttatggccgatttcgaagattcactggcaccagactggaacaaagtgatcgacgggcaaattaacctgcgtgatgcggttaacggcaccatcagttacaccaatgaagcaggcaaaatttaccagctcaagcccaatccagcggttttgatttgtcgggtacgcggtctgcacttgccggaaaaacatgtcacctggcgtggtgaggcaatccccggcagcctgtttgattttgcgctctatttcttccacaactatcaggcactgttggcaaagggcagtggtccctatttctatctgccgaaaacccagtcctggcaggaagcggcctggtggagcgaagtcttcagctatgcagaagatcgctttaatctgccgcgcggcaccatcaaggcgacgttgctgattgaaacgctgcccgccgtgttccagatggatgaaatccttcacgcgctgcgtgaccatattgttggtctgaactgcggtcgttgggattacatcttcagctatatcaaaacgttgaaaaactatcccgatcgcgtcctgccagacagacaggcagtgacgatggataaaccattcctgaatgcttactcacgcctgttgattaaaacctgccataaacgcggtgcttttgcgatgggcggcatggcggcgtttattccgagcaaagatgaagagcacaataaccaggtgctcaacaaagtaaaagcggataaatcgctggaagccaataacggtcacgatggcacatggatcgctcacccaggccttgcggacacggcaatggcggtattcaacgacattctcggctcccgtaaaaatcagcttgaagtgatgcgcgaacaagacgcgccgattactgccgatcagctgctggcaccttgtgatggtgaacgcaccgaagaaggtatgcgcgccaacattcgcgtggctgtgcagtacatcgaagcgtggatctctggcaacggctgtgtgccgatttatggcctgatggaagatgcggcgacggctgaaatttcccgtacctcgatctggcagtggatccatcatcaaaaaacgttgagcaatggcaaaccggtgaccaaagccttgttccgccagatgctgggcgaagagatgaaagtcattgccagcgaactgggcgaagaacgtttctcccaggggcgttttgacgatgccgcacgcttgatggaacagatcaccacttccgatgagttaattgatttcctgaccctgccaggctaccgcctgttagcgtaaaccaccacataactatggagcatctgcacatgaaaacccgtacacaacaaattgaagaattacagaaagagtggactcaaccgcgttgggaaggcattactcgcccatacagtgcggaagatgtggtgaaattacgcggttcagtcaatcctgaatgcacgctggcgcaactgggcgcagcgaaaatgtggcgtctgctgcacggtgagtcgaaaaaaggctacatcaacagcctcggcgcactgactggcggtcaggcgctgcaacaggcgaaagcgggtattgaagcagtctatctgtcgggatggcaggtagcggcggacgctaacctggcggccagcatgtatccggatcagtcgctctatccggcaaactcggtgccagctgtggtggagcggatcaacaacaccttccgtcgtgccgatcagatccaatggtccgcgggcattgagccgggcgatccgcgctatgtcgattacttcctgccgatcgttgccgatgcggaagccggttttggcggtgtcctgaatgcctttgaactgatgaaagcgatgattgaagccggtgcagcggcagttcacttcgaagatcagctggcgtcagtgaagaaatgcggtcacatgggcggcaaagttttagtgccaactcaggaagctattcagaaactggtcgcggcgcgtctggcagctgacgtgacgggcgttccaaccctgctggttgcccgtaccgatgctgatgcggcggatctgatcacctccgattgcgacccgtatgacagcgaatttattaccggcgagcgtaccagtgaaggcttcttccgtactcatgcgggcattgagcaagcgatcagccgtggcctggcgtatgcgccatatgctgacctggtctggtgtgaaacctccacgccggatctggaactggcgcgtcgctttgcacaagctatccacgcgaaatatccgggcaaactgctggcttataactgctcgccgtcgttcaactggcagaaaaacctcgacgacaaaactattgccagcttccagcagcagctgtcggatatgggctacaagttccagttcatcaccctggcaggtatccacagcatgtggttcaacatgtttgacctggcaaacgcctatgcccagggcgagggtatgaagcactacgttgagaaagtgcagcagccggaatttgccgccgcgaaagatggctataccttcgtatctcaccagcaggaagtgggtacaggttacttcgataaagtgacgactattattcagggcggcacgtcttcagtcaccgcgctgaccggctccactgaagaatcgcagttctaagcaacaacaaccgttgctgactgtaggccggataaggcgttcacgccgcatccggcaatcggtgcacgatgcctgatgcgacgcttgcgcgtcttatcatgcctacagccgttgccgaacgtaggctggataaggcgtttacgccgcatccggcaattctctgctcctgatgagggcgctaaatgccgcgtggcctggaattattgattgctcaaaccattttgcaaggcttcgatgctcagtatggtcgattcctcgaagtgacctccggtgcgcagcagcgtttcgaacaggccgactggcatgctgtccagcaggcgatgaaaaaccgtatccatctttacgatcatcacgttggtctggtcgtggagcaactgcgctgcattactaacggccaaagtacggacgcggcatttttactacgtgttaaagagcattacacccggctgttgccggattacccgcgcttcgagattgcggagagcttttttaactccgtgtactgtcggttatttgaccaccgctcgcttactcccgagcggctttttatctttagctctcagccagagcgccgctttcgtaccattccccgcccgctggcgaaagactttcaccccgatcacggctgggaatctctactgatgcgcgttatcagcgacctaccgctgcgcctgcgctggcagaataaaagccgtgacatccattacattattcgccatctgacggaaacgctggggacagacaacctcgcggaaagtcatttacaggtggcgaacgaactgttttaccgcaataaagccgcctggctggtaggcaaactgatcacaccttccggcacattgccatttttgctgccgatccaccagacggacgacggcgagttatttattgatacctgcctgacgacgaccgccgaagcgagcattgtttttggctttgcgcgttcttattttatggtttatgcgccgctgcccgcagcgctggtcgagtggctacgggaaattctgccaggtaaaaccaccgctgaattgtatatggctatcggctgccagaagcacgccaaaaccgaaagctaccgcgaatatctcgtttatctacagggctgtaatgagcagttcattgaagcgccgggtattcgtggaatggtgatgttggtgtttacgctgccgggctttgatcgggtattcaaagtcatcaaagacaggttcgcgccgcagaaagagatgtctgccgctcacgttcgtgcctgctatcaactggtgaaagagcacgatcgcgtgggccgaatggcggacacccaggagtttgaaaactttgtgctggagaagcggcatatttccccggcattaatggaattactgcttcaggaagcagcggaaaaaatcaccgatctcggcgaacaaattgtgattcgccatctttatattgagcggcggatggtgccgctcaatatctggctggaacaagtggaaggtcagcagttgcgcgacgccattgaagaatacggtaacgctattcgccagcttgccgctgctaacattttccctggcgacatgctgtttaaaaacttcggtgtcacccgtcacgggcgtgtggttttttatgattacgatgaaatttgctacatgacggaagtgaatttccgcgacatcccgccgccgcgctatccggaagacgaacttgccagcgaaccgtggtacagcgtctcgccgggcgatgttttcccggaagagtttcgccactggctatgcgccgacccgcgtattggtccgctgtttgaagagatgcacgccgacctgttccgcgctgattactggcgcgcactacaaaaccgcatacgtgaagggcatgtggaagatgtttatgcgtatcggcgcaggcaaagatttagcgtacggtatggggagatgcttttttgagtaaagcttccatataatttttctccgcaatgtatcgagggttatccgtaaagccaaagctttcagccatcttatttaatgtattaaggattaattcagcaataacccggtgaccaaattcaaaagccaactcaaaggcagagtatttttgtggggctttgtgttgccaaaaatccataatatcttcagcggtaaatccaaacaggcgtgcatggtcagataaagcaagataaaccgtctctacaacattttgttgtttatgctgtatcgctgaaaacaaaccgggatattcattagaattatttgccaggaggaggggcttcatattttttttatcgaatttaaacgtattaaacagagtgggtaatgcgttaaaaatagtattaataacgttcatgtgtccgcgctgcatggccataaacaaacccgtgtcgcgcgcaagacttttagcggtcagaagatctacaatatcggaagctgaaatgttaatttcctgggctaggctgggcaatgcttcaagaataactttcacgatatcgctatgtccattttgcatcgccagatatagtcctgggcaaccataaaaatcctttgccttcaggagatcgagtacctgttctttagtcaaatgacatgtgcgaattaacaaaggtaacgcgttcaaaacaattttcagcatgtcggcatcaccattcgccataacatggtataaaacatggctggacgttctatttttggcactcaggaatttatacacttgttcgttatctaaatgatgtgttgcggccagtttaggtaaggcgttcagaatcgaggttacaacatttttatccttacgtgatatcgctaaaaataatccagaaaaaccatttttatcttttgcctccagaatatgcatgagattttttttcgagagtaatccttcatatcctgtttctgacaatgaattgaaaatagtctcaacgatatccgcattaccataatttatagccaaatataaacctggcaggttaatactattataggcagtcaacatttctgttctatgtagttctggcattttctggagttgaatcatcagttgcgtaagttggtgattctgaccaattgccattagcaaattcatcgttgcaggtgataatggaggggttatttcatccacagatccttttaacatcaatagctgttctttcggaagtgctggaattattgcaacagattgattaataacatgatcatttgaccatttcaggaggctataatctacattcataaaatccatcagagaatagtgtttaatattctctttgctttcgctcataattcttattttatcgttagttacattaggatcataaaccgaaaccacgtaatgggtacatccttcagttgtgttctttattcttagccggaccgtcaaagcatggttatccaccagtaatatggctgccataacactgatgccatttgattccatcttgtcaaaatatgctttcataactagcccgaaatcaccgcaggcagcaacgcaacgcccctcaggacggctggaaaccaacgccaaagtctggtttttgcattttttgttgaagtgcgtgagaaatttttcagctgaagagtaatcatcttgatggggtttgtaatcaacattctgataaatatcattaatatattgtgcagcaatgtgtcggcatactatacggttttggggtcgccccggaaaataacattgaccattaagtttaattcttgggaattctttttcttttctatctgattttaggtttaattcttgtttatcaagagtgtctgagcgttgaggtaaaatttccattaggtatttttcaaatattggggcaatggtttgagtaagtgtcgtgttttcgtttttattaattatcgtaatttctttcttatcagcttgtaagacggacgtggaaaatttaatgacaaaatccttgttgctaaagatatgacgaccattttgtctacagttctctgagaagctttttaatagaggcgtcgccagctccttgccagaaaatttatcctcgagttctttataaaacaattcactcagggtttggtgttcatttgtctgggctgtattattaatatttgcagagaaagaactacgaggaatacgagtaatcatttaaatatctcattgtttattgatgtcttgaattttaactatcagaacagtgaaaaaatttaatatgattacaactaaagaaatatcataaatcgctcaatctcataatgcagccgtaaaagtttcggtggaatgagatcttgcgattttgttaataattaagtggtttgatgtttaaaaataatgctgagttaataaaagtgtgtgaagtgtatgacattaagttattttggcgtcaatgcgattaacagacacccttattctattgccactcaggtatgatgggcagaatattgcctctgcccgccagaaaaagtcagcgcattccaccgtacgccagcgtcacttccttcgccgctttaatcaccatcgcgccaaactcggtcacgcggtcatcggtaatacgtgaaatcggtccggaaatagaaattgcggcaaacggttcacggtgctcatcgaaaatacacgctgcaaggcaacgtagccccagtgcatgttcctcatcgtcaaatgaataaccccgtttgcgcgtttgggcgagatcttcttttaaatgcacaggagacaccagcgttgcgtgggtataggcatgtaaccctttgcggtgcagcagcttcgtcacctgttcttcgctcagttgggctaaaaaggctttacccgcaccggaagcgtgcatcggcaatttaccgccgataggcgcggacattcgcatcagatgcgtacactgtacctggtcgataataatcgcttcgtgatcgctttgatcaagcaccgccatattgaccgtttcgccagactcttccattagattgcgcaggatagggtgaacaatcgctaacaaattacggctctggagaaagctgctgccgaccataaaggcatgtgcgccgattgcccaatgtcccagttcgccaacctgacgcacgaaaccctgctgttgcatcgtggttagcaggcggtgggtcgtggaattgggtaacccggcttgttgcgccagttccgtgagtgccacactgccattggattcggcaatccactccagtaatttcaggccacgcgttaaagactgaacctgtccagtcgctggtgcggtggcaacggcgggttttctgccgcgtttcgcgggaatgggtgcgaccatgacagtctcttttttctgtatcgtggaaatcattttcatttttattgttagctaatgcaatagttactgaactgatccgatgagttaatgttgaacaaatctcatgttgcgtggtggtcgcttttaccacagatgcgtttatgccagtatggtttgttgaatttttattaaatctgggttgagcgtgtcgggagcaagtgtgagcagcaaagtggaacaactgcgtgcgcagttaaatgaacgtattctggtgctggacggcggtatgggcaccatgatccagagttatcgactgaacgaagccgattttcgtggtgaacgctttgccgactggccatgcgacctcaaaggcaacaacgacctgctggtactcagtaaaccggaagtgatcgccgctatccacaacgcctactttgaagcgggcgcggatatcatcgaaaccaacaccttcaactccacgaccattgcgatggcggattaccagatggaatccctgtcggcggaaatcaactttgcggcggcgaaactggcgcgagcttgtgctgacgagtggaccgcgcgcacgccagagaaaccgcgctacgttgccggtgttctcggcccgaccaaccgcacggcgtctatttctccggacgtcaacgatccggcatttcgtaatatcacttttgacgggctggtggcggcttatcgagagtccaccaaagcgctggtggaaggtggcgcggatctgatcctgattgaaaccgttttcgacacccttaacgccaaagcggcggtatttgcggtgaaaacggagtttgaagcgctgggcgttgagctgccgattatgatctccggcaccatcaccgacgcctccgggcgcacgctctccgggcagaccaccgaagcattttacaactcattgcgccacgccgaagctctgacctttggcctgaactgtgcgctggggcccgatgaactgcgccagtacgtgcaggagctgtcacggattgcggaatgctacgtcaccgcgcacccgaacgccgggctacccaacgcctttggtgagtacgatctcgacgccgacacgatggcaaaacagatacgtgaatgggcgcaagcgggttttctcaatatcgtcggcggctgctgtggcaccacgccacaacatattgcagcgatgagtcgtgcagtagaaggattagcgccgcgcaaactgccggaaattcccgtagcctgccgtttgtccggcctggagccgctgaacattggcgaagatagcctgtttgtgaacgtgggtgaacgcaccaacgtcaccggttccgctaagttcaagcgcctgatcaaagaagagaaatacagcgaggcgctggatgtcgcgcgtcaacaggtggaaaacggcgcgcagattatcgatatcaacatggatgaagggatgctcgatgccgaagcggcgatggtgcgttttctcaatctgattgccggtgaaccggatatcgctcgcgtgccgattatgatcgactcctcaaaatgggacgtcattgaaaaaggtctgaagtgtatccagggcaaaggcattgttaactctatctcgatgaaagagggcgtcgatgcctttatccatcacgcgaaattgttgcgtcgctacggtgcggcagtggtggtaatggcctttgacgaacagggacaggccgatactcgcgcacggaaaatcgagatttgccgtcgggcgtacaaaatcctcaccgaagaggttggcttcccgccagaagatatcatcttcgacccaaacatcttcgcggtcgcaactggcattgaagagcacaacaactacgcgcaggactttatcggcgcgtgtgaagacatcaaacgcgaactgccgcacgcgctgatttccggcggcgtatctaacgtttctttctcgttccgtggcaacgatccggtgcgcgaagccattcacgcagtgttcctctactacgctattcgcaatggcatggatatggggatcgtcaacgccgggcaactggcgatttacgacgacctacccgctgaactgcgcgacgcggtggaagatgtgattcttaatcgtcgcgacgatggcaccgagcgtttactggagcttgccgagaaatatcgcggcagcaaaaccgacgacaccgccaacgcccagcaggcggagtggcgctcgtgggaagtgaataaacgtctggaatactcgctggtcaaaggcattaccgagtttatcgagcaggataccgaagaagcccgccagcaggctacgcgcccgattgaagtgattgaaggcccgttgatggacggcatgaatgtggtcggcgacctgtttggcgaagggaaaatgttcctgccacaggtggtcaaatcggcgcgcgtcatgaaacaggcggtggcctacctcgaaccgtttattgaagccagcaaagagcagggcaaaaccaacggcaagatggtgatcgccaccgtgaagggcgacgtccacgacatcggtaaaaatatcgttggtgtggtgctgcaatgtaacaactacgaaattgtcgatctcggcgttatggtgcctgcggaaaaaattctccgtaccgctaaagaagtgaatgctgatctgattggcctttcggggcttatcacgccgtcgctggacgagatggttaacgtggcgaaagagatggagcgtcagggcttcactattccgttactgattggcggcgcgacgacctcaaaagcgcacacggcggtgaaaatcgagcagaactacagcggcccgacggtgtatgtgcagaatgcctcgcgtaccgttggtgtggtggcggcgctgctttccgatacccagcgtgatgattttgtcgctcgtacccgcaaggagtacgaaaccgtacgtattcagcacgggcgcaagaaaccgcgcacaccaccggtcacgctggaagcggcgcgcgataacgatttcgcttttgactggcaggcttacacgccgccggtggcgcaccgtctcggcgtgcaggaagtcgaagccagcatcgaaacgctgcgtaattacatcgactggacaccgttctttatgacctggtcgctggccgggaagtatccgcgcattctggaagatgaagtggtgggcgttgaggcgcagcggctgtttaaagacgccaacgacatgctggataaattaagcgccgagaaaacgctgaatccgcgtggcgtggtgggcctgttcccggcaaaccgtgtgggcgatgacattgaaatctaccgtgacgaaacgcgtacccatgtgatcaacgtcagccaccatctgcgtcaacagaccgaaaaaacaggcttcgctaactactgtctcgctgacttcgttgcgccgaagctttctggtaaagcagattacatcggcgcatttgccgtgactggcgggctggaagaggacgcactggctgatgcctttgaagcgcagcacgatgattacaacaaaatcatggtgaaagcgcttgccgaccgtttagccgaagcctttgcggagtatctccatgagcgtgtgcgtaaagtctactggggctatgcgccgaacgagaacctcagcaacgaagagctgatccgcgaaaactaccagggcatccgtccggcaccgggctatccggcctgcccggaacatacggaaaaagccaccatctgggagctgctggaagtggaaaaacacactggcatgaaactcacagaatctttcgccatgtggcccggtgcatcggtttcgggttggtacttcagccacccggacagcaagtactacgctgtagcacaaattcagcgcgatcaggttgaagattatgcccgccgtaaaggtatgagcgttaccgaagttgagcgctggctggcaccgaatctggggtatgacgcggactgattcacaaatctgtcacttttccttacaacaaacagggcgctcaatgagtgccctgtctctttattaatatgaaacacttatactggaaacaggctggaataatcttagccggaaaaacgaatgtcaaaaggcacagtaaagatgccagtcagcgtgtttccggtcctttggtcattcaattgcttcaggaacatataacgataaggagaacctgaactcgtgttaacgctgcttcacctgctttctgccgtcgccctgctggtctgggggactcatattgttcgaaccggcgtaatgcgcgtcttcggcgcgcgtttgcgtactgtccttagccggagcgtcgaaaaaaagccgctcgccttttgcgcggggatcggcgttaccgcactggtacagagcagtaatgccaccaccatgctggtgacctcgtttgtcgctcaggatctggtagccctcgcaccggctctggtcattgtgctgggtgcagatgtcgggacggcgctaatggcgcgtattctcaccttcgacttatcctggctgtcaccgttacttatttttatcggcgtgatttttttcctcggacgcaaacagtcacgcgccgggcaactgggccgcgtcggtattggtcttgggctgattttgctagcgctggagttgattgtgcaggccgtaacgccgatcacccaggcaaacggcgttcaggtgatctttgcctcgctgaccggcgatattctgctggatgcgctgattggcgcgatgttcgccattatcagctactccagccttgctgctgtactgctgaccgcgactctgaccgccgcaggcattatctccttccccgtggcgctctgtctggtgattggtgctaacctcggttccggtctgctggcaatgctcaacaacagtgccgccaatgccgcagcccgccgtgtcgcgctgggtagtctgctgtttaagctggtgggtagcctgattatcctgccgtttgtccatttgctggcagagacaatggggaagttgtcattgccaaaagcggaactggtgatctatttccacgtcttctacaaccttgtacgttgcctggtcatgctgccatttgttgacccgatggcacggttttgcaaaacgattattcgcgatgaaccggaactggatacccagctacggcctaaacatctggatgtcagcgcgctggatacgcccacgcttgctctggcgaacgccgcgcgcgaaaccctgcgcattggcgacgccatggaacagatgatggaagggttgaataaagtgatgcacggtgagccacggcaggagaaagagctgcgtaagctggcagatgatatcaacgttctctacaccgccattaagctgtatctggcgcggatgccaaaagaagagctggcggaggaagagtcgcgccgctgggcagagatcatcgaaatgtcgctcaaccttgaacaggcctccgatatcgtcgagcgcatgggcagcgaaattgctgacaaatcactggcagcacggcgggcattttcgcttgatgggttgaaggaactggatgcgctctatgagcaattgctcagtaatttaaagctggcaatgtcggtgttcttctctggcgatgtcaccagcgctcgtcgtttgcgtcgcagcaaacatcgttttcgcattcttaatcgccgctattcccacgcccacgtcgatcgcctgcatcagcaaaacgtgcagagcattgaaaccagttcgctacatttaggcttactgggagatatgcagcgcctgaactcgctgttttgttcggtggcttacagtgtgctggaacagccggatgaagatgaaggacgggacgagtattaatattgtgaatcctgtaggcctgataagacgcgtcaagcgtcgcatcaggcactatgaacaagatgccggatcatgcatccggcaattcacttaaaaacggtgaccagcttccagcggaaccgcttcttcaccagccttaaacacataagtggtgttcgggccacccagcgtagcgtgacctttactcactgtgatccagttaccttccggtagaccaataatcgtcagttctggcgcgacgaccagcagttcgcgaatacgctgctcacgggtttcacctttatggccttccggcagcgcgttggtgaagtgcgggttgatttgcagcgggaacagatttagcgcatcgaaaccttgcggatcgacaatcggcatatcgttggtggtacgaatagttgggcaagcaaggttagcgcctgcgctccagccaatatacagagcgccacgtttaaccacgtcagtaattggtgccagcagcccgcgctcgcggcactgtttcagcaactggaaagtattcccgccgccgacaatcacgatctcagcattttcaatcgcggcaacgggatcgacaacgctatgaataccggtgacagaaacacccagcggagcgagaaccgcagccgttttcgctgtgtaatcatcccaggtctgcgttacgccagcgaaagggataaacaccgctgagcggcgaccctgcaactgttcagcaattagcggcagtgcatgttccagccaggctttacccggcagcgtcgagttactcaataaaagcagttccattacttctccggttagtaagaaatcacgggaggcatgctaccactgcgaatttaaccacttactgacatggctcacgatgtcgcacattgcttctggaaagtgatttgagcaggtaacgaattcaagccaatggaaataacaaatagttcgctcatgactattttttatcaacccaaaggtacggtatattccgttttttacaggagaatttatgctgcccgactcatcagtccgtttaaataaatacatcagcgaaagcggaatttgctcacgccgcgaagcggatcgctatatcgagcaaggcaatgtgttccttaatggcaagcgagccaccattggcgatcaggtgaaacccggcgacgttgtgaaagtaaacggtcagttgattgaacctcgggaagccgaagatttggtacttatcgccctgaacaagcccgttggtattgtaagcaccaccgaagatggcgagcgcgataacattgtcgatttcgttaaccacagcaaacgcgtgttcccgattggccgcctggataaagactcccaggggctgattttcctcaccaatcacggcgatctggtgaataagatcctgcgtgctggcaatgatcatgagaaagagtatctggtgacggtcgataaaccgattaccgaggagtttattcgcggcatgagtgcgggggtgccaatcctcgggacagtgaccaaaaagtgcaaagttaaaaaagaagcgccgtttgtcttccgcattaccctggtgcaggggctgaaccgtcagatccggcgcatgtgcgagcatttcggctatgaagtgaaaaagctggaacgcacgcgcatcatgaacgttagcttaagcggcattccgctgggggaatggcgcgatttaaccgacgatgagttaatcgacctctttaagctcattgaaaattcctcttccgaggtaaaacctaaagcgaaggccaaaccgaaaacagcgggcatcaaacgtccagtcgttaagatggaaaaaacggcggaaaaaggcggtcgcccggcgtccaacggtaagcgttttacctcgccggggcgtaaaaagaaggggcgctgattaacgcctcagactgatgaaaacggcccaaaagtgcccggacagtcccctcgccccttcgggaaaagggttagggtgaggggaaaattgtgttcacactgacgagtgaaaatctcaggcgttgattgtggattagcgcctgccgcgcgtcgacgtatttgctgaccagctaaatgacgcttcaggatccggtttataagcctgctttttcttcaactggcgggcttttttcgcttcagcctcacgctcaaccattaatttatcgatgtaatctttcttaatgctgttggtttcggagttggtcaatacgcgaccatgcgcaatccgcgcccgatccagcagtgttttaagttcacgctgctcgcgttcagtcatctctttttgggtaatacgggggagtgccatgatggtgccctcagtgagccagagagttcagtgtacgggaattcgtttgcgagcagaactgataatattcattttgccttctcttaactatttatctctttcgataattaattagagatgcagataaaaaaattaaaggcaattattctccgataaagacgctggttaacagagtacaggctcgtttattgatgagcatagtgacaagaaaatcaatacggcccgaaatatagcttccaggccatacagtatttactcaaacaaattactatgcagtttttgcaccacctgctcggcatcttcgccgggcaccaggaagcacaggttatggctggatgcgccataacaaatcatgcgaatgttgaacggttccagtacgccgaatacctctttgccaacgccgcaggcttttgacaggtcattgccaatcaacgcgaccagcgccagaccttcttccacctccacccgacacagtgcggaaagctccatcagcagagattgcgtcagcaacgtatcgccagtggaggttgaaccggtggtatcaagggttaatgccacgctcacttctgacgtggtgattaagtctaccgaaatattatgccgcgcgaggatgccgaaaacttccgcgaggaaaccgcgagaatgcagcatattcaggctgtgcaaagtgagcagagtctgattgcgacgaagcgccagagcgcggaacagcggcggattttcagttttattgcacaccagcgtaccacctgcgcgtgggtctttgctggagccgacaaagaccgggatatcgctgcgtactgcgggtagcaacgttgccggatgcagtacttttgcaccaaaagttgccatctctgccgcttcggcaaacgcgatttcatcaatgcgttttgctgcggaaactacgcgtggatcggtggtgtagatgcccgggacgtcggtccagatatcaacacgagatgcgtgtaaagcctccgccagcaaggctgccgtataatcgctgcctccacggccaagcgtcgttgtacgacctttattttcgctaccgataaatccctgggtgatcactaagccttcattgagacgtgggagcagctgcagcgcggccagttccgccagcgcggctatatctggctctgcacgaccaaatcggtcgttggtacgcatcactttacgtacatcaaaccactgtgcctgaacatcgcgttcgcgcaggatctcaacaaacagcagggtcgacatcagctcgccgtggctgaccagctcatctgtcagcgccggagacgttgccagcgccgccgcttctgccagaacagtaatgttctccagcagacgttcaatctcttcacggataacgttcgggtaacgcagacgttccagaatggcaaactggatgttgcggatagcgtcgagtttttcgaatcgctcgccaggttccagtccttcagctaaagcgaccagcagattagtgataccagcagaagccgagaggacaactaaacgcacgttggcatcagaaagcacaatatcagcgctgcggttcatggcgtcaaaatcagctacgctggtaccgccaaatttggagacaacaatttcagacataactacctcgtgtcaggggatccattttcagccttggcacaagggaagagcggaagacgggtgggcgcagagcgatacttcgctactattttcacccagaagtgctccaccacttgcgaaacgcccgactgcgaacgcttctggtgacaacccaggggattcagcccctgtagccgatgatgaacgtggccagccgttcaatcacctcggcgatgcaccccctcaggtgttatcacaggactggctcctccaacaccgttacttgggcaacgcgcctcttctggcctgcgctagcgcaggtagtacatttataaataaagggtgagcggggcggttgtcaacgatggggtcatgcggatttttcatccactcctggcggtcagtagttcagctaataaatgcttcactgcgctaagggtttacactcaacattacgctaacggcactaaaaccatcacatttttctgtgactggcgctacaatcttccaaagtcacaattctcaaaatcagaagagtattgctaatgaaaaacatcaatccaacgcagaccgctgcctggcaggcactacagaaacacttcgatgaaatgaaagacgttacgatcgccgatctttttgctaaagacggcgatcgtttttctaagttctccgcaaccttcgacgatcagatgctggtggattactccaaaaaccgcatcactgaagagacgctggcgaaattacaggatctggcgaaagagtgcgatctggcgggcgcgattaagtcgatgttctctggcgagaagatcaaccgcactgaaaaccgcgccgtgctgcacgtagcgctgcgtaaccgtagcaataccccgattttggttgatggcaaagacgtaatgccggaagtcaacgcggtgctggagaagatgaaaaccttctcagaagcgattatttccggtgagtggaaaggttataccggcaaagcaatcactgacgtagtgaacatcgggatcggcggttctgacctcggcccatacatggtgaccgaagctctgcgtccgtacaaaaaccacctgaacatgcactttgtttctaacgtcgatgggactcacatcgcggaagtgctgaaaaaagtaaacccggaaaccacgctgttcttggtagcatctaaaaccttcaccactcaggaaactatgaccaacgcccatagcgcgcgtgactggttcctgaaagcggcaggtgatgaaaaacacgttgcaaaacactttgcggcgctttccaccaatgccaaagccgttggcgagtttggtattgatactgccaacatgttcgagttctgggactgggttggcggccgttactctttgtggtcagcgattggcctgtcgattgttctctccatcggctttgataacttcgttgaactgctttccggcgcacacgcgatggacaagcatttctccaccacgcctgccgagaaaaacctgcctgtactgctggcgctgattggcatctggtacaacaatttctttggtgcggaaactgaagcgattctgccgtatgaccagtatatgcaccgtttcgcggcgtacttccagcagggcaatatggagtccaacggtaagtatgttgaccgtaacggtaacgttgtggattaccagactggcccgattatctggggtgaaccaggcactaacggtcagcacgcgttctaccagctgatccaccagggaaccaaaatggtaccgtgcgatttcatcgctccggctatcacccataacccgctctctgatcatcaccagaaactgctgtctaacttcttcgcccagaccgaagcgctggcgtttggtaaatcccgcgaagtggttgagcaggaatatcgtgatcagggtaaagatccggcaacgcttgactacgtggtgccgttcaaagtattcgaaggtaaccgcccgaccaactccatcctgctgcgtgaaatcactccgttcagcctgggtgcgttgattgcgctgtatgagcacaaaatctttactcagggcgtgatcctgaacatcttcaccttcgaccagtggggcgtggaactgggtaaacagctggcgaaccgtattctgccagagctgaaagatgataaagaaatcagcagccacgatagctcgaccaatggtctgattaaccgctataaagcgtggcgcggttaatcatcgtcgatatgtaggccggataaggcgttcacgccgcatccggcaaccgatgcctgatgcgacgcggtcgcgtcttatcaggcctacaggtcgatgccgatatgtacatcgtattcggcaattaatacatagcacgattgattaaataaccttaataacaatgccgacgttatgtcggcatttttttatcagataaatccccttgtctgtaatttaacggaaatcataccgtgaggttaatcctaaaatagatttttaatcgttgtttatttcggaaaatacgcagattaattgcttttgtttttattttaagtttatgatttttattgttatttaaatataagttgaaacttatatttgatattcattccaattatcctaaaacgccatcgctaattccccgcgccgtaattcgcatgctttagttgtgtatactcgatcccgcccgaaatgtttttgggtaaatctccattcattcaatgaagggaaattgttatgaaaaaagttctgtatggcatttttgccatatctgcgcttgcggcgacttctgcgtgggctgcacctgtacaggtgggcgaagcggcagggtcggcagcaacgtcggtttcggcggggagttcctccgcgaccagcgtcagcaccgtaagctcggcggtgggtgtcgcgcttgcggcaaccggtggcggtgatggttctaataccgggaccaccacaaccacgaccaccagtacccagtaataaagtatgtatccccaaaataattcgagtcattgcatctgtggctagaagtatgaagggattaaccataaccacactccggtgtggttattctgcccctctggagaagagtcgtgaagcgacctgcactcattcttatctgcctgttattacaggcctgttcagccacgactaaagagctgggcaattcactgtgggacagtctgttcggcacgccaggcgtacagctgacggatgatgatattcaaaatatgccctacgccagccagtacatgcagcttaatggcgggccgcagttatttgtggtgctggccttcgctgaagacggacaacaaaaatgggtcactcaggatcaggctactctcgttacccaacatggccgtctggtgaagactctgctcggcggcgacaacctgattgaagtgaataaccttgctgccgacccgctgattaaacccgcacaaatcgttgatggcgcaagctggacgcgcacgatgggctggaccgagtaccagcaggtacgctacgccaccgcacgctcagtcttcaaatgggatggcaccgataccgtcaaagtcggcagcgatgaaaccccggttcgcgtgctggacgaagaagtctccaccgaccaggcgcgctggcataaccgctattggatcgacagcgaagggcaaattcgccagtcggaacagtatctcggcgcggattattttccggtgaaaaccactctcatcaaggcggcaaaacaatgattaaacaaactattgtcgcgttgcttttgagtgtgggagcgtcatcggtcttcgcggcaggaaccgtcaaggtgttcagcaatggcagcagtgaggccaaaacgctaacgggcgcagagcatttaatcgatctggtaggccaaccgcggctggcaaacagctggtggcccggtgcggtgattagcgaagagctggcaacggcggcagcattgcgtcagcagcaggcgttgctgacacggctggcagaacagggcgcagattccagcgccgacgatgccgctgcgattaacgccttacgccagcaaattcaggcgttgaaagtgacgggcaggcaaaaaatcaatcttgatcccgatatcgtccgcgttgccgaacgcggtaacccgccgttgcagggcaactacacgctgtgggtcggaccaccgccgtccacggtcacgttgttcgggcttatcagccgtcctggcaagcagccattcactccaggtcgcgacgtggcgagctatctctctgaccagagcctgctcagcggtgcggatcgcagctacgcgtgggtggtttacccggacggacgcacgcaaaaagcgccggtggcttactggaacaagcgtcacgtagagccgatgcccggcagcattatttatgttggcctcgcggactccgtctggagtgagacgcctgatgcccttaacgccgacattcttcagactctgacgcagcggatacctcaataatgaaaaaaagacatctgcttagcttactggcgctgggcattagcacagcttgctacggcgaaacatatcctgcgcccattggtccgtcgcagtcggatttcggtggcgtaggattattacaaacgcccaccgcgcgtatggcacgggaaggggagttgagtctgaactatcgcgataacgatcagtaccgttattactcagcttcagtgcaactcttcccgtggctggaaacaacgctgcgctacaccgacgtgcgcacccggcagtacagcagcgtcgaagcgttctctggcgatcaaacgtataaagataaagccttcgatctcaaactgcgtttgtgggaagagagttactggctgccgcaagtggcggttggtgcgcgggatatcggcggtacggggctgtttgatgcggaatatcttgttgccagcaaagcctgggggccgttcgattttacgctcggcctgggctgggggtatttgggcaccagcggtaatgtgaaaaatccgctctgttcagccagtgataaatattgctatcgcgataacagctacaaacaggcgggatctatcgacggtagccagatgttccacggtcctgcctcactgtttggcggcgtggaataccagacgccctggcaaccgctgcgcctgaaactggagtatgaaggcaataattatcagcaggattttgccgggaagctggagcaaaaaagtaagtttaacgtcggtgcgatttatcgcgttaccgattgggccgacgttaaccttagctatgaacgtggcaacacctttatgtttggcgttacgttgcgcaccaactttaacgatctgcgcccgtcttacaacgataacgcccgcccgcaatatcaaccgcagccgcaggatgccattttgcagcattcggtggtggcgaatcagttaacgctgttgaaatacaatgccggacttgccgatccacagatccaggcgaaaggcgatacgctgtatgttaccggcgagcaggtgaaatatcgtgattcgcgcgaagggatcatccgtgcgaatcggatcgtgatgaacgatctgccggatgggatcaaaacgatccgcattacggaaaatcgccttaacatgccgcaggtgacgacggaaaccgatgtcgccagcctgaaaaatcatctcgccggagagccgttgggccacgaaacgacgctggcgcaaaaacgcgtcgagccagtggttccgcagtccaccgagcagggctggtatatcgacaaatcacgctttgatttccatatcgatccggtgctgaaccagtcggtcggtggcccggaaaacttttacatgtatcagctgggcgtgatgggaacggcagatttgtggctgacggaccatctgctgaccaccggcagcctgtttgcaaatcttgccaacaactacgacaagtttaactacactaatcctccgcaggactcgcacttaccgcgcgtgcgtacccatgtgcgcgagtatgtgcagaacgatgtctatgtgaataacctgcaagccaactacttccagcatctgggcaacggcttctacggtcaggtctacggtggttatctcgaaaccatgtttggcggtgcgggggcagaagtgttgtatcgcccgctggacagcaactgggcgtttggtctggatgccaactacgttaaacagcgcgactggcgtagtgcaaaagatatgatgaaattcaccgactacagcgtgaaaaccggacatctgaccgcctactggacgccatctttcgctcaggatgtgttagttaaagccagcgtcgggcagtatctggcaggggataaaggcggcacgctggagatcgccaaacgctttgatagcggcgtggtggtgggtggctatgccacgatcactaatgtttcgaaagaggagtacggcgaaggggacttcaccaaaggcgtgtatgtctcggtaccgttggatctcttctcgtctggcccgacacgcagccgtgcggcgattggctggacgccgctgacgcgtgacggtggtcagcaacttgggcgtaagttccagttgtatgacatgaccagcgaccgtagcgtcaatttccgctaagtcatgggaaaggtgccagttttcgcactcactggcaccttcattcttaatggcctgtcgagccatcaggaacgcagttcactcccggtttgcgatctggtgtgtaaaggcgaaaacattctgtcttcctgtccgtcgatatcggttgcaggtctggttgcctgagcgactgggccatcattgggctggagacattgctttgcggtaggtcggctttatcagcagtaccgagcggaccagcataagcaggaagaacagagactgataacatcaaagcagcaaaataaggcttcatttttaccacctttatcaggttacgtttcatttgttccagaggaacattgtcgatttttcgcgcattgctggtggctgggaatcacctgaatgggtgatttttgaattaccggctttggtgcggtttgtcttgccggatgcgccgccaggcgcggcttatccggcctacgggtaggtatatccggctttggtggaggcgcgctccaaatccaggttgaacaaaacatacacaaaaaatatagatctccgtcacatttttgcgttatacaggaagctcgccactgtgaaggaggtactgctatgacgtcactctctcgtccgcgcgtggagtttatctccaccattttgcagaccgtactcaatcttggcctgctgtgcctcggcctgattttggttgtcttcctcggcaaagaaacggtgcatctggctgatgtgctgttcgcgccagaacaaaccagcaaatatgagctggtagaaggactggtggtttactttctctatttcgaatttatcgcgctgattgtgaagtactttcagtccggttttcacttcccgctacgttactttgtctatattgggatcaccgccattgtgcgcttgatcatcgtcgatcataaatcgccactggatgtgttgatctactcggctgcgatcctgttactggtgatcaccctgtggctgtgtaattcgaaacggctgaagcgggagtaaaaagtcagcacgccgaaatggcgcggcgtgctggacaggaagattacagcgtagcagtttgttgtgttttcttcgtttccggttcccagagcgcttccagctcctcaagggttttacctttggtttccgggacaaatttccacataaacagtgctgccagaacgcccatacaaccgtaaatccagtaggagaaaccgttgtggaaatgggccaccagccaggagtttttgtccatcatcgggaaggtccaggagacgaagtagttcgccagccactgggccgccaccgcgattgccagcgctttaccacgaatagcattcgggaagatttccgacagcagtacccagcataccggaccccaggacatggcaaaggcggcaacatagaacagcatcgacagtagcgccacaatacccggtgcctgagtgtaaaacgcggtaccgaggctaaacataccgattgccattccgagtgcgccgataatttgcagtggcttacgaccaaatttatccaccgtcataattgccagaacggtgaaggtgaggttgataactccgacaataatggtctgcaacagcgcgatatccgtgctggcccccagcgttttgaacacttccggcgcgtagtacagcaccacattgatgccgacaaattgctggaagatggagagcattacgccgattacaatcacgcccacgccaaacatcagcagacgaccaccggttttgcggccatgatccagggagtgtttaatttcctgtactgcctgagttgcaagcgtgttgcccataattttgcgcaggataccttccgcctgttcttgcttgccgcgcgacatcagccagcgaggactttctggcacggtatacagcagcattaagaacagcagtgcagggatacattccgaggcaaacatataacgccagccgtcagtattcagccagctggcatcaccggaacgggcaataaaatagtttacgcagtaaactaaaagttgcccgaaaataatcgcaaactggttaaaagagaccagtttcccgcgaatatgagctggagccagttccgcaatatacattggcgagagcattgaggctaaaccaacgccaataccgccaataatgcgataaataacaaattccgggacataacctgccagataaacaggcacagtgttgtccgggtttatagaggtaaaaccaagttctggccaggcagaacctacaccagaaataaaaaacaggacagcagcaatcttaagtgaatcacgacgaccgaagcggttactgcaataaccaccgagggcaccgccgatgatgcaaccaatcagagcgctggccacgcaaaaccctaacagggagttggcagcggattcacttaagttttgtggagcaacaaagacggtattgagtgactcaacagtaccggaaataacggcggtgtcgtagccaaataataaaccacctaatgtagcgactaaggtaatcgaaaatatataactggaattatactgggtattcattcagacctgccttagaccattctgatcttttatcagtgcattgatgttggaattgtcaggcagttaaggcaattatcattttttacaatgcgtttacgtaatgtcttttctgtgatcttaattgtgataattatccaaaattgataaaaacaatactattgccgtgactcagagcacgaaagagaattatcgtaagtgggaaaacaaataacgtaaaaataataagctctatgatggaaatattaaccggcgaacgattcagattgcagacgaaagaaaaaaaggcgctccgtggagcgccgaataacagtcacaagttgggataacgtaagttgagggtgcagcggcataacattggcagaacaacatctttaacctttcacaccacctgccgtcaggccgttgaccagccagcgttgagccagcaagaagacgatggtgatcggtaatgcagacatcacggcagcggcggcaaagtcaccccacaggtagttttgcgggttgaggtattgctgcatccccacggccagggtgtagctgtttacgtcacgcagtaacagcgacgcgaccggaacttcagtaatggcagcgataaacgacaggatgaataccaccgccagaatcggtactgacagcggcaacaggacaaggcggaaggcctgccacggtgtcgcaccatccagcgcagcagcttcttccagcgaactgtcgatggtttcgaaatagcctttgatggtccagacatgcagcgcaatcccacccagatacgcgaaaattacgccgccgtgagtattcaggccaatgaatggaatgtactcacccagacgatcaaacaacgcatacaacgcgaccagtgaaagtactgccgggaacatctggaaaatcagcattcctttcagcagcgtcgctttgcctggaaagcgcatacgggcgaaagcgtaggcgcaggtggtggagagcgccacaatgccaatcgcggaaatcccggcgacctttaccgagttccacagccacagcagtaccgggaatggcggtggcgtaatgcgaccatcagcctgttcaacgctaaaacctaacgccagtttccagtgatcccaggagatttgctccgggatcaggctgccggtcgcaaagtttccctgacgcagcgagatagcgacgaccatcagcagcgggaacataatcgctgcgataaaaagtagcagtagcaggtgagtaataaataaacgagctttttgcgatttcggttggaccattgccatttttgttatctcccttaatcaaacttcattcgcgtggctttcaggttcactatcgccagcgcacccaccagcaggaagatcagcgtggcaattgctgccgccagaccgaagtcctgacccccgccgccttcaaaagcgatgcggtaggtgtagttaacaagcaggtcggtataaccggctggcgtggtcgtgccaagacgatccgggccgccgttggttaacagttgaatcagcacgaagttgttaaagttaaaggcgaagctggcgatcatcagcggcgtcagcggtttaatcagcagcggcagcgtaatcttaaagaagttctggaacggacctgcgccatccattgctgaggcttcatacaaatcgtccggaatcgctttcagcaagcccatgcagaggatcatcatgtacggataacccagccaggtattgacgataattagcatcgtgcgggcggtggtcggatcgctgaaccaggcgggcttcacgccaaacagcgcgctcaacatcatgttgatttcaccgaagctctggttaaacaaccctttgaaaatcaagattgaaatgaacgatggcaccgcgtagggcagaatcagcaggacgcgatagaccgctttgccgcgcaacgcttcccactgcaccagacacgccagaaccatgccgaccgccaccgttaaaaagacagtgatcagcgagaacaccacggtccagacgaaaatggcgaggaacggtttctgaatgccttcgtcggtaaagacgcgggtaaagtttttccagccggtggtcacggtgtaaccggggcttagcttttcatcaccccagttgccgtcggcggtaatggactggtaaaagccaatttggttattcggacgatatttcacgccgctctgattattcgtcaacgtgccgtcaccgtcgagtgtgtagagcggctgcgtgccagaaaactggcgcagggagctcatcatcactttgttgccatccggcagaatggcggtaatgtcactcagcgcctgacgattctgggtaatcacgcgcagattcgcgcgttcgccttcgggctgggcggtcgtttctttcagttgcagtttttgctcgccgccaaatttaaaagcgtcggagaggtaatttttgccggtttcgccgtcgctgagcgccagttgccactcatcgcccgccgggtaaagaccaaagttataggttttgcctgcttgccaggagcgatctaacaacacttcctgcgcacgttcaaaagtcagctggttagtgctgctgtagttggtgaaggcaatggcgatggtgcagaccagagggaagaggacgaataatcccattccagccattcccgggtaaacatagcgccaggcgtaggctttacgattggcgaaaatatacagccccgctgaactcaatatcagcgtggtaatggcgaacaggtattccccttgtgcgtacattaaaacaacaaggtaacccaccagcaggccgagcagacctagcactgaccatttcagcgcgtcgctttgccaccaatgtttctttttaatgacatccatggggttcttcctcattccaggacggataaggctttcacgccttatccgacaacaactgcctgatgcgacgctgacgcgtcttatcaggcctacatacgtttcggttttgtaggccggacaaggcgttcacgccgcatccggcatttcacagcattacttggtgatacgagtctgcgcgtctttcagggcttcatcgacagtctgacgaccgctggcggcgttgatcaccgcagtacgcacggcataccagaaagcggacatctgcgggatgttcggcatgatttcacctttctgggcgttttccatggtggcggcaatacgtggatctttcgccaactcttcctcgtaagacttcagcgctacggcacccagcggtttgtctttattaaccgcttccagaccttcatcagtcagcagatagttttcgaggaactctttcgccagctctttgttcggactggcggcgttaatacctgcgctcagcacgccaacgaacggtttggatggttgacccttgaaggtcggcagtaccgttacaccataattcactttgctggtgtcgatgttggaccatgcccacgggccgttgatggtcatcgctgtttcgcctttattaaaggcagcttctgcgatggagtaatcggtgtctgcattcatgtgtttgtttttaatcaggtcaaccaggaaggtcagacccgctttcgcgccagcgttatccacgcccacgtctttaatgtcgtacttgccgttttcatacttgaacgcataacccccgtcagcagcaatcagcggccaggtgaagtacggttcttgcaggttgaacatcagcgcgctcttacctttcgctttcagttctttatccagcgccgggatctcttcccaggtttttggcgggttcggcagcagatctttgttataaatcagcgataacgcttcaacagcgatcgggtaagcaatcagcttgccgttgtaacgtacggcatcccaggtaaacggatacagcttgtcctggaacgctttgtccggggtgatttcagccaacaggccagattgagcgtagccaccaaagcggtcgtgtgcccagaagataatgtcagggccatcgccagttgccgcaacctgtgggaatttctcttccagtttatccggatgctcaacggtgactttaattccggtatctttctcgaatttcttaccgacttcagcgagaccgttatagcctttatcgccgttaatccagattaccagtttaccttcttcgattttggcgagagccgaggcggaaaacatcatcgtcgttaatgcggataatgcgaggatgcgtgcacctgtttttattttcataatctatggtccttgttggtgaagtgctcgtgaaaacacctaaacggactctagtttctttatacggcaacctctttccatcctccttgcccctacgccccaccgtcgctttgtgtgatctctgttacagaattggcggtaatgtggagatgcgcacataaaatcgccacgatttttgcaagcaacatcacgaaattccttacatgacctcggtttagttcacagaagccgtgttctcatcctcccgcctcctcccccataaaaaagccagggggtggaggatttaagccatctcctgatgacgcatagtcagcccatcatgaatgttgctgtcgatgacaggttgttacaaagggagaagggcatggcgagcgtacagctgcaaaatgtaacgaaagcctggggcgaggtcgtggtatcgaaagatatcaatctcgatatccatgaaggtgaattcgtggtgtttgtcggaccgtctggctgcggtaaatcgactttactgcgcatgattgccgggcttgagacgatcaccagcggcgacctgttcatcggtgagaaacggatgaatgacactccgccagcagaacgcggcgttggtatggtgtttcagtcttacgcgctctatccccacctgtcagtagcagaaaacatgtcatttggcctgaaactggctggcgcaaaaaaagaggtgattaaccaacgcgttaaccaggtggcggaagtgctacaactggcgcatttgctggatcgcaaaccgaaagcgctctccggtggtcagcgtcagcgtgtggcgattggccgtacgctggtggccgagccaagcgtatttttgctcgatgaaccgctctccaacctcgatgctgcactgcgtgtgcaaatgcgtatcgaaatctcccgtctgcataaacgcctgggccgcacaatgatttacgtcacccacgatcaggtcgaagcgatgacgctggccgacaaaatcgtggtgctggacgccggtcgcgtggcgcaggttgggaaaccgctggagctgtaccactatccggcagaccgttttgtcgccggatttatcggttcgccaaagatgaacttcctgccggtaaaagtgaccgccaccgcaatcgatcaagtgcaggtggagctgccgatgccaaatcgtcagcaagtctggctgccagttgaaagccgtgatgtccaggttggagccaatatgtcgctgggtattcgcccggaacatctactgccgagtgatatcgctgacgtcatccttgagggtgaagttcaggtcgtcgagcaactcggcaacgaaactcaaatccatatccagatcccttccattcgtcaaaacctggtgtaccgccagaacgacgtggtgttggtagaagaaggtgccacattcgctatcggcctgccgccagagcgttgccatctgttccgtgaggatggcactgcatgtcgtcgactgcataaggagccgggcgtttaagcaccccacaaaacacacaaagcctgtcacaggtgatgtgaaaaaagaaaagcaatgactcaggagatagaatgatgattactctgcgcaaacttcctctggcggttgccgtcgcagcgggcgtaatgtctgctcaggcaatggctgttgatttccacggctatgcacgttccggtattggttggacaggtagcggcggtgaacaacagtgtttccagactaccggtgctcaaagtaaataccgtcttggcaacgaatgtgaaacttatgctgaattaaaattgggtcaggaagtgtggaaagagggcgataagagcttctatttcgacactaacgtggcctattccgtcgcacaacagaatgactgggaagctaccgatccggccttccgtgaagcaaacgtgcagggtaaaaacctgatcgaatggctgccaggctccaccatctgggcaggtaagcgcttctaccaacgtcatgacgttcatatgatcgacttctactactgggatatttctggtcctggtgccggtctggaaaacatcgatgttggcttcggtaaactctctctggcagcaacccgctcctctgaagctggtggttcttcctctttcgccagcaacaatatttatgactataccaacgaaaccgcgaacgacgttttcgatgtgcgtttagcgcagatggaaatcaacccgggcggcacattagaactgggtgtcgactacggtcgtgccaacttgcgtgataactatcgtctggttgatggcgcatcgaaagacggctggttattcactgctgaacatactcagagtgtcctgaagggctttaacaagtttgttgttcagtacgctactgactcgatgacctcgcagggtaaagggctgtcgcagggttctggcgttgcatttgataacgaaaaatttgcctacaatatcaacaacaacggtcacatgctgcgtatcctcgaccacggtgcgatctccatgggcgacaactgggacatgatgtacgtgggtatgtaccaggatatcaactgggataacgacaacggcaccaagtggtggaccgtcggtattcgcccgatgtacaagtggacgccaatcatgagcaccgtgatggaaatcggctacgacaacgtcgaatcccagcgcaccggcgacaagaacaatcagtacaaaattaccctcgcacaacaatggcaggctggcgacagcatctggtcacgcccggctattcgtgtcttcgcaacctacgccaagtgggatgagaaatggggttacgactacaccggtaacgctgataacaacgcgaacttcggcaaagccgttcctgctgatttcaacggcggcagcttcggtcgtggcgacagcgacgagtggaccttcggtgcccagatggaaatctggtggtaatagcaaaacctgggccggataaggcgtttacgccgcattcggcaaccaacgcctgatgcgacgcttgcgcgtcttatcaggcctacaacggctgtcaaatgtaggccggataaggcgtttacgccgcatccggcataaaaacaggttgtcattatctgaaaggggcgaaagcccctctgattatcgggtttagcgcgctattgcctggctaccgctgagctccagattttgaggtgaaaacaatgaaaatgaataaaagtctcatcgtcctctgtttatcagcagggttactggcaagcgcgcctggaattagccttgccgatgttaactacgtaccgcaaaacaccagcgacgcgccagccattccatctgctgcgctgcaacaactcacctggacaccggtcgatcaatctaaaacccagaccacccaactggcgaccggcggccaacaactgaacgttcccggcatcagtggtccggttgctgcgtacagcgtcccggcaaacattggcgaactgaccctgacgctgaccagcgaagtgaacaaacaaaccagcgtttttgcgccgaacgtgctgattcttgatcagaacatgaccccatcagccttcttccccagcagttatttcacctaccaggaaccaggcgtgatgagtgcagatcggctggaaggcgttatgcgcctgacaccggcgttggggcagcaaaaactttatgttctggtctttaccacggaaaaagatctccagcagacgacccaactgctcgacccggctaaagcctatgccaagggcgtcggtaactcgatcccggatatccccgatccggttgctcgtcataccaccgatggcttactgaaactgaaagtgaaaacgaactccagctccagcgtgttggtaggacctttatttggttcttccgctccagctccggttacggtaggtaacacggcggcaccagctgtggctgcacccgctccggcaccggtgaagaaaagcgagccgatgctcaacgacacggaaagttattttaataccgcgatcaaaaacgctgtcgcgaaaggtgatgttgataaggcgttaaaactgcttgatgaagctgaacgcctgggatcgacatctgcccgttccacctttatcagcagtgtaaaaggcaaggggtaattacgccccacagtgctgattttgcaacaactggtgcgtctcctggcgcacctttttttatgcttccttcctgggatatgagcgattttttatagtaactcacttcttcttcactaagaatatccattatctcaatgccttatcagagattcttttcctttcgccggtagtgtctggacattcaggctacttttccaggttattttatttctgttatgcagaggttttatgataagtcatatcctaaattctggcggcaataactctttgatgaaacatgatgtggtgcaaggaaataatatagtagatcttgatttactacgtaatttaaatggggtgccaggtttaaacagagataactttatttatatcagcaatattttttcaaatataaaacaacggaacgaaaaaatcatgcaataaatatgtttcgtgaagtctcaatcagtaatgatactataagtgtaaaattctacagaaatgaaaaaaattgaatgcgcttgcaattttctgatggataaagatgcgcaggggtatatcgacctgtctgatttggatttaacaagttgtcattttaaaggtgacgttatatcgaaggtgtcttttttatcatcaaatctacaacatgtaacattcgaatgtaaagaaattggggattgcaattttactactgcaatagttgataatgtcatatttagatgtcgacgtttacacaatgtgatttttatcaaagcgagtggtgaatgtgtcgatttcagcaaaaatattcttgatacagttgacttctcgcagagtcaacttggtcatagtaattttcgcgaatgtcagattagaaattcaaacttcgataattgttatctttacgcttcgcacttcaccagagcagagtttctgtctgccaaagaaatatcatttattaaatcgaatttgacagctgttatgtttgattatgtgcgaatgtcgacagggaattttaaagattgcattacagaacaattggaattaactattgattattcagatatattttggaatgaagatctcgatggttatatcaataacattataaaaatgattgatacattgccagataatgcaatgatattgaaatccgttctggccgtaaaactggtgatgcaattaaaaatacttaatattgttaataaaaactttattgagaatatgaagaaaatatttagccattgtccttatataaaagatcccattatacgcagttatatccattctgatgaagataacaagttcgatgattttatgcgtcaacatcgattcagtgaggtgaatttcgatacccaacagatgatcgattttattaacagatttaatacgaataaatggctaattgataaaaataacaatttttttatccaacttatcgatcaggccttacgatcaacggatgatatgatcaaagcaaatgtttggcatctttataaagagtggattcgtagtgatgatgtttcacctatatttatagaaactgaagataatttaagaacctttaacacgaatgaattaacacgaaacgataatatctttatcctgttctcctcagtcgatgatgggccagttatggtggtaagctcccagcgcttacatgatatgttgaatcctacaaaagataccaattggaattccacgtatatctacaaatccagacatgagatgttgcctgttaatcttactcaggaaacacttttcagctccaaatctcatggtaaatatgcgcttttccccatttttactgcgagttggcgagctcatcgtataatgaataagggtgtttaagtaaaggaaaacatcaccgttcctggcatcctggacggtgatgcccctacggttgccctcgccagcacgggcatcggtaaagcgtaaggttcaacatcgttttaccacttcatgcgattgttgcgtttttgttgcgtattagatcacttaatttgctttacatctcccgtaaacacttttctgcgatacaatgcctttacgttatgtaacggagagttcggcatgtcacaccccgcgttaacgcaactgcgtgcgctgcgctattgtaaagagatccctgccctggatccgcaactgctcgactggctgttgctggaggattccatgacaaaacgttttgaacagcagggaaaaacggtaagcgtgacgatgatccgcgaagggtttgtcgagcagaatgaaatccccgaagaactgccgctgctgccgaaagagtctcgttactggttacgtgaaattttgttatgtgccgatggtgaaccgtggcttgccggtcgtaccgtcgttcctgtgtcaacgttaagcgggccggagctggcgttacaaaaattgggtaaaacgccgttaggacgctatctgttcacatcatcgacattaacccgggactttattgagataggccgtgatgccgggctgtgggggcgacgttcccgcctgcgattaagcggtaaaccgctgttgctaacagaactgtttttaccggcgtcaccgttgtactaagaggaaaaaaatatggagtggagtctgacgcagaataagctgctggcgtttcatcgcttaatgcgtacggataagccaattggcgcgttactgctgctctggccaacattatgggcgttgtgggtggcgacaccgggcgttccccagctctggatcctggcggtgtttgtcgcgggtgtctggctgatgcgcgctgccggatgtgtggtgaatgattatgctgaccgcaagtttgatggtcatgttaagcgcacggcgaaccgaccacttcccagcggcgcggtaacagagaaagaggcgcgcgcgctgtttgtcgtgctggtactgatttcgtttttactggtgctgacgctgaatacgatgaccattctgttgtcgattgccgcgctagcgctggcgtgggtgtacccgtttatgaagcggtatacccatctaccgcaagtggtgctgggcgcggcgtttggctggtcgattccaatggcttttgccgctgtgagtgagtcggtgccattgagttgctggttaatgttcctcgccaatattctctgggcggtggcttacgacacgcagtatgcgatggttgaccgcgatgatgatgtgaagattggcattaaatccacggcaatcctgttcggccaatacgataaattgattattggtattttgcagattggcgtactggcactgatggcgatcatcggtgagttaaatggcttaggctggggatattactggtcaattctggtggctggcgcgctgtttgtttatcaacaaaaactgattgccaaccgcgagcgtgaagcctgctttaaagcatttatgaataataactatgttggtctggtactatttttagggctggcaatgagttactggcatttctgatgatgtaaaaaagccggatgatcatccggctttcttctgggttgcctgatgcgcggcgcttctcaggcctacacaacacatcgcaatttattgaatttgcagattatggaaggccggataaggcgttttcgccgcatccggcaattctctctgattacccttcgccctgcgtcgcactctcaatcgtcaaacgcacgtctgatgtaatcaactccgccagcaactgataaaccttcatcgtttctgccggttcggcatcgccgctatcgctgatatacccttcatcacgcagtgtcagcaccagagaactgaacaccgccttgtcgaagaactccggcgcgttgatgccgtgcagcacggagagacgttgcgcgacggtgcggctctctttctccagcgtaccgcggttgatcgacgggttggcactcaacaaccagaaggtgatggcataacgttgcagcgtttcgcgcgcgcctgcggccagcagctgtagcgtgcgagaatgcgccgggttgatatgcaactcatcatcttgcagggtaatcagcccctgacgttgcatctcatttgccagcgcatcaataacgtccggcaactcgtcgcgatcccagcgcaggaacagctccgctttcagcattgggtaaagcacattgacgtgctccatcaatacgtcgcgggagatgtggcgatgctgggtgacgattgccgccatcagcgaaggcagcaccaacatatgcgcaatgttgttgcgatagtaggtcatcagcaccgcttgctcgcgcggcagaatgatgatgtcgccgattgtgtctttctcgacttcaaacttgttcatttgcagcgcgtgatcgataagctcgctggcgctggctgaaggaacggtagagtccgtggagtagggcacgttgcgcatcagatccaggtagcagttgagttgctcggttaactgctcgcgggtgagtgagcgctgacgtgatgccagtagcgcagtacagcacaggttcatggcgtttgccgcgcctgcgttgttaatgcgtaccatcagatcggcagcaatattattgaccgtcggcgttaaccatgccggacgcaccgcttcgatgggatcgatagattcacgccagtcaggtacatgctggttaaggtaggtcatcaacggcattggttcaccgaagttgacgtaaccctgaccgagattacgcagcttgcttaaaccgcgcagcatctgcggcaggctctctttctctttcgtcgcgccgcgcagttctttggcgtaagtacccacttccatgacgtgctcataaccgatatagatcggaatcagcgtaatcggacgcgtgccgccacgcagcatcgcctgaatggtcatcgacagcgtaccagttttcggatccagcaaacgccccgtacgggaacgaccgccttccacgaagtactcgacggaataaccacggctgaacagttcgccgagatactcccggaaaacggtggaataaagtttattgcctttaaacgtacggcgaataaagaacgcccccagacggcggaaaatcggcccggcaggccagaaattcaggttgatcccggcggcgatatgcggcggcaccagcccctggtgatacagcacgtaagaaagcagcaggtagtccatgtgactgcggtggcaaggcacatataccagctcatgaccgtcgtgggccagctggcgaacgcgctcagcgttatggacgttgatgccctggtaaagtcggttccaggtgaagcccagaatacggtcagtcaggcgaatcatctcgtaagagaaattcgccgcaatctcttccatcagtgcaatcgcgttctgctgcgctttttcatgggagatttttttgctgcgcgcttcatcttctaccgctttggcaatggcgcgggaggcgagcagcttattaaacagatcctgacgagcaggcaaacgtgggcctacggcagccagacgttgacgggcaaagtgcatacgcgccacgcgcgccagtttctgagcgatagttttatccgtgccgtgttcatccgccatacggcgcagcgaaactgacggcgagaaacgcacaaaactgtcgcgaccgagccacagtacagcgaaaaatttctgtacgccgttaagcatacgcagcggcgggttcacttcgcctttttcacgccccggcgcgcgaccaaacatcaccgacactggcaccatctgcacatccagatttgggttgctacggtgcaaatcgagatagtcgtggaacagcttaatagactcttctttcggcgtgtaataggtgaacacacgcggcccgccgtgaatgaacacatagcgcggcagtagcgtgccgtcgatttccagcggctctaacgggtcaggcaagtcatgtgccagacactgggcgcgcaacgtcagcaaatctgctttcgagttgtacggtaaaacgtacataattggacgagaggtatccagccccagttccggggcaggatctgccggaatagacttgctttttaccaggatgcttaatggtaaattcagtaatttgtagtaaattcgtggccagccggacataaacgatgtaaagcctctggttaataatgcaaatgcgcggcaaggatagcagaaagtcatgggaaattctgtggtatccgctcatgtttcgcgcggcgctacgcaaacccgaatcatcggatttaacggtacactgatattgacgctcataatgtaaaaaggttctttcaatggccaataataccactggattcacccgaattatcaaagctgctggctattcctggaaaggtttacgcgctgcatggatcaacgaagcggcattccgtcaggaaggcgtagcggtattgttggcggtggtcatcgcctgctggctggatgtggacgcgattacccgcgtgctgcttatcagctccgtgatgctggtgatgattgtggaaatcctcaatagcgccatcgaagcagtggttgaccgaattggctctgaataccatgagctttccggacgcgcaaaagatatgggatccgctgcggtgctgattgccattatcgtcgccgtgattacctggtgcattctgttatggtcgcattttggataacccttccagaattcgataaatctctggtttattgtgcagtttatggttccaaaatcgccttttgctgtatatactcacagcataactgtatatacacccagggggcggaatgaaagcgttaacggccaggcaacaagaggtgtttgatctcatccgtgatcacatcagccagacaggtatgccgccgacgcgtgcggaaatcgcgcagcgtttggggttccgttccccaaacgcggctgaagaacatctgaaggcgctggcacgcaaaggcgttattgaaattgtttccggcgcatcacgcgggattcgtctgttgcaggaagaggaagaagggttgccgctggtaggtcgtgtggctgccggtgaaccacttctggcgcaacagcatattgaaggtcattatcaggtcgatccttccttattcaagccgaatgctgatttcctgctgcgcgtcagcgggatgtcgatgaaagatatcggcattatggatggtgacttgctggcagtgcataaaactcaggatgtacgtaacggtcaggtcgttgtcgcacgtattgatgacgaagttaccgttaagcgcctgaaaaaacagggcaataaagtcgaactgttgccagaaaatagcgagtttaaaccaattgtcgttgaccttcgtcagcagagcttcaccattgaagggctggcggttggggttattcgcaacggcgactggctgtaacatatctctgagaccgcgatgccgcctggcgtcgcggtttgtttttcatctctcttcatcaggcttgtctgcatggcattcctcacttcatctgataaagcactctggcatctcgccttacccatgattttctccaatatcaccgttccgttgctgggactggtcgatacggcggtaattggtcatcttgatagcccggtttatttgggcggcgtggcggttggtgcaacggcgaccagctttctctttatgctgttgctgtttttacgcatgagcaccaccgggctgactgcgcaggcttatggtgccaaaaatcctcaggcattagcccgtacgctggtgcaaccgttgctgttggcgttgggggctggggcgttaattgcgctgctgcgtacgccgattatcgatctggcgctgcatattgttggcggtagtgaggcagtcctggaacaggcgcggcgctttcttgaaatccgctggttaagcgcaccggcgtcgctggcgaatctggtattactcggttggttactcggcgtgcaatatgcccgtgcgccagtaattttgttagtggtcggcaatatcctcaacattgtgctggatgtctggctggtgatggggctgcatatgaacgtgcagggcgcggcgctggcgacggttattgcggaatatgcaacattgctgattggtctgctaatggtgcgtaaaatcctcaaactacgcggaatttccggcgaaatgctgaaaactgcctggcgaggaaacttccgtcgcttgctggcgcttaaccgcgatatcatgctgcgttcgctgttgttgcaactctgtttcggcgcgatcaccgtacttggcgcgcgactggggagtgacattatcgctgttaacgcggttctgatgacgctactcacctttaccgcctatgcgctggatggttttgcctacgcggttgaagcgcactccggtcaggcatacggtgcgcgcgacggtagccagttgctggatgtctggcgggcagcgtgccgccagtcggggatcgtagcgttactgttttcggtggtttatttgctggctggggaacacatcattgcgttactgacgtcgttaacccagattcagcagctggctgaccgctatcttatctggcaggtgattttgccggtggttggcgtctggtgttatctgctggacggcatgtttataggcgcaacgcgtgccaccgaaatgcgtaacagtatggcggtggccgccgcaggttttgcgctgacgctccttacgctgccgtggctgggtaatcatgctttgtggctggcattaaccgtctttctggcgttgcgcgggctttctctggcggctatctggcggcgtcactggcgcaatggtacctggtttgccgcaacgtgacggttaaaaattctgaataaataatcctaagccaaattgctgactacacttaatctcacgttcagaagaaaagtgaacgtactctcattcacaacctaacgatgaggtcttgattatgaataaagatgaagccggcggtaactggaaacagtttaaaggtaaagtgaaagagcaatggggcaaactgaccgatgatgatatgacgatcattgaaggtaaacgtgatcaactggtcggtaaaatccaggaacgttatggttatcagaaagatcaggcagaaaaagaggtcgtggattgggaaacccgcaatgaatatcgctggtaattaatccctcctgcccgacgtgtacaaggatgtacgccctcttaacgcggtttctttttcacctgcacagagtgatcatgctggcactgttcaggatgacgacacgcttccacttctacacatgccgcacagagcccatgtgcttcaatcacattatgccgcagggcaaaccccatttttgccgccagcgtatgcataatgtcttccacgccttctgcacactcttctttcactgcgccgcagcgatcgcaaataaacatggctgacgtatgggtgggctgatcgaacagatgacagagcacataactgttggtggattccaccttatgcacaaaaccttgctcaagcagaaaatccagcgcgcgataaaccgttggcggcttggcttgcggttcagcttcgcgcagtaaatcaagcagatcataagcgctgatagcgccatcctgcagactcatcaggcgcaacacttccaggcgctgtggggtcaggcgcacattacgctgcgcgcagattttttcagcctgcgctaataactcctgcgttgtggtcttttccatcgggcacctcaaagtgggggttaagaatgtccttactttaccatgttccaggaaaaacaccgagaacccttattgttgccgtaatgttgattttctgttttgtaggtaaggtgttatgttgccttgtcgtaccattatcaacacgataataattaataattcatttttaaataaattgcttcaagttaactcgctatttatttaactgggtttaaacgcatacctgtagttcagaaattatgagcgatttttgatagtgaccagatggcaaaagaattataaggaggacacggtacgacaaaaaaggtagatgaatcatgttgaagataatacccggtgcaactggatactttaataaaacactcaattcaaatcaattcgataatgaagatgcaatcaaagataaattagataatagaggttcaatcaaaggtaaattaaataatatatatggtaaatctattgattatgcagcgctgcgtcatcgggatataattattgcaaaaatagatttgtttattcaacgaatcacgcataatttatggcatgcacgtaaaaaaatgtgtttttaattgtgcaaataaatgatctcaaaatgtgggtcaataagtatattgacgattgcactgatgaggatttaaacgatcgtgactttattgcatcagttgttgaccgggctatttttcatttcgcgattaatagtatatgtaatcctggggataataaagatgcaatgcccattgaacaatgtacttttgatgtagaaactaagaatgaccttccctccacggttcagctattttatgaggaatctaaggataatgaacctttagcgaatatacattttcaagcaataggttctggttttttaacgtttgttaatgcctgccaggaacatgatgacaacagcttaaaattatttgcttcgctgttaatttcactttcatattctagtgcctacgcagatttatcagaaacagtgtatattaatgaaaataatgagagctacctgaaagctcagtttgaaaaattatctcaacgtgatatgaagaagtacctgggagagatgaagcgtctggctgatgggggagaaatgaattttgatggctatctggataagatgtcacatctggtgaatgaaggaacgctcgatcctgatattttaagcaaaatgcgagatgctgcaccacaattaattagcttcgcgaagtcgtttgacccaacctcaaaggaagagattaaaatacttacagacacttctaaattaatttatgatttgttcggggttaaatcggagaaataatatgtgaagttcttcgatagtatggaaggcattatataaaaggacccaatatttattgggttcttttttctctatcaatactattagcagggagatatatcaccagagtttaatgtgtgattttttatttatcgtcgaacctggattgtttatcattggccttaacaaagttaacggctaataagattatttccatcacttcgtgagagcttcatgccttgagaggatctcaattttcttttgcaatgagacaggcgcttcctgttgttatggtatagtaccccgctattgagcctcctgaatagtgatgctgaataacataaccccatgatatatcgataaaataatctctacatttgaaaatgcacggtaattctgaaatgcaaaaaatcaaccaaaccagcgcaatgcctgaaaaaactgacgttcactggagtggtcggtttagcgttgcaccaatgctcgactggacggacagacattgccgctatttcttgcgtctgctttcccgcaatacgttgctgtataccgaaatggtgaccacaggggcgattattcacggtaaaggtgattatctggcgtacagtgaagaagaacatccggtagcgttgcaactgggcggtagcgatccggcggcgctggcgcagtgtgcaaagctggcagaagcgcgcggatatgatgagatcaacctgaatgtcggctgcccgtctgaccgggtgcagaacggcatgtttggtgcgtgtctgatgggtaatgcgcagctggttgccgactgcgtgaaagcgatgcgcgatgtggtgtcgattccggtgacggtgaaaacgcgtattggcatcgacgaccaggacagctatgaatttctctgcgatttcatcaataccgtttccggcaaaggcgagtgtgagatgttcatcatccacgcacgtaaagcctggctttcggggttaagcccgaaagaaaaccgtgaaatcccgccgctcgattatccgcgtgtgtatcaactgaagcgtgactttccgcatctgacaatgtcgattaacggtggtatcaagtcgctggaagaggccaaagcacacctgcaacatatggatggcgtgatggtcgggcgcgaggcgtatcagaatccgggtattctggcggcggtagaccgggagatctttggttcctcggataccgatgccgatccggtggcggtagtgcgcgccatgtatccgtacattgagcgtgaactcagccaggggacgtatctcggccatattacccggcatatgttgggcttgttccagggtattcctggcgcgcggcagtggcggcgttatttaagtgaaaatgcccataaagcgggtgcagacattaatgtgctggaacacgcgctcaaactggtggcggataagcgttaacttttcaccaaaaagtagtcaaattcaccacgccctgcgcaccgtcgcggggcgttttgctgttaaatcaatagattatttttggcatgattcttgtaatgccagcaagagatttcatatttgggagagcatcatgctggaactactttttgtgattggcttttttgtcatgctgatggtcaccggcgtttcgttgctgggcattatcgccgcgctggttgtggcgacggccattatgttcctcggcggtatgctggcattgatgattaagttgctgccgtggttactactggcgattgcggtggtgtgggttattaaggcgattaaagcaccaaaagtgccgaaatatcagcgttatgaccgctggcgttactaagggattgtgcggatgatcacaacctaaggttttatccttagaacaaaataggaattgataatcaaatctgtcactattgcgcctctaacagattcatcgtgctgtaccctacatacagccgaactataaaaagaaagggcttcccaggtggaagccctatttcttttatggaatcagcaggctggaaccttgcgtcgcccggctttccagaatctcatgcgcacgctgcgcatccttcagcggatatttctgctgctcggcgacatcgaccttaatcacaccgctggcaatcaaagagaacagttcattactggcctcggttaattcctcccgcgtggtgatatagccttgcagggaagggcgtgtcacatacaacgagcctttttgattgagaatgcctaagttcacaccggtaaccgcacctgatgagttgccaaaactgaccattaagccgcggcgttgcaggcaatccagcgaccgttcccaggtgtctctgcccacggaatcgtacaccacgcgcactttcttaccgccggtgatctcttttaaccgctcgaccagatcctcttcacgatagttaataacctgccacgcgcccgcttttagcgcgctctgcgctttttgcgcggttcctacggtgccgataagtttcgcgcccagggcttttgcccactggcaggcaattaagccaacgccgccagccgctgcgtggaacaggaactgttcatcgggtttaatttcataggttttgcgcagcagataataaaccgttaagcctttcaggaaggatgccgcagcttgctcaaaagaaattgccgcaggcagaatcgccgctttatccgcaataatgttatgcacagagctgtaagcgcctaacgccgactgcgcatagactacacgatcgcctgccttaatatgctttacaccactgccgactttactcacgatgcctgctgcttcggtgcctaatccgctgggtagcgatggcggcgggtaaaggccgctgcggatatatgtgtcgataaaattgatgccgatggctttattttcgacctggatttcattctccgccggatcggcaggagtgaactctacggcttgaagtacttccgggccaccgtgcttgtgaaattcaattcgtgttgccatgtgtcctccagaacgtatcgtcagggtctgcttcatatgataaagtttcgacccattctttatctcggtaactccattcactatggcaggaaataaacccttcaacaaacagcaggctgaaccccgcgaacgcgatccacaagttgccgggctgaaagtgcctccgcactcgatcgaagcggagcagtcggtgttgggcggtttaatgctagataacgaacgctgggatgatgtagccgagcgtgtggtagcagacgatttttacacccgcccacaccgtcatatctttactgaaatggcgcgtttgcaggaaagcggtagccctatcgatctgattactcttgcggaatcgctggaacgccaggggcaactcgatagcgtcggtggttttgcttatctggcagagctgtcaaaaaatacgccaagtgcggctaacatcagtgcctatgcggacatcgtgcgtgaacgtgccgttgtccgtgagatgatctcggttgcgaatgagattgccgaagctggttttgatccgcaggggcgtaccagcgaagatctgctggatctggctgaatcccgcgtctttaaaattgccgaaagtcgtgcgaacaaagacgaagggccgaagaacatcgccgatgtgctcgacgcaaccgtggcgcgtattgagcagttgtttcagcagccacacgatggcgttaccggggtaaacaccggttatgacgatctcaacaaaaaaaccgctggcttgcagccgtcggatttgatcatcgtcgccgcgcgtccgtcgatgggtaaaacaacatttgcgatgaacctcgtcgaaaacgcggcgatgttgcaggataaaccggtacttatcttctcgctggagatgccatcagaacagatcatgatgcgttctctggcgtcgctgtcgcgcgttgaccagactaaaatccgtaccgggcagctcgatgacgaagactgggcgcgcatttccggcaccatgggtattttgctcgaaaaacgcaatatctatatcgatgactcctccggcctgacgccaacggaagtgcgttcccgcgcacgccgtattgcccgtgaacacggcggcatcgggcttatcatgatcgactacctgcaactgatgcgcgtaccggcgctttccgataaccgtacgctggaaattgcagaaatctctcgctcgctgaaagcactggcgaaagaactgaacgtgccggtggtggcgctgtcccagttgaaccgttctctggaacaacgtgccgacaaacgcccggtcaactccgacctgcgtgaatctggctctatcgagcaggatgcggacttgatcatgtttatctatcgtgatgaggtgtatcacgaaaacagtgatttaaaaggcatcgcggaaattattatcggtaaacaacgtaacggcccaatcgggacggtacgcctgacctttaacggtcaatggtcgcgcttcgacaactatgcggggccgcagtacgacgacgaataataattattttatgaattaggtaattaaagcaaacacttatcaaggaacacaaatgcaagcggcaactgttgtgattaaccgccgcgctctgcgacacaacctgcaacgtcttcgtgaactggcccctgccagtaaaatggttgcggtggtgaaagcgaacgcttatggtcacggtcttcttgagaccgcgcgaacgctccccgatgctgacgcctttggcgtagcccgtctcgaagaagctctgcgactgcgtgcggggggaatcaccaaacctgtactgttactcgaaggcttttttgatgccagagatctgccgacgatttctgcgcaacattttcataccgccgtgcataacgaagaacagctggctgcgctggaagaggctagcctggacgagccggttaccgtctggatgaaactcgataccggtatgcaccgtctgggcgtaaggccggaacaggctgaggcgttttatcatcgcctgacccagtgcaaaaacgttcgtcagccggtgaatatcgtcagccattttgcgcgcgcggatgaaccaaaatgtggcgcaaccgagaaacaactcgctatctttaataccttttgcgaaggcaaacctggtcaacgttccattgccgcgtcgggtggcattctgctgtggccacagtcgcattttgactgggtgcgcccgggcatcattctttatggcgtctcgccgctggaagatcgctccaccggtgccgattttggctgtcagccagtgatgtcactaacctccagcctgattgccgtgcgtgagcataaagccggagagcctgttggttatggtggaacctgggtaagcgaacgtgatacccgtcttggcgtagtcgcgatgggctatggcgatggttatccgcgcgccgcgccgtccggtacgccagtgctggtgaacggtcgcgaagtaccgattgtcgggcgcgtggcgatggatatgatctgcgtagacttaggtccacaggcgcaggacaaagccggggatccggtcattttatggggcgaaggtttgcccgtagaacgtatcgctgaaatgacgaaagtaagcgcttacgaacttattacgcgcctgacttcaagggtcgcgatgaaatacgtggattaatcgttctgtaatatttgattgtctgtgccggatgcggcgtgaatgccttatccggccaataaaatcctaaaaattcaataagttgatgttctttcatgctcttataaaggtcgtgcctctggcggatgtacgtttgtcatgagtctcactctgttgctaattgccgttcgctcctgaacatccactcgatcttcgccttcttccggtttattgtgttttaaccacctgcccgtaaacctggagaaccatcgcgtgtttcaaaaagttgacgcctacgctggcgacccgattcttacgcttatggagcgttttaaagaagaccctcgcagcgacaaagtgaatttaagtatcggtctgtactacaacgaagacggaattattccacaactgcaagccgtggcggaggcggaagcgcgcctgaatgcgcagcctcatggcgcttcgctttatttaccgatggaagggcttaactgctatcgccatgccattgcgccgctgctgtttggtgcggaccatccggtactgaaacaacagcgcgtagcaaccattcaaacccttggcggctccggggcattgaaagtgggcgcggatttcctgaaacgctacttcccggaatcaggcgtctgggtcagcgatcctacctgggaaaaccacgtagcaatattcgccggggctggattcgaagtgagtacttacccctggtatgacgaagcgactaacggcgtgcgctttaatgacctgttggcgacgctgaaaacattacctgcccgcagtattgtgttgctgcatccatgttgccacaacccaacgggtgccgatctcactaatgatcagtgggatgcggtgattgaaattctcaaagcccgcgagcttattccattcctcgatattgcctatcaaggatttggtgccggtatggaagaggatgcctacgctattcgcgccattgccagcgctggattacccgctctggtgagcaattcgttctcgaaaattttctccctttacggcgagcgcgtcggcggactttctgttatgtgtgaagatgccgaagccgctggccgcgtactggggcaattgaaagcaacagttcgccgcaactactccagcccgccgaattttggtgcgcaggtggtggctgcagtgctgaatgacgaggcattgaaagccagctggctggcggaagtagaagagatgcgtactcgcattctggcaatgcgtcaggaattggtgaaggtattaagcacagagatgccagaacgcaatttcgattatctgcttaatcagcgcggcatgttcagttataccggtttaagtgccgctcaggttgaccgactacgtgaagaatttggtgtctatctcatcgccagcggtcgcatgtgtgtcgccgggttaaatacggcaaatgtacaacgtgtggcaaaggcgtttgctgcggtgatgtaatgcaggaaagcaggctggagctacccagcctgcagtgaaattaaactgtcgtcgctttcactctttctttatagatgatttttttgatgccatcgttctacgtgagagataataaacgttgttagttcttttattgttaagcttatcccaattatctggaattccttatcctgtttttttgggtggagtaataatttctgcacatctaaccattattaaatttaataataagtatcgggtttgttacgatagaatatttctatatcctcaagaatatgctttgccttattgcctgtgactttctgagattcaattatagtatcgttaaattctaatgttaaagagaactcttttttccgctttgtgtaagtttaaccttatattgattaccaatatcaaataaaaaggtcctgtaatgagaataatcacctttaacctcctcggcaaaacagcaaagcgtgcaaatatacataaagtctttcttacccctgattttgttaactaaatcaataaatgcgtgaaaaactttacttgcaatagaacttgatacttcttctccaggtctaaaaaatcttttgcaatttttaactgtgtttctatgtataaaaagaaatctttggcataagagatatctttattatttagtgcatctagctcaacaggtaaagatgtcgttttgttgctattcacatatgatatattcatatcatcatctccatcgcgagtaataaaattaatcaccattgtagggtagggggctggtcaatcagaaatcatctttataaacttcgattgtttttgtaatgctgtatcattaagttcattaaatcgtacagcagataaatgttctatcaaatttcgctcatttgccgaggattcatcataataaacgtaaaattaatgtatccttacatcgagtaataaacattttttatacaaaaaaagacaggaacgtatttactgggttaaatataatcatcctgcttttcatcacaaaaaccgcagataatccttcctttccccggcagctggcgttatggtcagatggtttttgcaacaaatctcacaataaaaagtttcaacatactgactatttagggaaaaatatgcgcaagatcacacaggcaatcagtgccgtttgcttattgttcgctctaaacagttccgctgttgccctggcctcatctccttcaccgcttaaccctgggactaacgttgccaggcttgctgaacaggcacccattcattgggtttcggtcgcacaaattgaaaatagcctcgcagggcgtccgccaatggcggtggggtttgatatcgatgacacggtacttttttccagtccgggcttctggcgcggcaaaaaaaccttctcgccagaaagcgaagattatctgaaaaatcctgtgttctgggaaaaaatgaacaatggctgggatgaattcagcattccaaaagaggtcgctcgccagctgattgatatgcatgtacgccgcggtgacgcgatcttctttgtgactggtcgtagcccgacgaaaacagaaacggtttcaaaaacgctggcggataattttcatattcctgccaccaacatgaatccggtgatctttgcgggcgataaaccagggcaaaatacaaaatcgcaatggctgcaggataaaaatatccgaattttttatggcgattctgataatgatattaccgccgcacgcgatgtcggcgctcgtggtatccgcattctgcgcgcctccaactctacctacaaacccttgccacaagcgggtgcgtttggtgaagaggtgatcgtcaattcagaatactgacagagcgggagagcgtgatgctctcccgaatgctgtttttttaatcacacctttatcctttcgctgtcttgctgcaaactgattaagagagttttatcaaggagcagcacatgtggtatcaaaagacgctcacgcttagcgccaaatctcgtgggtttcatctggtaacggatgaaattctgaatcagctggctgatatgccgcgcgttaacatcggcttactgcatctgttgctgcaacatacctccgcctctctgacacttaatgagaactgcgatcccaccgtacgccacgacatggagcgttttttcctccgcaccgttcccgacaacggaaattatgagcatgactatgagggagcagacgatatgccttctcatatcaaatcctcaatgctgggaacatcgcttgtattgccggtgcataaagggcgtattcagaccggcacctggcaaggcatttggctgggggaacatcgcatccacggcggatcgcgtcgcatcatcgcgacactacaaggggagtaaaaaatgaccatttcggagttgctacaatattgcatggcaaaaccaggcgcagaacagagcgtgcataatgactggaaagcgacgcagatcaaagtggaagatgtactgtttgcgatggtgaaagaagtagaaaatcgcccagctgtttcgctgaaaaccagcccggagctggcggagctgctacgtcagcagcacagcgatgtgcgtccaagccgccatctgaataaagcgcactggagcaccgtgtatctcgacggttcgctgccagattcgcaaatctattatctggtggatgcgtcttatcagcaggcggtgaatttactgccggaagaaaaacgtaaattgctggtgcaactctgaaaggaaaaggccgctcagaaagcggccttaacgattacagcatcggcttaaggaagcgtgccgtgtgtgatgcttcgcactccgcgacggtttctggcgtaccggagacgaggatctcgccgccaccactgccgccttctggtcccaggtcgacaatccagtcagcggttttgatcacgtcgagattgtgctcaatcaccacaatggtgttgccctgatcgcgcagtttatgcagtacgtcgagcagttgctgaatatcggcgaagtgcagaccggtggtcggctcgtcgagaatatacagcgtctgcccggtgccgcgttttgacagttcacgcgccagcttcacgcgctgggcttcaccgcctgaaagggtggttgcggactgccccagtcgaatgtacgtcaggccaacgtccatcaacgtttgcagcttacgcgccagtgcaggtacggcatcaaagaactcacgcgcctcttcgatggtcatatccagcacttcgtggatggttttgcctttgtacttaatctccagcgtttcacggttatagcgtttacctttgcactggtcgcacggcacgtagatatccggcaggaagtgcatctccactttgatcacgccatcgccctgacaggcctcgcagcgtccgccacgaacgttaaagctgaaacgtcccggcgtatagccgcgcgcacgggattccggtacgcccgcaaacagttcgcgcacaggcgtaaacacgccggtataggtcgccgggttagaacgtggagtacgaccaattgggctttggtcgatatcgatcactttatcgaaatgctccagcccctgaatatcgcgatacggtgctggttcggcgatggtcgccccattcaactggcgttgggcaatcgggaacagtgtgtcgttaatcagcgtcgatttaccggaacctgaaaccccggtgatgcaggtaaacagacccaccggcagcgtcagcgtcacgtccttcaggttgttgccgcgtgcgcctgtcagcttcagcactttttccggattcgccggaacgcgtttcttcggcacttcaatcttgcgtttgccgctcatgtactgcccggtcaacgactccggcaccgccataatcgcttccagcggaccttctgcgaccacttcaccgccgtgaacacctgcgcccgggccaatgtcgatcacatggtcagcggcgcgaattgcgtcttcgtcgtgctccaccacaatcacggtattaccgagatcgcgcagatggataagcgtacccaacaggcgctcgttatcacgctggtgcaggccgatagacggctcgtccagcacgtacataacgccaaccaggcccgcaccaatctggctcgccagacggatacgctgtgcttcaccgccagaaagcgtttctgccgagcgggaaagcgtcaggtaattcaggccgacgttaacgaggaatttcagacgatcgccgatctctttaaggattttttctgcaatcttcgcccgctgacctgcgagtttgagattgttgaagaattccatcgcatgaccaatgctcatgtcggagatagcaggcagcggcgtattctcgacatacacgtggcgcgcttcccgacgcagacgcgtcccttcgcagctggcgcacggacgattactgataaacttggctaattcttcgcgtaccgcgctggattccgtctctttatagcggcgctccatattatgcagcacgccttcgaacggatgacgacgaatggaggtatcgccacgatcgttcatgtatttgaattcaatgttttctttgccagaaccgtacaacaccactttatgcacgttcgcgctcaggctgccccacggcgcttcgacgtcgaacttatagtgatctgccagcgatttcagcatctggaaataatagaagttgcggcgatcccagccacggatcgcaccaccagccagcgacagttccggattctggatcactcgatcaggatcgaaatattgctgtacgccaaggccgtcgcaggtcgggcaggcccccgccgggttgttaaacgaaaacagtcgcggctccagttcacgcatactgtagccgcaaattgggcaggcgaagttggcggagaacagcagctcttccgctttcgggtcgtccatatccgccactaccgcggtaccaccggaaagctccagcgcggtttcaaatgactcggcaagacgttgggtaagatcgtcacgcaccttgaagcgatcaaccaccacttcaatggtatgtttcttttgcagttccagttttggcggatcggaaagatcgcagacttcgccatcaatacgagcacggatgtagccctggcttgccaggttctccagcgttttggtgtgttcgcctttgcgctctttaatgattggcgcgagtagcatcagacgcttgccttccggctgcgacagcacgttatccaccatctggctgacggtttgcgccgccagcgggacgtcgtggtccggacagcgcggctcgccaacgcgggcgaataacaaacgcaaatagtcgtggatttcggtgattgtccccaccgtagaacgcgggttatgagacgtcgatttctgctcaattgagatggcaggagaaagcccctcaatatgatcgacgtccggcttttccatcagtgacagaaactgccgcgcgtaggcggaaagggattcaacgtaacggcgctgcccttcggcatataaggtgtcgaaagcgagcgaggatttgccagaacccgaaagcccggtcacgacaatgagcttgtcgcgggggataacgaggttgatgtttttgagattatgggtgcgggcgccccgaacttcgatcttatccattcacctttcccggattaaacgcttttttgcccggtggcatggtgctaccggcgatcacaaacggttaattatgacacaaattgacctgaatgaatatacagtattggaatgcattacccggagtgttgtgtaacaatgtctggccaggtttgtttcccggaaccgaggtcacaacatagtaaaagcgctattggtaatggtacaatcgcgcgtttacacttattcagaacgatttttttcaggagacacgaacatggccagcagaggcgtaaacaaggttattctcgttggtaatctgggtcaggacccggaagtacgctacatgccaaatggtggcgcagttgccaacattacgctggctacttccgaatcctggcgtgataaagcgaccggcgagatgaaagaacagactgaatggcaccgcgttgtgctgttcggcaaactggcagaagtggcgagcgaatatctgcgtaaaggttctcaggtttatatcgaaggtcagctgcgtacccgtaaatggaccgatcaatccggtcaggatcgctacaccacagaagtcgtggtgaacgttggcggcaccatgcagatgctgggtggtcgtcagggtggtggcgctccggcaggtggcaatatcggtggtggtcagccgcagggcggttggggtcagcctcagcagccgcagggtggcaatcagttcagcggcggcgcgcagtctcgcccgcagcagtccgctccggcagcgccgtctaacgagccgccgatggactttgatgatgacattccgttctgatttgtcattaaaacaataggttatattgttttaaggtggatgattaaagcatctgccagccataaaaaagaagcctccgttatggaggcttctacgtatcaggtcaaaatcattggccattgtggcggtgtctgattcatctcttctatcatcaccgactcgatgttgtgccagatagcggtgatgtccgccattgtgatgccaagcaaccccattgcgaaccaacaggcggaaacaacgcccagaccgctgctgatcaccgcaagcccgacataatcagaccgacgaaaacggatgttgagtgtgctggccagaaacatcattacggcactaagaagttgccagcgaagaagaaccacgccagtggtgagggtagccatcaaacaattcctctgaaaagagccgatgccctggacagcgcggcgttgttcacgggaggcgtggtacactctggctatcgcggggcttgcagaacacaaaaatgaaacactctgtttgtttcattaattttgtgaactatatcacaattgattgtttgttagccatattaggccgtgacttttattgctgtacagattatgtggtttttcagtggcattaagggcatatcttcccgccgcctctgcattcctgtaggaaattaattttgaatatcaatgaattattttcatccaggtgacgattagaaaggtatcaatttcaaatcaggcaaaagtgctatttataccgtaagatttatctaaagacgtcggtacccagggttttcaccttgcaatggccgggtataaacaggcaggaaattgatagcaatgagtcatcgtgcacgacaccaattactggcgttgccgggcattatctttttagttctctttcccatcattctttcgctatggattgccttcctttgggcaaaatcagaagtgaataatcagctccgaacctttgctcaactggcactggataaatccgagctggtcattcgccaggcagatttagtgagcgatgcagctgaacgctatcaggggcaagtttgcactccagcccatcaaaagcgaatgttgaatattattcgtggctatctttatattaatgaattgatctatgcccgtgataaccattttttatgctcatcgctgatagcgcctgtaaacggctatacgattgcaccggccgattataagcgtgaacctaacgtttctatctattattaccgcgatacgccttttttctctggctataaaatgacctatatgcagcggggaaattatgtggcggttatcaaccctctcttctggagtgaagtgatgtctgatgacccgacattgcaatggggtgtgtatgatacggtgacgaaaacctttttctcgttaagcaaagaggcctcggcagcaacgttttctccgctgattcatttgaaggatttaaccgtacaaagaaatggctatttatatgcgacagtttattcgacaaaacgcccaattgcagccattgttgcgacttcatatcaacgtcttataacccatttttataatcatcttatttttgcgttgcccgccggtattttggggagtcttgttctgctattactctggctacgtattcgacaaaactatttatctcccaaacgtaaattgcaacgcgccctcgaaaaacatcaactttgtctttattaccagccaataatcgatatcaaaacagaaaaatgtatcggcgctgaagcgttgttacgttggcctggtgagcaggggcaaataatgaatccggcagagtttattccgctggcagaaaaggaggggatgatagaacagataactgattatgttattgataatgtcttccgcgatctgggcgattacctggcaacacatgcagatcgctatgtttctattaacctgtcggcctccgattttcatacgtcacggttgatagcgcgaatcaatcagaaaacagagcaatacgcggtgcgtccgcagcaaattaaatttgaagtgactgagcatgcatttcttgatgttgacaaaatgacgccgattattctggctttccgccaggcaggttacgaagtggcaattgatgattttggtattggctactctaacttgcataaccttaaatcattgaatgtcgatattttgaaaatcgacaaatcgtttgttgaaacgctgaccacccacaaaaccagtcatttgattgcggaacacatcatcgagctggcgcacagcctggggttaaaaacgatcgctgaaggcgtcgaaactgaggagcaggttaactggctgcgcaaacgcggcgtgcgctattgccagggatggttctttgcgaaggcgatgccgccgcaggtgtttatgcaatggatggagcaattacccgcgcgggagttaacgcgcgggcaataaaattacaggcggtggcgataatcgctgggagtgcgatcaaactgccgacggaaaacgcgggagaaggtctgctgcgagacataacccaggtccattgcgatatcaaaaatcggacgctcggtggtgcgcaactcaacggcggccagtaacaggcggcgttggcgaatgtaatcgccaagcgtctgatgcgtcaccgtgcggaacattcgttgcaagtaccactttgaatagcctgatttttttgcgactacatcaatgttaagcggctggtcaatatgctcgtcaatccatgcgataagatcctgaataattttctgatgggacataaatctgcctcttttcagtgttcagttcgttaattcatctgttggggagtataattcctcaagttaacttgaggtaaagcgatttatggaaaagaaattaccccgcattaaagcgctgctaacccccggcgaagtggcgaaacgcagcggtgtggcggtatcggcgctgcatttctatgaaagtaaagggttgattaccagtatccgtaacagcggcaatcagcggcgatataaacgtgatgtgttgcgatatgttgcaattatcaaaattgctcagcgtattggcattccgctggcgaccattggtgaagcgtttggcgtgttgcccgaagggcatacgttaagtgcgaaagagtggaaacagctttcgtcccaatggcgagaagagttggatcggcgcattcataccttagtggcgctgcgtgacgaactggacggatgtattggttgtggctgcctttcgcgcagtgattgcccgttgcgtaacccgggcgaccgcttaggagaagaaggtaccggcgcacgcttgctggaagatgaacaaaactaaagcgccacaagggcgctttagtttgttttccggtctttgtctttctctctatcccgctggtacacaggagggtttcccccgacgtcaacacacctcattcgagcacgtggtggaggttccggttggtgttgatgctttaattgtatgtcaccgacgtttcttcgccagtgtaaaagtatactttttaaccgcaatatttttgtcatctcagacgattttttatcgcaatcctgaacggtatacggctcgataacgctgcaatcttgcgcaccgacgataacgtttgcgcatcaattgcctggtttttcatcgtcaagacaataaaagagaaaaaagcagcaaacttcggttgaaaaagccgctatgatcgccggataatcgtttgctttttttaccacccgttttgtatgcgcggagctaaacgtttgcttttttgcgacgcagcaaattgtcgcaaacctggagcaggaagataacgtttcgctggcaggggattgtccgccacgcatcttgacgaaaattaaactctcaggggatgttttcttatgtctacgccatcagcgcgtaccggcggttcactcgacgcctggtttaaaatttcacaacgtggaagcactgtccgtcaggaagtggttgccgggttaacaacgtttctggcgatggtctactcggtcatcgtcgttccaggtatgttgggtaaagcaggcttcccgcctgcggcagttttcgttgcaacctgtctggttgccggactcggttctatcgtgatgggtctgtgggctaatctgccgttggcgattggttgcgccatctccctgacagcgtttaccgcattcagcctggtgctggggcaacatattagcgtacctgtcgcgctgggtgccgtgttcctgatgggtgtgctgtttacggtaatttctgccacgggtatccgtagctggattttgcgcaacttgcctcacggtgtggcgcacggcacggggattggtatcggtctgttcctgctgctcattgccgctaacggtgtcggtctggtgattaaaaacccgcttgatggtctgcccgttgcgctgggtgatttcgcgaccttcccggtgattatgtcactggtaggtctggcggtgatcatcggcctggaaaaactgaaagtccctggtggcattctgctgaccattatcggtatctcaattgtcggtttgatcttcgatcctaacgtccatttctccggcgttttcgccatgccttcattgagcgatgaaaacggcaattcactgattggcagcctggacattatgggcgcgctgaatcctgtagtcctgccaagcgttctggcgctggtgatgacggcagtatttgatgccaccggaactatccgtgccgtcgccggccaggcgaacctgctggataaagatgggcagatcatcgacggtgggaaagcactgaccactgactccatgagcagcgttttctctggcctggtgggtgcggctccggcagcggtatacatcgagtctgcggcgggtacggcggcgggcggtaaaaccggtttgacggctatcaccgttggcgtgctgttcctcctgattctgttcctctctccgctctcttacctcgttccggggtatgcaacggctccggcgctgatgtacgttggcctgctgatgctgagcaacgtggcgaaaatcgactttgctgattttgttgatgcgatggcgggtctggttacggctgtattcatcgtgctgacctgtaacatcgtaacaggcatcatgatcggcttcgcgactctggtgattggtcgtctggtttccggcgaatggcgcaagttgaacatcggtacggtcgttatcgccgtggcgctggtgaccttctatgcgggtggctgggctatctaatctttcatcggattctgaaaacgggtggcaatggctgcccgtttttattttctccgcacattgtgtgagcttttgcgatattctgaaaaaaatgagaattcaggcataacgtctttctcagatcataaaaaacatcgcaaacagggaacgcatggaaatcttcttcaccatactgataatgaccctcgtggtctcgctgtccggggtggtcactcgtgtcatgccctttcagatcccgcttccgcttatgcaaatcgccatcggtgcgctactggcgtggccgacgtttggtttgcatgtggagtttgatcctgaactctttttagtcttgtttatcccgccgttgctgttcgctgatggctggaaaacgccgacccgtgaatttctcgaacatggtcgagagattttcggcctcgcgctggcgctggtggtggtcaccgtggtcggcattggcttccttatttactgggtggtgccgggcattccgctgatccctgcctttgcgctggcggcggtgctttctccgaccgatgctgtggcgctctccgggattgttggcgaagggcgcatcccgaaaaaaatcatgggcattttgcagggcgaagcgttgatgaatgacgcctccggtctggtgtcgttgaagtttgccgtagcagtggcgatggggacgatgatcttcaccgtcggcggtgcgacggtcgaatttatgaaagtagccattggcggtattctcgccggttttgtggtgagctggctgtacggtcgctcgctgcgattcctcagccgctggggcggtgatgaacccgcgacgcagatcgtcctgctgttcctgctgccattcgcttcttatctgattgccgaacatattggcgtttccggcatcctcgctgcggttgccgccgggatgaccatcacccgctccggtgtgatgcgccgtgcgccgctggcaatgcgcctgcgtgcaaacagcacctgggcgatgctggaatttgtctttaacggcatggtgttcctgctgttaggtctgcagctgccgggtattctggagacgtcgctgatggcagcagaaatcgaccctaacgtcgaaatctggatgctgtttaccaatattattctgatatatgcggcgctgatgctggtccgtttcggctggctgtggacgatgaaaaagttcagcaaccgcttcctgaagaagaagccgatggagtttggttcgtggaccacacgagaaatcctgatcgcgtctttcgccggggtgcgtggggcgatcactctggccggtgtgctctctatcccgctgctcttgccggatggtaacgtcttcccggcgcgctatgagctggtgttcctggcggctggcgtcattctcttctcgctgtttgtcggcgtggtgatgttgcctattctgctacaacacattgaagtcgcggatcattcgcaacaattgaaagaggaacgtattgcgcgagcggcaacggcagaagtggcgattgtggcgatccagaaaatggaggagcgtctggcggcggataccgaagagaatatcgataaccagctgcttacggaggtcagttctcgcgtcattggtaacctgcgtcgtcgcgccgatggacgtaacgacgttgaaagttccgtgcaggaagagaaccttgagcgtcgcttccgtctggcggcattgcgttctgaacgtgctgaactttaccacctgcgcgccacacgggagatcagcaacgaaacgctgcaaaaattactgcacgatctcgatttgcttgaagcgttgctaattgaggaaaatcagtaagccgaaagcgacgtaaccaggcccgaggtaatctgaaaaaggtgcaatcttttgcacctttaacaggttagctcgggctaacattcatgattctaaaacaaataaattatctctcttttaaagtcaattcattggctgttcttcgacttaacctcaatctgcatcttgcataatatctgcagtaatcttcatagcgactgcatgaagattatcctcagtttgtgacatgccagtatgagtggcacaatcttcttcaaagaatttctgtagtgttaccaggatatcactattaatggagatattttcctcaccacggagaatggtaatacccattccctggacgctagcctcatcgaaattaacacgatagagacggatattaaacatccaggcttttgttaaaacagaacagttgaaatggcaattgcttaaattggcattattaaaattaacattagccatattagagtcggtacatataaccatttcgaggaacgtatttgttaaccgcgtaaaaaagagtttgctatcaattaagtttatattctggagggttgctttattcaggttgacacgagacagatcagcatgttcaaagttaattaaatcaagtttagagaagctaaggtcggctctaaataaattaatatatggcgctattactttataaagatttacctcagccatgtatgccatataaaaatttgaataatcaaggaaggtatttttaatattggctctattcattgttgcattgtagaattgaacatgcatagcggaacatgaatttagagttccgtcagtcatttttatctgagcgaaatttgagtcatcgagaatacaattatcaaaaagtattttttccattatggcgaaattaaaattcgttttatacatattacagtcctgaaaaatagcgttttgtagtctgcaacctgcaaaattcgaattggataaatcttcatctttaatcacgatacctttcaggctaaggtgtgaaaaatcgtaaccaccatttactgtctgtgggatttcgatagtattattatggacggtgacattatttataaaatataccaccttaattgacacttccttatctttattaaggtaaactcttctcgtaattctatcgtcacatttattatttgcatgtgaagctatatctataaaatatttatgtattttcctgtccgtttctttcgtgatttttcctgatggtaaactatcataaattcttttcattttctgaatcaagcctatcactttttcatgatcatccattttgaaaagagagagggctttattgtcaattaacgtgtttttatgatgtttgctgtaattatctgattttgttttctttgtatgtgatggacttgtgacagagtggttatcgttaatcaggcaaagagggaaaaacatattatttaaaccattatagcgcataaaatatccttataattaacaagaaagaaaaggcatattctctgcattatcattttctacgactgtcaaaaatcgctcattttttaatgagtttatttgtttaatattatgggaaaaggtgatgcatttgggagaggaagagtattccccggtcagacgaccggggaaggggagagattaatgcgcgcggccttgctcaacgccaaagccggtctgggagcggataaactgcgcgcggaacagttcacgctcacgcgcgccttccgctgagttatcggttgccgagaagaaccagatgccgaggaatgccacggtgatagagaacagcgccgggtattcatacgggaagatggctttttcgtgaccaaggatctgtacccaaatcgtcgggccgaggatcatcagtactactgcggtaatcagccccagccagccacccatcatcgcgccacgcgtggtcagtttcgaccagtacatagaaagcagaatgatcgggaagttacagctcgccgcgatggcaaacgccagccccaccataaaggcgatgttctgattctcaaacagcacgccgaggataatcgcaatcacgccgaggatcagtacggtgatttttgatacccgcagctcttcacgttcggtcgcgccttttttgaagacgttagcgtacaagtcatgcgaaaccgcggatgcgcccgccagcgtcagacccgcaaccaccgcgaggatagtggcgaaagcaaccgctgaaataaaaccgaggaacaggttgccgcccactgcattcgccaggtgaacggccgccatgttgttaccaccaatcagatggcccgccgcgtctttatattccggattcgcaccaaccagcatgatcgcgccgaagccgataataaaggtcagaatatagaagtagcccataaacccggtggcgtagaacacgctcttacgtgcttcgcgggcatcgctgactgtaaagaagcgcatcagaatgtgcggcaagcccgccgtaccaaacatcagtcccagacccagagagagcgcggagatcggatctttcaccagcccgcccggcttcatgatgtcgacacctttcgggtgtaccgccatcgcttcactgaacagattgttgaagctaaagccgacgtgtttcatcaccataaaggccataaagctggcaccgaacagcaacagcacggctttgataatttgcacccaggtggtcgccagcatgccgccgaacaggacgtacatcatcatcagcacgccgaccagcaccaccgcaatgtgatagttaaggccaaacagcagctcgatcagtttacctgcgcccaccatctgggcgataaggtaaagcgccaccaccaccagagaaccacaggccgaaagaatacgaatcggcccttgtttcagacggtaagaggccacatcggcaaaggtgtagcgccccaggttacgcagacgttcggcaatcaggaacaaaatgatcggccagcccaccaggaagcccagcgagtaaattaagccgtcatagccggaggtaaacaccagcgcggagatccccaagaatgaggcggcggacatatagtccccggcaatcgccagcccgttctggaagccagtgatattgccgcctgcggtgtagtagtcgctacgagaacgtacgcgttttgatgcccagtaggtaatgccgagcgtaaacacgacgaaaatcaggaacataataatcgcctgccagttcgttggctggcgctctacggccccgctaatagcatccgcggcgttagctgcgaaagggagtgtggcggcaagcgccgtcagaactcttttcatgatgcttgtacctcatgcaggacttcattattaagacggtcgaattcgccgttcgcccgccagatgtagataccggtgagaacaaaggagatcacaatcactccaacaccaattggaataccgcgtgtgacgctggtgttcggattcagcggcgtgcccagccagccgggcgcgaaggcgatcagtaaaataaagccgatataaactgccagcataataatcgacaggatggtggcaaaccgttgccgtttttcgactaactccctgaaatgcgcattgtcttctatccgctgataaatagtgccattcatcacagattctccagaggtaatgtagggattgttttaattcccgctcccttatgggagaaggttaacgctcgggtaacccttgccgaatgtaggccggataaggcgtttacgccgcatccggcaatcaatgcctgatgcgacgctgtcgcgtcttatcaggcctacaaaccgttaccgactcgcatcgggcaattgtgggttacgatggcatcgcgatagcctgcttctcttcaagcagcttctcgactacgccaggatcggcaagcgtcgaggtatcgcccaggttgctggtatcgcccgccgcaattttgcgcagaatacggcgcataattttgccggagcgggttttaggcagggagtcggtccagtgcagcacgtctggcgtcgccagcgggccaatctctttacgcacccagttgcggacttctgcgtacagttctggtgacggttcctccccgtgattaagcgtgacgtaggcgtagatcgcctgacctttaatattgtgcggaatacctactacggcggcttcggcaatcttcggatgcgccaccagcgccgactcaatctctgccgtccccagacggtgaccggagacgttcagcacgtcgtccacacgcccggttatccagtaatagccatcttcatcgcgacgcgcgccgtcgccgctgaaatacatatttttgaaggtggagaagtaggtctgttcaaaacgttcgtgatcgccaaacagcgtacgcgcctgacccggccaggagtcggtgattaccaggctaccttcggtggccccctccagcgggttaccttcgttatcgaccagcgccggttgcacgccgaagaacggacgtgttgccgaaccggctttcagctcggtagcgccaggcagcggggtgatcatgaaaccgccggtttcggtctgccaccaggtatcgaccaccggacatttctcgttgccgatttttttccagtaccactcccacgcttccgggttaattggctcgcccacggaaccgagaatgcgcagcgacgaacggtcggtgccttcgatcgctttatcgccttccgccatcagcgcgcggatcgccgtgggtgcggtatagagaatattgacctgatgcttgtccaccacctgcgccatacgggcaggcgtcggccagttgggtacgccttcaaacatcagcgtggtcgcaccgcaggccagcgggccgtacagcaagtaactgtgtccggtcacccagcccacatcggcggtgcaccagtagatatcacccggatgataatcaaagacatatttaaaggtcagcgccgcgtacaccagataaccgccggtagtatgcagcacaccttttggcttaccggtagaaccggaggtgtagagaataaacagcggatcttcggcgttcatctcttccgcctggtgctgatcgctcgcttgctcaaccaggtcgtgccaccacaggtcgcgcccttcctgccagtcaattttcccgccagtacgcttcagtaccaccacatgctctacgctggtgacgttcgggtttttcagcgcgtcatcaacgtttttcttcagcggaatactgcgcccggcacgcacaccttcgtcggaagtgatcaccagtcgtgagttggaatcaataatgcgcccggcaacggcttccggcgagaagccgccgaaaatcaccgaatgcaccgcgccaatgcgggcgcaggccagcatcgcaaccgcggcttccggcaccatcggcatataaatcgccaccacatcaccttttttaatgcccagctcgagcagggtattggcgaagcggcagacgtcgcggtgcagctctttatagctgatatgtttgctctggctggcgtcgtcgccttcccagatgatggcggtacgatcgccgttttcttgcagatggcggtcaaggcagtttgccgccagattcagcgtgccgtcctcgtaccatttaatggacacattaccgggggcaaaggaggtgtttttcaccttctggtaaggtttgatccagtcaagaatttttccctgttcgccccagaaggtatcaggtacgttaatagattgttgatacatcgcctcgtactgctgagggtttatcaggcaacggtctgcgatgttggcaggaatggtgtgtttgtgaatttggctcatgcttttgttctccttgtaggatgttaataatatgtggcataagcgttaaatgtaggggtattggcagttttgtttagtatttgggcgacagatcacgcaaaagtagaattgtgcaaataaacggcagggtaatttttgaaggtcagcaacaaaagttgattaattctttgaggaacatgcagttatgcatgctgttgaaaaagaggaagatactgactaactctaaagtggtattttacatgcacttacaattgattaaagacaacattcacagtgtggttatttgttacacataggggcgagcaatgtcatgacagtgtaggtgcggttactgtcgtgaaaaacaataaaaaccgccattgcaacaatggcgcaattcggatgaagcccctatgacaaggataaaaataaacgcacgccgtatcttcagcttattgattccttttttctttttcacttctgttcacgctgaacaaacggctgctcccgcaaaacctgtaactgtggaagcgaagaatgaaacctttgccccgcagcatcccgatcaatatctctcctggaaagccacctcggaacagtcagagcgtgttgacgccctggcggaagatccacggctggtgatcctgtgggcggggtatcccttctcgcgcgattacaacaagccgcgtggacatgcttttgctgtgaccgatgtgcgtgaaaccctgcgtaccggtgcgccgaaaaacgctgaagatggtccgctaccgatggcatgctggagttgtaaaagcccggatgtggcgcgtctgatccagaaagacggcgaagatggctacttccacggtaaatgggcgcgcggcggtccggaaatcgtcaacaacttaggttgtgccgattgccataacaccgcctctccagagttcgccaaaggcaaaccggagttaaccctttcccgtccgtatgcggctcgcgcgatggaagccattggtaaaccttttgagaaagccggacgtttcgaccagcaatcgatggtttgcggtcagtgccatgtggagtattacttcgacggcaaaaacaaagcggttaaattcccgtgggatgacggcatgaaagtcgaaaatatggagcagtattacgacaaaattgccttctctgactggactaactccctgtcgaaaacgccaatgctgaaagcgcagcacccggaatatgaaacctggacagcgggcattcacggtaaaaacaacgtgacctgtatcgactgccatatgccaaaagtgcagaacgccgaaggcaaactctacaccgaccataaaattggtaatccgtttgataacttcgcccagacttgtgcgaactgccatacccaggacaaagctgccttgcaaaaagtggtcgcggaacgtaagcagtcgattaacgacctgaaaatcaaggttgaagatcaactggttcacgctcacttcgaagcgaaagcagcgctggatgcaggcgcgacggaagctgaaatgaagccaattcaggacgatatccgtcatgcccagtggcgctgggatctggcgatcgcttcccacggcattcatatgcacgcaccggaagaaggtttacggatgctcggtacggcgatggataaagcggcggatgcacgcaccaaactggcgcgcctgctggcgaccaaaggcatcacccatgaaatccagatcccggatatctcaaccaaagagaaagcccagcaggccattggcctgaacatggaacaaatcaaggccgagaagcaggacttcatcaaaacggtgatcccgcagtgggaagaacaggcacgtaaaaacggtctgttaagccaataaccccgttccgcctcgcaaggggcggaaaacacaatggagtgaatatgagcgtattacgttcgttattaactgccggggtgctggcgtcgggcctgttgtggagcctgaacggaattaccgctacccctgcggcgcaggcatctgatgatcgctacgaagttacccagcagcgtaacccggatgccgcctgtctggactgtcataaaccagataccgaaggtatgcatggaaaacatgcttccgttatcaacccgaataacaaactgccggtcacctgcaccaactgtcacggccagccatcaccgcaacaccgcgaaggggtgaaagatgtgatgcgctttaacgagccgatgtacaaggttggagagcagaacagcgtctgtatgtcctgtcatctgccggaacagttgcaaaaagcgttctggccgcacgatgtccacgtaaccaaagtggcgtgcgccagctgccattccctgcatccacagcaagatacgatgcagacgttaagtgacaaaggacggattaagatttgcgtcgattgccacagcgatcagcgcaccaatccgaactttaacccggcgtctgttccgttgcttaaggagcagccatgacctggtctcgtcgccagtttctcaccggcgtcggcgtgctggcagccgtcagcggcaccgcagggcgcgtggtggcgaaaacgttgaatatcaatggggtgcgttacggcatggtgcatgacgagtcgttatgcatcggctgtaccgcctgtatggatgcttgtcgggaagtgaacaaggtgccggaaggcgtctcgcgcctgacgattattcgtagcgagccgcagggcgaatttcctgatgtgaaatatcgcttcttccgtaagtcttgccagcactgcgatcatgcgccgtgcgttgacgtctgcccgaccggtgcgtcttttcgcgatgctgccagtgggattgtcgatgttaatccggatctctgcgtcggttgtcagtactgcatcgccgcctgtccgtaccgcgtgcgctttatccatccggtcacgaagacggcggacaaatgcgatttctgccgtaagaccaatttgcaggccggtaagttgcccgcgtgcgttgaagcttgcccgaccaaggcgctgacgtttggcaatctggacgatcccaacagtgagatttcgcaactgctgcgccagaagcccacttaccgctacaagctggcgctgggaaccaaaccgaagctgtaccgcgtaccgtttaaatacggggaggtgagccaatgacgcagacttccgcatttcattttgaatcgctggtgtgggactggccgattgccatctacctgtttttgattggtatttctgctggtctggtgacgctggccgtgctgttacgtcgcttctacccgcaggcgggcggtgcagacagtacgttgctgcgcaccacgctgattgtcgggccgggcgcggtgatcctcggtctgttgatcctcgtcttccacctgacaagaccgtggaccttctggaagctgatgttccactacagttttacctcggtgatgtcgatgggggtgatgctgtttcagctctacatggtggtgctggtgctgtggctggcgaaaatctttgaacatgatttgcttgccctgcaacaacgctggttgccgaagctggggatcgtgcaaaaggttctgagcctgctgacgcccgttcatcgcggactggaaacattgatgctggtgctggcggtgttgttgggggcttataccggctttctgctgtcggcgctgaaatcgtatccgttcctcaataacccgatcctgccggtgctgttcctcttctccggcatctcgtccggtgcggcggtggcgctgatcgccatggcgatacgccaacgcagtaacccgcattccacggaagcgcagtttgtacaccgtatggaaatccctgtggtatggggtgaaatcttcctgctggtggcgttttttgtcggtctggcgctgggcgatgacggtaaagttcgtgcgctggtggcggcattaggtggcggtttctggacgtggtggttctggcttggtgtcgccgggctggggctgattgtgccaatgctgctcaaaccgtgggtcaatcgcagttccggcattcctgccgtgctggcggcgtgtggggccagtctggtcggcgtgttgatgctgcgctttttcattctctacgccggacagttgacggtggcgtaagccagaaaagaggtggtttctggacgtattccttcctgaagtcggttttctggcgttgttgttaagtctcggggtcaacgtgttgaccccgttgacggccttcgcgggagtgcggttgcgctggcctgccatgatgcgactcacttgcatcggcattctggcgcagttcgcgctcctgctgctcgcctttggcgtactgacgtattgttttctcatcagcgatttctcggtcatttatgtcgcgcaacatagctatagcctgctgtcgtgggaactcaagctggcagcggtgtggggcggccatgaaggttcgctgctgctttgggtgctgctgctttccgcctggagcgcgctgtttgcctggcattatcggcagcaaaccgatccgctatttccgctgacgttagccgttttatctctcatgctcgccgcactgctactgtttgtggtgctgtggtccgatcccttcgtgcggatatttccaccagcaatcgaaggccgcgatctcaatccgatgctgcaacatcccggtcttatctttcatccaccgctgctttaccttggctatggcggtttgatggtagcggcgagcgtggcgctggcgagtctactgcgcggcgagtttgatggtgcctgcgcccgaatttgctggcgctgggcgttacctggctggagtgcattaacggcggggatcatcctcggttcctggtgggcctactgcgaactcggctggggcggctggtggttctgggatccggtggaaaacgcctctttattaccctggctttctgccactgcgctgctgcacagtttgtccctgacacgccagcgggggattttttgccactggtcgctgttgctggcgatagttactctgatgctgtcgctgctgggcaccttaattgtccgttctggcattctggtttcggttcatgcgttcgcgctggataacgtccgcgccgtgccgttgttcagcctgtttgcactgattagccttgcgtctctggctctgtatggctggcgagcgcgggacggtggcccggcggtgcatttttcggggttatcgcgggaaatgttaatcctcgctacgctgttgctgttttgcgcagtgctactgatcgtgctggtgggaacgctttatccgatgatttacggcctgctgggctggggacgcctctccgttggcgcgccgtattttaaccgcgcgacgttaccgtttggtctgttgatgctggtggtgattgtgctggcgacgtttgtctctggcaaacgcgtgcagcttccggcgctggtagctcatgcgggcgtgctgttatttgccgctggggtcgtggtctccagcgtcagccgtcaggagatcagcctgaatttacagccgggtcagcaggtgacgctggcaggatacaccttccgttttgagtgcctcgatctacaagccaaaggcaattacaccagcgaaaaagcgatagtggcactgtttgaccatcagcaacgcattggtgaactgacgccggagcggcgtttttatgaagcacgccgtcaacaaatgatggaaccgtcaattcgctggaacggcatccatgactggtatgcggtcatgggggagaaaactgggccggatcgttacgcttttcgtttgtatgtacaaagcggtgtgcgctggatctgggggggaggattgttgatgattgcgggcgcattgttaagcggatggcgggggaagaagcgcgatgaataaagggcttctcacgctactgctgttatttacctgttttgcgcacgctcaggtcgtagacacctggcaattcgccaatccgcaacaacagcaacaggcgttaaatattgccagccagttacgttgtccgcagtgccagaatcaaaacttactggaatccaacgcgccggtggctgtcagtatgcgccatcaggtttacagcatggtggcggaggggaagaacgaagtcgaaatcattggctggatgaccgaacgctacggagattttgttcgctataacccaccgttaacgggtcagacgctggtgttatgggcgctgccagtggtgttgttactgctgatggcactgatcctctggcgagtgagggcgaagcgatgaaacagcccaaaataccggtgaaaatgctgacaacactcacgatattgatggtatttctctgtgtcggcagttatctgttaagcccaaaatggcaggcggtacgtgcggagtatcagcgtcagcgcgatccgctacatcagtttgccagccagcaaaccccggaagcgcagcttcaggcattgcaggataaaatccgcgctaatccacaaaacagcgaacagtgggcgttactgggcgagtactatctgtggcaaaacgattacagcaattcgttgctggcgtaccgtcaggcgttgcaactacgtggtgagaacgctgaactgtatgcggcgctggcgacggtgctttattaccaggccagccagcatatgaccgcccagactcgcgcaatgatcgacaaagccctcgcgctggacagtaatgaaatcaccgccctgatgctgctggcttccgatgcgtttatgcaggcgaactacgcgcaagccatcgaactatggcaaaaagtgatggatctcaactcaccgcgagttaaccgaacacagctggttgagtcgattaatatggcgaaattgttgcagcggagattggattaatcatctggtgatgaagattatgtcattgagctgcataaaaaataatcgaatgaacatatgccaaaaataatcactaatcagtattattgcagattaaacaaataaaaatctttccataacaaatggttattcattaatcctgccataaactcgcgttattatgcattaatgcagcgaaaagctctgttgttaaagggttgcgcaacataccgcgcaaatgatactgatcataagcgttaaaaaaatctacaaaccaacgcaacacaattcatgccctggcagtatgtcacgttctcgcgtttctgaacggggaacggcgctccattgaggaagtcattcatatgaaaaatataaaattcagcctggcctggcagattctgtttgctatggtgctgggcattctcctgggaagctacctgcactaccatagcgacagccgcgactggctggtcgtcaatttgctctctccggcgggtgatatcttcatccatctgattaaaatgattgttgtgccgattgtgatctccacgctggtggtgggtatcgcgggtgttggtgatgccaaacagctcgggcgtattggcgcgaaaaccattatctacttcgaggtgatcaccaccgtcgccatcattttggggatcactctggcgaacgtcttccagcccggtgccggggtggatatgtcgcagttggcgaccgtcgatatctcgaaatatcagagcactacggaagcggtacaaagcagttcccacggcattatgggcacgattttgtcgctggtgccgacgaacattgtggcgtcgatggcgaaaggcgaaatgctgccgatcatctttttctcggtgctgtttggtctggggctttcttccctgcccgcgacgcatcgtgaaccgctggtgaccgtgttccgctccatctctgaaaccatgtttaaagtgactcacatggtgatgcgttatgcaccggtgggtgtgtttgcgctgattgcggtgacggtggctaactttggtttctcgtctctgtggccactggcgaaactggtgctgctggtgcatttcgccattctgttcttcgcgctggtagtgctgggaattgtggcgcgcctgtgcgggttaagcgtctggatcctgattcgtattctgaaagatgagctgattctggcgtactccactgccagctctgaaagcgtgctgccgcgaattattgagaagatggaagcctacggagcaccggtgtcgatcaccagtttcgtggtgccgaccggttactcttttaaccttgatggttcgacgctgtatcaaagtattgccgctatcttcatcgcgcagttgtatggcattgacctgtccatctggcaggaaatcattctggtgctgacgctgatggtgacctcgaaagggattgctggcgtgcctggcgtgtcgtttgtggtgttgctggcaacgctgggtagcgtaggtattccgctggaaggtctggcgtttattgctggtgttgaccgtatcctcgacatggcgcgtactgcgctgaacgtggtgggtaatgcgctggcggtgctggtgattgccaagtgggaacacaaatttgaccgtaagaaagcgctggcttatgagcgtgaagtgctgggcaaatttgataaaactgcggatcaataattgaagattgccggggatatccacccggcaatgtgtgaatgcctgatgcgacgcttgccgcgtcttatcaggcctacgccagacagcgcaatagcctgatttagcgtgattttgtaggtcggataaggcgtttatgccgcatccgacatcaacgcctgatgcgacgcttaacgcgtcttatcaggcctacgccagacagcgcaatagcctgatttagcgtgattttgtaggtcggataaggcgtttacgccgcatccgacatcaacgcctgatgcgacgcttgccgcgtcttatcaggcctacgccagacagcgcaatagcctgatttagcgtgattttgtaggtcggataaggcgtttatgccgcatccgacatcaacgcctgatgcgacgcttaacgcgtcttatcaggcctacgccagacagcgcaatagcctgatttagcgtgattttgtaggtcggataaggcgtttacgccgcatccgacatcaatgcctgatgcgacgcttgccgcgtcttatcaggcctatcttaaccgttggttaatttttcaaactcttcacacccggtatcaaacccttccatacagctcaggttcaaccagtgcagcgccttttgcttgttcttctcgataaaaccttcttcaccgtttaagaacatcattcccgcccagtactcggaataaccggttcgggaaattgcagagctgcgtttgaaataccaggttgccttgtcatcgtcggccttaatgcccacgccgttggcgtaaatcaaaccaagcagcatttgggcatcgacggcagagtcgttctccagatcttccgaggcgttttctaacagcgaaattgcctttggataatccggtttacccgcttgagtatttaccagaatatgcgccagcgttacttcaccttctttactgcccgcttgcgccgctttctctgcaagaacttttgcttgtggatagtccagactgaccggattggtgattttgatctgcgccagcagcgcgcaggcatcagcatcaccgctgtcggcggctttctgtgcccaatattcggctttgctcaaatcgccggagctaaaccagctgtcggcaagaaaatattgtgcgcgtcggtccccggcctctgctgcctttaaatactggctgccaggctcggagtcgttggcgtgggcaaagaatgtcaaaaacaacatcaatgcgataatttttttcattttgataatacgattgggtagggagtaaccagtataaagagttcgaatggataaaaaaacagcctccgaaaggaggctgtagaaaggacggtattacgccagtgccgcttcgcgcaggcgagttttcaacttgttgtactcgtcaatcacgtactgctcggcggcgcgctgatcggcgatcggctcgacgcgaacggcgcagtatttgtactccggcgttttcgtaatcgggcttaagttttcggtaaccagctcgttacaggcaccaatccaccactggtaggtcatgtaaatcgcccctttgttcggacgatcgctgacctgcgcacgggtgataattttgcctttacgcgagtgcacccaaaccaatgcctcatcttcaatacccagacgtttggcgtcttcggtattgatttgtgcgtagccaggttcatcagccagcgccgccagtgccgcacagttaccggtcatcgaacggcaagagtagtgaccaacttcacgcaccgttgacagtaccatcgggtactcgtcggtgagtttgtcgattggcgctacccagtcgcaggtgaagaactgcgccagaccgttcggggtatcaaacttctctttaaacagataagaagtcccctgatcggcatctgaagtatcgcggcaaggccactgaatgaagcccagttcgcccattttctcgtaagtcgcaccgtagaaatccgggcacagatgacgcaactcatcccagatctcctgggtgttgttgtagtgcatcggataacccatacgggtggcgatttcactgatgatttgccagtccgttttcagatcccatttcggttcaaccgccttgaagaaacgctggaagccacggtcagccgcagtaaacacgccttcatgctcgccccacgacgttgacggtaaaataacatccgccgccgacgcggttttggtcataaagatgtcctgaacgataaccagttccagatcttcaaaggctttacgtactgccgacagctccgcgtcagtttgtagcggatcttcgcccataatgtacgcggcacgcacttcgccatgcgctgcgcggtgcggcagctcgctgatgcgatagccggtatgcgctggcaggctttccacgccccaggctttggcgaatttctcgcggttagccggatctttcacgtactggtatcccggatacgtatccggcagcgcgcccatatcgcaggcaccctgaacgttgttctgaccacgaaccgggttaacacccgcatgcggcttaccgaggttaccggtcagcatcgcgaggctggtcagagaacgcacggtttccacgccctggtagaactgggttacacccatgccccacaggatggcggcgcttttcgcctgggcatacatccgtgccgcctgacgaatctcactggcgctgacgccggtgatatcttcaaccgactccggcgtgtagccttcaacgattttacgatactcttcaaagccttctgtacgtgaagcgacgaacgctttgtcgtacagattttcttcaataatgacatggcccatcgcattcaacagcgcgatgttcgagccgtttttcagtgcaatgtgcatgtcagcaatgcgcgcggtttcaattttgcgcggatcgcagacgataattttcgccccgttacgtttagcgttaattacgtgattcgccacgattgggtgggaatccgccgggttgtacccgaaaacgaacactaaatcggtattatcaatttcgttaatagcattgctcattgcgccattaccgaccgattggtgcagacctgcaaccgatgggccgtgtcagacacgagcgcagcagtcaacgttattggtaccaataacggcgcgcgcaaatttttgcattacatagttggtttcgttacccgtaccacgcgaggagccggtcgtctggatggcatccggaccgtacttctctttgatggcgctcaggcgctcggcaacgtaattcagtgcctcatcccaggaaacaggttcgagtttgccgccacgctggcgacggatcatgggggttttcaggcgcggggtcaggatctgggtatcgttaatgaagtcccagccataataacccttcagacacagggtaccctggttggttttcccctgcgctgcctccgcccggacgattttgccgttatcgacgaccaggttgattttgcaacctgatgcgcaataggggcaaaccgtgacgacttttttcatcggtctcgctccagttaatcaaatcacgcatacgcgctctcgactacagtatgcatcttttatgccacattttatgtggggtcattccctgatattacgggcactatttattcaaaactctgacgaaaaacaggctgtcgtcagttttgacgtgacgaaacgaaataccgcgtgacagccatcacgcggcagacattttattttttctcgacgacgggacctgcctgatacccgccgcccagcgatttcatcaactgaatgctttggatcacccggcggctgtccagcatcagtaatgacatctcttcggcaagcactggcaaccgggcttcggtggcctgtaagcggctggttaagccgcgctgataggcggcctcggcagcgcgctgggtaaagcgcgtggcttccacgcgttcagcctgcatttctcgctcgtcgttgagcgtttgcagacgcgtgccgttgacggcaacgtcacgcaccgcgttcagtactgactggttgtaacgttcaatcatcatgttgctggcggcgcgcgtgccttcgagattggcattcaaccgtccaccgtcaaacagcggcaatttcagacccgggatgaagttgaactggcgactggtttttttgaataaggtatgcagatggatggagtccagaccgaaaaacgctttgatatcaaagctcggatagaacaacgcccgcgcggaatccacctgatctaatgacgcctgaacataccagcgcatggcttgcagatccgggcgtctggcgagcaactcataagagagtgtcgccggaatgccggtctggacttgcggtaatgccaccggtctgatctccggcatatcgctggctcccgcgccaatcaatgcacgcagagattctcgcgtttcggtgatttgccctttgacggcaacaatttgtttatcgaccgccagaatctgtgcccgcgcgccgtggaaaggcacttgcgcttccagaccgtgcgccactttactctggtgcgctttcaccgcgtaatcaatcacatcgtgagtttgttctaacagatcgagcatctgatagctggcctgcatactgtaataaagctgcgctacgcccgtggccagcgatagctctactgctgcggtttctgccagcgcggcattatgcgcgccaatggcggcggcaaccgctgagcgatgcacaccccacaaatcaagatccagtccggcaaacaaacctactgtggcttccgtatagtacggcccgtccatacccagtgctggcgcatccattgaataagggcttaaaaagccgttcgccgagacacgttggcggttgagcatccctaacgctgcgacctgtaattgtgaaccggcatctaacaaatcggcctgggactgcgctttttcttcccgcagtttcgcttcggcgagggtgtgtgaaccacttagcgtccgttggatcagcgcatccagctgcgggtcattgagttgtttccaccactgcgcctgcggccagccggagctggcaagatgaatatcgtcggccagtttgatttgttccggtttgagctgttgatgaggtgcagaatccttacgtaccagggcacagccggaaatcagcgtcgtgctgccgagaatgctgcacaacagcagacgtgaaagttgacgattgatcattgcgtggctccttgtgcctgttccgtggcgggcgttaatgccggggctgtccagtctggcaagcgggcgaaaagctggcagacgtgttgctcctgttttaataaggtgggcaggatggcctgagaggcgggtgtctcttcaagcgttatttgaggagaacggctgagtgcggttgccagaccggcagcgtatttctccagggcgtcggcaaactgacctgctctgtccggctgtagtgcgttatccagcgcctgcgccgagttccaggtggcatcccaggcgtgaagaagatcgcggccctgacgaataaccgtttgcgaacgttcaatcagtaatgcgcgttcttcgctgtccagttgacgctccagcgccacgcgttggcacatctcttcacaggcattaaacgccgcatgcagaccgatacgaatttgcagataagtgcgcagagccgtgacttcctgctggcgtgggatccgcattactttacttaacatacccagcgtgccagccagtttttgcggcagtgtgcgcgcttcactttcaggccagacaaaggtgtaaatcaccgcggacaccacggtaccaatgatgatacccagggcgcgatcgcgaatttccaccaggtcgtacactgggccaaaaacgttttcgagcgtggcgagcgcgaaggtgaccaccatctgtgtgccgatataagaagagcgttcagagctggtggcaatccatgcgcccaacaggaaaatcggtgccagcacaaacagcaattcgacaatattgtccagccagggcatgaccagtagcgtgaataacagcgccagaatcgcgccgcaaaaggccccgccaaaacgcagcaccatcttctggtacgacgaaccgacatttgggttagcgacgatcacgcatgtcagcatacaggtgtgaatgccttcccagtccacgccgctgtaaaaggtgtaacagatcaaacaggcgagcagcgtttttaccgcgtagcgcatatagtctggattggtaaaagcatcggcggccattgatggcggtttggctgcgggcgttggcggcgtattcgggtccatctgacccagttgtaacaacgtctggcagatattctccaggttacattcccgtgccgccatcgcttcactttcactgatccgccagtcgctttgccagcactgaccttcagcaacggcatgctgcagcttgttgatttctgaagctaatttttgtcggaattcaataattgcctgagaatcagcaaaagaggtgggatcgtagcgattcagcgtcgagtaaatgtaggttaccgttgccacgcagctttgccaccatgcgttttgagttcgccagttggcatcgtccgcgaggcaaaagacattgagtttttgtagcgccagcgcctctctttcaatccgcgtttcgggtagcggtgcgaggctgtctgtcaggtgactaatggcatcatcaagccgatcattaagcgcctgatgcatttgcgaaatggcacgactgggaaaccacagcacgccgattaacgtcatcagcaaggttggatagaggccaacaacgatacaccacagcgttaagcgcacgaccacttccggatagtcgagcatggcggggaaggtttgcccgtaaatagcgacaatggcgacggcgaaaaagaccagccccaagcgatgggtgcgcatcaaaaacatgcagcccatcaggatcggtccggcgatgatcaatcggatcaacggttcgccgtatgaccatttgtagatcaaaaacaggctgccgatctccagcaccgtggcaaccacaaacaagatcgcgacaaatttggtgtaaaacgcgttcgactgaataccgtaaaacagcactgccagcgataacgccacaaaagggatctcaaaggtcatcgagatcagaatcaccagcaggcagcctacccagagttgcacggtctgcggcacgcgacctggtcgccgctcgcttaactcttcatgaaagaacgccagcagcctgaccaccggtaatggcagggagttgagcgcgctcattattgcggctcaagattagcgactgccgaagcgccgatgcggaacatttccgggtcaggtttatcgaccatgattttgaccggaaaacgctgggcaacgcggacccagttaatagaacgagacactttcggcaggccgcccagcaccaggccgccgtcatccggtagcacgccgtagccaatcgaatccactttaccctcgaaggttttgccgctgtcactcatcaggcgaatcgttgcgggtgtacctgagcgaatatttttcagatcggtttcgcggaagttggcgatcacataccagtgacgagtgtcgattagggtaaaaatagggcgcatggcagaagcaaattgcccgacggaggttttgagggaaatgacccggccatcaaacggcgcgcgaacggtcgccatttccagatgcagtttggtcagggcaatatccgcttcgaccgccgcacgctgggcaactaatgcatccacgccgctgacggcgctggcggctgactgcgcctgtaacaatacggcattaagatccgcttctgcggcgcgctgcgccgttcttgcacggtcaacatcttccgctgagacaaaaccttctttcagtaatggctcggtgcggcgtaatgtatctgtggcctgtttcgcggcggcacgggctttttctaccgtggcattaaccgagtcggcaccaaactgttgcgcgtcaacgctacgctgggtgagcataatttgcttatccagcgccgcgagggaggcttcagctttcgccagattggcttcgtacgggcgcgggtcgatgcggaacagcaaatcgccctgtttgactgcctggttgtcggtgaccgccagttctacaatgcggccgctgacttccggtaccacatcaatggtatctgctgacgcgtaagcgtcattagttgatggcgcactgtctacgcgccagataacgaaaacaagggcaaccagcgccaacgcaaccactaacagagcagggaatttactgcgaggagcttttttcggcgtactttccatgagcgcgtctcaaatagattagaaaaatgccagccagaacagcatggcgtagagagcaaaaagggcggtataaataattccgacaaatgccagattgatatttgcccgctgaataactcgcctcgtgatgagcgtcaaaataaggctggcaatggcgcagaaaaaccagctgggataataagcgccgatcaccgggattgccggagataatgagcatcccgaaaccatgaagacgggaattatccaggctgtttttttgagttgcatcgccatgcgagagagaactgttggcatattaaatacatcctgtctgctgcgaacaatatctgtagtgaatatcaatatccattgaaggcgtcagtatggctattttcttgatgaataaaaatagctttattcagccaccgcattcataacttatatattttatttattaattggctgtatatatttttaaaataaatacttttgggggcttcagcgcccccaaaagcgagtgacattaatttggggttacgatattcacccacaaatcgaaattatccagacaggcgataatttcttccagtttcgcgccattgccaataattttggctttcttcgcttttaccagatccgccattttggcttgtccggtcagcacggcgtgcagatcttcacggctgatgtagaaagaggcgtcggcttgcggttgcagcgttttccggtagttaagcacgctatcgttcagcgtcaggttgaggttatcgccgttgctcatattgaagttcaggctgatatttttacccgcagctttcgcgctatcgaggcgaacggccataaagtcgaacagcatttcgaccgacatcccgcgaatggtgtccggggaaccggtggtgccgtggctgaacttatgcaccccttcgcgcagctctttcgcgccggtcaggtagaaaccgcgccatgtggcggactcggcctgatagcccagctgttcaaagttattcgcttgcagattcttcgcgacctggtcacccgggttggcggcaatcacctgtttcagcagttctgccgaccagcggtaatcaccttgcttgttcgcttcttgcgccaggttgatgacacgggcagaaccgcccagcgcctgcacgtaacgtttacccatctccacctgaccatacggatgcaggttagccgggttaccgtcgtaatagccaagatagaagttatacaccgcgcgggcgttgtggctgacagaaccgtaatagccgcggctggcccagttattggcaagtgcaggcggcagcttaatcatgtcgccgatttcattcatggtgtagccctggttcgccaggtgcagggtctggtcgtgaatgtacttgatggtatcgcggtatttaccaatataatcattgatatgcttattgccccagaccggccaggtgtgcggcataaacagcacttccgcgtcgttaccccacatatccagcgtttcgttcagatactcggtccacttgctggtgtcgcgggttttcgcgccgcgcagagtgtagaagttgtgcagggtatgcgtggcgttctcggcggtacacagggctttcagggccggaatatagaagtgcatttcggctggcgcttcgctacctggggtcatcaggaagtcaaactccaggccgtcgataatcatcttctcgccagttctgacgatagttttcgtcggtgcaataatgctcgggtcgcccgttgccagcgtcacgccaaggccattacccacattgccttgcgcgttgtgcggcagtaacagaccgtaagagtagagcgcacggcggctcatgatgttacccgccagcacgttttcgctgatggcttcgtccataaagcctgcaggggcaatcacctgaactttgccggatttaacatcggcttcagagataatgcctttcacgccaccatagtggtcggtgtggctgtgagtgtagataacggcaacaatcggtttttgcggacgatgctggaagtaaaggtcaagtgcggcttttgcggcaggcggcgtcaccagcgggtcgataacaataatgcctttctcgccctcaacgaacgtaatgttagagatatcctggccgcgcacctgatacattttatcggtgactttgaacaggccagaaataccgttgatttgcgactgacgccacaggctggggtttacggtttccggcgctgcggcattaatatcaaatttgtaatcgtccgcgcggtagtaaactttaccgttcgcatcacgcagaataccttcatccagcagcggggcgataaatccacgctgggcatcgtcaaaatcctgacgatcgctaaacggtaatgatttggcgtaattctgattaacctgttgggtatattgagtggcggctttcgcttcctctttcgcgttagcggtatttaccatcatgccgctggcggcagttaacgcaataacaatcctgctcaaacggaataaccgagagttattcatataaatctccatttatcatttatgtcgtaaatatgtaatccatgcaaaatacgtcatttaaagctggcgttatcataattgggaaattgcgactttaataagtggaagtgtgagcggaacgcgccattttattaggcatttgtgctgaagagggaaaattacagtaaaactatcattgcagaaaataatatgagtcgttttatgtgtttattatatatattgtacctgtcgttggcacagcgggacattgcgctactgtgccaacgttttactcatggggctttagcacagaactgtggcaaaaaacgttgatgcgccaatattgctgcaccctgagcgccattaaagtcagaagatgaggcggcaataaagcgcacgacctgatgcggcagtggacggcgcaggtacttttgggtcatggcaacgagagtctcgcgtgggaaggcgggcatatccatcacgccaccgcccaggatcaccgcatcgggatcgaacagattaatgctggtggcaatggcccgtgccgcgttttcaagcagactctggacgaaaggggcgttttccgcatggacgaaaagatcgcgcaatgggtaatttcggggctgttgttcgtaccagcgtcttagcgccattccagagcaattggtttccaggcacccaggattgccacacgcgcagtgttgggtcatatctcccagggggatatgacccagttcgcctgccacaccgtgtgcacccgtccacggcgcaccgttcatccacactgcgaaccccatccccgtaccgagataggccgccagaaccagttgttgcgtaaggcggttttctactacgtcccaggagagttgcaggttaacgtcgcgggaaaactcaaccggacaattcagcgtattttcgagcttatcggcgagatcatataaatccgccgctgttaacggcaggttaggcgtagaaataatggtgcgtttatctttactgaccagcgccggaaatcccatcaccagaccatgacagcgagcgttaaagcgcctgagttgctcgtcaatcatttcgccgatacccgacaccaggccgggagcaatgacttctgcggtccgctttttttcgcagtgtagcgtttcaccttctgctgtccgcagacaaaagcggatatgcgttgcccccatatccacgcccgctacgacgttatgctgtttttgcatgaggctgtacctcgctttttgcagccagaatctgcgcggtcataattctccatgcttcgtcgatattttccgcatgattaaacaggccggaagtgccgacgataaagacatccgcccctgccgccatcagtttttcgtaagttgcctggttgcaggaaccgtccacctcaatttcgtactccagaccttctcgttcacgccatgccttcagttcggcaagtttatccagcatttcaggaatgaacggttgtccggcaaagccgggatcgacagtcatgaccgtaattttatcggccttatggatatagtatttcatggcctcaactggcgtctccgggttaaggatcagccccactttcatgtcatgacggcggatttcatcaatcaggcggaacgcctggccgttgatggtttccggatgcagagtgatgaaatctgctcccgcacgcgccagttgagcaatgtaatcctgcggccgcgtcaccatcagatgacagtcgagcggtttagttgccagttttttaacctgacttacgaagaacggtgagagtgtcagattggggacaaagtgaccgtccatgatatcgatgtggaagtaatcggcatggctgtcgataaattcgatctgttctttaaatttcagcagatccatacacattaacgagggggagattttcatgttcaattccttacttactgataagacggtcaagggcgacagccgcgataattaatccgcccatcaccaccagttggtaataggtttgtacctgcaaaatattcagaccgttgttgatggtgccgatgatcaacccgccaatcaccacagagaaaatgcgccccttgccgccgaagaaactggtgccgccaatgatggcgctggcaatggcataggtttcaaaacccataccggcaagcggttctgcggcaccgagtcgtgcagttgagacgacgcctgccagacctgcacaaacaccggagatgataaacaccaccaggatgtggaatttcacgtcaatcccggaatagaacgccgaatttttgttgccgcccagtgcgtagatgttgcgcccgagccgcatacgcgttgtcagaaaccaaaggatgagcgcgacaattagtgagaagataacggggacaggtatcccaattacgctggcggcaaagaagttcacgaagtcaaatgagaagccgtataccgagttggcatcggagatcaccagcgtgatcccacggaaaatcgcgttggtgccaagggtgatgatgaacgggtgtagccccgtccagttgaccaggcagccgttgatcgcccccagtgcgccgccaaccagtacaccgccaatcatcgctgcgagaaacgggtcaacacctgccaacatcagtttggcggtcaccataccggaaagcgccagaatcgcgccaaccgagaggtcgataccagcgaccaggatagcgaaaaactcgcccatgccgatcaataccgtcacggagctttgaacaaaaatctgggtaatattattggtggtcagaaaatattctggtgacagcgaaccaaagatggcgacgatgatcgccaggataaaaaaggtgccgtatttatcccagaacagcgcaaagttgaacggtttcttctcgctcgcttcgctttttactcttgtggtaaagcccatgccataatctcctcttcgctcatgtcatcgcgattcgtcaggatttgcgtcagtcgtccttcgcagaacacggcgatgcggtcgcagacggtgataatttcaggtagttcagatgacaccatcaggatgacttttccgtcgtccgccagttggcgcatcactttgtaaatttcggctttcgcgccaacgtcgatgccgcgggtaggttcatcgaaaataatcacttccgggcaacagcacagccatttggagatcaggactttctgctgatttcccccggagagttcggtgatattctggtttaccgaatgacatttcagcgccagcagttcgcgttgattttcagcggtacgttgctcgtcaacttcatgaaacaagcccatcgcgcctttatagccgccgtctttcagactgcggctgatcgccatgttctgagcgatggaaaagttggggaaaaaaccgttatcccggcggctttcagtgatgtaagccatcccttttttcacggcatccaggggtgaacgtggagagatatctttgccattaagacggatttctccgccagcgcgtttatccacgccaaacagacaattcatcagttcagtacgtccggaaccgaccagtccggcaaagcctaatatttctccccggcagacgctaaatgagatatcccggaccttttttctgtcacgactggtgacgttccgcacctcaaaaaccgtttcgtgcgcaaggttgctgacattctccttcatcgcgttaaaacggttttgcagttcgcggcctaccatcagacggacgatatcgtcatttgacacatcgcttactatgccgctgcaaacgctgctgccgtctttcatcaccgtatagcggtcgcaaatacggcgaatttccgccaacttatgcgagatatagacgatggccgtaccctctttacgcaactgattcatgatcagaaacagatagtccacctctttattggtgagtgaggaggtgggttcatccatgatgatgactttggcatcgagcatcagcgttttggcaatttctagcatctgcttgtggctgatagataaattcgccactttctcatctagatcaactttcaagcccacgcgtaataacatcatggcggcgcggacacgcatttctcgccagtcgataatattgacgccacagatttttttcgtcagatgacgaccaatatataaattttccagtacggttaattcatcaataacgctgagttcctgataaataatcccgataccgagttgtgccgctaatttatgatccagcttgttatagctaatgttattaatggtaatggtgcctttggtcggctcatgtattccggataaaactttcattagcgtggatttacccgcgccattttctcctagtaatgcatgtatttcaccaggataaaccgttaaattaaccgactttaatgcgtgaaccggaccaaaggacttgccgatccccgccatcgatatatatggcgtggccataaataacctctctgcacgaaatatcgtattattgcctgatggctacatttatcaggtctacgttcaggttattttgttggccggataagacacttcattagcatcatcatccggcatcattcagttttattgagtgaccaggattgaatcgaccagtttaaattccggtgctttatccagcgggataaccttgccggatttctcagcgtcaaccatcagcttcagacccgttgcgccgatatccgccgggttctgggcaaccgtcgcggtcatttgtccggcttccaccattttgcgggcttccggaatgccatctgtaccgacgaccagcacttttcccgtttttccggcgtttgcgactgcctgagcaacacccattgccatcgtgtcattcgcgcaatagatcgctttaatattcggattacgttgcaacacgttagtggcgacatccagtgctttaatgcggtcccagtcggcaggctggctggcgacaagcttgatctggcttgcttttttgaaggcttcggtggcaccattacgacgcgcttcaccggaggcgttaccggctttaccctcaatgattgcgacttcaccaccttcagcgcccaatttgtcaataatgaacgacgcgcctttcgccccgacagcaacgttatcggtggtgacaaaagcttccacattgccgccagcttttttcagattatccatgtcgattttttcatcgagattaaccagataaatgccttttttccatgcgcgggcgacaggcatgaccagattcactgaggataatggagcgaaggcgatacctttgtaatttttattactgagatcttcaaataactgcaattgagattgaaaatcgccttctgaaggagaggcaaaaatatcaacgctgacgcccagtgtttttgcttcatcttcaatgccttttttcatatctacccaaaatgggttggagagggttttcaatacgacagcatattcggcggcagcaaaagcgctggttgacaacattaagcccacgagtgtgccgctgaaatatttcagatatttattcataataatgttctcacggtaaggggacaggtaactccgcgatggcggaattacctttttcttatttcagcgcgcctggtgagaagaaatcaacaattgcgccggttttttgcatattaatattagcttgttcaatgttgagctgggcgacagagacaaaaaaagcgtccagcaaagttagttgtaatattcttgccgaggcattacgacctaataacggcgtttccggggctggtgagcaaataatataatcggccagtttcgctatcggtgaatggtagctatgggttatacaaataatctttgccccgttcttttttgccagttctacggccgcttttacatcactggttcgcccggaatgggtcactaccagcacaacatctccttcctgtaacaacgaagcggacatcatcatgatgtgagcatcaggataggcctgacagcgtacgccaatgcgcaagaacttgtgctgtacatcagcacagatagcatttgatcctccggcaccgtacaaatcccgctgtctggcctgatagaaaaagcgggcggcacggtggatctcatcaacgttgacgatcgactgaccttccataatggtgcgtaaagtgatgttaaataccttattcaccacatcctgcggcgcttcatcaaaagccaactcggaaggcaatacctgttctgactgagaaaaataatcttccagcgcactgcgtaagttacgaaagccgctaaaccccagcagctttgataccttaactatcatcgcttcagataccgccagagcttctgcgacatctttaattgcgggtgcacaactcaggttaccgggtttgagtaaccactccacgatgcggctttcattttctgtcattccttcctgcttcattcgcaggtaaggcgctaaccctataccgttcggaagcgctgaatcaaactctgactggctcatcacgttctcttgtccttgaattgaagacgccactatatcaccacagcaagaacagaaaagatgctggcgacttcacaaaaaaataaaatttataaagtttattttattgtgaacaatggcgagtggcttaaaattttatttcatttaattagtttaaaaacatgatgttatttgtttttctggttttttagatgatagatgttgctggatggtgagtgtctttaacgctattgcgctgtcagatgtaactctgtaaaacagatcaggaaggcgtaattcatcgattttgggtgtttttaattcattaacatcacaaatgttttttgattgtgaagttttgcacggacggggaagatgaatgaaaaagattgcatttggctgtgatcatgtcggtttcattttaaaacatgaaatagtggcacatttagttgagcgtggcgttgaagtgattgataaaggaacctggtcgtcagagcgtactgattatccacattacgccagtcaagtcgcactggctgttgctggcggagaggttgatggcgggattttgatttgtggtactggcgtcggtatttcgatagcggcgaacaagtttgccggaattcgcgcggtcgtctgtagcgaaccttattccgcgcaactttcgcggcagcataacgacaccaacgtgctggcttttggttcacgagtggttggcctcgaactggcaaaaatgattgtggatgcgtggctgggcgcacagtacgaaggcggtcgtcatcaacaacgcgtggaggcgattacggcaatagagcagcggagaaattgagattcatccactacttgcatggatgagtaatgattaatgtggatagagtttctttttgaggttggctaatgaaacgctttccgctatttcttttattcaccctgctcacgctgtccaccgttccggcccaggccgatattatcgacgacaccattggcaatattcagcaggcgattaatgacgcttataaccctgaccgtgggcgagactatgaagattcgcgcgacgacggctggcagcgtgaagtgagcgacgatcggcgcagacaatatgacgaccgccgccgccagtttgaagatcgccgcaggcagctggacgatcgccagcgccagcttgatcaggagcgtcggcaactggaggatgaagagcggagaatggaagatgagtatgggcgatgaggttgggtatggagcaggcatcgcccctcaccccaatggggagagggagaaaacgagcgcaatattcaatatcgagcacaatcggtcccctcgcccctctggggagagggttagggtgagggggccagcgcgcacattccctctcatcacgccaccccaatctccatcccatcaaaccccacctcaaaccctgacggtagtgcgttttccatcagccacgcatcaaactggtggctgatatgggtcagaatcacccgtggcgagcggataacctgattcagcgcaagcacggtatttaaatcacagtgattacgcggtgcatccgcgcgcggcgggtgactgcaatccatcaccattacctgcggctgattattgcgtaaaaatttcagcgttttttccggcaagcctgcggtgtcagacagccacgccacccggctgtgtgccgtttccagcagataaccgaaggtcagttttgagtggttgagcggcaggggcgtgacctgtaacccctgcaaatcaaacaccacaaacggttccaccgtgtggctgaaatcaagcaggcccggatgtttaaacagatcgtcgcagccctgttcatccggcgggccgtaaaccgggatcggatcgccaacgccccagcgcagcggaaacagcccctggacgtgatccatatgataatgcgtcagcaaaaactgctggaacgatccgggcgaccagcgatcggcgagatcgtgcagcccggcgtcgatcagggtgattgcgtcgttaaacttcactacgccgctgcacggttggcggcgatactgcggcgagcgccgcgctctggcgcaggccgcacactcgcagccccatgccggaacgccctgtgcgccgccggtgccggtgagcgtgagggtcaggctcatgttacagcgccttggtgaagcggaagtggctctgctcgtagccttcgcgcagatagaaacggtgcgcgtcgtggcgcttcacgttggtcgaaagttcggtcatttcggccccggcctggcgggcttcttcttctgcccacgccagtaacttactgccgacgttcagaccgcgcgcctgcggcattaccaccaactcctgaatttcgccgatccagttgacatgatgcagatgaaactgcaaatgcaggccgatcatgccgacaacttcgccatcaagcagcgccagatggtagcgcatgtttgggtcgcgcagattggcgttaaaacccacgcgaaacgcgtggtggtcaaactccgcctgttttagctcacaaatcagcgcgtaaaccgcgtcggtgtcgtactgcgtggccgggcgaagctcacaagcaggcatggtgtttctccttctgatggatcagcgtcagcagcgtgtcgaccgactggcgcaggctgccgtcattgttgagcgtatggcaatcctgtggagtatagcgggcggcgcgcgccaggcgggcgttaatttcactggcgttttcacggccacggttttccaggcgctggcggaggatctccggcgaaacctgtaaacagacgggcagcagcgccgattgatagcgcgcccgcgcctgcggcagatgggcgcgtgagccgttgaccagcacgtcgaatccggcgtgcagccagagatcaatctcgacgccgacgccataatacagaccgttagcgtgccagcttaaggccaacagattttgccccgcgcgggtaaaaaactcctgctcgctcagggcgatatggttttcacttccggcgctggcatcgcgcgtgatgtagcgatgcgccaccagtaactgagtttgttcccgcaggcggagttccgccagcaggctgtctttcccggagccggacggccccattaaccaaatcagttttcccatcatcagaacacccttttaccctgacgccagacgtggtcgatatgaatatgattgtccttgcgatgcgccagcaccaggtcggcgcgtttgccctcgccaatcaccccgcgatcctggagattaagcgcctgcgctggatttttagtcaccagcttcaccgcctgcggcagcgtaaagcggttgctctggtcatcggcgacgcgaaatgccgcatcgagcaggctggcggggtagtagtcggaagagaggatatccagcaggccaagctgcgccagttcactggccgccacgttgccggagtgcgagccgccgcgcacaatattcggcgcgcccatcagcacgttcatgccatgcttgcgcgaggcttccgccgcttcgaacgtggtgggaaattcggcgatcacgctgccaagctggtgagattcagcaacgtgggcgtgggtggcgtcatcgtggctggcaagcgcaatttttcgcgcgcggcacagggcggcgatggattcgcgattcggctgcgaccagcgtgcggcgagcgccagttgctcttcttcgtactgctgcatctgcgcatcagtgagggagtatttgccctgataatattcgcgatacttctcgcggttggcgaactggcgctggcccggcgagtggtccatcagcgacaccagcgtcaccggctcgcgctgcaccagtttttcaaacagcggcagcgtggtgtgatgcggcagttcgcagcgcagatgcagacggtgctcggcgcggttgacgccgcgtttctgcgtctcttcgatggcgttgatcatcttctccagattctccagccgatcgccgccgtcgcgcacgtcgccaattgccacggcatccagtacggtggtgatgccgctcgccaccatcagcgcgtcgtggctgctcatcgccgagtgggcaggccagtcaactttcgggcgcggggtgaagaatttatccagattatcggtatgcagctcaatcagccccggcagcagccagccgccttcgccgtccatcgcctccggcaggcggctctggctttcggcaaaggcgcggatttcgccgttctgcacctccagcgaaccgcttaccacctcgttttccagcaccagcttaacgttattgataatcatgaagaggctcccattgggtgcaggcggtcggcgacgtcattacgtacagcttcgtcatggaagatgcctacgatggctgcgccacgggttttggcttcgcgaatcagttccaccaccgcggcgctgtttttggcgtccagcgaggcggtaggttcgtcaagcagcagaatggggtagtcgacgataaagccgcgggcgatgttgacgcgctgctgttcgccaccggaaaatgtcgatggtgccaggtgccacaggcgttccggcacgttcaggcgggtgagaagacgcgcggctttagcggcgcaggcttcacgcggaacgccggtatcgagcagcggctgcatcaccacttccagtgctgagatacgcgggatgacgcgcagaaactggctcacccagccgacggtggttttgcggatttccaccactttgcgcgctggcgcggtgaccaggtctacccactcgtcaccgtgtttgatctggatttgaccttcgtcgggcagatagttggcgtacagcgagcgtagcagagttgatttgccgctgccggaatggccgtggagcaccacgcattcgcccgcgttgacggtgagcgaggcgcgattgaggacgggcaggcgcacgccgttttgctggtgcaggatgaaggttttactgacgttttgtacgttaatcatttttcgcctcgtggttcgggtgtcggatgcgacgctgacgcgtcttatccgacctacggggagcgcatttgtaggccggataaggcgtttacgccgcatccggcaccggctcaattctgcaaaaccgatgacaccagcagctgtgtatacggatgatgcgggtcgtcgagcacgcggtcggttaacccactctccaccacttgcccctgcttcatcaccagcaaacggtccgccagcaggcgggcgacgcctaaatcatgggtgacaatcaccaccgcgaggttcagctccaccaccaggccgcgcagcaggtcgagcaggcgggcctgcaccgacacatccagcccgccggtcggttcatccataaacaccagcttcggatgcgtcaccaggttgcgggcaatctgcaaacgctgctgcataccgccggaaaaggtggtcggcaggtcgtcgatccggttggcgggaatctccacctcttccagccacttctgcgcggtggcacgaatatcgccgtaatgacgtgccccggtcgccatcagccgctcgccgatattgccgcctgccgacacctggcggcgcaggccgtcgagtggatgctgatgcaccacgccccattcggtacgcagcaggcgacggcggtcggcctcgctcattgcatacagcgaacggttctcgtagtgaatttccccctgctgcggcgtcaggcgcgcggagatcgacttcagcagcgtggtcttcccggagccggattccccgacaatgcccagcacttcccccggccataaatcaaaagagacatcgctaaagcctttgcccggcgcgtaaaggtgggtcaggttattgaccgaaagtaacggttgattcattggttttttgcctcgctctgttggcggcaataatcggtatcggagcagacaaacatgcggtttccggcgtcatccagcaccacttcatcaagatagctgtgggtcgatccgcagatggcgcatggctcatcccactgctgaacggtgaacgggtgatcgtcgaaatcgagactttccacgcgggtaaacggcggcaccgcatagatgcgcttctcgcgccccgcgccgaacagttgcagggcgggcatcatgtccatttttgggttatcgaatttcgggatcggcgacgggtccatcacgtagcgcccatttaccttcaccggataggcgtaggtggtggcgatatgaccgaagcgggcgatatcttcatacagtttcacctgcatcacgccgtactcttccagcgcgtgcatggtgcgggtttccgtttcgcgcggctcgataaagcgcagcggctcggggattggcacctggaagataattatctgatcttcggtcagcggcgtttcggggatgcggtgacgcgtctggataaccgtcgcatcgtccgtacgttccgtggtgtttaccccggtcacgcgcttgaagaagttgcgaatcgacacggcgttggtggtgtcatccgcgccctggtcaatcaccttcagcacgtcgctttcgccaatcacgctggcggtaagctgaatgccgccggttccccagccgtacggcatcggcatctcgcgcccgccaaacggcacctgataaccggggatcgccaccgcttttaagatggcgcggcggatcatgcgtttggtctgctcgtcgaggtaggcaaagttgtagccgctcagattagccatggttctgctcctgttgcagacgtttgagtagctccagttcggcctggaaatcgacgtagtgggggagtttgaggtgtgagacaaagcctgcggcttcgacgttgtcggcatgtgccagcacgaactcttcatcctgcgccgggcctgtcgcgtgctcgccgtactccggggcttgcagagcgcggtcgaccagcgccatcgccatcgctttgcgctcgctcatgccgaacaccagcccgtagccgcgcgtgaagtgcggcggctcacccggcgggtcgataaaaccgttaaccatttcacactcagtcatcagcagttcgccgacgttcaccgcaaatcccagctcttccggcacaatcgacacgtcgatatagccgctgcggatctcgcctgcgaacgggtgattgcgcccgtaaccgcgttgggtggagtaggccagcgccagcaaatagccttcgtcgccgcgcatcaactgctgcaaacgggaggagcgtgagcaggggtaaaccggcggcgtgcgggtgatgtcatccggctgtgcgccgctatcctcttcaaacttcgccagcccctgacgcgccagcaggctgaaaacgtgcggcgacggctgctgttcgctgtcggcggtggtcagcgtcggcgcttcgccgtttgccagcagggtaaaatcgagcaggcgatgggtgtagtcgtaggttgggccaagcagctggccgccgggaatgtctttataaacggcggagatacggcgttcgagacgcatcccggtggtgtcgagcggctcgcttaccgccagcttcgccaacgtggtgcggtaggcgcgcagcaggaaaatcgcttcaacgttatcgccgctggcctgtttcagcgccagcgccgccagttcgcggtcggcaatgccgccttcggtcatcacgcgatctaccgcgaggttaagctgctgttcaatctgggcgacgctcagttcgggcaaatcggtatcgcctcggcgtcggctctcttgcagggcgtgggcggcgtcgatcgccttctcgccccctttcacggcaacgtacatcagcacacctccacatgagtggttcgcggaatagccagcaggcgctcgccacaggtcaggatcaggtcgatgccgagcgggaacggatgcgggcgctcggtgagttcgtgcagaatgcactccggcagctgcggagcgatcattcgttcttcggcaatacccgcaccagtaaggcgcaacatgcgtccgccgctcaggctggcgacctgtaaaatcagcgtcgcacccgcttccggcgcaacggcggtgccggtggaaagggcgttgagctgttcgctggaaatcgcctcatccgtcaccgcgaaggtcgcctgttccggctggctgaccagcggcgcgttggtatgaaaacgcaggctctggttgacgatatcgttatttaatggggtagaaagccacaccggcgtgtcgttatcggccagcgtcagcagcacgctggtggtggcgatattcagcggttgccagccgcgtttgagctgatgcagggcgacaatcacgcccggctcgctcatggcctttaacaggcgacgaaaactgtgctgggcatcctgcacgggaagcataaaagcggtttccagggtcatgcgttgtctccgcgaaccatcgtaaagaagtcgacccggctggcgttcacttcggcctggcgtgcggcaatgcgtgccatacggtcagcgtccagcggggcaataagggtttctgataagttttgaaagtggcgagattgctgcatcagcgcgtcaatcagcgcgcagcgttcggcgtgctgtttatcacgcccctgcacccagctgtagccgagcgtgccgtcagtcaggcgcacggcggcgcgggtcagcgtggcgtcgccggcaaaaaaacgttcgccggtgccgcccatccgcgcctgaatctgtaccaggccagtttcagcggcgcggatcacctcatagtcggcggtgatgtttagcgcgttcaggcgtgctgccagttcagccggttggctgtgcgccagcacggacatccagtgctggcgggtcgcggtatctgcgtgcattcagtgctccatagtgaattcaatcatgtcggcgcgcgtcaggctgacggagtactccgccgggctgctttcaccgtcacggtggttaagggtgcgcacgcacagcagcggcgacatattcgggatttcaagacgctggcactctttggcctgggcgcggcgggcgctgatccgcgtctggctgcggcgcagcgcaattccggtttgctcgcgcagaaaatcgtgcagcgagccgctgtcgaagcgttgcagcgtcggccagagggtgaggtccgcgaagtagtggtcgattaaacagagcgcgacgccgttgacacgacgcagggtgcgcaggtggatgacgttctccccctcggtaatccccagtgcgtcagcgacgtggccggacgcggggcgcaataccgaaagcagtttttcgctggtgggatggctgccctgatccagcagattctggctaaaacgcgcctgggcgttgagcgggtaatcgaacgggcgcatcagcaccagcacgccgacgccctgacggcgctgtacccagcctttttccaccagttggtcgatggcgcggcgcagggtgtggcgattcacctcaaagcgcgctgccagttgctgctcggcgggaagatagtcgccgcagcggtagtgttgacgaagctcctgctcaagttttgcggctatctcttgatagcgtgttgggtagctggtcggatgtgtagacaagtgcatagatatcaatgcctcgcttatcagataaagtgcttacgcaaccgttgagagaggaaatccagcaggctgaccgtgacgatgataagcaccatcagggcgcaggtttgttggaactggaaaccgcgaatcgcttcccacagggtgacgccgatcccgcctgcgccgaccatgccgacgacggtcgccgagcggacgttggattcgaagcgatagagggagtaggagatcagcagtggcatcacctgtggcagcacgccgtagaggatctcttcgagcttgttggcaccggtggcgcgaatgccttccaccgggccgggctcaatcgcttccaccgcttcggaaagcagcttggagagcacgccggtggtgtggataaacagcgccagcacgccagcacgccagcgaacgggccgaggccgacggcgaccacgaacagcatggcgaagaccatttcgttaatggcgcggcaggcgtccatcaggcggcgaacgggctggtaaacccaccacggcaccaggttttcggcgctcatcaggccaaaggggatggagagaaccaccgccagcgcggtgccccagacggcgatttgcagcgtgacggccatttcggtgaggtaatcctgccactggctgaaatcgggcgggaagaagtcggcggcgaacgtcgccatgttgccgccgtctttgatcagcgtaagcggggccatttccgcgccctgccacgagacgaccaacacggcgagtacaacggcccagctcagaagcgagaaccagctgcgcttgggtggggcgatggtgatggtttgcatgtttggctccggtctgtaggccggataaggtgcttgcaccgcatccggcatcaacgcctgcacattgtcggatgcgacgccggggcgtcttatccgacctacgatttactgcaccgctttactcaccgaactcatcgcgcttagcgcgttgttcaggcggtccaggtcatccagctgcgcctgaatctcggtggtttttgccagcttgtcctgctcattcagtcctttattgcttttcacgccctgcatctctttaaacagcgcgagctggcgaatcggcaccagttgcaggtcgctggaagcgcggaatggcgcccagcccaggcgttccagcaccgctttttcttccggcgttttgccgtagttcataaagaagtcgtagatcttgtctttggtggtttcggaaagattcttgcgccagacgatcggatcgcctgggatcagcggcgacttccagatcaccttcagttctttcagcttctctggcgcggaggttttcagcttgtcgaggttttcggtgttgttggtggcaacatccacctgcttgttggcgacggccagcgcgttggtttcatgcccggcgttgacggtgcgcttgaagtcgctggcggagatattgtttttggcgaagacgtagtagccggggacgaggaagccagaggtggagttaggatcgccattgccaaaggtgagatctttccgcttcgccagcagatcgttcaggttgttgatcggactgtctttgttgacgatcaacacgctccagtaacccggcgatccatccgccgcgaccgtctgggcgaagacctggccattggcgcgatccaccgcttccatcgccgacagattgccgtaccaggcgatatccactttattgaagcgcatcccctggataatgcccgcgtagtccggggcaaagaaggcgttgaccttcacgcccagcttcttctccatatcctgcaagaacggcgtccattgcggtttcaggttttgctgtgattccgttgaaataatgccgaaattcaacgccttttcctgctcttcggcgtgcgccgggcttaacagggtgctgaggctgaacatgctggtgaaggccagcgaggcaattatcttagcgttcattcgttttcctcaatgatggggatgtcaggcagctttcgcgttctcttcgacgcggttaatgctgcggtagagatggtcaaaacgttcgttatcaaactgttggctgctgccgtcgtagaagacgtgcccctggcgcagggcgacgatgcgttcgcagtagcgcagggcgtaatccacctgatgcagcgtgacgaccacggtgatgccgtcgttctggttgatgtcgcgcagggtgtccatcacgatgcgcgctgattctgggtccagcgaggcgatgggttcatcggccagaatcactttcgcctgctgcatcagcgcacgggcaatcgccacacgttgctgctggccgccggagagggtggaaacgcgctgatgggcaaaatgcaccatgccaacgcgggtcagcgcctgtaacgcgcgctgtttctgctcgccggtgaaccagctaaaacaggtgcgccagaacggcgtgctgccgagcgcgccaatcagcacgttctccagtacgctcaggcggttcaccaggttgaattgttggaatatgtagccggtatgggcgcggcttttgcggatatcgcgggccaggcggccttcgcgctggactgtgcggcccagcagctcgatatggctaccgacagatttatcgccggtaatcaaaccgcttaagtgacgtaaaagggtggattttccggaacccgacggcccaagcagagccaccatttcaccgtgatgaatgttcagatcaaccgcatgcagcgcctgatgctgattgaaggttttggcgagcttctcgacacggataatcgtttgcatgatgcagcctccctaaaaaagtggctccatcgtggcggattattgtgacgatttggttaattaaaagtgactaacagatgaagagttaacgggaattcgatgacagtgcgggagggcgggcctcccggcgggttattgcgttggttgttgtttgacgacattaatcatccacggtacgccaaatttatcggtgactttgccaaagccatgcgcccagaaagtttcctgccaggccatttcgatttttccgttagcggcaagattgtcaaaccagcgttttccttcttcgacctgttgcgaatcgagcaccagcgtaaagccggagtagctggcttttcctgacggcatggcatcgctcatcatgatgtcgcttccggcaatgcgcacattggcgtgggcgatggcggtatcgggaaattgcattccggaagggcagttctcggcgctgtcctgcgctgattttggcatttcgccgaagctgattttatagagcagttccgcgcccaacgtacgttgataataggcaatcgcgtcggaacagttaccggcaaaagagaggtagggacttaacggcatgatggtgacctcagttaagagaagccagttaagtgtagttcgaaatttatacagatgagaggcggcctgataagacgcgcgagcgtcgcatcaggcagtcggcactgttgccggatgcggcgtaaacgccttatccggcctacggagggtgcgggaatttgtaggcctgataagacgcgcaagcgtcgcatcaggcagtcggcaccattgccggatgcggcgtaaacgccttatccggcctacggagggtgcgggaatttgtaggcctgataagacgcgcaagcgtcgcatcaggcagtcggcaccgttgccggatgcggcgtaaacgccttatccggcctacggatggtgcgggaatttgtaggcctgataagacgcgcaagcgtcgcatcaggcagttggcactgttgccggatgcggcgtaaacgccttatccggcctacggagggtgcgggaatttgtaggcctgataagacgcgcaagcgtcgcatcaggcagtcggcaccgttgccggatgcggcgtaaacgccttatccggcctacggagggtgcgggaatttgtaggcctgataagacgcgcaagcgtcgcatcaggcatctggcaccgttgccggatgcggcgcgagcgccttatccggcttaccgatcacaatacaatcagttctttttcacaaactcagatttcagtttcatcggaccaaaaccgtcgattttgcaatcgatgttatggtcgccttcaaccaggcggatgtttttcactttggtgccaattttcagcatcgaagagctacctttcaccttcagatctttaatgatggtaacgctgtcgccgtcagccagcagattgccgttagcatctttaacgatcagctcgtcgctttcctgtgcaggttctgcgtcgttccattcgtaggcacattccgggcagatgtacatgccgttatcttcgtaggtgtattcggagttgcattttgggcagtgtggtaatgacatgtggatttcctcaaaagtcagcagggcaaaagcgccaaaaaacggcagattgccgaaaaaggccgcaattatacacaaaatccctgagtttgtcgggggtactgctgattttagacgacgatcgttttcatttgaaaggaaacgcaaaaagaaaataatctttttgcctctatttattatttaagataatgttaatgctctacttgttctttttttaattcacatgatatttttatctttctgacgttttaaacgtatcagaagacgttatttattctgataaaaaacaacacactaaatataaaattatttcttgcagtaattataaaagccgaaaacagaactcaaaaacaatctggctaaataaaataacaaaatttgctttaaggaagaattttctatgtacacacagaccctgtatgagttaagtcaggaggctgaacgcctgttacagctttctcgccaacagttgcagttactggaaaaaatgcctctctctgtacccggagacgacgcgccacaactggctttaccctggagtcagcctaatatcgccgaacgtcacgcgatgctgaataatgagttgcgtaaaatttcccgactggaaatggtgcttgcaattgtcggtaccatgaaagcagggaaatcaaccaccattaatgccattgttggtacggaggttctgcctaatcgtaatcgcccaatgactgcgctgccgacgcttattcgccatacgcccgggcaaaaggaaccggtactgcatttttcacatgtcgcgccaatcgattgtttaattcaacaattacaacagcgcctgcgtgattgcgatattaagcatctgaccgatgtgctggaaatagataaagatatgcgtgcgcttatgcagcggatcgaaaatggcgtcgctttcgaaaaatattatctgggtgcccagcctatttttcattgtctgaaaagtttgaatgatttagtgcgactggcgaaggcgctggacgtcgattttcctttttctgcttacgccgccattgagcatattcccgtgattgaagtggagtttgtccatctagcggggctggagagttatcccggtcagttgacgttactggatacccccgggccaaatgaagccgggcaaccgcatctgcaaaaaatgcttaaccagcagctggcacgcgcctcggcggtactggcggtgctggattatacgcaactgaaatcgatctccgatgaagaggtccgtgaggcgattttggcggtggggcaatcggtgccgctgtacgtgctggtcaataagttcgatcaacaggatcgtaacagtgacgacgccgaccaggtgcgggcactgatttccgggacgctgatgaaaggctgtattacgccacagcagatatttccggtgtcgtcgatgtggggctacctggcgaatcgggcgcgctatgagttagccaacaacggtaagttaccaccgccagagcaacaacgctgggtggaagattttgcccatgccgcgcttggcaggcgctggcgtcatgccgatctggcggacctcgaacatattcgtcatgctgccgatcagttgtgggaagattcgctgttcgcccagccaattcaggcgttgcttcatgccgcttacgctaacgcctcgttgtatgctctgcgatctgccgcgcataaactgttgaattacgcgcagcaggcgcgggaatacctggattttcgtgcgcacgggttaaacgtcgcttgtgaacaattgcggcaaaatatccaccagatcgaagaaagtttgcagctattgcaactcaatcaggcgcaggtgagcggcgagattaaacatgaaatcgagctggccctgacctccgccaaccactttctgcgtcaacagcaagatgcgctgaaggtgcagttagccgccttgtttcaggatgattcggagccgttaagcgagattcgtacccgctgtgagacactgttacagacggcgcagaacaccatcagtcgcgactttacgctgcgttttgccgagcttgaatccaccctttgccgggtgttaaccgatgttattcgccccattgagcaacaagtcaaaatggaattgagcgagtcagggtttcgtcctgggtttcattttcctgtttttcacggcgtagttccccacttcaacactcgccagctgttcagtgaagtcatttcgcgccaggaagcaacggacgagcagagcacgcgtttaggcgttgtgcgtgagactttttcgcgctggttgaatcagcccgactggggacggggaaatgagaaatcaccgacagaaacggttgattacagtgtgttgcaacgagcattaagcgcagaagtcgatctctattgccaacaaatggctaaagttctggcagagcaggtcgatgaatctgttacggcaggcatgaatacttttttcgctgagttcgcttcatgtttgacggaattacagacgcgtttacgcgaaagtctggctctgcgtcaacaaaatgaatcggtggtcaggctgatgcagcagcaattgcagcagactgtgatgactcacggctggatttacaccgacgcccagctgttacgcgatgatattcaaacacttttcacggcagaacgatattgaccaagacgttacttgacggccccggtcgcgtgctggagtcggtttatccccgctttttagtggatctggcgcagggtgatgatgcccgccttccacaagcccatcagcagcagtttcgtgaacgactgatgcaggaacttctttcgcgtgtgcagcttcagacatggacgaacggcggcatgttaaatgcgccgcttagcctgcgtctgacattggtggaaaaactggcgtcgatgctggatcccggtcatctggcactgacgcagatcgcgcagcatctggcgctgctgcaaaaaatggatcaccgccagcactctgctttcccggagctcccccagcaaattgccgccttgtatgagtggttttcagcccgttgtcgctggaaggaaaaggcgttaacgcaacgaggcctactggtgcaggcaggtgatcagagcgagcaaatttttacccgctggcgtgctggggcgtataacgcctggtcgttgcctgggcgctgttttatcgttctggaggagttgcgctggggggcatttggcgatgcctgccgtctgggaagcccgcaagcggtggcgttgttgctgggtgatttgctcgagaaagcgacacaacatctggcagagagtatcaatgcggcaccgaccacgcgtcactattaccatcagtggtttgcctcttcgaccgttccgacgggcggggagcatgctgattttttaagttggctgggaaagtggaccacggcagataaacaacccgtttgctggtcagtgacccaacgctggcaaactgtcgcgctggggatgccacgactctgttcagcgcagcgtctggcgggggcaatgctcgaggaaatcttctctgtaaatttggcgtaaataatcagttacatcaatgagtcctaaacgaaatccatgtgtgaagttgatcacaaatttaaacactggtagggtaaaaaggtcattaactgcccaattcaggcgtcaactggtttgattgtacattccttaaccggagggtgtaagcaaacccgctacgcttgttacagagattgcatcctgcaattcccgctccccttttgcggccgtcgcgctgatttttctggcgtttgcggaaatgggccaactctgcgaggaaagctatgctgaaaaggaaaaaagtaaaaccgattacccttcgtgatgtcaccattattgatgacggtaaactgcgtaaagccattaccgcagcatcactgggtaatgcaatggaatggttcgattttggtgtttatggttttgttgcttacgcattaggtaaagtttttttcccgggggctgaccccagcgtgcagatggttgctgcacttgccactttctccgttccctttctgattcgaccgcttggcggactcttctttggtatgttgggcgataaatatggtcgccagaagatcctcgctatcactattgtgattatgtcgatcagtacgttctgtattggcttaataccgtcctacgacacgattggtatttgggcaccgattctgctgttgatctgtaagatggcacaaggtttctcggtcggcggtgaatataccggggcgtcgatatttgttgcggaatactcccctgaccgtaaacgtggctttatgggcagctggctggacttcggttctattgccgggtttgtgctgggtgcgggcgtggtggtgttaatttcgaccattgtcggcgaagcgaacttcctcgattggggctggcgtattccgttctttatcgctctgccgttagggattatcgggctttacctgcgccatgcgctggaagagactccggcgttccagcagcatgtcgataaactggaacagggcgaccgtgaaggtttgcaggatggcccgaaagtctcgtttaaagagattgccactaaatactggcgcagcctgttgacatgtattggtctggtaattgccaccaacgtgacttactacatgttgctgacctatatgccgagttatttgtcgcataacctgcattactccgaagaccacggggtgctgattattatcgccattatgatcggtatgctgtttgtccagccggtgatgggcttgctgagtgaccgttttggccgtcgtccgtttgtgctacttggtagtgttgccctgtttgtgttggcgatcccggcgtttattctgattaacagtaacgtcatcggcctgatttttgccgggttactgatgctggcggtgatccttaactgctttacgggcgttatggcttctaccttgccagcgatgttcccgacgcatatccgttacagcgcgctggcggcggcatttaatatttcggtgctggttgccggtctgacgccaacgctggcggcctggctggtcgaaagctcgcagaatctgatgatgcctgcctattacctgatggtagtggcggtggttggtttaatcaccggcgtaaccatgaaagagacggcaaatcgtccgttgaaaggtgcgacaccggcggcgtcagatatacaggaagcgaaggaaattctcgtcgagcattacgataatatcgagcagaaaatcgatgatattgaccacgagattgccgatttgcaggcgaaacgtacccgcctggtgcagcaacatccgcgaattgatgaataagctgaaacggatggcctgatgtgacgctgtcttatcaggccaattgaactcttaaggttcacttaatctctgacgcgcatactctcctccaggttaacggaggagagtgcaatgaaaaaccgtgtttatgaaagtttaactaccgtgttcagcgtgctggtggtcagcagctttctttatatctggtttgccacgtactgatctttcttcagccgtacccaggcccgcgtgccggaagtctcttgccggttttgcaggaaaaactgcccgtgatgcaactgtgtaatgcggctgacaatacttaaccccagaccaatcccgccataacggctgtccatacgtacaaacgctttactcaactccccgcatttactctcatcaatacctggtccttcatcttcaactgccatgaccgctccgtcatcttcttgcagcttaatcataatgttgctgccttgcgggctgtaacgatgggcgttttctaccaggtttcgcaataacatccgcagcagggttgcatcaccctgaacggtgatgtcggcggcgctctctggcaatagcagggtttgctgtcgctggtcgagcatggtactgagttcgtcatacgaggggagaatgacatcttccagcagttttacatgttgataattaccggaagaaaatgactgtccggcacgcgccagttgcagcagctgggagacgctctccatcatctgatcaagccgtgccactaacggtgctacatcaatgtgatgcgttttcgccagcagttccagatgcaaacgcacccccgccagtggcgttcgcagttcgtgcgcgacgtcagcggtaaacaacctttcgttatccagcgtgctggtcaggcgactgaccagatcgtttaacgccgaaaccaccgcttcgatttcgagggtggcgctgtgaatggcaatgggcgttaagttgtcggcggtgcgcgcttccagctctttttgcagctccgccagcgggcgggtgatgcggcgtaccgcctgatagcagataaatagcgtcaggctgaccataaagacgccggggacaatcaggctggcgaccgcctcgcggatctcacgcatgatgtggcgatcgttgttgcgattgtcgcgtagcgcctgctcaaacagctgaatctgctcggtactttcatgccatagccagaagacgctgatcagctcaaacaccaacaaaatggccccgatggtcaatatcagccgttggcgcagcgatattggtcggcgcagaaaatgcatcagattcaattagttttcctcattcgcgaccagcatatagccaaagccgcgcacggtgcggatacgggctttgcccactttgtcgcgcagattgtggatatgcacttccagggtgttggtcgagggttcattgtcccagttatagatgtcgttgtagagaatttcccgatgcaccggactgcctgctttgagcattaaccgtgacagcagagcatattctttgggcgtcagaatcaactcttcaccgcccatccatacctgacggcgacccatgttcagcgtcagattgccaacaatcagctcactttcgccctgattattatggcgtcgtagcagggcgcggatacgggcatgtaactcttccagcgcaaaaggcttcaccagatagtcgtcggcaccgacatccagcccggcgattttgtcggtcagcgtatcgcgagcggtgaggatcagtaccggcagggtatattttttctgccggatacgggcgagaaaatgcagtccatcttcgtcgggtaaccctaaatccagtaccaccaggctgtaatgacctgcctcaaggctttgttccgccatccgcgcggttgtcacgctatcgcacgcgtagccttcggtttgcgccgccagaatcagtccctgcaataacagcgtatcgtcttcaacaatcagaattttcattcactcactctcctgcaagtttgcagaatatcatccgcagcctggtaatacttcgtctcaacgccagttaatcccaatagcgtggagaataaattgtcttgtgaatagtgttgcgtttgcgcctgtttttgcaggcagttctggtcaacctgataccgtttttgataatcctccgacagccacagcagcatcggcacctgtttttggctatccggggcgatggcataaggcagaccgtgcagatagatgccattttcacctaacgattcaccgtggtcagaaagataaaccaggctggtggtaaatttatcctgatgttctttcagcagattaatcgctttatcaacaatatagtcgacgtaaaccagcgtgttgtcgtaagtgttcaccagttgctctttggtacaggtctggatctcattggtgtcgcaggttggggtaaatttcctgaactgaggcggatagcggttgtaataggtcggaccgtggctgccgatggtgtgtaagacaatcacgccatcaccttgcaggttattgatgtactcttcaagcccgtggaacagcacttcgtcatagcattcgccgttgatgcactgatcaggtagattcagcgcggtgacgttctggtgaggcacgcggtcgcaggcacctttacagccgccatcgttgtcattccacagcacgttgatgcccgctcgctgaatgatatccagcacgccttcctggtgctgtgccagctcttctttgtagtgctcacgcggcatatccgagaacatgcacggtactgaaactgccgttgccgtgccgcaagatgcggtattagggaaatagaccacgttatctttcgccagccgcgggttagtttcacgcgggtagccgttgagggagaagttctccgcccgcgaggtttcgccgacaatcaggatggtcaaatttttacgtttttcgttctgcattaacgggttgcggtgcgcgtcttcaccaattcgcaccagcggcagatttgccagtcgctgatgggagtaccatgaccagctggcaacaatgctgttagaggggcttaaggatttcaccagctctttgttattgcggaacaacgaggcgtagtctttataaaacagtgcggcgaccagcaaaatcagtagtacagaaaccagaatattggctccacggaaaagaacactgcgcagacgcgaggtggcaggtttgatttttatccagcaggcaatcagcgcagcaagcacgccgctgaatcccagcgttaataacatttgcggtgtcatcagcgcataactttctgccggagtggtatcaataatattggcaatcatcgagcggtcgatgacgatgccgtaagtcattatgaaatattgtgcagccgcgccaaccagaataaacaggcaggccagtggtcgattaagccataagaaagagcttagtgtcaggacaatattaatcacgctgaaagcgacgaccggcatcgacaagaaaaccagtacgttatgcagcgaatccagcggcagcgcctgcaacacctgtttaaaaaaggcaatattcaggcagatagagatataaaaagcggccaacaatagccaggcgagtaaattcaaagagggtctttttagtaggcgcttcaacatcacggtgtttccatcgaacaaagtgcgcatatgctcgcaaagcaaaattaagccaaccttaagttcttaaggttggcttttatgtttgctggattaaggggaattaatctttgcttattggtgcatctaagggatacgggtttttatgtagccggttgtaattcagcgcatacatggcggtgatgaccatcagggtgacaaatgaccacataacctctttcgctccggaccccaccacggcccagatgcagtagaggaaggcaatggtagtaactgccagatatgccgggcgtgctttaccaaagtgaccgtgtccgagcagcagtaacgccgcacaggtgtaaagatatggcaccagtgtaaagatgaccgagacggaagaaaccagaccgaactctttggtcgcgtttggtgaaatgctgctgagctggaagatggtcatcaaaataccgacgataatcagccccgccactggcgtacccgctttatttacacgggcaaaaatcggtgggaacagtccgtcatcggcagcggctttcgccgtttgacccgccagcaacgtccagccgcccagtgaacctaagcaacccgcagctgcgcagaaggaaacaatggccccggcggtgtcacccaacgccatccgtgcggcatcaccgaatggcgaagcagaaacgcgcagtgcggcattagggatcatccccataatcgcggtggtagaaagtacatagcaaacggcggcaatcaataccccaccaatggtggcgatagggacattgcgtttcgggtttttcaccacacctgcggcaacggaggcactttccacaccgatgaacgaccacagcgtaacgttaagggtactttgaattgcaccgaaggtgcccaggccgctgacgttccatgccgccatataggtttcaccacggaaccagaaccagccaaatacggcaatcccgacgatggggatcagcgccagcacggtggcaactgcctgcacacgggtgatcattttcggaccgacaatgttcagcaggacgaagatccacagcaccacgacgcaggtgatggttaataccaatggatctttcagaatcgggaagaagtaacttaaatatcctacgccaatgaccaccatggcgatattgccgatccagcaggccagccagtagaggacgttggtttgataaccgagaaacgggccaaagcagcggcgggcgtaagcgtaagaaccaccaggacttgggtcgaggaacgacattttggcgtataccatcgagagccccagtgcaccgataatcgtcaccaaccatccataaatggcaatcccgccagtagaggccaggtttgcaggtaacagaaaaacacctgaccccataatattccccgacaccatcagggtgacggggattaagcccactttgtgagcatcagcatccgaagacataattaaactcctgcgaaggcgagcttcgtgacaataaattacgtcatatcatacgcctgcattcgatagttgaattattatcgaccgggttatcgctgatgccgttattaatatagctcttcgttaaggttaaaaatcaggcgacagtgcgttctctgtgctgactaacataatgcagcggcgtcataccgtagaagtctttaaagacagaaataaagtacgacgtactgttgtagccgcaggactgtgatacctgagagatatttttaccgtccatcattaattcatttacggcataacgcatgcggcaggtggtgattatttggctataactggtgttttcgcttttcaactttttctttaacagacttgggctaagacataaacaactggctaccatactaagattccagtctttgtgaatatcgctttcaataatttgataaacgctgtcacttacacaattacgtaacatatacatcattaatgaaacgaattttttactgtcgagaaaacgggatagcaccgtgaataataatgcgcgtgttcgttccttttctgactcagtttctgcgggcatcatgctgtgttgcgcggcaacgcgaaagacgtctggcgtcaggcatggcagggtgagtatgggcgtagcgctacgttgccatactggtatttgcgagagatctttattcagaaaccggaggtaatctttgatgatgtcgtgactaatatgagcaaccaaagtgttgttaagagaggagacgtcgataatattattttcacaatttaataacgccatatggttagctttaaggctaataggttctttcccattcacccttatccagacatctttttcagtcaataaaacaatacaaggttggtcgctgcaaatcctcatacatgtactcctgagtgcgaataaaagaccagttctcgctaaagcaaagcgataccgggaaatggttatataattgtatgatgaatataaacatgcataaaaataacgagttttactaatagtacaaatttttatagtaatttctcatgtacatatttttttacaggataaataacaggcaaaaaaaagcgcggggtggggccgcgcaaaaagtatgacatttttgtttgcagcaatttttatgaaaacgttgccatactcaaaaggcctaaggccaggcggcgtaatgttatttaaacaattacgccttcagcggaatagtggttacgctttcacgcacataacgtggtaaataccgtcaataatttcagtcccttcagtttcgtgttcaaatccagggaaatggtggtcccaggattgcagcgagcgtaaataacttacttgcggactgtttttatcgccgaagttttcaccagacagcagcatcgggattcctggcggatacgggataactgagtttgccgcgatgcgtcctggcagattttcaatggataccagttcgacattgttgtcgacaatcgcgttgtacgcttcacgcggggtgacttccgccaccggcaggccggaataggcttcgttcaaccgtgcgccagggttgttttctttcagccaggcaaacatggtgtcacccagatcgtgaatccccatgttcgcgtaagtgtcaggatattgttcaacaagttccggcatcacctgcgccagcggtgtgttggcgtcatagtggcgtttgaaggagcaaagggtgttaaccagagttccccatttcccacgggttacgcccatagagaacaggaacataatttggaagtcagtggtgcgggtaggtacaatgccgtggcgaccaagccaggcagtgaccagcgccgccggaacaccggtttcttccagttcaccatcttcacccattcccggagcaaggatgctgactttaatcgggtcgagcatactccagttatccggaatatctttgaagccgtgccagctttcgcccggatgcattacccagcagtcctgaacggtggtcagcagtttggttggtgcgtcagcaaagtcataggttttgccggtttgtgggtcggtgacgacttctttgttccacggtttgaagaaccagctaccgtcagcggtgaactctttatatagccgcgccatcgcctgacggaaatcaaccgcttcgtcaatcacttcctgtgtcagtgacaggccgctgttgccgtccatcatcgacaccgccacgtcgttggatgcgcagatggcatacagcggggaggtggtggcatgcatcatgtaggcctggttgaagcgggagaagttaatcgccccacgaccttcacgtacatgaatataagaagcctgtgacagcgcattcagcagtttgtgggtggagtgggtggcgaaaacggtaggaccgttgtgatcgccaggttcgccgcgcatggcatagtgatcggcatagatcgggttgaaacgtgcatagccgtaccaggcttcgtcaaagtgcagacgatcggaggttttttccagcagatcctgcgcttctttagcgttataacacacgccgtcataggtgcagttggtcaccacgcagtaagacggtttttgcccggctttgtctttggtcagcgggctttcactgattttcttctgcaaggtttcaggttgcatttcctgcggatagattggcccgataatgccgtagcggttgcggcttggcaccatatagaccggtttcgcgcctgtcagcatcaaaccttgttcgatggatttatggcagttacggtcaacgaccacgacatcgttatcggtcatgcaagcctgcatgatggtgcggttagagccggaagtaccgacgactaccgaccaggagcgatcggcaccaaatacgcgtgcggcatatttttcgctttcgccaaatgcgccagtatggtcaagcaaagaaccgagggaagttcgttcgatgcccatgtcggtgcggaacagattttcaccatagtagtcatggtagaaacgtccggcgggtgttttggtaaaaccaacgccgccctggtggcctggcgctgcccaggaatattcatggatgtcactatatttcatcagcgcgctgaacagtggcggcaacagctgctggcggtagcgggtcatcgcggcaacggcgcgtccggcgataaagtcggcggtatcttccagaatccaggcgaattcatcgacaagctccagcaggtcgcgatccattgcggcgagggctttttcccgatcgcccaacaggaagaccggcacgttttgttggcgctcatgaagcttaccgatcaattgtctgacgttttgatgttcgtccggatgttccatttgatagctgaacatcaggcagtcaatggcttcgtttgaagagagaatggcaaaaccatcatcaaaggaggtggatttaatcacggtaacattttgctggcttaaagcatctgccagacgctcaacggcgttaccgacccaggtgtcttgatggagaaactcgctttcaacaattaatactttcatcattgcttacccggttatgaaggaatcttcgttgcgggcaagtatcttccggccttttcgggctgtaaagcgcgtgaaaaacaaacatttttgaaatatttagttttataaacaatacgttatgtgattattttaaattattttcactgcttattatcgacggctaaactatttttttggctgatactgatatcgtctttagccgggaaacgtctggcggcgctgttggctaagtttgcggtattgttgcggcgacatgccgacatatttgccgaacgtgctgtaaaaacgactacttgaacgaaagcctgccgtcagggcaatatcgagaatacttttatcggtatcgctcagtaacgcgcgaacgtggttgatgcgcatcgcggtaatgtactgtttcatcgtcaattgcatgacccgctggaatatccccattgcatagttggcgttaagtttgacgtgctcagccacatcgttgatggtcagcgcctgatcatagttttcggcaataaagcccagcatctggctaacataaaattgcgcatggcgcgagacgctgtttttgtgtgtgcgcgaggttttattgaccagaatcggttcccagccagagaggctaaatcgcttgagcatcaggccaatttcatcaatggcgagctggcgaatttgctcgttcggactgtttaattcctgctgccagcggcgcacttcaaacgggctaagttgctgtgtggccagtgatttgatcaccatgccgtgagtgacgtggttaatcaggtctttatccagcggccaggagagaaacagatgcatcggcagattaaaaatcgccatgctctgacaggttccggtatctgttagttggtgcggtgtacaggcccagaacagcgtgatatgaccctgattgatattcactttttcattgttgatcaggtattccacatcgccatcgaaaggcacattcacttcgacctgaccatgccagtggctggtgggcatgatatgcggtgcgcgaaactcaatctccatccgctggtattccgaatacagcgacagcgggctgcgggtctgtttttcgtcgctgctgcacataaacgtatctgtattcatggatggctctctttcctggaatatcagaattatggcaggagtgagggaggatgactgcgagtgggagcacggttttcaccctcttcccagaggggcgaggggactctccgagtatcatgaggccgaaaactctgcttttcaggtaatttattcccataaactcagatttactgctgcttcacgcaggatctgagtttatgggaatgctcaacctggaagccggaggttttctgcagattcgcctgccatgatgaagttattcaagcaagccaggagatctgcatgatgtctgcacccaaaattacatttatcggcgctggttcgacgattttcgttaaaaatattcttggtgatgtgttccatcgcgaggcgctgaaaacggcgcatattgccctgatggacattgaccccacccgcctggaagagtcgcatattgtggtgcgtaagctgatggattcagcaggggccagcggcaaaatcacctgccacacccaacagaaagaagccttagaggatgccgattttgtcgtggtggcatttcagattggcggttatgaaccttgcacggtgactgatttcgaggtctgtaagcggcatggtctggaacaaaccattgccgatacgttggggccgggcggtattatgcgcgcgctacgtaccattccgcatctgtggcaaatttgcgaggacatgacggaagtctgccccgatgccaccatgctcaactatgttaacccaatggcgatgaatacctgggcgatgtatgcccgctatccgcatatcaaacaggtcgggctgtgccattcggtgcagggaacggcggaagagttggcgcgtgacctcaatatcgacccagctacgctgcgttaccgttgcgcaggtatcaaccatatggcgttttacctggagctggagcgcaaaaccgccgacggcagttatgtgaatctctacccggaactgctggcggcttatgaagcagggcaggcaccgaagccgaatattcatggcaatactcgctgccagaatattgtgcgctacgaaatgttcaaaaagctgggctatttcgtcacggaatcgtcagaacattttgctgagtacacaccgtggtttattaagccaggtcgtgaggatttgattgagcgttataaagtaccgctggatgagtacccgaaacgctgcgtcgagcagctggcgaactggcataaagagctggaggagtataaaaaagcctcccggattgatattaaaccgtcacgggaatatgccagcacaatcatgaacgctatctggactggcgagccgagtgtgatttacggcaacgtccgtaacgatggtttgattgataacctgccacaaggatgttgcgtggaagtagcctgtctggttgatgctaatggcattcagccgaccaaagtcggtacgctaccttcgcatctggccgccctgatgcaaaccaacatcaacgtacagacgctgctgaccgaagctattcttacggaaaatcgcgaccgtgtttaccacgccgcgatgatggacccgcatactgccgccgtgctgggcattgacgaaatatatgctcttgttgacgacctgattgccgcccacggcgactggctgccaggctggttgcaccgttaaaacgcgactaaacgctactgcgccgggggatttattccggcgcacacctctgacgataccaataacagaaggcgggcgttggtaacagcgacccgataccctatgagcatttcaatgactacaaaactcagttatggatttggagcgttcgggaaggattttgcgatcggcattgtgtatatgtacctcatgtattactacaccgatgtcgtcgggctgtctgtgggtttggtcggtactttgtttctggtggcgaggatctgggatgctattaacgatccgattatgggatggattgtaaatgctacgcgatcgcgatggggtaagttcaaaccctggatcctgatcggtacgttggcaaactctgtaatcttatttctcctctttagtgcgcatctgtttgaaggtactactcagattgtctttgtttgcgtgacctacatcctctggggcatgacttacaccattatggatattcccttctggtcgctggttccaaccatcacgctcgataaacgtgagcgcgaacaactggttccttatccgcgtttttttgccagtctggcaggctttgttacggcaggtgtgacgctaccatttgttaattatgtcggcggtggcgatcggggatttggctttcagatgttcactctggtactgatcgccttttttattgtttcaaccatcatcactctgcgcaatgtgcatgaagtcttttcgtcagacaatcaaccgtctgctgaaggaagccatctgacacttaaagccatcgttgcgctaatttataaaaacgatcagctttcatgcctcttgggtatggctcttgcttataatgtagccagcaacattattaccggctttgctatctattatttctcatatgttatcggtgatgcggatttgttcccctattatctgtcgtatgcgggagctgctaacctggtgacgttagtattcttcccacgcttagttaaatcattatcccgacgcattttatgggccggagcatctattcttccggtgttaagctgtggtgttctcctgttaatggcattaatgagctatcacaacgtcgtcctcattgtgattgcgggtattttgctgaatgtgggaacggcgcttttctgggtattacaggtcatcatggtggcagatatcgttgattacggtgaatataaactgcacgtacgctgtgaaagtatcgcttactccgtgcagactatggtggtgaagggcggttcagcctttgcggcttttttcattgcggttgtgttagggatgattggctatgtaccgaatgttgaacagtctacgcaagccctattaggtatgcagtttattatgattgctctaccaactctgtttttcatggtaacgctgattctctacttccgtttctatcgcctcaatggtgacacgctgcgcaggatccagatccatctgctggataaatatcgcaaagtaccgcccgagcctgttcatgctgatattccggtcggtgcagtgagtgatgtgaaagcctgacgtggacaatagctaacgaaaatggcctgatgcgatatgtttatcaggccacgtcttaatgtaatgctttggatttgcaaattttgtagaccggataaggaattcacgccgcatccggcatcaacaaagcgcaagttgttatccggttatcaagccaaagcgccgtagctggcggcaatgaaagcgagcgaggaatatcaccgtcgttaatgcgccaagcagcgcgcagaacatatcggattgcgtgtcccactggtcgccctgggtgccgagaaaatcatccgctccctgacccattgccagcgctgcccaccactcgattaattcatacatcgcgcttatcgccagcgccacgcagcagaccaggaacgccaccattttacgtccgcgcacgtacatcccgcgaacgagaatttctcgtgccaccagtgcaggcaccagcccctggaaaaagtgccccagcttgtcatacggattacgactcaaccccagccattcctgcacctcaaaaccaacggggactttcgcgtaggtgtattgtccgccgaccatcaggatgatggcgtgaaggaaaatgagcgtatagagcagcggcgttaacggataacgtctggcggtggcaagcagtagctgcacgacaataatcaccggtgtcacttccatcagccaggtgagtttgtcatgggccgaaatgccggtataaatcaggattaacgttagcgtcagtgcgctggtgttaagaattaacggcttgagtgtgcgggtcatggtgagttcgcaaatcagggaaaatactgactattcaccagcaagcgtgaaattacaatcgcaaaagaggtggccagggggatcacctggcagcatgctgccaggcgctgggccgaagaggttacttagtgcagttcgcgcactgtttgttgacgatttgctggaagaagtcgttacctttgtcatcgaccaggataaacgccgggaaatcttctacttcgattttccagatagcttccatacccagctccggataagcgacgcactccagatgcttgatgctctgctgcgccagtaccgccgccggaccgccgatgctaccgaggtagaagccgccgtgtttatgacacgcgtcggtaacctgctgactgcggttacctttcgccagcatgatcatgctgccgccgtgggattgcagcagatccacgtaggagtccatacggcctgcggtggttgggccaagtgaacctgatggataaccggcaggggttttcgccggacccgcgtagtagatcgggtgatctttgatgtactgcggaagttctttaccggcgtcaatcagctctttcagcttggcgtgtgcaatatctcggcccacgataatggtgccggtgagcgacaaacgagtggataccgggtattgcgaaagctgggcgaggatctctttcatcgggcggttaaggtcaactttcaccgcttcgccttcaccggcctggcgcagttcttgtggaatgtactggcctgggttgtgttccagtttttcgatccagataccttcgcggttgattttcgctttaatgttacggtcagcggagcaggagacgcccatgccgaccgggcaggatgcgccgtgacgtggcagacggataacgcgaatgtcgtgcgcgaagtatttaccgccaaactgcgcgccaagaccgagtttctgggcctcttccagcagttcctgttccagctggacatcgcggaacgcctgaccatgttcgttcccttccgtcggcagttcatcgtaatagtgagcgcttgctaacttgacggttttcaggttggtttccgcagacgtaccgccaatcacaaacgcgatatggtacggcgggcaggctgcagtaccgagggtacgcattttctcgacgaggaagtttttcagtttgccgggagtcagcagggctttggtttcctggtagagatacgttttgttggcagagccgccgcctttcgcaacgcaaaggaatttgtactcatcgccatctaccgcgtacaggtcgatttgcgcaggcaggttagtgccggtgttgacctctttgtacatgtccagcgccgcattctgtgaatagcgcaggttatcttcgatataggtgttatagacgcctttcgacagcgtttcttcatcaccgccgccggtccacacgcgctggccttttttaccgacgatgatcgcggtgccggtatcctggcaggtcggcagcacgcctttggcggcgatttcggagtttcttaagaattgcagcgccacgtacttgtcgttttcgctggcttctggatcgtgaagaatagccgcaacctgtttctggtgtgccgggcggagcataaaagaagcgtcgtgaaaggcttgctgcgccagcagggtcagggcttctggttccactttcaggatggtttcgccgtcgaagtcggcaacgctaacgtaatcggaagtgagtagatagtattcggtattgtctttccccatcgggaaaggtgcctggtagataaagggtttgtttgacatagcttccagcctgtaactctgtatttgttattcgaaaatggcgtgccgcgtagtcacgggcggcacgcaaagtgcatttataagaacccgtacatcgcggcgaagatccagccgaagacgcacgatacgctcacaccaatcaaccccggcagaataaagctgtggttgatgacgaagcgaccgatgtgggtggtgccggaacggtcaaactgaatcgctgccagatcgctcggataagtcggcaggatgtaataaccgtagcaagccggtgctgaagccacgatgtatgccggatcaacgccgatcgccagcgcgaccggaacaatcgccgccagcgccgcagcctgagagtttacaaacttggaaaccagcagcagaacaatggcataggcccacggatactctttcaccatttcacccagtacgccctgaatttcagacatatgcgcaccgaacatggtttctgccatccatgcgataccgtacaccgccacgatggcgatcataccggaacggaagacttcgttttttgagatagacgcgggattggttttggtcaggataataatcagcgccccggtcagcagcataaacatctgaataaccagtaccatcgacagcggtttgccgccgaaggatggacgcaggtccgaatcagcaccaagaagggcgactacagcgattgccccgaggaaaatccacattgccagccagttgcttttcggcagttttttatccagcagcgtcgcggtatcaccgtaaacatactcacggttttccggtacggagatgaatttctggaactcttcgtctttatccagatctttaccgcggaaccagctgaagataccgatcgccaggataccgattaacgtcgatggaatggtgattgccagcagatcgaggaactcaagatggcgaccatcaaaggtgacattacccagcatcgcaaccagagacacgaccgcaaccgacaccggactggcgataatccccatctgtgcaccgatagaacttgccgccatcggacgttccggacggatgttgttcttaatggcgacgtcgtagatgatcggcagaatggtgtaaaccacatgacccgtaccgcaaagaatggtcagtgtacaggtcacaaacggcgcgacaattgagacatatttcgggttgcggcgcagcagcttctcggcaatttgcagcatgacatcaagaccgcccgaagcttgcaaggtcgccgatgccgccaccaccgcaatgataaccagcatgacatcaactggtggtttacctggctgaaggtggaagacgaagaccagaatgaccagaccgataccgcctaataaacccagcgcgataccaccctttctggcaccataaaacagacatatcagtattatgataagttggatagtaaataacatgtgtgaaccctcgcgataatcctatttaaatttttgctgaatagatcacagtcacgttctgttttgtatgaactgttttcagagcctgactaaatatccgtttggtcgttaccggctttagcaaatacctcacagtgaatattggctgattaaagcagcggcaaatttatgcactgtgataagcggctttttcagagagaaagactctctggcgatgggtttatagtttgtactgcgcagatgttaatgttttgtttgctgttatcttattgatatttatcggtctattttttgttctcagggcagatgtcattaggtttatagattaatctgatctacccatttgtgggtaaaaatacacataatgcgggtgacataatagttaattaacttttgttagcgttttgaaattaaaaacaccgttcacctgaagagatattaatttttagcgatgatggagggataattatatttgatctggcacaagttttactgatgaaggatgtaacttgtgccaggggtattttgcattacggtaataattattacttacagataaccagcgatccgttattggcaatattgtttcagtagtgagtagtgttctgcctgaatacggtaacggtaaactggacgccccgtgacgccataatggatactggtgaacaagatgtggcagttgaccagccagatgaggtatttacggcaggaaacacgcgaaatgttaacctcgttggctagctcgtcggttgaaaattcatagtcctgatgcgcgtcaatccactggcacagtgtgcgtaacgtctgcggcgttaagccttttggcaagcgacgaggatcctgttcgttggagctgctgccgtggattagctgatcaagctcggcctggtcataatactgatgtttttccagcgccattttcttttgccgccagccggtgagcgcctcttcaaagcgggaagcctggaagggtttgatcaggtaatccacgacaccgtaatgcagcgaatctttaatggttgccgcatcggctgcggaggagatgacaatcacatcacttttgcaacgcgcgttatgcaggacaggcagtaaatcgagcccgttctctttttgcatatagatatcgagcaatatcaggtcgataggcgtatcgctattgaagataatctctttggctttctccagcgtcgaggctgttccacagcattgaaagcctgggatttgtgctacgtatcggcgattcagctccgcgaccattgcgtcgtcatcgataattaatacattgatcatctgttcgacctctccccgtcccagggtatctggacaaaaaattgtgtgaaaatcccgggttccgattccacggcgatgctgccgccgagattttctacctgttgtttgacaagtgctaaaccgacgcctcgctcgcttccttttgtcgagacacctttgtcaaaaatgtgatcgattttatcgggtgcgatccccggtccatcatcattaacttcacagtgcagccagccgtgacggtagtgcaatgttacgctaatttcgcctccgggttccggccctaatgcctccagcgcgttttctatcagatttcccaacgtggtaatcagcgtcgcgacctggtcctcactgccgctgtctggcagctggctttcactgtttaaaatcagcgtatggcctaaatcggtcgcgcggttaatcttgctgattaaaaaaccagcgataaccggagatttgatcttacccagcagagagccaatctcttcctgatagttattggctgttttgagaatgtaatcttccaactgcttataactcttcagatgcaataatccgagaatcacatgcaatttattcataaattcgtgggatcgttcacgaagtgcgtcagcatagttgaccagaccgtcgagtcgctgcatcagtttacgtacttcagttttgtccctgaaggttgaaatggcaccgatgataacgccattactgcgcaccggaacggtgttgatcagtaatagccggtctttaatcgtaatctcttcgtcgcggcgcggggtaccgtcgcgtaacacttccgagacatctaccacctgtgaccatgagtggcttagcgtcgacagtttctcatcgtcctgcgacttacggtaattcagcaattcttgtgcggcatcgttgatcagcgtgacctcgccgcgatcgtccacggcaacgacgccttctttgatagactgcaacatggcctggcgttgctcaaacagcgtggagatttcgtagggttccaggccgaaaaggatttttttcagtaccttaaccagaatgcaggtgccaatcagtccgaccagcatgccaaataataccgaccagataatgctccagcgactgtcattgatctgttgggtcacacggcttaactcaaggccgatcgccaccacgccaatttgtttatgattttcatcgtagatgggggtaaatacgcgtaaagcctgcgccagaaaaccgcgattgatagcgacattttcttcgccattcagcgctttaaggatgtcatcacctttaaatggctgaccaatacgctgggcttcaggatgcgagtagcgaagactttgcatatcggtaacgacaataaacagcagatcgttgcgtttgcgtacggcttccgcgatggcctggatgccactctcctgcggttttttctgcaagccctgacggatttccggcgagtcggcgagggtacgcgccactgccagtgccttgttggctagcccatctcgcgtcatatcactgatttgcgagaagtaaatcagatgcaccaccaatagcaccgagaacagtaccgcactgaccattaagatcactgtggtactcaatttcatcggacgtttgcgtaacatgcggtagggcaatgaatgtctcatcagcttccttgtgtgacaaatttcttaagcattatctctgatgaggcgggtaattcaaagggagtaagaatgattggctatataggggaagagactctggcaacggaaactgccagtgctgtatgaagattccggggctatgcttatagcgataatcatactgatgagagagggaaggtcatggatcaggcgctactggacgggggttatcgctgttataccggcgaaaagatcgatgtctatttcaacactgcgatatgtcagcattctggcaattgcgtacgtggcaacggcaagttatttaatctcaaacgaaagccgtggatcatgccggatgaagtcgacgtcgccactgtggttaaagtgattgatacgtgcccgagcggcgcgctgaaataccgtcataaataagcgagggtaaaatggaaatacgcgaaggccacaataaattttacattaatgacaaacaaggcaagcaaatcgctgaaattgtctttgtgccgaccggagagaatttagcgattatcgaacataccgatgtcgatgaaagcctgaaagggcaagggattggtaaacagctggttgcgaaagtcgtggaaaaaatgcgtcgggaaaaacgaaaaattatcccattatgcccatttgcgaaacatgaatttgataaaacgcgggagtatgatgatattcgcagttgatgggagagtacagagtcacgatatttttcattctctccgcgatgtgatgcaggagagcatctgaagggtagggggatgcacaaagaatgggcagagagcgcgtttttttgtcccaagtcatcccctttactgagcaaaaaaaagaatatctcctatatgagaatcatcaatcggggttaataagttttgcgtccccagagcgtttaatattgataggagtcatattatggaaggtaaaaacaagttcaatacttatgttgtttcttttgattatccatcatcttattcctcagtgttcttaagattaagatcattgatgtatgatatgaatttctcctctatcgtggctgatgaatatgggataccacgacaattgaatgaaaactccttcgcaataacgacatcgttagccgcaagtgaaatcgaagatttaatcaggctcaaatgcttagacttaccggatattgattttgacctcaacattatgacagttgatgactatttccgtcagttttacaagtagccaggaaggataagaagaacataaaaaatggcactattctctaaaatattaattttttatgtgattggtgtgaacatatcctttgtcattatctggtttatctcacatgagaaaacacatattcgtttacttagtgcattcctggtcggaataacctggccaatgagtctgcctgtggcattacttttttctctcttttaggagctgtagttgagtggacccgctggttatcgtgaaacgaagcgtctctcctcaaaactggatttgcggaacgatgaacgaagcagtcgcctgactgcttcgttcattaaagtgaaatttatttctgtgggcgcatcgccgggaagagaataacgtcgcgaatagtatggctgttagtaaacagcataatcattcggtcgataccaatacccagaccagcggttggcggcagaccatattccagcgcagtcacgtaatcttcgtcatagaacatggcttcgtcgtcacctgcagctttagcattaacctgttcctggaaacgttcagcctgatcttctgcgtcgtttaattcgctaaaaccattaccgatttcacgaccaccgatgaagaattcaaaacggtcggtgatttccgggttaacatcattacggcgtgccagcggggacacttctgccggatattccgtaataaaggttggctgaatcagatgtgcttctgccacttcatcaaagatctctgtgacaatacgtcccaacccccagcttttctctaccgtaataccgatagattcagctaatgctttagcagcatcaaaattatccaggtcggccatatcggtttctggacgatattttttgattgcttcgcgcatggtgagtttttcaaacggtttgccgaaatcaaacacatgctcgccataagtgactttagtggtacccagaacctcttgtgccagggtgcggaacagtgactctgtcagttcaatcaaatcgtggtaatccgcatacgccatgtagagttccatcattgtgaactcaggattatggcgaacagaaataccttcattacggaagttacggttgatttcgaatacccgttcaaaaccgcctacaaccagacgtttcagatacagctccggcgcgatacgcagatacatatctaaatccagagcattatgatgggtaataaacgggcgagcagatgccccacctggaattacctgcatcatcggggtttctacttccataaagccgcgcgcgaccatgaattgacggatagcggccagaatttttgaacggacaacaaacgtttgacgggatttatcgttagcgatgaggtccagataacgttgacgataacggacttcctgatcctgcagaccatggaatttatctggtaaaggacgtagtgctttagtcagcaggcgcagctcagtacagtgaatggaaagctcacccgtttgcgtcttaaacagcgtaccgcgggcaccgataatgtcacccagatcccattttttaaactgatcgttataaacaccttctggcaggctatctcttgcaacgtacagttgaatacggccaccgacatcctgcaacgttacaaaggaggctttccccatgatacgacgggtcatcattcggccagcaaccgagacttcaatgtttaaggattccagttcctggttatccttcgcatcaaactcttcgtgcaactggtcagaggtatggtcgcggcgaaaatcattgggaaacgccacaccttgctgacgtagtgccgccagtttttcgcggcgatttctcagttcatcgttaaaatcaatagcctcattggctccccgtgtttcttgttcagacattttggttcctctaaatccagctttcaatttagcgtagataaagagacagatcggtacactgtattatctgcctcgactattagtaactcagtttatcttatcgaaactaacgcttacctcaagttgatatcactaataaataaccatcaaaatggtttaaatgacttattaatctcgatttgttagtgttataaactgaaagttaatttattcataaccaattgtttttacgacagttaatcgttgctctcctgtatcatattcgtcggcgtgctaaacagaaaacgggtagcaaaggccaatacgacgatgatcgcgacacaagccaacgtccactctcccatctgagaaaagaatcgctggtaagctgcaattgccataccgctaatttgcgactctgtcgtctgctgtgccacgacgcctgccagccagttggcgaccgcgcctgttgccagcatataaatcccggttaatacgccagacattttcagacgcgtgatttgcgcaatcgccaccgggtcaataaagagttcggcaaagcccattagcgccagcccggatatcatcacgcccattgacgcttgaccgtcagccgctgcatgtcgggcatcaaatgccaacaacataaagccacaagccatcagcagtaagccaaaggcaaacttcagccagacgcgcaatgttgagttgccgcggctttctggcgacgccagccaggccagtacaaccccagcgagcatcaccgcaattgcattcaccgactggaatagtgctgtaggtacttcaatattgaatgcctgacgattcacaaagcgatcgataaacaagctgatggtactgccgccctgttgtgccagtacccagaacaatgtcccgacaaacatcaacaatacaatttgccaaagagcacggcgatgttcggggaatttgatcatcatgcgggcaatgatttgtgcggcaatgaggcaaacgatcgccagcaaatatccggaccagtcgttctccagcagcagagtaaaaaatactggggctaaacagagcatcaccactaaccagctccatactggtaaggcaaatttgacactagtgagcgcttttttatccatactacgtgtggactggaaatgacgatgaccgcttaagaaaatcaacaaaccgataaacatgccgccacccgcaagggcaaagccaacatgccatccataccactgagcagccaggccgcaggcgattggggctgcgatagaaccgatattgcccgcagcatacagcagcgaaaaaccgccatcacgtcgatgatcgttctcgtcgtagagctcgccaagcaaacagctgatgtttgatttgaataaaccgtagccacaaataatgattgccagcgccagatacaggctaaaggttgaatttgtatcaatacccagcaccacatggccaagggtcattaacagcgcgccggcaatcactgcagtgcggttgccgagcaggcggtcggcaagccagccgccgagaataggggtaacgtaaaccagagaagcatatgcgctgaacaggctgatggcatggttatcatcaaaaccaagctgatgggtgagatagagaatgagtaaggcacgcatgccgtaaaaactgaagtactcccagatttggatcgccacgatatagtatatcgcgcgcggctgtgagggtgttttcatgtgttctccttatgagcaaaaaagggaagtggcaagccacttcccttgtacgagctaattattttttgctttcttctttcaataccttaacggtatagcggccatcagcctgacggtatgcaccgtgaatatcggtttcaaagcccggatagtgagcgccgatttcacacagcatctgcaggaactccagaaccggacggctttcttcggtgatcatttcacccggcattaccagaggaactcccggcgggtacggaaggatcatattggcgttaatacgacctaccatttcgtcgaggtaaacttcttcggtcataccgtgcagctctttctggaatgcagcatacggagtcattaccatcgtcggcagcacttcaaatgcgcgatacatcagatccggcagattgtggtgaacaatcagtttgtggatattctgagccagttcctgaatacgcatgttttcatagaattcaggatcttcacgatacagagacggcagcatgtttttcacacgcaggttcaggtcgaacgcacgtttaaagtcagtcagagcacgcagcaggctcagtgctttggtcttatcgataccgatgctgaacaggaacagcaggttatacggaccggttttctcaacaacgatgccatgttcgtcgaggtatttcgccacgatgctggccggaataccaaagtcgctcatggtgccgtctttttccatccccggagtcagcagggtgactttgatcgggtcaagatacatgtgctcgttatcgatgtttttgaagccgtgccaggtgctgtcagaacgcagcggccagcattcagtcgtatcgatatgatccggctgccatacatcaaagaaccagccatcagattccgttctcagacgtttgatctctttacggaatttgatcgcacgttcaatagaaccgttgatcagacgcttacctgcattgcctttcatcatcgccgcagcggtttcagtggacgccacgataccgtagtgcggagaagtggtggtgtgcatcatgtaggcttcgttaaaggtttcttcgtttacgtcacctttaacgtggatcatggaagcctgagagaacgccgccagcagtttgtgagtggactgggtttcgtaaatcactttcccttctacacggccaccgctcataccgcatttaccttcgtaaatcggtgagaagttggtgtaaggcacccacgcggagtcaaagtggatggatttcacatccagtgttttcttgatgaagtcggtgttgtacagcagaccatcataggtagagttggtaattacagcatgtaccggccaggttgcgtttggtgtttctttcacgcgcttagcaatggtagcgtgctggaattcactctgtgggataccaccaagaataccgtaagcgttacgggtcgggcggaaatagattggcgtaacatcgctcatcatcatcaggtgggtcagcgatttgtggcagttacggtcaatcagaatggtgctgcctgctggagcagagtacataccaacaattttgttcgcagtggaagtaccgttggtcaccatgtagctgcggtctgcgttaaagacgcgagcgatatactgttctgcttctttgtgtggaccactgtgatccagcagagaacccagttcagatactgaaatggaaatatcagatttcatggtattcggaccaaagaaatcatagaacaggctacctaccgggcttttctggaatgcagtaccgcccatgtgaccaggagtacagaaagtatatttaccttcacgaacatatttaaacagtgctttagtcagcggaggcagaatagtgttgatatattcgtcagtggtctgcttgatcttattagcaatatcttcagcagcacccagcgcatattcaaagaagctaatctgtaaacgcaggtcattcaggcttacatcgagagtggaatacgtattagcgaacgcgtacaacggcaggttctcgttcattttgctaatttcttcgcacagctcgagattatatttatcccagtcaaaaataacgccgcacagacgcgcattgttttcgatcagttttaataagtcgtcacggtcgttcgggtaaacaatctggaagttcagacgttcaagcgcgcgatgaagttcacggatgggttcttctttaaaataaacccccatgtgattcaatattgcaataacgttcatagtcatatctccaggtaaaaaaggcccctcccaacacatgggacaaaatgaaaggaggagcctcggaaaatacttttaattaatgtgcgttagacgcggtgtggttatccattgagtggctctggcgctcgtgcattttgcgagcgtagaacatcaggataatcaggctgacgatgaaggtacctgccagctcgaaggagcttgcgcccatcagcgcgatgaagcagaacacgcaacccagtacagagcagatcaggctgacaaagttgcggatgttaacgccttcaaaacgaatcaggtcaacgcaagagtagaaatacggcagcatagtcagcagtactgcgataccggtcagttcaccgaacaggtcagatgctttaccaccggcagagttcatcagagtgataaggatcatcagggcagtcattttcactgcagccagcagcagaccttttttcggaataccgttgctgtcgacttcaccataaactttcgggaagttaccgtcgttagcggcacgtacacctgcctggcctaccaacatcatccaggagcccagagaagtcaggcacgcaaaggcggtgaatgcagaaaccagcggcgcagcccagttaccgaggatagttgaagcactgattgcaaacggagcaccggaagccgccattacagaagacggatacataccggaaagcacctgagtcgcagcgatgtaaacaatacctgctaaaccagtacccagcatggttgccagcggaacggtacgtttcgggtttttaaccataccagtacttacagctgcggattcaacacccacgaaggcccacaggcagagcagaatacttttaatgatcgcatgaccatcagtggtatccgcagtattccagttagctgcataagttgccgcatcaaaccaatgccagccaacaatagcagtcatcaccacaggaataagaaccagcaccagaccaatagtggttaaacggcttacccaagtaccgccgagcatatttacaaaggtaaatacccagacgatagcaatacaggcgatacccgccggaacaggatcatttaatactgggaagaaggtggaaagataagatacagcggtaataccaatcgccaggttaccaatccagttagcatggtaataaagaacacctgtctgaaaaccaaatgcaggggaaatttctccggcataagcaattgggccaccttgttgcgggttttttgttgccagtcgggcatatacatacgccagcgacattgcaccaataatagagataatccaaccccagatagcaataccaccgatacttgctaggttcgcaggtaataatgcaataccgctccccatcatattaccggcaacaacaccggtacaggcaaatagcccgatcttcttggcagaactcatgctcttctcctaatttcatttttgaatttggagtccgggtcatgatgtataactatttcctgaccagaccaaactggcgataagattactcacgaaaaaaggattaatcctaaagattaggtgaaataacacaaaagtttctgtaagtgagaacttgaggttttttattaacacatcaggatcgcaagttgatatcatgaaaagataaacatttaatgtttacaatggattgcgtgacattctctggttaaatttatgtaataaaaattatgcggcaaataaattgccgcaacatattataccaacaggaacatacaaaaactcaacaacaaatatttccgagcataaatcaacccggagttacttattctgaagcaagaaatttgtcgagataaggtacaacataaggaacagaagtctggaatataccattttcaatccagtaaagggtgtttgcccctgggcgtaaattaaaggcggtgagatatgcatcagctgcttcccggttcatccccttcatttcataaaccttgccaagcaacacataatttagccaggacatttcaagatcaatgccagtatttatcgcctggtaagactcatctgttttaccttttaccagagcactgaccgcttttatttgatatataatggacaggttgttcaattccggcagtgtaacaatgttatctatttctgtgttcagtgctgctaattgtttttcatctaaaggatgttgagaatggcgcacgatatcaactaatgctttttctgctctcgcgtaggtaaattctggggatgattgaacaatctcacctaataattcactggcacggttcaatgatttatcatcgccatgcagtaaataatcatgtgcctgataaaaattagttaataacgcaccacgatgcggcaaaattttctggagcgtctcctgcattcgttgtggccacggttggtttaacgcttttgataaactctccagtaaatcattttgaatcgccagctgattaccgttagtgatgacataacgtttatccagcatggttgaaccatctgcattgtctaccaattttatcgacataaagcattgttgagcacggtattggcgctgattaacaaacgcaatagataatgttttaccggaactgctcggttcatcaatgttgtagttgattttgtcatgcaccataaaggtggagaaggtgttaagtgatgtcgccaccaaatcacccacgcctatcgcgtaagagagctgatacggggaactccagctgttacaacttttatttaccatattaatgtcaatatcgcgtggattgagcaaaatacgcgatttgctcataggaagacgtgtatcaagacttgaaaacgctaccagtgctacacagatacctaacgacaacaggaaaaaaaaccatacccaaaaggtagtgaatcgtttgcttttaactggggattgttcaggtggcgttgcggtgttttgaatgttaagactgtgggagggagaatctgtggcaggaaccgcctctggtatagggggaggcgaagatagcattatttcctctccctcttcttcgctgtaccagataaccggcaccattaatttatagccgcgctttggtacagtagcgatatagacaggactatcttcatcattatcttttaatgacttacgtagttctgagatactctgcgtcacaacgtgattggtgacaatacttctcttccagacattatcgataagttcatccctgctaagtacttcgccactgtgttgagcaaagaaaaccagaagatcgattaatctcggctcaagggtaagttgacgcccattgcggctaatttggtttatggacggagtaacaagccattcgccaacgcgaactacaggttgttgcataatagaaactcattcgaaaagggaatgatgcaatgataattgccacaacctatttttaccatctatagatgggtttatttacatattattggtgaatgcaagacgttatttttaccagccataaacttcttgattacatagtattacgaaaggattttactgagaaccagaagtaatattccttaccatcaaaattcatcatctttgccaaagaaaaatgttcagaaaataatccatggaaaattgtccggagcacttactattttaatggattgttagtctttgcatgagcaagcgaactgatacatttctctttgttctcattcagaaaatctcatcagtcgccgttcagaccggtgttgtgctttatggatgcgttacgctcctgatgacgtcatttgacgttcaacagcatcacggggccgcacgacatttcacgtcagttagtgctatagctcaggaacaaattttcccgaattgggatatgcccgcaaattgctggtgatgtggggagaatctggttgagttcggtagaattgatttggaggcagaacgcttaaatcgtggcgtcctgaaacgaaaaacggacctccgtggaggtccgtttatatgaatttggtgcccggactcggaatcgaaccaaggacacggggattttcaatcccctgctctaccgactgagctatccgggcaacggggcgcattaaaccgtaatctgcacatctcgtcaacctaatttcagtaaaagcgattcaactgcttaagattgcggcaaatcgcttcttttctgtgtttctgtcaggtcaatgcaccaccctggcggcagcgggcgaagcgcaggatatcttccgccagccgatgtgcagtgtcgacatccgcctggctacgattcaccagcattcggcttaaacagccttccagcaccagttccatctgctttgctaccatcgccggatcgtcaacttccagtgtggttaacagttcgtgggtgaaatcgtaggccgcgcttttttgctgatcggccagttgatgaatagggtggccaggatcgggataaaacgtacaggcagcgataaatagacagcccggatagcggttgtttttaacgcactccgataacgcctgataacgtgccagcagcttttgttcggcggtttgcgtttcgtccagcatcagctgacgacgccagacatctatctgttggctaagataacgcagcgcatcgtagaggattgcctctttgtctggccagaagcggcgtagctcgtccagtggataatccacacgttcagcaaccatctccagcgtggtgttggcaatcccttgtaattctaataatttcagggcttctcccagtacatcttcacgttgcacgctattttcctccgtctttcccactgcaagtgtcgttcacggttggcgatcgcgcaaatgtgcgctgaaggtttcagcatccataaagcccgtgacgcgtgcttgtggatgctcctggccttgtccgtcaaaaaagagaattgtcggtaggccaaggacattaagatgctttaacagcgccacatcttgtgcgtcgttggccgtgacgttggcctgaagtaagaccgtgtctgctaacgctttttgcacctgcgggtcgctgaaggtgtatttctcaaactctttacaggcgacgcaccagtcggcataaagatctaacatcaccggtttgcctttggcttcaacgagcgcctgatttaactcatctaccgttttgatttgtgtaaagttgagatgcgtctgagtttgcgcggtatgcgtcgcaccaaatgcccaatcctgaagtgggcgcacgctaaccaatgccgctgccagcagaataatttgcacaatacgcatccagccgcgtttagcctgtaggctggtgataaaggcccagccaaagaatgcgacacccagcgccgaccacaagcgtaatccccatacatcaccaatcactcgctccagcaggaagaccggcagtgcgaggatcacaaaaccaaacgcggttttgacttgttccatccacgggccgcttttcggcagcaagcggttaccaaagacggtaattagcatcagcggcaggcccatgcccaacgcatagagataaagcgtgccgccgcccagccacatgttcccgctttgggcgatatacagcagaatcgcgctaagcggtgcggtggtgcatggtgaacagatcagtccggcaatcgcccccataacaaacacaccgccaggtgagccgccctgttggcgattgctcatcaacgtgagacgtgtttgcagcgaagaggggagttgcagggtaaacaagccaaacattgacatcgccagcaaggtaaagacgatggcgaggccaatgagcacgtatgggtgctgtagcgccgcctggaactgtaaccctgcggcggcaaccaccagacccagcgccgtgtaggtcagcgccatcccctgcacataaataaaggtcagcaacaatgctctggcagtggagagccgctgtttaccacccagcacgatgccagaaatcagtgggtacattggcagcacgcatggcgtaaaggcgataccaataccgatcaacaacgcccagagcgcggaaaagggcaattgcgcggtgggctgctcttgctgcggaacagacacaggctgtggcgctgcgttgttggcgaccacttcgcttaacggaacggttttggtttctggcggataacagaaaccggcatcagcacagccctggtaggtgacagttaacgtcgctcccgcactcgcctggttgatggtgacgggaagcgtcagccgatcgcggtaaatctcgcttttgccgtaaaactcatcttcatgccagacgccttgcggcagctgcacgtcggcaattttcgcgtgttccggcgtaatgcggatctgtttacggtagaggtagtaaccgtctttgatctgccaggtcagattaaggtcatgttggttttgctgaaaatcaaaagcaaaggcttgatccgcggggacaaattgtgaacgtcccggcgcgtcgaataatccggcaaaaacggaagtgctgcaaagtagcaggatcagcgtaaagatgcgttgagccatgagaggtaatctgtgtctccgtgtgtaacaggtaaaaccagaagttccggggtttgatatggatgatgagacttcaggcattccagcagtgcctgctggtgagatacggtagtttttaaaatcatctgcacttcgtattcttgctccagcttaccttcccagtaatagagagaggtagcgccggggatcaaggtcgcgcaggccgccagtttttccgccagcactttggcggctaaatcctgggctgtcgcttcatctggtgccgtacatagcaccacgacagacgcggtattcgaacttttttcatcaagcataaacacctcgcaagaacagatggaaccgcaagagagaggtcactatacaacggacgggggaaggatgttagtcggcgggaaagaaagcggggcgtgaacgccccgcgattgatcattacagcatgaagctacccagcacgaagccgaagcaaacggccagggcaacacccagagtacccgggatgaagaacggatggttgaagacgaatttaccgatacgggtagtacccgtgtcatccatctgtaccgcagcaaccagcgtcgggtaggtcggcagaatgaacagaccagacaccgcagcgaaagaagcaacagcggtcagcggtgaaacgttcagtgccagagccatcggcatcagtgcttttgcggttgcagcctgagagtacagcagagcagaagcaaagaagaagatgacggccagcagccacggatgaccctgaatcacttcaccagcggtatctttgatccagtcgatgttgttggaaacgaaagtatcgcccagccacgcaacacccaggatacaaatacaggcgctcatacctgctttgaaggtgctggagttgaggatgttgtcggtatcgactttacagataacggtggtcagagttgcaacgctgagcatgatgatcaggattgcgttggtggtgttcatcagcggtttttcaaccagacccatgcttgggctgttgatgattgcatagataaccacgccaactacgcccagcaggaacagccagacggacgtttttgcaccggatttgatttcaatctgcttttcaccgcgcagttcaaccaggccctcttccagacgcttgcgataaatcggatcgtcagagagtttggagttgaacagcatagtgaccaggaaggacatcaccagaaccgccagcagggtggacgggatgaccacggagagcagatggaggtagctgatgccatgaccttccatcacggaagacatgtaaaccactgccgctgagattggcgatgcggtgatcgcaatctgcgcggataccactgcagtagacagcggacggcaaggtttaacgccttgttccttcgcaacttcagcgataactggcagtgtcgccagagagatgttgccagtaccagcaaagatagtcaggaaataggtcacgatcggtgcgaggatcgtgatgtatttcgggttacggcgcagcagcttttctgtctgatgaaccagatagtccagaccgccagcaacctgcatggcagaaatagcggcgataaccgccatgataatggagatgacatcgaacgggatgttaccgggtttaacgccaatagcggcaagaaccagcacccccaatccgcctgcaaaaccaatacctattccccccaatctggcgcccaagaagatcgccagcaaaactatgatgagttctacaactagcatattagccttccttgttttttaacaagttgatattagattgttatttttaagttactgctcacaagaaaaaaggcacgtcatctgacgtgccttttttatttgtactaccctgtacgattactgttcgctttcatcagtatagcgttttgctttgtaagccgggtgcatcagattctgtacggagaaaatatcgtcaagttccgcttcagtcaacagaccgcgttccagaacgacttcacgtacactcttaccggtttcggcacagattttacccacgatgtcaccgttgtggtgaccgatgaacgggttcaggtaagtaacgataccgatagagttgtaaacgtaaccttcgcacacttctttgttagcagtgatgccgttaatgcatttttccagcaggttgtagcaagcgttggtcagaatgtgaacggattcgaacatggcctggccaatgaccggctccataacgttcaactgcagctgacctgcttctgctgccatggtaacagtggtgtcgttaccgatgactttgaagcatacctggttaaccacttccggaacaaccgggtttactttagctggcatgatggaagagcccgcctgcagttccggcaggttgatctcgttcaggccggcacgtgggcctgaagagagcaagcgcaggtcgttacagattttggacatcttcacagccaggcgtttcagcgcgccgtgaaccataacataagcgccgcagtcagaggtcgcttcgatcaggtcttcagccggtacgcatgggaagccagtaacttcagccagttttttcactgccagcggagagtactctttcggcgtgttcagaccagtaccgattgctgttgcaccaaggttaacttccagcagcagttcagcggtacgttggatgtttttcacttcttctttcagcaggatgctgaaagcgcggaattcctgaccgagggtcatcggtactgcgtcctgcagctgggtacgacccattttcaggatgtcctggaattcgacagctttacgttcaaagccttcacgcagttggttaatcgcatctaccagcttaatcagggaagagtaaactgcgatacggaaaccggtcgggtaggcgtcgttagtggactgacatttgttaacatggtcgttcgggttcaggtactgatattcacctttttggtgacccatcagttccagaccgatattggccagcacttcgttggtgttcatgtttacggaagtacctgcgccgccctggtagacgtctaccgggaactgatccatgcattttccgttgttcaggacttcatcacatgcggcaatgatggcattcgctacacttttaggaatggtttgcagctctttgtttgccatagctgcggcttttttaaccattaccataccgcgaacaaattcaggaatatcactgattttgttgttgctgatatagaagttttcaatcgctctcagagtgtgaacaccatagtaggcatcagctggaacttccctggtacccaacagatcttcttcgatacgaatgttgtttgacatgtgaaccttctttttcaagctgccaatgatttgctttaaacacacagaatatatgtggtttcgaatgtttttcgaccgacgattatcccctgcatcgaccgaatacccgagatcatatgctgcttgaggatttctaccgtaatctggatcactttaagtgtcggtttttaccccttaattattaatttgtgaaatagatcaccgctttgggattactaccaaaaatagttgcgcaaacatcttgaaattttgctaatgaccacaatataagctaaacgcgattcgcaacccattcaggtagccggggttaaccggctgctattacaggagaaacctttgcgctggttaccttttattgccattttcctttatgtctatattgagatttcaatctttattcaggttgcccatgtattgggggtattgctgaccctcgtgctggttatattcacgtcagttatcggtatgtcactggtacgtaaccagggctttaagaatttcgtgctgatgcagcaaaaaatggcggcgggtgaaaacccagcggcggagatgattaaaagtgtttcgctgatcattgctggtttgctgcttttattaccgggcttttttaccgacttcctcggtcttctacttttattgccgccggtgcaaaagcatctgacagtgaagttgatgccgcatttgcgcttttctcgcatgcctggcggcggttttagcgccgggaccggtggcggtaatacttttgatggtgagtaccagcgaaaggatgatgagcgcgaccgccttgatcataaagacgatcgccaggattaatgtcgaaacgccggattatgtggttatgccattttccggcgtttttcgttttggcagcaacagccataaccccgccagcatgatcagcgcatagagacttttccagccgaccattgccagtaacagaacgcataacagcccgccaaccaccgccagtagtcgataacgtccttgcaataatttacagcctgccagcatgcataacagataaatcataataaagatgccattggcataaataataagagcgtccagattgatctctaaagcatgaatcaccaaagtgctcaccacacagcagccgagcaccgcattgagggcattattcgggatatggcgagaagagaggcgtgccaggtagtggtcaggattatgttgcgcctgcgaccagaccaggcgggcgaagctctgtatataaatgttgagactggcaaagcaggccagatagccaatcacgcaggcaatccataacgctcctacaccgaacaactgcactacaatttttggaagcgatgctgccgccgccattttttcaccataggcgtcgaagtgtaagacgactaccgtacagccccagtagactaatcctgccagcagcagaccaatcatcaaagcacgaggaaaatcacgctctggatttttaaattccgaggcgagatgggcaaatgcctccagaccgacaaaacaccagaacatcactgataacgcagcaaataacccggtaagttcgatattaccaggtgccggaaaggggatattcgcaggtttgatatcgcccgcccaccagatagcgacaatcagcgcgacgataagtccggcaataacggtttgtagattagcactggaactggcaccgcgagtaccgatataccacaccagcgccagcgtaccgagttctgccaacaacagttgccagctatgccagccaaacatcgcctggccgaacccggcggcaatttgtagtgcggcaggcaaacccacgggaatgaccgataaaaacagccagccggtgactcgctcaagccgcgaaccaaacgccataccgacgaagtgcgcgacgccgcctgcgctgggatagtggcgacccagaatcgcaaacacaatcgcaatcgggaacactaagataatcaaaacgggccacgcccacaggctgttattgcccgctaccagcgcagctaacgcaggaacggcaaacacgccagtgcctaataatgacgtcgatagcaggccaatgccctgggccagccccagttcttgtttgagtccactcatgggttgatgtccgattgcgcccaaattttgggcaactgcgtagattttcgatggtagcacaatcagattcgcttatgacggcgatgaagaaattgcgatgaaatgtgaggtgaatcagggttttcacccgattttgtgctgatcagaattttttttctttttcccccttgaaggggcgaagcctcatccccatttctctggtcaccagccgggaaaccacgtaagctccggcgtcacccataacagatacggactttctcaaaggagagttatcaatgaatattcgtccattgcatgatcgcgtgatcgtcaagcgtaaagaagttgaaactaaatctgctggcggcatcgttctgaccggctctgcagcggctaaatccacccgcggcgaagtgctggctgtcggcaatggccgtatccttgaaaatggcgaagtgaagccgctggatgtgaaagttggcgacatcgttattttcaacgatggctacggtgtgaaatctgagaagatcgacaatgaagaagtgttgatcatgtccgaaagcgacattctggcaattgttgaagcgtaatccgcgcacgacactgaacatacgaatttaaggaataaagataatggcagctaaagacgtaaaattcggtaacgacgctcgtgtgaaaatgctgcgcggcgtaaacgtactggcagatgcagtgaaagttaccctcggtccaaaaggccgtaacgtagttctggataaatctttcggtgcaccgaccatcaccaaagatggtgtttccgttgctcgtgaaatcgaactggaagacaagttcgaaaatatgggtgcgcagatggtgaaagaagttgcctctaaagcaaacgacgctgcaggcgacggtaccaccactgcaaccgtactggctcaggctatcatcactgaaggtctgaaagctgttgctgcgggcatgaacccgatggacctgaaacgtggtatcgacaaagcggttaccgctgcagttgaagaactgaaagcgctgtccgtaccatgctctgactctaaagcgattgctcaggttggtaccatctccgctaactccgacgaaaccgtaggtaaactgatcgctgaagcgatggacaaagtcggtaaagaaggcgttatcaccgttgaagacggtaccggtctgcaggacgaactggacgtggttgaaggtatgcagttcgaccgtggctacctgtctccttacttcatcaacaagccggaaactggcgcagtagaactggaaagcccgttcatcctgctggctgacaagaaaatctccaacatccgcgaaatgctgccggttctggaagctgttgccaaagcaggcaaaccgctgctgatcatcgctgaagatgtagaaggcgaagcgctggcaactctggttgttaacaccatgcgtggcatcgtgaaagtcgctgcggttaaagcaccgggcttcggcgatcgtcgtaaagctatgctgcaggatatcgcaaccctgactggcggtaccgtgatctctgaagagatcggtatggagctggaaaaagcaaccctggaagacctgggtcaggctaaacgtgttgtgatcaacaaagacaccaccactatcatcgatggcgtgggtgaagaagctgcaatccagggccgtgttgctcagatccgtcagcagattgaagaagcaacttctgactacgaccgtgaaaaactgcaggaacgcgtagcgaaactggcaggcggcgttgcagttatcaaagtgggtgctgctaccgaagttgaaatgaaagagaaaaaagcacgcgttgaagatgccctgcacgcgacccgtgctgcggtagaagaaggcgtggttgctggtggtggtgttgcgctgatccgcgtagcgtctaaactggctgacctgcgtggtcagaacgaagaccagaacgtgggtatcaaagttgcactgcgtgcaatggaagctccgctgcgtcagatcgtattgaactgcggcgaagaaccgtctgttgttgctaacaccgttaaaggcggcgacggcaactacggttacaacgcagcaaccgaagaatacggcaacatgatcgacatgggtatcctggatccaaccaaagtaactcgttctgctctgcagtacgcagcttctgtggctggcctgatgatcaccaccgaatgcatggttaccgacctgccgaaaaacgatgcagctgacttaggcgctgctggcggtatgggcggcatgggtggcatgggcggcatgatgtaattgccctgcacctcgcagaaataaacaaacccccgggcagaaatgtctgggggtttttcttttggtcatctttctagtataagattcagacacggacgacgcgagtggcgtccagctcattgattatggggaataacatgcacgtaaaatacttagcagggattgtcggtgccgcgctactgatggcgggttgtagctccagcaacgaattgagtgctgccggtcagagtgtacgcattgtggacgagcagccaggcgcagagtgccagctgattggtactgcgacaggtaagcaaagcaactggctttccgggcaacacggagaagaaggcggttctatgcgcggcgcagcaaacgatctgcgcaaccaggcggctgcaatgggcggtaacgtgatttatggcatcagtagcccgtcgcagggaatgttgtccagttttgtcccgacggatagccagattatcggtcaggtttataagtgcccgaactgatgtgatccagaggctgggtgacaaacgtataattgcctgatgcgcttcgcttatcaggcctacataaggcattgcaactgattgaatgcttgagaatttgtaggccggataaggcgtttacgccgcatccggcatgaccaacgatcacgttatcagtcatttcaggctggatggctccagcctcgcattagcaaagatgagattatttcgcctgtggtgcagttttgctggtggattgaacacgtaagtgatgcagcgcgcgtaagcattgatcctgggttagcggttgggcgttattcgccgctacggtgcgaacatagacctgacatggcacacccgcgagttttttcagtcgtgggctgaaatcaagcattcggcgagtgatcgcttctatttctttacccggcgttgcttcacgcgttttcaccactgcgccgctaaattgttctttgccactttcatctttaaagcggtaaagcaccgccagataatggtcgaacaagttatgtttccattccggttgggaataggtgtcatattccagattgccattgtcctggcagtcaacgtcgtataacggcaggaaatctaacagtgaggtaatacgtaatgccagttcacgcatttccgcattattaattgcatgaatgattgctcgcgccagcatttcaatctgcaactcattgacgactaactcacatttgctaccgtcatgtagcgttaatacgaaggtaagattttcgccttgattatcggtaagttccagcgtgttaacccgacgattaatatcggcatttttaagctcatcaaccagaatttctgggatgttttctgccattttcttaatgactttatcgcgagcttgctcatactgaaggtgtgcagcagcatccagtttatgcttttgatgcagacgactttccagcgcaatcagcaggtcgcgcagttccatgacagacataaagaacaacgattctttattgcgaggttctttaattttcagcgccagtgcaatgaaattattactcttgcgaataacaccggtattaacacccttgatgcttatggccatgtaggttctccctaaccatttctcaattaaataattaattttaatttataagccagataaatgggcttggtagtaatagttgttaaaataacataaatagccgtactcactctatataaacagaaaagaaaggttaattattggtgttagctatataaaaagtaacaacagcaatgcatatgaataattaaaggttatgcaacgggcaaagattaaacttcccagtttaatgacaggttgctgtacttgcgtttgttgctcttgccggatgcagcgtaaacgccttatccggcctacagttcattgcaaatccattcaatttcaatgcacgatgtaggcctgataagcgtagcgaatcaggcaattttaatgtttaacttccctgtttaatcagttactgctggcgtagctggagatccagcggcgttttgctgggttcgccgccaatttctcgcgccagtttcggcaccagatatcccgacaccagtgtcagcaactcacgcataatctgccgtgcttcgtcatcactcaccataaaatgcgccgcgccctgtactttatcgagcacatgcaggtaatacggcattacgccggcatcgaacaacgcattactcaggtttgccagcgtttgtgcgttatcgttcacatcacgtaacagaacgctctggttcagcaaagtaacgcctacccggcgcaacttagccatcgcctgacggaatgtttcatctacctcattggcatggttgatgtgattcaccagcaagatttgcagcgtagaacgggcaaagcattcaaccagcgcctcggtgatacgtgccgggatcacaatcggcagacggctgtgaatccgcagacgttttatatgcgggatggcttccagttgtgtgagcaaccagtccagctcgtgatctttcgccatcagcggatcgccgccggagaaaatcatctcgtccagttccggatgcgcagcaacatactcaagtgcagtttgccagttacgcttgttgccctgattttcggcataggggaagtgacgacggaagcaatagcggcaatttaccgcgcagccgcctttgaccagcaaaagcgcccggttgtggtatttatgcaacaaaccaggcactacgctgtgctgttcttccagtgggtcggtggagaatccgggcgcgatgacaaactcatcttgcgaggtaagtacctgacgcaaaagaggatcgtccggattgcctttctccatgcgatcgataaatgagcggggcacacgcagggcaaaaagctttttggcgctgcgtccggctaacagtttttcctccgcgtctatattcaaaagacgcagaagttcatcaggatcggtcacaacatcggcaagttgcgttaaccaatcttctctggatggggtatttagggttacaatatgcgccattttgtggcttagctaccaattaacaaatttcagagggccttatggcaacgtactatagcaacgattttcgtgctggtcttaaaatcatgttagacggcgaaccttacgcggttgaagcgagtgaattcgtaaaaccgggtaaaggccaggcatttgctcgcgttaaactgcgtcgtctgctgaccggtactcgcgtagaaaaaaccttcaaatctactgattccgctgaaggcgctgatgttgtcgatatgaacctgacttacctgtacaacgacggtgagttctggcacttcatgaacaacgaaactttcgagcagctgtctgctgatgcaaaagcaattggtgacaacgctaaatggctgctggatcaggcagagtgtatcgtaactctgtggaatggtcagccgatctccgttactccgccgaacttcgttgaactggaaatcgttgataccgatccgggcctgaaaggtgataccgcaggtactggtggcaaaccggctaccctgtctactggcgctgtggttaaagttccgctgtttgtacaaatcggcgaagtcatcaaagtggatacccgctctggtgaatacgtctctcgcgtgaagtaatgcggttgtggtgcggcctgcaggctgcaccatcacttattcaggtcagagatgatgaaacgccttatcgttcttgttttgcttgccagcacgctgctcacgggctgtaacaccgctcgcggtttcggcgaagacatcaaacatctcggcaactccatctctcgcgctgccagctaatttttcttctcttccgaaaaatcatcagattcccatcatttttggcgatgttgtctattattaatttgctataggcaaacataaataacattacctaaaaggaagacgttatggtgaagaagacaattgcagcgatcttttctgttctggtgctttcaacagtattaactgcctgcaacaccacgcgtggcgttggtgaagacatttctgatggcggtaacgcgatttctggcgcagcaacgaaagcgcagcaataagcaataacggtacgacagctgtgtcgtgccgtttgttttttctgcgatagtcacaaaggtaatagttgaaattcccctgccacctggcaaaatatccgttcaaccatcagctttgcaggacgacctgcaaacgcctcttttcaccggggacggccccaattctccggagcctgatatgtcctggattatcttagttattgctggtctgctggaagtggtatgggccgttggcctgaaatatacccacggctttagtcgtttgacgccgagtgttattactgtgacggcgatgattgtcagtatggcgctacttgcctgggcgatgaaatcgttaccagtagggacggcttatgccgtgtggacgggtattggcgcagtcggcgcggccataaccggcattgtgctgctcggtgagtccgctaacccgatgcgcctggcgagtctggcgttaatcgtattggggattattggtctgaaactcagcactcactaactaccaggctgctgtacccaaataaatttactgacatcaaacccttcccgggtcgcgactgccagcatctcctgtttcacttcgtcagaaatggttggcgtgcgggagagtatccacaggtagtcgcggtccgggccgcaaaccagcgcatggcggtattcccgatcgagtgcaataacgttataaccgccatagaaaggaccaaagaatgacactttcagcgcagcgcgagttggtgcgccggtaaagtacgctttcccttcactctgctgccacattcctctgtcagggttatagcctttattaatgacattcaggccgccgtcatcacgcaggctgtatgttgcggtgactttttccagtccacgttcaaagcggtgatcaaaacgggcaatctcataccaggtaccgagataacgtttggcgtcgaaattatttactacggtcacgccacgcggcggcgtaggagaactgcaggcaacgaccagaaatgcagctgtcgctgcggcaacgagagggagcaggcgcataaatgtttccttactggtttttttctaagtgtagatgacagcaaggaaaagcggagaaaaggtccgaaaattcggacccgatggaattttactgtagagcgttaagaatctgccaggcggcgtcgactctcgctggattgggatagtttttgtttgccagcatcacgatacccagctctttttctggaataaacgcgacatagctaccaaatccgccggtcgcccctgttttatgtacccatgatgcgcgtactgcaggagttgggggcgtaatcgcttttacggggcgtgctgccagtgcaattttattgtcactgccgttaatgatgctgtcaggatttaccggccagtccagcatttcccagcccaggccctgatacatatcgccggtttgccagtagcgagattgtgccagttgtatcccttgttgaagcgttttctcattgatatcaaggggttttaaattgctttgcacccagcgggccatatcttcaatggtcgacttcacaccataagcttcagcatctaacgccccaggcgaaacatgcactgccttaccttcgcgatatccccaggcgtaattcttttcttctgcgggcggtacattaatccacgtatggttgagtttgagtggctggaagacacgagtttgcatcgcctgctcaaaactcaaaccagacggcttcacagccagtgcgccgaacaaaccgatactggagttggcatacagacgttgtgttcctggagcccatgcaggctgccagttttgatagaagcgcagcaagtcgcttgaggatttcacctcatccggcacctgcaatggcaggccgccagcagtgtaggttgcgagatgtaatagtgtgatcccattccactgtttagcggtaagttcaggccagtattttgttgtgggatcgcttaacttgatttcccctcgagcaatagcgtcgccaccaagcacgccagtaaatgttttgctgaccgaacctaactcaaacaacgtttgctgtgtgacgggctgctttttggcgatgtccgcatagccccaggtaaagtaataaggtttaccctgataaattaccgccaccgccatacccgggatcttttgttgctctataagcggggtaattgtgcgatgcacaatatcgttgatttgttgaggggcagcaaatgtggagcaagaggcggtaattaataaggcgcagagcgtcgttttgaacatagggtctggtttccatacaaaacggcccgccataggcgggccggatttacattggcgatgcgttagattgtaacgacaccaatcagcgtgacaactgtcaggatagcagccagaccgtagaaaacccatttgcccgcaggtacgtggattttcagatcgtgcatcgcgtggtgcatacggtgtaaaccacaccacagcggcagaacgatcatcaggaacaggaatacgcgaccaatgaagctctgcgcgaacgccagaacgcgctcgtagctcagcgcatcacccggaaacaaccccagtggcagcagaatacccaccagcaggatcatcaccggcgcaatgatggcgctccacataccaccggccccgaagaggccccagaataccggttcgtcagaacgctttggatttggattaatcatctcaggctccttaccagtacagggcaacaaacaggattacgatggtggcaaccacagttaccgcccagagacttttgataattggctctggtcccattttttcgtcttttacaatgatattggccgctttcggtgccagttcaaaccaggttttggtgtgcagcagagctgccgccagagtgatcaggttaatgatcacgataaccgggttttgtaaaaagtcgacgaatcccgcccaggcttccgggccatttttcagggcaaacagcccgaaaatcagttcaatgctgaaccacacagccggaaccgccgtgccttcgcgcagcatgtaaaagcgataaaacggcaattttttccaccaggtggacgtcattggccgtacatacggtttacgtttagtcgtcatgttgcactccttagcgtggtttcagggtcgcgataagaaagtctttcgaactttctactttgccctgctgaatggccgcagccggatcgacgtgtttcgggcagacttcggagcagtagcccacgaaagtacagctccatacgccgttctggctgttcaactgcgccatacgctccttcttaccgtggtcgcggctatcttcgttataacgatgcgccagcgtaatggcagccggaccgatgaactctgggttcaggccaaactgcgggcacgcggcgtagcacaaaccacagttgatgcaaccggagaactggtgatacttcgccatctgcgccggggtctggatgttagtaccctgatccgcggtgcgggagttgccgatgatgtacggtttgatcgcttccagactttcgatgaagtgggtcatatcgaccaccagatcgcgttcaatcgggaagttagctaacgcttcaaccttcataccgtcggtgtaatcacgcaggaaggttttacatgccagttttggcacgttgttaaccatcatgccgcaggaaccacaaatcgccatacggcaggaccagcggtagctcaggtccggtgccaggttgtctttgatgtagcccagcgcatccagtaatgaggtagttgcgtcataaggcacttcatagaatgcgctatgcggtgcggtatcgacttccgggttatagcgcaccacctcaattttcaggtttttcatctcagccattcgccttctccttcttattggctgcttccgccttatcggctgcatccgcttcgccaccgtaaacgcgtttagctggcggcagcgtagtaatcttcacgtcgctgtactccaggcgagtcgtgccatcagcatcgcggaaggcgagggtgtgtttgaggaagttgacgtcgtcacgctcggtgcaaccttcgtccagacgctggtgcgcgccgcgggactctttacgtgccattgcggagtgcgccatacattcagcaacgttcagaccgtggcccagttcaatggtgtagagcaggtcggtgttgaacacgctggaagtgtcggtgatgcgcacgcgcttgaagcgttcctgcagctctgccagcttgtcgatggttttctgcatcagttccggcgtacggtagataccgcagccttcttccatagccaggcccatttcgtcgcggatcttcgcccagttttcgccgccatcctggttaaccagatctttcagacgttgttcaacgccagctgcctgcgcttcaattgccgcttcgttgccattaccggcagttgctgcacgctctgtcgcttgttcaccggccagacggccgaagaccaccagttccgccagggagttagaacccagacggtttgcaccgtgcagaccaacagaggaacattcacccacggcgaacagacctttaatgcgggtttcacagttctgatcggtttcgataccgcccatggtgtagtgtgcggtcggacgtaccggaatcggttctttaaccggatcgacgccaacgtacgctttcgccagttcgcagatgaacggcagacgttcatgcagttttttctcgccgaggtgacgcaagtcgagataaaccacatcgccacgcggcgtggagatggtgttgcctttacgccattcgtgccagaaggcctgagagactttgtcgcgtggacccagttccatatatttgtttttcggctcgcccagcggagtttccgggcccatgccgtaatcttgcagataacggtagccatttttgttgaccagaataccgccttcaccgcggcaaccttcggtcatcaggataccggaacctggcagaccggttgggtgatactgaacgaattccatgtcacgcagcggaacgccgtggcttagcgccatacccataccgtcaccggtaacgatgccgccgttggtgttgtaacgataaacgcgacccgcaccgccagtagccataacgaccgcgttagcacggatctgcaccagcgtgccttccatcatgttcattgctaccaggccgcgaacatgaccatcatcaaccagaatatccagcacgaaatgttcgtcaaaacgctggatctgcgggaattgcagagaggtctggaacagcgtgtgcagcatatggaagccggtcttatcggcggcgaaccaggtgcgctcgattttcatgccgccgaagcgacgtacgttgacgctaccatccgggcgacggctccatgggcatccccacagttccagttgggtcatttcggttgggcagtggtggacgaaataatccacgacatcctgctcacacaaccagtcgccacccgctactgtatcgtgaaagtgatattcgaagctgtcatgatcctgcgcgacagcggcggagcccccttctgcagcaacggtatggctacgcatcgggtatacttttgagattagtgcgatttttgcattcggatttgcctgcgcggcagcaattgcagcacgtaatcccgcgccaccggcgcctacaatggcaagatcggcttgaaaggtttgcacgacattcctccagattgtttttatcccacagccacgtacttcagggtaagtacctgaaagttacggtctgcgaacgctattccactgctcctttataggtacaacagtatagtctgatggataagtctgaaatttgacgagatcgatttttttagtgcgcaagagggctaaattatcactgaagatgattaatttaattactaaaccatcagatcgtgctttttttagtcactgcccaccgctgtttgattcctgcgtaaaatttgtctcgccgtcgcgttgcgagtagacttcgtgcccttgtcaaaaactggagatttaactatgagcgaaacggcatcctggcagccgagcgcatccattcctaacttattaaaacgcgcggcgattatggcggagatccgtcgtttctttgccgatcgtggagtgctggaggtggagacgccttgtatgagccaggcgacggtaaccgatattcatttggtcccgtttgagacacgtttcgttggccccgggcattcgcaggggatgaatctctggttaatgaccagcccggaataccatatgaaacgcctgctggttgccggttgtgggccggtattccagctgtgccgcagcttccgtaatgaagagatggggcgttatcacaaccctgagttcactatgctggagtggtatcgaccgcactatgatatgtaccggttgatgaacgaggtggacgatctcttacaacaggtgctggactgcccggcagcagaaagcctttcttatcaacaagctttcttgcgttatctggaaattgacccgctctctgccgacaaaacgcaactgcgggaagtcgcagcgaaactggatttgagcaatgttgctgataccgaagaagaccgcgacacgctgctacaattgctgtttacctttggcgtagagccaaatattggcaaagaaaaaccgacctttgtgtaccactttccagccagccaggcatcactggcgcaaatcagtaccgaagatcatcgggtcgctgaacgctttgaggtttattataaaggtattgagctggcgaatggtttccatgaattgacggatgcccgtgagcagcaacaacgctttgaacaagataaccgtaagcgcgcggcgcgcggtttgccgcagcaccccattgaccagaatctgattgaagccttgaaagtcggtatgcctgactgttccggcgtggcattaggtgttgatcgtctggtgatgttggcgctgggcgcggagacactggctgaagtcatcgcctttagcgttgaccgggcataattctgaaaaattactgaattaacagcgaagaatggcgtgataagcgccattctgtagcatatgttttcatttttccgttaaaggccacaatttaagactggatatttgatatcatccaggtatcaattctgtattggtttttacgctgcctgctcaatgttgcgcagtgcagttcagtgggcacgtgttatacacgcgctgaaatgaaggatggtttcatgcctcacacgataaaaaagatgagtctgataggactcatattgatgatctttacttccgtatttggatttgccaatagcccatcggcttattacttaatgggttatagtgcgattcccttttatatattttctgcattgttattctttattccattcgccttaatgatggctgaaatgggagctgcttatcgcaaagaagaaggcggtatctattcctggatgaataatagtgtcggaccacgttttgccttcattggtacgtttatgtggttttcctcttatatcatctggatggtgagtacctccgcgaaagtttgggtaccgttctcaacattcctctatggtagcgacatgacccagcactggcgtattgccggactggagcctacgcaggtggttggtctgctggctgtggcatggatgattctggtcaccgtcgttgcttctaaggggattaataaaattgcccgcattactgcggtgggcggtattgcagtaatgtgtctgaatttagtattgctgttagtaagcattactattttgttattaaatggtgggcatttcgcgcaggatattaatttccttgcatcaccgaacccgggttatcagtccggtctggcaatgctatcgtttgtggtatttgccatttttgcctatggcggaattgaagcggttggtggtctggtcgataaaacggaaaatccagaaaagaactttgccaaaggtattgtttttgccgctattgttatttcaatcggttattcgctggcaatatttttatggggcgtcagcacaaactggcagcaggtattaagtaatggttccgttaacctcggcaatattacctatgtgctgatgaagagccttgggatgacgctgggtaatgcactgcatttgtcacctgaagcgtcattgtcgctgggcgtatggtttgcgcgtattactggactttcgatgttcctcgcctataccggtgcgttctttacgctttgctattcaccgttgaaagccatcatccaggggacgccgaaagcattgtggccggaaccgatgacgcgcctgaatgcgatggggatgccgtctatcgccatgtggatgcagtgcgggttggttactgtcttcatcctgctggtttcgtttggtggcggtaccgcatcggcgttctttaacaagctgacgctgatggcgaacgtgtctatgacgcttccttacctgttcctcgcgctggctttcccgttctttaaagcacgtcaggatctcgacagaccgtttgtgattttcaaaacgcatttgtcggcaatgattgcgacagtggttgtcgtactggtggtgacatttgcgaacgtcttcaccatcattcaacctgtggttgaagccggagactgggacagcacattgtggatgattggcggccctgtcttcttctcgctgttagcgatggcgatttaccagaactattgcagcagagtggcaaaaaatccgcagtgggcggtggaataacccgatgccctatcgtctacctgacgatagggcgtaaagacaggaaatgttatggatgacaccagccgggacccggcaataaccgaagatgaaatcagggcgctgcaattttctgccggggatgtagcggaaatagagcagacgattctctcttttgtcgatgcctgccacacccgtaaagtggcgatggtggtgggtagcaccattaacaccctcaaagatcgcgatggtaaacggtggggaaacctgccggatatttattgcgcttatcttatccgatgtctggtttttcgcggggaattagtgggatacggcgatttgtttcgtatgcgctatagcgaaattaagcgaccggttaccttatgagtgcgcgcatgtttgtcttatgctgcatctggtttattgtggcgttcctctggataaccatcacttccgcgctggacaaagagtggatgattgatggacgcgggattaacaacgtctgcgatgtgttgatgtatctcgaagaagacgatacccgtgatgttggtgtgataatgacgttaccgctctttttcccttttctctggttcgctttgtggcgaaaaaaacgcggctggtttatgtacgccaccgcgctggctattttcggctactggctgtggcagttttttctgcgctatcagttttgtttgtgagccggattggttcatccggcacacaaacttacaaacttcccgcctgacgacctttgcccgcagacgtcagcgttctccccgtttgtttaccgttgaggctttccagacgcatctggaagggcgggaatggcatatcgataccgtgggcatggaagccagccagaatcagctggtggatctcatggcgtagcggcatacggtgacccatctcagcggcgtaaatacgcagctcgaaaatctgaatcccctgttgcagatccaccaggaagacttccggtgccgggttgtcgatcaccagcgagcagcgacgcgctgcggtgagcaggatttccgtcacttcttcgctattggcatcggcaggggccggtatcgtcaacaccacgcgcgtgaccgagtcagagagcgaccagttgataaactgctcggtaataaacgccttgttcggcacgattatctctttacggtcccagtcgctgatggtggtggcgcgggtgttaattttcgtcacgctaccggtgagatcgcgaattgtcaccgtatcgccaatgcgaatcggtttttcgaacaggataatcagaccagagataaagttggcgaaaatttcctgcaaaccaaaaccgagaccaacaccgagcgcggcaaccagccactgcaatttcgaccactcaataccaatcattgagaagccgaccagcccgccaatcagcatcagcagatatttggtgatggtggtgatggcgtaacccgtacccggcgttaaatccaggtgctgcaaaatcgccagttccagcagcgcgggcaagttgcgcaccagctgcgtggtgatgataaacaccagaatggcaatcagcaccgcaccgagggtaattggctccagactttctacgccctgtaccgtggaggtgacatcccacagcgaaatattttcgaggaagccgaaagcggaatggatttctgaccacagcacaatgacagaaagcagggcgatcaacatcaaaattgagcgcaccagccgcaaggattgcgcactgatggcatcgagatcgacttcgctttcatcgacttcaattgctccttccgggctactgtgatgatgcgcttcctcttcgccacgcgcacgttgcgctaacatctctgcccggcgatgcttcgcccgatcaaacgccagcctgcggcgctggatcagcatccagcggcggataacgtgataaaccaccagtagcaggaaccagatggcaaccgaggtttcaagcctcgctaacagcgcctgtgccgttgccagataacccaccgccgacgccagaatggcaaccaacggcgcgccaatcatcatgttccacagcatatggttggtaatgttgtcgccgctgccctctttgttgagatacagcggaatcccggcctttttcaggctgagggtgaccaccgccagcgcaccgcaaatgaggataaagcaaagccgtcccagcgaaccggagaattcacggtcgtcgaggttatcgaacatcatcagcgccataatcagcggcacaataagcccgatgctcatcaggtagtagcgcatcccacgggaaacacgttcgcgcggccagccaaaatgagcgataaacaagccgttcgggcgggcaaaggtggcgcaaatcatcactacccacagcagcggcacggtggccgttacaccatcgccaatcgcgaccgccagcggataaggccacgcctcgcgcaagccgtaacccagcgtcatccacagcaccggtaacggtgacgcgacgagaatcgaccagaaaagagtgcgcaacgtcagccagaagtgatcctgagtcactttgccaactttcgccgccgaacgttcaagaaaacgggtgaaatagcggcgcgagtaaatactgcaaccgaccagaatcaacgcgccaaacagcggcaaaattgtctctttgctggtcagcatcatcacactggctttgcccaactgactgaaggtgtccagcgaaatgagacgacgcagatcctgggcgatttccagcggccaggcgatggtcatcgggcgcacgtcagaggtccagaacagatagcggtgcgttgcttcgttcacctctttcagcgcatcctccagttgcccgttggagactttcagcttggtcagttccaatagtagcgtgtcgccaccctgcaacaatgagttcagcaactcacgctgagtgcgcagttgtgcttccagaatacggttttgctcggcagtcagcggctgaccgtcggcctgatgaatttgccgtagcagcggctgtttattaagcagatcctcataacgtaaccgttgcacacgcaactgcgccatttcggtatcaagctgttgtggtttcggcatttccggcagccgtgccacctgcgcccgcagcgcttcgccgagcagattggacgatcccagccattgcgactgttcacgcagcgtattcaacgcctgccggacctgtaacgtctggctggcagcctgacgctgttgcgaggcaacgagatccatccgctgcgcctgttgattcaaagccgccgatagttcgcggttaattttgaattgcgcgacgatatctttcggcaaatcggcgctgttttctgccagcaattcggtactttccagcgcccgctccgcctcaagctgacgttggctgtttaattgattacgcaaggcctgcaaatacgcatccagttgctggctctctttttccgccagctctgagcgtaagcgcgctaattcctggcggttattggcagacagctgcgccagctccagttcatcaacgagcgccttaagacgtgcagagtcagactgcaacgcgaaattttgtgcctgattgagcggagtattgccggtaagcgttcccaggcggcgctcgatctcatttaactgacggcgggcgtcggtttgctgttgcggcagttgattcagcgaatcggcaatctcgcgggcgcgctcctgctcttgctgggcctgacggcttttatccagcaactggctgctgacctggagaatttcctgattcagcgcgtcggtagacattcccggcgacacgctgcgcggctcgtcacgcatgttgtttaattgtgcgcgcagagtagcggagagtttcggataattatcgataacttgctgatattgtttgatgcgctcaagggaaccttttcgttcctcaagcgcatttaaggcagactggagcgcctctacgacttccggctgtgcgggtttcgccgcttttgcctgctccagttcctgagtgatttgtttgctatcgggggccgtcgcggcgtacgccccccaactgaggcaccaggccatcagaaaagtgataatcaggcgcacgtcagcgtttcctttgatggattagacctggtcttttttgtcgtcaaccaatgggctggcgtcgtgttctgcttcgatctcttcagcaggaagcggggcaggttcagcgtctggcgtaacaaaggtttcggtagatactgccagcggctggccaattttcgtgacagacaggctttccagttgctcaaccagattcactttacccggtgcaaacaggttgataacggtggaaccgagtttaaagcgacccatttcctggcctttcagcagtgccacagaaccgtcgttttccccggcaggccaggtccagcgcttgatgataccttcgcgcggcggcgtaatggtgcccgcccagaccgtctcaatgctgccaacaatcgtcgctccgaccagaatctgcgccattgggccaaattcggtatcgaaaaggcaaatcacgcgttcgttacgggcaaacagattcggcacgttctgagccgtgagatggttaacggagaagagatcgcccggcacgtagatcatctcacgcagaataccgttgcacggcatgtgtacgcggtggtagtcacgcggggagaggtaagtggtcacaaacgtaccgttgcggaacaggtccgccatcagatagttgcctgccagcagggcttcgaggctgtagttgtggcctttggcttgcaggattttatcttcttcgattttacccaactggctgataacgccatcggcaggcatgaccagtacattcggatcggtatcgattgggcgtacttcgtcacgcagcggacggacaaagaattcgttaaaggtgcggtagctggcggtgtccggcttttgcgcctctttcatgtcgaccttgtagtatttaacgaacagatcgataaccagttttgtcagccatcctgcccgcttgcttgcgccccaacccgccaggcgagtaagccatagtttcggcagaatgtactgtagcgaaagtttaaatgaatttaacaaggtagcctccaggccattgttttgtcgttcctgatccggcctacatgccggatcctgaaaaaaaggggacgattctaacgacggttagcttaattgtcagtcatccgtatcagaaaagtttttacgcgtttttacctgcgccatgctttccagaatacggtgatagttttcgaaacgggtttccgcgattttcccttcctcaaccgcttcccggatagcgcagcccggatcggtatcgtgtttgcaatcgcgatatttacacagacctaaatagtcatggaattcgacaaagccctgagtgatttgttccggctccaggtgccagaggccgaactcacgcactcctggggagtcaatcacatcaccgccgtgcgggaagtgatacagccgagcggcggtcgtggtgtgctgaccgagccccgagttgtcagagatatcgttggtcaggatctctttttgcagccccagcaacgcattcagcaggctggatttgccgacgccagactgcccggcaaaaatgctgatgcgcccggtcaacgcctcttccagcggttttagcccatcctgagtatggctggaaaccatcaatacgcgataaccgatattgcggtagatatccatctgctcgttgacgaacgccatgccttcgtcgtccagcaggtctatcttgttgagcacaataatcggctcaatctgcaaggtttcgcaggccaccaggtaacggtcgataatattgagcgacagctccggcaaaatggcggagacaatgacaatctggtcgatgttggcggcaataggttttacgccgtcgtagaaatccggacgcgtcaacaccgaggtacgctcatgcaccgcttccacgatccctttgacatttacgccttccgccgccggtttacccggacgccagactacgcggtcgccggttaccagcgaacggatggtacggcgaatattgcagcggtgaacgtcgccatcggcggattccacatcagcgtgcataccaaagcggctgatgacgataccttcatcaggctcgccaaacagattgtcgtcgtagtcgggcttctccttagacgttttaagacgacgctggtgattggcgttcacgcggcgctgctggcctttggagagtttatttttactcaatcgtacagactcctggtcgcccctgatgggcaaaacatctatgatacacgcaattgtggatcaatatagtcactgtgaatgggtggaaaatagcatgagtgccaatgaaaacaacctgatttggatcgatcttgagatgaccggtctggatcccgagcgcgatcgcattattgagattgccacgctggtgaccgatgccaacctgaatattctggcagaagggccgaccattgcagtacaccagtctgatgaacagctggcgctgatggatgactggaacgtgcgcacccataccgccagcgggctggtagagcgcgtgaaagcgagcacgatgggcgatcgggaagctgaactggcaacgctcgaatttttaaaacagtgggtgcctgcgggaaaatcgccgatttgcggtaacagcatcggtcaggaccgtcgtttcctgtttaaatacatgccggagctggaagcctacttccactaccgttatctcgatgtcagcaccctgaaagagctggcgcgccgctggaagccggaaattctggatggttttaccaagcaggggacgcatcaggcgatggatgatatccgtgaatcggtggcggagctggcttactaccgcgagcattttatcaagctgtaaaatttttcctggtcacgtaagcgccggaatccacttgcggcggcgtgattttgacgctaaattgaacgtcttgctgataatttcagcacttgagataaaaacgcaaaaaaaacttttttggggggttgcagagggaaagatttctcgtataatgcgcctcccgtaacgacgcagaaatgcgaaaattacgaaagcaaaattaagtagtacgcgggaatagctcagttggtagagcacgaccttgccaaggtcggggtcgcgagttcgagtctcgtttcccgctccaaaatttgaaaagtgctgcaaagcacagaccacccaagcgggaatagctcagttggtagagcacgaccttgccaaggtcggggtcgcgagttcgagtctcgtttcccgctccaaaatttgaaagtgctgtaaggcacagaccacccaagcgggaatagctcagttggtagagcacgaccttgccaaggtcggggtcgcgagttcgagtctcgtttcccgctccaaattcttctctcaataaaatatccacagcgacgcgatgcgttattgctggtttttgttgtctctgacaaactcttgtaaacagagttatccacagcctcaggctgtaatcttaatttcaaagaaacttcgcacggtgaatagtatttttttaacctattgatagataagttaaaaattaagattccgttttgtcgagtcgatcacttgacgattttattcgtcttgaattgcaatgcgtttttatttttattcacaagctgtggatgaatcaggcgtcacgcggtaaccctttttcaatcacccgaaccagacgctgttttttcggcaattgcacttcgactatgcacgcatttcgtctctctatttgctgcgcaatcgcccacgctatgtgctcatcgagaagtgggtgctcacctttacgactttccagcgctgtcaaaatcgtttcatcccaaggggcattgcctaatgctacggcgatattacgcagccaacgcaggtgaccaatacgacgaatcgccgatccttccgtgacttttaaaaacttctcttcgctccaggcgaataactcaatgagttccggtgcgtgtagcggcttacgcgggctgaaatcctcttctgtggtgagttgtgaatagcgattccacgggcagataagctggcagtcatcgcaaccgtaaatacggtttcccattaacggtcgcaactcttccgggatcgccccttcaagttcgatggtgagataagagatacagcggcgagcatcgacggtatatggctcgacgatggcaccggtcgggcaaatcgtcatacaggccacgcatttgccgcatccttcctcgactggttgatccacgggcagcggaatatcgaccagcaattcgcctaaaaagaagaacgaaccggcctcgcgattgaggataagtgagtgcttacctgtccagccgagcccagctttttcagctaacgggcgctcgagaataggcgcagaatcgacaaacggtctaaaattcagcgaaacacaatgttgctgaatcatctcgcccagctttttgagtcggttgcgcagaagtttgtgatagtcacggcccagcgcataacggctaacatagccgagtttggggtttttcagcgtgctggcaaatgcggcgttagcaggaaggtaattcatccgcacgctgatcacgcgcagcgtaccgggcaataactcatgagggcgagcgcgcagcataccgtgacgtgccatccagtccatttcgccgtggtattgtttgtccagccatgcttgcagtttgggctcggactcgctgagatcggtatcggtaatacctacctgctgaaagcccagttccagcccccactgtttaattttttgcgctaactgattgagatcgaggggctctgacatgacggaccatacaatgaagaaaaaccccgtaagtataccacacaccgtctggtacgccgacgatatccgccgcggagaacgcgaggcggcagatgtgctggggctcacactctatgagctgatgcttcgcgctggcgaggccgcattccaggtgtgtcgttcggcgtatcctgacgcccgccactggctggtgctgtgcggtcatggtaataacggcggcgatggctacgtggtcgcgcgactggccaaagcggtcggcattgaggtcacgttgttggcccaggagagcgacaaaccgttgccggaagaggccgcgctggcacgcgaagcatggttaaacgcgggtggcgagatccatgcttcgaatattgtctggcccgaatcggtagatctgattgttgatgcgctgctcggtaccggtttgcggcaagcgccccgcgaatccattagccagttaatcgaccacgctaattcccatcctgcgccgattgtggcggttgatatcccttccggcctgctggctgaaactggcgctacgccaggcgcggtgatcaacgccgatcacaccatcacttttattgcgctgaaaccaggcttgctcactggaaaagcgcgggatgttaccggacaactgcattttgactcactggggctggatagttggctggcaggtcaggagacgaaaattcagcggttttcagcagaacaactttctcactggctaaaaccgcgtcgcccgacttcgcataaaggcgatcacgggcggctggtaattatcggtggcgatcacggcacggcgggggctattcgtatgacgggggaagcggcgctgcgtgctggtgctggtttagtccgagtactgacccgcagtgaaaacattgcgccgctgctgactgcacgaccggaattgatggtgcatgaactgacgatggactctcttaccgaaagcctggaatgggccgatgtggtggtgattggtcccggtctgggccagcaagagtgggggaaaaaagcactgcaaaaagttgagaattttcgcaaaccgatgttgtgggatgccgatgcattgaacctgctggcaatcaatcccgataagcgtcacaatcgcgtgatcacgccgcatcctggcgaggccgcacggttgttaggctgttccgtcgctgaaattgaaagtgaccgcttacattgcgccaaacgtctggtacaacgttatggcggcgtagcggtgctgaaaggtgccggaaccgtggtcgccgcccatcctgacgctttaggcattattgatgccggaaatgcaggcatggcgagcggcggcatgggcgatgtgctctctggtattattggcgcattgcttgggcaaaaactgtcgccgtatgatgcagcctgtgcaggctgtgtcgcgcacggtgcggcagctgacgtactggcggcgcgttttggaacgcgcgggatgctggcaaccgatctcttttccacgctacagcgtattgttaacccggaagtgactgataaaaaccatgatgaatcgagtaattccgctccctgatgagcaggcaacattagacctgggcgagcgggtagcgaaagcctgcgatggcgcaaccgtaatctatctgtatggcgatttaggcgcaggtaaaaccacctttagccggggctttttacaggctctgggtcatcagggtaatgtcaaaagccccacttatacgctggtcgaaccctatacgctcgacaacttaatggtctatcactttgatttgtaccgccttgccgatcccgaggagctggagtttatggggatccgcgattattttgccaacgatgccatctgcctggtggagtggccacaacaaggtacaggtgttcttcctgacccggatgtcgaaatacacattgattatcaggcacaaggccgtgaggcgcgcgtgagtgcggtttcctctgcgggtgaattgttgctggcgcgtttagccggttaacctttgaaaggtggcgggatgatgtatcgcatcagaaattggttggtagcgacgctgctgctgctgtgcacgccggtgggtgccgcgacgctctctgatattcaggtttctaacggtaatcaacaggcgcggataacgttgagttttattggcgatcctgattatgcgtttagccatcaaagcaaacgcaccgtggcgctcgatatcaaacaaacgggcgtgattcagggactgccgttgttgttcagcggcaataatctggtgaaggcgattcgctctggaacgcctaaagatgcacaaacgctacggctggtggtcgatcttaccgaaaacggtaaaaccgaagcggtgaagcggcagaatggcagcaattacactgtcgtctttacgattaacgccgatgtgccgccaccgcctcctccgccgcccgtggttgcgaaacgcgttgaaacgcctgcggttgtcgcaccgcgcgtcagcgaaccggcgcgcaatccgtttaaaacggaaagtaaccgcactacgggtgttatcagcagtaatacggtaacgcgtccggcagcgcgcgcgacggctaacactggcgataaaattatcatcgctattgatgccggacacggcggtcaggaccctggcgctatcggccccggtggtacgcgggagaaaaatgtcaccatcgccatcgcgcgtaaattgcgtactttgctcaatgacgatccgatgtttaaaggcgttttaacccgtgacggggattactttatctcggtgatggggcgcagtgatgtggcacgtaagcaaaacgccaatttcctcgtgtcgattcacgctgatgccgcaccgaaccgcagtgcgactggcgcttccgtatgggtgctctctaaccgtcgcgccaacagtgaaatggccagctggctggagcagcacgagaaacagtcggagctgctgggtggggcgggtgatgtgctggcgaacagtcagtctgacccctatttaagccaggcggtgctggatttacagttcggtcattcccagcgggtagggtatgatgtagcgaccagtatgatcagtcagttgcaacgcattggcgaaatacataaacgtcgaccagaacacgccagccttggcgttctgcgctcgccggatatcccatcagtactggtcgaaaccggttttatcagcaacaacagcgaagaacgtttgctggcgagcgacgattaccaacaacagctggcagaagccatttacaaaggcctgcgcaattacttccttgcgcatccgatgcaatctgcgccgcagggtgcaacggcacaaactgccagtacggtgacgacgccagatcgcacgctgccaaactaaggacgattgatgccaattcaggtcttaccgccacaactggcgaaccagattgccgcaggtgaggtggtcgagcgacctgcgtcggtagtcaaagaactagtggaaaacagcctcgatgcaggtgcgacgcgtatcgatattgatatcgaacgcggtggggcgaaacttatccgcattcgtgataacggctgcggtatcaaaaaagatgagctggcgctggcgctggctcgtcatgccaccagtaaaatcgcctctctggacgatctcgaagccattatcagcctgggctttcgcggtgaggcgctggcgagtatcagttcggtttcccgcctgacgctcacttcacgcaccgcagaacagcaggaagcctggcaggcctatgccgaagggcgcgatatgaacgtgacggtaaaaccggcggcgcatcctgtggggacgacgctggaggtgctggatctgttctacaacaccccggcgcggcgcaaattcctgcgcaccgagaaaaccgaatttaaccacattgatgagatcatccgccgcattgcgctggcgcgtttcgacgtcacgatcaacctgtcgcataacggtaaaattgtgcgtcagtaccgcgcagtgccggaaggcgggcaaaaagaacggcgcttaggcgcgatttgcggcaccgcttttcttgaacaagcgctggcgattgaatggcaacacggcgatctcacgctacgcggctgggtggccgatccaaatcacaccacgcccgcactggcagaaattcagtattgctacgtgaacggtcgcatgatgcgcgatcgcctgatcaatcacgcgatccgccaggcctgcgaagacaaactgggggccgatcagcaaccggcatttgtgttgtatctggagatcgacccacatcaggtggacgtcaacgtgcaccccgccaaacacgaagtgcgtttccatcagtcgcgtctggtgcatgattttatctatcagggcgtgctgagcgtgctacaacagcaactggaaacgccgctaccgctggacgatgaaccccaacctgcaccgcgttccattccggaaaaccgcgtggcggcggggcgcaatcactttgcagaaccggcagctcgtgagccggtagctccgcgctacactcctgcgccagcatcaggcagtcgtccggctgccccctggccgaatgcgcagccaggctaccagaaacagcaaggtgaagtgtatcgccagcttttgcaaacgcccgcgccgatgcaaaaattaaaagcgccggaaccgcaggaacctgcacttgcggcgaacagtcagagttttggtcgggtactgactatcgtccattccgactgtgcgttgctggagcgcgacggcaacatttcacttttatccttgccagtggcagaacgttggctgcgtcaggcacaattgacgccgggtgaagcgcccgtttgcgcccagccgctgctgattccgttgcggctaaaagtttctgccgaagaaaaatcggcattagaaaaagcgcagtctgccctggcggaattgggtattgatttccagtcagatgcacagcatgtgaccatcagggcagtgcctttacccttacgccaacaaaatttacaaatcttgattcctgaactgataggctacctggcgaagcagtccgtattcgaacctggcaatattgcgcagtggattgcacgaaatctgatgagcgaacatgcgcagtggtcaatggcacaggccataaccctgctggcggacgtggaacggttatgtccgcaacttgtgaaaacgccgccgggtggtctgttacaatctgttgatttacatccggcgataaaagccctgaaagatgagtgatatcagtaaggcgagcctgcctaaggcgatttttttgatggggccgacggcctccggtaaaacggcgttagccattgagctgcgtaaaattttaccagtagagttgataagcgttgattctgcccttatttacaaagggatggatatcgggacggcgaagccgaacgctgaagagttactcgccgcgccgcaccgattgctggatattcgcgatccgtcgcaggcttactcggctgctgattttcgccgcgatgcgctggcggaaatggccgatatcaccgcggcggggcggatcccactgttagtgggcggtacgatgttgtatttcaaggcattgctggaagggttgtcgccgctaccgtcggcagacccggaagtacgggccagaattgagcaacaggcggcagagcaaggttgggagtcattgcatcgtcaacttcaggaggtagatccggttgcggcagcaaggattcatccaaatgatccacaaaggctttcccgggcactggaagtttttttcatttcgggtaaaactttaacggaactgacgcaaacgtcaggagacgctctaccgtatcaggtgcatcagttcgccatcgccccggcgagccgtgaactgctccatcaacgcattgagcagcgttttcatcagatgttggcttcaggttttgaagcagaagtccgggcgctttttgcccgaggagatttgcatacggacttgccttccattcgttgcgtgggttatcgccagatgtggtcttaccttgaaggcgaaatctcatacgatgaaatggtttatcgaggtgtttgcgccacgagacagttggcgaagcggcagataacctggctgcgtggttgggaaggggttcactggcttgacagtgaaaaaccagaacaggcgcgtgacgaagtattacaggttgttggtgctatcgcaggctgaatgtgtacaattgagacgtatcgtgcgcaattttttcagaatcgaaaggttcaaagtacaaataagcatataaggaaaagagagaatggctaaggggcaatctttacaagatccgttcctgaacgcactgcgtcgggaacgtgttccagtttctatttatttggtgaatggtattaagctgcaagggcaaatcgagtcttttgatcagttcgtgatcctgttgaaaaacacggtcagccagatggtttacaagcacgcgatttctactgttgtcccgtctcgcccggtttctcatcacagtaacaacgccggtggcggtaccagcagtaactaccatcatggtagcagcgcgcagaatacttccgcgcaacaggacagcgaagaaaccgaataaggtttcgggctgtttttttacacggggagccagcgatcctgcgttccccgctgatctatttagagggttatacgcttgtttgaccgttatgatgctggtgagcaggcggtactggtacacatctattttacgcaagacaaagatatggaagacctccaggagtttgaatctctggtctcttccgccggtgtcgaagcattgcaggtgattaccggtagccgtaaagcgccgcacccaaagtattttgtaggtgaaggtaaagcagttgaaattgcggaagctgtcaaagcgacgggtgcttcggtcgttctttttgaccatgccctgagcccggcgcaagagcgtaacctggagcgtttgtgcgagtgtcgtgttatcgaccgcaccggccttattttagatattttcgcccaacgtgcgcgtacccatgagggtaagttgcaggttgagctggcgcagctgcgccatctggctacgcgcctggtgcgtggctggacccaccttgaaagacagaaaggcgggataggtttgcgtggtccgggtgaaacccagctcgaaaccgaccgtcgtttgttgcgtaatcgcatcgtgcagatacagtcgcgcctggaaagagttgaaaagcagcgtgagcaggggcggcaatcgcgtatcaaagccgacgttcctactgtttcgctggtgggatataccaacgccggtaaatctacccttttcaatcgcatcaccgaagcgcgggtctacgcggcagaccagttgtttgccaccctcgacccgacgttgcggcgtattgacgttgcagatgtcggtgaaaccgtacttgcagataccgtagggtttattcgccacctgccgcacgatctggtggcggcatttaaagccacgttacaagagacgcggcaagccacattactgctgcacgtcattgatgcggcggatgtgcgtgtacaagaaaacatcgaagcggtgaatacggttcttgaagagatcgacgctcacgagatcccaaccctgctggtgatgaacaagatcgatatgctggaagatttcgaaccgcgtattgatcgggacgaagagaacaaaccgaaccgtgtctggctttccgcacagaccggagcggggataccacagctttttcaggctttgacggagcggctttccggcgaggtggcgcagcatacattgcgtctgccaccgcaggaagggcgtctgagaagtcgtttttatcagcttcaggcaatagaaaaagagtggatggaggaggacggcagcgtaagtctgcaagttcgtatgccgatcgttgactggcgtcgcctctgtaaacaagaaccggcgttgatcgattacctgatctaacggcgtagcgtctgaagcgtggagtcatatcctctggcgtcgaaagacaacagggatcaccgcataacaaatatggagcacaaacatggcgtggaatcagcccggtaataacggacaagaccgcgacccgtggggaagcagcaaacctggcggcaactctgagggaaatggaaacaaaggcggtcgcgatcaagggccacctgatttagatgatatcttccgcaaactgagcaaaaagctcggtggtctgggcggcggtaaaggcaccggatctggcggtggcagttcatcgcaaggcccgcgcccgcagcttggcggtcgtgtcgttaccatcgcagcggcagcgattgtcattatctgggcggccagtggtttctataccattaaagaagccgaacgcggcgtggtaacacgctttggtaaattcagccatctggttgagccgggtctgaactggaaaccgacgtttatcgacgaagtcaaaccggtgaacgtggaagccgtgcgtgaactggccgcttctggtgtgatgctgacgtcggacgagaacgtagtgcgcgttgagatgaacgtgcagtaccgcgtcaccaatccggaaaaatatctgtatagcgtgaccagcccggatgacagcctgcgtcaggctaccgacagcgccctgcgtggagttatcggtaaatacaccatggaccgcattctgacggaaggtcgtaccgtgattcgtagcgatactcagcgcgaactggaagagacgattcgtccgtatgacatgggtatcacgctgctggacgtcaacttccaggctgctcgtccgccggaagaagtaaaagcggcgtttgacgatgcgattgccgcgcgtgaaaacgaacagcaatacattcgtgaagcagaagcgtataccaacgaagttcagccgcgtgcgaacggtcaggcgcaacgtatcctcgaagaggcgcgtgcgtacaaggcccagaccatcctggaagctcagggtgaagtggcgcgctttgctaaacttctgccggaatataaagccgcgccggaaattactcgcgagcgtctgtatatcgagacgatggaaaaagtgttgggtaacacccgcaaagtgctggttaacgataaaggtggcaacctgatggttctgccgttagaccagatgctgaaaggtggtaacgcccctgcggcgaagagcgataacggtgccagcaatctgctgcgtctgccgccagcctcttcctccacaaccagtggagcaagcaacacgtcgtccaccagtcagggcgatattatggaccaacgccgcgccaacgcgcagcgtaacgactaccagcgtcagggggaataacgatgcgtaagtcagttatcgcgattatcatcatcgtgctggtagtgctttacatgtctgtctttgtcgtcaaagaaggtgagcgcggtattacgctgcgttttggtaaggtactgcgtgacgatgacaacaaacctctggtttatgagccgggtctgcatttcaagataccgttcattgaaacggtgaaaatgctcgacgcacgtattcagaccatggacaaccaggccgaccgctttgtgaccaaagagaagaaagacctgatcgtcgactcttacatcaaatggcgcatcagcgatttcagccgttactacctggcaacgggtggtggcgacatttcgcaagcggaagtgctgttgaaacgtaagttctctgaccgtctgcgttctgaaattggtcgcctggacgtgaaagatatcgtcaccgattcccgtggtcgtctgaccctcgaagtacgtgacgcgctgaactccggttctgcgggtacagaagatgaagttactaccccggcggcagataacgccattgccgaagcggcagagcgcgtaacggctgagacgaagggcaaagttccggtcatcaacccgaacagtatggcggcgctgggtattgaagttgtcgatgtgcgtatcaagcagatcaacctgccgaccgaagtgtctgaagcgatctacaaccgtatgcgcgccgagcgtgaagcggtagcgcgtcgtcaccgttcacaaggtcaggaagaagcggaaaaactgcgcgcgactgccgactatgaagtgaccagaacgctggcagaagctgagcgtcagggccgcatcatgcgtggtgaaggcgatgccgaagcagccaaactgtttgctgatgcattcagtaaagatccggacttctacgcattcatccgtagcctgcgtgcttatgagaacagcttctctggcaatcaggacgtgatggtcatgagcccggatagcgatttcttccgctacatgaagacgccgacttccgcaacgcgttaatataacgactgcggtacaggtcaataaagccaccgcatcctcagggatgtcggtggttttctttttctataaggataatgaatgaattcgacaatctggctggcgcttgccctggttttggtactggaaggtttagggccgatgctttacccgaaggcatggaagaagatgatctctgcgatgaccaatttgcccgataatattttacgtcgttttggcggtggacttgtggttgcgggcgttgtggtctactacatgttgaggaaaacgattggctgaacaaaaaacagactgatcgaggtcatttttgagtgcaaaaagtgctgtaactctgaaaaagcgatggtagaatccatttttaagcaaacggtgattttgaaaaatgggtaacaacgtcgtcgtactgggcacccaatggggtgacgaaggtaaaggtaagatcgtcgatcttctgactgaacgggctaaatatgttgtacgctaccagggcggtcacaacgcaggccatactctcgtaatcaacggtgaaaaaaccgttctccatcttattccatcaggtattctccgcgagaatgtaaccagcatcatcggtaacggtgttgtgctgtctccggccgcgctgatgaaagagatgaaagaactggaagaccgtggcatccccgttcgtgagcgtctgctgctgtctgaagcatgtccgctgatccttgattatcacgttgcgctggataacgcgcgtgagaaagcgcgtggcgcgaaagcgatcggcaccaccggtcgtggtatcgggcctgcttatgaagataaagtagcacgtcgcggtctgcgtgttggcgaccttttcgacaaagaaaccttcgctgaaaaactgaaagaagtgatggaatatcacaacttccagttggttaactactacaaagctgaagcggttgattaccagaaagttctggatgatacgatggctgttgccgacatcctgacttctatggtggttgacgtttctgacctgctcgaccaggcgcgtcagcgtggcgatttcgtcatgtttgaaggtgcgcagggtacgctgctggatatcgaccacggtacttatccgtacgtaacttcttccaacaccactgctggtggcgtggcgaccggttccggcctgggcccgcgttatgttgattacgttctgggtatcctcaaagcttactccactcgtgtaggtgcaggtccgttcccgaccgaactgtttgatgaaactggcgagttcctctgcaagcagggtaacgaattcggcgcaactacggggcgtcgtcgtcgtaccggctggctggacaccgttgccgttcgtcgtgcggtacagctgaactccctgtctggcttctgcctgactaaactggacgttctggatggcctgaaagaggttaaactctgcgtggcttaccgtatgccggatggtcgcgaagtgactaccactccgctggcagctgacgactggaaaggtgtagagccgatttacgaaaccatgccgggctggtctgaatccaccttcggcgtgaaagatcgtagcggcctgccgcaggcggcgctgaactatatcaagcgtattgaagagctgactggtgtgccgatcgatatcatctctaccggtccggatcgtactgaaaccatgattctgcgcgacccgttcgacgcgtaattctggtacgcctggcagatattttgcctgccgggcgaacagtgtgatacattgctgtgtcgggtaagccattacgctatccgacacagtgttaaatcctcgcttttttccttccccgaactgaaataaattagcgacacagcttgtggctggtttatcatcaatataaatgtattttttcccgatttcccttttgaggttgatgtgcagttaacgagtttcactgattacggattacgtgcgctgatctacatggcgtcattgccagaagggcggatgaccagtatttctgaagtgactgacgtctacggcgtctcccgtaatcatatggtcaaaataatcaatcaacttagtcgtgccggctacgtgactgctgttcgtggaaaaaatggcggcattcgcctgggtaaaccggcgagtgcgatacgtattggtgatgtggtgcgcgagctggagcccttatcgctggtgaattgcagcagtgagttttgccacattacacctgcctgtaggttgaaacaggcactttctaaggccgtgcaaagttttcttacggaactggataactacacgcttgccgatttggttgaagagaatcaaccgctttataaattattgctggtggagtgacgaaaatcttcatcagagatgacaacggaggaaccgagatgtcacaagatcctttccaggaacgcgaagctgaaaaatacgcgaatcccatccctagtcgggaatttatcctcgaacatttaaccaaacgtgaaaaaccggccagccgtgatgagctggcggtagaactgcacattgaaggcgaagagcagcttgaaggcctgcgtcgccgcctgcgcgcgatggagcgcgatggtcaactggtcttcactcgtcgtcagtgctatgcgctgccggaacgcctcgacctggtgaaaggtaccgttattggccaccgtgatggctacggctttctgcgggttgaagggcgtaaagatgatttgtatctctccagcgagcagatgaaaacctgcattcatggcgatcaggtgctggctcagccgctgggtgctgaccgtaaaggtcgtcgtgaagcgcgtattgtccgcgtactggtgccaaaaaccagccagattgttggtcgctactttaccgaagcgggcgtcggctttgtggttcctgacgacagccgtctgagcttcgatatcttaatcccgcccgatcagatcatgggcgcgcggatgggctttgtggtcgtagtcgaactgactcagcgtccgactcgccgcaccaaagcggtgggtaaaatcgtcgaagtgctgggcgacaatatgggcaccggcatggcggttgatatcgctctgcgtacccatgaaattccgtacatctggccgcaggctgttgagcaacaggttgccgggctgaaagaagaagtgccggaagaagcaaaagcgggccgtgttgatctgcgcgatttaccgctggtcaccattgatggcgaagacgcccgtgactttgacgatgcagtttactgcgagaaaaaacgcggcggcggctggcgtttatgggtcgcgattgccgacgtcagctactatgtgcgtccgtcaacgccgctggacagagaagcgcgtaaccgtggcacgtcggtgtacttcccttcgcaggttatcccgatgctgccggaagtgctctctaacggcctgtgttcgctcaacccgcaggtagaccgcctgtgtatggtgtgcgagatgacggtttcgtcgaaaggccgcctgacgggctacaaattctacgaagcggtgatgagctctcacgcgcgtctgacctacaccaaagtctggcatattctgcagggcgatcaggatctgcgcgagcagtacgccccgctggttaagcatctcgaagagttgcataacctctataaagtgctggataaagcccgtgaagaacgcggtgggatctcatttgagagcgaagaagcgaagttcattttcaacgctgaacgccgtattgaacgtatcgaacagacccagcgtaacgacgcgcacaaattaattgaagagtgcatgattctggcgaatatctcggcggcgcgtttcgttgagaaagcgaaagaaccggcactgttccgtattcacgacaagccgagcaccgaagcgattacctctttccgttcagtgctggcggagctggggctggaactgccgggcggtaacaagccggaaccgcgtgactacgcggagctgctggagtcggttgccgatcgtcctgatgcagaaatgctgcaaaccatgctgctgcgctcgatgaaacaggcgatttacgatccagaaaaccgtggtcactttggcctggcattgcagtcctatgcgcactttacttcgccgattcgtcgttatccagacctgacgctgcaccgcgccattaaatatctgctggcgaaagagcaggggcatcagggcaacaccactgaaaccggcggctaccattattcgatggaagagatgctgcaactgggtcagcactgttcgatggcggaacgtcgtgccgacgaagcaacgcgcgatgtggctgactggctgaagtgtgacttcatgctcgaccaggtaggtaacgtctttaaaggcgtaatttccagcgtcactggctttggcttcttcgtccgtctggacgacttgttcattgatggtctggtccatgtctcttcgctggacaatgactactatcgctttgaccaggtagggcaacgcctgatgggggaatccagcggccagacttatcgcctgggcgatcgcgtggaagttcgcgtcgaagcggttaatatggacgagcgcaaaatcgactttagcctgatctccagcgaacgcgcaccgcgcaacgtcggtaaaacggcgcgcgagaaagcgaaaaaaggcgatgcaggtaaaaaaggcggcaagcgtcgtcaggtcggtaaaaaggtaaactttgagccagacagcgccttccgcggtgagaaaaaaacgaagccgaaagcggcgaagaaagacgcgagaaaagcgaaaaagccatcggcgaaaacgcagaaaatagctgcagcgaccaaagcgaagcgtgcggcgaagaaaaaagtggcagagtgatcaataccctctttaaaagaagagggttagattgctgacaaaatgcgctttgttcatgccggatgcggcgtgaacgccttatccggcctacataatcacgcaaattcaatatattgcagagatcatgtaggccggataaacgtagtgcatcaggcaaaacgtaaacaacgagtacattaatgagcgaaatgatttacggcatccacgcagtgcaggccctgctggagcgcgcccctgaacgttttcaggaagtctttattttaaaaggccgtgaagataaacgtctgttaccgctgattcacgcccttgagtctcagggcgtggttatccagttggcaaaccgccaatatctcgacgagaaaagcgacggtgccgtgcatcagggcattatcgcccgcgtgaagccaggacgtcagtatcaggaaaacgatctgccggatctgatcgcttcgctcgatcaaccgttcctgctgatcctcgacggcgtaaccgatccgcacaacctcggcgcgtgcctgcgtagtgcggacgccgcaggcgttcatgcggtgattgtgccgaaagatcgctccgcacagctcaacgctacggcgaaaaaagtagcctgcggcgcggcagaaagcgttccgctgattcgggtgactaaccttgcgcgcaccatgcgtatgttgcaggaagagaatatctggatcgtcggtacggcaggcgaggcggatcatacactctatcagagcaaaatgaccggacgcctggcgctggtgatgggtgcggaaggtgaaggtatgcgtcgcctgactcgtgaacattgcgatgagttgatcagcatcccgatggctggaagcgtttcttccctgaacgtttcggttgcgaccggaatttgcttatttgaagcggtgcgccagcgcagctaatttctcagaattatgaaaagccatccagatttggatggtttttttttgtctatagctggtaagataattacgtattgcaaatattcattttattaatatttaaacttaatctatatggaataatatatgacatggaatccgttggcgctagcgacggcgctgcaaactgtacctgaacaaaatattgatgtaacaaatagcgagaacgcattaattattaaaatgaatgattatggcgatttgcaaatcaatattctttttacttcccgccaaatgattatcgaaacctttatttgtccggtgagtagtatcagcaatccagatgaatttaataccttcttattaagaaatcagaagatgatgccgttgtcatcggtagggatctccagcgtacaacaggaagagtattacattgttttcggggcgttatcgcttaaatcttctcttgaagatatcctgcttgagataacctcgctggtagataacgcattggatctggctgaaattacagaagaatattcacactaattacaaggacgggtatttatgggaattttaaaaagtttatttacgctggggaaatcgtttatctcccaggcggaagaatccattgaagaaacccagggcgtgcgcatgctggaacagcatattcgtgacgctaaagctgaactcgataaagccggaaaatctcgcgttgatctgctggcgcgggtgaaattaagtcacgataagctgaaagatttacgtgagcgcaaagccagtctggaagcccgtgcgctggaagcgttaagcaagaacgttaatccgtcgttgattaacgaagttgctgaagaaatcgcgcgccttgagaatctcattaccgctgaagagcaagtgttgtcgaatctggaagtctcccgtgatggcgtggaaaaagcagttacagcgacagcgcagcgtatcgctcagtttgagcagcaaatggaagtcgttaaagccactgaagccatgcagcgtgcacaacaggctgtaacaacctctaccgttggcgcatcttccagcgtttcgacagcggcagaatccttaaaacgcctgcaaacgcgtcaggccgaacgtcaggctcgcctggatgctgccgcacagttggagaaagtcgcagacggtcgcgaccttgacgaaaagctggcggaagccggaattggcggtagcaataaaagtagcgcccaggatgtattagcaagactgcaacgccaacagggcgagtaatttttttgccagcctcgctaaaaggctggcaactattttaaggataaaatatgtctggttttttccagcgtctgtttggcaaggataataagccagctatcgctcgtggtccgctgggacttcatctcaatagtggctttacgctcgacacgttagcgtttcgtttgctggaagatgaattgctgattgcgctgccgggtgaggaatttacggtagccgccgtcagccacatcgatctgggcggcggtagtcagattttccgctactacacttcaggcgatgagtttctgcaaatcaataccaccggcggcgaagatattgatgacattgatgatatcaagctctttgtctatgaagagagctacggtatcagtaaagagagtcactggcgcgaggcgatcaacgccaaagcgatgggagcaatgaccttaaactggcaggaaaaacgctggcagcgattttttaacagcgaagaaccgggaaatatcgaacccgtctacatgctggaaaaagtagaaaatcaaaaccatgccaaatgggaggtccataattttaccatgggctaccaacggcaagtaaccgaagatacttacgaatatttgctgctaaatggtgaggaatcttttaacgatctcggcgagccagagtggttattttcgcgcgcgttgggtgtcgatatcccgctgacatcacttcatattattggttaattacaaggacgtttacaatgcatatactggattcacttcttgcctttagcgcctatttttttattggcgtggctatggtgattatttttctgtttatctattctaaaattacaccgcacaacgaatggcagttaatcaaaaacaataataccgcggcgtcactggcgttcagcggtacattgttgggttacgttatccccttatccagtgcggcaatcaatgcggtgagtattccagactatttcgcctggggcgggattgcactggtgattcagttactcgtttttgctggtgtcagactttatatgcccgcattaagcgaaaaaattattaatcacaataccgcagcaggaatgtttatgggaaccgccgcgctggctggcggtatttttaacgcagcttgtatgacatggtaatggacgatcatggccagaaaacgcaaatcaagaaataacagtaaaattggtcacggagcgattagtcgcattggtagaccgaataatccttttgaaccgtgccgcaatcgctacgcacaaaaatacttaacgttggcgctaatgggcggtgccgcttttttcgtattgaaaggttgtagcgatagtagcgatgtcgataacgacggcgacggaacgttttacgcgacagtgcaggattgtattgatgacggtaataatgccgacatttgcgcgcgtggctggaacaacgccaaaacggcattttatgccgatgttccgaagaatatgactcagcagaactgtcagtctaagtacgaaaattgctactacgacaatgttgaacagagttggatcccggtcgtttctggatttttgttaagccgggttattcgtaaagatcgcgatgagccgtttgtttataacagcggcggttcctcttttgcttcgcgcccagtctggcgcagcacttctggtgattactcctggcgctccggttctggcaaaaaagagtcttactcttcgggcggctttaccaccaaaaaagcgtctaccgtttctcgcggcggctatggtcgttcttccagcgcccgtgggcattggggaggctaatcatgctgagacacaacgttcctgtgcgacgggatctggaccagatcgccgctgacaacggtttcgactttcatatcatcgacaatgaaatctattgggatgagagtcgggcttaccgttttactctgcgccagattgaagagcagatcgaaaaaccgactgcggaactgcatcagatgtgccttgaggtggtggatcgcgcggtaaaagatgaagagatcctgacgcaactggcgatcccgccgttgtactgggatgtgatcgctgaaagctggcgcgcccgcgatccttcgctgtatggacggatggattttgcctggtgtggcaatgcgccggtgaagctgctggagtacaacgccgatacgccaacttcattgtacgagtcggcttatttccagtggctgtggctggaggatgcccggcgcagcggcattattccgcgtgatgccgatcagtacaatgctattcaggaacgcctgatttcacgctttagcgagctttacagtcgggaaccgttttatttttgctgctgtcaggacaccgatgaagacaggagtaccgtgctgtacttgcaggactgcgcccagcaggcagggcaggagtcgcggtttatctacattgaagatctcggtttgggcgtcggcggcgtactgaccgatcttgatgataatgtcatccagcgtgcatttaagctgtatccgctggagtggatgatgcgtgacgataacggtccgctgctgcgcaagcgtcgcgagcaatgggtggagccgttatggaaaagtatcttgagtaataaagggctaatgccgctgctttggcgcttcttccctggtcatcctaatcttcttgcgtcctggttcgatggcgagaaaccgcagattgccgctggcgaaagctatgtgcgtaaaccaatctattcgcgcgaaggcggcaacgtcaccatttttgacggcaagaataacgttgttgaccacgctgatggtgattacgccgatgaaccgatgatctaccaggcgtttcaacctctgccgcggtttggcgatagctacacactcatcggtagctggattgtcgatgatgaagcgtgcggaatggggatccgtgaagataacacactgatcaccaaagacacctcacgtttcgttccgcattacattgctggataagaatgttttagcaatctctttctgtcatgaatccatggcagtgaccatactaatggtgactgccattgatggagggagacacagtgcactggcaaactcacaccgtttttaatcaacctataccattaaataacagcaacttatacctgtctgatggcgcgctctgcgaagcggtaacgcgtgaaggtgctggctgggatagcgattttctagccagtattggtcagcagttaggaacggctgaatcccttgaactggggcggctggcgaatgtgaatccgcctgaattattgcgctacgatgcgcaaggacgccgtctggacgatgtgcgttttcaccccgcctggcacctgctgatgcaggcgctatgtaccaatcgggtgcacaatcttgcctgggaagaagacgctcgctccggcgcatttgtggcgcgcgcggcgcgttttatgttacatgcgcaggttgaggcagggtcgttatgtccgataaccatgacctttgccgccacgccattgttgttacagatgttacccgcgccgtttcaggactggaccacgccgctattgagcgatcgctacgattctcacttattgccaggtgggcaaaaacgcggtttgttgattggcatgggaatgacggaaaagcagggcggttccgatgttatgagcaacaccacccgtgcagagcgtctggaagatggctcttatcggctggtggggcataaatggtttttctcggttccgcaaagcgatgcgcatctggtgctggcgcagaccgcgggtggtctgtcctgcttttttgtgccgcgctttttgcctgacgggcaacgcaacgcgattcgcctcgagcggctgaaagataagctgggtaatcgctctaacgccagttgcgaagtggagtttcaggatgccattggttggttgttggggctggaaggggaaggaattcgtctgatcctgaaaatgggtgggatgacgcgttttgattgcgccctgggtagccatgccatgatgcgccgtgcattttcgctggcgatttatcatgcacatcaacgccatgtttttggtaatccattgatccaacagccccttatgcgtcatgtcttaagtcgcatggcacttcagcttgaagggcaaacggcgttgctgtttcgtcttgcgcgagcgtgggaccggcgtgccgatgccaaagaagccctgtgggcgcgtttatttacgcctgcggcaaaatttgtgatctgcaaaagaggtatgccgtttgtggccgaagcgatggaggtgctgggcggcattggttattgcgaggagagtgagctgccgcggctttaccgggagatgccggtaaacagtatttgggaaggttccggcaatattatgtgcctggatgtgttgcgcgttctcaataagcaagcgggcgtatacgacttattgtcggaagcatttgtggaagtgaaagggcaggatcgctattttgatcgcgcggttcgtcgtttacagcagcagctgcgtaagccagctgaagaactggggcgagagattactcatcagctattcctgctgggctgcggtgcgcaaatgttgaaatatgcttctccgccaatggcgcaggcgtggtgtcaggtgatgttagatacgcgcggcggcgtacggttgtcagagcagatccagaatgatttattgctgcgggcgacggggggagtgtgtgtgtaagcgtatacgactgatgcgacgctggtttcgattaactaaatgaaatatgtgaaaattgtaggccggacaaggcgctcgcgccgcatccggcattgttcatttgctgtagatgacactcatgcatacagtatcgcctgtacgcgccagttatcaggctgctggtcttcgtacatggtaataatgcggtaccatgacgcaccttgttcatcggcctttaacgccacgatacgttccacgtcctgcggatcccctgaaatattgctaactgagatctgacctatttcattcaggcccgtcacgcagtcagcactggcgaattctgcagactgtgccgtggcgctcgcaggataagtcactaattgcagcgagggtgaggcaagtaattgtttcatcgtcagctccatttttcgtttccccacatgttgcagggcattccatcgcggtaataaacgcccaggcttccagccggtaatttattgtgcacaggtaaacgcatagggacgcaaagcaatgtaaagctgactatgtaagttgtctgatttatttacggtacaaaatggcttgtgaataccactgtcctgtcacgatggtttcgtccaccatgacgacaacgtaataatcagcttttgcagcgacagctttcgctttgatttctgctaatgcgtcatccggagaaccccgaaccatcgtgcttacgctacctattcgctgtaacccttgcgtctggtcgcggcgaatctcttgcggatggtccgttactggcggtgctggctgtggcgtaccttgcagtgcgctacaggcacttaacatcaacaccaataataaactggcaaaccggtaaataacgctattacgtttcctgctaaccatagtgtagtgccttattaatttaactttgggggaatgttcccgaattgttacctggtacgcgattttcgaatgaaaacgtgacgaaagcgtaacccacatctcaacattatgaactaataccgccagcagaaacttgtgctaaggatttcttcatgtcataccagacaaaaaggagagacagatgattgaaatagaatcacgcgagctggcagatattcccgttcttcatgcttatcctgtcgggcaaaaagataccccgttaccgtgcgtaattttttatcacggctttacttcatccagtctggtgtatagctattttgccgttgcgctggcgcaggctggtttgcgggtgatcatgccggatgcgcccgatcacggtagccgttttagtggtgacgcagcgcggcggttaaatcaattctggcaaatcttgctacaaagtatgcaggaattcactactttacgtgcggcaatagccgaagaaaactggctgcttgatgaccgtctggcagtcggtggcgcgtcgatgggcgcgatgacggcactggggattaccgctcgccaccccacggtgagatgtaccgccagcatgatgggatcgggctattttacatcactcgcccgttcactgtttccaccgctgatacctgaaacggcagcacagcagaatgaattcaataacattgtcgcgccactggcagagtgggaagcgacaaaccacctggaacaacttagtgacagacctctactgctgtggcatggcctcgacgatgacgttgtgcctgccgacgaatcactacgtttgcagcaggccttaagcgagacgggacgggataaactgctaacctgttcatggcagccaggcgtgcgtcaccgcattacgcctgaggcgttagatgctgccgtgacatttttccgccagcatctttaaacacgcagaatgctgaccccttgcgcttccagttgttgcaggatttccgggttagcatttttgccggtgataagcatatcgatttgatcggcacggctaaaaagcattcccgcgcgttcgccaatcttactgctatcaaccagtaccaccagtttccctaccacgctcagcatcttctgctctgccattgctgtcagcatatcggttttatacaacccttctgcggtcagcccttttccgctggtaaacatccagtgcccggcatagagactgttttcgctgccctgcgggcttaaagtgatggactgacttttgttgtactgtccgcccataatgatcacgctgtcatgttcttgatcgatcaggtaatttgccagcggtagataattagtgatgatttgcactggcttgccacacatttcccgcccaagcagaaacgcggtggagccgcagttgatgactacgctttcgcccggattaaccagctgcgaggccgctttagcgatacgtactttttcatcgtgattctgcgcctgatgcagattcatcggcgtccagcgcgggcgctgttgggtaatagcttctgcgccattgcgcacttttttcagtttgccgctttcgtcaagtttattgatatcgcgtcgcgcagtggcaggcgaaattcccagacgctcaacgactttctcaacggtcacaaagcccaattgtgcgagcatttccaggaggatttgatgtctttgtgcttcagtcatgagctattccgataaaatttgatttttttagatgatatttgaaatagccaggaaatactacgccggatagcgcgaacttctccacgctacccggtataaacgacagattacaggaatgacttgaacggcagatccggttcaatagtgaagcaatcatcgaaaccgcgcggatagtggtactcgaagttgtctttatccagcggccaggtaaatttgccacccacctgccagataaacggcttgaagccatacttcaggcgatcttttttcatctcccacagcacgcggatctcttgcggatcggcctggaagtttgaccagatatcgtggtggaacgggatcactactttcgcattcagcgcttcacccatacgcagcatatcggcgctggtcattttgtcggtgataccgcgcgggttttcgccgtacgatcctaacgccacgtcgatctgatgttcgttaccgtgcttcgcataatagttagagtagtgggagtcgccgctgtgatacagggagccgccaggcgttttgaacaggtagttcaccgcgcgatcgtccatgccatctggcagtacgccagccgctttttgatcggcaggcagggtgatcagtgcagtacggtcgaaagcatcaagcgcatgaatttcaatgtctttcacttttactacatcgcccggtttgaccacgatgcaacgctctttcggtacgccccagccaatccacaaatccacacaggttttcggtccgataaacggtacgtcatctgcacaattctgcatcacggcagcagcgacgttaacgtcgatatgatcgttgtgatcgtgagtcgccagtaccgcgtcgatctggcgaatcgcaaacggatcaagaacaaacggggtggtacgcaggtttggctgcagttttttcacgccagccatgcgctgcatctggtgaccctgtttcattaacgggttaccgtgactttgtttgccagtgccgcaccagaaatcaacgcaaacgttggtgccaccttccgatttcaaccagatcccggtgcagccaagccaccacatcgcaaatgtgccaggagcgacctgttcttgttcaatttcttcattcaaccagctaccccactccgggaaagtgctcaggatccaggattcacgggtgatacttttcactttactcatcgccatttaccttcatgatagttcaattcgaatcaatatgtgattggttttgattaatcctgacactattttttcaggaaggcaatgaccattttttgactttttgccagggaagttgttgttgattttgagtatggaaagatttaatggaatgtgtaattcaattaactaaatgaatttaaatggataattgtttcgttgtgtgaatcccactctatccatgtggaattatttgcgggtcgcgtcacatttaatcataaataatcttgttgtgattacttttgaaaattagagtgagtgcacaacattccgggtgtgtggaatacccggttacctcttcttcaggagatcgttatggagatcctctacaacatctttaccgtgttttttaaccaggtcatgaccaatgccccgttgttgctgggtattgtgacctgtctgggctacatcctactgcgcaaaagtgtcagcgttattattaaaggcacgattaaaaccataattggtttcatgttgttgcaggcagggtccggcatcctcaccagcaccttcaaaccggtggtggcgaaaatgtccgaagtctacggcattaacggcgcaatttccgatacctacgcttcaatgatggcaaccatcgaccgcatgggcgatgcctatagctgggtgggttacgccgtattgttagcgctggcgctgaacatctgttacgtgctgttgcgtcgcattaccggcattcgcacaatcatgttgaccggccacatcatgttccagcaggccgggttgattgccgttacgctgtttatcttcggctactccatgtggaccaccattatctgtaccgcgattctggtttcgctctactggggcatcacttccaacatgatgtacaagccgactcaggaagtgacggatggctgtggtttctccatcggtcaccagcagcagtttgcatcatggattgcctataaagtcgcgccgttcctcggcaaaaaagaggagagcgttgaagacctcaaattgccgggctggctgaacattttccacgacaacatcgtctccacggcgattgtgatgaccatcttctttggtgccattctgctctccttcggtatcgacaccgtgcaggcgatggcaggcaaagtgcactggacggtgtacatcctgcaaactggtttctcctttgcggtggcgatcttcatcatcacgcagggtgtgcgcatgtttgtggcggaactctctgaagcatttaacggcatttcccagcgcctgatcccaggtgcggttctggcgattgactgtgcagctatctatagcttcgcgccgaacgccgtggtctggggctttatgtggggcaccatcggtcagctgattgcggttggcatcctggtcgcctgcggctcctcgatcctgattattcctggctttatcccgatgttcttctctaacgccaccatcggcgtgttcgctaaccacttcggcggctggcgtgcggcgctgaagatttgtctggtgatggggatgatcgaaatctttggttgcgtctgggcggtgaaactcaccggtatgagtgcctggatgggcatggcggactggtcgattctggcaccgccgatgatgcaaggcttcttctccatcggtatcgcctttatggccgtcatcattgtaattgcactggcttatatgttcttcgctggccgcgcgctgcgcgcagaagaagatgcagaaaaacaactggcagaacagtctgcttaataaggagttttgattatgaccgtacgtattctggctgtgtgtggcaacggacaaggcagttccatgatcatgaagatgaaagtggaccagtttttaacccaatcaaacattgaccatacggtaaacagctgcgcggttggcgagtacaaaagcgagttgagtggcgcggatatcatcatcgcttctacgcacattgcgggcgaaatcaccgtgaccggcaacaaatacgtggttggcgtgcgcaacatgctctctcctgccgactttggcccgaaactgctggaagtgatcaaagagcatttcccgcaggatgtgaagtaaggacgcgccatgaaattacgtgattcgctggcggaaaataaatccatccgcctgcaggctgaagcagagacatggcaggaagcggtgaaaatcggcgttgacctgctggtggcggcagatgtggtagagccgcgttactaccaggcgattctggatggcgttgaacagttcggtccttatttcgttatcgctccgggcctggcaatgccgcacgggcgtccggaagagggcgttaagaaaaccggtttctctctggtaacgctgaaaaagccgctggagttcaaccacgatgacaacgatccggtggatatcctcatcaccatggcggcggtcgatgccaatactcaccaggaagtgggcatcatgcagatcgtcaacctgtttgaagatgaagagaattttgaccgtttacgcgcctgccgtaccgagcaggaagtactggatctcattgaccgcaccaacgcggcagcttaagaaggaattgaacatgtcattaccgatgttgcaagtcgcgctggacaaccagactatggatagcgcctacgaaaccactcgcctgattgccgaagaagtcgacattatcgaagtgggcaccattctgtgcgtgggcgaaggcgtgcgtgcggttcgtgacctgaaagcgctctacccgcacaaaatcgtactggcagacgccaaaattgccgatgcaggcaaaatcctttcgcgtatgtgcttcgaagccaacgctgactgggtgacggtaatttgctgtgcggatatcaacaccgccaaaggcgcgctggacgtggcaaaagagtttaacggcgacgtgcagatcgaactgaccggttactggacctgggaacaggcgcaacagtggcgcgatgcaggcattgggcaggtggtttatcaccgcagccgtgacgcgcaggccgcaggcgtggcgtggggcgaagcggacatcaccgcgatcaaacgtctttccgatatgggcttcaaagtcaccgtcaccggaggcctggcgctggaagatctgccgctgttcaagggtattccgattcacgtctttatcgcgggccgtagtatccgtgatgccgcttctccggtggaagccgcacgtcagttcaaacgttccatcgctgaactgtggggctaaggagcggatatgttgtccaaacaaatcccgcttggcatctatgaaaaagcgctccccgccggggagtgctggctggaacgcctgcaactggcaaaaacgttaggcttcgattttgtcgaaatgtcggtagatgaaactgacgatcgcctgtcgcgcctcaactggagccgcgagcagcgtctggcgctggtcaatgcgattgttgaaaccggcgtgcgcgtgccgtccatgtgcctttctgctcatcgtcgtttcccgctgggcagtgaagatgacgcggtgcgggcgcaggggctggagattatgcgtaaagctatccagttcgcccaggatgtcggtattcgcgtgatccagctggcgggctatgacgtttactatcaggaagccaataacgaaacgcgtcgtcgtttccgtgacggcctgaaagagagcgttgagatggcaagccgcgcgcaggtgacgctggcgatggagatcatggattatccgttgatgagctccatcagcaaggcgctgggatacgcgcactatctcaacaatccgtggttccagctctacccggatatcggcaacctgtcggcgtgggacaacgatgtgcagatggagttgcaggccggaatcgggcatatcgtcgcggtacatgtgaaagacaccaaacctggcgtcttcaaaaacgtgccgtttggcgaaggtgtagtggatttcgaacgttgtttcgaaacgctcaaacagagtggctattgcgggccgtacctgattgagatgtggagcgaaacggcggaagacccggcggcagaagtggcgaaagcgcgtgattgggtgaaagcgcgcatggcgaaagcgggcatggtggaggcggcataatgcaaaagctaaaacagcaggtatttgaagccaacatggagctgccgcgctacgggctggtgacctttacctggggcaacgtcagcgctatcgaccgcgaacgcgggctggtggtgatcaagcccagcggcgttgcctacgaaaccatgaaagcggccgatatggtggtggttgatatgagcggcaaggtggtggaaggggagtatcgcccatcttccgacactgcgacgcatctcgaactctaccgtcgttacccgtcgcttggtggcattgtccatacccactccactcatgccaccgcatgggcgcaggcggggctggcgatcccggcgttaggcaccacgcacgccgactacttctttggcgacattccgtgtacgcgcgggttaagcgaagaagaggtgcagggcgagtatgaactgaacaccggcaaagtgattatcgaaacgctgggcaacgccgagccgctgcatacgccgggaattgtggtgtatcagcacgggccgttcgcctgggggaaagatgctcacgatgcggtgcataacgcggtggtgatggaagaagtggcgaaaatggcgtggattgcccgcggcattaacccacaactcaatcacatcgacagcttcctgatgaataaacacttcatgcgtaaacacggtcctaacgcttattacgggcagaagtagaacacgcgctgcggaaatttccttcctcgggagataactggtctaattccgcagccgtttttcaaaaaaaagccccctgcgaagggggcaaagcaaactatggcaatgtttcgttggttatacctggtgctagcgataaatatccgcgctggcgtgcatattgccgttactccccggttcccgcatcagaattacgtggtagtacgttgcgccttgcgcatctgtttcttcatttaatgcctgacgtgcttcgctttcagtggcgaaattatgattgatataaatcacgcctaagctttgcacatcgtccatatttctggcctggtggttattaatttcaatggctgcccatgtatttgcacttagcaaaagcacagccagaagggctaaaacacgactgaacatagatacctcctcgacggctgactttgtgtgctctcctctgtgatgatcttctgatttaattttaatcaatgataaagaagttgatggtgaccatttctgatgcagttgttcaaaaaaacaccatgatgaagtgtgatgaacttcaaatcagcgtgttagaggttaattgcgaaaggggagatttatttcggctctgcccttgagtttagcgaggcatacaagtactataacgcgtcatttttcagccgacctttaacacgttccttgcctccccgggattcggctgacccagacaggaggctgaataatccgtaaggagcaattcgatgcgtcattacgaaatcgtttttatggtccatcctgaccagagcgaacaggttccgggcatgatcgagcgctacactgctgccatcactggtgcagaaggcaagatccaccgtctggaagactggggccgccgtcagctggcttacccgatcaacaaactgcacaaagcacactacgttctgatgaatgttgaagctccgcaggaagtgatcgatgagctggaaactaccttccgcttcaacgatgccgttatccgcagcatggttatgcgtaccaagcacgctgttaccgaagcatctccgatggttaaagcgaaagacgagcgccgtgagcgtcgcgatgatttcgcaaacgaaaccgctgatgatgctgaagctggggattctgaagagtaatttctgatgaccaaccgtctggtgttgtccggcaccgtgtgcagggctccccttcgaaaggtcagtccatcaggaattcctcactgccagttcgtgcttgagcatcgttctgtgcaggaggaagccggctttcaccggcaggcgtggtgtcaaatgcccgttattgttagcggacacgaaaaccaggccattactcacagtataacggtcggcagtcgcataaccgttcaggggttcatttcatgccacaaggcaaagaacggactgagcaaaatggttttgcatgccgagcagattgaattgatagattctggagactagccatatggcacgttatttccgtcgtcgcaagttctgccgtttcaccgcggaaggcgttcaagagatcgactataaagatatcgctacgctgaaaaactacatcaccgaaagcggtaagattgtcccaagccgtatcaccggtacccgtgcaaaataccagcgtcagctggctcgcgctatcaaacgcgctcgctacctgtccctgctgccgtacactgatcgccatcagtaatcggtcacggtccattaatacgactttgagaggataaggtaatgcaagttattctgcttgataaagtagcaaacctgggtagcctgggtgatcaggtaaacgttaaagcgggctatgctcgtaacttcctggtaccgcagggtaaagctgttccagctaccaagaaaaacattgaattcttcgaagctcgtcgcgctgaactggaagctaaactggctgaagttctggcagctgctaatgctcgcgctgagaaaatcaatgcactggaaactgttaccatcgcgtctaaagctggcgacgaaggtaaactgttcggttccatcggtactcgcgacatcgctgacgctgtaactgcagctggcgttgaagtggctaagagcgaagttcgtctgccgaacggcgttctgcgtaccactggcgaacacgaagtgagcttccaggttcacagcgaagtattcgcgaaagtgatcgtaaacgtagtagctgaataattcgttattcaacgagacgtaaaaacgccgaccattggtcggcgttttgctttctatttttcgtcaggtattagtttcgcaagtagatccattcaccattctcttgtgtccataagtcaggatggtttgctggcgttagatacatacgagcgcaactgatgtctcgctcctgcggcactcgctcgaaacccaaacccgagtagattgcggctgaacttgataaggaacgcagaccaattttcaaatcatggggtaaatcagaatacgcgtttagcaatgcagcaatgatgaatccgagggcattagaaacgcctgtaacagtgcgaagttggtcgatataaagatcgattgttggtagttcagatgaccagcaattaggcatttgggcaggaagggttacaacgtatcctatcgtttggccggtatagtctggagtaccataaccaggtcccaaaaccacttcgtgtattgtgtatttactgttgggttcgaaggattcgacatcttgcaataaatatttcagttctgcggttaacctcgcacccgcgtaagctttattgtatttctgggcgtgaatattatctaatgtagcttcatggttccatccaaaagaattatcaccattcattgtgattccatcgtaagcattacacctcgtcgctaacttattgaatgcttgccagtctgagagatctagtttgtggatctcaacagtacgtctgccatcgcaattatgatctcttccacgatttgaaagtaatgtagcgcgtgcgtattgatgaaattttaattttactggtttgtcggtggacgaaaaacgagataaatatgcaggaaatgaataaatagtcgttggtaatgtcattgtaatgttacctgtttaatgtttttataaatatcgcagctgaatgttcacagaaaaaaatcgatattaataaaaataagtttgttttctgaagtggtgaaaatagcggatggtgaaagatattaatatcaaaaatcgctcattatggatataacgatgcacccggggagaaaatgacttccacgccttacaccgtacattcttgttgtgcggtatgtaattattctacgctgtcggtatcggtgtattcgttaatcagcaggttagccagccacaaaaagccattgagaaaattattgattttacatgggattattatattgctaatccttggtttttaaaaattgtgcatagtgaaaatcaaagtaaaggtgtgcattatgcaaaatcacagcgtctcttagaaattaaccatgcgcacttgcagttaatggaatccttattggatgaagggaagaaacacaatatttttaagccagatatcgacccattgcaggtgaatattaatattgctgcgcttggcggatattatttgatcaaccagcatacgcttggcctggtttatcacatcagtatggtttcaccccaggcactggaagccagacgtaaggtcatcaaagagacaatccttagctggcttttggttgacccttcatctaccgcgcacgaataaaactgccatccggctggcgggtgaacaggacctgttgattattccccgtatcaatggttaagcccgtcaccacgccgctggcgttctggcggattttcaccatctgcccgttttgcaaattactcagcggcttacccgcgccttctacctgcgccattgcatagacatcggtagcgggcagtccgtggtcgcggaacagctgcgccatcgttttaccgggttcgacacggtaagagcgccattgattatcaattccgctatctggctggaatggttgcgtttgggtagtttgcggctgctcttctggctggccttcctgtataggttctggagcgaccggagccacctgatcaggatcattttgtggggtaactaattgcgcccgcagctgttcttctgtcggcggttgtgattgcgactgaatatctaactgcgcttcacgcgtcaccaccggcgcgttgggcgtatcatcagatggaagcagaaatccgaccaccaatacaatggcggcaataatgatcccccgacgatgcatcggcggcagcgggtccatgaagcgaaaattgtccggcgcgtgccagactttctccagggttggttttagttcaaagcgcccgggcatggtttcctcctgctccgcgtcttgttcctcaatcatagcctatgaataagctaacgctatgatgtccgtggtaaacccgcctttattatattcatacgggatattgctattgtttctttttccctgggatttgtcatcattcccgcgacaaagttttacccaaagaagtgtggctgatatgctgcccgctactttataccctaagaaaggaaatacgatgaccaccccaacttttgacaccatcgaagcgcaagcaagctacggcattggtttgcaggtagggcaacaactgagtgaatctggcctggaagggctgctgccagaagcactggttgcaggtattgccgatgcgctggaaggcaaacatccggctgttccggttgatgtggtgcatcgcgcgctgcgtgaaatccacgagcgcgccgatgccgttcgtcgtcagcgtttccaggcgatggctgctgaaggtgtgaaatacctggaagaaaacgccaaaaaagaaggtgtgaatagcaccgaatctggcctgcaattccgcgtgatcaaccagggtgaaggcgcaattccggcacgtaccgaccgcgttcgtgttcattacaccggtaaactgatcgacggcaccgtgtttgacagctccgttgctcgtggtgaacccgctgaattcccggttaatggcgtgatccctggctggattgaagcactgactctgatgccggtaggttctaaatgggaactgactatcccgcaggaactggcatatggcgagcgcggcgcaggcgcatccatccctccgttcagcaccctggtgtttgaagtcgaactgctggaaatcctctaagcagcgcattctgttcccctcgaacgagaggggagcaggcattcagcaataaacccttcagtttgccaaacggcgctattttgtgttgcaaagaccccgtaagcgtgtatttttgtgagctgtttcgcgttatcaccgtgatatgacactcactttaaacataaaattaacattagatctaaatcttagtattcatcccgcgtattgttacctaatatcgatgagtcccgatacagattcgtcgtatcatagactgactaaaggccgtagagcctgaacaacacagacaggtacaggaagaaaaaaacatggtagatcaggtaaaagtcgttgccgatgatcaggctccggctgaacagtcgctacggcgcaatctcacaaaccgacatattcagcttattgccattggcggtgccattggtacggggttgtttatggggtctggcaaaacgattagccttgccgggccgtcgatcattttcgtttatatgatcattggttttatgctctttttcgtgatgcgggcaatgggggaattgctgctttcgaatctggaatacaaatcttttagtgacttcgcttccgatttactcgggccgtgggcaggatatttcaccggctggacttactggttctgctgggttgtaaccggtatggcagacgtggtggcgatcacggcttatgctcagttctggttccccgatctctccgactgggtcgcctcgctggcggtgatagtgctgctgctgacgctcaatctcgccaccgtgaaaatgttcggtgagatggagttctggtttgcgatgatcaaaatcgtcgccattgtgtcgctgattgtcgtcggcctggtcatggtggcgatgcactttcagtcaccgactggtgtggaagcgtcattcgcgcatttgtggaatgacggcggctggttcccgaaaggtttaagtggcttctttgccggattccagatagcggttttcgctttcgtggggattgagctggtaggtacaacagctgcggaaaccaaagatccagagaaatcactgccacgcgcgattaactccattccgatccgtatcattatgttctacgtcttcgcgctgattgtgattatgtccgtgacgccgtggagttcggtagtcccggagaaaagcccgtttgttgaactgttcgtgttggtagggctgcctgctgccgcaagcgtgatcaactttgtggtgctgacctctgcggcgtcttccgctaacagcggcgtcttctctaccagccgtatgctgtttggtctggcgcaggaaggtgtggcaccgaaagcgttcgctaaactttctaagcgcgcagtacccgcgaaagggctgacgttctcgtgtatctgtctgctcggcggcgtggtgatgttgtatgtgaatcctagtgtgattggcgcgttcacgatgattacaaccgtttccgcgattctgtttatgttcgtctggacgattatcctttgctcgtaccttgtgtatcgcaaacagcgtcctcatctacatgagaagtcgatctacaagatgccgctcggcaagctgatgtgctgggtatgtatggcgttctttgtgttcgtggtcgtgttgctgacactggaagatgacactcgccaggcgctgctggttaccccgctgtggtttatcgcgctggggttgggctggctgtttattggtaagaagcgggctgctgaactgcggaaataaccgcattatcatgctggatggcgcaatgccatccagcttttagatcactcacccgccagcgcgcgtgggaacagtacattgttttccagactgatgtgatccatcaggtcatcaatcagttcattaatgccgttatacatcgctttccaggtggtgcaggcttctggcggcggtgtgacgttattggtggtgtgtttaatcacttccagcagttcgcccgcttcatcgtgctcgctttccattacgctgattggccccattgcctggctgcccatgccttgtttgatcatcgggaagaggatctgctcttctttcatcatgtggctggaaagctcttcatgcagcatggtcaggtattttgtcagcccttttggcacgctcggtttgtcggcgtgaacgcgctcgactttagtcgcttgcagaatcagctccggcagttgctcgcggtgacgatcgtggtagcgcacgatgatatggtcgatgatttctgccagcggggcgctacgccagtctttctcaatcggttgttcagcgagctttgccagttcagcttcaatgacctcaacatccagttctttacgtgccgccgcgcgcgccagcgtctgcttaccgccacagcagtaatccatatcatatttacgaaacagagctgaagcgcgaggaatagagagcgccagttcacctaaaggttggtcgcgataagccatagctgatacctcattcttaataagataagatgtattttaaatgcatctttaaggcaaaagctataacccttacgtagcagaggcttatttaactcactgccagcgtgtcaactttctgagacagattcagttaaaggtttttctggttttgctctgaccgcgatgaccacgccaatcactaacagcgcgataccgctcagcgtcattagcggcggcatttgctggcggagtaaaaaggtgtacagcaaacctgccagcgtttcgaaaacaatcagcggcccgagaatcactgtcggtaatagctggctggcgacgttccagcagagtgcgccaacccatgagcaaagcacggctatcgcaaccatcagactaataaacaccagcggacgggggccaaagggtagggagaagtccggcgtttgcgtattcagccagtaacaagcgacgagatagccgataagtgaaaccggcagtgtgaccagcgcctgcgctgttgcccacatcatcggatgtttgtcgggattttcccgcagccagcgggcgttgcgcagggcataccacgcccagcagaccacggaaactaacgccagcacgatgccagaggtataacgtgcccagtcaaaatcggggagtccgtggtttaactcagcaatattcacacacgccaggccgatgccaatacaaatcagtgctggggcgagttttccccacgcgagtttgccgtcgcgctggctataaagcagattggcaaagacaggaatgaccaccggcagggtgccgataatcatcgtggaaacaggcgcgccagtacgttgaatggcactggcaaggcagaagtaatagatgaggttgcccatcatagtgagcatcaaggcggtaagccagtcgcgacgcgccaactgacgcagacgcacgcgtcccagccaggcaatgggcagcgcaattaaccctaacgccagataacgccccatcgactgcaacatcgccgggtattccggcacgatcaacggcccgacaaaaataagcccccacatcaaccctgctaacagggcgtacagcacgccgctaatcattactggcatccattgatctgtcagaagaaagttcaggaagcagacatgattgctcccggcatcccgtcattatcagagaggatgcgggaggatgccactttaattaactagttattaacattaaaaagatggcttacgctttcggctaacgttgtcgttgggtggccaatcaatttgctaagtgttttgctgtcatcaaacagaccgcctttcgatgcgccaacgtcagaatccgccagcatatccgccagtccgtcgggcagtccgacgcttttcagtgccgcggcgaaatcggcttcgctcagattttgataggtaacctgtttgccgctctgtttggtcagctctgccgctaactgtgtcaacgtccaggcactatcgcccgccagttcgtaaaccttgccttcgtgaccggcttcgctaatcacgcgtgccgcagctgccgcataatctgcccgcgttgctgaggcgattttgccatcgcccgccgcaccgataaatacgccgtgttccagtgctgccggggcgctggcgaggtagttttcgctgtaccagccgttgcgcagcagggtgtaaacgatgccagaatcagccagcattttctccgtctcgatgtgctcatcggcgaggccgagcggggaggtatctgcatgtagcaggctggtataagcgataaatttcacgccagccgcctttgcggcattaataacattacgatgctgcggggcacgttgacccacttcgctggaagagatcagcagtagtttttccactccctgaagtgcagatgtcagtgcggcttcatcgccgtagtcagcctgacgcacggtaatgccttgtgctgccagggcttgggcttttgccggattacgaacgatagccactatttggctggcaggaaccgttttcatcaaggattcaataacatagtgaccaagttggccagtggcaccagtaatagcgatcatgggaagtctccatcgttttgtcttgtgtttaaatacgctaacacctaaacttacttttagtaagtacgtacaaaaaggtaagtatgaaatgagtcaggttagcctgtcgcaacaactgaaagagggtaatctctttgcggaacagtgcccgtcgcgcgaggtgttgaaacacgtcaccagccgttggggggtgttgattctggtggcgctacgcgaaggtactcatcgctttagcgacctgcggcgcaaaatcggtggggtgagtgaaaagatgcttgcgcagtcgttacaggcgttagaacaggatggttttcttaaccgtatcgcgtatccggtggtgccgccgcatgtggaatatagcctcacgccgctgggcgagcaggtgagcgaaaaggttgctgcactggcggactggattgagttgaatttgcccgaggtgttggcggtgcgggatgaacgtgcggcataactgccggatgcgctgagcttatctggtctacggtgcatggcttgtagggcggataagatgcgccagcatcgcatccgccaataaatgccggatgcggttgatgatttataggccgaaaaagaagtgttttacttactcaaatccacctgataaatcgcaaacccgatatcatcggtcgcgactttattcatcggatactgccctttctctttaataaacgctgcggctttatctgacggagaggtttcgaaacggatatccagtttcttatcgccagctatcggtgctaaacgccagttgttatctgccgccgggtgaatttcccccgcacgtttcgactcatcagcaatccacgctgccagcaccgagcggttctcatccggtgaagcaaaagcgatatggctgtcgcccgtaccggcaaatttgccgccgtaagcgcgatagttattggtggcaaccaggaacatggcgttcggatcaatcggcttgccattaaaggtcaggttcttaatcctttccgcattggcattaatcatctggcactcgccgtcataacgggcgggctgggtaacatcaatctgataattcacaccatcaataacatcaaagttataagtgcggaaaccatcccagttgatgagtgactgtggtttcgtgctgttgggatcaatctggttaaactgtcccgcggagcactccagccactctttcacctctttaccgctggctttcaccacaatcagcgtattgggatagagataaagatcggcggcattacggaaggtcaactggcctttttccacctccacatagcttgccgggtcatttttgcgaccaccgactttaaacggtgcggcagctgaaagcaccggcagttttgccagatccggatcgccctgaatgtaatgctcgacatacgctttttgcgcgttgttcaccacctgcacggtcggatcgtcctgcaccagcgccagatagctatacatattgtcggcagatttaccgattggcttgctgacgaactggcgtgtggcatcgtgatcggctttgagtgtttctaccagcttgctgtcttccgccgcgagggattttttattagcgatgtcgtaaatcggtcgtgcttccgctttcgcctgcgtcacctgccatttaccgctgtcattactgagttgtaagtcgaccacaccaagatgatcgccccacatgcctggcattaccgccggaacaccattcagcgtgcctttggcgatatcagccccttcgatatcagcaaaatctttacctgggaaaacggcgtgagcatggccaaacataatggcgttaacgcccggaatttcactgaggtaataaactgagttttccgccatcactttatacggatcggcagatagcccggaatgtgccagaacgacaacaacatcggcacctttctcgcgcatttcaggcacgtatttgcgcacggtttcggtaatatcattcaccgtcactttcccggataaattagctttatcccagcccatgatttgtggtggcacgacgccaatatagccaatcttcagcgtctgtttttttccgtctttatcgaccacttcggtgtctttaattaaatacggtgtaaacattggctgtttggttctggcgtcaatgacgttggcatttacataagggaatttcgctcctgccagcgcatttttcaggtaatccagaccgtagttaaactcgtggttgccaagcgttccgacggtatagtccagcgtatttaatgccttatagaccgggtgaatatcacctgcttttaatcctttcgccgacatgtaatcggccagcggactcccctgaatcaaatcgccgttatcaaccagtacgctgtttttcacttcattgcgggcatcgttaatcaggcttgccgtacgtaccagtccgaatttttccgtggcggtgtctttgtaataatcgaaatccatcatgttgctatgcagatcagtggtttccatgatacgcagatcgaccgtcgctgcattcacactggcggcaatcagcgtggccaggagcgttgcgctaaacttaatcatcagggacatccttttatcatcgggaatacgaaagaaaagggagaataaacgtcttacttatagaacagtgaagaatgccacaattttacgctttgaaaatgatgacactatcacagttggcgcattcattaacgatagggtataagtaaaacaataagttaacaccgctcacagagacgaggtggagaaatgttagatcaagtatgccagcttgcacggaatgcaggcgatgccattatgcaggtctacgacgggacgaaaccgatggacgtcgtcagcaaagcggacaattctccggtaacggcagcggatattgccgctcacaccgttatcatggacggtttacgtacgctgacaccggatgttccggtcctttctgaagaagatcctcccggttgggaagtccgtcagcactggcagcgttactggctggtagacccgctggatggtactaaagagtttattaaacgtaatggcgaattcaccgttaacattgcgctcattgaccatggcaaaccgattttaggcgtggtgtatgcgccggtaatgaacgtaatgtacagcgcggcagaaggcaaagcgtggaaagaagagtgcggtgtgcgcaagcagattcaggtccgcgatgcgcgcccgccgctggtggtgatcagccgttcccatgcggatgcggagctgaaagagtatctgcaacagcttggcgaacatcagaccacgtccatcggctcttcgctgaaattctgcctggtggcggaaggacaggcgcagctgtacccgcgcttcggaccaacgaatatttgggacaccgccgctggacatgctgtagctgcagctgccggagcgcacgttcacgactggcagggtaaaccgctggattacactccgcgtgagtcgttcctgaatccggggttcagagtgtctatttactaaattcagatggcagaaacagtgtatttcctgattctgccatcctgatttctcccaacctaaaaagttataaataaaaagagattgtatttaaagtgcaaaaattcaattgctaataagttacattttaataatgagcgttttttgatagtttacttctatagtgagatatttaatggcgacataaagtaaccaaataaaataaggttgtcatatgttacccaggatcagacacaataattttattggtgcggtggagttatttgtaaagtcttcgtatacaaaaacacattcaaacaatttttttaacaacatccatcatgcatttaagaaaaaagattggatttcgaattatgatagcctgttaactttgagggagttctttcgttgcgcaactcagattgataaaagtggttatcaggtgctttcatcaaaaaatgaaactgttcacgccatggataagtttcttatcagtttcagccttaaagataacggtgccgaatatacaatgacattgcgaggtagtggatttgaatacgaagaaatacccataacaataaatgaatataactcattcatggatttcaaaaaccgtgaatttccgttagaacaaaacagacgattgtatgcctgggatattctacagaaaaaacagtctgacataccgaaaaggattaaaggttatattcaccaggcgattggtgacgtgtctttaggttatgccttattggaggatatagtaagcaaattaaaacggggtaaatttgaactccaaataccaggaggtggaattaaagaatgcgatggatggtatatttacgaaaaaataattgatgataattttgccatagtcatagaatctttgggctttgcgcttaaaatctatggaggggatgaacgttttcgtaatggttcctctgttgttttggaggatgaagattactctcttatttataattttctggttaatgcaggttgccaacaagtcgaattagccgaacaagtggatgcgatagtaagtgcgaatctggccgcagatagcgatattaccaaagaaaagatttgcgagaaatataaatcgaccattgaggcgtttaaaaaagagcaactagcgttaccagtattagttcggcgtaagaactcagagacttaattcccctatcccatagataacgataggggaaaattatttttgcagaatttatgttattgccattatttgagcaacttttgcagcaggtccatcacttgctgcacctcttccggtgtgagcgccccgtctttggcccattgcacgcgaccatccttatccagcaccactacagcggaactttcttcatccagctgccaggcaccgagcgcgacgccattgctatcgacaataaactgcgaccagggataaagctttttattactctccagactgctgcgcacaaacatccctgaacccggaatcgcgtcgtcggtgttaacaatggtggtggtctggtaacgatcgtgcggtaacttcgctgatttaatcgcttcaatcagcgtcgcgtttttctcttttgcagaggtgcgaccagcaatatgttgcagtactcgcacttttcccactaactgcgcgctgttccaggttttgtagctaaactgatctttatcaagcaccaactcgccccgatcggtaatgccaatcggcggcactcgctgaccggtttcgaactgatgtgcggaagccatcatcggcaacagcaggcaggtgagtgccagaatcttgcgtagggtcatggtgtttccttcttatgatatgcaggtgatccgaccacttgggtctgagttttaatcatatgtgctatttatcgaatttcccgcaagtgtgatgccagtttgcggtcaagcgcacaaatcatatgaaaaatgaatgcttatactgaagaccgcgcttcggtaaaaagataattctgaataattgtaacctttaggtaaaaaaagttatacgcggtggaaacattgcccggatagtctatagtcactaagcattaaaatttgcgcctcataatagttgggccgattgtggcaccgcacaggcgtaatactcagcaggagataacaatgaaaattttccaacggtacaacccacttcaggtggcgaagtacgtaaagatcctgttccgtggacggttatacatcaaggacgttggcgcttttgaattcgataagggtaagattcttatcccaaaagtgaaggataagctgcatttgtcagtgatgtccgaagttaaccgtcaggttatgcgtctgcaaacagagatggcttaaccaaagtgctatgcagtaaaaagtgctatgcagtaataagacggctcctgattcaggagccgttgatgtttctgggggttacgcgacgctttcttctttatctttagcgtcaggcagttttggcgaaagggcggtggccttgctgtcgatccgggtcaccagcagctggtcgatgcggtagttatcgatatccaccacttcaaatttgtagccggcgaatttcaccgaatcggtgcgtttcgggatcttacgcagcataaacatcataaagccgccgatggtttcgtagttgcccgactgcgggaactcgtcaatatccagcacgcgcatgacgtcgtcaattggggtgccgccgtcaatcagccatgagttctcatcacgggcgacaatctgctcttccagcccctgaccgaccagatcgcccatcagcgtggtcatcacgtcattgagggtgatgatccccaccaccagcgcgtactcgttcatgatcaccgcgaagtcttcacctgcggttttaaaactttccaacgcctctgaaagggttaacgtatccggcacaatcagcgtgttgcgaatttgtacgccgctgttcagtgccaggctttggttagccagcacgcggttcagcaggtctttagaatcgacataaccgatgatgtggtcaatatcttcattacagacgaggaacttagagtgcggatgttccgccaccttattcttcaggctttgctcatcttcgtggagatcaaaccaaatcacgttttcacgcggtgtcattgaagacggaacggtacgggattccagctcaaagacgttttcaatcagctcgtgttcctgtttacgtaacacgcccgccagcgcaccggcttccactaccgcgtagatgtcatcagaagtgatgtcatctttacgtaccattggcagtttgaaaatacggaagattatgttcgccaggccgttgaagaaccacaccagcggggtgcaaacgtacaggcagaagcgcatcgggttgatgatacgcaaagccacagcttctggcgcaatcataccgatgcgtttcggggttaaatccgcaaacaggataaacatgccagtcactaacgagaaagagagaataaagctcagttgctcagagagctctgccgacatatagcgggagaacaggctgtgaaaagctggagaaaatgccgcatcaccgacgataccgccgagaatcgccactgcgttcagaccgatttggaccacggtaaagaacatgccgggattttcctgcatattcagaacgcgttgggcatttatattgccttcatcagccagcagtttaagtttgattttgcgtgaggcggcaagcgagatctcggacatcgagaagaacgcacttacagcgatcaagcagagtatgactaaaatactgtttaacatatcttatccgacctttcaggccagatcctcggaaggggaagttgattaatttgtgtgaaatacacattgaaagccgattcgaagaaagtgaaccggcattttcagtggctagtatagcgtaaggtactgtaaagccgccagagggttaaaattcagacagctgaaaaatgcaaaactgcctgatacgctatgccgatcaggcctacgcagtccttgcaatatattgaatttggacgattttgtaggcctggtaagtcgtttacgccgcatcaggcatagacaaagagcactttatcaacaaactacatttgtacccgtaacgctatgcttccggcggcagacagacgccaattccgccaattccacagtaaccatacgggtttttatgcagatattgctggtggtcatcttcggcataataaaacggtgtggcgttagcgatttccgtggtgatgtgacgatcgtcatcggcggcaagcatcgccgcctgaaaacgttccagactggcgcgagctgcggcatcctgttctggggtcagcggataaatcgctgaacgatactgcgtgccgtggtcattgccctgacgcattccctgggcgggatcgtgattctcccaaaatacctgtagcaactgctcatagctgatgacggaaggatcgtaaacaatgcgtaccgcttcggcatgacccgtatcaccggagcacacttcccgataagtcggatttggcgtatagccgccggtatagcctgcggcggtgctgtaaacgccgggtaactgccagaacagacgctccacaccccagaaacaacccatcgcaaaaatggcaatctccattccgtcaggtacattggtcattgagtgaccgttgaccgcatgcagcgtggctacgggcatcggggtgttacgtccaggcagggcatcggcgggggaaaccagatgctttttatcaaataaactcatggtgtcgctctcccgaaaatcggtcattggggttaaggttgtaacaagaggcgtatttgcacacaataaccaccgtgaataggtctaaagtaaaacataagaaatatttggggtttagtctgctttttaatccatattactggatttttgttaagccgtttaacggcgttccaggggcaggaaaaaaggatattcaggagaaaatgtgcgctatatccgacagttatgctgtgtaagcttactctgcttaagcggatctgccgtcgccgcgaacgtccgtctacaggtcgaggggttatcgggacagctggaaaagaacgttcgtgcgcagctttctacgattgaaagtgatgaagtgacgccagaccgtcgctttcgcgcacgcgtcgatgatgccatccgcgaaggtctgaaagcgctgggttattaccagccgaccattgaatttgatctccgtccaccgccaaagaaagggcggcaggtattgatcgccaaagtcacgccaggcgtgccggtgttaattggcggcaccgatgtggtattgcgcggcggcgcgcggaccgataaagactatttgaaattgctcgatactcgcccggctattggcacggtactgaaccagggcgattatgaaaatttcaaaaagtccttaaccagcattgcgttgcgtaaaggttatttcgatagcgaatttaccaaagcgcagctgggcattgcgctcggcctgcataaagccttctgggatattgattataacagtggcgaacgttaccgctttgggcatgtgacctttgaaggatcacaaatccgcgatgaatacctgcaaaatctggtgccgtttaaagagggcgatgagtacgaatcgaaagatctggcagaactgaaccgccgactttctgctaccggctggtttaactcggtggtggtggctccacaatttgataaagcgcgcgaaacgaaagtattaccattgacgggcgtggtttcgccgcgaacagaaaacaccatcgaaaccggggtcggttactctacggacgtgggaccgcgcgtgaaagcgacgtggaaaaagccgtggatgaactcttatggtcacagtctgaccaccagtactagtatttccgcgccggaacagaccctcgacttcagctataaaatgccgctgctgaagaatccactggaacaatattatttggtgcagggcggttttaagcgcactgacctgaacgataccgaatctgactccactacgctggtggcttctcgctactgggatctctccagcggctggcagcgtgccattaacctgcgctggagtctcgaccactttactcagggtgaaattaccaataccacgatgctgttttatcctggggtgatgattagccgcacgcgttctcgtggtggcctgatgccaacctggggcgactcgcaacgctactctatcgactactccaacacggcctggggttcagatgtcgatttctccgttttccaggcgcagaacgtctggatccgcacactgtacgatcgccatcgttttgttacacgcggcacgctgggctggattgaaaccggtgatttcgacaaagtaccgccggatctgcgtttcttcgccgggggcgaccgcagtattcgtggctacaaatacaaatctatcgctccgaaatacgccaacggtgacctgaaaggggcctcgaagttgataaccggatcgctggaataccagtacaacgtgaccggaaaatggtggggcgcggtgtttgtcgatagtggcgaagcggtaagcgatattcgccgcagcgactttaaaaccggtaccggggtcggcgtgcgctgggaatcgccggtcgggccaatcaaactcgattttgccgtaccggtcgcggataaagacgaacacgggttacagttttacatcggtctggggccagaattatgagtttatggaaaaaaatcagcctcggcgtggttatcgttatcttactgttgctgggatcggtggcgtttctggtgggcaccaccagcggcctgcatctggtatttaaagcggcggatcgctgggtgccaggactggatattggcaaggtcaccggcggctggcgcgatctcaccttgtctgacgttcgttatgagcagccaggcgtggcggtaaaagcgggcaatctgcatctggctgtcgggcttgagtgcctgtggaacagcagtgtttgtattaatgatctggcgctgaaagacattcaggtcaacatcgacagtaaaaaaatgcctccttctgaacaggttgaagaagaggaagatagcggtccgctggatctctccacgccgtatcccatcaccctgacacgggtggcactggacaacgtcaacattaagattgatgacaccacggtatcggtgatggacttcacctccggcctgaactggcaggagaaaaccctgaccctgaaaccgacgtcgctgaaaggcctgctgattgctctgccgaaagtggcggaagtggcgcaggaagaagtggtcgaaccgaaaattgaaaatccgcagccggatgaaaagccgctcggcgaaacgctgaaagatctcttttctcgcccggtattgccggaaatgaccgacgtgcatttgccgcttaacctgaacattgaagagtttaagggcgagcagctgcgcgtgacgggcgacacggacatcaccgtgagcaccatgctgctgaaagtgagcagcattgacggcaatactaaactggacgccctggatatcgattccagtcaagggatcgtcaacgccagcggcacggcgcagctgtcagacaactggccggtggacatcactctcaacagtacactgaacgtggagccgttgaaaggtgaaaaagtgaagctgaaaatgggcggcgcgctgcgcgaacagctggagattggcgttaatctttccggtccggtggatatggatttacgcgcccagacgcgactggcggaagccggattgccgctcaacgtggaagtgaacagcaaacagctttactggccgttcactggtgagaagcagtatcaggcggatgatctgaaactgaaacttaccggcaaaatgaccgattacacgctctctatgcgtacggcagtgaagggacaggagatcccgcccgcgactattaccctcgacgccaaaggtaatgaacagcaggtcaatctcgacaaactcaccgtcgcggcgctggaagggaaaactgaactcaaggcgttgctcgactggcaacaggccattagttggcgcggtgagctaacgcttaacggcattaacaccgccaaagagttcccggactggccgtcgaaactcaatggcttgattaaaacccgcggtagcctgtacggcggcacctggcagatggacgtgccggagttgaagctgaccggtaacgttaaacagaacaaagtgaacgttgacggcacgctgaaaggcaacagttatatgcagtggatgatcccagggcttcatctggaactcgggccaaacagtgccgaagtgaaaggcgagctgggggtaaaagatctcaatcttgatgccaccatcaacgcgccggggctggataacgcgctgccggggcttggcggtacagcgaaagggctggtgaaagtacgcggcacggtggaagcgccacaactactggcagatatcaccgcgcgcggcctgcgctggcaggaactttccgtggcgcaggttcgcgtggaaggcgatatcaaatccaccgatcagatcgccgggaaactcgacgtacgcgttgagcaaatttcgcagccggatgtaaatatcaacctcgtcaccctgaatgccaaaggcagcgaaaagcagcacgagctacagttgcggattcagggggagcctgtctccgggcagcttaatctggcaggaagttttgatcgcaaagaagaacgctggaagggaactcttagcaatacccgcttccagacgccggttggcccgtggtcgctgacccgcgatattgcgctggattaccgcaataaggagcaaaaaatcagcatcgggccacactgctggcttaacccgaatgcggaactgtgcgtgccgcaaactatcgatgcgggggccgaagggcgtgcggtggtgaatctcaaccgcttcgacctcgccatgctgaaaccgtttatgccagaaaccactcaggccagcggtatcttcacgggtaaagcggacgttgcctgggacaccacgaaagaggggctgccgcagggcagtatcaccctttcggggcgtaacgtgcaggtaacgcaaaccgtcaacgatgcggcgctgcccgtggcgtttcagacactgaatctgacggcggaattgcgtaacaaccgtgccgaattgggctggaccatccgcctgaccaataacggccagtttgatggacaggtgcaggtgaccgatccgcaaggccgccgtaatcttggtggcaacgtcaatatccgtaacttcaaccttgcgatgataaaccccatctttacccgtggggaaaaagcagcggggatggtgagtgccaacttgcgtctgggtggtgatgtgcaaagcccgcagttgtttggtcagcttcaggttacgggtgtggatatcgatggcaactttatgccgtttgatatgcaaccgagccagcttgcggtcaactttaacggtatgcgctcgacgcttgccggtacagtacggacccagcagggtgaaatctacctgaacggtgatgccgactggagccaaattgaaaactggcgggcgcgggtaacggcgaaaggcagtaaagtgcggatcaccgtgccgccgatggtacgaatggatgtatcgccagatgttgtattcgaggctacaccaaacctgtttaccctcgatggtcgcgtggatgtcccttgggcgcgcatcgtggtgcacgatctgccggaaagcgcagtaggcgtctccagcgatgtggtgatgcttaacgataacctgcaaccggaagagccgaaaacggcgtcgattccgattaacagtaacctgattgtccacgttggcaacaatgtgcgcattgacgcctttggcctgaaagcgcggctgacgggcgatctcaatgtcgttcaggacaaacaagggctgggtctgaacgggcagatcaacatccctgaagggcgcttccatgcctatggtcaggatctgattgtgcgtaaaggtgagttactgttctctggtccgccagatcaaccgtatcttaatattgaagctattcgtaacccggatgctacagaagacgacgtaatcgccggagttcgcgtcactggtctggcggacgaaccgaaagcggagatcttctctgacccggcgatgtcgcaacaagctgccttgtcttatttgctacgtggacaagggctggagagcgatcagagcgacagtgcggcaatgacctcgatgctgattggtttgggggttgcgcaaagtggccagattgtgggtaaaatcggcgagacgtttggcgtaagcaatttagcgctcgacacccagggagtaggcgactcctcccaggtagtggtcagcggctatgtattgccaggtctgcaagtgaaatacggcgtgggtatatttgactctatagcaacactcacgttacgttatcgcctgatgcctaagctatatctggaagccgtgtctggtgtagaccaggcactggatttgctctatcagttcgagttttagcaatgcgaatatttgtctacggcagtttacgccacaaacaaggcaacagtcactggatgaccaatgcccagttactgggcgatttcagtatcgataactaccagttgtatagcctgggccactatccaggcgcagttccggggaacggaacggtacacggtgaagtttatcgtattgacaacgccacgctggccgaacttgatgccttgcgcaccaggggcggtgaatacgcgcgccagttgattcagacgccgtacgggagtgcatggatgtacgtttatcaacgacccgtcgatggattaaagctaattgaaagcggcgactggttagacagggataagtaaccatatgcatacgccaccttcgggtggcgttgttttttgcgagacgactcgcattctgttttgtaattccctcaccttttgcttttctctccgagccgctttccatatctattaacgcataaaaaactctgctggcattcacaaatgcgcaggggtaaaacgtttcctgtagcaccgtgagttatactttgtataacttaaggaggtgcagatgcgtattaccataaaaagatgggggaacagtgcaggtatggtcattcccaatatcgtaatgaaagaacttaacttacagccggggcagagcgtggaggcgcaagtgagcaacaatcaactgattctgacacccatctccaggcgctactcgcttgatgaactgctggcacagtgtgacatgaacgccgcggaacttagcgagcaggatgtctggggtaaatccacccctgcgggtgacgaaatatggtaaagaaaagtgaatttgaacggggagacattgtgctggttggctttgatccagcaagcggccatgaacagcaaggtgctggtcgacctgcgcttgtgctctccgttcaagcctttaatcaactgggaatgacgctggtggcccccattacgcagggcggaaattttgcccgttatgccggatttagcgttcctttacattgcgaagaaggcgatgtgcacggcgtggtgctggtgaatcaggtgcggatgatggatctacacgcccggctggcaaagcgtattggtctggctgcggatgaggtggtggaagaggcgttattacgcttgcaggcggtggtggaataaggtgtgtttatttatcgcgggcataaaaaaacccttactaaccgaagcccggcgttcagggttattacgccagaagaacttatttattctttgcgcgctcgaaggaggcaacgatttcagctttagcggcttctgcgttttcccaaccttcaactttcacccacttgcctttttcgaggtctttgtagtgctcgaagaagtgagcgatttgcgctttcagcagttcaggcagatcgttaacgtctttaatgtgatcgtattctttgctcagcttgctgtgcggaaccgcaaccagtttcgcatcttcaccggcttcgtcggtcattttcagaacgccaaccggacggcaacggatcacagaacccggctgcagcgggtacggagttgggaccagtacgtcaaccgggtcaccgtccagagacagggtgtggttgatgtaaccgtagttgcatggatagaacatcgcggtggacatgaagcggtcaacgaacagtgcgccgctctctttgtcgatttcgtatttgatcggatctgcgttagccgggatctcaataacaacgtagatgtcttccggcagatctttacccgcagggacgttgagtaagctcatgtctgtttcctttaaaaatatgtggcaaacaagtgccgagtattatagccaactcgcgccgaatgtcttcgcttgttttcgtcttcattttcctttttcaccagttttaagacggtatacagagcaggaaaatccataaccgtagccgcatttttcatagtgagatgaaagcgattacaaacttgtgattaacgttttatttacttttttgaagtgtgatgtaacgcaatctgttacataacgaattgtctatagttttttcgcgaacatcttttaaccaataataactaccccgacgaggacaaccctatgtggaaacgcttacttatagtctctgcagtctcggcagccatgtcgtctatggcgttggccgctccattaaccgttggattttcgcaggtcggatcggaatcaggctggcgtgccgcagaaaccaatgtggcgaaaagtgaagccgaaaagcgcggaatcacgttgaaaattgccgatggtcagcaaaagcaggaaaaccagattaaagcggtacgttccttcgttgcacaaggggtggatgcgatctttatcgctccggtggtcgcgacaggttgggaaccggtattaaaagaggcgaaagatgccgaaatcccggtattcttgctcgatcgttccattgatgtgaaagacaaatctctctatatgaccaccgtcactgccgacaacatcctcgaaggcaagttgattggtgactggctggtaaaagaagtgaatggcaaaccatgcaacgtggtggagctgcagggcaccgttggggccagcgtcgccattgaccgtaagaaaggctttgccgaagccattaagaatgcgccaaatatcaaaatcatccgctcgcagtcaggtgacttcacccgcagtaaaggcaaagaagtcatggagagctttatcaaagcggaaaacaacggcaaaaacatctgcatggtttacgcccataacgacgacatggtgattggtgcaattcaggcaattaaagaagcgggcctgaaaccgggcaaagatatcctcacgggttccattgacggtgtaccggacatctacaaagcgatgatggatggcgaagcgaacgccagtgttgaactgacgccgaatatggcaggtcccgccttcgacgcgctggagaaatacaaaaaagacggcaccatgcctgaaaagctgacgttaaccaaatccaccctttacctgcctgataccgcaaaagaagaattagagaagaagaaaaatatggggtattgagggttgctatgcctgatgccgattcgtaggccggataaggcgctcgcgccgcatccggcgatggtgcactgaagcctgatgcgacgcttaccgcgtcttatcatgcctactgggagcacgctttacaccgggggaaaccatgacgaccgaccaacaccaggagatcctccgcaccgaaggattaagtaaatttttccccggcgtcaaagcgttagacaacgttgatttcagcctgcgccgtggcgaaatcatggcgctgctcggtgaaaacggggcgggaaaatcaacgctaatcaaagcattaactggtgtataccacgccgatcgcggcaccatctggctggaaggccaggctatctcaccgaaaaataccgcccacgcgcaacaactcggcattggcaccgtctatcaggaagtcaacctgctacccaatatgtcggtcgctgataatctatttataggccgcgaacccaaacgcttcggccttctacgccgcaaagagatggaaaagcgcgccaccgaactgatggcatcttacggtttctccctcgacgtgcgcgaaccgctcaaccgcttttcagtcgcgatgcagcaaatcgtcgctatttgtcgggctatcgatctctctgccaaagtgctgatcctcgatgaacccaccgccagtctcgacacccaggaagtggagttactgtttgacctgatgcgtcagttgcgcgatcgcggcgtcagcctgatttttgtcactcactttctcgatcaggtctatcaggtcagcgatcggatcaccgtcttacgcaacggcagtttcgtaggctgtcgggaaacgtgcgagctaccgcagatcgaactggtaaaaatgatgctggggcgcgagctggatacccacgcgctacagcgtgccgggcgaacattgttgagcgacaaacccgttgccgcgttcaaaaattacggcaaaaaaggaacgatcgcaccgtttgatctcgaagtacgccccggcgagatcgtcggtctggctggattgctgggatcaggacgtaccgaaaccgccgaagtgatcttcggtatcaaacctgctgacagcggcacggcgttgatcaaaggcaaaccgcaaaacctgcgatcgccacatcaggcttcggtactgggcattggcttctgcccggaagacaggaaaaccgatggcatcatcgctgccgcctcggtgcgggaaaatatcatcctcgctctccaggcccagcgcggctggctacgtcccatttcccgcaaagaacagcaagagattgccgaacgctttatccgccagcttggcattcgcacaccttcaactgaacaaccgattgaatttctctccggcggcaatcagcaaaaagtgttgctttcacgttggctactgacccgaccgcaatttctgatcctcgatgagccaacccgcggcattgatgttggtgcccacgccgagatcatccgcctgattgaaacgctatgcgccgatggtctggcgctgctggtgatctcctccgaactggaagagctggtgggctatgccgatcgggtgattatcatgcgcgatcgcaaacaggtggcggagatcccgctggcagagctttccgttccggcgatcatgaacgccattgcggcgtaaggagaacagtgtgatgcctcaatctcttccggacaccactacgccaaaaaggcgctttcgctggccgacggggatgccgcagctggtagcactattgctggtgctgctggtcgatagcctggtagccccgcatttctggcaggtggtgcttcaggatgggcgtttgttcggtagccccatagacattcttaaccgtgcagctcccgttgcgttactggcgattggcatgacgctggtgatcgccaccggtgggattgatctctccgtaggggcggtgatggctatcgccggagccacaacggctgcgatgacggtcgcgggattcagcctgccgattgttttgttaagcgccctgggcaccggcatcctggcgggattgtggaacggcatactggtagcgatcctcaaaattcagccgtttgtcgccactctgatcctgatggtcgccgggcgcggcgtggcgcaactgatcaccgccgggcagatcgtcacgtttaactcgccggatctctcatggttcggcagtggatcgctgttgttcctgccaacgccggtcattatcgcggtgctgacgcttatcctgttctggctgttgacccgcaaaacggcgctggggatgtttatcgaagccgttggtatcaacattcgggcggcaaaaaatgccggggtaaacacgcgaatcatcgtcatgctcacttatgtgttgagcgggctgtgtgcggcgattgcgggcattatcgtggcggcggatattcgcggtgccgatgccaacaacgctgggttatggctggagctggacgccattctcgcggtggtgattggcggcggatcgctgatgggcgggcgctttaacctgctactttcggtggtgggggcgctgattattcaggggatgaacaccggaattttgctttcgggctttccgccagagatgaaccaggtggtgaaagcggtggtggtgctttgcgtgctgattgttcagtcgcaacgctttatcagtctgattaaaggagtacgtagccgtgataaaacgtaatttgccactgatgatcaccatcggcgtctttgtgttgggttatctttactgcctgacccagtttcccggttttgcttccacaagagtgatctgcaatatcctgaccgataatgcctttcttgggatcattgccgttggcatgacctttgtgatcctctcaggtgggatcgatctctccgtcggttcggtgatcgcctttactggcgtgtttctggcaaaagtgattggcgatttcggcctctcgccgctgctggcgtttccgctagtgctggtgatgggctgtgccttcggcgcatttatggggcttctgatcgacgccctgaagatcccggcatttatcattacgcttgcggggatgttctttttgcgcggcgtcagctatctcgtttcggaagagtcgattccgataaaccatcccatttatgacacgctctcaagccttgcgtggaaaatccctggcggcggtcgcttaagtgcgatgggactgctgatgttggcggtggtggttatcggcatattcctcgcgcatcgtacccgttttggtaatcaggtatacgccattggcggcaacgcaacgtcggcgaatctgatggggatttccactcgcagcaccactattcgcatttatatgctctccaccggactggcaacgctggcggggattgtcttctcgatttatacccaggccggatatgcgctggcgggcgtaggtgtggaactggatgctatcgcctcagtggtaattggcggtacgcttttgagcggtggcgttggaacggtattagggacgctttttggcgtggcgattcagggactgattcagacttacataaactttgatggcacgctgagttcctggtggacgaaaatcgccatcggtattttgttgtttatttttatagcattacagcgtggattaacggtgctgtgggagaatcgtcagagttcgccagtgacaagagtcaacattgcgcagcaataaaaacgcctctccgtgtggagaggcgcaggagattacgcgtccgggaactcacggataaagcgttcgacatcttcaaccatatggtcgttgccgacaaagaatgaacggcgctggtgcagggtttccgggatgatatccagaatacgctctttgccatcgctcgctttaccgcccgcttgttccgccaggaatgccatcgggttgcactcatacagcaaacgcagtttgccgtccgggtggctggcggtgcttgggtagagataaataccgcctttcagcaggttacggtggaaatccgcgaccagtgaaccgatataacgtgaggtataagggcggttggtggatttatcttcttcctggcagaatttaatgtacttcttcaccccgttcggaaacttaatgtagtttccttcgttgatggagtaggttttgcctttctccgggaagcgcatccgttcctggcacaggcagaaaacgccgagcgaaggatcgtaagtaaaggcgtgaacaccgcatccggtggtgtaaaccagcatggtagaggagccgtataccacgtaacctgccgcaacctgtttgttaccaggctggaggaaatcttcttccgttaccggcgtgccaacaggcgtaacgcggcggtagatggagaaaatggtaccgacagagacgttaacatcgatgttggacgagccatccagggggtccatcagcaccacgtattttgcgtgttcacagccttcaaagacgacaatctcatcttcttcttcagaggcaatgcccgcaacgatatcgcgtgctttcagtgcggctttcagtttttcattagcgaacaagtcgagtttctgctgaacctcgccctgcacgttctcagcaccgctggcacccaggatatcaaccagtcctgctttgttgatatcgcgatggataatcttggcgcccagttttattgccgacagcaaagcagtgagctcaccggtagcatgagaaaactcgtgctgcttttcgacaataaattcacctaacgttttcataaaactttccctgcaatgtttatggagtaaagcgaccgcaacaatcttaacaaataatctcaatgttgcgctcaggtgaatcgcgccagcaaattacggattatcctgaaatgcgtttctcacttgcccgacatatgcgtaaaatgagcggcagattaaaaaaggatagtgacgtatgcgcattcatattttaggaatttgtggcacatttatgggcggtctggcgatgctggcgcgccagttaggccatgaagtaacgggttcggacgccaatgtgtatccgccgatgagcaccttacttgagaagcaaggcattgagctgattcaggggtacgatgccagccagctcgagccgcagccggatctggtgattattggcaacgccatgacccgtggaaatccgtgtgtggaagcggtactggaaaaaaatatcccttatatgtcaggtccacagtggctgcacgattttgtgctgcgcgaccgctgggtgctggccgttgccggtacacacggcaaaaccaccaccgcgggaatggcgacctggattctggaacagtgtggttacaaaccgggctttgtaatcggcggtgtgccggggaactttgaggtttcggctcatctgggcgaaagcgacttctttgttatcgaagcggatgagtatgactgcgccttcttcgacaaacgctctaaatttgttcattactgcccgcgtacgctgatcctcaacaaccttgagttcgatcacgccgatatctttgacgacctgaaagcgatccagaaacagttccaccatctggtgcgtatcgttccggggcagggccgtattatctggccggaaaatgacatcaacctgaaacagaccatggcgatgggctgctggagcgagcaggagctggtgggtgagcagggtcactggcaggcgaaaaagctgaccaccgatgcttccgaatgggaagttttgctggatggcgaaaaagtgggcgaagtgaaatggtcgctggtaggcgaacataatatgcacaatggcctgatggcgattgcagcggctcgccatgttggtgtagcgccggcagatgccgctaacgcgctgggttcgtttattaatgctcgtcgccgtctggagttgcgtggtgaagcgaatggcgtcacggtatatgacgattttgcccatcacccgacggcgattctggcaacgctggcggcgctgcgtggcaaagttggtggtacggcgcgcattattgctgtgctggagccgcgctcgaataccatgaaaatggggatctgcaaagacgatctggcaccttcattaggtcgtgccgatgaagtcttcctgctgcaaccggcgcatattccgtggcaggtggcagaagtggcagaagcctgcgttcagcctgcacactggagtggcgatgtggatacgctggcagatatggtggtgaaaaccgctcagcctggcgaccatattctggtgatgagcaacggcggttttggtgggatccatcagaaactgctggatgggctggcgaagaaggcggaagccgcgcagtaattcggccttagccagatatagtatgcgtaggccggataaggcgttcacgccgcatccggcatttgagcatagtgcctgatgcgacgcttgatgcgtcttatcaggcctacaggtgcaccgtatccggcaaaccatactcacatcaacaacgaaaattacccttcgttctccgctaactcgcgcagatactggaaaatctggcgtgcggatttcggcggcttattcccttctttctctttcttcgcgttgcggatcagagtacgcagttgctgacgatcggcatcgggccacagatttaatacctcagcgatggcgtcatcaccttgatcgatcagacgatcgcgcaggttttccagtttatggaacagcaccacctgctggttgtgacggtttttcagcttatccagcgcctgacgaataggctctacgtcgcgctggcgcagcatcttaccgatgagctgcaactggcggcggcgaccttccatcttaatacgctgggcgagctcaatagccgcgcgcagatccgcatctaacgggatcttatccagcgcgtttttccccagatcaacaatttccgcgccaaggcgttttagctcctcggcatcacgtttaatttcacttttactgacccagataatttcatcgtcttcgtcttcgatgtcatcaccgggaacgtcgtcgagccagtcttcgggctgcttagtcatctcaggctccttaaaaaaagaggctaatgttaccagttaagatgcgcactgaaaaacggttctctgttagacttcagagaaactctctacattatggcacttgcaatgaaagtaatctctcaagttgaagcgcagcgcaagattctggaagaagcagtttccactgcgctggagttggcctcaggcaaatcggacggtgcggaagttgccgtcagcaagaccaccggcattagcgtaagcacgcgttatggtgaagtggagaatgttgaattcaatagcgatggcgcgctggggatcactgtttatcaccagaaccgcaaaggtagcgcatcatccaccgatttaagcccgcaggccattgcccgtactgtacaggcggcgctggatattgcccgttatacctcgccagatccctgtgccggcgtggcagacaaagagctgctggcctttgacgcaccagatctcgacttgttccaccctgcggaagtttccccggatgaagccattgaactggcggcccgcgcagaacaggcggcattgcaggcggacaaacgcatcaccaataccgaaggtggcagctttaacagccactacggtgtcaaagtttttggcaacagccacggcatgttgcagggttactgctcaacgcgtcattcgctctccagctgtgtaattgccgaagaaaatggcgatatggagcgtgattacgcctacaccattggtcgtgcgatgagcgatctgcaaacgccagagtgggttggggccgactgtgctcgccgtactttatcgcgtctgtcaccgcgtaaactctccaccatgaaagcgccagtcatttttgccaatgaagtggcaaccgggctttttgggcatctggtgggggcgatagcgggtggatcggtttatcgtaaatctaccttcctgctggattcgctgggtaaacaaattctgccggactggctgaccattgaagagcatccgcatctgctgaaagggctggcgtcgacgccattcgacagcgaaggtgtgcgcaccgagcgtcgcgatattattaaagatggcatcctgactcagtggctgctgaccagctactcggcgcggaaactggggctgaaaagcaccggacatgcgggcggtattcacaactggcggattgccggacaaggtctaagcttcgagcagatgctcaaagagatgggcaccgggctggtggtgacggaattgatgggccagggcgtgagtgccattaccggtgattattcccgtggtgcagcgggcttctgggtagagaatggcgaaattcagtatccggtgagcgaaatcaccatcgcaggtaatttaaaagatatgtggcgcaatattgtcaccgtcggtaacgatattgaaacacgcagtaatatacagtgtggttctgtgctgttgccggagatgaaaatcgccggacagtaaaaaaactggcgcgacctgccgcgctataaactaaaaaattacacaaaatcattcgcactgcatcgagacggaaagtgaatgagggccggggagcgtactcgcagtacgtgacccggtcgaatgagcgtagtcgtcgatgaggcagtgtgaaggatgaagtgtaaataaaaaaggaactattcttgcagtctcctcgttggtattcagttcggcgtcatttgctgctgatctcgaagacaatatggaaaccctcaacgacaatttaaaagtggtcgaaaaagccgataacgcggcgcaagtcaaagacgcgttaacgaagatgcgcgccgcagcgctggatgcgcaaaaagcaacgccgccgaagctcgaagataaatcaccggacagcccggaaatgaaagatttccgccacggtttcgacattctggtcggtcagattgacgacgcgctgaagctggcaaatgaaggtaaagtaaaagaagcgcaggctgctgcagagcaactgaaaacgacccgcaattcatatcacaagaagtatcgttaattcctcatttccctgttgcctgcactcaggtaacagggaacttatcatcgcaaatgatgcaccacctgattgctgctgccgcgccagatcagggaagggtcttttaaatcctgcacaaatttgccgtcgaccagcacgttaatcaaatcaacaacctgcatttgcgcagcgttgagttcgtcgagtttatagcctgtccacacccagatgtctttacccggacactcggcgcggatgcgttgtaccagtttcagaatatccggcacgttttgcggatgcagcggatcgccgccggagagggaaataccctggcgtttgatacgagtgtcattcagatcgttaatgatctggtcttccattgctttggtaaatggctgaccggaatttacccgccatgtgcttttgttatagcaaccggggcattcatgaacacacccggagacaaacagggtgcaacgagtgccggggccgttgacgatgtcgacaggatagtactgatgataattcattatttcgcctggcttatcagtccgcgtgtaggctgcatccggtaatcaatgcctgatgcgacgctgtcgcgtcttatcagacctggagcaattgccaaatgtaggccggataaggcgtttacgccgcatccggcatttgcttagctcagagtgaagattaacctatctgcccattccccaaatgtttaacgcggcgcttaacttcttcctgcttaccagcgttaaacggacgtgcatccgggctacctaaatatccgcacacgcggcgagttaccgacacacgggaggcgtcatggttaccacatttcgggcaagtgaagcctttgctggtgcactcgaactcaccggtaaagccacactcgtagcactcatcaatcggtgtattggtgccgtaatacggtacatgctgatagctgtaatcccagacatcttccagcgccttcaggttgtgctgaatgtttggatactcgccgtagcaaatgaaaccaccgttcgccagcggcgggtaaggcgcttcaaagtcgatcttgtcgtacgggttcaccttcttctccacatcgaggtggaaactgttggtgtagtaacctttatcggtcacgcccggcaccacgccaaactcagcagtatcgagacggcagaagcgatcgcacaggttttcactcggcgtgctgtagagactgaaaccataacccgtttcttctttccactgatccactgcctgacgcagacgttcaacaatggcgatacctttcgcgcgaagctgctcgttgtcgtaaacatgctcgccgccgaacagcgcgttaatggtttcgtggatgccgatgtaacccagcgaaatagacgcacgaccgtttttgaagatttcagaaacatcatcgtcagcattgagacgcacgccacaagcaccttccatatagaggatcggggccacgcgcgctttcacgccttcgagacgagcgatacgggtcatcagcgccttacgtgccagcaccagacgttcatccagcagcttccagaaggtggcttcatcgccttttgcttccagagcaatacgcggcaggttcaggctgatcacgccgaggttgttacgaccatcgtggatctgctcgccgttttcattttcccacacgccgaggaagctgcggcagcccatcggagttttaaacgaaccggtgactttcactacctgatcgtagttcaggatatccggatacatgcgcttgcttgcgcactccagcgccagctgtttgatgtcgtagttcggatcgccttttttatggttcaggccatcgcgaatcgcaaacaccagtttcgggaacaccgcagttttacggtttttaccgaggcctgcgatacggttacgcaggatcgattcctgaatcaggcgcgattcccagctggtgcccaggccaaaaccaaaggttacaaacggcgtctgaccgttggcggtgtgcagggtgtttacttcgtactccagtgactggaaggcatcgtagcactctttgatggttcgagagttagcgtagccttcggcgtccgggatgttccactcttctgcggtcttgcgatgtttgttgtagctggcagtgacaaacggtgccagcacttcatcgatacggttaatggtggtgccgccataaatatggctggcaacctgagcaataatctgcgcagttaccgcggttgccgtagagatcgacttcggcggttcaatctcggcgttccccattttaaagccctgggtcagcatgcctttcaggtcgatcaacatgcagttgaacatcgggaagaacggtgagtaatcgagatcgtgatagtgaatatcgccacgctcatgtgcctgcaccacgtcacgcggcagcaggtgctgacgtgcatagtgtttagccacgatcccggccagcaggtcgcgctgggttggaatcaccttgctgtctttgttggcgttttcgttgagtaacgaggcgttggtctgctcgaccagaccacggatctcctggttcaggcgaccgcgtttttcacgttcaatgtcgcgatcgtgacggtactcgatgtaagcacgagccagttgtttgtatggacctgacatcagctgattttcaactgcggtctggatctcattgatatccacctggttgcggccctgcatctgctcgctgacaaccgcggcaacagtggcgcaataatcggcatcatcgacttccgctgctttagctgcacgcagaatcgcttctttgatgcgctctgatttaaacggcactttgcagccgtctcgtttcatcacatgcggtgtcatgatcgctccatatttttaagaacaggttatccacagaaattgggaaaggcgttttccggttttttcgtttcgttttccggtgctttccgcaatcgccatccgcttatccacaacgccgcacctttttcgtggggagctgtagtagcaattatagtcgattaatacaacatattgggttgggacgcattttaaagtctatatatagtgctttgcatcaaggatgtttgagctttttttgatgtagctcaaagtaaaaagcagagcgtacggatgacgggcgctacagcgatatgtaaattttttaatgaatttgctggttgaaaaatcaacaaaaacaacatactgacagacaaaaccccggaatgaccggcattaccggggcttagggaagatttacttctgtaaccaccagacagcctcaaaaggccgtaaattcatggcacagggttgtggtgaggcttcttcgtagttatgcatcacaagctgccagttgccgcgcatttgccctgcctgccagggttggatctcacggctaaggttggcaatgaccagcaaggtttgccccttccattcacggcgatagcaccacaatacagggctgtttggcagcagatcctggtaattgccccatgtcaggatggcttcctgcttacgcagtgcgattaacttttggtaggtgtaaaacaccgaggaatcatcggccagcgcggcttctacgttgatttgttgatagttatcgcccaggccaatccacggttcgccagccgtaaacccggcattatcgccgttgctccattgcatgggcgtgcgactgttgtcacgggatttactggcgaggattgccaataactcgtcggcatcacgcccatcgttgcgcagctcggcaaacatattgaggctctctacgtcgcgatagtcagtaatgcgcgtgaaatgcgggttggtcatgccaatctcttcgccctggtagatatacggcgttccctgcatgccatgcagcaccatcgccagcatttttgccgcaggcacgcggtattcaccttcatcaccaaagcgagaaacaatgcgcggctgatcgtggttacaccagaacaaggcattccatgctacgttgtgcattccttgttgccagtggcggaacaatgttttcaacgccacaaagtcaggtttagccagcgtccatttttcaccaccgggataatcgaccttcaggtgatgaaaattaaaggtcatcgacaattcactgcctgtcagagccgcgtatcgctggcaatgctcaaggctggtggaggacatttcacctacggtcattaacccgcgtggcgtaaacacatcgcggttcatctcgtgcaaaaactcgtgtgctcgtggcccgtcggtgtagaagcgacgcccgtcgccgtccaggtcttcagggaaacgcgggtctttggagatcagattcaccacatccaggcgcaacccgtcgaccccacgatcggcccagaactcacagacttttttcagctctgcgcgtaccgctggattctcccagttgagatccgcctgttctggtgcaaagagatgcaaatagtactgttcgctttccgcatgccagcgccacgcactaccgccaaattttgaacgccagttgttcggtggcgtttctggttctccatcgcgccagatataaaactggcggtaagggctttctttgttcagcgcctcgcgaaaccaggcatgttgggtagaggtatggttaaacaccatatcgagaatgatacgaatcccgcgcgattttgcctgcgtcaccagttcgtcaaaatcgtccagcgtgccgtaggtgggatcaatcgccgtatagttcgctacgtcgtaaccgttatcgacctggggagagacataaaagggggttagccagatggcatcaacgcccagtttatgcagatagtccaggtgttggataacgccacgtaaatcgccggtaccgctacccgtggtgtcctgaaaactctttggataaatctggtagataacgccgttttgccaccagtggggaagatgagtcattacgttattcctgcgaatgcgagggggcgcaattgcgccccgaagaaaattaaacaatgtccagcgtgcccaggcggtatttccgctgatagataaacgaggtgagtacaatcgggatgatgatggcgatagccattgccagcgcaaacacctgccagtagctcggttgaatcgagagaattcccggcaggccgcctacgccgatgccattcgccataacgccgttcaggccgcatagcaatcctgccagaccagaaccaatcatcgcgcacagcatcgggaagcgatatttcaggttgatgccgtacattgcaggctcagtgaccccaagccaggcggagatagcggcaggcacggagatctcgcgttcattgtgcttgcggctggaaatgataatgcctatcacggcggagccctgagcgatattcgacagcgcaatcagcggccacactggcgtaccacccatgctttgaatcatctgcaaatcaatagcaagcgtggtctggtgtacaccggtgatcaccagcggggcgtacaggaagccaaacaatgctgcgccaatcggagcaaagctgccggtcatcaggtgacgtaccgcaaaggcaacgccatcgccaatcatgcgaccaaacggaccaatcagcgcatgggcgaggaacaccgcgaggatcagcgaacagacgggtaccaccaccagatagaggtaatccggcacgatgcgtttaaggcgagtttcaataacgcccagcgccagtccggctaacagtgccgggatcacctgcgcctgatagcctactttggcgatgctgaacatgccaaagtcccacacttccggcagctgctgcccgagcagataagcgttcatcagctgtggagaaaccagtgtcacgccaagcacgataccaaggatcggcgtgccgcccatttttttcaccgctgaccagcaaataccgaccggcaggtagaagaagatcgcttcaccgatcaaccacagaaaatcgtagatcgtttgcagggaagggtacatttgcgccagcgtctgaccgttgctcatgggcaaatcgccgatcacattgcgaaaaccgaggatcaaaccgccgctaatcaacgcgggcagcaacgggaagaagatcaccgcgaaatgagagatcaactgctcatgccatttcatattatgccgggcggctttttttacctgctctttatcaacctgcgcctgtccggttgacgcaatcagtgcttgatagtaatcacccacgttggtgccaatcaccacctgaaattgcccggcattggtgaaacagcctttcaccatagggagttgctcaatttctttcggtctggcattggccggttggttgaggacaaagcgtaggcgagtaatacagtggctcaccgtcgcaatattgccgcgcccgccgaccagttcaatcaaccgatcgatatccgtttggtttattttgctcatcataaagccccatggcagatgacatttttggttggctgcagaatatattgcgcggaaaaatttaaaaacgggaacgttcccgaaacgcagcgaagatcacaatttatcgttcaggaaacgatcaggacagggtggcggggatgatgatttgttgcggttcgctgcgcccggttacctgcgcgatcaactggcaagccgcctggcgtccagcttcggcgtaaccgggatctacggttacgatctccggatggaggaatttcattaacggcgtattaccgacgctcgccagttgcaaggtgtcgatgcgttgctcttgcaggtatttacttgcgccaagtgccagcgtgtcggttgcgcacagtaaggcggtagtttcaggcgtaatcacttttgcaacgttctcatagccttgcttcatagcaagccctggcagggcggcaacgggatgcagtttatgcgctttgcagaacgccaggtaggcttcgtgacgtcgcttaccggttgtcacgtcactgtgcggcacgccgagataactgatattacgatgcccctggtcatacagccgttgcatcaggattttgattgccccttcgtcgtcataacagaccgaagcaaagccttttgcgtcacgcgccagcagaaccagcgatgactgccagtgggctaacatttcttctgttatgccagtaaaaccgaacagcactacgccgtcgatattacgccgtttcagcactcccaaatgttcggcaactaattgcggggaaaactgactttccatcatgattgggtcgtaaccttgttcatagaacgctggcagcatggtttgaacggcgagattttctgacaacgaatccagacgggtaacaatgatggcgaccactttatcgctttgcccacgcatagcgcgcgcagagcgggaaggggaaaatccatgctgattcatcactgcttcaacacgctcgcgggtgagctggctcacgccgctttcgttattcagcacccgggaaactgtagatttccccacgccgcttaagcgcgcgatatctttgatggtcagccgattttgcatcctgttgtcctgtaacgtgttgtttaattatttgagcctaacgttacccgtgcattcagcaatgggtaaagtctggtttatcgttggtttagttgtcagcaggtattatatcgccatagatgctacgaatattattggattctccttattatttgcggcgcttttttcacttaccggaggttatatggaacctgatcccacgcctctccctcgacggagattaaaacttttccggtaagcccgtcttttcacggcgttaccggatgcgtaaggccgtgacgttttaacgtccctgctcagctttattaccttcaggtaaggcttcgccacgcctgaagacatttctgtactgtttcagacagtgcggagggactccttatgtttaaagaaatttttacccggctcattcgccatttaccttcccgtctggttcatcgtgatccattgcctggcgcgcagcagacagtgaatacggtggtcccgccgtccttaagtgcgcattgcctgaaaatggcggtgatgcccgaagaagaattgtggaaaacgttcgacacccatccggaagggttaaatcaggcggaagtggaatctgcccgcgaacaacatggtgaaaataaattacccgcacaacaaccgtcgccgtggtgggtacatttatgggtctgctatcgcaacccctttaatattttactcaccattctcggcgctatttcttacgccacggaagatttatttgctgcgggcgttatcgcgctaatggtcgctatttctacgttgctgaactttattcaggaagcacgttccactaaagcggcagatgccctgaaagcgatggtcagcaatactgcgacggtgctgcgcgtaattaacgacaaaggcgaaaatggctggctggagatcccgatcgaccagctggtgcccggcgatattataaaactggcggcgggagatatgatcccggcagatttacgtatcttgcaggcgcgggatctgttcgtcgctcaggcgtcgttaaccggtgagtctctgcccgtagaaaaagccgctaccactcgccagccggagcacagcaatccgctggagtgcgacacgctgtgttttatgggcaccaccgtggtgagcggcacggcacaagcaatggtgattgctacaggtgccaatacctggtttggtcaactggcggggcgtgttagtgagcaggaaagcgagccgaatgcctttcagcaagggatcagccgcgtcagtatgctgctgattcgctttatgctggtgatggcaccggtggtgctgttaatcaatggttacaccaaaggcgactggtgggaagcggcgctgtttgcgctttcggtcgcggtaggcctaacgccggaaatgttgccgatgattgttacctcgacgctggcgcgcggcgcagtaaagctgtcgaaacagaaagtgatcgtcaaacatctggatgctattcagaactttggcgcaatggatattctgtgcactgataaaaccggcaccctgacgcaggataaaattgtgctggagaatcataccgatatctccggtaaaaccagcgaacgcgtgctgcatagcgcgtggttgaacagtcattatcagaccggacttaaaaacctgctcgatacagcggtgctcgaaggtacggatgaagagtcagcgcgctcgctggccagtcgttggcaaaaaattgatgagattccgtttgatttcgagcgtcgccggatgtcggtggtagtggcagaaaataccgagcaccatcagctggtttgcaaaggtgcattgcaggaaatcctcaatgtgtgttcgcaggtgcgtcacaatggcgagattgtgccgctcgatgacatcatgctgcgtaagattaagcgggttactgatacgctgaatcgtcaggggctgcgcgtggttgcggtggcgacgaaatacctgccagcgcgtgaaggagattaccagcgggcggatgaatccgacctgatcctcgaaggatatattgcttttcttgatccgccaaaagagacaaccgctccggcactgaaggcattaaaagcgagtggaattaccgtaaaaatccttactggcgacagtgagttagttgcagcgaaagtgtgccatgaagtggggctggacgcgggagaggtggtcattggtagtgatattgaaacgctatctgacgacgaactggcaaatcttgcacagcgtaccacgctgtttgcccgcctgacgccgatgcataaagaacgcattgtgaccttactgaagcgcgaagggcatgtggttggctttatgggcgatggtattaatgatgcgcccgccttacgcgctgcggatatcggcatttctgtggacggcgcggtagatattgcccgtgaagcggctgatatcatcctgctggaaaaaagcctgatggtgctggaagagggggttattgagggacgtcgcactttcgccaacatgctgaaatacatcaaaatgacggcgagctctaacttcggtaatgtgttcagcgtgctggtagcgagtgctttcttgcccttcctgccgatgttgccgttacacttgcttattcagaacctgctgtacgatgtgtcacaggtggcgatcccgtttgataacgtcgacgacgagcaaattcaaaagccgcagcgttggaatccggcggatctggggcgctttatgatcttcttcggaccgatcagctcgatcttcgatattttgacgttttgcctgatgtggtgggtattccatgccaacacgccggaaacgcaaacgctgttccagtcgggatggtttgtggtgggcttactgtcgcaaacgctgattgtgcatatgatccgcacccgccgtgtgccgtttattcagagctgtgcatcgtggccgttaatgatcatgaccgtgatcgtgatgattgtcgggatcgcattgccgttttcaccgctggccagttatctgcaattacaggcgctgccgttaagctatttcccgtggctggttgcgattctggcagggtatatgacattaacccagttggtgaaagggttctatagccgtcgttacggctggcaataaagaataaactgggcacgatagccccgattcagattgtagacaaagtgagttttgttcatgccggatgcggcgtaaatgccttatccggccaacaaattcaataaattgcaggaatcacgtaggcctgataagcgtagcgcatcaggcgattttgcgtttgtcatcagacttaatccgggcatgatagcccggatttccatcaagattagcgacgaacagcgatcgcttcgatctcaatcttcacgtctttcggcagacgggcaacttcaacgcaagaacgtgccgggaaggtggcgttgtgttcggtgaagaaggcttcgtaagtggcgtttacggttgcgaagtcgttcagatcttttacaaacacggtagttttaacgatgtcgcccactttcaggccagcggcttcgacgatcgcttttacgttatccagcgactgacgtgcctgtgcagcgacgtctgccggtacttcgcccgttttcggatttaccgggatctgaccggaggtgatgatcatattgcccagatcaacgccctgtacgtaaggaccgatagctgccggtgcattttccgtcgcgatagttttgctcatgatttctcctttattacagcggtaaaaagtctggctcattatagggagccagacttttattaccaaccgcaattaattggccagcaccacattatgggaaaactctttttcacagtatttgcatttgagcgcgatatcattggcgcgttttcgcacggcaaagctggatgaaaccggttcggcatggctgatacagttgctgttcgggcagaccagcacattgtcgatgcgctccggcagacttgggcgcgatttacccaccacttcatagttgtcgatacggttaaccgtggcttgcggcgcatacaatgccagttgatctacttgatcttcactcaaaaaggtattttcgattttgatcagatctttgcggcccatctcgccagaaggcaggttcagaccaatggtgatgcgctgatccgtttcggtcagcttgaacagactcaacagcttaaaaccgatctgggcggggatatggtcaattaccgtgccgcgtttaatagcttcaacctgcaatttattatcgtgtgtcatctctatttccccttacagtaccagatcgcgattcagaaccagtgccagtaacgcctggcgagcgaaaatcccgttgcctgcctgctggaagtaccaggcgtgtggcgttttatcaacatccgtcgcaatctcatcaacacgcggcagcggatgcagcactttcatattggctttggcgttgtggagatcgctggcgcgaagaacaaactgcgctttcacgttggcgtactcggacgggtccagacgctctttttgcacgcgggtcatgtacaggatgtctacttccgccatcacttcttcaatagagctgtgcagactccatgcgatccctttttcatcgagcatatccagaatgtattgcggcattgccagcgcgtccggcgcgatgaagtaaaaacggttgccgtcgaacttcgctaacgcctgagtcagggagtgaacggtgcggccatatttcaggtcaccaaccattgcgacgtggagattgtccagacgcccctgggtttcctgaatagtgaataagtccagcaaggtttgcgtcggatgttggttggagccatcaccggcattcagtaccggtacattgccggaaaactcggtggccaggcgcgccgcaccttcctgcggatgacgcatcactatcgcatcgacgtaagtgctgataaccgaaatggtatcggccagcgtttcgccctttttacccagtgatgtattggcgctgtcggagaagcccaccacgctggcccccaggcggtgcatagatgtttcgaaagagaggcgggtacgggtagaggcttcgaagaaacagctggcaatgactttgtgcttcaacagctctggttgcgggtttgctttcagtttcgccgctgtcgccagcaccagattaaggtcatcgcgactaaggtcgtttatggaaatgatatgtttctgatatagcggattagccatcttttatctcctgacgcctgggcaaaaaaaagcccctcgattgaggggctgggaatgggtgatcaacgggaagaaaaacggcaggccagcgtcttttttcagacgcggtaagacaaaatgtcgaacacactgaaccatacatcctcccggcaaattgtccggcattatactcatcgtcagaagcggcgcaagcatttgatgcaatattttgtcagcgcaaacggtttatttgaattaaaagtcaaggtatatgcatttttatttgatgtgattctgcaggggaactgtccttcggtatcaataattgcagacattccctgctttttcctttttcactttcacgcaatcagatatgcattttattccattcatccgacttatagggcggagtgtgaaagcgaacggctaacactattgcttactgctcagggatgcgcgctatcactttaatttcaaaatcaaagcctgccagccatgtaacacccaccgccgtccagtttggataaggtggggcgctaaatatttcatttttcaccgtcatgatgtcttcaaattggttttctggatcggtatggaagctcgtaacatcaatgatatcgtcaaaagtgcatcccgcagctgccagggtcgcatgcaaattatcaaatgccagtctgacttgttgctgaaaatcgggttctggtgttccgtcctctcgacttcctacttgcccggaaacaaacagcaaatcgccggaacgaatagccgcagaataacgatgctcagcatatagtgaatgtcggccagcagggaaaacagcggttctttctaccatttggttatcctcaagatttacgacatgaacagaagatttctctttaccgggagccgcttttagcggacgacgtgagtaaacaaaacccagacatcatggataatggctgggcttaattgagcgtagtcggttatgcgccaaacgcgccatcaatggtatgcatcgcgccggtaacaaaactggcttctggccctgctaaccatgcgaccataccagcgacctcttccggttgcccatgtcttttgatagccatcaaactatgcaacatatcgcgcattggcccgttggcgggattagcgtcggtatcaattggccctggctggacgacgttaatggtgatcccacgcggtccaaaatcacgggccagcccgcgcgccatgccttgcagggcagatttgctggcggcataagcagccatgcctgcaacaggcatacgatcgccattcacggagccgatgattaagatgcgcccgccttcgggcatctgccgggcggcttcaacagaggcatgataaggagcatgaatattgattttgaaaaggcgatcaatatcgtcggcatttaattccagggcctcgccaaagacgccaatacctgcatttaccaccaggatatccaatgcgccgctcttacgaacgacatcaatgacagcgtctctgtcagcactatctgtgaatactgctgtcgctccagtctcttgtgccaggcgtttagcggcatctttcgaccccgcataggtgaatcgtacattggccccatcggtgacgaaacgacgtacgatagcggcaccgataccacgactgccaccgaggatgagaactgtcttacctgtaaaagcgcccataaggactccttgatttattatgtaacatgcattacaaaactgttttaactttctgtcaacaggttttgtaatggtcactaaaaaacaatctcgcgttccaggtcgtcccagacgtttcgctcctgagcaggcaatctctgcggcaaaagtgctttttcaccaaaaaggtttcgatgctgtcagtgttgctgaagttactgattatcttggtattaaccccccgagcctctacgcggcttttggcagtaaagctgggttatttagccgtgtactcaatgaatacgtcggtacggaagctattccgcttgccgatattcttcgtgatgatcgtccggtaggcgagtgcctggttgaggtattaaaagaagcggcgcgcagatatagccaaaacggcggctgcgctggctgtatggttcttgaaggtattcatagtcatgatccacaagcgcgtgatattgccgttcaatattatcacgccgcagaaacgaccatttatgactacatcgccaggcggcatccacaacgcgcacaatgtgtgactgattttatgagtaccgtgatgtctgggctttctgcgaaggcacgagaggggcactctatagaacaactctgtgcaacagctgcaatggcgggggaagcgataaaaactattcttgaggagtgatgcgggccttgacccgaaaggcgggaaagcgcctgccgataagttgtgataagacaataattcacgcgttaaggctagcggaattgattatcttttcgtataacgatagaaatgaaacgttgttttaattaaggagtggaaaagatgatcatcggaaatattcataatcttcagccgtggctaccccaggagttacgccaggcgattgagcatatcaaagcacacgttacggcagaaacgccaaagggcaagcacgatatcgaaggcaatcgactgttttatcttatctcggaagatatgaccgagccgtacgaagctcgccgtgcggagtaccatgcccgctatcttgacattcagattgtgttaaaaggtcaggaaggcatgaccttcagcacgcaacctgcaggcgcgccggataccgactggttagctgataaagacatcgcatttttgccggaaggcgttgatgagaaaacagttattctaaatgaaggtgattttgttgtgttttatccgggggaagtgcataaaccgctgtgcgcagtgggcgcgccagcccaggttcgcaaagcagtagtgaagatgctgatggcgtgatgacttttcgccgtaaataactcaaggtttacggcgagtttgtgaaaagagcgttttttgatatttttttgtgagtaaaatttgtaatgcttagacgttcttattcactcaaggagttcgtcatgagcaaaatatcagatttaaattattctcaacacattacattagccgacaattttaaacaaaaaagtgaagttttaaatacctggcgtgttggaatgaatgattttgcccgtattgccggggggcaggataacagaaggaatattctttctcctggagcatttttagagtttttggcaaagatatttaccctgggttatgtggattttagcaaacgctccaacgaagcgggtagaaatatgatggctcatattaagtcctcatcttattctaaagatactaatggcaatgaaaaaatgaagttttacatgaataatcctgtaggggaacgagcggattcacccaaggtgattatagaaatttcactttccactatcactactatggggactcgtcaaggacatacagccattatatttccacaacctgatggttcgactaaccgttatgaagggaagtcctttgaaagaaaagatgagagttcattacacctgattactaacaaggttctggcgtgttaccaaagtgaagctaacaagaaaatagcgcgtctattaaataataatcaggagttaaataatctacagaaattaaataatctacagaagttaaataatctactgaagttaaataatatacaggggttaaataatcctcaggagttaaataatccgcagaatttaaatgattctcaggagttaaataactcgcaggaattaaatagtccacaggagttaaatgatccgcaggagttaaataattctcaggacttaaataactctaaggtgagttgtacagtttcagttgattctacgattacgggtttattaaaagaaccattgaataatgcattattagcaataaggaacgaacatctgctattaatgcctcatgtatgtgatgaatcgatttcatacttactgggcgaaaaaggtatacttgaagaaatagataagctctacgcattaaatgatcacggaattgataatgacaaagtaggtaacaatgaaattaatgacatcaaagttaacctgtctcatattcttattgattccttagatgatgcaaaggttaaccttacaccggtcatcgattcgattctggagactttttcaaaatccccatatattaatgatgtaagaatactggattggtgttttaataaaagcatgcaatattttgatgatactaaaaagataaagcatgcatgctccgtaataaatcatattaatcttcgcagcgatcagtctaaaatagctgagacattatttttcaatctcgataaagaaccctataaaaatagccctgaattacaggggttgatttggaataagttggttgtatatgtcaatgaatttaacttaagtaatcgagaaaaaacaaatttaatacaaaggctatttgataatgttgagtctatatttaatgaagtacctgtcagcattttagtgaatgatatttttatgaatgatttctttatgaaaaatcctgagatgattaattggtacttccctcagttacttaagagttatgagggtgaaaagatttattttgataatttaaaatatgatttaaatgataatgataaggaatctaataaagaaattttgaagaatcaaccagataatgttatcaaagaaaaactgaataatgaatacaaacttagatttagaatgatgcaaactatcttgcaatcgagagttaatgtattaccatatattaatgaacagcgtttaaataaactaaatccaccggaaaatttacgtatagcaatagaacactttgggtggaagaatagacctatcactgcataaaataatgtgatgccgggatggtttgtatttcccggcatctttatagcgatagcaattatttactgagcgtcgcgaccatcaccgctttgatagtatgcatacggttttccgcctgatcaaaaacaatgctggcggcagattcgaagacctcatcagtgacttccataccgccatgtaggccaaattcttccgccattttcttgccaagcgtcgtttggtcgtcatgaaacgcgggcaggcagtggaggaatttgacctccgggttaccggtcaactgcatcatcttgctgttcacctgatattcacgcagcaatgcaatccgttccgcccatttctcttttgcttcccccatcgacacccacacatcggtatagataaagtcagcaccttcaactcccttcgcgacatcttcagtcagcgtaatattcccaccattttgctgtgccagggcgcggcattccgtaaccagcgcagcttccggccagcacgcttgtggcgcgaccagacgcaaatccagaccggtaagcgccgcagcttcgagcatcgaattgcccatgttgttacgcgcgtcacctgcatagaccagcgtcatttcgttgaacgctttgccgggcaaatgctcctgcatggtgagaagatccgccagcagctgcgtgggatggaactcattggtcaggccattccataccggcacgctagcgtattccgccagtgtttcgacaatctcctgaccatagccgcgatactgaataccgtcatacatgcgaccaagcacgcgggcagtgtctttaatcgactctttatgaccaatctggctgccgcttgggccgagataagtaacgcgagcaccctggtcatatgcggcaacttcgaaagagcatcgggtacgagtcgagtctttttcgaagatgagcgcgatgtttttaccagtgagtttggcttcttctttaccgcttttcttatcggctttcagcttcgcggctaactgcagcaggctgttgagttcagctggcgtgaaatcgagtaatttcaggaaatgcttatgataaaacccggacatagatccctcctgtggctaacgcctcaatgaattaaaattcaatttatatggatgattattcatttgcaagtctaaagcataaatctttgtcacaaaggtggaggcaatgtcagtggtgtgtgacaataagagtatcggcaggacattaagaggaatgagccatggcaaacccggaacaactggaagaacagcgtgaagaaacacgtttgattattgaagaattactggaagatggcagcgatccggacgcgctgtacaccatcgaacaccatctttccgcagacgatctggaaaccctggaaaaagcagcagttgaagcgtttaaactcggttacgaagtgaccgatccagaagagctggaagttgaagatggtgatatcgtgatttgctgcgacatcctcagcgagtgcgcgttgaatgccgatctgatcgatgcccaggttgaacaactgatgacgctggcagagaaatttgacgttgagtacgacggatggggcacttactttgaagatcctaacggcgaagatggcgacgatgaagattttgtcgatgaagacgatgacggagttcgccactaattaagcgtagcgcatcaggcccaggtagttcctgcaacctggtgaatttgtagcccggataaggcattcatgtcacatccggcataaacaaaacgtacgttgttaatgttcgaatgcccgcgagttgaacacgcgggcatttttttagagttcgcgcaacatccgcacttcacaatcgacatggcccgtgcagccaagcgcatagtcgatatgctcaaagcccaaatgctcataaagcgcaatggcttcctttaaaaaagcggtcgtttccagatagcagcgtttgaaacccatctctcgcgcctgctccatcgccattaaggccagtttttttgccagccctttgccgcggatagccggaagaaaatacatcttttgcagttcgcaaatatccgactcactcccggttaatggcgctatcccaccgccgccgaccacttcaccctcgtactcaacgacccaatatgcatggccaggctgactatatacttgatacagctcgtcaagattcggatcggcgacggtgtagcctttatcagcggtaagaccgtattcggcggatacctgacgaatgacgcgggcgatagcaggattatcctgcagcgtcaggcgacgcattacaggtgattgcggcgcaatgttattcatagtttaacccaataaaaataaagtaattatacatttgtttaataccactctcttcttacgtacgcaagcgacttataaagtaataaagtttttgccagcctattactgataagagtattgtaacgtggcagaacattttactgtctgtatatataagttatatcaatggattttttaattcagggaatttttatggctcaagttattaatgaaatggatgttccgtcccattcgtttgtttttcatggtacaggtgagagatattttcttatttgtgtggtgaatgtgttgttaacgattataacgctaggtatctatttaccatgggcattaatgaaatgtaagcgttatctttatgctaatatggaagttaacggacaacgattttcttatggaattaccggtgggaatgtttttgttagttgtcttttttttgtttttttctatttcgcaatcttaatgacagtgtcagcagatatgccgcttgttggttgtgttttgactttgttactgttggttttgcttatatttatggcagcaaaaggactgcgtcatcaggccttaatgaccagtctcaacggcgtaagatttagttttaattgctctatgaaagggttctggtgggtgacctttttcttgccgattttaatggccattgggatggggactgttttctttatctcgacaaagatgctacctgccaatagttcaagtagtgttattatatccatggttctgatggcaatagttggtattgtttccattggtatttttaatggtactttatatagtctggtaatgagttttctctggagtaataccagtttcggtatacatcgtttcaaggtgaaattagatactacgtattgtataaaatatgccattctcgcatttttagctttattgccttttctcgctgttgctggttatattatcttcgatcaaatattaaatgcgtatgatagttctgtatatgcaaatgatgacattgagaatttacagcaatttatggaaatgcaacgtaaaatgataatcgcgcagttaatctattattttgggattgctgttagcacaagttatttaacggtgtctttgcgaaaccattttatgagcaacctgtcactgaatgatgggcgtattcgttttcgcttaactttaacgtaccacggtatgctttatcgcatgtgtgcgttggtggtgatatccgggattacgggcggtctggcttatccactgctgaaaatatggatgattgactggcaggcaaaaaatacgtatttgctgggcgatttggatgaccttcctttaatcaataaagaagaacaaccagataaaggcttcttagccagtatttcacggggagttatgccttctttaccatttctgtaagagataaaaaaggccggagcatgctccggccttcgttttcatcactgtgttttgattacagcgcggcgataacagcctgctgttcaatcagtttcgctttcgcttccgcatagccttccagcttctcacgctctttcgcgatgaccgcttccggtgcgcgggcgacaaagccttcgttcgccagtttgttctcgatacggctgatttcaccttcaatcttcgccacttctttcgccagacgcgccagctcatcttctttgttgatgaggccagccatcgggatcagcagctctgcaccgtcgatgatcttcgtaacggaaaccggacctttgtcatcggcaggcagcacggtgatactttccagacgcgccagggtttgcaggaagccacggttttcatttacgcgacgttctgcatccgcgctgcaaccacgcagcagcagctccagcggtttgcccggcgcgatgttcatttctgcacggatgttacgtaccgcaacgatcgcctgtttcagccattcggtgtcggccagtgcggcttcatcaacctgagatgcatcgtactgcgggaacggctgcagcatgatggtgtcggcagtgataccgcaaagtactttcacacgctgccagatggtttcggtgatgaacggaatgatcggatgcgcgaggcgcagcagaccttccagtacagtcaccagcgtatggcgagtaccgcgcagttctgcttcggtgccaccgttcattaccggcttggtcagctcgagataccagtcacagaactggttccaggtgaactcatacagaatgcctgcggcgatatcgaagcggaagctgtccagcgcttcgcggtacgctttgatggtctggttgaactccgccagaatccagcggtccgccagcgacagcgtcatttcgccgccgttgaagccgcaatcctgaccttctgtgttcatcagcacaaagcggctggcgttccacagcttgttacagaagttacggtaaccttccagacgcttcatatcccagttgatgtcacgaccggtagacgccagcgccgccagggtgaagcgcagcgcgtcagtaccgtgcggctcaataccgttcgggaactgcttctcggtgcgcttacggattttgtccgccagctgcggctgcatcatattgccggtacgtttttccagcagttctggcagcgaaataccgtcaaccatatccagtgggtcgataacgttacccttggatttggacatcttctggccttcgtcatcacgaatcaggccggtcatgtaaacggtgtggaacggcacctgcggtttgccattttcatctttgatgaagtgcatggtcatcatgatcatgcgggcaatccagaagaaaatgatgtcgaaaccagataccatcacgctggttgggtggaactgacgcagggcgtcggtattttccggccagccaagggtagagaaggtccacagcgcagaagagaaccaggtatcgagaacgtcttcgtcctgacgcaggacaacatcagcaccgaggttattttctttacgcacttcgtcttcgttgcggccaacataaacgttacccgcttcgtcataccatgccgggatacggtgaccccaccacaactgacgagagatacaccagtcctgaatatcgcgcatccaggagaagtacatgttttcgtactgcttcggtacgaactgaatgtcgccgttctcaaccgcttcaaccgccggtttcgccaggacatcggcacgcacgtaccactggtcggtcagcattggttcgataactacgccgccacggtcgccgtaaggaacggtcaggtcgtgcggtttaatttcttccagcaggccaagcgcgtcaactgcggcaacgactgctttacgtgcagcaaaacgctccagtttctggaactctgcagggatttcgctggaataaacgtcagattcgttacctttggtatcgaacacctgggcgctttcacggatatcgccgtcaaaggtcaggatgttgatcatcggcagggcgtgacgtttacccacttcatagtcgttaaagtcgtgcgccggagtgattttcacgcagccggtgcctttttccatgtcggcgtgttcgtcgccaacgatcggaatacgacggttaaccagcggcagaatgacatatttgccaatcagatctttgtaacgcggatcttccgggttaacggctacgccagtatcgcccagcagggtttctggacgggtagtcgcgaccaccagataatctttaccgtctgcggttttcgcaccgtcagccagcggatagcggatgtgccacatcgaacctttcgattcgcggttttcgacttccaggtcagagatagcggtgcgcagtttcggatcccagtttaccaggcgtttgccacggtaaatcaggtcttctttatacagacgaacgaaaacttctttcaccgcattggacaggccttcgtccatggtgaagcgttcacgctcccagtcgacggagttgccgagacggcgcatctgacgggtaatggtgccgccagattccgctttccattcccagattttgtcgatgaaagcttcgcggccgtagtcgtgacgggttttaccttcttctgcggcaatcttgcgctcaacgaccatctgggtagcgatcccggcgtggtcagtaccgacctgccacagggtgtttttgccctgcatgcgctgatagcggatcatggtatccatgatggtttgctggaaggcgtgacccatatgcaaactgccggtgacgttcggcggcgggatcatgatgcagaaactttcctggctttcatcgccattaggcttaaagtagccctgcttttcccagtgctcgtaaagcggctgttcgatatcttgtgggttatatgtcttttccattatttccaggttgccgtattcaggttgaaaccagccacgcggtaggctttatagcgttcgcgcgccagttgtttcagagaatcttcataaggaacgaagtctaccacttctgtgaaagcggtggcaaaatctgcaaagcttgttcgcagactaatcaatatatcgcgccggctgctgctacgcttttgcggccaggcgatctccaccggtgcaccgccgcgcggtccttctcccgctaaattatgcggaacaaagctttctgccggacgcgcccacagggcttcatccagccggtaagcctgcttttcatcttcacaggcgatgagcacgcgcttaccgctgcgccaacgttctgcggcaatttcacacaccagttgctcaacggcgcttaagccatcgacggtggtgtcattgtccagaaggtagaacgtcgcgtttttcataaatggggcttcttgtggtggatttaaatacgcatcaggtatacaccgcagcgcctgatgcgacgctgttgtgtcttatcaggcctacgagttcagtgctgtgtaggtcggataaggcgttcacgccgcatccggcaataacagccttgcctgacgcaattactcttcgccgttaaacccagcgcggtttaacaggaactgtgccagcaacgctaccggacgaccggtggcgccttttgctttaccagaacgccaggcggtaccggcgatatccaggtgcgcccagttgtacttacgggtaaagcgtgacaggaagcaacctgcggtaatcgccccaccaggacgaccgccaatgttcgccatatcggcaaaattggactccagttgttcctgatactcgtcacccagcggtaagcgccatgcgcggtcaccggattgttcagacgcggcaatcagttcatgggccagcggattatggttcgccatcagaccagtaatatgatgacccagcgcgatcacgcaggcaccggtcagcgtcgccacgtcaatcaccgcttccggctcaaaacgctcaacgtaagttaacacgtcgcacagtaccaggcggccttcagcgtcggtgttcagcacttcaacggtttgaccggacatggtggttaacacatcgcccggacgataggctcgtccgccaggcatgttttcgcagcctgccaacacgccgataacgttaatcggcagttgtagctccgcgaccatccgcatcacgccgtaaaccgctgccgcaccgcacatatcgtacttcatctcatccatgccttctgaaggcttgatcgagataccgccggagtcgaaggttaaacctttacccaccagcacgattgggcgtgcatcttccgacgcgttgcctttgtactcaatcaccgacatcagcgattcgttttgcgaaccctgaccgaccgccagataggaatgcatccccagctctttcatctgctgttcgccgataacgcgggtgatgacattcttgctgtagctgtcagccagctggcgcgcttgtgaagcgaggtaagcggcgttacagatattcggcggcatattgccgagatcttttgctgctttaatcccggcggcaatcgccagaccgtgctggatcgcgcgctcaccgctggtcagttcacggcgggtcggcacgttgaacaccatcttacgcagcggacgacgcggttcgctcttgttcgttttcagctgatcgaaactgtagagcgtctcttttgccgtctcgacagcctgacgcactttccagtagttgttacggcctttaacgtgcagctcagtcagaaagcagaccgcttccattgagccagtatcattcagcgtattaatggttttctgaataacctgcttgtactgacgctcatccagctcacgttctttgccgcaaccaataaggagaattcgctcggaaagtacattcggaacatggtgcagcaacaatgtctgccccggttttccttccagttcgccccgacgtagcagggcgctgatgtacccatcgctgattttatcgagctgttctgcaatcggagaaaggcgacgtggttcgaagacgcccacgacgatgcaggcactccgctgtttctccgggctaccgctttttacactaaactccatgcactacgctcctgaatcttaaagacaacggcggtggctacagatagaattgcaagctttcgtaactcatgtccgctgttgcgatgacttcgtgttaatcttaacgttattacggcattggcacgtcagaacaaaatctgagaggtgaatccgttgagtataattatcttagcgacgatttcgacgactcaagagaataaatgacgtttaagccatgaaacaagctaaaatcctgcaaaagacgagtttttacgggcgtatttaaagtgataatcataagatatctggtgcgggagacgctcaaaagccagctggcgatactcttcatcttgcttttgatcttcttctgtcaaaagttagtgaggatcctcggcgcagcggttgacggcgatattccggcgaatctggtgctctcccttctcgggttgggcgtgccggaaatggcgcagcttatcctgccattaagcctgttcctcgggctgctgatgacgctgggcaaactgtataccgaaagtgaaattacggtaatgcatgcctgcggcctgagcaaagcggttctggtgaaagcggcaatgatccttgcggtattcacggcaatcgtagcggcggttaacgtgatgtgggcgggaccgtggtcatcgcgtcatcaggatgaagtgttagcagaagcgaaagcgaaccctggcatggcggcgctggcgcaagggcaattccagcaagcgactaatggcagctcggtgctgttcatcgaaagcgttgacggcagcgatttcaaagatgtgttcctcgcgcaaattcgaccaaaaggtaatgcacgtccttctgtggtggtggccgattccggacatttaacccagctgcgcgacggctcccaggtcgtcactctcaaccagggaacgcgcttcgaaggcactgcattgttacgtgatttccgcattacggacttccaggattatcaggcgatcattggtcaccaggcggtggcgctcgacccgaacgataccgaccagatggacatgcgcacattgtggaacactgacaccgatcgtgctcgcgcagaactgaactggcgtatcacgttggtattcaccgtgtttatgatggcacttatggtcgtaccgctgagcgtggttaacccacgtcagggacgcgtactgtcgatgctgccagccatgctgctgtatctacttttcttcctgatccagacctccctgaaatcgaacggcggtaaaggtaagctggacccgacgctgtggatgtggaccgttaacctgatttatctggctttagcgattgttctcaacctttgggacaccgtgccggtccgccgcctgcgcgccagtttttcgcgtaaaggagcggtgtgatgcaaccttttggcgtacttgaccgctatatcggtaaaactattttcaccaccatcatgatgacactgttcatgctggtgtcgctgtcgggcattatcaagtttgtcgatcagctgaaaaaagccgggcaggggagttacgacgcgttaggcgcaggaatgtataccttgctgagcgtgccgaaagatgtgcagatcttcttcccgatggcggctctgcttggggcgttgcttggtcttgggatgctggcgcagcgcagcgaactggtggtgatgcaggcttctggttttacccgtatgcaggtggcgctgtcggtgatgaaaaccgccattccgctggtcttgctgacgatggcgattggcgaatgggtcgcgccgcagggcgagcagatggcgcgtaactaccgtgcgcaggcgatgtacggcggctcgttgctctctacccagcaaggcttatgggcgaaagatggcaacaacttcgtctacattgagcgggttaaaggtgacgaagagttaggtggcatcagcatttatgcctttaacgagaatcgtcgtctgcaatccgtacgctatgccgctactgcgaagtttgacccggaacataaagtctggcgtctgtcgcaggttgatgaatctgatctgaccaatccgaaacagattaccggttcgcagacggtgagcggcacctggaaaaccaacctcacgccggacaaactgggcgtggtggcgctggacccggatgcactctctatcagcggtttgcacaactatgtgaagtatctgaagtcgagcggtcaggatgccggacgttatcagctcaacatgtggagcaaaatcttccagccgctatctgtggcggtgatgatgctgatggcgctgtcgttcatctttggcccactgcgtagcgtaccgatgggcgtgcgtgtggtcaccggtatcagtttcggttttgtcttctacgtactggaccagatcttcggcccgctgacgttggtttatggcatcccgccgatcatcggcgcactgttgccaagcgccagcttcttcttaatcagcctgtggctgttaatgagaaaatcgtaaccgaatgaacgaataaagggagcgaaagctccctttattattgttagcaaagtgtgcttcgttcattcctgaaaaataattaaaattcaatatattgcagtggggtgggcatgataagacgcgccagcgtcgcatcaggcaaagacaaatctcgcctgacttaccttcttctcccccccagcaaactccccaacatcccgcgtacaatctgattcgtcacttggcgagcggcgcttttggccattgtttgcaccacaccatctttcttcccgccgcgtggtccggtagtgccgaacaaaatatccttcaatccaccaagaatgccgtcatccaccgctacctctttccctttcgcgggaggattattttgctgctcggtactggcctgaaagcctttttgcaacatctcataggcggattcccggtccacctcatcctcatatttgccatacaccggagagtgattaatcaagccattacgctcatcttccgtcaccggccccatccgcgaacaaggcgcgatcaccatcgcacgctccaccacagaagggcttcctttcgcatccagaaaagagatcaacgcctcgccggtgcccagttcctgaatcgccttttcggtatcaaacgccggattggcccgcatggtttgcgccgctgccttcactgctttctgatcttttggcgtaaaagcccgcaaagcatgttgaacgcgattaccgagctgcccgagcacattatccggaatatcagacgggttttgcgaaacgaaccagacgcccacgccttttgagcgaataagccttatcacctgctcaatcttatccagcagtacctgcggggcatcgttaaacagcagatgtgcctcgtcgaagaaaaacaccagttttggtttctccagatcgcccgcttccggcaattgttcatacaactctgaaagcatccacagcaggctggcggcgtacagtttcggcatctgataaagtttctcggcgctgaggatattgataacgcctttaccgttggcatcggtgcgcatccagtctttgatatccagcatcggctcaccaaagaagtgtgctgcgccttgctgttccagcgacaacagcccgcgctggatggcaccaaccgatgcgctactgatattaccgtactgattctggaaggatttggcgttatcgccgatgtactgggtaattgcccgcagatctttaaagtcgagcagtaacagcccctgatcgtcagcaatgcggaagatgatattcagcacgccagattgcacatcgttgagattcaacagtcgtgccagcaacagcggccccagatccgaaaccgtcgcccgcaccggatggcctttctcgccaaagatatcccacaccaccaccggattggcatgcggttgccagtcattgacgccgatatttttaagccttgcgagcagtttttccgacaccgttcctgcctgcgcgacgccggtcagatcgcctttcacatcagccataaacaccggcacgccgatttccgacaatgactccgccagtttttgcagcgtaacggttttacccgtccccgttgcgccggtaatcagcccatgacggttagccattcccggcagtaaaaacagttctgtgtccggcgtgcgggcaattaacaggggttcactcatgagatatcctccagtttcctgcctggagtataggcaacgtccggcaaagagaatacgtgtaatgaagagaaaataacctaaagcgtgttgccgtgataaatctgatacccgaggtcaacagtgttgtggttgtgatcgttatttttaattttgctcagcaacatttgggcggccatccgaccaatatcaaaacggggagtaattacgctggcgaggcttgggatcatttgcctgccaatctccagcccatgaaaacccgcaatggaaatttgttctggcacggcgaggtttcgctcgcggcacagcagaagcgcacccatcgcaatatcgtcattggtgcaaaatacaccgtctaaatccgggtttgcgctaagggcatcacgcattaactgcattcctaaatgaatggatgagatggcgcgtggattcatgcgtaatggggaaagattatgcagcatcatcgcatcgcaatacccctgataacgctgttcatcgcgggtgtcatctttggaaccgagatacagaattttgtgcctgactcgcttctccagcatggtacacaccatgtcaaaagcggcctgccgattatcaaaaccgacctccatatccagccgttctccctgtacatccatcaattccacgaccggaatggtggctgaacgcagaaatttcaccgtcctgatggtgtgatatttttccgaaagtataatcccgtcaatgttataagagagcaggttaatcaccgactcttcttcggaatcgcgatcgtaattgtaattagcaataagggtctgataattatgctcagaggtgacggattctattcccgcgagaatgtcagcgaagagttgattttgaaatgacggaatcaagataccgagggtataactttgtgcattcaacaacatgccgggagcgcgattagggatataattgatctcttccataattttggcgatgcgctcgcctgtttcctttgccacctttttcggcgagcggatataacgactcacggtcatttttgttacgccagccagcgtagcgatatcctgtaaagaaattctgtgattgcgcataacttctcccaacgtcgggggaatcttcaatcttcccccgaaactacatcacaatattttattctttcagtgcaatacggcgttaatggctaacacgcccagcaaacccataatagaaataagggtttccatcaccgtccaggtacgcaacgtttcaccaaccgtcagattaaaataccctttaaatagccagaagccagggtcgtttacgtgtgacgcgatcacgctgcccgcaccggttgccagtaccattaaagcgggatcggcatgggtaacgttgataatcggcaacaccacacccgcggtggtaatggccgcgacggtggcagagcccagagcgatacgcaacagcgccgcaacagtccagcacatcaataacggcgaaagtgtagttccggtcattaagtgtgaaatatagtgcccgacaccgctatctactaatacctgcttaaacgcgccgccgccagcgataataaacacaatcatcgcgatagcgcctatagaatccccaatgatatccatgatttgctcgatggtgcgtccattacgtcggcccagtgtgaaaatcgcaataacaatggcaataaacagcgcaacggcagggttaccgacaaattcaaagaagaggcgcacggtgttagttttcggtaacgtaatttcacaaacggcggcgatagccatcaggatgaccgggatcacggcagcgaaaatactgttccagaaggagggcatctcctcttcgctaaacagatgaggattaaataagccttccggtggtgctttctcaaagcgagttagcagtttagaaaacagcggtcctgcgacaataactgtcggaatggtaatgataaatccatacagtaaagtcgttccgagattagcctcaaagatagtcgcgatggcagtaggccctggatgtggcggcagaaaacagtgggttacagagagcgctgctaccattggtacgccaacatacaacaggggtaatcctgatgatgctacgatggtaaataccaacggcaacagcaggacaaaacccacttcaaaaaacatggcgaggcccacaaccagaccggtgatcactagcgcccattgcacgcgttttttaccaaaagtagcaatcagcgtagtggcgatacgttgtgccgcacccgtatcagaaatcagcttgcctaacatggccccgaaaccgaggatcattgccagcccgccgagcgtgctgccgataccattttgtatagagtgcaggacggcctgtgcatccatcccttcggcaaatccgacgacggcagctaccagaacgagggcaataaagccgttaactttaaagccgatcatcaggataagaagcagcgcgacgcctgccgcaataatgattaatggcatagtctttatctcttattagtgccagaaaagcagcgctttcgcgctgcacgtaggggggctgttaaacagccactaacatgccgccatcaacaaacaacaggtggccgtttacgaaatcagaggcttttgaagaaaggaacaccgcagcaccaatcagttcctgcggatctccccagcgtgcggcgggggtccgtttgcacaaccaggcggtgaaggcttcgtcctcaaccagtgctttagtcatttctgttttgaaatagcccggcgcaataccgttgacctgaatattgtggcgcgccagctcgacgcacatgccgcgggtgagcatttttaccgcccctttcgatgcggcataaggggtgatggtgtcacgtcccagttcgctttgcatcgagcaaatattaataactttacctgccttgcgttcaaccatgtgacgagttaccgcttgcgataccaggaacacggcggtctggtttactgcgatcacatcattccactcttgttcagggaactcagtaaaaggatgacggcgctggataccggcgttattcaccagcacatcaatggggccgatgtccttttcgatatgttcaacggcggcatcaatttcatgtttatgagtaacattaaaaggtgcggcaacggcctgaataccctcctggtggagtttttctacagcaagttctgcgcgttcggcagtaatatcattaataattatttgtgcgccatatttacccaggccggttgccagtaaaaagccaatgccctgtgctgaaccggtaatcaagatattttttcctgccagtgaaaatagatcgttcattgtattattcctttatttatctcttagaaaacaagctggacttttgctgcctgggttttatcaccggcgaaacgtagcgcctcttccaggtcagtgaagggatattcagcactcagtaaaggcagtggattgataacgccattcgccagccatgacactgcggtattaaattcgctggtaaaacggaaagagcctctgagtgaaatctccttaccaatcaacgtcatcattgggaattctgccatcgcgcctcccatacctacctgcaccattacgccgcgtgcacgagtgacctccagacaggtattcactgatgaaggatgaccggacacttcaaagctgacatcgaaatagcctttttccgctttccagtgatccatgtcgtcgttttgtgggtttacgagcacatccgcccccatctctttgcccagcgaaagggaacggggactcacatcagcacagacaatttccgcggcccccagtgttttcactgcactgacaatcaggcagccaatgggtccaacaccggaaataaatactcgcttgccctgtaactcgccggcctgatgtgcggcatgaatcgcgacggctaaaggttcggcaaaagccataaccttttcgtcagctttggccggataagggacacattgcgacgtttcgaccattttataacgggtaaaaccaccatcaacatgagggaaatacatggcactgccaaaaaaacgcatatctgtacactgattctcgttatgttcaatgcagtatttgcagtgaccgcacggtttagacggattaatggctaccgtttgcccttcatgtaattctgatgagtcgctatgaataactttaccgataacttcatgacctaacaccatcggtgcctttatcatgaaattacctacttttccttcctgataataatgtaaatcggaaccgcaaattccacctcgggttatttgtactaatgttccattattattccaatctatcgtctgctcggtaacggcaacagttttcttgcccgcaacaacgcaggactgtgttttcacttgcataaattcctcactggtcaggtagacacctcggaagcatttaagcggttttaactgtcattatttgtgatgaagatcacgtcagaaaattgttacattactatgttacgcataacgtgatgtgccttgtaattcttatcagtagaaataaaaaaacgtgaaattattatgccgccaggcgtagtatcgcagcaggtaagatgattcaggagattttaaatggcgggtgaaagctttattttgatgggcgtttcagggagtggtaaaacattaattggtagcaaggttgccgcgttattatctgctaaatttattgatggtgacgatcttcatccagccaaaaatatagataaaatgtcgcagggtattccattatctgatgaagatcgacttccctggctggaacgcttaaatgatgcttcatacagtctttataaaaagaatgaaacaggatttattgtctgttcatcattaaaaaaacagtatcgtgatattttacgcaagggtagcccccatgttcatttcctctggttagatggcgactatgaaactattctcgcgcgaatgcagcgtcgggctgggcattttatgccggtagcgttactaaaaagtcagtttgaggcactggagcgtccacaagcagatgaacaggatattgtgcgcattgatatcaaccatgatattgccaatgtcaccgaacaatgtcggcaggctgtgctggcgatacgacaaaacagaatatgtgcgaaagagggcagcgcctcagatcagcgctgcgaatgattttcaaaaatcggctttcaacaccacgcggtaacgcgccttaccgtcgcgcacatgctggatggcgtcgttaattttcgacatcgggaacagttcggtggtcggcgcaaccttgctgcgggcggcaaaacgcatcagcttacgcagctcataaggcgtgccggtagcagaaccagagacgctgcgatcgcccgcaattaacgtaaaggccggaacagacagcggcgtgagaaccgcaccgaccgtatggaaattaccgccataggtcagcgcctcaaaatagggctgccagtcgaggctgacgttgacggtgttgataatgagatcaaactgccccgccagtgctttcagtgcctgcggatcgcggctattcaccactttatcggcacccatcgccagcacttcctgctctttcgccggattagaactaaaggctgtcacctcgcatcccattgcgtgcagaagttttatagcgatatgccccagcccgccaataccaattaccccaacgcggctggtagcagtgatatggtgcatcaacagtggtttaaagaccgtgataccgccgcacaacagcggcccggcggactcgatatcaatattttctggcagtggaatcacccattgccagtccgcacgcaacttctcggcaaagccaccgcgattcataatcgtcggcaccgcaccttgctcgcagttgatctgattaccgctaatacaggcgtcgcagtgaccacagctacgcgccgtccagccaatcccgacacgctgaccgacctgcaaacctttatcctgcgcggcgctcccgagtgccaccacgcgcccaatcacctcatgcccggcaaccagcggatattgtgaaaatccccattcgttatcgatcatcgacagatcggaatggcagatcccgcagtaatccacctgcacttcaacatcttgtggcctcagctcaccgggatcgtactcataaacttccagttcgccgcccgcttcttttgcggcatagctttttatcatcgacattttttggtccttctctggtgttgtttgggaagtgtagagcatggcagggcggggtgcctggagtgtgacaaaggttacacatcgctgtatgcaatgctgaaaatttcagcacttagcgaggtgcgagcaagctggcgcttgcatggtggcgtgcgacaggtataatccacaacgttttccgcatacctcttcagtgccgaagtggcgaaatcggtagacgcagttgattcaaaatcaaccgtagaaatacgtgccggttcgagtccggccttcggcaccaaaagtatgtaaatagacctcaactgaggtctttttttatgcctgaaatccagtgtttatctatctttcccgctatattaactctctcaaggtcaaccgatatcaacgtacatctaccaacatatgttggtacagatgatggtatttccggttcgataatgcttgtaccaacagggagggaatacgatggcattaacagatatcaaagtcagagcagccaagccaacggataagcaatattagctgactgatggtggcggtatgcatctgcttgtccatccaaatggttctaagtactggcgtttgcagtaccgttatgagggaaagcaaaaaatgctggcacttggggtttatcctgaaatcacactagcggatgccagagtacgtcgtgacgaggcgcgtaagctgcttgcgaatggcgtcgatccgggagacaaaaagaaaaatgataaggttgaacagagtaaagcacgaacctttaaagaagtcgcgattgagtggcatggcaccaataaaaagtggtctgaagatcacgcccatcgtgtgctaaaaagtcttgaagataatctttttgcagcgcttggtgaacgtaatatcgctgagttaaaaactcgagatttattagcacctattaaggccgtagaaatgtctggacgtcttgaagtggccgctcgtcttcagcagcgcactacagccatcatgcgctatgcagtgcaaagtgggttaattgattataacccggcacaagagatggctggggcggttgcttcctgtaatcgacaacatcgtcccgcgcttgaattaaagcgcatccctgagttgcttacaaaaatagatagctatactggtaggccgctaacccgatgggcgatagaactcactttgctgatctttattcggtccagtgagctgcgttttgctcgttggtcagagatcgatttcgaagcgtctatatggactatcccaccggagcgggagcctattcctggagtgaaacattcccatagaggctcaaaaatgcgtacaacgcatctagtgcctctttcaacgcaagctcttgcaattttaaagcagataaaacagttttatggggcccatgacttgatatttattggtgatcacgattcgcacaaacccatgagtgagaatacggtaaatagtgcgttacgggtcatggggtatgatacaaaagtagaggtttgtggtcatggctttcgaacaatggcctgtagttcattggtcgaatcaggtctgtggtctcgtgatgctgttgaacgtcagatgagccacatggcgcgaaattcagtgagggccgcgtatatccataaagcagagcatctggaagaacggcgattgatgctacagtggtgggccgattttctggatgtaaacagagaaaggtttatcagtccatttgaatatgcaaagattaataatccattaaaacagtaatcatcccgggcaaatgcccgggaattattctaggattattttctttgttaaaaaagacaaacggtattaactgatgtatttactatttaccgctccctgcaggggggattatcagaatccgcggttattcattatttatatacattcaataaaaaagtaacctcataaaaaatcctgtactcacagggtgatgcgggataactgacgtaaggagtgctgcagggatttgatggtcccttgtagactggccccctgaatctccagacaaccaatatcacttaaataagtgatagtcttaatactagtttttagactagtcattggagaacagatgattgatgtcttagggccggagaaacgcagacggcgtaccacacaggaaaagatcgcaattgttcagcagagctttgaaccggggatgacggtctccctcgttgcccggcaacatggtgtagcagccagccagttatttctctggcgtaagcaataccaggaaggaagtcttactgctgtcgccgccggagaacaggttgttcctgcctctgaacttgctgccgccatgaagcagattaaagaactccagcgcctgctcggcaagaaaacgatggaaaatgaactcctcaaagaagccgttgaatatggacgggcaaaaaagtggatagcgcacgcgcccttattgcccggggatggggagtaagcttagtcagccgttgtctccgggtgtcgcgtgcgcagttgcacgtcattctcagacgaaccgatgactggatggatggccgccgcagtcgtcacactgatgatacggatgtgcttctccgtatacaccatgttatcggagagctgccaacgtatggttatcgtcgggtatgggcgctgcttcgcagacaggcagaacttgatggtatgcctgcgatcaatgccaaacgtgtttaccggatcatgcgccagaatgcgctgttgcttgagcgaaaacctgctgtaccgccatcgaaacgggcacatacaggcagagtggccgtgaaagaaagcaatcagcgatggtgctctgacgggttcgagttctgctgtgataacggagagagactgcgtgtcacgttcgcgctggactgctgtgatcgtgaggcactgcactgggcggtcactaccggcggcttcaacagtgaaacagtacaggacgtcatgctgggagcggtggaacgccgcttcggcaacgatcttccgtcgtctccagtggagtggctgacggataatggttcatgctaccgggctaatgaaacacgccagttcgcccggatgttgggacttgaaccgaagaacacggcggtgcggagtccggagagtaacggaatagcagagagcttcgtgaaaacgataaagcgtgactacatcagtatcatgcccaaaccagacgggttaacggcagcaaagaaccttgcagaggcgttcgagcattataacgaatggcatccgcatagtgcgctgggttatcgctcgccacgggaatatctgcggcagcgggcttgtaatgggttaagtgataacagatgtctggaaatataggggcaaatccaccttgtgctgatatgaatacggatattttatacagaatacttttcagtacaagcgactgtattacagtctgccatatatgattacctgtgatcaggaagaataagtggctgaggtttcaaactgtctgccggtatattcctctctcccttaaaaaccataacaggttagttatcttcgtctgtcagcggattgaatggcggtatattttcagtacaaataccggtcatccactgaaaaatacctgcgaaatgacgggcactgatttttctactgacgggctgatgagacgttatgtcactggcggtaataatcagtggcacactgtagcctccctgcacatgaccataatgatgaacaggattggcactgtcgctgaccgacagcccaaggccagaaaagtaaagcatggcgaaatgacgtgagtaccggcgaaggataccatcaagctggccaagaaagttatccagtttactgatgctggcgaggtaacaggcaatttttcggggatactgctccaggtaattattcggctaggagttaaggctgtcacacggatttggatgagaacccatcatgtgcaggaaaattatcttcggagaggatgtatccgccagcgcacgttctgtttcctgtaacaacagtttgtcatctgttttacgggaagcgaagctgcctttcttgaggaaagtggcatgctccgcatcagaagcaataacagagatgcgtgtgtcatgctcccccagttttccttgattggatatccaccatgtgctgtatcctgcttttgctgccagcgccaccacattgttgccggaatcagggttctgctcatagtcataaatcagtgtccggctcagggaagacactgtactggaggctgtcgaggtataatcgtcaataaataaaccgggtgccgtattcagccacggtgtggttggtacgggatagtcatacactgacatataatccctgcgcacactctcaccagtgacaataacaatcgtatcatataacggtgctcccggctggattttccagttgtcagccccgtgctactcagttgttcataacgctgcatttcacgtaatgtgtcagttgtccccacaactgttcctttaaccatccgcaatggccaacggtttacagagcataatacgaatagccgtagagccagccagttacggtggtcgcgatggtgtgtccgccagaaaatcaccacgaataccagaatcgcggcactgaccagaaaatgataaacaggaaacacggggcggttcactttgctttctcctgtagtgttttctgtaggttctgaaccggttctagcggggttgtgaggctgatggcaatcgccgggctcttcctgcatgttacactggtactgcaagagggggccttcgctcctctgacattactcagtattttcactactacaccccatctgccatccataacaaccgattcaccccctcgcgaggcgttgttgcccgtcacccggacagacaccgttatggacttctcttgttgcacgatcgatcaattgttatgcatgctgacaccacaaccccggtgggtatgaccgatgcctttctcactctcttcccggtcatcgtcggccttccccgttattgtggcgtgtcagcaccctcgacggcatttcgatggctgctcagtgttcactcacgttacggcccgcataacccgttgacttcctgaagaagtcgtttcagggagagattcagcccttttgttacctcctggaccgcttcttgtccttccagtcggagcgagagttagccggggcggactttcaccgacggaaagatcgtgcatttcaaggcacacacaacaatatctgcgagcgtgctatccgtccggtcgttatgggacgaaaggcctggttgttcgctggttcactggtggccgggaaccgcgcggcacagataatgagccttctgggaaccgcagtctggagccacatgcttggctgacggacgtcctgacgcgtctgccggagtggccggaggagaggttggctgagttactgcctcttgagggctttaccttcttcgggtaagtgatacctgccgtcaggtgtttgtgcaccgggccataacctgcagttgggaattgaacgcctgacaacaggaaatgagctagagcagtaaacacgcgggctgacaatgggtcagaatatgagttagcccggcgttattcctggggtcagtacttcagatctagcctccggtaccagactagctagcccctacgcaaccaaataaatcaaccatcgtcagagtgcaatcgttcatatacactgtcggtgatgcgctaaaaaatgcgttaatgttgagttcctcgaacccttaccaattaagggacatagccagatacgcaactggctgatgcaagcagtctaatgtctttagatccgctggcctgcgggcatgacaatgtcaaacagtcaaagattgtggcgttgacggtcagtcttggggacaaaaaagctcagtattctcgttggcaaccagataatttaacagttgatgctgaaacgaaataggcatcttggttctgtaatgccagtcagttaagcaactgactggctctttttcggggctgtggggtatttccagggcctctcctttaccactctcgggaaggccctttcccttcttgtcggtaatttcacaagttgtcccatacttgcaagatcgcgcatcagctccggtatacgtcccggtgaagcgccctgcaatgtcatcagcattctcatcaccattccgcatgattctgagaaactcagttgattcggccagtaacctttcagatgttccgccattttaatcatctgatatctcaccagattataagccagtaagacaccccacagctcttgctccacaagctccggctttttacttctcagcgtcagcctgctccgttgcatcgtctgttttatctccctgtatcccagttcgatttcccagcgatgactgtacagatcccccatttctcctccggggaagcgcatggcgtccgtcatcgacgtcagcagatggcagacttttcctttgcgcgtcacggtcagcaggcgggcagtcacttcatttcccagtcccggccacttttttcgtgcctgcgggctggttttcagcttcaccagatgatcgcctttacccagttttctgatctcttcatattgcgctccctttctgagaggtatcatccagtggcggtgttctcccgccaggctccaggcatttaacagtcccagtgagtaataacctttatccattaacgtcagagtgttatcgccggtttgttctataagttgctcagcaagctcattttcgctgttcttcatcgtgccgaaggctgcagccgtcagcagatggctggtcagttccatctggcagaccattttgacctgcgggtagagcgccgggttcccggcatgtgtctggcgggggaaggctgcatcgttctctggtgtatccggtgtgcgccagaacacaccatcgatggccagcagggtcaggccgcaccagtgcggatgcggcgtggcgttatgccagagctgcgctgttttcgtgaacacgcggcggacagcctcacttcccaggcgctggcgggcctgaataacggcactgggggcaacgaaggggcgattgcccggcagcatgatgtccaggcgattcacaatctggtgaagaggttctttacgctcaagcgccatgccaacaatacaccagaccatcatttcgaggggaagacggcgcttgcgtagcgttacagtacctgattcggcaaggcaacgagagatgagttcggggtcgaggtaatcccccagagaagtcagtgggttacgcagagaatcgtaacgggataccagatcaagagcctgtccaatgtgcataaaaaaatccggaaacaagtgagcgtttccggattcttacacagccactggatcggtcaactgatccttaactgatcggcattaatcttggttctggtgtttgtaacaaactatcagctacaaaaatatgctcaatttgtgacatcagtaacaaaacgcgttttgttatgtggattgcttgttttttgatctggtataacaggtataaaggtatacagaaaagcaaagaaatactgcaaaggaaaacagctataacgtaagctaaagtaataacctctcagtctttcctcatttgacgaagggagttttattcaacctgaacggactacgaaaatgagcacaatgaataagtcaatttttgaagcagggttgaactgtgccagtggtggaatatctggcgaacattgttttttgttggtgacccaaaactgtaggtgggtatcagttttatctttcatagagtgaaatatgttaagaagaaatggaggaaaagattgtactgattaggtattgataacaatcaatagtactggcgtatttgaagacaatataattatttctggatattgttgaggctccctaatatttactttaagggctatattagaataacacaggaaacaaatatggcaacagcatggtataaacaagttaatccaccacaacggaaagctcttttttccgcatggcttggatatgtatttgatggctttgattttatgatgatattttacattcttcatattataaaagcagatcttggcattacggatattcaggctactttaatagggacagtggccttcatagccagacctattggaggtggtttttttggtgccatggctgataaatatggtcgtaagccaatgatgatgtgggcaattttcatttactcagtcggaacaggccttagcggtattgctacaaacttatatatgctcgcagtttgccgttttattgttggcttagggatgtctggtgaatatgcatgtgcttcaacttatgcggtagaaagttggcctaaaaatcttcaatctaaagctagtgcttttttggtaagtggtttttctgttggaaatattattgcggcacaaataatccctcagtttgctgaagtatatggatggagaaactctttttttataggcctgttaccagttttactagttctttggatcagaaaaagtgctccagaaagtcaggagtggattgaagataaatataaggataaatcaacatttttgtctgtcttcagaaaaccacatctttcaatctctatgatcgttttcctcgtctgtttttgtctatttggtgcaaactggccgataaacggactacttccttcctacctggcagataatggagttaatacagtggtcatttcaactctgatgacaatagcaggtttaggaacactgacaggtacaatattttttggttttgttggtgataagattggtgtaaaaaaagcctttgtagtcggtctaataacttcatttattttcctttgtcctcttttttttatttctgtgaaaaactcttctcttataggattatgtctctttggattaatgtttacaaatttaggtattgcagggttggttccaaaatttatatatgattactttccaacaaaattaagaggattagggaccggtcttatttataacttaggggcaactggaggaatggccgcacctgtattagctacatacatttcaggatattatggcttaggtgtttcattattcattgttacggttgcattctctgccttattaattttgttagttggttttgatattccaggtaaaatttataaactatccgtggctaaatgattggaggctttatgattaattatggcgttgttggtgttggatactttggcgctgaattagctcgttttatgaatatgcatgataatgcaaaaattacatgtgtatacgatcctgaaaatggagaaaatattgcccgtgaattgcagtgtatcaatatgtcaagcttggatgctttagtctcaagtaaattagtcgattgcgtgatcgtagccaccccaaattatctgcataaagaaccagtaattaaagcagcaaagaataagaagcatgttttttgtgaaaaaccaattgcattaagttatgaagattgtgtggatatggtcaaagcgtgtaaagaagctggtgtgacctttatggccgggcatattatgaattttttcaatggggttcaatatgcacggaagttaattaaagaaggtgttatcggcgaaatattatcatgtcatactaagagaaatggctgggaaaacaaacaagagagactttcctggaaaaagatgaaagaacaatctggtggacatctatatcatcatatacatgagttagattgtgttcagcatttacttggagaaataccagagacggttactatgattggtggaaatttggcccattctggtccaggatttggcaatgaagatgatatgttatttatgaccttggaattcccgtcaggaaaactagcaaccttagagtgggggagtgcatttaactggccggaacattatgtcatcatcaatggaactaaaggctctattaaaattgatatgcaagaaacagcagggtcacttaggattggcggtcagacaaagcattttttggtccatgaaacacaagaagaagatgatgatcgtcggaaaggcaatatgacctcagaaatggatggcgctatagcatatggtcatccaggaaaaaaaacaccattatggcttgccagtttaataagaaaggagacgttattcctccataatatcctctgtggtgcaaaacctgaagaagattatattgaccttctcaatggtgaggcggccatgtcggcgattgctactgctgatgctgccactctttcaagatcgcaggacaggaaagtgaaaatcagtgagatcattaaacatacatcagtaatgtaaaaactatacgcctcttgatttaattcaggaggccttttatgtatgatcaagaattttatcttcgataatctcataattttagcagtgccatttatgataaaaacatcccttaaaaccaatctaatctttttcttcctctgtgtatttgttccccatatggcgtcataatttacgctacgtaatacgggatagttacgatacgcagcgatagcgctaagttttagttaaaatcccccatcagcgggatatggggatctctgggaggttcaggttttagcatcgcgactttaatacgacagacgctggtgacgatgatgccaagtagtgactcttccgaataaggttcccactgaccaattggcgcgcgcttcgcaataaaatctcccttcgcccagtattgggaaaagtagatacattcaaactgtgtacgctgtttcgtctcacagttcacgacattgctggccgatgagctgaccattgggcctatccgggctgtcccgatggatattacgccgaagtatgtgggaattgccagcggattgatgaacgccggttccgctgtcgccgacattatttcacctatcgcctttggcattattatcgacaaaacaggcaactggagtttaccattctacggttccgtcgcattgcttgttattggtatattcctgacgttcttcatgcgtccagataagtcattgtaaaagtcgaatcagggctgaagtggcacactgaatttggccacctgaacagaggtgatatgctcacctcagaacaacacaggtgctccaatgaaaaaaagaaatttcagcgcagagtttaaacgcgaatccgctcaactggttgttgaccagaaatacacggtggcagatgccgcgaaagctatggatgttggcctttccacaatgacaagatgggtcaaacaactgcgtgatgagcgtcagggcaaaacaccaaaagcctctccgataacaccagaacaaatcgaaatacgtaagctgaggaaaaagctacaacggattgaaatggagaatgaaatattaaaaaggctactgtagattcaatctgtcaatgcaacacccctttcaattatctctttcggtgttttgaacttcagtgtctttctcggtctgttgtttagctgagcagcaaccagatctagttcatgttgagtatattgggcaagacatgtctttttaggaaagtactgccgaattagcccatttgtgttctcatttgttccccgctgccaaggactctgaggatcgcagaagtaaactttaacgccggtgctgacagtaaattctagatgtctggccagttccattcctctgtcccatgtcagtgattttctgagttctgacggtaaactcaggaatttgtcggtaagagcctgatttactgagacagaatctttgcccctgagtctaaggatgatcgtataacgtgattttcggtctacaagtgtggctatatgagagttttttgtacctgagactaaatcgccctcccaatgccctagagagcgtctgttatcgatatttcgggaacgttcgtgaattggtgttccgttcactatgttaatcgtacctctttcgcctttgcgggtatgacgcctgccatggcgaaggctatgcgaccgtcgcagatgctgtatattcaggtggtgtagcgcttcacggctacgaaagtacagcgttttataaattgtctcaggtgatattcgcagcgttttttgacgtggttttgttcgccttaaccatcctgatatttgctctggagaccatttcatctccagcttttccagaacaagctttcgcaatggtaaattttgatccagtaagcacggttttggccttttcgccattctgttggctcggttattagcatcaacagctttgtaatagcgtctgccccgattacgctgaacttcacgtgagatcgtcgaaggactgcgattcagcgcagtagctatcgcacgaatgctcattttggctgacaaaccagctcgtatctcctcgcgctcagacagtgtcaggtgagctacagcccgcttacgctcatggggttttatgccgccagtatcccttaacatagtgaagatcgttccgggttttgaacccaggatattcgctatttcactgaagcctgttccgttcttccatagttcaaaaacagaggctttttcctctgctgtaaatgttcgtctcattcaaaaaacctccgcaaccccatgttttcacataactgttgcgttgaccaattgaatctacagttgctttttttaatatatctcgctcaaggcgagcttcatttaacgccttacgcagttgcagaatttcagattccagttcagccaccgtgcgggaaccaggagtaccgagcccttttctggcggcggtaacccattgtcctaaagtgccttcaggaagagataatcgggaagcgccttcactgatcgaaagttgattttcaagaaccgttctgacagcttcggctttgaactttttagagtaacgttgggtttttctgctcattattagctccttctgatgccattctatttcaggaaggagtgtccgttaaactcaggctacctcaggaaaaaccgtcctgaaaaaccagacggcagacgggctgtattacgcagtcaggtacttgagctacatggcatcagccacggttcggccggagcaagaagcatcgccacaatggcaacccggagaggctaccagatgggacgctggcttgctggcaggctcatgaaagagctggggctggtcagctgtcagcagccgactcaccggtataaacgtggtggtcatgaacatgttgctatccctaactaccttgaaaggcagttcgccgtgaccgagccaaatcaggtgtggtgcggtgatgtgacctatatctggacgggtaagcgctgggcgtacctcgccgttgttctcgacctgttcgcaagaaaaccagtgggctgggccatgtcgttctcgccggacagcaggcttaccatgaaagcactggaaatggcatgggaaacccgtggtaagcccgtcggggtgatgttccaagcgatcaaggcagtcattatacgagcaggcagttccggcagttactgtggcgataccggatcaggcagagtatgagtcggcgtggaaactgctgggataacagcccaatggagcgcttcttcaggagtctgaagaacgaatgggtgccagcgacgggctatgtaagcttcagcgatgcagctcacgcaataacggactatatcgttggatattacagcgcactaagaccgcacgaatataatggtgggttaccaccaaacgaatcagaaaaccgatactggaaaaactctaacgcggaggccagttttagttgaccacaacagactacctgaagggagccgcggtcgcctggcagttgcagtagcaggagatcatccagccgcagtacaggtcacgatgactctggttaatgataccggctttgaccccgtattttccggctctatcgctgaatcatggcgtcagcagccgtgcacaccatcctattgttgtgactgggaggctgccaccatgcttcgcgctttccctctggcgaaaaagggagaaggacgggcccgtctgccttcactttatgccagcttcggtaagctgggtgagacaccgactcatgaagatatcattgataacaatcgatccatcaactggcctgtataacgtggctgccggtgattaagaaagctgcacctacctaagtagtagcaaacgcacactttttagaaaaatcgatggtcagaaactggattagcaattccgttccatggttgcttttgatttacgttggcgtctgatcattgatttatcctcaaaagcccaacctcattggtaatgaaccagctccgtgaatgtccgctctggcacagagcgaaattttttgatctcccccctgaaatctaaacttagtcatgtcacgtttttgggtttctaaaattttaacttcgcgtttttcgttgccgtaagggttatacagaaatgtccgttaagcagagttcaaaattgattgccgtgatcacgactggtttgaaagccgcgcccaagcctgtacagctctggtttgcgttgattatgaacctgtcagcctaaagcaagcggatggacgatgagtattggtaatctttcagagtccggaaaagttcagccccagtctgaacaggcttgctggcgccagtccagtttcattcagtcgtggtttggttcttacggcctgtgcaatctacctcattaggcacatcggcctgccagataccggctcggggtgtatttccgcttccacgctgaatactgttctcagcaatcctggggtcatcacctcttctggtgtgccttgcgccataacatgtccgtttgccattaccaccagttgatcgcagtaccggctagcctgattaaggtcgtgcagcacagcgaccaccgttttcccctgagtccggagttcgcccatcaaccgcatcaggtccacctggtgattgatatcaagataggtggttggctcatcaagtaatacaacgggcgtattctgggccaggaccattgccagaaatgcgcgctggcgctgaccgccggaaagctcggttaaccgacgaacggcaagatgattgatccgggtctggttcatggcgacattaactcgtgcattgtcttcagcggagagacgcccccagagtgacagccagggattacgaccatacgaaaccagctcctggactgtgatcccctctggcgttaaatggtgctgaggcagcagcgaaagcctgcgggccaactggcgcgatgagagcatatttatgggattatcgccgagaaatacggtgccagactgcggcattaaaagccgcgaaaaacagtttaacagcgtcgatttcccgcaaccgttaggaccgatcagggcggtgatcttccccgttggcagtgagagtgaaacgtcgttaagtaccttgtctgtcccgtaactgaccgtcagattttcagttcgtaaagtcatttatcgcattctcacaagcaaccagacaaaccacggcgcaccgataatggcggtcagcacgccaaccgggagctccagtgggggatgaataattctcgccagcagatcggcaaccaccaacagcaacgcacctgtcagggccgaaacaggcagcagtctgcggtgacgtccaccggtgatgctacgcatcatatgcggcaccacgagaccaataaagctaatcgggccgcaggcggccacgccggtagatgtcatggcgacagctagtaacaaagcccagaatcgggtatggggcaccgacacaccgagcgtggtggcgcgcgcatcgccgagtgcaaggaggtcgagatcgcggcaaaaactcaggctcagcggcagaaataaaatcatcagcgggatggcaatcttcacaaagctccagtcacggccccataagctgccggtcagccacagcagggcgttgttcacatcctgcgggcgcgagagcatcagataatccgtcaggctggcccagcatgcagaaagcgccacgccggtgagcgccagcttcatcggctggtgggtctttgccagcatcttcagcaatatcaaccccgccatgccgcccgcaaaggccagcagcggcagcaccatcacgggcagtgacggcataagaagtagagcccccacagaggccaggctggcggcatggttaacaccgagaatatccggtgatgccagagggttgcgcacaatcccctgtatcagcacgcccgccacggcgagggctgcaccgacaaacagtgccagcagcaagcgcggcagtcggtactccatcaatacataataatgctcgtgtccggcctgccagtcggtcagcagcgcgcgccacggcacggggatcactcccatatggagtgataacagcgcacagcccgccagggcaagggtgatgaaaataaccagcgcaattttcatcctcgcctcctcacaagccagacaaagcaagggctgccaatcagcgccagcactgcgcctgcgggcagatctccggggaaggccagcgcgcgtgcgagtacatctgccagcagcatcagcgtggcccccagcagcatgctcactggcagtacgttgcgctgatcgaagcctgcccagaagcgcgccagatgtggcaccagcagaccgataaacgccaccggacctgctacgctgacgcacgcaccaaccagaagcagcactaacatattgatgaccaaacgtagcctcgtcaggttcactcccagcgtatgggcggtgctgtcgctgaggttgagcaggttcagttgattcgccagcagcaacacgacagggactgcagtgaccaccaccggcaagagctgccagacatcctgccagcgggcgtgggacactccgcctgccagccagtaaaagatgccgtaagcatgatcttcggccagcagcagggtgatgcgggtaaggcccatacaaaaggccgacagcgcgatacccgcgaggatcagtttgtttctgtcatgggtatgacgaaatccgcctcctgcggtcatgaccagcagccagctcacgccgcccccgcatgccgcgatgaatgacagagaatagcctgcaatcggcgtcggactcagcgcgctggtaagcgccatagccagcgccgcgccgctgttaatgccgagcagtgaaggagaggccattgggttgtgggtcagggtttgcagcagcgtgcccgcgagcgccaggcttgcgccgatcagaacggcgaccaggcttcgtggcaaacgaaggttttgcaccagcgcttctggtagcgttggcgtgtgtccaggcagcagggcgcgggttgcatctgctccggaaacaggaatggccgagtagcaaaacagactcagccagaaaataataataagtgctgcaacgggaagcccccacagcagcaccgggtgttttatcgcggtcatttcacaacggtaagcggctgatggtggaagatttttaccgtgtcagcggcaatacgctctgcagcaaaaataccgcgcatccgcgcccaggtgttactgtcgaccgaagcaacctgctgcttctgcgcggcggttaacatctgccagagcggatcttgttgccagcgtttaacaatgctctcttcgcgatagtgggcaaccagcagccaggcaggattgaccgccagcagttgctccaggccgatggacggcatggacgcacccgccatcgcagcgggaacgttcagccccagagaggccagcacgctgccggtccaggtctcctgagtatgcaggttgaattgctgttcgcgtgatgtgccaaaggccacgcgtgtccctttgggaagctggctggcccactgcgccatcctctctttatgttgttccagacgtgcctgcatctctcgctttttacccaccatttcgccgatgatagccgcagattgcaaattttcagcgtaggtttcgttgcgggacttaagcagcagtaccggcgcgatttgctgcaaggcgatgtaaacccccgcatggcgactgctgtcggcaatgatcaggtctggtttcagagcggcaatggcttccaggctcggctgcgcgcgcgttccgacggactgccacggtttcaggtgcgcacgcacttcgggcaggatgcgttttgcatcgttatcgtcggcaataccgatcgggatgacgtccacggcggccagcgcatcggcgaacgagagttccagcaccacaatccgttgtggcgttttttcgagtgtaaacgtgccgtgttcgtcctgaaccgtggcggcaaaggcgtggctgatcaccagcagcaggcctgcaaaaagaaaacggataaatgccaacataatcacattccagctaaaagcccggcaagccgggcgttaacacatcagaacttcaacgacccctgcatatacagcgtgcgcggctggcctgcatagatgcctttgttgttgtcgtcataagagcggatgaagtagtcctggtcgaagatgtttttcacaccgaatgccaggttcagatctgccatctgcgggccaaagtcatacgccacgcgtgcgccccagagcatgaagccgggaatgcggccggtactgccgtcggcgctctctttcaccgtattggcgttatccgcaaactggctggactggaaatcgctgttcagattgaacgtccagtttcctggcttgtagtccacgcccagcgtgcctttatgtttcggggagaatggtaccagattgccgtaggtgtcgcctttctcgcggatttccgcgttcacatacgcatagctggcgtagatggaaacgttatcaagcgttggcgttagcgtacccagatcgtaacgtgcctgcgtttccagcccggtatggcgcgttttgccacgtgcagtgacggtgtcgttggtctggttggagtcgtactgattgttaaagttaatcaggaacagccccatttccgccgtcagcgcgccgtcgtcgtagcgggtaccgagttcccaggttcgcgctttttccggttcaacattgccgctttgcacagccttgccaatctggctgtactgtacggtgccgaacgagccttcagtgtttgcataaagattccagctgtcagtcaggtgatagagcacgttcaacgccggaagcggtgcgttatagctcacttcttcgtgcgtgcctgtgatggcgttgttctggtatgactcgatatgttcgaaacgcatacccggcgtgatggtccagttgccgatgtcgattttgtcatccagataccaggcgtgcgcctcggtgccggaacgcgtatcgcggtcgtaagggcttgagccggacggcaactgcccgctgctggtggcggtgtagtaacgcatttcatgcgttgattcattcaaatagcgatagcccacgcccacttcgtgcgcggaagggccgatcataaagatctggctgtagcgtggctcaataccgcgcacccagtagttacgcggcgagagggtgatgcgtttgccttgctccaggtagccgctgcgcagggtttgggtgtagaacccctgaatgttgaatttatgctggctgtctggctggaactggtagcccaggctcgccagcttgcgacgaccccagaagcggtcatacgggcgggtggattgccagcgatcggcgtcgtaatccgcgcgagacaggccaccgggcatgtcggcttcaccgtcgtaatattgcagcaggctgttgaaggtgtgcacctcatccggcgcatatttgcttttcagcatcaggtcgtcgatgcgggtggcgctgtgctcgcgccagtcactgccgcgcgtgccggagtagagcagcgcggtgccaaaaccgttgtccgctgtgccgcccaccatcaggttgtgcgtctctttcgggttgttttgtgaagaggttgggctgagctgaccttccacgcccgcctcgataccaaagtcctgcggaatggcacgggtaacaaagttcaccacgccgcccacgctctgcggtccgtaacgcaccgcaccaccaccgcgtaccacgtcaatggcatccatgttgccgagcgaaacgggagccagtgaaagctgcggctgaccgtaaggggcgaaggggacggggatgccgtccatcaggacggtcgagcggctggcgaggcgcgggttcaggccccggatgccaaagttcatcgccaggtcgtggctgccggtgccgttgttttccggcgcgctgacgccagggatgcggttaagtacctcacgcatggtggttgcgccggttttggcgaaatcctcacggcggatcacgtcacgcgcgccagcatgttcaaatacgtcgttttcacgcgcatcacccagccagtcgccgaccacggtcagggcatcttcttttggtgcgggcgcgggctccagcgtccagctgttatttcccagcggttttacctgcagtccgctgccgtccagcagttgttgcaggccgctctcgacgtcgtaatcgccgtgcaggccgttgctctgcttgccgcgcgtcaggctggcgtcaaccgagagggtaaatccgctgtgtgcggcatactgattgagcgctttatcgagcgatcccggtgcgatattaacctgtgcagcaaaagcggaaaacgagagaccggccagcggcagcaggctcaggcgaatggtgttaaccaaaggtgttgttttacgaaaaacgcgtaacggcgtcataccttccccatcatcatttttgttgtgttcagctatgagtcgaacgagaagggtaaaaaggacaatcgaaataagaattattttccttacagtggtgaaatgtttatccagtaccgcgtaatagactgaattttaacgggaagcgtttgcgcgataacgttcaggatcgcatcggtatttttcagcgggaacgtcccgctcaggcgcagcccggcaacggcgggatcgcagcgcagcacgccgttgcggtaacgggttagcgtggctatcacctcacccagcggtttatcgctgaagctcaggatgtccttcgtccagcttgtactctcgtcatccagcggtttcactgcgccaaactcagaggcgctgaactgcaggctttcaccagcgttcacgatgcgtttttgcgcgggggcactggcgagaagcacttccacagcgtgctgctgcacgtcaagctgcgtgaaattatcctgctggcggacggtaaattctgtccctaaagcagtgagctggccctgacgggtcaggacacggaaggggcgttgcagggcatctttcgcggtagtaatggcgatttcaccgtaccagagccggacggtgcgctgatgcgcatcaaaacgcacatccgccgcgctttgggtattcagcgtgagcagggagccatcttccagttgctgacggctgactgtgcctttggcggtgcggtaatctgcccgcagaccttcgccggtttccgactgccagagctgccagcctccgccagcgccgagcaacagcagtaatcctttcatcacgtgacggcgggtgaggcgggtatcgtgcaacgcccggctggcaacgtcgccaggcacaccgccaagctggttgcgcaggttttcaacctgctgccaggcccactggttatcctgatcctgttcataccactgttgccagcgcgcttcctgttgtgggctgacgcgctcgccgcttagcacggcataccagtgggaagctgaacgcagcgcctgacggcgggaatcggttaacaaaggattcataacccatactccagacggaacagcaggcagtgctcgacggctttcgccacgtattttttcacggagctgatggaaacaccgagtttgtgcgcaatctcgctgtatgtcagaccatccagttgcgaaagcagaaacgcttcacgtgttttgccgtttagcccgtccagcatgctgtcgaggagttgtagggtctcgagttggctttcgcgttcctcaggtgaaggcgctcccccctccggcataagcgccagcatctccagatacgctttttccagcgcgtttcggcgaaacaggtccaccatcacgcgtttggcgatagtgcagaggaaggagcgaggatcgcggatcgtcgagagcgtttcgctgaccattacccgcaaaaaagtgtcctgggcaatgtcatctgcatcaaaagcagactggagtttgcgcgtcagccagcttttcaaccagccgtgatgtgtgccataaagcgactcgaacgttaaggaagctgtggtagtggcgcggtcagacatgcggagtgcatcaaaagttaattatcacgtagtcatattaatatgagaatggttatcattacaattggaaataaaattgtttccaatagacatttttaacatgttgtttttctaagtgttataaggtaggtataaaatgggatggagcctctgcttctggcatgtgtcggtcagaatgactcatgatgtggtctgctattattgacatcctcactgccctaaaggatggggatttcggtaatgctgccaacttactgatttagtgtatgatggtgattttaaggtgcttgcgtggcttccatttccatcagatgtccttcctgctccgctactgaaggcgtggtgcgtaacggcaaaagcactgccggacatcagcgctatctctgctctccttgccgtaaaacatggcaactacagttcacttacaccgcctctcagcccggtaagcaccagaaaatcattgatatggccatgaatggcgtcggatgtcgcgccagtgcacgcattatgggcgttggcctcaacacggttttacgtcacttaaaaaactcaggccgcagtcggtaacctcgcgcatacaaccgggcagtgatgtgattgtctgcgctgaaatggacgaacagtggggctacgtcggtgctaaatcacgtcagcgctggctgttttacgcgtatgacaggatacggaggacggttgtggcgcacgtcttcggtgaacgcactctggccacactggagcgtcttctgagcctgctgtcggcctttgaggtcgtggtatagatgacggatggctggccgctgtatgaatcacgcctgaagggaaagctgcacgttatcagcaagcgttacactcagcgcattgagcgacataatctgaatctgagacaacatctggcaaggctgggacggaagttactgtcgttctcaaaatcggtggagttgcatgacaaggtcatcgggcattatctgaacataaaacactatcagtaagttggagtcattaccgaccatgtttatttcatacattgtgggtattgttcttattatcgccgctaatcaataaaatcctgccccatatctacatggggcagttgttcattcttttagtgtggtaattcacacgccagcaaaaactctgccgttccttcatcaacaatcaggtccgtgacatatcctcccagcagggcacccaacgttgcgtcatagcctctttccccaccagcaaggaagatcttccgttcaatctgccttagctgagccagactgattcccagaatacgctggtcaacatcagccacgacgggcatcccttccttgtcatagaagcgaccacaaatgacacctactgcgcctaaatcccgatacgtctgcatttccttcttattcagcacgcccacccgaatcaggggattttcatcaagcgcgttacccacgacaaaaaaggctttcgtacagcgagtcagaacgtcaaaattcgatcgaataataggctctgcctgtaactccatggccagtctggcgcttgataccacggcgggcacgtgcagcgaggcgacacggcctgaaagcttgtaggcgatttgcgatgaggattcaatgatcgtcaggtctggctgagatggcatggaaccgagcatctgtataacggtgacatttttacatgacttcggcgtcatggttttgctcatctgatggattgttcttccccaggcaacccccagcacatcaccattctcaatcacctgattcagatacatgccaccggcacgtgaaaggcgagtccgcatcagctttgtatcatcacgttttccggcatgttcgccatccggcacgatgatcactctctggagattgaatttatcgcgaatttgcaaagcagcgtcgatagagccaaagacattcacatccaggttgatatgaaccagtccattttcccgggctgtttgcaggtatttgacaaccgtgacgcgggacacccccatgatagctgcaacttcagtctggcttttgccttcctgatagtacagccatgttgcatgaagtacgggatcatcattgaacaggctgctgtttgtttgatctctatccacttttgtatacctgtattaaaccggggaaatgctcatcttaaccctgtttacccggagagttgatgcagattgccagtggcatgattttatacagatattttattcttttacatgaaataaaccagcataccatttgagcgatcgcccgctgttcccccatactgtaaagccggagacatgctccggctttacagtattactgagaatacacccatcaagcataatcgaaggttcaatatcgcccctttttgatcgccagcgattcgtcaccgtgcagacggttgccgtcactcactaaattatgggggacagtgaacaacaggttggctcactggcaagaacccgattataaaactaagctggcgagcagaataaaaatcagcccactgatggataagagtgtggacatcagcgtccaggataacagcgtttctttggtggtcaggccaaaaaagtctttaatcatccagaaactggcatcgttaacgtgagaacaaatacaggatccggcaccggtagccagcgtaatcaaggccaggttggtattgggatgtactgccaacaatgggatgaccagaccggcggtagagatcgccgcgacggtggctgaacccagacaaatacgcaggaatgcggccacgccccaggccatcaggatcgggttaatatccatacccgaaaccagggtggaaatatactgaccaacgccagagtcgatgagaacttgcttgaatgcaccaccaccaccgataatcagcagcagaccggcaatacccgcgatagcttttccgcaagaatccatcaggtcagggattgttttcccgcgccccaggcccatggtatagatcgcgaatagcagtgaaatcagcatggcgatcgttgaattacctaagaacagtatcacgttgtaaaataagcctgaatccgcggcacttttggcatgagtcatctggatgatggtgacaaccgccatcaggatcaccggcagcattgccgtgagaaaactgatcccaaagcctggcatttcgctttcgctgaatcggcgggtcgcgccgagagaggctatattcccctcttttttaaaggcgtccggaataatgcgctggcagaatttattcaataccgggccgcaaagaataaaggttggaatgccgacaatgataccgtatatcagtaccaatcctacatcagcgccatattccctggcgataacagtcgggccggggtgcggcggcaaaaaaccgtgtgcgaccagcaaaccagaaagcatcggcacacacataaacatcggtgatatttttgcttcacgggcaatagcgaataaaataggtaccagaagaattaaaccgacttcgaaaaaaagtgcgataccgacaataaacgccgaacagaccactgcccagtcaagtttatttttcccgaaataattcagcatggtcagcgctattcgctgcgcaccacccgcatcggccagcaagcgaccgagcataacaccgaagccaaatatcaaaccaatatggcccagcgtaccgccaagtccggattcgactgaggtgacgactttactcaaatccataccactggcgatggcgacagcaatcgagacaataattaacgaaacaaacgtattaagcttaatttttatggttaaaagcaggagtaaagcaatccctgccacaacgataattagtggcataacgtcctctcataacagggtagcgacccatcattatccgactgagcaaataacgaatgatgcagagtcggataattcaggtgtctggatgtttttatttatgctttcagtttttattcataaaatcgcgcaaagccgcgccaattttgtttacatcataaatacaaccggtccatgtcccaccactcacggcctgaagcattgcccatagccgggtatcatctggcaattcaggatcgggaagtaaatcctgatggctgggtctggcatttaatattgcagttgcctcctcctgtgaaggtaattgttcatcgctacgggttccgaggaaattgacttcgccgtgaagctcgcgacaatcaattttaatttcaattaaatccccggtgcgtaatttaccgatggggcctccggccagcgcttctggccccacatggccgatgcacgcgccagtagaaacgcccgagaaacgtgcatcggtgattaacgaaacatgcttaccgtatgacagatgcttcagggcactggtaacctggtaggtttcttccatccctgtacctgaaggtccaacgccaataatgaccagaatatcgcccgccttgatcttgtcatgtttgatatcgtaaatcgcacttttctcggacagataaaccttcgccacacctttatggtaatagataccttgctcatcaatcatcgaggggtcaatggcggtggatttgatcaccgaaccttctggcgcaatattgcccaccgggaaggtgatagttgaggttaatccgcgcgcttttgcttgctgcggagacatgatcacttcgtcagcgttgatttgttcctgatcgagcaggagttgcttgaaccgctgacgccgttcggagtgctcccaccagtcgaggttttctttcagcgtgctgccggtaaccgtcataacgtcttcatgcaacaatccgaggctgcgcagatgcaacatgacttccggcacaccacctgccataaaggcattgaccgttggatgataaaccgggccattaggcagtacgctcaccagtcggggcacgcgcttgttgatgcggatccagtcatcaacggtcgggatatggcaacctgcctggtgagcaattgccgggatgtgtaacagcaggtttgttgaaccaccgaacgcggcatggaccgtcatcgcattctctatcgctttatcggtgagaatttcccgggtggtgatgcctttttgactcaggttcagcgcagctcgcgcggaagctctggcgatctcccgccacacaggctcaccggaaggggccagggctgaatgtgggattgccagtcccaatccttcggccaccacctgagatgtcccggcagtgcccaaaaattgacagccgccgccggaagaggcacaggctttacagcccgcacggcgtgcgtcctgtagagataattcgccattggcgaagcgtgcgccaatggtttgcaccttgccgttgtcttctccatcctttgcgggcagcgtcgcgccgccggggaccagcacggttgcgatgttgtgctgcgcggcgagtgccatcatggtggccggaagccccttatcgcaactcgccacaccaataactgctttcgcgtcgggcagagagcgaataaggcggcgcattaccatcgatgcgtcatttcggtatggtagcgaatcaaacatccccgttgtaccctgagtacgcccgtcacaaggatcggagacgtacacggcatagggcagggcatggttggctttaataacctcggccgccgctttcatctggatgtccagttcgtaatgcccctggtgcaacgccagcgccacgggtttaccgtctgcgccgcgtaagccaccgagtgtactgagcagtaaaataccgtcccgatccagctcgtccggagaccaacccattccggcattcatggtcataccgaacagatccccgctcgggcggttgataagcatctctgcggttaatgggagttcgccgtccgggccatcggcgtgcgttctgacggtgtaaatatcgtggctctcgtcagcaaaaatattgcgaacagacatgagtttctcctcagactggtaaaatgccctgcgcggtaagcagcacgtggactttatcttttgcttcttcagatgcttcaagaatcggtggtaagcaatatgtctctacaggcagcccgacacactgcatgctgtatttgatcagtgagacaaacggtgtttcgagggcgtaaatagcgggcagttgtagtagttttttattcagcgtcgcagcggtcgccagatcgccttcacgccaggcgcggtagatgccgacggagagttccggagcaaagttagcgctggcggttatcgcaccgtcgccgcccagcagcatcgtattcagcaaatgatcatcgtaaccgcagaataccgaaaacgacgggcgtaccgacttaactgtgttgatcatcgtacgcaagtgaccaacgctgtcgatggtgtctttgatgccaacgatattctcgttttgcagagccagacgcgtcacggtttccggggttaagtcctgacccgtcagatccggaaagttgtacaggatcaccggtagggtgacgctacgggcgatctgctggtaatagtcgtcaagatttcgtggtgcgactttccagtagtaggggttgatggcgacgataccatcagcgccgtaggcttgcgcatgctgcgccagtttgaccgcttcgtcagtggaaggggaaccgacgccaatcaataccggcactcgcccgtcgacaatggttacagcttcttcggcgagtgccatgcgctgggctgtattcatttggctaaattcaccaccggtacccagataaaacagcccgtcgacccctttattaatcaggaagtcggcaacttcgcgcattgcctttttatcaagggttccgtcacgatgaaacgtgctggataccggtggaataatgccgctgaattttttcattacctcagtttccttttcgtaagtgctcattttcgtttctgtatcccagcccatatgatatttgctcagcgcatttccggagcaattccagatagctgtctatcttatttcctgaataaactaccggatcgccagaaagtgagattgcatagttaactctgttatacatattgaataccggcatacttaaacataccgccccataggttgattcttcgttgtctatggcccatccccgaaggcgtgttttttgtaattcttccagaaacaattttttatcggtaaatgtattgcgcgtatgtggagttaacgtgagtgcttctaaaaaataatccagttcttctcgtgtcttccaggctaataatgccttacccaacgcggtaatatgcaactcaagttttttgccaatccagcttttgctcgtcggtacagagtccggactttcgatcttgtcgagatagatagccgaaatgctctccatcgccccaagatgacaaaccagtccacttttcagcgacaactcctgcattggccgcttagtcacctcaaatatattttgacggtgtaacgcctgacaacccaattcgtagttttttattcccagtgaatagtagccgtttttgtttttaattaagaaaccacaatccaccattacattcaataaattaagcaggctgcttttggggtactggaatttatttaataactccatataacttgccataccaacccatgcaatgtgggttaatattttttcagcacggactaatgaattacaccctttgcgaaccataatggctcctccttgctcatggaataaatggtatcggcattacatagtggaaaatatgctttgttcagcatgctgaaccgtaatgatgtgattaaatgtgatcttgtacacactttgaataatgaatccagaacagccacatttagtgaatgagaataaaaagtagatggcgtgttgttgcaacatcgtagtgtgtggattgcgcctagagcttctttattcgttcgagcgcatcgccaatattttctattgggtgccattgattatttttgcttgaaatccctctcgaatgaacttacttatcactttattgaatgaggtaaaaacaactgacatccggctcgctgataacgctgtgcaatagtctcaggtaacccgctgtcactgatgatcgttttaatacatgatagtgttgctacagcatgcggctcaacggcatcaaattttgagtgatcggccatgagaataacttcacgcgagcgttgaataatccgtgttttcaccccgacctcaaacatggtggcattggtgatccccgtctccagcgacagcgcatcgcaggagataaacgcacgttctacggaaaaggcattgatcatctccagcgccagactctctcctaccgaaaaataacctgggcgaatcagtcctccgataatgtaactttccacatggggaaaacagcccagttcattggcgattttaatgtcgttgcagatgacctttacccgcgcatcggccaggcatttcgccagttcgaggcaggttgagccggagtcgagaaaaaagcagtcgccatctttgatcattgttcgggcaagggcagctatttctcttttcgccacagattgcaatgtacgtttcacgtcgaagacgtactctttgtcgtctgtactgtcgtcgaagtccaggcaaccgtgaccgcggatcatgcctggatactggttgacaatatactggaaatcacgacggacagtcgcttccgcatagccaaaaagctccatggcctgctgtgtggagaggtgacgatgttgccacaggtagtgcagcatctgtttgatacggtcaggtctctgttggctcatcagaaacaatctcctcttacagggtggcgaattgagctaaggtcgcgcgatagtcagatgaagagaacagggcgcgcccaatcaccatatgttgcgccccagctgctgccagttgctgtgcagctgccagcgtaattccaccgtcggcccagcactcggtctgaggaaaagccgtgcgtactttttggattttctcgcacatggagggaataaaccgctgtccctgcccatcgggctcactggtcatcaccatcactccgtccagctcagacgccagatatcgccaggcgtcgatcggggttgccggattaaataccagtccggctcgtgcgccggtatggcggatctcagttaacgtttccgaaggatagtccagcgtttctgcatgaacgaagatccacgcgggtctgatttcagccagcgcgttaaaccagcgctgtggccgggcaagcatgaaatgaaaggacaagggatgaggcgtctgtctggcgacggcctgcaccgttttcatcccaaacgtaatgttgttaatgaagctgctgtcctcaatatccagatgcaggctcccaaaatccagattgtccaatgccgtcagctcacgaccatagtgcagaggatttgcgctggcgagagaagggtgcaggatcataagcgcctccgttaacctgataccagcgcaaacagtgcatcgtctgtgctggcatttcccactgccgttaagcgttgtggcgaatcaataaactggctgatgcgctgaatggtcaaaatatgtgcgttggcatccgtggcgctgacgcagagaagcagccagacggggtcgcactcctcgttaccaaaggcgaccggggtgcgtagcgtggtgatactgacctgattatagtttgcgccttgctctggtcgggcgtgaggcaaggcgattcctggggctatcagataataaggcccccagttaagggtattttcgatgatcccattaacgtagcatggctgcgcggcaccataggctaccagcgggcgggtggcgatttccacggcctgacgccagtcggtggctttacgttgtgcctgtacccatttaatatcgttaatcatccgtcgttgactccatgccgattcgggttaatctggtagcgatccccgtcgatacttttgacgaaggcggcagggatcgcagaagggttattgctctttgccggggataagcgctctgcttatccccatcttatcggcgtatatgatgcactttctccataaactgactgactcgcgcctggtcaacgaaattggcaaaaacgccgtcctttttaaaggtggttgcggtcacacagccatcggcgatactgagttgttcctccacgttttccaggcagacgcccgtgttggccaacacgacggtgtcaggcaccgtttctttgacccgttttaacagcgcgctgtcggtacgcgtcccggcggtcaggccagaaacacagagcgcatcaggatggttgttaaatactgtcgatttagcaatagaacagatatcgcgattgcccagatacacggcggcctctgggacgatattgaacaaggttttcacttcgcctgcaccaatccggtgttgatgacggatggtctcaccgacgttagtgtcccagacgccaaagtcgctggcataggcaccggtaaatatctcgcggataaacttagcgccggtagccatcgccaggtcgaatgaggcgaccggatcccacagaacattcacgccaaacgggatgcggatatcgctcattaattgcccgatgattcgtgccattgccgcagtggtttccggacgcaccttcgtgagatagggaagactaaactcgttggagaacatgactgcatccaccccaccattttggagcgccatcagatcgtcccaggctttgtcgataacccagttcatccccaactgcgcatcaaaactcgggtcgccgggcaatgcacgtagatggcacatggcgatgaccgctttttccgtcccaataacctctttcagccaactcattgaaagtactccttattccgataattcacgtttacgtaagaacagcacgacgctggcgacaataccgaccgccacgacaacgccaataatcccaagcgacatcaattcagaaatcgaccaaccgaacatattgcccacggacaacgctgagatttgcgcactttcaccggcaaaactgaaaccgcctttgagcgccatttcagtgaagtaaggcgcgaactgggtggcgatcagcaggacggtaatcatcacgatgaccccgcttatcaacgtcctgaccaggtctccgcggtggataaccgtagccatacagataaagaacggtgctaccggcaggtctgcgaggggtaacactttgttgcccggtaaaatgctggccagaattaacataatgggtatcagtagcagaccgacagcaatggtggttggatgccccagcgtcacagcagtatccagaccgatatacacttcacgtcctttgaaatatttctggaagaactttcttgcaccgtcggagatgggcagcaggccctcaacaatcaggcggatcatgcgcgggaacaacaccatgattgccgcaacggtaatcatcagactggcgcaacctttaaagccttcaccagccgccaggccaaaaatcagaccgagcactacgccgataatcaccggatcgccgaccatgccgtagcgtttctggatctcctgagcatcgatattgcgtcccttcatgaaagggattttttcatagatagcatcaagtagaacgaaaagcggtactgaactggaaccgtagccttgcggtatcgaaataccttccagcccgacgatgttctgtacccgttttgccgtccagtcggccatttttaacgatagcgccgcatggcagattgcccccagcacaccataaatcaggctaccggtcataagctggaccaccgtacccgtaatggcgtagtgccagtaattgtaaatatcgacgttcatcgttttggtcagacgggtgaccagcatggcgacattgagaagaaaaataactgggataatcatggcgccaatggctgtcgcataaccaacgccggaggcagggcctgcgccaacgtcaaagacatgcagggctaggccgaaacgctcaatcatcactttgatagggggactgaggctgtcgatcgccatgacgatcaccagtcccataccgacaaaaccaatcccaaccgttacccctgccttaatcgcctgcagccaggggatgcggaagataaggccaatcacgatcatgatgatagggacgaaaacggtaccgccgagagacaggatgtaatcaaacataatgcctccttttattgagttaacagagccttgatttgttgttttaacgcgtcgtcgttgatccctgtgagcagggcggcgccattaagcgtagggatgccgtaatcactgttggttcgcatggaggttacaataaggtccataccgttacagttaagagggatctcattcagacagcattgggcggtagtggctgaaatgccctgttcagtcaggaactcttgcagcttgtgtgcaatcatggttgaagtcgacatgccggtaccgcatgccacaaggatctttttcataatggatgtgcctcttgtgtagtgcctgaatcaggctcaacggggaaatgtgctgctgacatacctgccagagcggtcaataggcggatgcaatcagtcaaatcacgcaggctggcaacctccgccggagaatgggtatagcgacaaggaatagagagactggcgcagggaataccatcctgctcaacctggatataaccggtttctgttatcacgccgggagccacttctcgctgcaccggaatgttgtgttcaagagccgtctgttccaacatccgtatcaggcgaggaggcgtgattaatccggccagcgttccccgaccatggtagttcaggcaggtgatcccaacgccctgattaatcctgacctcggaataatcgtgtaaatcaggggtgtcacacgatggagtgatatcaataccaatcgccaggtcaggttttacacggcgtaatacgggaacaatgccgcggatattaaattcttcctgtaccgaagccaccagataaacggcgatatcaagctccatagtactgatagcatccgctacaccgagcagggcagtacagcctagacgatcgtctagtgctttactgcacaccagatcgtttgccaggagttgcggcgggttatacagagtgacaggcgtaccgacctgaatgcccatccgtatagcgtcgtctttgtctttggcaccaatatcaatccacagtttgtcgacagaaggtgactgcgtgcgctcgtcgcctttggcaaagtggtaggacttaatgccgatacaccccatgactggccctttgtccccggtgagggtgacgatggaaccagccatagtgacctgcgcaggaccgcctacgcgttcaaagcgtaaaaatccagacggctctattttgcgcaccataaaaccgacttcatccatatgcgcaaaaatcatcagtcgcagcgcatcgggtttatcactaccgtagcgcgcgacgacattcccaagcctgtctcgccagacctcttttgcctgacgcctgaattcgcacagcatgacgtcagcgacagcgttttcgtgtcctgaaatcgcattgtgctgcaaaagcgagaacagggtttcctgcacagaaaatgacatagctatctccgtagaccgtaaaacaatcactcgttgagcgttttataggcgcagactggtcgaataattgtgagaacgttcacgtgaaaacgcgcaaagctgaacaaataaaaaattatgtgagccgagtggaataaaagcgctcaacgtttgtgaaagttacgggctggagagaccagtgattatggttgaaataatgaggatgaataaaacgcggtaactgttatagcaccactttgttgcaggacgctccctcttcattacgtcctgcacgtggataccccagcatctccatcagcggatcttagaatgtaatggcgcgtggcaggtcgttggttcccagcataatgtaagaaaacatcggatctcctgaatagattcagagggagtatagataatcagctcaaatcactctccgctttatgagcccaggctggcattgccgtcagataacgttttgcacgcttatgtgcttcctccgggccgactttttgccaggaatcaaggaagctggctaaacctgataccgcttcttcccagggtttgagattgccgttgctgtcgctgcattacgcacaatattgatcactggcactgtgtgcatctggtgccgacatcggcattccgcaagcctgacagaactgttcatgttgtgacatatgatgctccttatggtgacatcttgattaataaacatactgaatatgtattgtgcaggtgatacatcagatcaaagcaaaggtaaagcctcgatatttccagccagaaataccgggaacctgttgttaccgggcgatgagtgcgaacacgccccagccaaagcattcccgcgcgtaggtcacgtagcgtttcggcgcgatgtttagttcggccctgacttcggcggcgaagtcatcgtcaggattcgcttccagccagcggcgcatggtcagccattttgcggcttcataccggtcccagccttcctggtctgccagtaccatttccaccacgtcatagccgagatcgtcgaacgctccgacaagtcctggcagcgtcaggaaatcgcttgtcgagctgacgccgcaggcctgggctatttcttctgttgctggtagctgacgccagtagggttcgccgataagcatgatcccgcccggtttcaggctttgcgctagcagctcctccgccccggcaaacccaccggcaatccatgtcgcgccgacgcaggccgccacgtcacatttttcatttgcgacgtaaccggccgcatcgttatgaataaaatgtacgcgttcgctgacgccgagttcttccgcgcgacgctttgcctgcgcggtgaagagcgaactcatgtcgatgccagtccccgtaatgccatgatccctggcccaggtgcagagcatctcgcccgagccgctgccgaggtcaagaatgcgggtgcccggcttcatgcgcagcacgcgacccagcgtggcgtacttctcttcggtgaacgggttatggatgcggtgttcactttcgctgatggtaaaaatacgtgggatatccattatttaattcctgttattgggttaagccttaaaaaggacacaacaagattgttattcacgtcagtgctccggtttcatcagggtctgcgcaccggatgtggccggtcagggtcatgggctgagcggtgagtgattgcatcatccagcaggctttgtgctcctccgggatgggataaggtgccggatagcctttgtctccggcacagggttcgaacccatgtcgggggtaataggtggcgtggccgagaacaaaaaccgtctggcagcccatcaacctcaggtgctcgatgccagtgcgtatcaaccgtcctcccacgcccatcccttggtattccggtatgaccgccaggggagcgaggatgtgcatcaacggtgaatccatttctcctttgaaggttgcccgggtaaataaaatatgcccgacggctttgccttcataccgggctagcagcgataacgcggggcgcgcgctttcatcctcaagtaaagaggccactaaatcggcttctttgctgaagccaaatgcgcgggtttcgacttcccggatatcactggcatcacttttatctgtgatatgaaaagtgaagtggtgtactgtcatagaaactctccttagcgattatcgagctgagcgcgaactttattcagctcggtggtgttgattcgatagggctggccattgacggacttgataagttttttggttttgagttttttgaagacggcgagcgtgcagtcggtcagcaacagcccttcgcggctgtagcattcaacggaagtgacgcggcctgaagaatcgcggacgtgcgcaatacgtctacctttagcgagaacgtgtaaggtatgttgttcctgacgggataaattcatactgaagaacctatttaatcatcatgtgcaaaacgtgcaaacacaccgcggtgtccgcattcgatttcggcgcattgataatcagtccggcctgaaaaggtcggggaactgattatcggatgattacattctccagcatcaaagcctcgggttgagttgaaaggtatttacggagcgaatattaacacgtagttataggagggatatgtttcagtagaaaaagtgtgatgtactttggaaattgaatgccaacccatttactggaaaaggcagatgacactgacgaatgcatgttgaagtacgcctgaaatggcctcatcggcttttcccttcgggagattattctccttttgttaaatccagaacataaatatgctcacccatcttcgatgcttgaaaaattgaagccaatcctgataagtaatttttttgaaagggtattttccggattcacaccggctttgatgagtgaaaaaccgttctcttttattcagtcaatcgtggcggtaattgcttcaattgcatatccctggcgagcataagcgggactgatggtatagccgagccaaaacacatcgcattgctgacgtaaatagatatcaccaatcaaaacctgcgtcatttgttgacaatggccaattgaatatcgcgagcaagtgtaagaactcccagcaagaccctgtaaataattctgtgtaactgcccacgattaaaggtggccgctcaggcggtcaccgtattcgataataaatgggtctggaaaaagtgcagcatctggcagcgtaatgcaggtagcccagttcaactctcactaccagtatgatcccaagttcgagcgcggaatgtatctgtatgagcatcgtcgctgtttcaataacatcatcgactactgtaactcactttgctatcacggtaagttgcagcctaaaagagggatggaaaaaggacgattttccccgcaatgggatatttacatattgatggtagaggcatgaagccaaatggagggagccgtcataaccctcttgaagctgaaacaatagcagcatggctggtggcacataaggatgatatagagcgccattacggggaaccactgtacaaagttgttggtgttgtgacgccattttcggcgcaggttaatgctatcaaaatgtcattgcgtaagctggaaattaatggcaaagacgagcagggtttactgacagtggggactgtgcactccttgcagggggcggaaagggcgattgttctcttttctcctgtctactcaaaacatgaagatggcaggtttcttgatagcaacagcactatcctcaatgttgctgtctcacgcgctaaagatagttttctggtatttggcgatatggaccttatcgagatgcagcccgcattttcgccgcgagggttattggcaaaatatctcttttcttcagataataatgcgttgcaatttgagtttcagaaacgacaggatttaatttccgcacatacacaaatttcaacgctgcatggtgtggagcagcatgatgaatttttgaacaagactcttgccggagctcaaaagaaaataacgattatttccccttggttatcctggcaaaaagtggagcaaacgggatttctggcatcaatggctttggcccgttcccggggcattgatattaccgtggtgacggataaaaactgcaatatagcgcatgtcgatgatgataagcgtcaggagaaacaacatctgctgaatgatgctgttgaaaagctcaataagatgggtatcgctacgaaattggttaatcgtgttcacagcaaaattgtgattgaggatgaagaactgctgtgtgtcggatcttttaactggttcagtgctacacgggaagataagtatcaacgatacgatacgtctttggtgtaccgtggtgaaggcgtaaaaaatgaaataaaggcaatatatggtagtctggatcaacgtcagctttaaatgtgatgagccgttcatgatacaggagtagtaaagggcatattttaccaatgttaaggcgactttccgttttattgcgagtcgcctttcctgattataaatcttattgtttacctaatcattttcctttgcataatgcgcctgggattaatggcgggtgcttttaggaatgaaagaaaatgcaagcaataatataataatggcctaatttctttgaacatcattaagcatatcatcatcgtctatttgccagaatccgtcgacttataatcgccagaacggcatatcaggacggtgctgcgaacgctgtggcccaaaacgttccagtaaactgtgtagatgttcgtagatttccgagccataatcgaaaaggcgcggatgtctattaaggcatccggctaatctgtaagcaataacaacggtttatgcggtgcgcgtttttcacccttgtgccagattattatattggcaattgcctgctgttcgagcccgcaagtgaagagatattaccttgatctcatttgttttttgttgtctactctgagaacgaacaaggacatcccccatgaataaactccccgctcacctttcgcgccaaaactgcaaaattgcttctacaaatctgtcagaaataatcccccgacgggctgcagtgctgaaatgactgcttcgcagtgccgtcgtccagttctccggtgaccggtacgctgaaccgtaatatcccgtgcttaaatcgtccgggtcttcatcaggcgcgttcgtcagtcctctttcaccttgttgctggaagtcgacgaaaataatattggctaaaacattattttgataattgccataaatagcttcatacgaatgcgggaaattttctttccagtaccaggtggtatcgccgcaaaaccacggcgcgtcagtaatattattaagctgagaatggtattgttttagatccctacgaaaggcttcaaccatatgattaaagtgttgagggtgtgacgcgtagtcactggtcattaagtcaaattcgccttgcatccagcatgcgccgaggaatttgttctgcggattttttgccagtgcggctcgcgttctgctgactaaatcctggtacagcggagtatccgttccccaacgacaagcatcatggctggctccgtgccgttctgaatatgtcccttcgctgcccgcggtaaaagccgatccgccacggcaacacggaacgataagaatccctgcattatcaggaatgaagggcagtaatttccgtgcaatatgcagtgcctggccaacggtgccgtactgtgtttgatgattcgttgccagaggatggtgataaccctgcatatcctgaacatcgtgtgggcagtgagtcagtggaataatgtcgttaaagtgacatggcgggcctccgggatgcgtatgcgcaaatctcgctaattgtttaattctgggatgaggcgcatcttccctgtccggtaatggcagtccttcgccatacgccatggcattagactgaccagcaacggtaagaacatagtaataatcgggcgatattattgcgttcatataaatttcgcgtaattgaaatgacaaattgatagcagggcccctttaccggggccctgaagcgttagttttgtactgtgactttattatccttcacagtgatcaaaactgaatccgtcaccgctttgccgcctgcagtttcaccgccaataatcaatagactattattccagggcaatgatactccgtaggcccgaccttgcgataattcacccgatttatcccatttcccgttatgccaaagatgaatatcagtgctatatgattttttcaggccttcatgcgcatagttcttaccgttctggtaattttctcgtgaacctttgaatccggcccctccggcaaatataagagaatcattgcttatccccgcaaaaccgccagctacgccatctggtgatgagacgggagcaagcttattccattttaaattattaccggtgaaatcaagttcaaatacggcatccgttcgcaatcctggtttggcttcgccattaataagccaggttttatcacctttattcacaaccgccgcaccagccgttccgtaccagggcgattcgccagcgtaactccattgctgtgttgagggatcaaaagacaacagaaacttattgaagaaataatcttctgcttttttgtcaaaatagtgagcattgattttatctatagcggttgaatcttttccagcctcgttgagatcttcaaaatagccattgaagatattctggttaacaccaccagtaacataagccttgccgttgtgtacaaaagtcacatggcccgccatgcccatcggcgcgtgcgacatcaatttaacccaactattggttttggggttgtatttgtgtacgtcattaaatacctgagtcaagccctcgctgtttttgccaatgccgccaaacacatacagattgccatcaataaatgcagaggttgcttgatctcttggtccgccagggaatgcagctaacgctgtccattttttatctttggcctgtgtatccagcttgtaccatgccgtacctgcgctacctaaaccaatgtagacagtgtcgttatcaattgctccggtaccacttttaaatggcacaggagtttccggtaatacagacgcgtttgcggcaaatgaagccatcatgatagcaagcgccgttattgttttattcattgtgactgtctcctgtctactacagtttaaatgacacaccaatgcgataactgttttccgataaattatctctgccgttgtaaacaccctgacggtcaaggtagtcatattctatgtatggcgtaatatcgggcgtcatatggtattgtagaacaaatgcattttccgtcgcccatttcttatggtttgcatagcgataatcgttctgtttgctgtatagcgtcgtttgccatgcgaaggtgaaatcactattaatatggtaagtgacatatccatcccaacgatgaacgttatcacgagacatatcaccggataagtcttgttgtcggtaagctttccagtcgtaacgatagcgaatgccaaaattaagatcttttgtcgcgtcccaggacagttttacgtagggtccgtagcgtgtgccgttgctgctaaaatgcgttaacattcccgggcgcaccgtccattgatcatcaagtttaatcgcgtaattaacttcaacctgaacatcattgagtgcggcattttcctttttattatcatgaatggtattccaggtattactttccatgcttgcccaccatccattttgccatccctcactgactttgagtcgagtctcataggcgtggcttccactacgatatccaccacgtacgtccagtgtcgcagcctgagaaattaatggggacgaaaagcacagtaataatacgccagaaagtattttagcctttttcataaatttcactcatttgtaggatacagaaagcaatacaaagcccgcataaacaattagcatttatgttgtgtaatatttttttgccaggcttatagtgtctttggcaaccggtagctgtattttatatttttttgtataaggtctcctgtgaaaaatctcttttcacattatttaaataaacagagatccagattaaatacctgagtataaaatctcttctgatgtttaattgatttgaatgttcgtaagctatatcacttactcaatccattttacccagagtcataaaatagaatgtctgttgatctcattttcatattcctttcagactgaagtgcgttttcatcacccgatgagaaagaactgaagtgatgtttgccatagattgcgagatgccctgtctcattgactatcttggtgcacctttatacctgttataccagatcaaaaatcacgcaatccatacaacaaaaccagatttgcaattcgtgtcacaaaatatgtcgatctttttctaagaggaagatgccatgtgaagccagacgaacacttgcggtggtcttcaaaaactaaagatcttagtttaactatttgttttataaataatttattaagagtctaaacaaggggagctttgcaagctaactcagtgagcttggtgaaaatcagtgtttacccgccatcaggctgagcataattctcatcatgaaatatgtttcctggtttgtggcttgtaactggtcacttctgaagtcgatctggagaggcttgttgatgttggtgttttcaggatgatgtttcacttagtttgtttgccgtatcgcccggcgaatggctgtgattgaggaaggtttaagtcgtagtgaccaaagctatatttaccaacgaatgtagatgaaaaaatcatctcctgcgttcccccatatctctaggataaaaaggaatgtaacaatctcatggcgtaagctgacgaatcagcaggaataatcgctagggacctaagaattagcatgataatagccactaagaaattactgcgctccatgaaatagccattttgtggcaaatggagttgactaataatgtcatatgtgagacggctagttgaacgaatattaaattttgctgaattttttatgttgattttacttgttacagaacatatcacatgatatatagataagattagttgcattaatgatgagggttattattagattcgtatccgattgataaatatataaaggtacatagcatgcaagagcatggcgtttgtatggcaacgttattataattaacagttgctactccatttaagttcactcagaagaactggtccacttacgttagttattaagcaaacgttcgcttttataaacataatcaggataaaaatgttggattattgctaacccagcacagctagtgcgcgtctgtaattataagggaaaaacgatgaagaataaggctgataacaaaaaaaggaacttcctgacccatagtgaaatcgaatcactccttaaagcagcaaataccgggcctcatgcagcacgtaattattgtctgactttgctttgttttattcatggtttccgggcgagtgaaatttgtcgattgaggatttcggatattgatcttaaggcaaagtgtatatatatccatcgattaaaaaaaggcttttcaacaacgcacccgctattgaataaagaagttcaggctttaaaaaactggttgagtatccgtacttcgtacccgcatgctgagagcgagtgggtatttttatcacgtaaggggaatccgctttctcggcaacagttttaccatattatctcgacttccggtggtaatgccgggttgtcactggagattcatccgcacatgttacgccattcgtgtggttttgctttggcgaatatgggaatagatacgcgacttatccaggattatcttgggcatcgcaatattcgtcatactgtctggtataccgccagcaatgcagggcgtttttacggcatctgggatagagccagaggacgacagcgtcacgctgttttatagagatagttgagataccagggatggtgttaaaaactacattattcttacgatatatcaaaaatgattaaccatttattaattgatgttattgtaagtgtgattcttaattatcataataaacattaagttaaccatatccatacaaaatacaatggtttatgttcttcaaaataaataaacaaaatcattcataaatttacacatcacttaaaatctcctgtttccgcacttttttctttattttttaagcaactggaagttaatccactgcaatctattgttatattgaatcaaatcaatgaaaatagatgttgtcacatcagtgatattttatttttgtatgatatttaatgtaattgactgatagccacatcactccgtgtgtggttatctttttatctattgggctaattttgaccgattgaggtttcctataggtattcattcaaatatatctcagttaggagtactactattgtgagtaaacgtcgttatcttaccggtaaagaagttcaggccatgatgcaggcggtttgttacggggcaacgggagccagagattattgtcttattctgttggcatatcggcatgggatgcgtattagtgaactgcttgatctgcattatcaggaccttgaccttaatgaaggtagaataaatattcgccgactgaagaacggattttctaccgttcacccgttacgttttgatgagcgtgaagccgtggaacgctggacccaggaacgtgctaactggaaaggcgctgaccggactgacgctatatttatttctcgccgcgggagtcggctttctcgccagcaggcctatcgcattattcgcgatgccggtattgaagctggaaccgtaacgcagactcatcctcatatgttaaggcatgcttgcggttatgaattggcggagcgtggtgcagatactcgtttaattcaggattatctcgggcatcgaaatattcgccatactgtgcgttataccgccagtaatgctgctcgttttgccggattatgggaaagaaataatctcataaacgaaaaattaaaaagagaagaggtttgatttaacttattgataataaagttaaaaaaacaaataaatacaagacaattggggccaaactgtccatatcataaataagttacgtattttttctcaagcataaaaatattaaaaaacgacaaaaagcatctaactgtttgatatgtaaattatttctattgtaaattaatttcacatcacctccgctatatgtaaagctaacgtttctgtggctcgacgcatcttcctcattcttctctccaaaaaccacctcatgcaatataaacatctataaataaagataacaatagaatattaagccaacaaataaactgaaaaagtttgtccgcgatgctttcctctatgagtcaaaatggccccaaatgtttcatcttttgggggaaaactgtgcagtgttggcagtcaaactcgtttacaaaacaaagtgtacagaacgactgcccatgtcgatttagaaatagttttttgaaaggaaagcagcatgaaaattaaaactctggcaatcgttgttctgtcggctctgtccctcagttctacagcggctctggccgctgccacgacggttaatggtgggaccgttcactttaaaggggaagttgttaacgccgcttgcgcagttgatgcaggctctgttgatcaaaccgttcagttaggacaggttcgtaccgcatcgctggcacaggaaggagcaaccagttctgctgtcggttttaacattcagctgaatgattgcgataccaatgttgcatctaaagccgctgttgcctttttaggtacggcgattgatgcgggtcataccaacgttctggctctgcagagttcagctgcgggtagcgcaacaaacgttggtgtgcagatcctggacagaacgggtgctgcgctgacgctggatggtgcgacatttagttcagaaacaaccctgaataacggaaccaataccattccgttccaggcgcgttattttgcaaccggggccgcaaccccgggtgctgctaatgcggatgcgaccttcaaggttcagtatcaataacctacccaggttcagggacgtcattacgggcagggatgcccacccttgtgcgataaaaataacgatgaaaaggaagagattatttctattagcgtcgttgctgccaatgtttgctctggccggaaataaatggaataccacgttgcccggcggaaatatgcaatttcagggcgtcattattgcggaaacttgccggattgaagccggtgataaacaaatgacggtcaatatggggcaaatcagcagtaaccggtttcatgcggttggggaagatagcgcaccggtgccttttgttattcatttacgggaatgtagcacggtggtgagtgaacgtgtaggtgtggcgtttcacggtgtcgcggatggtaaaaatccggatgtgctttccgtgggagaggggccagggatagccaccaatattggcgtagcgttgtttgatgatgaaggaaacctcgtaccgattaatcgtcctccagcaaactggaaacggctttattcaggctctacttcgctacatttcatcgccaaatatcgtgctaccgggcgtcgggttactggcggcatcgccaatgcccaggcctggttctctttaacctatcagtaattgttcagcagataatgtgataacaggaacaggacagtgagtaataaaaacgtcaatgtaaggaaatcgcaggaaataacattctgcttgctggcaggtatcctgatgttcatggcaatgatggttgccggacgcgctgaagcgggagtggccttaggtgcgactcgcgtaatttatccggcagggcaaaaacaagagcaacttgccgtgacaaataatgatgaaaatagtacctatttaattcaatcatgggtggaaaatgccgatggtgtaaaggatggtcgttttatcgtgacgcctcctctgtttgcgatgaagggaaaaaaagagaataccttacgtattcttgatgcaacaaataaccaattgccacaggaccgggaaagtttattctggatgaacgttaaagcgattccgtcaatggataaatcaaaattgactgagaatacgctacagctcgcaattatcagccgcattaaactgtactatcgcccggctaaattagcgttgccacccgatcaggccgcagaaaaattaagatttcgtcgtagcgcgaattctctgacgctgattaacccgacaccctattacctgacggtaacagagttgaatgccggaacccgggttcttgaaaatgcattggtgcctccaatgggcgaaagcacggttaaattgccttctgatgcaggaagcaatattacttaccgaacaataaatgattatggcgcacttacccccaaaatgacgggcgtaatggaataacgcagggggaatttttcgcctgaataaaaagaattgactgccgggtgattttaagccggaggaataatgtcatatctgaatttaagactttaccagcgaaacacacaatgcttgcatattcgtaagcatcgtttggctggtttttttgtccgactcgttgtcgcctgtgcttttgccgcacaggcacctttgtcatctgccgacctctattttaatccgcgctttttagcggatgatccccaggctgtggccgatttatcgcgttttgaaaatgggcaagaattaccgccagggacgtatcgcgtcgatatctatttgaataatggttatatggcaacgcgtgatgtcacatttaatacgggcgacagtgaacaagggattgttccctgcctgacacgcgcgcaactcgccagtatggggctgaatacggcttctgtcgccggtatgaatctgctggcggatgatgcctgtgtgccattaaccacaatggtccaggacgctactgcgcatctggatgttggtcagcagcgactgaacctgacgatccctcaggcatttatgagtaatcgcgcgcgtggttatattcctcctgagttatgggatcccggtattaatgccggattgctcaattataatttcagcggaaatagtgtacagaatcggattgggggtaacagccattatgcatatttaaacctacagagtgggttaaatattggtgcgtggcgtttacgcgacaataccacctggagttataacagtagcgacagatcatcaggtagcaaaaataaatggcagcatatcaatacctggcttgagcgagacataataccgttacgttcccggctgacgctgggtgatggttatactcagggcgatattttcgatggtattaactttcgcggcgcacaattggcctcagatgacaatatgttacccgatagtcaaagaggatttgccccggtgatccacggtattgctcgtggtactgcacaggtcactattaaacaaaatgggtatgacatttataatagtacggtgccaccggggccttttaccatcaacgatatctatgccgcaggtaatagtggtgacttgcaggtaacgatcaaagaggctgacggcagcacgcagatttttaccgtaccctattcgtcagtcccgcttttgcaacgtgaagggcatactcgttattccattacggcaggagaataccgtagtggaaatgcgcagcaggaaaaaacccgctttttccagagtacattactccacggccttccggctggctggacaatatatggtggaacgcaactggcggatcgttatcgtgcttttaatttcggtatcgggaaaaacatgggggcactgggcgctctgtctgtggatatgacgcaggctaattccacacttcccgatgacagtcagcatgacggacaatcggtgcgttttctctataacaaatcgctcaatgaatcaggcacgaatattcagttagtgggttaccgttattcgaccagcggatattttaatttcgctgatacaacatacagtcgaatgaatggctacaacatcgaaacacaggacggagttattcaggttaagccgaaattcaccgactattacaacctcgcttataacaaacgcgggaaattacaactcaccgttactcagcaactcgggcgcacatcaacactgtatttgagtggtagccatcaaacttattggggaacgagtaatgtcgatgagcaattccaggctggattaaatactgcgttcgaagatatcaactggacgctcagctatagcctgacgaaaaacgcctggcaaaaaggacgggatcagatgttagcgcttaacgtcaatattcctttcagccactggctgcgttctgacagtaaatctcagtggcgacatgccagtgccagctacagcatgtcacacgatctcaacggtcggatgaccaatctggctggtgtatacggtacgttgctggaagacaacaacctcagctatagcgtgcaaaccggctatgccgggggaggcgatggaaatagcggaagtacaggctacgccacgctgaattatcgcggtggttacggcaatgccaatatcggttacagccatagcgatgatattaagcagctctattacggagtcagcggtggggtactggctcatgccaatggcgtaacgctggggcagccgttaaacgatacggtggtgcttgttaaagcgcctggcgcaaaagatgcaaaagtcgaaaaccagacgggggtgcgtaccgactggcgtggttatgccgtgctgccttatgccactgaatatcgggaaaatagagtggcgctggataccaataccctggctgataacgtcgatttagataacgcggttgctaacgttgttcccactcgtggggcgatcgtgcgagcagagtttaaagcgcgcgttgggataaaactgctcatgacgctgacccacaataataagccgctgccgtttggggcgatggtgacatcagagagtagccagagtagcggcattgttgcggataatggtcaggtttacctcagcggaatgcctttagcgggaaaagttcaggtgaaatggggagaagaggaaaatgctcactgtgtcgccaattatcaactgccaccagagagtcagcagcagttattaacccagctatcagctgaatgtcgttaagggggcgtgatgagaaacaaacctttttatcttctgtgcgcttttttgtggctggcggtgagtcacgctttggctgcggatagcacgattactatccgcggctatgtcagggataacggctgtagtgtggccgctgaatcaaccaattttactgttgatctgatggaaaacgcggcgaagcaatttaacaacattggcgcgacgactcctgttgttccatttcgtattttgctgtcaccctgtggtaatgccgtttctgccgtaaaggttgggtttactggcgttgcagatagccacaatgccaacctgcttgcacttgaaaatacggtgtcagcggcttcgggactgggaatacagcttctgaatgagcagcaaaatcaaataccccttaatgctccatcgtccgcgctttcgtggacgaccctgacgccgggtaaaccaaatacgctgaatttttacgcccggctaatggcgacacaggtgcctgtcactgcggggcatatcaatgccacggctaccttcactcttgaatatcagtaactggagatgctcatgaaatggtgcaaacgtgggtatgtattggcggcaatattggcgctcgcaagtgcgacgatacaggcagccgatgtcaccatcacggtgaacggtaaggtcgtcgccaaaccgtgtacggtttccaccaccaatgccacggttgatctcggcgatctttattctttcagtcttatgtctgccggggcggcatcggcctggcatgatgttgcgcttgagttgactaattgtccggtgggaacgtcgagggtcactgccagcttcagcggggcagccgacagtaccggatattataaaaaccaggggaccgcgcaaaacatccagttagagctacaggatgacagtggcaacacattgaatactggcgcaaccaaaacagttcaggtggatgattcctcacaatcagcgcacttcccgttacaggtcagagcattgacagtaaatggcggagccactcagggaaccattcaggcagtgattagcatcacctatacctacagctgaacccgaagagatgattgtaatgaaacgagttattaccctgtttgctgtactgctgatgggctggtcggtaaatgcctggtcattcgcctgtaaaaccgccaatggtaccgctatccctattggcggtggcagcgccaatgtttatgtaaaccttgcgcccgtcgtgaatgtggggcaaaacctggtcgtggatctttcgacgcaaatcttttgccataacgattatccggaaaccattacagactatgtcacactgcaacgaggctcggcttatggcggcgtgttatctaatttttccgggaccgtaaaatatagtggcagtagctatccatttcctaccaccagcgaaacgccgcgcgttgtttataattcgagaacggataagccgtggccggtggcgctttatttgacgcctgtgagcagtgcgggcggggtggcgattaaagctggctcattaattgccgtgcttattttgcgacagaccaacaactataacagcgatgatttccagtttgtgtggaatatttacgccaataatgatgtggtggtgcctactggcggctgcgatgtttctgctcgtgatgtcaccgttactctgccggactaccctggttcagtgccaattcctcttaccgtttattgtgcgaaaagccaaaacctggggtattacctctccggcacaaccgcagatgcgggcaactcgattttcaccaataccgcgtcgttttcacctgcacagggcgtcggcgtacagttgacgcgcaacggtacgattattccagcgaataacacggtatcgttaggagcagtagggacttcggcggtgagtctgggattaacggcaaattatgcacgtaccggagggcaggtgactgcagggaatgtgcaatcgattattggcgtgacttttgtttatcaataaagaaatcacaggacattgctaatgctggtacgcaatattacctgaagctaaaaacctgcacgttagccctttgtaggccagataagacgcgtcagcgtcgcatctggcataaacaaagcgcactttgctggtctgttcccctcaccctaaccctctccccggaggggcgaggggactgtccgggcacatttttagactttgtcatcagtctgagcctgccattggcaggctctggtgtccttttacgctaccatgctaataatcagcacaataatcagcccaaccacggagttgaccagctccagcagaccccaggttttcaacgtgtcttttactgacaggtcaaagtaacctttgaacaaccagaaagatgcatcgttaatgtgggtgagggtgttggaacccgcagccgtcgccagtaccagcagcgccggattcacgccaaccagctgaccagttgctggatctaggattgcagcactgataatcccggcggcggtcatcgccgaaacgacaccctgacccgtcgccagacgaattagcacagtgatcagccatgccatgatgtagggcgagatattgccgtgggacatcaacatgccgatggtgtcgccaatgccggtgtcgatgatggtctgcttcagcacgccacccgcaccgatgatcagaatcaccattgcaatactcttcaccgcgctttcaaaagcgttcatcacccactgcatgtcatgaccacgtgcggtgccaaagagtacgaatgcaaccaccatcgcaataaacattgcaatcggcgaggaaccgataaagttaaccacttcccaggcaggggtatcttttaccagccagatattggcgatggtggtagagatcataatgatcgccgggatcagcggcaccagaatcgaaacgccgaaagagggcagattattcatatctaccggttgatctgctttcaggaatgatggcgttgggcgctcaagattgccgaggaacttcggcaggatcagacctgcgcagattacacttgggatcgtcaccagtacgccatagatataaaccatccccatatccgcgccataagcattcaccagcgccaccggacccggctgcggtgggaacagtgaatgtgcggtagtggcagctgctactgccgggatcgccagtttcaggaacggaattttagcttcggcggcaataacaataaccagcggcgctaacatgataaaggccacttcatagaacatcgccagaccaaaaatcaggccgatgataatcaccgacagctgtacatagcgcagaccgagacgcgccagcagcgtatgcgctatctggtgagccgcgccggagtcgaccatcaatttaccgatgaccgcaccgaacaccacgatgatagccagttcccccagcgtgttgccgaagcccgctttcatagtgtgcagcagcgacatcaaatccatgcccgccagcatcccgacggacagcgccgccaccaacaaagccaccattgaattgattttgaacttcaaattcagtaccagcatcagaccaatgccgaataccacccagagaatgttaagcacatgcataacgttttaccttacctggttgaaccgttgttattttgggcgatatgttatgtaaattggtcaaccattgttgcgatgaatgtcacatcctctgatcaataaccatcgattaccctttgctgcaatttgcagcaacaaccatgagagtgaaattcttgtgatgtggttaaccaatttcagaattcgggttgacatgtcttaccaaaaggtagaacttatacgccatctcatccgatgcaacgccacggctgcggtctggttgttcatccggatacctaaacaactccagggttccgcgtctctttgctgtggaacccactatgtgaaagaggaaaaatcatggaacagacctggcgctggtacggcccaaacgatccggtttctttagctgatgtccgtcaggcgggcgcaactggcgtggttaccgcgctgcaccatatcccgaacggcgaagtatggtccgttgaagagatcctcaaacgcaaggcgatcattgaagacgcaggcctggtgtggtctgtcgtagaaagcgtgccaattcacgaagatatcaaaacccacactggcaactatgagcagtggatcgctaactatcagcagactctgcgcaacctggcgcagtgtggcattcgcaccgtgtgctacaacttcatgccggtgctcgactggacccgtactgacctcgaatacgtgctgccagacggctccaaagctctgcgcttcgaccagatcgaattcgctgcattcgaaatgcatatcctgaaacgcccaggcgcggaagcggattacaccgaagaagaaattgctcaggcagctgaacgcttcgccactatgagcgatgaagacaaagcgcgtctgacccgtaacatcattgctggtcttccgggcgcggaagaaggctacaccctcgaccagttccgtaaacacctggagctgtacaaagatatcgacaaagcgaagctgcgcgaaaactttgccgtcttcctgaaagcgattattccagttgctgaagaagtcggcgtgcgtatggctgttcacccggacgatccgccgcgcccgatcctcggcctgccgcgcattgtttccaccattgaagatatgcagtggatggttgataccgtaaacagcatggcaaacggttttaccatgtgcaccggttcctacggcgtgcgtgctgacaacgatctggttgatatgatcaagcagttcggtccgcgtatttacttcacccatctgcgctccaccatgcgtgaagataacccgaaaaccttccacgaagcggcgcacctgaacggtgacgttgatatgtacgaagtggtgaaagcgattgttgaagaagaacaccgtcgtaaagcggaaggcaaagaagacctgatcccgatgcgtccggaccacggtcatcagatgctggacgacctgaagaagaaaaccaacccaggttactccgcaattggtcgtctgaaaggcctggccgaagttcgcggtgtcgaactggcgatccagcgcgctttctttagccgttaatatccaccggcatggctgcgcgccgtgccggttccttcttccttgccgtcactctttgaagacggattctggagtttacgatgactactattgttgacagcaatctgccggttgcccgcccgtcatgggatcattctcgtctggaatcacgcattgtgcatctcggttgcggggcgtttcaccgcgcgcaccaggcgctgtatacccatcatctgctggaaagcaccgacagcgactggggcatctgcgaagttaacctgatgccaggcaacgaccgcgtgctgatcgaaaacctgaaaaaacagcaactgctgtacaccgtagcggaaaaaggcgcagagagcaccgagctgaaaattatcggttcgatgaaagaagcgctgcatccggaaatcgatggctgcgaaggtattctcaacgcgatggcgcgtccgcaaacggcgattgtctctctaacggtcacggaaaaaggctactgcgctgatgcggcaagcggtcaactggatctcaataacccgctgatcaagcacgatctggaaaacccgactgcgccgaagtccgcgattggttacatcgtcgaagcgttgcgtctgcgtcgtgaaaaagggttgaaagcgtttacggtgatgtcctgcgataacgtgcgtgaaaacggtcatgtggcgaaggtcgcggtactggggctggctcaggcgcgtgacccgcagctggcggcatggattgaagaaaatgtcaccttcccgtgcaccatggttgaccgcatcgttccggcggcgacgccagaaaccttacaggaaattgctgaccagctgggtgtttacgacccgtgcgccattgcctgcgaaccgttccgtcagtgggtgattgaagataacttcgttaatggtcgcccggattgggataaagtgggcgcacagttcgttgcagacgttgtgccgttcgaaatgatgaagctgcgtatgctgaacggcagccactcttttctggcgtacctcggttacctcggcggctatgaaaccattgccgacaccgtgactaacccggcttatcgcaaagcggcctttgccctgatgatgcaggaacaagcgccaacgctgtcgatgccggaaggtacagacctgaacgcctatgcgacgctgctgatcgagcgtttcagcaacccgtctctgcgtcaccgtacctggcagattgcgatggacggcagccagaagttaccgcagcgtctgctggacccggtgcgtctgcacctgcaaaacggcggcagctggcgtcacctggcgctgggcgtggctggctggatgcgttacacccagggcgtggatgagcagggtaatgccattgacgtggtcgacccgatgctggcggagttccagaagatcaacgcgcagtatcagggcgcagaccgcgtgaaagcgctgctgggcctgagcggtatttttgccgatgatctgccgcagaatgccgactttgttggcgcagtgacggcggcatatcagcagctgtgcgaacgcggtgcgcgcgagtgtgtggctgcgctgtaactaactgattaccctacagacttactggtcaatcaaactgatatttggttgaccagttttcgtttttttgcccacctgtacgtgccaacttccagtgctaatggtatagtttgagattaacgggggccgtaaaattgcccgttgtaggccggataaggcgttcacgccgcatccggcaaaaatttgattaaccgcacctaacggacacaacaccatgaaatctgccacctctgcgcaaagaccttaccaggaagtcggggcgatgatccgcgatctgatcataaagacgccgtacaatcctggcgaacggctgccgccggagcgtgaaattgcagaaatgcttgatgtcacgcggacggtggtacgtgaagcgctgatcatgctggagatcaaagggctggtggaagtacgccggggtgccggtatctatgttcttgataactcaggcagccagaacacagacagtccggatgccaacgtctgcaacgatgccggtccttttgagctgttacaggcgcggcagttattggagagcaacatcgccgagtttgccgctttgcaggctacccgcgaagatatcgtcaaaatgcgtcaggcattgcaactggaagagcgtgaactggcttccagtgcgccgggcagcagcgaaagcggtgacatgcagttccatctcgctattgccgaagcaacgcataacagcatgctggtggagctgttccgtcagtcctggcagtggcgggaaaacaatccaatgtggatccagttgcacagccatctggatgacagcctgtatcgcaaagagtggttgggcgatcacaaacagatcctcgccgcgttaatcaaaaaagatgcccgagcggcgaagctggcaatgtggcagcatctggaaaacgttaagcaacgtctgctggaattctcgaacgttgacgatatttattttgatggctatctgtttgattcatggccgctggataaagtcgacgcctgacttattataataagcgcaagggtaaacgttccttgcgctttcttaaattaagaagtcgcaatgagtattactttgtaaattgcagggtattgtttagctatctgtataacctgaatgttagtactcattcttcctggtagttatttaccaatataattccattcaccattttttaattcaaacagttctggaagagatgacggttgcagagtcatacgtttgagtggtgcattttcatcacccgggataactttatatcccatttttgcatggatctccgcggtaccgggataggcttctataccaattattgggtcattacccaactcaatattagcattaagtaatgcggcaagggcgaatccggaagaatttgctacccctgttaccgtcattatctgatcaatatagatatcaatccttggctgctcattggtccatctttttgcctgagaagctggaagggttgaaatatatcctatcgtggttccggcataaccaggaacattgcaaccagggcctaatgttatttcatgaactgtatagtcctcaacaggatcgaaagggctcttcataaataaatttagccgtaaaccttctgctaactctgtggtagcatgcgcctttttacatatgccaccatatatttcgtctaaagctgaggtgattttcaagttccgatagagcatacgtcctgttgttgtaataccatcggattctctgcatgctcctgtcacataattaaatggccaaggctctttactaatatcaagttttctaatttcgacaacgctttttccatcgtaattatggttattgccacgagtaagaggcggaagatagatgttttccgaatccatgcgtgcatattttaatttacgtgtaaactcactgtcgactattgggtgatgaaggaagtgagcatctgtaataatttgactctgaagggcattgcttaatggcatagacataatagttaccttttatgagtatttcactgatgtttagaaaaatagataaatttttctgtagtaaaaagagaagtaaacaaatgacatgcatgtttctgttgtagtgatatcaactctacacggtgatattaaagggtaggaaacactctaaagtatcaaaaaacgctcatttaaaattatttgcatgcaatttaaaagcatatcttattactaattggaatttgatgttgctatattgaggtctatattaataatgcctgtgaatggtatttttgatgtatttgatatgttatcaatttatattatttacaaactaattgtttcaaataatacatggctgattatgcggaaataaataatttcccaccggaattaagtagcagcggtgacaagtattttcatctacgtaactattcggaatattcagaatatactagcggtttttttttgagtttgatgatttttatcaaatcatgacttttttcctgaaaagtcagtagatattcataggcaagtaaggttttatactttgctgacaggattcaggcctgtctcagactgacatggatgtaatgaacaaaagggaatggctatggaaaatgagcatcaatacagtggtgcccggtgttcagggcaagccgcatatgttgctaaacgtcaggagtgcgcaaaatgatgcgacaatcacttcaggctgttttacctgaaatttcaggcaataaaacgtcatcgctgcgtaaatcggtatgcagcgatctcctcactctttttaattctcctcattcggcattaccgtcattacttgtttcaggcatgcccgagtggcaagtgcataacccgagcgacaaacatctccagagctggtattgccgtcagctgcgttctgcactgttatttcatgagccacggattgcggcgttgcaggttaatttgaaagaagcgtactgccacactctggcgatcagccttgagataatgctgtaccacgacgatgaaccgctaacgtttgatctggtctgggataatggcggttggcgcagtgcgacgctggagaatgtcagctaagcacaatctccagctcgcgcagttcacgccagaagcgttcggcaacgggattcatgcgggtattcatccggtatgcataggcctgaatcgggatcaccagttcgtcccgattcagtacaacgagcttcccgctgcgaatttcttgttggatggcgtactccggcagccaggcaatcccacagccgtcgagggcaacctgctttaaaagctcgctcatcgaagagacaaaaaaggtgctgaaacttaactcactgtggcgcgtcagggtgcgattaatcaatcgccccatgtaggagttgcggctgtaattcagtaacggaaagtgtggctgcgcgaggttaaaaagtgcttctccgtgttcgtcactggcgcagacagggaacaattgagattcaaataagcgaatgtggtcaaacggcgcttccagcaaatcttcgtcgtgaaaggaaaaaatacagtcactttgcccttcacgcagtttatcgaccgcttcatcgacatcaatagcttcaattgcccaggtaaagagcggcggcatctggctgataatggacggtaacagcccgagggaaagagagtgtgcagcggctatcttgatttttcgttgcgcgtaatcgctgccgccacgcagctctgccagattgctctctaactgttgcaacagatggcggatctgcgaatggaagattttcccttgttctgagagttgcagcggcgttacctggcggttaaacaattcaacaccaatcgcctgttccagcgcacggatgcggcggctgaatgccggttgcgagacgttgcgactgactgccgcctgggaaaaattgcggcatttttccagggtcagaaaatcataaagccatttggtttcaatattatgcaaaatcgcaccacagtcatccattacgttttactctgtcagccgcccttgcgggcattctacgtccattcgggcggctgacaaccgtttaagccgtttcaaacgttcctttcacgcaggctttgccgtctttgaccatcagtttgccgcgagcgtatacctgctcaatgcgcagttctggcgtcatgaccagcaagtcagcatcattgcctggcagaatttcgcctttcccggtcaggttaaggaaaccggctacgctactggtgagcgggcgcagggcatcgctgatactgaaatcatagtctttgaccagcacctgcacggtttccagcaacgtttcaaaaccggcaacaccgatatgggttaaattcccttcgtcatcgaagaacggctggctaccgttgccgtcggagctgagggtgacgcgtgccagcggaatacccgcctgaacggcgcgggcaataccttcggcaggggcgaccggttcgtcaatgctgctggtgatatcgatggtgccgcctttgcgcgcgaactccagcgcctgctcaaacaacggtacgttgcggttaacgtgggtcggcagcagcttgctgatcggcacatcgcagttttccagcaggtcataaataggctgtaacgcctttttactgtcgcccatgtggaacacggtgacgccaggtttaccgccgagcaaaccgccaacgcgggattctgccgccatattggccaggtgataaacgtccggtgcggcagaacggtgatcagagatggcgcatttcacgccaatcacacgatcgataatcgccacgtctttttccacggaacccgtaatggtgcgggaagggacatgataagcgccggtcagcatccaggcgctgatgccttcttcattgagcgcacgggtcttggcgagcagggattccgggtggcgagagatagagtcggtgcccagcagaccaaccactgacgtgacgcccgcttccgtcaggcgacttagcgccacttccggcgtgcgcgtcgtgggacctgcttcgccgccaccgccaatcaaatggacgtgttgatcaataaaacctgggcagaggatctgcccactgagatcgacaaccgtgcagttcggtacaatgtcagaagggatattgctggcaacggcgataattttgccgttagcgacgaggacatcgcaaattccccgatcttccggcgcatacaaatgcgctccctgcagcagggtaaaaccggctgcggtataatcaatcatggtaactccttgttaaacaataagctgcataacccagatcgacagcaatgcgttaatcacgcagaccgtaatgatatgcgggtaatatttggcattcacttcggctgtccccaggcagcgaccgacattttgcaccgggttgcccattaaatacatcgcgggcagtaaaacggtgacatcgtgaccggttaatgcgccagcggttgccagactggcggcaacaccgactgcgccacccatactcattaatgcggctaaaaggacggttgccgcttcaccgggtaatccccacagcgccattacgggttcacagatatgccccacccagtcgagcaggccggtaattttcagcgcctgaatgatgacaaacgccatcaccacgtttggcagcaggttggtcgtggcgatagtaaagccacggcgcgcgccatcgataaacatatccatgacgtttttgcggacctgagttgtcatgcttgcgctccttgcgttgggttgcgacgttcttcgaagttaagccagacgcgcaaaatgttggctccgacaaatttaaacaccaggatgacggctaaaggtacgattacggacgtgcccagaaaggcaaacaccgcgacgccggaagagaagtagttggtgatgatggcgctaccgctggtttgatatgcggcgaaaatcactttatcgcgttcggtaatttcaccttcctgcgccagctctttggtcataccggcggcggcatcggtgttttgcaggttagcgatcagcgccagcgagcagatccctggaatgcccaacaacggttttagcacaggtgtcattaactgctgcgcggcgcgtaatccaccaagaccatcggtaattgaaataatccccagagagagaatgactgacggtgccagctccagcgcaaagagaaagccatctttagcccccgcgccacccgcgccgcgaaatgaggtggtggctccgttcgcaccaggcagttgcccaaacgatccgttcagaacggaaaaatcaaaaacgcgccaccagctgtctgttccggaaaaaacaccggaaaaaaagattatggtgagaaaaaaggccagataccctttaatgcccactttttctgtcgccagctccccggctacagcatccccttgttgtgtcataacaatccccattgtttttttgtgtttgtgtgttgcttgagccaggaaaattcctggaactgaaaaaccttatcagccatgtgggtatggggaaaatgcaagtatgtttctggctatgcgttttttgcatagcggaaaaattacgctgtgtggaaaaggctctgcgcaggattgagttgcagaaaattcataaaccaagtgacaatgacatcagtaaataaaaacagaaaatccagggacgaaaacgagatggcaaagtacaacgaaaaagagctggcggatacgagcaagtttttaagttttgtcctccgacacaaaccggaggcgattggtatcgtactggaccgtgaaggatgggcggatatcgataagctcatactttgtgcccaaaaagcgggcaagcggttaacccgtgcattgctggatactgtggttgccaccagcgataaaaagcgttttagttattccagtgatggtaggtgcatccgcgcggttcaggggcattcgacttcgcaggtcgctatttcctttgccgaaaaaacaccgccacagtttctctaccacggtacggcaagccgtttccttgacgagataaaaaaacaggggctgattgcaggtgagcgtcactacgtacatctctctgctgatgaagcaacggcacgcaaagtgggagcaagacacggatcgccggttattttaaccgtcaaagcacaggaaatggcgaaacgaggcctccctttctggcaagcggaaaacggggtctggctgacatcaacggttgcggttgagtttcttgagtggtaagggaaacttccctcatgaagtgaccacttgtagcttaaataattgcactgtgctgataagcgcagcaataaacaacgccgccgcgccgcagagagtggcgctggcaagcgccgatgttccattgctgagcatactggtcagcgccgggccgaggatttgcccaatgccgtaaatgagcgtcacaaagcctaaaagattgagatttcccggtacgctcagttggcgggcgatagtcatcaccagagatgtcgtgcccataaaggtaccgccaaaaccaagactgctgatgataagcaagagaggcgagtcgctggcgagagtaagcagcacacagatagcctgcaccagcaaattcgccgtcaggcagggcaaagccccccaacgttttgctgcccatagccagccaaagcaaccaggcacaattgataagccgactaacgtccagagatgggcggttaacaatggtgagcctgcatctttcgccatgagcggcaggtaagtcgcgacgatgatataaccaaatcccgccaggccgtacagaatagccagtaaccaccagctcattatctgttgctccgtttttgccaatggcattggtgtgatggcgtgttttttcgagggcattaaaagcgtaagtgcaatcagcatcatgccagaaagcgccccggcgccttgccataacgtttgcgaggagaggtcaaaatgcaggcctgccagaacatattcattgcccagtgcgatgccaatgccaacgccagaaaacaaagctgccagcacaaaaggatggcgcgtgtgctgcataatcagcgtcgaaccaaaaatcagcataccggcgctggcgacacccgccaggacgcgaatcaataacaccagaataaatggcggcaaccatgccattgcgaggatcaacaacccgctcgccagggcagaagccaacagaaatgggcgcaggcgcgatggctggtgaaatgcgccaaaagaaaatagcagactgccagccagataccccgcatagttgccgctggcaatccacgagagctggctaaatgaaaacgatccttccgccatcatgacgggcaacataggcgtataaaggaagcggcctaaacccatacctaaggtcagaaccagcatcccgaaaagcgcggtgctgaaagaaaagcgttctacgggatgcgtggacgaaggcatgtttaaccttgtttgtcatttttgttgttaacaagttaataacaaaaaggtgaagcatgccagcctgttaatgcgatgattgaggggtaaagcgataaaaacgatttggttcgctaacgatataaatattaccagaggcatccatcgcaaccccttcggcctgtttgatgttatgcgacaaacctcgactgcctttggttagtgacatttcaccgataacctcgccaaccagggttacttcctggagtgcgcgagattcatgagacagcaccagaagcgtatttttttgctggttaaattctgcgccggacacatcatctaaagtaaattgccgttgtagtgcctcgtctttgctgatgtgtaattcattgctacttaacagcccgttaactttgtagacctcaatcggatttttctctttaaaaaaccagaaagtgtgatcctggcgagaataagccaacccttcaaaaccgcaattggttggggagtcttgcagcgggatttttatttttttgaggatttttacttccgagtttggggtcagtgaaatcacataaatggcgtaatcgcgctcatcgctaatgacaaactgattatcgccaatgtattcgatcgtctcgagatccttaacaaaatccagaggaattgtgcggataaaatcaccattggtggtcatttcaacaatggcggcaggtttgttgatagtgctaaaaagagtattgctttgtgccgaccaggtcagcgaagagatattattcgttatgcctgcaatttctttgccgtcaatggtggcgtggtaattctgaaatgatgctgcatgattgcttttacgggcgcaagattgcacgaagaaagtacacactgccacaatggcaaaaagaatcacaataatggagatgcgtttacttaacgaaatactttttgtcacggtaatccctttaaggcaaatcaataagatatcgagaagtatacgtagcgaccttaatgaatccttaacgcggagaaaccccgtaatgtgcaatgcagcgccagacaccatcctgctggcaataaattgactcagtcagcccagggatcacccattgtatttcctcgccggggggacaggtcagccaaatgcataacccgcagccgccgcgtaaatcacggggaatatcgctgacgcgaaaagtcatgcccgctgcctgcaacgctttgcgggtttgtatgacgccgaccgtggagtgaaataaaaataaaaactctttcatcggcgtgtcctcactcgttgaccaattaccgccgcgccaattgcgccagcaaattgcgcatcaggatgggtatttaccggcattcgcaggtgagattccagcatccgggcaaacttctggcaatgactaacgccaccagtaaacagaatcggcgcttcacaggagagacgagcaatgaaattggcactcctccgcgccatcgcgttaatcactcctgcgagaatcgcttctggcgcgacgcccgctgagcgcaggctgatcgcttctgattcagcaaacactgtgcacatactcgtgatggcgtgcggcgtgacattttcggtaatgctgtcgagttgctcgacgctggtgccaagcgtgcgcgagatcacctccaggaaacgcccggtgcccgccgcgcatttgtcattcatcaggaaatcgcacaggttaccgtcatcatcaagctgaatcactttgctgtcctgaccaccgatgtcgattaccgcgcgcgttgctggcgcaagaaaccgtgcgcccagcccgtgacaggagatttccgttacctgtttatcggcaaaatccaccagttgccgcccgtagccggtgagcgtcagaaacggcgttgtctctaacccttcgcgcagagtttcccaggcttcagtaattgctgttgccgggcgaaagggggttggaacgaggaaacggcgcgtaatcacgccgtctgccagtaagatccctttggtggcggttgagccggaatcaatgccaatcgaatatgccactgccactccttacagcatctcaataaaggccgcgacacgggtactgagctgcccgacatccgaggtggagtagtctgtttcaatagcgatataaggaatgttgtgctgctggcgcacatgacgtttaatcgccagcgattccaccgcgtaggtatggcacgcctgcaaaatcacatcaactacgccatcgacctgatattcctccaccatctggctgagcattttcaggcgctgatcgttcggcgaaacacaggagcagccaatcgccagatatttatccgccagcgcgtcgtagacatcgcccgtttctgccacgcattgctcggtcgctttcgccccggtgcagttttcataaccgacaacccagccgccattctcttcaatcgcgcgcaccactttttctgctgcgccgccaatcgggcagccggtgattaaaatgcgcggacgcgggtccagtcgctggccttcttcccactgctgacgaacgcgggcggtcattgcatccagttcattgatcaacgcctctttatcgaaccggaaggttgcgccgtaaaccactttcagaatgtcgctgccgctaagcgccggaggatttaactgcccaagatgataaaaattagccagtgcgcgacgttcgcggtttttcagcgcaatggcatcgcgcagagcatcttcgctaatctcgtgcccaaaacgttcttctaccgttttttgcaagcgcagcatctcggctttccataacgcacgcgaggcatcgtccttaacgctgttgggcaattgcatcacatgaacaggcttaaactccgccatgtattcatacattttctttttgccgtcgcaggtggtttcaccgaccaccagatccgaaaagtagaagtaggggcatttatcggttttgccgaagccgtagctgcttttaatcagcgggcagaggttgcgcggcagatctttctccgcttcttcaatggtttcatcagaggtggaacagagcgaaaccacaaccgcaccggctgccatcgggatctcttgcggcataaaggtgcagtaagtgccaaccagcggaatgccgcgctccttgagatccatgacggtgagaaagcctgtctggcgagcttcagagaactgatcgaaaatggcgggtagatcggtgacaagtgacatgattttccttccccgtaccacgggagataatgaaaagaggccacattattaccattcttttagtatggtttatttgatctctctcgcggttagccacttagtttttcatggatttctaaaaattgccgagggggaacaaggccgggagctgcgacagcaaatataaaattagcccaatacaaccgccaaccagcgtaccgttgacacgaataaactgcagatctttgccgatatttaactctatttgccgcgacatatcccgcgcatcccagctttttaccgtatcgctgatgtggcgcgtcaggaatgcggaaaactcaggcgcgacgcggtgcgcggcttgttcaagatgaccatttaacgacgcccgcaaggcatcatcggcaattaacgtttcgccaaaccattgacccgctcgtgcgatgcgttctttcacacgagaatcttcactgttgatatccactttcagccattcccgtaaatccccccacaattcactgagatagcgattaaaagcttcatcttctttcagatagctttttacggcatcggctcgcgctgccatttccggatcgtttttcagcttgtcgatcagggcgaaggtggcgcgatcaaacgcatggcggatctgatgcgcacgatcgcgactaatatcatcaagcaaagaattcaccgcgtcagaaaccaactccgcgctatgttcgcccaaccattcggtggggagaattttggctttcagtggatgctcgctctccagccagcgaacaatttgctgggcgataaacttgcgcgatttatcgcgctggagaagggcgatcaactgtgcgatcagcgtatccagcagcacctgatgacgatcgtttttggtcatactctccagcatcaacgcactggtgccggaaagatcgaccttatcaatcgcccgatggaccgcgcgcttaagcaggcgctgaatacgcgcatcatcggtaagttcgagaaaaccgctcatgatctgcaacagatgctgaccaacgcggcgggcgttttctggctggctaaaccagttgccaatcagcaacgccggttcgtggcgtcgaatcaatgccaccagggattgagtatcaagaaatttttcctgcacgaactggccgagattttcgccaatccggtctttattacgcgggataatcgccgtatggcgagaaatgatcggaatcggcacgcggcgaaacagcgccaccaccgcaaaccagtccgccagcgcgccgaccatcgccgcttcagcaatcgccttcacgccgctcacccaaaaattgggcggcaaaaacagcgtaacgacaaaggtagcagcggcgataagcagtaaagagagcgccaaccttttggcgcgtctgagttcgatgagtttattcataacgttaagaatagagcctgacggccggatcgcgcaaaaatcactgctcctccactagctcggctgcctgatgctggcgcacgcgattgagcaatcccgccagggtgaaaacgacgataacgcccgccacaacggctaacagatgaaacggcaagcgaccgccgttaaaccatagccagcggccgatttcgaccgagaccgacatcaccatcaggatcaccatatttagcgatgcggagacggtccctttcggtaacttattggaaaacagcgtaaagcggaataaggtcgggaaaatcaaaccaatcccgaaagcatacagactggtgcccagcaccgaccacagccagacgtgcggcgacagcagattgccgacaatcaacagcgagaggccgaccagttgaatgggtacggcacgccagataaaccgcggttcggtcggatctttaacaaaacgcgccacgatggcattcgcaacaatcaccgcgccgaacaccggaacctgtgtccaggcgaactgcgaagttgttaagctgcctgcatcgataaggatcaccggcgagacagccacccagctcatcatcgggatatagcttaaagagatggttgctgcgccaaagaggaacagccgattgcaaaagacattacgaaaatcgcgcaagacgcttttggcgctaaacggaaccgcgccgcgcttcaccgtctctggcatcgccaacagtaagccaacaaatgagataaaacccataaccgcaatgatggcaaaaaggactttccagtgcataaagtgcatcagagctgcgccggaaagcgggccgataatcggcgcaatcagtacgatggaggtgataatcgccatcaacttgatcccttttgtctgtccgaacgcctcctgcaccgtgacataaccaacggtggcaataaaacagatactggtgccctgaattgcacgcgcgataagaaactgtgtcatagacgttgtgaacattgtcgcggcgcaggcaagggtaaaaattagcgccccggtaatcagcaccggcctgcggccaattctgtcggaaagcggccccagcagccactgtaacgccataccgccagcaagatagagactgacggcagcaggggccagactgacatcggcattaaaatcacgtaccacattaatgatcccaggctggatcagatccgtcgacagatacgcagcaaagtcatacaaaatcaacgccatcgggaaaaacagcgtggcggcatggcgggtaaaaaaacgtggcataacaaacaactccttgtccggagaaccccaacggggaaaacgaaattcaataccgtcggtaatgacgaaaggcaggtgagaagggcaacgagactgcaaatgtactgaatttcatgtaatcaaccacactgcctgtgaacacacagacagagaaatactttctgacttcgggtcagaatgtataacgattacaaatagtcatcagcacattacacctcttgaattgatgggttgcatagaaaatatacaccttaagtgtaattaaaatttgcggttaatcaaaagagcgcggtggaaaggggaatatctgccgggtacaggacatgtaaaacgcgagcttgtttccggaaaaatgtatcgtttgcagaagaataaaaatagcctggaaagcgcctcggggaatgggaaattgccgggtgagaatggttttgttagtcgctaaagtcaggccatctttttcaacaggtgatggatcgccatgacaaacttcacgaccagcacgccgcatgatgcattatttaaaacctttctcacgcaccctgacactgcgcgggattttatggagattcacttacctaaagatttacgtgaactgtgcgatctcgatagcttaaaactggaatccgccagctttgtcgatgaaaaattgcgggcgctacactccgatattttatggtcggtaaagacccgcgaaggcgatggctatatctatgtggtgattgaacatcagagccgcgaggacattcatatggcctttcgcctgatgcgctattccatggcggtgatgtagcgccatatagagcatgataaacgccagccgctaccgttggtcatcccgatgctattttatcacggtagccgtagtccttacccctggtccctgtgctggctggacgaatttgccgacccgactaccgcacggaagctttataacgccgcgttcccgctggtggatgttactgtcgtgccagacgacgagattgtgcagcatcgcagagtcgccctgttggagttgatccaaaagcatattcgccagcgcgatctgatggggcttatcgatcaactggtagtattactggttacagagtgtgctaatgacagccagataactgcgctgttaaattacattttactgactggcgatgaagcgcgttttaatgagtttatcagtgaacttacccgtcgaatgccacaacacagggagcgaataatgacgattgcagagcgaattcataatgatggatatataaaaggggagcagcgcattcttcgattgttgttgcagaatggggcggatcctgaatggatacaaaagattaccggactttcggcagagcaaatgcaggcattaaggcagcccttgcctgagcgtgagcgctattcatggctcaagagctaatcagagacggatgacaaacgcaaagcagcctgatgcgctatgcttatcaggtctacataacccattaaatatattgaactttaaagatttttgtagacctggtcaggcgttcacatggcatccggcatgaacaaagcgtactttgcttaattcaggctggaacgtggcgatgacccagcaaagataaaacgagtcacaggttatgcatgagaggaaatcaggcgcttcgccgctatttcgaatttattccattgcccgatacacggcctcgccaatttgcttcagtgcttcgcgataggtttcgctgagcggcaaagcgcagttgatgcgcagacaattacggtatttgccggaagctgagaaaatcgagcctgccgccacctggattttcatgcggcacagctgccgcgcgacgcagaccatatcgacctgttcaggcaattctatccacagtaaaaatccgcctttcgggcgcgtaatacagatttcgcagggaaaatattcccgtatccagcaggtataaagcgccaaattgcgctgatagatctgccgcatccgccggatatggcgatgatagtgaccttccagcacaaacgttgccgccgccatttgcgtggacggcacattaaagctgctgatggcgtatttcatatgcatcagtttatcgtgataacgccccggtgcgacccaacccacgcgcaggcctggtgcaatacttttactgaacgagctgcacaacagcactcgcccgtcgatatcccaggaatgaatggtccgcgggcgcggatactccgtcgccagttcgccatagacatcatcttcaaaaatcacaatatcatgacgctgagcgagagagagaacggcccgtttgcgcgcgtccggcataataaatcccagcggattattacagtttggcaccagaatgatgcctttaatcggccactgttccagcgccagttccagcgcttcaacgctgatgccagtttctggatcggttgggatttcaatcactttcacgcccatgccgcgcagcatctgcatcgaaccgtaataacagggggattcgaccgcgacaatatcgcccggtttacacactgccattaacgccagcgacatcgagttatggcagccgctggtgatgatgatgtcatcggcggtgaccaccgagccgctgtcgagcatcaggcgggcaatctgctctcgcaatactcgctgaccggctaacaagtcataaccgagaacggtttgcagattatgctgcaccacccggcttagctcccgccacagcggtttcaggctgggcgcttcgacatccggtgtgcttttgcttaacggaacaatggaactgtcgctatgcgcctccagcatatccagcacctgatcccactgggtaatttccaccgggcgctgcaccggacgcgtcatcggcggtactggcggctgggctttacgttgtgcgacaaaataacccgaacgcggctgcggagtgatgagcttcatcgtctccagcgtctgatacgcctgctgcacggtgctgatactgacgccgtgctcctgacttaagctgcgcaccgacggcaatttctccccgtgacgatacagcccttgctcaatccgttcggcaagcagagtcgccagatgttgataacgcgtcatgctgtattccttatgtggaccatacagagagaaaaaccggtacagatgaggctaaaaaaccggatgcagatgctgttttaacctgtctgtatgttaaataaaagtaatatttgaatctgtattgtgaactgccagaaggtggatgatgaagcctctgaaagatgaggaggtagcagatggaatttcacgaaaacagagctaaagcgccgtttatcggcctggtgcaactctggcaggcggtgaggcgttggcggcggcaaatgcagacccgacgcgtgttacagcagatgagtgatgagcggttgaaggatatcgggttacgcagggaggatgtggagtgaggggggatatagatttatatataataaaacgtttttatgtttttaaattaagttataaaaattttcccgagacaattcatcaataggtatggagtgtacaggaatatcttcttcactaacctctttaaactcatgtcgataacggtcaaaaaacgcacagtgattacttgtgttttttgactgactttacaactctcattattcgctattgtgcagtttctctaattgttttataccctggaaagttaaatgtcagctactgaatactttttgattgtttgagatttattttcatttgaaattataaaatcaggtgataaatgagttgtgattaatagatggttgatatcatttttatctaaaattgatttatagtatcgacctgaaaaaatagttgttgccgcctgagtaactatacaatattctgaaaggttttctttcaaattagaaatgttgtggggttttgtttttgtatcttttatctctaaggagcttgctttgggtcaatcagaatacatttcatgggtaaaatgtacttcctggctaagtaactttgtgaatcttagagggttgagacaaccggatggccgtcctctttatgaatatcatgcaaccaatgatgaatatacccaattaacgcagctactccgtgcagtcggtcaatcacaatctaatatatgtaatagggactttgctgcctgttttgttcttttttgctctgagtggtaccgcagggattatgaacggcaatgcggatggacgtgggaccctatatataaaaaaatagggatttcattcaccgccacagagcttggtactatcgtaccgaaagggatggaagattactggctgcgcccaattcgattttatgaatctgaacgacgcaattttctcggaacattattcagtgaaggtggtttacctttccggctactcaaagaatcagacagtcgctttctggctgttttctccaggatccttggacaatatgagcaagcaaagcagtcaggtttttctgccctttcgctggcaagagctgtcatagaaaaatcagcgctgccaactgtttttagcgaagatacctctgtagaacttatcagtcatatggctgataacctcaattccttagtacttactcacaacctaataaatcacaaagaaccagtacaacagcttgagaaggttcaccctacctggcgaagcgagtttccaataccgttagatgatgaaacaggaacgcattttttgaatggactgctatgcgcagcctctgtagaggctaagcctcgactacaaaaaaataagagtacgcgttgccaattctattggtcagaaaagcatccagatgagcttagggtgatagtatctcttccggacgaagtttcctttcctgtaacaagcgagccgtcaactacgcgctttgaacttgccatttgtgaagatggtgaggaagtctctggccttgggccagcctatgcttctctggaaaacagacaggcaacagttcgattacgtaaaagcgaagtgagatttggcaggcaaaatccatcggcaggtttgtcgttagtggctcgtgctggagggatgattgttgggagcattaaacttgatgacagtgaaattgccattggtgaggtgccgttaaccttcatcgttgatgcagatcaatggctgttacagggacaggcttcttgcagtgtgcgaagcagcgatgttctgattgtgctccctcgggataatagcaatgttgctggttttgatggccaatcgagggcagtaaacgtattaggactaaaagcactacctgtgaagggatgtcaggacgttacagttacagcaaatgaaacttatcggattcgcaccggaagagaacaaatcagcatcggaaggtttgctctaaatggaaagcgtgcaagctgggtttgtcatccagatgaaacatttattggtgtaccaaaagtcatttctacactaccggatattcaaagcattgatgtaacgcgttacacgtgctgacaaaacagcattacagccagcaggaagtactgcgttggatcgatgtctgttcagggactcaacctaatgcaaaggatcccgcatttcttaaagtcagggcgcatatcttccagcgtaatacctagggaatatgggcttgtgttgataaagattgcagattaaagcacggtacaccgctcgacaaaggctggccctttggctatgtgtatgtgaaccagcgacaaaattgtgactgtggaagccctgtatacgaagttgcattctgtaatgattgtaatgagcctcatcttctggcacgggacaaaaagggcaaactagtccagtgggaaaataaaggtggcgatgaattctctttgcaggatgaagtacctgttgaacatgacgctacagaagaaaaagtcgaaaaagagaacagttttcagcctccgttgattattgccgcaggagagaccagcgaggcaggttataccctacaacgcctcgaccgtcagacgcgccgtattggcgttattaacaatgacagcattccgctgattattaatgatattgaacaggtttgtagtgccagtggctgtggctacagaggcatgagtgggaaacagcccttccggcgtgcactattaggtgggccattttacgttactaatatcgtgcccaccgttctagagtattgtcaggactttaccagtgatgaaggcaaagagggcgtcggaccagattcgttgccaggacgaggtcgtcgactcatcacctttacagacagtcgacaagggacagcccgaatggcggtgcgtatgcagcaagaagcagaacgcagtcgcttacgcggaagcgtagtcgaaattctcagctggcatcaaaggacgcaaacgtctacagcgccgaatgccaatgccgatctggaaaaattagcggccagggcgaagcaagcccgtgagcaggcagaagaatatcgaagctggggaatgccagaccaggcgaaattgtcacaagcacaggctgaacagcttgaacaggcttatcaggctgcaaccggtgggaaagccgcgactatcctggtatcccgaacctggacggagatggttaacgagcttaaagagagagccgatatccgcgggccggttctgcaatataaccattatcttaagcctgaagtgtttaatgaaaacggcggcccccttaagctttctgaaatgttgttgttccgggaattcatgcgtcgccctaaacggactaacagcctggaaacacaggggctggttcaggttggttaccaggggctggagaaaatacataagagccccttgcactggcaggaaaaaggattaacgctggatgactggcgcgattttctcaaggttacgttggatcattacgttcgcgagagcaacttcacacagctggatgatgagctgaaaaactggattggtagccgtttttcatcaaaattcgtccgtaacccggaatcaaaagatcctgaagataatcagaacagacgctggcctcaaattcgtaatggcaacgtatcccatcgtttagcgaagttgctgatgctgggggctggattcaaaaccgtcaatgcggcaactattgatattatcaatacatggctgaaagaagcatgggcccaacttaccggaccgcttgcagtactgaaacccgatggcaaccgtttttatttaccgaaagagcatatgactttttctttaatcacggatgcctggatttgcccggtaaccaataaaatcctggatacggcttttaaaggcttaaccccttatctgcctacccatatttcgttcgagcatcttaccctggcgcaatatgacacttttgtcgcgcagaaagtcacaatgccggaaatctggaagctggatcgttcacaggaagactacgcagagggtctggcaaaagcacgcgactgggtcagccatgatccgctgatcgcacaattgcggtcggaaaacgtctggacagacattaacgatcgtgtcgtggaaggcggcttctactatcgtactgccgagcactctgcccagcagtcgtcagaacgtctgcaaagctatgaaaagatgttcaagaatgggcaactaaatgttctcaactgttccaccaccatggaaatgggggttgataccgatcgcgtgatgacgctggcctctcgcagccagcaggcaacgattccggggccggagtggcacctgaatgacgaactggtggtgcgtagtctcggttataaaacggtagaactgaacgagtttattctgccggctaaagccaccaacgctgtcgagcgggtcaaagacattcagatccacaaacagttgaatggaccactgtcgcagtttgggcaacgcttctgggacgtgctgtttaacgaccatgaagaagcgcagtcactgatgaataacacgcgaattaccggcgttcactataccgatcgctatctgcaaaacccggttgcgctggcgttgttgggatcaattctgagaccgctaaaaacaaagctgaccgatggcgctgaagtgacgctggatacgctatttaaagataaagatcgccccggtaaccggcctttccatgactggatgagcatagcggattttcaggatttcgctgatcagtggtttgctgctgcgctgggcaggccggtagaactgacggtgttcgactcgccgcgcgatatccctcaccatcgtaaactgacggtgacttttgaggatggtcaggtattgaagatccgcttcgatcaggggatgggctactggcgcatcaacttttcatcgcaatggcattactttgatttccgcgatgacgtttctttccagttagtcaaaatggctcaggcctgcaaggaagggaatgtcgccaacagcgaagagagttgggcaacggatgtgctggtggaggtgatcgcctcctgatgatgagccgctcccgatgtggtgtcgggagcggtattttctataaaacttaccgcttatttgagatattcatcgaaaatgtcgagtaattcttgatgtatacacggccattcctgacctaaattgacggtacacaagccaatatcgaagccattaattttataacgatgtttcactgcggtatctacgtggggatatattaataacccccctatgttttcgccattttcaggctttaacgaccataagtaattcatcagttgataaagattttgcgaatgaaatttttctgttcccattcgtcgtgaaaaaatgctcttatagtatttggcgtcaacgataagtattttttctgatgagcgaatggtgatgtcagtttccattcgaggtaacaaattaagtgactgatccgatatactcgatgcatcccattttaaataagagcgggttgtgtttgcagacgttaattcacgacggcaaaattcataaagaaacttttgataaagtaatgacatctctttttcgtttctttcaaaatcatagaaacggtagtgtcctttgttttgacctggaatagaattattgacgatgaatttgcagacactgataacgaatttataataacgcgtattttttccgccattcagatagctgaaatgctgcggagttaaatgaagagtgctaatgcccggtaattttctataaagtgaacgagcttcatctctgatagttgaatttaacttttcatgcttaattaatatggctaatgtgctttttataattcggttagccagcgtgtcttcattaagcatatcaaaagtactgacggttttcccatgattaagatggaagccgcgtattgttttagcaaactctattcgccctttgatgccaggaatgatctcggtgttaggattgtaatcaagctcaagccctcggcgtgaaagctgtaaaacccctttatttaatacataccccaggatatcaagaagattgttaccgggtatggcttcaaggtttgcctgcttaatttcctgtaaataaccccatgcataggtaagcatgtaatagatattacggacaggtatcacgggctgttccactatgagtcccctaataatttgttggtccatttctgttgtttataggggtcatcaaagaaatattcttcgagtaaaggggcgatatccgtcatcacaatttcattaagccattgcgtatccggagaggtgccatcttccaacccacagcagaagtaactatgcccaatgcggaatcctttcccaaggatagtggcctctttgctgatttcctggttcaactcgttcattttttggcataaagactcaacaaatgaaggttctgcttttttattcagtaaaaaattccggaactgtggtgtatcaaaacctggctcaatatctatgaaagaaaatcgtctgcgtagggcatagtcaacaacggccagagagcgatcggcagtattcattaaaccgatgatataaacattctccgggacatagaatcgttcttcatcgttttcggagtaggttaggggaacagaccagttttcacctcgtttatcatgttccattaacatcatcacttcgccaaatactttactgagattggcacgattgatttcatctataataaaaatatactttttctctggctgctctttagcttgctgacaaaaattgtaaaatatgccgtctttacgtcggaagccgacgccattcggacgatagccctgtataaaatcctcatagctataagattgatggaactgaaccatattgacgcgttgcggagccttttctcctgtcagcaagtaagccagacggcgtgcaacaaaggtttttccaacgccgggcggcccctggaggataatattttttttgatggttaatcgtttgagtatcgtctctattgtggtttcagggataaacaaatcatttaacgcatcttccagacagtatgattcagtttttgacataggtggaataacactcttgccagaattaaatattaatttatagtcgttgattatgttgtccagcatagaggcaaatcgggtgtaatcaataccctgtgagactttttgggaacaggcgtaataggactgtccgtattttttaggatatacacccgaagttgcctgaaaatactctgcgattgttttaggtatgtctgaagagaactgccattgggcatgtggttcattcgtgtcgcttataccataagccaaaaccaactcatcaaaatctttataatagagaataacgggatatataccgttagaagcttcctgaccttctccaagaaatgcaaaccagggaatagacgtaaaattaccataaccgaaactcaattttactcgcaggttacggtaagacgttggataatctttagtggattgcgaacgttgttgctgtgcttgcttaataaatttttcaatccagggttgaatagattccataagatatgccttcctcattgctaagcctctattatcgctttcgcaacgtactgaaacaatagatttttactgcaaaatcagactggtaaatatttactgagggggaaagtttctattgagtcagtggaaggctcccggtggttaaccgggagtaaacgctgttacgcgactttctgtttaccggcaatcactccaataaacgcctgcacctgcttttgtttacgcgccgacagtttgcacacctggcgtagcgactgcatcagttcgctctcctcggcggcgggtggttgggcggtgaggacaatacagccttccatcactttgacatctaccgccgtgccagtggcaaaaccggcggcttccagccactgacctttcagggtgatggcgggaatacggctgtaatccgggtagcgactcgcataaccgacggtgacatgacggttatttgccggggagacttctgcttcgaacggttgtgcaatagaatgcgtgtcagtcataactgctattctccaggaatagtgattgtgattagcgatgcgggtgtgttggcgcacatccgcaccgcgctaaatacctgtatatatcatcagtaaatatggggaaagtccagctaaaaatagaataaaatgggcaatttctggaatgatttaaatatatttatgtgggttatgattggcgtgaaataataaaaagcgcaccggaaaggtgcgccagaaaataatgttcaggattttttacgtgaggcttttttacccccgctagctgcgcgttcagctttgattttttccagcaacgcggcggcgctgttttctccgctgatcaaatccgggttttcggcccgccactgggcggtaagttcaccacggaacgcttttgccaggatggattgcgtcaggttgttgacgcgggctaaggcgttgttgacctgtttttctatggtgtcggcgtaggcgaagagttgctcgacgcggcgaacgatttcggcttgttcttttactggaggtaataaaacaacttgggatttgatatcttttcctgaaatacctttttgaccagaagttgttttcacgcagttcatcattgcatttcgtgctgagggggatgaaaaaaatatttcgatatattctggtaaagcatctttggttaatcgagctcgaataagtttatcaggatatagcaaattttgatgttgtaattttttcaataacccacaaacaccaacaaattctaaacttccgttatagcgagtaaataaaagatctccatcttgtaatttgtggcggtttagttcactttctgaacattctagaaaccgaatatcgttttgatctacatggccagcacgtacagaactaatgcgtagtattggatgaccaacaccactttcatttggctttgatgaaagaccattacgtaattcagttaagatagattcaaaatttaacttcttaaatacagaatgttgcggctcaaaattacgccatttttctgtcaattttccattaactgcgccccccaataccgcttgacgaaaacgtttcaggatttgtgggatttgctcaaaacgtgctttggtgctgtctacctgcgccagcagcgtatcgagtttttcagcgatgattttttgttcggcaagtggtgggattggtatatttatcaaatcaaagcttgccggcttaatattattaatatttgcaccagcagaaagtgatgaaattttgtttcgataaagagaagattttgtgaaatgagcaataaaaccagaaaatataagtttttcaggacgtaatacaccgcaaaatgcgccgaaactacattcaaatggtagatgctgatgtgcggatttaccaactacggatttgctccctgatgacattgcaataacaatatcttcaggagatattttttgactttctttaacaagatttttaggaacaaaaaccaagtccgtagtatcaaacttgccattctgaatattgttcgcacggataagaggcaaataatcatcttttagataatttattgcctgctcttttttatacgttactcctcggattagagttgtgaccgtagatactggggcgataacccacccctccggcaatttccccgcactcattccttcaccccaccaaacgcttcttccagcaactgacgctgcaaatcggcctcatcgctcgcccccagttcacgcatcagcgcatccagttcagacagcgcctgtaccagttcgcccatcgcttctgccgctaatacatccggctccggcaggctgtcggcatcaatactgtctttatctttcagccaggagatatccagcgaatcggattttgcggtgcggatccactcacggctgaacttgcgccagcggctggtagcaagatgctggtcggtgtttttgttctcttcgctgtcggcaacttccgtctcttcggcgttaaaactccattcaccttcagtgcgcgggcttaaaccgtgcgggtcttcgccatacacgcgctcaaacggctgcaaatgctcgtcggtaaacggtgtgcgcttgccgaaactcggcatattggtacgcaggtcatacacccacacatcatcggtacagttcttatcctgattcgggttcgccaccgtccctttggtaaagaacagcacgttggtcttcacgccctgagcgtaaaaaataccggtcggcagacgcagaatggtgtgcagatgacacttatccatcaggtcacgacgaatgtcggtgcctttgccgccttcaaacagcacgttatccggcaccaccaccgccgcacgaccgccgggatgcagcgtttcgataatatgctgcataaagcacaactgtttgttgctggtcgggtgaacaaaggtgcgggtaatgttggtgcctgcggcgctgccaaacggcgggttagtggcgacaatatgcgccttcggcaggttttcaccgtcgctacccagagtgttgcccagacggattgcgccgccgtggtcgaggttgccttcaatatcgtgcagcaggcagttcatcagtgccagacgacgggtgccgggcaccagttcgaggccgataaacgcgcggtggatctggaaatcctgcgtgtcgccatcaaggtcgtccagatcattggtttgcgacttaacatagcggtcggcttcaatcaaaaagcccgccgtacctgccgccgggtcctgcaccacttcacgcggctgcggtttcagcagatgaataatggttttaatcagcggacgcggggtgaagtactggcctgcaccagacttggtttcattcgcgttcttctgcaacagcccttcgtacatatcgccgaagtcatcgcgcgacttaccgtgcgcgccgttgtaccagtccagcgaatccatattgctgaccagtgcggttatttgtttcggctcggtgatggtggtactaacattatgaaaaactgcctgtaccagctttttgtcatcttcgcctaaatgcacgagcatttttcggtagaactgcaactgctcctggccgatgcgggatttcaggtcatcccagcggtaaccttccggcaggtattccgcttcctgaccggtctctttacacattttcaaaaacagcagcgaggcgagttcattgacgtagttttgataggaaacgccgccatcgcgcaggttgtcgcacagcttccacagcttcgcgaccagatcgttattgttcattgtgagttccgtaaattaagcagcggcccaaattcatcgagccgcagaagaagaaattgccgagggtaatatacacaaaatcattcaggttgcatcaaggcggcaagtgagtgaatccccgggagcgtacagaagtacgtgaccggggtgaacgagcgcagccaacgcagaggcagcctgaaggatgaagtgtatacgtgtcaggccagctcgtcccagatataatcgctgaatttgcccagcagggtatcgagattatcgtcaaaggttctttgcagcatcgccttcccgccgcgacggtggaagttgccggttttgaagacatcgtcgtcgagcaccactttctctttcagcgcctgcgctaaacgatcgagccagcttaattgctcgctgctccagtcgttttcgcccttaatgcgcgtcagcgcgtgatcgacacgttcctcaaacggtttcagcgcatcgcccaccgcagcgcggcgaatatgaccaatcagccgggcggcgatatcttcattgcgcgtctctttccatgctttgcgcagggaagattcctcaaagtgctggcggtcaaaccactcctgtagctcgaccagccctttacgggtgagatcgcgcgggcgattaataactgcctgcaatgccggttgcgcgttcggggaacgttgcaccagcgagtcaaaggcttcgaggaaatcctgcggcgtgtcgtaatcaccgtacagcgattttacactcaccacttcatcgtcgatatcgaggaagatcggcgcatcattcaggttgttgatgtccgttttcagcttttccagacgggcgataaagccaggcagtttgttaaagacttcggcgctccagtgcggccctttttcccgcaggcgcgaggcgaagccgttaaagttcacgcccgccgcgtcctggcatagctcatccagacgacgcacctgtttatctatcgtttcgctgcggtcacggttaaacgtggccagaccgatgatacgctggagcttcgccaccagttgttcatggctgtgctcggcaaaactgcggccatccgcttcggtgattttataggtttctgaatcggtaatttcattgaccagcgtttgcagttccaccttcgggcgcaccaccaccggacgcatggtgtcgacgctctccagcgtgctgtagatatcgacacagtcaaaaatcttaaagctggttttattcacctccgggcataagcgcgtggcgcggcctttcatctgttcgtacagaatgcggctgcgtactttacgcaggaacacgatattacagatcgacggaatatcgacgccggtcgtcagcaggtcgacggttaccacgatattgggcagccgctctttattgaagcgggtgatcatggtctgcactttgcgcgcgtctttatcggcatcaccggtgatcttgatgatcgcgtcgtgctccagttgcggatactttttcttgaacgcggcacgcagctcttccaccaccatatcggcatgggcattggtgacgcagaagaccagcgttttttgcgatccggtcgggtcaagataattggtgagttcgttacagacggcgcggttaaacgccgggatcaccaggccacggttaaagtcggcgacttcaaaatcctgatcgtcttccagggtgtcattgatcacttctccctgcgggctgatgcgctctacctgctcgcctttggagagataaaccccctcctgcgcgttgcgggtgatgatctgaataggcggatcctggtcgatcagaaaaccgtcgataaccgcggtacggtaggtataacggtaaaccggctcgccgaaaatctgcacagtatgtagcgccggggtggcggtgagagcgatttttaccgcatcgaagtgatcgagaatgcgacggtaggcagagacgtaatccagctggctgcggaactgcagttcgccttcggtctgctctttatcgagaatatagccgcgatgcgcttcgtcaacgacgatacagtcgtaacgggccaccggcatcggttcatctgattgcagggtgcgtttcaccagcgactgtacggtggcaacgtgaattttggtgctgtcttccgggaatttatccgtcagccctttaatgtcgaaaatgctgttgaaggtgtcgccgttaatacgcgtatcttcaaacgcgcccagcgcctgttcgccaagagaacggcggtcgacaaggaagagaatgcgtttaaaacgctgggactggatcaggcggaacatcatggcgattgccgtacgggttttaccggtaccggtcgccatcgccagcaggatctcttgttgccccttgacgattgccttttcaaccgcgcggacggcatcttcctgataataacgcaggcccagctcgctcatgccagggttatcggcaaaccactgattctgtttttgcggttcgctgccgagcatttccagcagctcttccgggcggtgccactcgggtaaggctttcgacatattgcgggtatcacgcacgtcgcgataccagatgccgcttttggtcttcattgttgcgcggtattcgcgcccgttggtcgagtagcagaaggggattttaaaccgttgtttgccgctggtgtcctgccagctggtttcatactctggcactgcttcatgcacttcatccggtgagtagtgctcaagcaaggtttcccgcaggaagccattatcgaaacatttactgtagcgatacgactcattgagcctggcgggaacgtcgatattgttacgtttcgcctctaccaccgcgatgggtttgaggccgacaaacagcacataatccgcaaagccctgattacccgtttcatcttttccggtcggccattcggcaatggctttattgacgccgggttccggacgtgcgcctttggagaagcgcagggttttgctgtcggcctgccagcctgctttacgcagttgcgcatcaatcaggaagcgactctcttcttcgctaaggttgagtgtgcgcttgatggcctgatcggtaatttctttgtggtaagccttacgttcctgttcggtctgttttgccagttccgcgttcttctcggcgagctgtgcttccagtgccgcaaggcgagcctgggtttgcgcttcggtttcctgctgtttgccttccagaatggcgatatagccgttcagggcaaccagcttctgctgttgcgcttcgacttctgcctgagtctgcgctttttctcgcacctgctgttcaagctgttgttttagcgtcagcacttcctggtgatagaggttttcaccacgttccggcaacacaaacaccggcaccgggaagtcataatctttagtgaccagacggtagtaccagacagccaggcggaacccgagtcgcaggcacatctgggcatcgttgagatcgttatgatattcgtgcaccgcctggttaccaatgcggcgtaatttgtgaaatacagagaggatgttgtcatcaacaaaggcgattttgccgagttcacgcaggagatcgtgttgattctcacaaggggggatgttgagtaacagaccaagatgtttcgctgtggcttcgccaaacatacgcattttaatcagcgtcgtgttgggatcatccgggtagttattttccgccgcacaggcgatggcataagtgaagtcgttgacgcccttcaggaattcaaaattggatttattcatcattgttattaatccattgctgtgcgggcctgtccaaatatttaaggcccataacatctcatcttagctttctgtacctttccgggcaatgaccacggtcacagcaactgactcatttctaacgtgttcgtctatttttgtagtgctatagtagccgaaaaacatctacctgattctgcaaggatgtactatgacggttcctacctatgacaaatttattgaacctgttctgcgttatctggcaacaaaaccggaaggtgcagccgcgcgtgatgttcatgaggctgccgcggatgcattaggactggatgacagccagcgagcgaaagtcattaccagcggacaacttgtttataaaaatcgtgcaggctgggcgcatgaccgtttaaaacgtgccgggttgtcgcaaagtttgtcgcgtggcaaatggtgcctgactcctgcgggttttgactgggttgcgtctcatccccagccaatgacggagcaggagacgaaccatctggccttcgcttttgtgaatgtcaaacttaagtcacggccggatgccgtcgatttagatccgaaagccgactctcccgatcatgaagaacttgcaaagagcagcccggacgatcggttagatcaggcgctaaaagagcttcgtgatgcggtggctgatgaggttctggaaaacttattgcaggtttctccttcgcgctttgaagtcattgttctggatgttttgcatcgcctggggtatggcggccaccgtgatgatttgcagcgtgttggcggtactggagatggtggcatcgatggtgtgatatcgcttgataaacttggcctggagaaagtttatgttcaggcaaaacgttggcagaatactgtaggcaggccagaattacaggcattttacggcgcactggctgggcaaaaagcgaaacgtggggtgtttattaccacttctggatttacttctcaggcgcgtgactttgcccaatccgtcgagggtatggtgttggttgatggggaacgcctggtgcacttaatgatcgaaaacgaagtaggggtttcttcacgtttgttgaaggtgccgaaactggatatggactattttgagtgaaatatcaggccggatgcggctgcgccttatccggcccataaccccttacttcctcaaccccgcaaacgcagcccgaatctcttcctccggcagctggatcccgataaacaccatcgtgctatgcggtttttcatcgccccacggcctgtcccagtcggcgctgtagaggcgctggacgccctggaacagcaggcggttaggttcgccgtcaatccacagcatccctttgtaacgtagcagtttatccgccgactccagcagcaggttttccatcacgcgggaaacttcgctgatatctaccgggtaatccagttccaccacaatcgacgaaatatcgttttgtttatctgcgataaagtggaaacgcggtttggtgctgacgacgttttcttccagcataaaaccgttggtgttgaacagcaggcccagatcgatgtcgccgtgggtgacggtgtagaccggtgcgcgggcgttgatgcgcgccaggcgttcatgcagtttttctgcttcgcctgcgacgtcggttttggtcagcagaatgcggtcggcgtagccaacctgtgactgggcgatggtgaactggttcatctgctcatcggcatgtaccgcatccaccagcgcaatcacgccgtccagcagataacgctggcataaaacttcatgggagaaaaaggtctgaataatcgggccgggatcggccatgccggtgcattcaatgaccagacggtcgaactgaatattgcccttgtcgagattgtccagcaggtcgagtagcgcgtcctccagctcgttggagcgcgaacaacagatgcagccgttggtcagcgttttgatctgcgtggcgcggtcgccaatcagttgatcatcaacagagacttcgccgaattcgttttcaatcacggcaatcttgtagccgtgctgttcgttaagaatatggcgcagcagggtggtttttcctgcgcctaaaaaaccggtgagtagggtaactgcaatcgggttcatgctctctccattaacaacagcgcataccgcctttaccatcgccgccgtagcgcgcgttctggcgttcgcggaagaattcttcatagctcatgtacggcttgtcgggatggttggtcttcatatgctcgacgtagttgtcgtagtctggaatgccaatcaacatcttcgccgcctggccgagatatttttttgcctgtcctaagttaccaaacatagttcactctgataagaacaaagccccgccgaagcggggctaaacacggttagtggtgcgaagagatcttcacgccgccttccgggattggaacgtacggtgtttctttgtcagtacgtttgtcgctgttacgcaccgcaagccaggttttgaaaccgtagaagatgatgctgtacaccacaatcaggaacagaatactcagacctgcgttggtgtagttgttcacaacgatgtggttcatattggcaatctgctgcgccgtcaggtcagtaccgttagcaatcttctctttgtactggcttgccatgtagaagaagccttccatctgcgggttggtgctgaacagtttcaggcccagcgcccaggtggtgcagataagcagccatacagccggaacaacagttacccagatgtattgggtgcgcttcatcttaatcagcacaacggtgcccagtaccagcgctacggctgccagcatctggttggagataccgaacagcggccacaggctcttaacgccgcccagcggatcaaccacgccctgatacagcaggtagccccacagacccacacagcccgcagtaccgatgataccggcaaccagagaatcggtttttttcaggaacgggatgaagttacccagcaggtcttgcagcataaagcggccagaacgggtacccgcatccagcgcggtcaggatgaacagggcttcgaacagaataccgaagtgataccagaagcccatgtcagccatcggcagcactttgtggaacacgtgcgcgatacctaccgccagcgtcggcgcgccacctgcacggttcaggacagaaggctcaccaatgtctttcgcggtttgcaggatctgctctggcgaaatcacgaagccccaggagctgacggtcgctgccgcgtgtgcggtaacgtctttcagctgcgccatgatgatcggcgcgttctcgccacccatttcatgcaggttaggcatggtgatgccaaggccagcaggcggggtgttcatcgcgaagtaaagacccggttcgatgatggacgcagcaaccagcgccataatcgccacgaaggactccatcagcattgcgccgtagccgatgaaacgcgcgtcggtttcattagccagcagttttggcgtcgtaccggaagagatcagcgcgtggaagccagataccgcaccacaggcgatggtgatgaacaggaacgggaacagagcgcctttccacagcgggccagtaccgtcaatgtactgggtcatggcaggcattttcagttccgggttcagcaccacgatacccagcgccaggccgacgataacgccgattttcaggaaggttgccagatagtcgcgcggtgcgaggatcagccacactggcagcagtgcggaaacaaacgcatagccaatcagcgcgaaggtaatggtggtgtctttaaaggtcagtgccggaccccagtacggatcgtgagcaatcacgccaccgaagtagatagaggcaaccagcagcacgataccaatgacagagacttcacccacacgccccggacgaataaagcgcatgtagatacccataaacagcgcaatcggtacggttgagcaaacggtgaagacaccccacggactttcggccagggctttaaccacaatcagcgccaggacggcgaggatgatgatcatgattaagaaacagccaaacagcgcgatagtccccggtactggtcccatctcttctttgatcatctcaccaagagatgcgccattacggcgagaggagataaacagcaccataaagtcctgaaccgcaccggccagcacgacccccgccagcagccacagcgtgccaggcaggtagcccatctgcgcggcgagaaccggacccaccagcggaccagcaccggcgatagcggcgaagtggtgaccaaacaacacgtaacggttggtcggaacgtagttcagaccgtcgttgttaataaccgcaggcgtcgcgcgcgtggggtcgagtttcatcaccttctgggcgatgtacagactgtagtagcgatacgccaccagatacaccgatacagaggcgaccacgatccacagggcgctgatgtgctccccccgacgtaatgcaactaccgcgaggcagaatgcaccgatgattccgagaatcacccagggtatgtgcttgaatatctttttagtatccatagtaaaacctggcatgtattgattaatagttggccgaagccgttctaggtttgcgttgcgtttgaggaggtaaattgaccgctatcctgtagtgatgttgccagagttacgcgcgcgtaaagtaaggtaaataactgagtggttattttagggatgtaagcggtcagttttgcggttgagcggcaaaggcgtcgtttaagtgacgataaatatgtgattcatatcacatatttatattgtgaataatttatgtaaataatggctttttaaattcagagtgtgaataaaattcactcggcgtaatctccgcgggatattcataaagtttttcctttccaggccgaaaatcttgcatcggtccacaggaaagagaaaccatgttaaaacgtatcaaaattgtgaccagcttactgctggttttggccgtttttggccttttacaactgacatcaggcggtctgttctttaatgccttaaagaatgacaaagaaaatttcactgttttacaaaccattcgccagcagcaatccacgctgaatggcagctgggtcgcgttgttgcagacgcgtaacaccctcaaccgcgcgggtatccgctacatgatggatcagaataatattggtagcggttcaaccgttgctgagctgatggagagtgccagtatttcgctgaaacaggcggaaaaaaactgggcggattacgaagcgttgccgcgtgacccgcgtcagagcaccgccgcagcggcagagatcaaacgtaattacgatatttatcacaatgcgctggcggagctgatccaactgttaggtgcaggcaaaatcaacgagttctttgatcagccgacccagggatatcaggacggtttcgagaagcagtatgtggcttacatggagcaaaacgatcggctccatgatatcgccgtcagcgataacaatgcctcctacagccaggcgatgtggattctggtgggcgtgatgatcgtcgtactggcggtcatcttcgccgtctggttcggtattaaagcctcgctggtagcgccaatgaatcgcctgattgacagcattcgtcatattgcaggcggcgatctggtgaaaccgattgaggtggatggctctaatgagatggggcaactggcagagagtttgcgccatatgcagggagagctgatgcgtaccgtcggtgatgtgcgcaacggggccaatgccatctatagcggtgccagcgaaatcgccaccggcaataacgatctctcttcgcgcaccgagcaacaggccgcttcgctggaagagacggcagccagcatggagcaactgaccgcaacggtgaagcagaacgccgaaaatgcgcgccaggccagccatctggcgttaagtgcttctgaaacggcgcaacgcggcggtaaagtggtagataacgtggtgcagactatgcgcgatatctccaccagttcgcagaaaatcgccgatattatcagcgtaattgacggcattgccttccagaccaatattctggctttgaacgcggcggttgaggctgcgcgtgcgggtgagcaagggcgcggttttgcggtggtcgcgggagaagtgcgtaatctggcccagcgcagcgcccaggcggctcgtgaaattaaaagcctgattgaagactcggtggggaaagtggatgttggctctacgctggtcgaaagcgccggggaaacaatggcggagattgtcagcgccgtgacccgcgtgacggacattatgggcgaaattgcttctgcttctgatgagcagagccgtggtatcgatcaggttggcttagcggttgctgagatggaccgggtaactcaacagaacgccgcgctggtggaagagtctgccgctgccgccgccgcgctggaagagcaggccagtcgcctgaccgaagcagtggcagtgttccggattcagcaacagcagcgtgaaacatcggctgtggtaaaaaccgtgacgccagctgcgccgcgtaaaatggccgtggcagatagcgaggagaactgggaaacattttaatcgccatgaaaatgcccgataagcaaaatgttatcgggcataaggagattaatctttacgtgggtcgttgatcggctgacgaaccaggaagatgtacgccagtgcccccgctgcggtgacgcaaccgcagatgattagtgccagacggaatgagtgggtggtatcaacaataaaaccagtaatgatcggcgcaaaagaggcgcagatgaagctggcaaagttctggatactgcccaccgacgcagtcatgcgagaagcaactgcgacgtggatcaagccccagcaggatgttccggcaaagtgaatacagaacagtgccatgccaatcagcagaaccgccgtcatggatgttgtcgcttgtggtactatcagcgtaaaggcggcagaacagaacatcccggcaataatgcagatcttacggcttttaatcggagccattccccctttgaccagccagtcggtaacgtaaccgttgaccagcatcccggcagccccaaacaggaaagggatagccgccatcaaccctgtgctttttaaatccaggttataggctgtttgcaggtaaccaggaagccaggccagatacagccacgcagtgtagttgatgccactgaatccgagcatcattccccacattgtacggttacggaacaggctgcgccattcggcaaaactgagcggatctcggcgggcattgacgctacctgcattgagataagcttgctcaacggcagtcagttctacgtgctcgcggttgcgatagagcatataccagccgatggcgagaaaaatccccagtacaccaatggtaataaacatcccgcgccagcccatcaccagcatcatcgccgccagaatcggtgggcttacggcaacgccaatggtagaagctgcgttgaagaagcccatcgggcgtccgcgctctttgatgttgaaccagtcgttaatgacttttacaccgcatgggttcatcggcgcttcaccaatccccataccgatacgcaccaacacgaactgcgtaaagttgtgcaccatgccagacattgcctggaacagtgaccagaagaacatccccagtcccagcatcaggcgtgggcctttacgatccaatagtgggccgcaaggaagttgcgcaatcccgtaagcgagtgaaaacacggagagcaaagcgccgatttcggtggcacttaatcccaattcttcacgaatcgttaaatttgctaccgacagcgaactgcggtcgagataattgattaccgccgcaaaaaataataacaacatggcggtggtttgaatgcgtttaattcgggtactgcgttgaactaatccatctggtggcacgggaatatctgccgacgaagatggagtaaatgaagaacgcggatcgatggtgatattttctttttccacgccggactcctgtatttataattttaattgtttacgtaattgtgcattacgcaaggttgacattaacggcaggttaaagttttaggactttactaccgctcacaaaaacatttttagtcgactgattgtgagcataggtaagcgggaatttcccggtatttatcttttgataaaaccgtgcacccgctaatagtttgctgtttttaatccgtacttaatgagcataacgcgtgttctcattaatggatcgaatcattgattgtttagctgaattcaaatggttacggagcgcaagggtggcatcaaggtcactgcggcaaatcagagcgctgagaatggtcatatgctcatcgacggcaatgatattgcgctgtttaagatcgctttcgtcccattgatagtgaaaatgaaagatgactgagatgatctcaagcgattgatcaaaaaagatattgtcggcagctgaaagcagtaaggagtgaaaatctctgtcaagttgcgagaacatgcgaaagctattgccgatgttgtcacgcagtagccgatgacgttcgagcatggttttcgcctgcagccagcggggatcatgatcaggcaggttgagaaagtgctgaagtgaatgtgtttcgagcatttcgcgtagctcaaacagctgctcggcgtaggattgatcgaattgcttcatgctccactggccgcgcttttcgctgtgaataagattataacggccgaattttaaaagatattctcttactacaaccgggctgacacccgcggcccgagccagttgcagttcagaaaacgtttcccctgggcgtaactggcgctggtttatcatcgtgaaaaaagcctgctcaaacactttgttttgttcactcattgaagcggtagtacaggcgaaaccgtcatcatggtcaggtttacgcgcaataacatagtcgtttccaacctgcgtcaagacgccgcattcgcgtaagtggctgagaatatgacgcactgtggtgcggctgatgttgtacatttccgccagcgcactttgcgatggaagtggggaagggatatgaccccgcgccatatcatcaatgacctggttaatcacattgtggcgtaaattttgtgaacgactcatattttcctccttgtgagtccattaaaacccgatttaaaacatttttatgcgtgtgttttcacaaaaaagattttccgttccgctgccatttttcattttcattgatatctaaggcaacaaaaagtggagagccgaatcatgtctacgatgaatgttttaatttgccagcagccgaaagaattagtctggaaacaacgcgagatacctattccgggtgacaatgaagcattaataaaaattaagtctgtcgggatttgcggtaccgatattcatgcctggggtggaaatcaaccattttttagttatccacgtgttttaggccatgaaatatgtggggagattgttgggctgggtaaaaatattgctgatcttaaaaatggtcagcaagttgctgtgatcccttatgttgcctgtcagcaatgcccggcgtgtaaaagcgggcgtaccaattgctgtgaaaaaatttcagtcattggcgtgcatcaggatggcggttttagtgagtatttgagcgtgccggtggcgaacattttgcccgcagacggtattgacccgcaggcggcagcattgattgaacctttcgctattagcgctcatgcggtgcgtcgcgcagccattgctcccggcgagcaggtgctggtggtcggggcggggccaatcggtctgggcgcggcggcaatcgctaaagccgatggcgcacaggtggtggtggcggataccagtccggcgcgccgtgaacatgtggcaacgcgtctggaattacctttactggacccgtcagccgaagattttgacgcgcagctacgggcgcagtttggtggttcgctggcgcagaaagtgatcgacgcgacaggtaatcaacatgcgatgaataacaccgtgaatttgattcgtcacggcggcacggtggtatttgtcggcctgtttaaaggtgagttgcagttctccgatccggaattccataaaaaagaaacgacgatgatgggcagccgcaacgccacgccggaagattttgctaaagtcggtcgactgatggcggaaggaaaaatcactgctgacatgatgttaacccatcgctatccgttcgccacgctggcagaaacctacgagcgcgatgtgattaacaatcgtgagttaattaaaggcgtaattactttctgataaggcgagattattaaagttgccatgcagcgtccggggaagtgttgggcgctgttttttttgtttcttaataatgtgttgtaagccgtagaaggcgtgtaggtcgcaccctatgcgacctacacatcagtcaggaattacccttcacgttctaccactttaatttccaccatgccgatcccgagcttacgcggcgagtgtccgaggatattcccttcgttggttgagacaggttccggcggcacaattaccagtgtgtcggcatcggttgggttatcgaaatgcagtgtggtggtggtcacttcattgcccagcacaagagtttgttcttcattgcctacgcgtaccggaataggacggctggcgttattgccgtatgctttggcggtaatcaccaggtcaaatttcttcggcagcggatgcttgtactcgatttttacttcatcgcccagctgcgcgttggaccagcggccccacgactccggacgggaaatcccgctaaactgtttcacctcttctggcgcaccggcgacgttaaagatgaaactgtcggctttgtagcgaatatcgttatcaacaatcttcagcgtatcgacattgcctttgtaacgcgccatgtcgatgaccgtatctttaaatgccgttttgccctgccatgttgttttgtcaacatgctgaacaatttgctgaccgccaagctgcccttgcgagacacaccagtcggtggaaagtgccagttccggagcccagagttgtgccatcttgtagcaacggtcaacccagacgaaattgtcgcgtggagcgaaatcggccagctggaaacgcagcggtgctgagtattcgctttccggcagcggttccacgcgtttgtctgaaacccgcaacagcagcggcaaacggaaatggctacccgagaaggcaatcatgtttttctgctggtcgatggtgaactctttcatctctttagggaatttccacaggcggatgatatctggcttccacgccaatgttttctctttgatattgaggaagatttccgacatcgactgcccggataaactgctacgaccaagtccgagatagttatcgccaccgagaatgtccagcaccgtcgcgccgttatccatcgtgttacgcttcactgccagcgtctcttgctgcggcttgtcgccacgaatgacaaaaaacaggttattgcgatcctgcttattgaggtatttccacgccgtgttgttcatcgctaaatggtcagaagagacgacgatgacggtatctttaaaccacggtgacgctttgattttgttgataaacgtcgcgatgttctcctggctgcaacttaccgcgctgaatgactgattcggtttaccgtcaaaatcatattttttgcggttacaggtacgagagataaaaccatccgggtgatgggtatcgactgtcagggtaaacagtgagaatcgctgacctgagcgggaaagctcttcaaactttttccacgcttcatcgagaacggtatcgtcgtagaatccccagtcgttgcgatagtgcgggtcggctaccacgcttttcagctcttctgagccgtataagtggtcgaagccatgcgacttcaggaacacatctttaccggcaaaacgcagattcgcgccctgcacgaaatagttctgataacccgagtttttcaggatatctcccagacagatgttctgcgggaagaagctggagacagaggcggaggcgttgccttcaaagggggcaaacagcggtatgccgcactgagaagccaccatgcccgcaatcgtgtaatctgttcccggcagctgctgcgtgtggctgaaatccaggccttcatttttcaacgcgcccagttcaggcgtgagatccgggaaagcctcgttatcaaaataggtccgctcgagactttcgccgtagatataaaccaggttgagtttcgggtcagggatagttttcgacggctctttataataagccgcaaagtccgggtcgccgtcgcgtgactgggatttcaccagttccgttatctgacgaaatgccgggctggcgtccaccgaacccagcgccagtaagagcgccagcaggctgtaaccaaaatggtgcggatgatggcgacgacggcgcaggatccagcccagcgcaccgaacaccgctgtcagccccagcacaatgccgatacccggcaaaatgtatttgctgacgccagcaccggtcaggctgttggttaaggtatagagaaccgcgtcgttaataccatcgccagtaaaatagtcgctggcaaacagggtgatatttaaaacgacaaatagccccagcaccgttaacgtggctgcaaaccaccaggtgttacgtcccgctttccatgcgtaaatcagcacagaggcgagaaaaagggcgaaagagagtagttctgacaacgggcgatcctcactaaaccgggccgtttagccaacgtttaagctttttgagaagcacaatgtaatggcgtcgccatattgctgcaattctagtgtcaaaaaaatgcgatgttgttaggaattagtttataaacagacttttttgattacggtcacttcccgtgtaacaggggtaaaaccgtccaggagcagggaaaagggcaggagagagccgcgtcagccgggtaacagctaaaacgcggcgtttcgcggttcaggaaatgaagttcagcccctgttttaacaccagatcgcaggctttggttttcaccttttctgccagcggagttgttccgatgttatccagattgagttgctgaccatctttggttttcagcaaaccctgaatgccgtccagatagttggtgtcttctttttgctcttcactgttcaggcccagcttttccagcacctggttcttgatgttttcggcatcggttaccgacgccagcttttgcttcgcgcagtattgcagaatgcctgcggcattgttcatgttatctgcgcttaaggcctggtttccgctgctaagcaagttagttaatgacgcgagcgaccaaccgccttcctgtgtcgtgctgttttggttgccaagttcgctggcggcgctggagagcgcatctttccaggacgcagcatgcaccccggtggaaattaatgcgctggcggcaatggcacagcacagaagatgtttaacagttttcatcatcattactcaaggtggaattgtgtcgcagtataccgccagaaacggggattaatactctttacctgttacccggctacggtagctatcccagttgaagatcacccacaaactgttacccaggcgcatacggtccatcacgcgttcgcccagcaacttggtcatctcttccatattactgttggtcagcatcccggttgggcgtttggaagaagagcggcgatcgacgatctggttgatgatcactttttcgtatttcgattcggtctgcacgccgatctcatcgatcaccagcagatcaacgttgctcagatcgttaagcagttgttcttcgctggtaccgctattcctgaaggtatctttcatcgccgacataatatcggccacggtgatgatcaatacggatttaccgcgtagcagcagctcgttgcagattgccgccgccagatggtttttgccggttcctggcttaccagaaaagatgaagctggcgatgttgccgtcaaactcttcgacatactggcgcgctttgcttaacgcattcatctgcccttcacactcaacgcgatagttctcaaaggaacagttctgatgcagtggacgaataccggagcggttaaaggtgcgctgcattttcatcgcccgattttcacgttcgagagcggcggagcggatcgctccttgttctttttgccaggccagtagttcttcacccgttttgaatgcgggtttgatatgggcaggcatcattttttgcaggcgttgcatcaggtcgccaacgtttttcatcgttaccctctgaatcctggtggaatttggctgtcaggttcgctgaccgtattcacatctcgtttcggcagtccgccgttgctggcacgaccgatttgcaggctgcgcgccagtttttgttgccactgcacatggtgaaagactttaccttccgcctgccagtaggcaatgaatgaggccagttcttcggtggtcaccggctctcttagcgccacgccccatagcgccgccaggcggataaaatcggcatcgggttgccagtccggatacatggcgaatttccccatgggtacagcaacgggagcggcttgcggttcctgatagagttgatcgtccagagcgacatcgcttcccggacgcgccagcttttcttccagcgccagcagttcagccaggcgtgcaggcgtgacggcataaaacgccggggcattgttagcaaatacggcaaccacaccgccttcagcttttgccagaacggtttggtgatcgtgtaccagggcgtcaataccaacgacgtccggggtcaaaactctggaagacatactgtttctcaaatatggaacgatgaacgagaagggagataacttttatagtaacacacggaggagaggaggctgtctctcatccgtgtgcttaagcgaggcaattttatacgcgagggcgcttgcggtacaaccataatccaggaatggaaagaccgatggataacgcaccaacaatcgatgaagctgtaagaaagttggttaacagggtaatcatcaacggttcgctgtaacctaactggctgatttttaccgccgaaatcattgcggtataagccgatatgcccgggaacatagggataacggccgccacggtaaacactttcggatgcgccagataccagcgcgaccattgaataccaatggtaccgaccagcatagaagccataaaggttgaccactcaatattcaacccgctggtcatcaagatcattcgggaaccatgacctatcgagccaagcagcgcacaccagcgtaacgcccgcacgggaacgttgaacaccatcgcaaagccgaccgcaggaatggcggcgaggatcatatcctgcgccaacgctaacagaaattcgatcacacccatccgcgtagcccccaaatcgtcagtgccatcactacgccgacgcaggtagccagtgtcagcagactggcgatcgcccagcgtgccagtccggtattgatgtggcctttaaacatatcggcgacggcattaatcaacggaaagcccggcactagcagcagaacgctggcggccatcgcaatggtgggggtattgctgaaagtggggagttgcaaaagcaatccggaaatggtggtggcggcgaaagcggtaaggcaaaagttgatctgtggatgaagatgacgttgtgccagcagctggcggatatacatcgcggtcgtactggcaaagaaggtgatgacggcaccatcccagccaccgttattgagtttacagaaacaggcgcaagaaaggccaaccattaaggctaccagccatcttgggtaacgtaatggctgaatttggctaaatcgtttctctacgcctttgtaatccagcagatgatgctccgcaagaatcacaatgtgctggacttcagtcaccacatgcatattaatgccgcgatcgtgatttttacgtgtcgatgtcaggcattgcccatctttaatagttgtcagcactatggcgttcgaagagatagaactttcgacgctgtccattcccagtgcccgacccagtcgtgaggaaagctcatcaaccaacgcgctttccgcaccatgttgcaaaagaaataatccacactggatacaaagccgtgttacggctcgctgttgctcagtttgcataactcgccctttgtcatagacgtgctgcgtattgttcagataatgagaatccatttgtatcatgaagcacggttgttttgcggtaggttaagatcaaaattgcgctgattaatcctggttatcgggagaagctcggtgataaaaagcgaattatctctcgccgcaaacaaactatcacatgaatattatcatcataatgaatttattgtttggcctttacgaatcaggataatagataaccgggcacgttttttaatgttaacaagctaaaaccatcagatttcattgaataaatattggttgtgtgattttgcattctgcgggaagggatatcatttaattataaattaaatgaatgtgatttctgtttttcattaagtattcctaacaacttaatgtagatattttaaatgtctccaggctatttcaccaggttatcatttgatgctaaccttctgacacatgcagtggagttgttgtgcagcaggagtatgctgatatgaaagtgaatgctaaggataatttattcgcttaatctattaatttgctggaaacatttaaggaatgaatatcctgaataaaccatcataatttttagacagtggatgtggaggaaatatgttgccaggatgctgcaaaaatggaattgttatcagtaaaatacctgttatgcaagcagggttaaaagaggtcatgaggactcacttccctgaatatgaaataatatccagcgcctctgcggaggaccttaccttattacaattacgtcgttccggattagtcattgctgatttagccggtgaaagtgaagatccacgttctgtttgtgaacattattattctttaatctcacaatatcgggaaattcactgggttttcatggtgtcacgctcctggtattcccaggcagtagaactgctcatgtgccctacggcgacgttattgtctgatgttgaacccattgagaatctggtcaagaccgtacgttccggcaatacgcacgcagagcgtatcagcgccatgctgacctccccggcaatgactgaaactcatgattttagctatcgctccgtcattctcactctttcagagcgcaaggtactgcggctattaggtaaaggatggggcatcaaccagatagcttcattgcttaagaaaagtaataaaactatcagcgcccaaaaaaacagtgcgatgcgtcgactggcaattcacagcaacgctgaaatgtatgcatggataaatagcgcgcagggtgcaagagaacttaacttgccttctgtttatggagatgccgcagaatggaacacagccgaattaagaagagaaatgtcgcactcatagaaaaatgcgtcatgagtagtatcggtattgagagtttattcagaaagtttgcgggtaacccttataagctccatacctataccagtcaggagtcatttcaggatgccatgtcgcggatctcgtttgcggcggtcattttttctttttctgccatgagaagtgagcgcagagagggattatcttgcctgactgaactggcgattaagtttccgcgtacccggcgtttagttattgcggatgatgatattgaagctcggctgattggttcattgtcgccatcaccgctggacggtgtattaagtaaagcgtcaacgctggagatttttcatcaggaactctttttgtcattaaatggtgtacgtcaggcgaccgaccgactgaacaatcagtggtacattaaccaaagccggacgttaagcccgacggagagagaaatattgcgctttatgtcgcgtggctactcaatgacacaaattgccgagcagcttaaacgcaatatcaaaacgatccgtgcacataaatttaatgtgatgtcgaaactgggcgtcagttctgacgcagggttgttggaggccgcagatattctgttatgtatgcggcattgcgaaacaagtaatgtgttgcatccctattaatccgcatgatgccgggtttacttccccggcagtgctttcatttcagcgtacaatcgccacattgctgcacatccggtaagcgataacgctggcagcaagtgcggcgcaccagcaggccgtcgcgcagtaccacggtacgccagagtggattatcttcaccgttcgtgagcgttttctcaaaaaagagggcatggcgcagcgattcaacagtagcctcgccgagcagttgcttcatctcagtgagataccagttgatcaaataaccggtattactccagataagtttgccgttgatctctccggtcgcttctagtgcttgcacaaccggaaccagcgcctggctgattaacgtttccattcgatgctgcggcgaatgtggtgttgcgtttttatcttcacacacatcgacccagaaacaggcgacgcgtccggtttcgtgaaactcagcatggaaatgttccggcgacacatctaatgccttttcctgcgtcagtagcgccagcattaatggtggcaccatcaggccgatataccattgtgcccatagtgagatcagcggtttgttctcgcggatcatcatcggttggttgcgatagatatgatcggaatagaccgccagcagagaacttagcacattcggtgatgaccattgcgccagcgtcatggcgttaagtggggcaggttcatccaggcggataaactccagcaaatgttcacgatgttttgcgatcgtcgcccgcacggcttgcgcaagcgtgggatcctgcggctggagatgcgttcgccagatgacatcttcatagagcggtgcggaacgataggccataatcgggatagtaatctaaatgataatgattgctaatcatagcgataggtttacccgatagcaagggatttatctggcttgcaaatgataaaaattatcatatgatattggttatcattatcaatgaaagagatgaaatcatgttgcaacgtacgctgggcagtggctggggagtgttgctgccgggattgctgattgcagggctgatgtatgcggatttatcgtcagatcagtggcggattgtcattctgatgggattagtattgacgccgatgatgctgtatcacaaacagttgcggcattacattttgctaccatcgtgcctggcacttattgctggcatcatgctgatgataatgaatttgaatcagggatgaaaaatcaaggaagaaacaagaaaggaagtaaagataattggtgcgaggggggggacttgaacccccacgtccgtaaggacactaacacctgaagctagcgcgtctaccaattccgccaccttcgcacagtcatcttactttttttgatatcgcctcgtttggtgcgaggggggggacttgaacccccacgtccgtaagaacactaacacctgaagctagcgcgtctaccaattccgccaccttcgcccagtgcgagcaatatcaacgtggtttttggtgcgaggggggggacttgaacccccacgtccgtaaggacactaacacctgaagctagcgcgtctaccaattccgccaccttcgcataccatcaattcttaaaaagaattgctaccacggaggcgcattctagtggttttcagcttttcgtcaatagttaattatcgacagaggtgtaattgctggaaaaatgtccatcaggaaactagcgtgcaggtttggtatgcatgcgggggcagatgccagatgcgacgctggcgcgtcttatctggcctacgaagggctaacgtgcaggttttgtaggtcggataaggcgttcacgccgcatccgacacggtattcggcgagataattaacctttcttcgcctggcgggtcataatggcgcgatacaccttgaagcgccctgtttgcgcgatcacttcgtggaagccaaatgtctcatccagcacgtccggataaggcaggaaggcgttcgctacaattcgcagctcgccgccgctattaagatgacgcaccgcaccgcgaatcagcgtttgcgccgcatccaggctggtttgcatcccatcgtggaacggcgggttggagatgatcatatcaaaacgacctttcacctcggaaaagacgttgctggcaaagacttcaccttcaacaccgttggccgcaagtgttgcgcggctggcttctaccgccggggcagagacatcgcacaaggtgagacgaattttcggcgaatggcgcgcaaaggcaactgaaagcacgcccgcgccacagccgacatccagcactttacctttcgtgtgcggagttaacgtcgagagcagcaactggctaccgacatccagaccgtcgcggctaaacacgccaggcagcgttttgaccgtcaggccatcgacgctgtattcgccccagaatttctccgcatcaaataccggctgtttttccagacgaccaaaatagaggccacagcgacgagcgctgtcgactttattcaacggcgcataatctgccagcatctgctcggcgctgcgcacgccgctgcggttctcgccaacgacaaaaatatctgtccccactggcagcagagaaagtaaattcatcaactggaactgggcttccggtttgttcttcggccagtagtaaatcagcgtatcgcaatctgcgacgtcatccgccgtggcgaccagactgaaacgggcgttatcccccatctggcggcttaatacctgccagtggtggaattgctgggtatgagcacggctggccgcggtatctaaacgcgcgggcaggtcatcctgtaagtctccggcaaacagaatacggctttgttcgaaatcatcactgtgacgcagcaagacttcacttgccggggtaaatgcagacatggaatgctcctcaattgatactggcggcgattatagccatatgttggcgcggtatcgacgaatttgctatatttgcgcccctgacaacaggagcgattcgctatgacatcccgacgagactggcagttacagcaactgggcattacccagtggtcgctgcgtcgccctggcgcgttgcagggggagattgccattgcgatcccggcacacgtccgtctggtgatggtggcaaacgatcttcccgccctgactgatcctttagtgagcgatgttctgcgcgcattaaccgtcagccccgaccaggtgctgcaactgacgccagaaaaaatcgcgatgctgccgcaaggcagtcactgcaacagttggcggttgggtactgacgaaccgctatcactggaaggcgctcaggtggcatcaccggcgctcaccgatttacgggcaaacccaacggcacgcgccgcgttatggcaacaaatttgcacatatgaacacgatttcttccctcgaaacgactgatttaccggcggcttaccacattgaacaacgcgcccacgcctttccgtggagtgaaaaaacgtttgccagcaaccagggcgagcgttatctcaactttcagttaacgcaaaacggcaaaatggcggcgtttgcgattacgcaagtggtgctggatgaagctacattgttcaatattgcggtcgatcctgactatcagcgtcagggattgggaagggcgctgctggaacatctgatcgacgaactggaaaaacgcggcgtggcgacactatggctggaagtccgtgcttcaaacgctgccgccattgccctgtacgaaagtttaggctttaacgaggcgacgattcgccgcaattactaccccaccacggacggtcgcgaagacgccatcatcatggcgttgccaatcagtatgtaatacaaggtggaataatgaagtgggactggattttctttgatgccgatgaaacgctgtttacctttgactcattcaccggcctgcagcggatgtttcttgattacagcgtcacctttaccgctgaagattttcaggactatcaggccgttaacaagccactgtgggtggattatcaaaacggcgcgatcacttcattacagcttcagcacgggcggtttgagagctgggccgaacggctgaacgtcgagccaggtaaactcaacgaagcctttattaatgcgatggcggaaatctgcacgccgctgccgggcgcggtttctctgcttaacgccattcgtggcaacgccaaaatcggcatcatcaccaacggctttagtgccttgcaacaggtgcgtctggaacgcacgggcctgcgtgattacttcgatttgctggtgatttccgaagaagttggcgttgccaaaccgaataagaaaattttcgattatgcgctggaacaggcgggcaatcctgaccgttcacgcgtgctgatggttggcgacactgccgagtccgatattctcggtggcatcaacgccgggcttgcgacctgctggctgaatgcacaccatcgcgagcaaccagaaggcatcgcgcccacctggaccgtttcttcgttgcacgaactggagcagctcctgtgtaaacactgattgcctcccccccgttgatgggtaaaatagccgcaatttttcgttttcaacaagcgcggcgcgatgccgcttactcaagaagaaagaattatgacgttgtctccttatttgcaagaggtggcgaagcgccgcacttttgccattatttctcacccggacgccggtaagactaccatcaccgagaaggtgctgctgttcggacaggccattcagaccgccggtacagtaaaaggccgtggttccaaccagcacgctaagtcggactggatggagatggaaaagcagcgtgggatctccattactacgtctgtgatgcagtttccgtatcacgattgcctggttaacctgctcgacaccccggggcacgaagacttctcggaagatacctatcgtaccctgacggcggtggactgctgcctgatggttatcgacgccgcaaaaggtgttgaagatcgtacccgtaagctgatggaagttacccgtctgcgcgacacgccgatcctcacctttatgaacaaacttgaccgtgatatccgcgacccgatggagctgctcgatgaagttgagaacgagctgaaaatcggctgtgcgccgatcacctggccgattggctgcggcaagctgtttaaaggcgtttaccacctttataaagacgaaacctatctctatcagagcggtaaaggccacaccattcaggaagtccgcattgttaaagggctgaataacccggatctcgatgctgcggttggtgaagatctggcacagcagctgcgtgacgaactggaactggtgaaaggcgcgtctaacgagttcgacaaagagctgttccttgcgggcgaaatcactccggtattcttcggtactgcgctgggtaacttcggcgtcgatcatatgttggatggcctggtggagtgggcacctgcgccgatgccgcgtcagactgatacccgtaccgtagaagcgagcgaagataaatttaccggcttcgtatttaaaattcaggccaacatggacccgaaacaccgcgaccgcgtggcgtttatgcgtgtggtgtccggtaaatatgaaaaaggcatgaaactgcgccaggtgcgcactgcgaaagatgtggtgatctccgacgcgctgacctttatggcgggtgaccgttcgcacgttgaagaagcgtatccgggcgatatcctcggcctgcacaaccacggcaccattcagatcggcgacacctttacccagggtgagatgatgaagttcaccggtattccgaacttcgcaccagaactgttccgtcgtatccgcctgaaagatccgctgaagcaaaaacagctgctcaaagggctggtacagctttccgaagagggcgcggtgcaggtgttccgtccaatctccaacaacgatctgatcgttggtgcagttggtgtgctgcagtttgatgtggtggtagcgcgcctgaagagcgaatacaacgttgaagcagtgtatgagtcagtcaacgttgccactgcccgctgggtagaatgtgcagacgcgaagaaattcgaagagttcaagcgtaagaacgaaagccaactggcgcttgatggcggcgataacctcgcttacatcgctaccagcatggtcaacctgcgcctggcacaggaacgttatccggacgttcagttccaccagacccgcgagcattaattcttgcctccagggcgcggtagccgctgcgccctgtcaatttcccttccttattagccgcttacggaatgttcttaaaacattcacttttgcttatgttttcgctgatatcccgagcggtttcaaaattgtgatctatatttaacaaagtgatgacatttctgacggcgttaaataccgttcaatgcgtagatatcagtatctaaagccgtcgattgtcattctaccgatattaataactgattcagaggctgtaatggtcgttattcatcactcatcgcttttgtgatggcgaccattgacttctgtagagggtgaagtctctccctattcagcaatgcaacctcgtgttgccaggctcaaattacgagcaaacatacaggaataaatcgatgactatgacaagactgaagatttcgaaaactctgctggctgtaatgttgacctctgccgtcgcgaccggctctgcctacgcggaaaacaacgcgcagactaccaatgaaagcgcagggcaaaaagtcgatagctctatgaataaagtcggtaatttcatggatgacagcgccatcaccgcgaaagtgaaggcggccctggtggatcatgacaacatcaagagcaccgatatctctgtaaaaaccgatcaaaaagtcgtgaccctgagcggtttcgttgaaagccaggcccaggccgaagaggcagtgaaagtggcgaaaggcgttgaaggggtgacctctgtcagcgacaaactgcacgttcgcgacgctaaagaaggctcggtgaagggctacgcgggtgacaccgccaccaccagtgaaatcaaagccaaactgctggcggacgatatcgtcccttcccgtcatgtgaaagttgaaaccaccgacggcgtggttcagctctccggtaccgtcgattctcaggcacaaagtgaccgtgctgaaagtatcgccaaagcggtagatggtgtgaaaagcgttaaaaatgatctgaaaactaagtaattcgtcgtaattcgtcctcccgaactttgtcgggaggcgcgatgtgcaccacactaaaaatatcgcattgagtgattttcacgctcatatcaagcggtgacattaactatggtaaaggagacgcttatgtttcgttggggcatcatatttctggttatcgcgttaatcgccgccgcacttgggtttggtggtctggccggtaccgctgcaggcgcagctaaaattgtctttgtcgtcgggattattctgttcctggtgagtttgttcatgggccgaaaacgaccctagatttcagaccattaagaaaattttatccaaagccagtccagcggactggcttttgcggttttagcgaataataaattgcgttactttgtcattctttcacaacaaaaacaggaaggcagaggtggggcagcgaatacctgtaacgcttggtaatattgcgccgttgtcgctaaggccgttccagcctggacgaatagctctggtgtgcgaaggcggcggacagcgtggaattttcacggctggcgtgctggatgagtttatgcgcgcgcagtttaatcctttcgatctttatctcggcacatctgccggggcgcagaacctctcggcgtttatctgcaatcagcccggttacgcgcgcaaagtcatcatgcgctataccacaaaacgcgaatttttcgatccattgcgctttgtccgtggaggaaatcttatcgatctcgactggctggtggaggccactgcaagccagatgccgttgcaaatggataccgccgcgcggttgtttgacagcggcaaatcgttttatatgtgcgcctgtcgtcaggatgactacgcgccgaattactttttaccaaccaaacaaaactggctggatgtgattcgcgcctccagtgcgatacctggcttttatcgtagcggagtgtcgctggaaggcattaactacctggatggcgggatcagtgatgcgattccggttaaagaggcggcaaggcagggcgctaaaacgttggtcgtcattcgcactgtgccgtcacaaatgtactacacgccgcagtggttcaaacgcatggaacgctggctgggtgacagtagcctgcagccgctggtcaatctggtgcagcatcatgaaaccagctatcgtgacattcagcaatttattgagaaaccaccgggcaagctgcggatattcgaaatttatccgccgaagccattacatagtatcgcgcttggcagtcggattccggcgctgcgtgaagactataaacttgggcgtttatgcggtcgttatttcctcgccacggttggcaagctattaactgaaaaagcgccgcttacccgccatctggtgccagtggtgacgccggaatcgattgtcattccgcctgcgccagtcgccaacgatacgctggttgccgaagtgagcgacgctccgcaggcgaacgacccgacatttaacaatgaggatctggcttgatttgccgttttatcgacacccactgccattttgatttcccgccgtttagtggcgatgaagaggccagcctgcaacgcgcggcacaagcgggcgtaggcaagatcattgttccggcaacagaggcggaaaattttgcccgtgtgttggcattagcggaaaattatcaaccgctgtatgccgcattgggcttgcatcctggtatgttggaaaaacatagcgatgtgtctcttgagcagctacagcaggcgctggaaaggcgtccggcgaaggtggtggcggtgggggagatcggtctggatctctttggcgacgatccgcaatttgagaggcagcagtggttactcgacgaacaactgaaactggcgaaacgctacgatctgccggtgatcctgcattcacggcgcacgcacgacaaactggcgatgcatcttaaacgccacgatttaccgcgcactggcgtggttcacggtttttccggcagcctgcaacaggccgaacggtttgtacagctgggctacaaaattggcgtaggcggtactatcacctatccacgcgccagtaaaacccgcgatgtcatcgcaaaattaccgctggcatcgttattgctggaaaccgacgcgccggatatgccgctcaacggttttcaggggcagcctaaccgcccggagcaggctgcccgtgtgttcgccgtgctttgcgagttgcgccgggaaccggcggatgagattgcgcaagcgttgcttaataacacgtatacgttgtttaacgtgccgtaggccggataaggcgttcacgccgcatccggcagttggcgcacaatgcctgatgcgacgcttaacgcgtcttatcatgcctacaggtttgtgccgaaccgtaggccggataaggcgttcacgccgcatccggcagttggcgcacaatgcctgatgcgacgcttgtcgcgtcttatcatgcctacaagtctgtgccgaaccgtaggccggataaggcgttcacgccgcatccggcagtcggcgcataatgcctgatgcgacgcttgtcgcgtcttatcatgcctacaggtttgtgccgaaccgtaggccggataaggcgttcgcgccgcatccggcagttggcgcacaatgcctgatgcgacgcttgacgcgtcttatcaggcctacaagtctgtgccgaaccgtaggccgtatccggcatgtcacaaatagagcgccggaaatatcaaccggctcaccccgcgcacctttaacgcatcagccaacggctcaacgtcttccggcgtggcgctcgcccagctttgcgcctcgccatacacgccgtgggcatgaaacgcgttcaggcgtaccggaacatcgccgagtcccttgataaacgccgccagttcttcgatgtgttgcaaataatccacctggccagggatcaccagcaaacgcagttccgccagcttgccgcgctctgccagcaaatagatgctgcgcttaatctgctgattatcgcgtccggtgagttgttgatgacattcgctcccccacgctttgagatcgagcattgcgccgtcgcacaccgggagcaatttttcccagccggtttcgctcaacatgccgttactgtccaccagacaggtgagatggcgcagttgcggatcgtttttgatagcagtaaacagcgccaccacaaacggcagctgggtcgtggcttcaccgccactcaccgttatcccttcgataaacagcactgctttgcggacatggctaagcacttcgtccacgctcatggattgcgccatgggcgtggcatgttgcggacacctcttcaggcaggtatcacactgctcgcaaaccacagcgttccacaccactttgccgtcaacaatctgcaacgcctgatgcggacactgtggcacgcactccccacagtcattgcaacgtcccatcgtccacggattgtgacagtttttgcagcgcagattgcagccctgcaaaaacagagccagacgactgcctggcccgtcaacgcaggagaaggggataatcttactgactaaagcgcatctgctgttcatggcttatcacgcgcggctggcgttccagaatacgagtgttgcgtgcggcttcttcgcccagccaggtggtgttggtgcgtgaaccttcggcgcgatatttttctaaatccgacaaacgcaccatataaccggtaacgcgaaccagatcgttaccgctgacattggcggtaaattcacgcattccggctttaaaggcaccgaggcaaagctgtaccagtgcctgcgggttacgtttgatggtttcgtcgagcgtcagaatgtcgctgatgccggaataataataagcatgatgcggggcgacagtttgcagatgggtgatcggatctggctcatcgccatacggcaaacgcgcgcccggcgtggtgccgatatcggaactgatccccgactgtgcgtgtaacatggcgcgtttttgccagccatatttcacgggggtattggcgacaaactccgccagttgcgcgctgatgcgataacctacttcatttgcggcggcttctttaccgtagcgcgcggcaatcccttctttttcacacagcaagttaaccgcttccgccagcccatacatgccaaacattggcacaaaacgttcagggttaatcagcccttctttcaccaggaagctattctcaaagaagtgtgattgttgatagaggaattcacaccgcgcatcgatgatggcgatctgctgctggcagtagtgcggtagagtgcgcgtaaagaagtcatccagcgattcgctgcgctcggcaatggctttcaggttaaggcgtaccagcgtgctgccaccacccgccagcggcagtgagttgtaacagctcacaatcccgtagcccccttttgtgaaaattttatcatgcaccggaccgttggcgatgtgcggtttgctacattcacagatgttcttcgccacttccagcagcaggtcatcaggggtgatttcaggatcgtagataaaggtcaggttcggtgaaacctgcttcaactctgcatctgcacgtaagatcgcgcgggtaatgggcgaatcagacgggccgatattggcgtgcataaaggcgtctggcagggttctgtcgaggtaacgccagaaacgttttattcgaacatcgatctcgtcttgtgttagaattctaacatacggttgcaacaacgcatccagttgccccaggtagaccggcatcgatgtgaccgacggtacgtggtggtaaagaatggtcagcagagagagtgcgtcatcaagatctttcgcgccttccagctccagccattcggaaccgttcgccagaaaacgggcgtaatcgggtaagacatagcgcggtttgtacggcgcatgaccttcaaacatatcgcagattacaccttcatccagcgcgcggcgggcttcggcaggaagctgtgggtaaggcagattgttttctgcttccagtgccagaaaatggcgcttctgctccgggctaagcactgggctggtgacaatttgctggcaacgttgttgcagtgcattttcatgagaagtgggcatcttcttttccttttatgccgaaggtgatgcgccattgtaagaagtttcgtgatgttcactttgatcctgatgcgtttgccaccactgacgcattcatttgaaagtgaattatttgaaccagatcgcattacagtgatgcaaacttgtaagtagatttccttaattgtgatgtgtatcgaagtgtgttgcggagtagatgttagaatactaacaaactcgcaaggtgaattttattggcgacaagccaggagaatgaaatgactgatctgaaagcaagcagcctgcgtgcactgaaattgatggacctgaccaccctgaatgacgacgacaccgacgagaaagtgatcgccctgtgtcatcaggccaaaactccggtcggcaataccgccgctatctgtatctatcctcgctttatcccgattgctcgcaaaactctgaaagagcagggcaccccggaaatccgtatcgctacggtaaccaacttcccacacggtaacgacgacatcgacatcgcgctggcagaaacccgtgcggcaatcgcctacggtgctgatgaagttgacgttgtgttcccgtaccgcgcgctgatggcgggtaacgagcaggttggttttgacctggtgaaagcctgtaaagaggcttgcgcggcagcgaatgtactgctgaaagtgatcatcgaaaccggcgaactgaaagacgaagcgctgatccgtaaagcgtctgaaatctccatcaaagcgggtgcggacttcatcaaaacctctaccggtaaagtggctgtgaacgcgacgccggaaagcgcgcgcatcatgatggaagtgatccgtgatatgggcgtagaaaaaaccgttggtttcaaaccggcgggcggcgtgcgtactgcggaagatgcgcagaaatatctcgccattgcagatgaactgttcggtgctgactgggcagatgcgcgtcactaccgctttggcgcttccagcctgctggcaagcctgctgaaagcgctgggtcacggcgacggtaagagcgccagcagctactaagtaagatgctttacgcctgatgcgctgcgcttatcaggcctacgagacgtatctacccgtaggccggataaggcgtagacgcatccggcaaaagccgcctcatactcttttcctcgggaggttaccttgtttctcgcacaagaaattattcgtaaaaaacgtgatggtcatgcgctgagcgatgaagaaattcgtttctttatcaacggtattcgcgacaacactatctccgaagggcagattgccgccctcgcgatgaccattttcttccacgatatgacaatgcctgagcgtgtctcgctgaccatggcgatgcgagattcaggaaccgttctcgactggaaaagcctgcatctgaatggcccgattgttgataaacactccaccggtggcgtcggcgatgtgacttcgctgatgttggggccgatggtcgcagcctgcggcggctatattccgatgatctctggtcgcggcctcggtcatactggcggtacgctcgacaaactggaatccatccctggcttcgacattttcccggatgacaaccgtttccgcgaaattattaaagacgtcggcgtggcgattatcggtcagaccagttcactggctccggctgataaacgtttctacgcgacccgtgatattaccgcaaccgtggactccatcccgctgatcaccgcctctattctggcgaagaaacttgcggaaggtctggacgcgctggtgatggacgtgaaagtgggtagcggcgcgtttatgccgacctacgaactctctgaagcccttgccgaagcgattgttggcgtggctaacggcgctggcgtgcgcaccaccgcgctgctcaccgacatgaatcaggtactggcctccagtgcaggtaacgcggttgaagttcgtgaagcggtgcagttcctgacgggtgaatatcgtaacccgcgtctgtttgatgtcacgatggcgctgtgcgtggagatgctgatctccggcaaactggcgaaagatgacgccgaagcgcgcgcgaaattgcaggcggtgctggacaacggtaaagcggcagaagtctttggtcgtatggtagcggcacaaaaaggcccgaccgacttcgttgagaactacgcgaagtatctgccgacagcgatgctgacgaaagcagtctatgctgataccgaaggttttgtcagtgaaatggatacccgcgcgctggggatggcagtggttgcaatgggcggcggacgccgtcaggcatctgacaccatcgattacagcgtcggctttactgatatggcgcgtctgggcgaccaggtagacggtcagcgtccgctggcggttatccacgcgaaagacgaaaacaactggcaggaagcggcgaaagcggtgaaagcggcaattaaacttgccgataaagcaccggaaagcacaccaactgtctatcgccgtatcagcgaataacggtatactgatctgatcatttaaatttgaagcactgagtacggagaacatatgaaacgtgcatttattatggtgctggactcattcggcatcggcgctacagaagatgcagaacgctttggtgacgtcggggctgacaccctgggtcatatcgcagaagcttgtgccaaaggcgaagctgataacggtcgtaaaggcccgctcaatctgccaaatctgacccgtctggggctggcgaaagcacacgaaggttctaccggtttcattccggcgggaatggacggcaacgctgaagttatcggcgcgtacgcatgggcgcacgaaatgtcatccggtaaagataccccgtctggtcactgggaaattgccggtgtcccggttctgtttgagtggggatatttctccgatcacgaaaacagcttcccgcaagagctgctggataaactggtcgaacgcgctaatctgccgggttacctcggtaactgccactcttccggtacggtcattctggatcaactgggcgaagagcacatgaaaaccggcaagccgattttctatacctccgctgactccgtgttccagattgcctgccatgaagaaactttcggtctggataaactctacgaactgtgcgaaatcgcccgtgaagagctgaccaacggcggctacaatatcggtcgtgttatcgctcgtccgtttatcggcgacaaagccggtaacttccagcgtaccggtaaccgtcacgacctggctgttgagccgccagcaccgaccgtgctgcagaaactggttgatgaaaaacacggccaggtggtttctgtcggtaaaattgcggacatctacgccaactgcggtatcaccaaaaaagtgaaagcgactggcctggacgcgctgtttgacgccaccatcaaagagatgaaagaagcgggtgataacaccatcgtcttcaccaacttcgttgacttcgactcttcctggggccaccgtcgcgacgtcgccggttatgccgcgggtctggaactgttcgaccgccgtctgccggagctgatgtctctgctgcgcgatgacgacatcctgatcctcaccgctgaccacggttgcgatccgacctggaccggtactgaccacacgcgtgaacacattccggtactggtatatggcccgaaagtaaaaccgggctcactgggtcatcgtgaaaccttcgcggatatcggccagactctggcaaaatattttggtacttctgatatggaatatggcaaagccatgttctgatggatttgggcggagcgttgactccgcctttgttatgtcacaaaaaggataaaacaatggctaccccacacattaatgcagaaatgggcgatttcgctgacgtagttttgatgccaggcgacccgctgcgtgcgaagtatattgctgaaactttccttgaagatgcccgtgaagtgaacaacgttcgcggtatgctgggcttcaccggtacttacaaaggccgcaaaatttccgtaatgggtcacggtatgggtatcccgtcctgctccatctacaccaaagaactgatcaccgatttcggcgtgaagaaaattatccgcgtgggttcctgtggcgcagttctgccgcacgtaaaactgcgcgacgtcgttatcggtatgggtgcctgcaccgattccaaagttaaccgcatccgttttaaagaccatgactttgccgctatcgctgacttcgacatggtgcgtaacgcagtagatgcagctaaagcactgggtattgatgctcgcgtgggtaacctgttctccgctgacctgttctactctccggacggcgaaatgttcgacgtgatggaaaaatacggcattctcggcgtggaaatggaagcggctggtatctacggcgtcgctgcagaatttggcgcgaaagccctgaccatctgcaccgtatctgaccacatccgcactcacgagcagaccactgccgctgagcgtcagactaccttcaacgacatgatcaaaatcgcactggaatccgttctgctgggcgataaagagtaattgtgtttcgctgcaaggcgattgccttgtgaagccggagcgggagactgctccggctttttagtatctattcatttttctctccagcttgaatattttcgctatacttttcagtgaaatgtgttaataaatctattcaagtatctattcacgaatctattcattaatgagcgagctgactgatcttttactgcaagggccgcgttctgccccggaattgcgccagcgtctggcaatcagtcaggcgacgttctcacgccttgttgccagagaagatcgggtgattcgctttggtaaagcacgggcaacgcgatatgcactgctgcgtccttatcgcggaattgagcgtattcccgtctggcgggtggacgataccggaaaggcgcataaattcgccgacatccggttgtgctggccgcagggaagttgtctggtaacaggcgcagatggcgacgaacagtggtttgatggtttgccctggtatttgaccgatctccgaccgcagggctttttagggcgcgcgtggggcaggaagttagccgcgcaactgaatctgactgatgatatacgtctctggcaggaagaagatgtgctctacgccctgaccgtatttaacggtgaatatactggcggttggttggtcggggaggggaattatcagcgatggattactgcacaacaccctgcggaaattcctctggatcaaaaactcacccattacgaacagctggcaagtgatgcactggcaggagaaattgtgggttcttctgcgggcggcgagcagccaaaatttacctactatgcacaaacgccgtcaggcaataaacatgtgttggtgaaattcaccgtaccacagcaaaccgcggtcagccaacgttggggtgacctgctaattgctgaatctattgccgcgcaaatcctgcgtgacggtgggatccacgccatcgagtcaacggtgcttgtaacaagtaacaggcaggtattcctcgaagcggaacgctttgactgcaaaggtaacgatggtcgcttgcctattgtgtcgctggaggcggtgcagagtgagtttatctcttctccgggatcgtggccgcaggcaatgcgccgtttgtgtgagcaacaacttgtcactcaccagagcgtggcgcaaacagaagtgatctgggcatttgggcgacttatcgccaacagcgatatgcacgcaggtaatttatcgttttatttatctgaaccgccatttgcgctgacgcccgtctacgacatgctgccgatggtctatgcaccaaacagcgctggaatgctgcgtgatgctgccattgaggtgaagtttgatcttaacgtcagtaaaagcgcttggttaacggcgatcccgctggcgcagcagttctggcaaacggtcgccagagatccgcgtatcagcgaggcgtttcgccacattgcgcaagaaatgccggaaaaaatccggcaaatcgaagagaaagttgcccgcatgggcgggtaactaccttacagcccccgccatccatgccgataactcccgtagctctttttcctgttccgggaagtcaaccaacagcgcttcgcactcctgttgcagcatatctgcgcggtacaggcagccttgcagtcgtccggcgagggcttccagcggcgcggggttgaggctgtcggtaaacacctgggcgcgggtgatatggcctttttcaacgtcgaaatgcagttccacgccgccccaggtaaagcgttcatccagcagatgcgagaatgccggagcctgaccgaagttccattcccagctactctggcgggcaaaggtttcggcgaagtttggcaagtctggcgttttgttcggggagatgatttccgcttccacgcgctcgccataatgggcgaaaaaggcctcggttatggcctcgcaaacctgctcatgggtgatccccggcaacagctcggtgaggttggtcacgcgggaacgtaccgacgtaatgcctttcgccgccagtttctttttatccggattgagatagtttgccaggcggctgaggtcggcattgagtagcaaggtgccgtggtggaagccgcgatctttggtttcgcgataggccgagcctgagactttgcggtcgccttcgacggttttcaccaccagatcgttacgtccggacgcttcggcgctgacgccgagcgcgttcagcgcattgagcacaatcgacgtggagatagttttatcgtactccggcttgccagccataaaggtaaagcaggtattgccgagatcgtggaacaccgcgccgccaccgctactgcgccgcgccaggcggacgttatcttcttccatccgccgggtattacactctttccacgggttctgcgcgcgaccaattactaccgtgtcggcattgcgccagagaaacagaacgcgctgcgtggcgggcatttggcgaaaaatacactcttccaccgccaggttaaaccacgggtcgtaagagtcagagatgagcaggcgtaatgtggacataacgatttcctttcttgtagtaatgggtcactcttttttctcgctttcttcctcttccggcaccggtttgctggcggttaacaggaagggcgattgctgccagcgggtgcgtttaccctgtagcagcgtgcgggtcagcactacaccgattgccagtgagagcagcaacatcaggcgtaaaatgttagtggtgttatccacctgttgggcttcggtggcgagcgtatgggtgtcgagtgtcaggcgcagatagccgagcggtccgtttttacccgcaattggctcgacaatctgctggttaaaatagccgcctgcttttttaccgtcgagcgccagccggtcgcgcacttcgacgctttcgccagaacgtgcgataagatcgccttgttcgtcatacacacccgcgtcgaggatacggctttcatccgttaactgatcgaggatcgcctgaatgcgtttttcatccggtgagtcggtacgcatcagcggtgcaacgttcagcgtcacctgacgcgccagggtgcgggccagttcttccagctgtggattacgctgtcgctggtggttttgactaaaccatgacgctccctgcatcagcgccactaacaaggcaagacagaacaggacaatcactgcccgatgcagccggaatttcagttttgtgcgagccatcttccaccctttgaaaatttgagacttaatgttgccagaagcaatggatacaaggtagcctcatgcgttattttccctgcttcgaacgattttacaggagccttaatgcctaacattacctggtgcgacctgcctgaagatgtctctttatggccgggtctgcctctttcattaagtggtgatgaagtgatgccactggattaccacgcaggtcgtagcggctggctgctgtatggtcgtgggctggataaacaacgtctgacccaataccagagcaaactgggtgcggcgatggtgattgttgccgcctggtgcgtggaagattatcaggtgattcgtctggcaggttcactcaccgcacgggctacacgcctggcccacgaagcgcagctggatgtcgccccgctggggaaaatcccgcacctgcgcacgccgggtttgctggtgatggatatggactccaccgccatccagattgaatgtattgatgaaattgccaaactggccggaacgggcgagatggtggcggaagtaaccgaacgggcgatgcgcggcgaactcgattttaccgccagcctgcgcagccgtgtggcgacgctgaaaggcgctgacgccaatattctgcaacaggtgcgtgaaaatctgccgctgatgccaggcttaacgcaactggtgctcaagctggaaacgctgggctggaaagtggcgattgcctccggcggctttactttctttgctgaatacctgcgcgacaagctgcgcctgaccgccgtggtagccaatgaactggagatcatggacggtaaatttaccggcaatgtgatcggcgacatcgtagacgcgcagtacaaagcgaaaactctgactcgcctcgcgcaggagtatgaaatcccgctggcgcagaccgtggcgattggcgatggagccaatgacctgccgatgatcaaagcggcagggctggggattgcctaccatgccaagccaaaagtgaatgaaaaggcggaagtcaccatccgtcacgctgacctgatgggggtattctgcatcctctcaggcagcctgaatcagaagtaattgctcgcccgccatcctgcgggcggcacagcattaacgaggtacaccgtggcaaaagctccaaaacgcgcctttgtttgtaatgaatgcggggccgattatccgcgctggcaggggcagtgcagtgcctgtcatgcctggaacaccatcaccgaggtgcgtcttgctgcgtcgccaatggtggcgcgtaacgagcgtctcagcggctatgccggtagcgccggggtggcaaaagtccagaaactctccgatatcagccttgaagagctgccgcgtttttccaccggatttaaagagttcgaccgcgtactaggcggcggcgtggtgccaggaagtgccattctgattggcggtaaccctggtgcggggaaatccacgctgctactgcaaacgctgtgcaaactggcccagcagatgaaaacgctgtatgtcaccggcgaagagtcgctgcaacaggtggcaatgcgcgctcatcgccttggcctgccgactgacaatctcaatatgttgtcggaaaccagcatcgaacagatctgcctgattgccgaagaagagcaaccgaagctgatggtaattgactcgatccaggtgatgcatatggcggatgtacagtcatcgcctggtagcgtggcgcaggtgcgtgaaacggcggcttatttgacacgcttcgccaaaacgcgcggtgtggcgattgtcatggtggggcacgtaaccaaagatggttcgctggctggcccgaaagtgctggaacactgtatcgactgttcggtgcttttggatggcgatgccgactcccgttttcgcaccttgcgcagccataaaaaccgcttcggcgcggtgaatgagctgggcgtcttcgcgatgaccgaacaggggctgcgtgaagtcagcaacccttcggcaattttcttaagtcgcggcgatgaagtgacctccggtagctcagtgatggtggtatgggaaggaacgcgtccactgctggtggagattcaggcgctggtcgatcactcgatgatggcgaacccacgccgcgtggcagtggggctggaacaaaaccgtctggcaatcctgctggctgtgttgcaccgtcacggtggtctgcaaatggccgatcaggatgtgtttgtgaacgtggtcggcggcgtgaaggtaaccgaaaccagtgccgacttagcgttactgctggcgatggtttccagcctgcgcgacagaccgctgccgcaggatctggtggtgtttggtgaagtcgggctggcaggggagatccgcccggtgcccagcggtcaggaacgaatctctgaagcggcgaaacacggttttcgccgggcgattgttccggcggctaacgtgccgaaaaaagcgccggaagggatgcagatttttggcgttaaaaaactctccgacgcgcttagcgtgttcgacgacttataatgagatatacggagggagatatgtcgtcatttgattacctgaaaactgccatcaagcaacagggctgcacgctacagcaggtagctgatgccagcggtatgaccaaagggtatttaagccagttactgaatgccaaaatcaaaagccccagcgcgcaaaagctggaggcgttgcaccgttttttggggcttgagtttccccggcagaagaaaacgatcggtgtcgtattcggtaagttctacccactgcataccggacatatctaccttatccagcgcgcctgtagccaggttgacgagctgcatatcattatgggttttgacgatacccgtgaccgcgcgttgttcgaagacagtgccatgtcgcagcagccgaccgtgccggatcgtctgcgttggttattgcaaacttttaaatatcagaaaaatattcgcattcatgctttcaacgaagagggcatggagccgtatccgcacggctgggatgtgtggagcaacggcatcaaaaagtttatggctgaaaaagggatccagccggatctgatctacacctcggaagaagccgatgcgccacagtatatggaacatctggggatcgagacggtgctggtcgatccgaaacgtacctttatgagtatcagcggtgcgcagatccgcgaaaacccgttccgctactgggaatatattcctaccgaagtgaagccgttttttgtgcgtaccgtggcgatccttggcggcgagtcgagcggtaaatccaccctggtaaacaaacttgccaatatcttcaacaccaccagtgcgtgggaatatggccgcgattatgtcttttcacacctcggcggtgatgagatcgcattgcagtattctgactacgataaaatcgcgctgggccacgctcaatacattgattttgcggtgaaatatgccaataaagtggcatttatcgataccgattttgtcaccactcaggcgttctgcaaaaagtacgaagggcgggaacatccgttcgtgcaggcgctgattgatgaataccgtttcgatctggtgatcctgctggagaacaacacgccgtgggtggcggatggtttacgcagcctcggcagttcggtggatcgcaaagagttccagaacttgctggtggagatgctcgaagagaacaatatcgaatttgtgcgggttgaagaggaagattacgacagtcgtttcctgcgctgcgtggaactggtgcgggagatgatgggggagcagagataaccgtgatgaaactgctcaaaggcgaggtataaaatgagtttttttgatgagttgaaaacctctctggaagaggctgtcgagattaaacaaggtttgaaaaaacctgcacgggtgacccgccacgaaattgaggatgctaaggctgttgtagaccggaaacggtgttcacgccgcatccggcattcggtgctcaatgcctgatgcgacgcttaccgcgtcttatcaggcctacagttttacaacgtattgaaattgctggttttgtaggccggataaggcgttcgcgccgcatccggcattttacgcattacttcgcaatacgcttgtacttgatacgcttcggctccagcgcgtctgcgcccagcgtgcgtttcttgtactcttcgtactcggtaaagttaccttcgaagaactcaactttaccttcatcctggtaatccagaatgtgcgtggcgatacggtcgaggaaccaacggtcgtgcgagataaccatcgcacagcccgggaactccagcagggcgttttccagcgcgcgcagggtttcgatatccaggtcgttggttggttcgtcgagcagcagcatgttgccgccaacctgcagcagcttcgccagatgcagacgaccgcgctcaccaccggagagttcaccaacgcgtttaccctgatcaacccctttaaagttaaagcggccaacgtaggcgcggcttggcatctcggtgttgccgatcttcatgatatccagcccgccggaaacttcttcccaaacggttttgctgttatccattgagtcacggaactgatcaaccgacgccagtttcaccgtttcacccaaagtgatggtgccgctgtccggctgttcctgaccagagatcatacggaacagggtcgatttacccgcaccgttcggaccgatgatcccgacgatcgctcctttcgggatcgagaagctcaggtcatcaatcagcagacgatcgccataggatttacgcaggttgctgacttccagcactttatcgcccagacgcggtccaggtggaataaacagttcgttggtttcgttacgtttctgatattcggtgctgttcagttcttcaaagcgcgccagacgtgctttacctttcgactgacggcctttagtaccttgacgtacccattccagctctttctcaatcgacttacgacgcgccgcttcttgtgaagcttcctgcgccaggcgctgatctttctgctccagccaggaggagtagttaccttcccacggaataccttcaccgcggtcaagttcgaggatccagcctgcaacgttatcgaggaagtaacggtcgtgggtaatcgccacaacggtgccttcgaagtcgtgcaggaagcgttccagccaggccacggattcggcatccaggtggttggtcggttcgtcgagcagcagcatgtctggtttttccagcagcaggcggcacaacgctacgcgacgacgttcaccaccggagaggttagcgattttcgcgtcccagtccggcagacgtagcgcatccgccgcacgctccagctgtacgttcagattatgaccgtcgtgagcctgaatgatctcttccagacggccttgttcagcggccagcttgtcaaaatcggcatccggatcggcgtacagcgcatacacttcatccaggcgtttcagggcgttaaccacttctgaaaccgcttcttcaatggactcacgcacggtgtgttccgggttcagctgcggttcctgcggcagataaccaatcttgatgtctggctgcggacgcgcttcaccttcgatgtctttatcaatgcccgccataatgcgcagcagggtggacttacccgcgccattcagacccaggacaccaatttttgccccagggaagaaactcagagagatgtttttcaaaatatgacgtttcggcggaacaactttgccgacacgatgcatggtataaacgaattgagccacgttggacttcgcctctatgtttatcgtgataatgagttttcaaaggcgaagtgtagcctttttccccgcctaatcccagccggtcgatcaccctcgcagtaaaagtaaaaaagtgtccgtaacgtggcgtaaacggcaatgactggttagcataaatctattacgcggcatgacgctgcattgatgtatttacacttagaggatgcgcttgtggaaaaagccaaacaagttacctggcggctgttggctgccggtgtctgtctgctgacggtcagcagcgtggcgcgagccgactcactggatgagcagcgtagtcgttacgcgcaaatcaagcaggcctgggataatcgacaaatggatgtggtcgaacaaatgatgcctggactgaaggattatccgctttatccctacctggaataccgccagatcaccgatgatctgatgaatcaaccggcggtgacggtcactaactttgttcgcgctaaccccacgcttcctcccgctcgcacgctgcaatctcgtttcgtcaatgaactggcgcggcgtgaagactggcgtggcttgttagcctttagcccggaaaagcccggaactaccgaagcgcaatgtaattactactatgcgaaatggaacaccgggcagagtgaagaagcctggcaaggggcgaaagagctgtggctaaccggcaagagccagcctaacgcctgtgacaagttatttagcgtctggcgtgcgtcaggtaaacaagatccgctggcgtatttagagcgtatccgtctggcgatgaaagcgggtaacacaggcctggtaacagtgctggcagggcagatgcctgccgattaccagactatcgcctcggcaatcatttcactggcgaacaaccctaatacggtactgaccttcgcgcgtacaactggcgcgaccgattttacccgtcaaatggcggcggtggcgtttgccagtgtggcgcggcaggatgctgagaatgcacggctgatgatcccatcgcttgcccaggcgcagcagcttaatgaagatcagattcaggagctgcgcgatatcgtcgcctggcgtttgatgggcaacgatgtcaccgacgagcaggcgaaatggcgcgatgacgccattatgcgctcgcaatctacttcgcttattgaacgccgtgtacgaatggcgcttggcaccggcgatcgtcgcggcctgaatacctggctggcgcgtctgcctatggaagcgaaagagaaagatgaatggcgttactggcaggcggatttattgctggaacgcggacgtgaagctgaagcaaaagagattttgcatcaactcatgcaacagcgtggtttctacccgatggttgcagcacaacgcatcggcgaagagtatgagctgaagattgataaagcgccgcagaatgttgacagcgccctgactcaggggccggagatggcgcgcgtgcgcgagttgatgtactggaatctcgataataccgcgcgtagcgagtgggccaatctggtgaagagcaagtcaaaaacagagcaggctcaactggcgcggtatgctttcaacaaccaatggtgggatcttagcgttcaggcaacgatcgccgggaagctgtgggatcatctggaagagcgattcccgctggcttacaacgatcttttcaaacgctacaccagcggtaaggagatcccgcaaagctatgcgatggcgattgctcgtcaggagagcgcctggaatccgaaagtgaaatcaccggtaggggccagcggcttgatgcagattatgcctggtacagcgacccatacggtgaagatgttctctattcccggttatagcagtcctgggcaattgctggatccggaaacgaatatcaacattggcaccagttacctgcaatatgtttatcagcagtttggcaataatcgtattttctcctcagcagcttataacgccggaccagggcgggtgcgaacctggcttggcaacagcgccgggcgtatcgacgcagtggcatttgtcgagagtattccattctccgagacgcgcggttatgtgaagaacgtgctggcttatgacgcttactaccgctatttcatgggggataaaccgacgttgatgagcgccacggaatggggacgtcgttactgatccgcacgtttatgatatgctatcgtactctttagcgagtacaaccgggggaggcattttgcttcccccgctaacaatggcgacatattatggcccaacaatcaccctattcagcagcgatggcagaacagcgtcaccaggagtggttacgttttgtcgacctgcttaagaatgcctaccaaaacgatctccatttaccgttgttaaacctgatgctgacgccagatgagcgcgaagcgttggggactcgcgtgcgtattgtcgaagagctgttgcgcggcgaaatgagccagcgtgagttaaaaaatgaactcggcgcaggcatcgcgacgattacgcgtggatctaacagcctgaaagccgcgcccgtcgagctgcgccagtggctggaagaggtgttgctgaaaagcgattgattttgtaggcctgataagacgtggcgcatcaggcatcgtgcaccgaatgccggatgcggcgtgaacgccttatccgtcctacaaatacccgtaatttcaatatgtttggtaggcatgataagacgcggcagcgtcgcatcaggcgcttaatacacggcattatgaaacggactcagcgccaggatcaccgcctggtgatagacgctggcgcgagtgagtttcccggcggtaaacacgccgatcgccccttccttacgaccaatctcatcaataccggtataacgcgacatcacgggaccaagcgcctcaccttcacgcactttttccagaatcaccgcaggcaacggcaaagtagccgaacgcgcctcgccgcgctggctggcgttttcaatcaccacccaactgaaagtgctgtcaccatcgatgccagcttcaatcgccacccaaaaatcagcctctggaagtaaacggcgggcattggctacccgatttcgtgcgccagcgcgcgtttcctcactgccaaagggctgttccggtacaccgctctcgacggcaacggatgcaatatggcaggatccttcgccgaagatctcgtgaaatgcctgcagaatggcctgaattttagcgggattggtggtcgcacagacaacttggtgcataatcagcattactcagaaaattaacgttacagcagtatacggaaaaaaagcatgttacaggtatacctagtccgccacggtgaaacgcagtggaacgccgagcgacgtattcagggccagtctgacagcccgctgaccgccaaaggtgagcaacaggcgatgcaggtggcaacccgtgccaaagagcttggcattacgcatatcatcagtagcgatttaggacgcacccggcgtacggcggaaatcatcgcccaggcctgcggctgtgacatcatctttgattctcgcctgcgtgaattaaacatgggtgtgctggaaaaaagacatatcgattctctgaccgaagaagaagagaactggcgtcggcagctggtcaatggcaccgttgacgggcgtattcctgaaggcgagtcaatgcaggagctcagcgatcgcgtcaatgcggcactggaatcttgccgggacttaccgcagggaagccgaccgctgctggtgagtcatggtattgcactgggatgcctggtgagtacgattctcggattaccagcatgggcagagcgccgcttacgtctgcgtaactgttctatttcgcgcgtggattatcaggaaagcctgtggctggcgtctggctgggtcgttgaaaccgcaggggacatctcgcatctggacgcccctgcattagatgagctgcagcgttaacgacggatcggaatcagcagttcacagcgtagattaattgggcgatctcccgctttggcatcttctgccgggtagtatcgctcaatatcctgacctttacggcgcgtcaggttgagcattggcatgcacgttccgtataccgtcaggataaactcctgcacgccggttcccagaccttcataggtaaacatcacatattcgccgccctgcagcatcaccggatgccccgtcagtacatagccatctgcctgatcctgggctaacgcggtggtatagaatacctcttgctcgtcgtctttatcctgactcggacgcgtttcattcaggccgtagagcaccggcggaatggtcggcgcgttgccgagaaaatcgtgccagaactgataacgcatttcatggcggaaatcagagatttgctccagcgaacaggagtagctctgggtaacaccaatcagcggcgtatcttccagggtgacaaatttgtgctctggcatagtgaattcacccaggcgtagcggcgggcgaataccaaaggcgctccattcaggagaacggcggtaaagtgcaggagtctgggcaaactgcttcttgaatgcgcgggtaaatgtctgttgagagtcgaagcggtattgcagcgcgatgtccagaatcggacgcgcagtcaggcgtagtgcgaccgccgatttcgacaaacgacgagcacgaatatacgcgccaatagcatggccagtgacatctttaaacattctctgtaagtgccacttggaataacctgctttcgccgctacattgtcgagcgacaggggctgatccagatgaccttccagccagattaaaaggtcgcgaataatgccggcctgatccataaaatatcctcatcctttcaacaacgagcacctgacatcaggtaattggataatagcattttttgctgttttagcattcagtgtttttttcttagtagagtatgttttagggcttgacggaaataaaagtattgagattttgttcttaatcaatatgttatttaccgtgacgaactaattgctcgtgtaatagataaaaatggtaacaatatgaaatacaagcatttgatcctgtctttaagcctgataatgctggggccattggctcatgcagaagagattggttcggtcgacaccgtatttaaaatgatcggcccggatcacaaaattgttgtggaagcctttgatgatcccgatgtgaaaaatgtcacctgttatgtgagccgggcgaaaaccggtggtattaaagggggattgggtctggcggaagatacctccgatgcggccatttcttgtcagcaagtcgggccgattgaactgtcggatcgtattaaaaacggcaaagctcagggcgaggtagtattcaaaaaacgcacgtccctggtctttaagtcgttacaggtcgtgcgcttttatgatgccaaacgcaacgcgctcgcttatctggcttactccgacaaagttgtagaaggttcgccgaaaaacgcgattagcgcggttcctgtcatgccgtggcggcaataacagaggcgatttatgcaacgggaaacggtctggttagtggaagatgagcaagggatagccgacacgctggtctacatgttgcagcaggaaggttttgccgtcgaggtctttgagcgaggcttgccggtgctggataaagctcgcaagcaggtacccgacgtcatgattctcgatgttggtctgccggatattagcggctttgaattgtgccgccagttactggcgctccatccggcgttacctgtactgttcctgacggcccgaagtgaagaggtcgatcgcctgcttgggctggaaattggtgctgacgactacgtggctaaaccgttttcaccccgcgaagtgtgcgccagggtgcgcaccttactgcgtcgggtgaagaagttctcgacgccgtctcccgtcatccgtattggacattttgaattgaatgaacccgcggcgcagatcagctggtttgacacgccattagcgctgactcggtatgagtttttattgttgaagacgttactcaagtcaccgggccgcgtctggtcccgccagcaactgatggatagcgtatgggaagatgcgcaggacacctacgatcgcaccgtcgatacccacattaaaacgctgcgtgccaagctgcgcgccatcaaccccgatctttcaccgattaatactcatcgcggcatgggatatagcctgaggggcctgtaatgcgtatcggcatgcggttgttgctgggctattttttactggtggcggtggcagcctggttcgtactggccatttttgtcaaagaagttaaaccgggcgtgcgaagagcaacggaggggacgttgatcgacaccgcaacgttgctggcggagctggcgcgtcccgatttgctctctggggacccaacgcatgggcaactggcgcaggcgtttaatcagctacaacatcgcccgtttcgcgccaatatcggtggcattaacaaagtgcgcaatgaatatcatgtctatatgaccgatgcgcagggcaaagtattgttcgattcggcaaataaagccgttggacaggattattcgcgctggaatgacgtctggctaacgttgcgtggtcagtatggtgcgcgcagcacgttgcaaaatcctgccgatcccgaaagttctgtgatgtatgttgccgcaccgattatggacggctcgcggcttattggcgttttgagcgtaggcaaaccgaacgcggcgatggctccggtcattaagcgtagcgagcggcgaattttatgggccagcgccattttgttggggattgcactggtgattggcgcaggcatggtttggtggatcaaccgctctattgcccggctcactcgctatgctgattccgtcactgacaataagcccgttcctctccccgatctcggtagtagcgagttgcgtaaactcgcgcaggcgctggaaagtatgcgcgtgaagctggaagggaaaaactatattgagcagtatgtttacgcattaactcatgagctaaaaagcccactggcggcgattcgtggagcggcggaaattttacgcgaaggtccgccgccggaagtggtggctcgttttactgacaacattctgacgcaaaatgcgcgtatgcaggcattggtagaaacgttactacgccaggcaagactggagaatcgtcaggaagtcgttctgactgctgttgatgtggcggcattattccgccgcgtcagcgaagcgcgcaccgtgcagttggcagaaaaaaaaatcactctgcatgttacgcccaccgaggttaacgttgctgctgaaccggcgttactggagcaggcgctgggaaatttactggataacgccatcgattttacccccgagagcggttgcatcacgctaagcgccgaagtggatcaggaacacgtcacgcttaaggtgctggataccggtagtggtattcctgactacgcgctttcacgtatttttgaacgcttttactctttgcctcgtgcaaatgggcaaaaaagcagcggtctggggttggcgttcgtcagtgaggtcgcccgtttgtttaacggcgaagtcacgctgcgcaacgtgcaggaaggtggcgtgctggcctcgcttcgacttcaccgtcacttcacatagcttcaaattcttcccacatagtcttcgtatcctgctgccattgcaaaggagaagactatgttgaaatcccccctgttctggaaaatgactagcctgtttggtgcagtattgctgttgttgattccgataatgctgattcggcaggtgattgtcgaacgtgctgattaccgtagcgatgtggaagatgcgattcgccaaagtaccagcgggccgcaaaaactcgttgggccgctcatcgctattcctgtgaccgagctttatacggtgcaggaagaggataaaaccgtggagcggaaacgaagttttatccatttttggttacctgagtcattgatggttgatggcaatcagaacgtggaagaacgcaagatagggatttataccggtcaggtctggcacagtgatttaacgttaaaagccgatttcgatgtttcgcgtcttagcgaactcaacgcgccaaatatcaccttaggcaagccatttattgtgattagcgtcggggatgcgcgtggtattggtgtggtgaaagcgcctgaagttaacggaacggcgctgaccattgaacccggcaccgggttagagcaaggcgggcagggcgtgcatatccctttacctgaaggggactggcggaagcagaacctgaagctgaatatggccctgaatttaagcggtaccggcgatctttctgtggtgcctggcgggcgtaatagcgaaatgaccttaaccagcaactggccgcatcccagttttttaggtgattttctaccagccaaacgggaagttagcgagtcaggttttcaggcgcactggcaaagcagctggtttgctaataatctcggtgagcgttttgcttcaggcaatgataccggctgggaaaacttcccggcgtttagcgtcgcagtaacgacgccagccgatcaataccaattaactgaccgggcgactaagtacgccattctgctgattgcactgacttttatggcgttctttgtttttgaaacgctcaccgcgcaacgtttacacccaatgcaatatttgctggtggggctttcattggtgatgttttatttgctcttgctggcgctttctgaacataccggttttaccgtggcatggataatcgccagtctgattggggcgataatgaacggtatttatttgcaagcggtattgaaaggttggtgcaacagcatgttgtttaccctcgcgctgttgttgctggatggtgtgatgtggggactgctcaactctgccgatagcgcgctgttgttgggaaccagtgtgctggtggtggcgctggccggcatgatgtttgtgacccgtaatatcgactggtatgcgttttcactgccgaaaatgaaagccagtaaagaagttacaacggacgatgagttacgtatctggaaataaggttgaaaaataaaaacggcgctaaaaagcgccgttttttttgacggtggtaaagccgattaatcttccagatcaccgcagaagcgataaccttcaccgtgaatggtggcgatgatttccggcgtatccggcgtagattcgaaatgtttacgaatacggcggatcgtcacgtctacagtacggtcgtgcggtttcagctcacggccggtcattttcttcagcagttcagcacgggactgaattttgcctgggttttcacagaagtgaagcatggcgcggaactcgctgcgcggcagcttgtactgctcgccatcagggccgatcaacgaacggctgttgatgtccagttcccaaccattgaacttgtagctttcaacgctacgacgttcttcgctgacagtacccagattcatggtacgggacagtaggttgcgtgcacgaatcgtcagttcacgcgggttgaacggtttggtgatgtagtcatctgcaccgatttcgaggccgagaattttatcgacttcgttgtcacggccagtcaggaacatcaacgcaacattcgcctgctcgcgcagttcacgcgctaacagaagaccgttcttacccggcagattgatatccatgatcaccaggttgatgtcatattcagagaggatctgatgcatttccgcgccatctgtcgcttcgaaaacatcatagccttccgcttcgaaaatacttttcaacgtgttgcgtgttaccaactcgtcttcaacgataagaatgtgcggggtctgcatgtttgctacctaaattgccaactaaatcgaaacaggaagtacaaaagtccctgacctgcctgatgcatgctgcaaattaacatgatcggcgtaacatgactaaagtacgtaattgcgttcttgatgcactttccatcaacgtcaacaacatcattagcttggtcgtgggtactttccctcaggacccgacagtgtcaaaaacggctgtcatcctaaccattttaacagcaacataacaggctaagaggggccggacacccaataaaactacgcttcgttgacatatatcaagttcaattgtagcacgttaacagtttgatgaaatcatcgtatctaaatgctagctttcgtcacattattttaataatccaactagttgcatcatacaactaataaacgtggtgaatccaattgtcgagatttattttttataaaattatcctaagtaaacagaaggatatgtagcattttttaacaactcaaccgttagtacagtcaggaaatagtttagccttttttaagctaagtaaagggctttttctgcgacttacgttaagaatttgtaaattcgcaccgcgtaataagttgacagtgatcacccggttcgcggttatttgatcaagaagagtggcaatatgcgtataacgattattctggtcgcacccgccagagcagaaaatattggggcagcggcgcgggcaatgaaaacgatggggtttagcgatctgcggattgtcgatagtcaggcacacctggagccagccacccgctgggtcgcacatggatctggtgatattattgataatattaaagttttcccgacattggctgaatcgttacacgatgtcgatttcactgtcgccaccactgcgcgcagtcgggcgaaatatcattactacgccacgccagttgaactggtgccgctgttagaggaaaaatcttcatggatgagccatgccgcgctggtgtttggtcgcgaagattccgggttgactaacgaagagttagcgttggctgacgttcttactggtgtgccgatggtggcggattatccttcgctcaatctggggcaggcggtgatggtctattgctatcaattagcaacattaatacaacaaccggcgaaaagtgatgcaacggcagaccaacatcaactgcaagctttacgcgaacgagccatgacattgctgacgactctggcagtggcagatgacataaaactggtcgactggttacaacaacgcctggggcttttagagcaacgagacacggcaatgttgcaccgtttgctgcatgatattgaaaaaaatatcaccaaataaaaaacgccttagtaagtatttttc
